European Patent Application EP 4 722 372 A2, published April 8, 2026. Title: PLANTAS COM CARACTERÍSTICAS AGRONÔMICAS APRIMORADAS MEDIANTE SUPRESSÂO DE GENES DA REDE REGULATÓRIA AIP10/ABAP1. Applicant: HAPISEEDS PESQUISA E DESENVOLVIMENTO LTDA. The sequence listing filed with the application follows.

SEQUENCE LISTING (263 sequences)

SEQ ID NO: 1 - DNA, 1705 bp, Arabidopsis thaliana
  source 1..1705: mol_type = genomic DNA
aaaaaaaaacagtttagaaaaggattaaagatgaattcataaaaaaataaagaaggttaaaggttgcatgaaaatttagcaaaggaataaagagggaaaaggtcccaacctaaagaatacgataagacaactattttcgacttctgattttttttctttttgtaagaataaaaaacattttcacaagcctctgtagctgaagcacaaagcaaaagcatttggtagtcgtaaccaaaacgccaaatcattaccgttcaactgaaatctaacagagagccctcttttcttgggaattcgattccttgtacgttatcttcttcttcttcttctctttctcaaaattcgtgtatcttctgggaaattttcagatttagatggagaaaggggttggatttgagaaagacatgaagacagtcagtgatgggtttgtcggaggttttttccctgtctctaccaccaagatcgcgtggaaatcaagaaaaagatcaggttttttccactgtttcttgttttctcagaccattaaagattctagacctttattagctaccctttctatttctggtctgaaagatttggaattttttttaagcatcaattgttttagctctatgtgaactatttcctcgagatctagacatggagctttagtcttcttctctctgtcttaagcttgtaaaatcaaagactttgtaactttcgttttgatctgatccgtttgcatgtgattttggaactcaaagcattaactattttgatcgcagcattgttgaacctagacaaagcaccggaggctgttacggaggtcacaccagagaagaacgagataacagcaatggataccgagaaagttggggaaccaatgaccacaactcctcttctgtccgagaaaaggaaagctctgttcgagccacttgaacccattacgaacttgaacggaaagcgaccaactgcggctgattcattgttgccaccgccggatttcgagactgcaaactacccaaaaggctggttgatcggtaagaagaggaagcttgtgaatgttgatgtagttgagagcatgcgtagaatagctgtccaagaaatgaacagaaaggtaaaacaaactaaacatgatgcagatttttgctggagtttgatttacggattgtgggattgtgacaggatcgagagatagatgggttaaacgagcagctagaagaggattcacggtgcttagagcatctacagcttcagctgctacaagagagaagcaagagaacagagattgaaagagagaacacaatgttgaaagagcaagttgatatgcttgtgaacatgatacaagaagatgacgaagaaggagctgaagaaccctaagctagttctcatcaaatttatgtctcacctataatagctgtgttctgttttttttattcttttgtagatttgtctcgtccacaaaaaagaagaaaagaaagaagcttaaccatctattatttggttaagctactcttgttcccttgtgtgatagaacaaaacataatcaagaacattatatattctaagttatgagttctcctgcaagatttgaacctggcatttgattgaatcgattatgttcattgaagctcttaggaggaaaaagaaccatttggtgtgtgtgtgtgtgtgtgtatctttcttcagcaagaaacagaggcaaaataaatacaagtttcagaaa

SEQ ID NO: 2 - protein, 213 aa, Arabidopsis thaliana
MEKGVGFEKDMKTVSDGFVGGFFPVSTTKIAWKSRKRSALLNLDKAPEAVTEVTPEKNEITAMDTEKVGEPMTTTPLLSEKRKALFEPLEPITNLNGKRPTAADSLLPPPDFETANYPKGWLIGKKRKLVNVDVVESMRRIAVQEMNRKDREIDGLNEQLEEDSRCLEHLQLQLLQERSKRTEIERENTMLKEQVDMLVNMIQEDDEEGAEEP

SEQ ID NO: 3 - protein, 175 aa, Arabidopsis thaliana
MEKGVGFEKDMKTVSDGFVGGFFPVSTTKIAWKSRKRSALLNLDKAPEAVTEVTPEKNEITAMDTEKVGEPMTTTPLLSEKRKALFEPLEPITNLNGKRPTAADSLLPPPDFETANYPKGWLIGKKRKLVNVDVVESMRRIAVQEMNRKVKQTKHDADFCWSLIYGLWDCDRIER

SEQ ID NO: 4 - protein, 151 aa, Arabidopsis thaliana
MDTEKVGEPMTTTPLLSEKRKALFEPLEPITNLNGKRPTAADSLLPPPDFETANYPKGWLIGKKRKLVNVDVVESMRRIAVQEMNRKDREIDGLNEQLEEDSRCLEHLQLQLLQERSKRTEIERENTMLKEQVDMLVNMIQEDDEEGAEEP

SEQ ID NO: 5 - protein, 158 aa, Arabidopsis thaliana
MEKGVGFEKDMKTVSDGFVGGFFPVSTTKIAWKSRKRSALLNLDKAPEAVTEVTPEKNEITAMDTEKVGEPMTTTPLLSEKRKALFEPLEPITNLNGKRPTAADSLLPPPDFETANYPKGWLIGSRDRWVKRAARRGFTVLRASTASAATREKQENRD

SEQ ID NO: 6 - DNA, 4134 bp, Arabidopsis thaliana
  source 1..4134: mol_type = genomic DNA
atgataatctcaaaatcgttcaaagcaccgctcaaattctccgtcaaatcttctactgcgccggtgatatcaaaccatccgccaatggagaaccatcccaagcgccagcgaacaacacgcctcgccgccagaaacttgaagcgaaaactcagtcacaacacagatggagcgccaatcgtcacacaacttattgatattgacgacgaacccatagatctcgtcgtcgcgattcgccgtcacgtcgaggttcttaactccagcttctcagatcctgattttgatcacgaagctgtcaaagaagctgctgctgatatcgccgatttggctaaaatcggtaccgtacttcttcattttacctctaatcggcggctaaaactgaaaacgtgttactctctttgcttgttcgtccttgagttgctcaattttgagtcaattctcgacaacggattcactctaattttggattctacatagaaattgttttgttcttgcccatagtactttgattttcagtaaggcgagacctagaagtgtttttttttggcttaattgattttctcatctgtttatatagatgaaaatgttgaaatcatcgtggaaaatggagcgatccctgctttggtgagatatctggaatcccctttggtagtttgtggcaatgttcccaaatcttgcgagcacaagctagagaaagattgtgctcttgctcttggacttattgctgcgattcaggtaacccttctttcgctgtttttgatgaaattgtggatgagatgttgtgtaatttcaatctctgttggaagttaacattagaatttttgaaatgggcgatttgcaactatcttagatgtacttagcttggattgatgtatattgatattagctttctctgttaaatagcctggttaccagcagcttattgtggatgctggagccatagttcccaccgtgaagttgttgaagagacgtggggaatgtggtgaatgcatgtttgctaatgctgttattaggagagccgctgatataattactaacattgctcatgacaatccaaggattaaaacaaatataaggtactaatatctcatgatccttactggttatggtgatgactagctgttttcacttgacaccttttaaaaatgctttacagggttgaaggtggcattgcaccacttgttgagcttctcaattttccggatgttaaagtacagagggctgcggcaggggccttgcgaacagtttcatttagaaacgacgagaacaagagtcaagtatgtttttactatgattatgttttgtttaggcttatgaaaggcatgattctcacataatgcgcaactatgtagattgtggagttgaatgctttacccacacttgtattgatgcttcaatcacaagattctaccgttcacggggaagcggttagttcttcatcttgctttagatcgttgcaattggtttgatttgttcagttctttctaatgtactatggactttcagattggggcaattggaaatcttgtccactcatctcctgacatcaagaaagaggttatccgtgctggtgccttacaaccagtaattggtctacttaggtatgcttattttactttctttctacttctgctggaacagatgctagctcttgaaattttgaattatgttttgtaactgtttttcatgatatctgctacagctccacttgtttggaaacacagagagaagcagcattattaataggtcaatttgctgcgcctgattcagattgcaaggtatgggattgtctctttcttgttgtactataatattagcacatgttatgttcactcaaactcgtttttttctacgatataactgaatggattctaactagagagaacatatttaacataactggcaacatgatcatgcaggtgcacattgcccagagaggtgccattacaccactgattaagatgcttgaatcatcagatgagcaggtcgtggaaatgtcagcttttgctcttggtcgtttggctcaggtatatatgtttttgaattagcatgtgaatgttttgttgcttttaatatctgactctttgtagatgattgttaaatcagaccttttgtgataaaacaaaaattgtatgttttgaatgttgcaggacgcacacaatcaagctggcattgcacatagaggaggcatcatctcactactaaatcttcttgatgtgaaaacggggtctgtgcaacacaatgctgcctttgctttgtatggccttgcagataacgaggtaaactcgactcgcaatgaatagtattatatgtagctatactctttgcttacttgacataccgtgagtacttaattaattttcccgtcaataggaaaacgtagcagatttcataaaggctggaggtattcaaaagcttcaagatgacaactttactgtccaagtatgcatttgactgcttatatttgcaaaaccaatctaataagaatttcaaactttaattgtaagtaatctatttgcagccgactagagattgtgtggttcggacattgaagaggctgcagaacaagattcacggacctgtgagtacctacttctgttagaacttctgggtctcaattatgttttgcgatgtttctaatcccctgatgtctcaaccttcttaggtactaaaccaattattgtacctaatgagaaccgctgagaagacagtacaaatacgaattgctctggctcttgcacatctttgtgaccctaaagatggaaaattaatctttattgataacaatggtaagcatctcatatattcagaatttcattttctaataaaattttctgtggttttttgtttctgatctattgaagtattacttatgcaggagtagagtttttgttggaacttctctatttctcaagcaataagcagcagagatatagttcaagtgctttatacgagttagctaaaaaagctacatcctttgcaccagaggattcagctccttgttcacccacacaacaggtaaaaaaatctccatttcttctttcaagcatcaaataatttgtgatttgaggtcttgacttgttgttattgattattatactgaaggtgtttctgggtgaaaaattcgtgaacaaccccactatgtccgatgtcacattcctaattgatggtataacatttaaccccatttatgattctatagaatccaccggtgagaacattctttaatgagtatatccatgtcctatgttaggtaaacaattctatgcacacaagattggcttggtagcttcctctgatatatttcgtgcaatgtttgatggtctttacaaggtaagctactgaatcacgattgtggtaacttatctcatcagaatatcatctaactaactttgagaactggatataggaacgcaatgctcaaaatgtggagataccaaatataagatgggaagtgtttgagcttatgatgaagttcatttactcaggaagaattaacatcgccaaacatttggcaaaagatctgcttgtagcagctgatcaatatcttctcgaaggtctcaaacgtcaatgtgaatacaccattgcacaggtaacaaacgtaaaaccaaggtcttaatttttctgcacagaaggactaatctctcttgtgtgtttttaataagatggactttacttgtgcaggaaatctgtctggataacataccagagatgtatgagttagcagatacattcaatgcttcagccttaagaagagcttgcacgctctttgttcttgagcatttcactaagctcagctctcaattatggtatgcaaaatcattacatcgttataatttttttgggaaatttaacttctatttcactcatcaagtttcgattgatttacctaatgcaggtttgcaaagtttgtcaagcaaattatacctgaaattcggagttacatgactgatattctcacacggccggtcgaagctagtcccccaaccgtcgtataaaacatataggattccggtttgaagtagttgatttactttacttaggtaaaattgtttttcttttgataaccggtctgtattttgttactgctatatctctaatataaactgcttaactcaataataccaaagaggctct

SEQ ID NO: 7 - protein, 737 aa, Arabidopsis thaliana
MIISKSFKAPLKFSVKSSTAPVISNHPPMENHPKRQRTTRLAARNLKRKLSHNTDGAPIVTQLIDIDDEPIDLVVAIRRHVEVLNSSFSDPDFDHEAVKEAAADIADLAKIDENVEIIVENGAIPALVRYLESPLVVCGNVPKSCEHKLEKDCALALGLIAAIQPGYQQLIVDAGAIVPTVKLLKRRGECGECMFANAVIRRAADIITNIAHDNPRIKTNIRVEGGIAPLVELLNFPDVKVQRAAAGALRTVSFRNDENKSQIVELNALPTLVLMLQSQDSTVHGEAIGAIGNLVHSSPDIKKEVIRAGALQPVIGLLSSTCLETQREAALLIGQFAAPDSDCKVHIAQRGAITPLIKMLESSDEQVVEMSAFALGRLAQDAHNQAGIAHRGGIISLLNLLDVKTGSVQHNAAFALYGLADNEENVADFIKAGGIQKLQDDNFTVQPTRDCVVRTLKRLQNKIHGPVLNQLLYLMRTAEKTVQIRIALALAHLCDPKDGKLIFIDNNGVEFLLELLYFSSNKQQRYSSSALYELAKKATSFAPEDSAPCSPTQQVFLGEKFVNNPTMSDVTFLIDGKQFYAHKIGLVASSDIFRAMFDGLYKERNAQNVEIPNIRWEVFELMMKFIYSGRINIAKHLAKDLLVAADQYLLEGLKRQCEYTIAQEICLDNIPEMYELADTFNASALRRACTLFVLEHFTKLSSQLWFAKFVKQIIPEIRSYMTDILTRPVEASPPTVV

SEQ ID NO: 8 - DNA, 3341 bp, Sorghum bicolor
  source 1..3341: mol_type = genomic DNA
agtacgccgtttccgccatcgttaggcgttacgtccctgaaaggaaaacccaagccaacgatgaccacgacgacagggccaagaaacggggagtgtattccaaggcgaccaccgcccccctctcgcactccaaacagcacacgtccatccgtcagcccagagccacaagataacgcaaccaacaagacacagcgagcgagcgagcgaggagaagggagtagcgcgcgcggcgcagcgcggcaaccaggtccaggagaaagggaagcccagttagcctggagccgagaagccgccgaggtgagattttgattgacatggttagctcacggaggcctggaagcgaggaggaatttgaggcggaagaagcagagatttattagcacagctggaagctgatgggtgcaattcgttttgtgctgtagggagcgagggagcagccaggcatggaggagcccgttccggctgatccccccaggattttctggaagtcaaggagatcaggtgcctgctgttctcaatcaattcctgttcctgcaacctgcatacaaaatctcactgatttcaagtgcctattttttttacccccgcaagaatcgtcttctcatcatgtctcatcgtctatttctctgttcttggaagatggccaatttcagctcagttttcttcaaatttctctgtaattctgctcaaaagaaagtaatacagttcatataaaagcaatataattagattaacatctaaacactattaatctcagctactttgtttccctccacaagcaccgtggtttttttctctcgaccggaacattttcctttttgttcatataagttctggtactgatgcccgggactgtgccggtgagatatttcgtgtggggggatgaatgatagacagctcactcgcgtgacgtaccggtagtccagtactagttaacaattaacatagcacgttaatcacgcatccgtggtacttaacttttattggataacctcccgtttggtagttcgatcacgtgagcgtagctggtcatttcaataccttgtcaagttgtcagctaccagaatagcagacgtctttgcttgtcttcaaggctaatcccaagcctgcagctgcggtgtggtgcttagtaacagtggtcccaggaatatgcttgcagcaagaaatcatattcctagataccctttgcagcaaagagtaatttctaatcttgctaccgtgggattagatttctgtgtgttttcttgtctgtttctgcctttccaatattttcctctctttgccgctgttcagacgaagccaaagactagtatgcaaccggtgtagcatcctagagtttcttggtgtggcagcagacaagtatgaacaattctaaccgagtagccgtctaggcatggtcaagtatggaacaaacagataaactacaatctagtcgtatatgagtattttgtagcatatgtccagagggcagtattgtcgtgtctcgtgtgggtcagattatgtatggctcatgtgggctggcttattggaatgctaatcaggtcaatctgatgctacatctggttgatactgaccaatatgtgacgctgacagattagtttagggcaaaataaatcaaccttggaaattactctctagcagacataaaaacaatgtatcagtcttggaatgcagaaattttgcccttaagggaacatgctcttgctactgtgagccacatgtttgacactgagattcatgcccacgagagagatactagaatattgtctctctcctgctggtgctgtgcacgaatcacagtgcgaaacttgtggctcacaacatcagagcttgtgctctttgggcaaattttactttctcatcagccttctttttagagcttatggtattgttcatgaatagatctttatgttcaatacagtgtgttatttcggtcccttattactttacttctttgtgaaggatggtacatatacatatagcatacttgcaagacactgaaggcctgtgaagaattaaagaagcctcacaaaagaatgaaagcaagagctataaaaatatttctaagaaatgaataaaagcatcccctagactctgcataagctattcacatgacagccaaactcatcctcacaactcactaacatattggttgtcaaaatgaatgaacttccaactgatcatattgtatagagcgaatggtcatgtgtgcattagattttaactggggaagtgcactgactcttgatctgactaacaatatgtatgttccagccaatggccggagcttgcaacaagaacctgacaaagatgctaccgaagaaactaatgagcaggctcaagaggaacccatgaagaccgacgatgcaacagatacaacagctacagctgaggatgtacaaccagacccaaaagctaacttatctgagaagcggaaggctctctttgagcctcttgagccgatcaatggaaagcgcagtgctgaaatgctgcttccaccaccggactttgagcccgcatcatatcctaagggatggctggtgggcaagaaacgtaagctcgtcaatgtagatgttgtggagagcatgaggaggattgcaatccaagaaatgaacagaaaggtttataatctttctagtggtctgattctacatacctgcatgatatcaatgcggcatgcaatgctatttttctagtaaatgcatcgatgatcaagctgaaaatcctgaaacgatggcttctgcttttatctgcgataagagtatcatgcttgtgtgctgcctaaggtaaactgtaggcaattttgttgctgaacgtgcatcaaagactgacaattgttattactgtggaaacggtgtggcaggaccgtgagatcaatggactgaacgagcagttagaggaagactcccgtgtgctggagcttctacagaagcagcttgccgatgagcgcaagaagcgggcagagattgagaaggaaaattctatgcttcatgagcaggtgaacatgctgatgaacatgcttgacgaaaatgagggtttcgatgaggacggagaagctccaccgcccgattcctttgattaagcattacattactatccattttccaacaatatcaagtcatacatctctaggtaccggtttcagagtatccaagggatatatgctgtgtagaatttcatttatcgtattccattacatggcttgtgtttctgtagataaagagtgcatgtctgttgcaccaactcctttctaggcttcaaatgtatgtgagaaactagtaacatattatatttgaatcgaagtgtatgtacatgttatatgaaattcttccttgctatgc

SEQ ID NO: 9 - protein, 207 aa, Sorghum bicolor
MEEPVPADPPRIFWKSRRSANGRSLQQEPDKDATEETNEQAQEEPMKTDDATDTTATAEDVQPDPKANLSEKRKALFEPLEPINGKRSAEMLLPPPDFEPASYPKGWLVGKKRKLVNVDVVESMRRIAIQEMNRKDREINGLNEQLEEDSRVLELLQKQLADERKKRAEIEKENSMLHEQVNMLMNMLDENEGFDEDGEAPPPDSFD

SEQ ID NO: 10 - DNA, 3123 bp, Saccharum spontaneum
  source 1..3123: mol_type = genomic DNA
atgcatgccccgcccccgatccgtcgtcggttgacgggagaagtacgccgtttccgccatcgttacgtccctcagaagcaaaaaccaagccaacgacgaccaggacgacacggccaagaaacgggagcgtcttccaaggcgaccgcctcttgcactccaaacagcacacatccatccgtcagcccagagccacaagataacgcaaccaacaagacacagcgagcgagagggcggggagaaaagagtagagcgcgtggcgcggcaaccaggtccaggagaaaggaagcccagctagcctggagccaagaagccgaggtgagattttgattgacatggttgctcacggaggcctggaagcgaggaggaattcgagccttcgaggcggaggaagcagagatttagcagctggaagctgatgcgtgcaatttgttttgtgctgctgctgcagggagagagggagcagccaggcatggaggatcccgttccggctgacccccccaggattttctggaagtcaaggagatcaggtgcctgctgtctcaattcctgttcctgcatacaaaatctcgctgatttcaagtgcttttttttgccccccagaatcgtcttctcgtgacttaaccatccttatctatttctctgttcttgaaaaatggctaatttcagctcagttctctgcaaattcctctgtaattctgcccaaaagaaagtaatacagacatacagttcatacagcaatctatttagattcacacctaagcactattaatctcagctactttgtttccctccacaagcaccggtttttttcctcgaccagaacattttcctttttgttcatataagttttggtactgatgcccgggaatgtgccggtgggatatttcgtgtggggatgaatgatagccagctcactcgcgtgacgtaccggtagtccagtactagttaacaattaacatagcacgttaatcacgcacccgtgctacttaactgctgttgataactaacagcccatttggtggttcacgtgagagtagctggtcattttaatcccttgtcagctacaagaagcagagcagacgtcaacgtctttgcttgtcttcaccgctaagatgtaagatcccaaacctgcggctgccggtgttgtgcttagtaacagtggtctcaggaatatgcttgcagcaagaaatcatattcctagacaccctttgcagcaagagtaatttctaattttgctaccgtggaattagatttctttgtgttttcgtgtctgtttctgcctttccattattttcccctctttgccactgttcagacgaggccaaagactagtatgccgctgttcagacgaggccaaagacaagtatgaacaattctaaccgagtaggcatggtcaagtatggaacaaacagataaactacaatctagtcgtatatgagtattttatagcatatgtccagacggcggtatggtcgtgtctcatgtgggtcagattatgtagcgctcgtgtgggccggcttattggaatgctaatcaggtcaatctgatgctacatctggttgatactgaccaatatgtgacgctgacagattagtttagggcaaaataaatcagccttggaaattactctctgacagacataaaaacaatgtatcagccttcttttcagagcttatggtattgttcatgaatagatctttatgttcaatacagtgtgttatttcggtcccttgttacttttacttctatgtgaaggatggtacatatacatatagcatacttgcaagacactgaagggctgtaaagaattaaagaagccgcacaaaagaatgaaagcaggggctataaaaatattcctaagaaatgaataaaagcatcccctggactctccataagctaatcacatgacagccatactcatcctcacaactcactaacatattggttgtcaaagtgaatgaacttccaactgatcatattgtagagcgaatggtcatgtgtgcattagattttaactggggaagtgcactgactcttgatctgactaacaatatgtatgttccagccaatggccggagcttgcaacaagaacctgacaaagatgctaccgaagaaactaatgagcaggctcaagaggaacccatgaagaccgacgatgcaacagatacaacagctacagctgaggatgtacaaccagacccaaaagctaacttatctgagaagcggaaggctctctttgagcctcttgagccgatcaacggaaagcgcagtgctgaaatgctgcttccaccaccggactttgagcccgcatcatatcctaagggatggctggtgggcaagaaacgcaagctcgtcaatgtagatgttgtggagagcatgaggaggattgcaatccaagaaatgaacagaaaggtttataatctttctagtggtctgattctacatacctgcatgatatcatgcggcatgcaatgttatttttctagtaaatgcatcgatgatcaagctgaaaatcctgaaatgttggcttctgcttttatctgcaataagagtatcatacttgtgtgccgcctaaggtaaactgtaggcaattttgttgctgaacacgcatcaaagactgacaattgttattaatgtggtaacggtgtggcaggaccgtgagatcaatggactgaatgagcagttagaggaagactcccgtgtgctggagcttctacagaagcagcttgccgatgagcgcaagaagcgggcagagattgagaaggaaaattctatgcttcatgagcaggtgaccatgctgatgaacatgcttgacgaaaatgagggtttcgatgaggatggagaagctccaccgcccgattcctttgattaagcattacattactatccgttttccatcaatatcaaatcatacatctctaggtaccggtttcagagtatccaagagatatatgctgtgtagaatttcatttatcgtattccattgcatggcttgttttatgtagataaagggtgcatgtctgtttcaccaactcctttctaggcttcaaatgtatgtgagaaactagcaacatattatatttgaatcgaagtgtatgtacatattatatgaaattcttcctt

SEQ ID NO: 11 - DNA, 3102 bp, Saccharum spontaneum
  source 1..3102: mol_type = genomic DNA
gccggtaatggatgccccgcccccgatccgtcgtcggttgacgggagaagtacgccgtttccgccatcgttacgtccctcagaagcaaaagccaagccaacgacgaccaggacgacacggccaagaaacgggagggtcttccaaggcgaccgccccctctcgcactccaaacagcacacatccatccgtcagcccagagccacaagataacgcaaccaagacaagcagacagagtagagcgcgtggcgcggcaaccaggtccacgagaaaggaagcccagctagcctggagccaagaagccgaggtgagattttgattgacatggttgctcacggaggcctggaagcgaggaggaattcgagccttcgaggcggaggaagcagagatttagcagctggaagctgatgcgtgcaatttgttttgtgctgctgctgcagggagcgagggagcagccaggcatggaggatcccgttccggctgatccccccaggattttctggaagtcaaggagatcaggtgcctgctgtctcaattcctgttcctgcatacaaaatctcgctgatttcaagtgctttttttttgccccccagaatcgtcttctcgtgacttacccatccttatctatttctctgttcttgaaaaatggctatttcagctcagttctctccaaatttctctgtaattctgcccaaaagaaagtaatacagacatacagttcatacagcaatataattagattcacacctaagcactattaatctcagctactttgtttccctccacaagcaccggttttttttttcctcgaccagaacattttcctttttgttcatataagttttggtactgatgcccgggaatgtgccggtgggatatttcgtgtggggatgaatgatagccagctcactcgcgtgacgtaccggtagtccagtactagttaacaattaacatagcacgttaatcacgcacccgtgctacttaactgctgttgataactaacagcccatttggtggttcacgtgagagtagctggtcattttaatcccttgtcagctacaagaagcagagcagacgtcaacgtctttgcttgtcttcaccgctaagatgtaagatcccaaacctgcggctgccggtgttgtgcttagtaacagtggtctcaggaatatgcttgcagcaagaaatcatattcctagacaccctttgcagcaagagtaatttctaattttgctaccgtggaattagatttctttgtgttttcttgtctatttctgcctttccattattttcccctcttttgccgctgttcagacgaggccaaagactagtatgccgctgttcagacgaggccaaagacaagtatgaacaattctaaccgaatagtcgtctaggcatgatcaagtatggaacaaacagataaacaacaatctagtcgtatatgagtattttgtagcatatgtccagacgacggtatggtcgtgtctcatgtgggtcagattatgtagcgctcgtgtgggccggcttattggaatgctaatcaggtcaatctgatgctacatctggttgatactgaccaatatgtgacgctgacagattagtttagggcaaaataaatcagccttggaaattactctctgacagacataaaaacaatgtatcagtcttcttttcagagcttatggtattgttcatgaatagatctttatgttcaatacagtgtgttatttcggtcccttgttacttttacttctatgtgaaggatggtacatatacatatagcatacttgcaagacactgaagggctgtaaagaattaaagaagccgcccaaaagaatgaaagcaggggctataaaaatattcctaagaaatgaataaaagcatcccctggactctccataagctaatcacatgacagccatactcatcctcacaactcactaacatattggttggcaaagtgaatgaacttccaactgatcatattgtagagcgaatggtcatgtgtgcattagattttaactggggaagtgcactgactcttgatctgactaacaatatgtatgttccagccaatggccggagcttgcaacaagaacctgacaaagatgctaccgaagaaactaatgagcaggctcaagaggaacccatgaagaccgacgatgcaacagatacaacagctacagctgaggatgtacaaccagacccaaaagctaacttatctgacaagcggaaggctctctttgagcctcttgagccgatcaacggaaagcgcagtgctgaaatgctgcttccaccaccggactttgagcccgcatcatatcctaagggatggctggtgggcaagaaacgcaagctcgtcaatgtagatgttgtggagagcatgaggaggattgcaatccaagaaatgaacagaaaggtttataatctttctagtggtctgattctacatacctgcatgatatcatgcggcatgcaatgttatttttctagtaaatgcatcgatgatcaagctgacaatcctgaaatgttggcttctgcttttatctgcaataagagtatcatgcttgtgtgccacctaaggtaaactgtagtcaattttgttgctgaacgtgcatcaaagactgacaattgttattactgtggtaacggtgtggcaggaccgtgagatcaatggactgaacgagcagttagaggaagactcccgtgtgctggagcttctacagaagcagcttgccgatgagcgcaagaagcgggcagagattgagaaggaaaattctatgcttcatgagcaggtgaccatgctgatgaacatgcttgacgaaaatgagggtttcgatgaggatggagaagctccaccgcccgattcctttgattaagcattacattactatccattttccatcaatatcaaatcatacatctctaggtaccggtttcagagtatccaagagatatatgctgtgtagaatttcatttatcgtattccattgcatggcttgttttctgtagataaaggatgcatgtctgttgcaccaactcctttctaggcttcaaatgtatgtgagaaactagcaacatattatatttgaatcgaagtgtatgtac

SEQ ID NO: 12 - protein, 319 aa, Saccharum spontaneum
MHAPPPIRRRLTGEVRRFRHRYVPQKQKPSQRRPGRHGQETGASSKATASCTPNSTHPSVSPEPQDNATNKTQRARGRGEKSRARGAATRSRRKEAQLAWSQEAEGEREQPGMEDPVPADPPRIFWKSRRSANGRSLQQEPDKDATEETNEQAQEEPMKTDDATDTTATAEDVQPDPKANLSEKRKALFEPLEPINGKRSAEMLLPPPDFEPASYPKGWLVGKKRKLVNVDVVESMRRIAIQEMNRKDREINGLNEQLEEDSRVLELLQKQLADERKKRAEIEKENSMLHEQVTMLMNMLDENEGFDEDGEAPPPDSFD

SEQ ID NO: 13 - protein, 313 aa, Saccharum spontaneum
MDAPPPIRRRLTGEVRRFRHRYVPQKQKPSQRRPGRHGQETGGSSKATAPSRTPNSTHPSVSPEPQDNATKTSRQSRARGAATRSTRKEAQLAWSQEAEGAREQPGMEDPVPADPPRIFWKSRRSANGRSLQQEPDKDATEETNEQAQEEPMKTDDATDTTATAEDVQPDPKANLSDKRKALFEPLEPINGKRSAEMLLPPPDFEPASYPKGWLVGKKRKLVNVDVVESMRRIAIQEMNRKDREINGLNEQLEEDSRVLELLQKQLADERKKRAEIEKENSMLHEQVTMLMNMLDENEGFDEDGEAPPPDSFD

SEQ ID NO: 14 - DNA, 3030 bp, Zea mays
  source 1..3030: mol_type = genomic DNA
gtacgccgtttgcgccatcgttacgtccaccagaaggaaaacccaagccaacgacgacggcacggccaagaaacggggagtgccttccaaggcgaccgccccctctcgcgctccatacgtccatccgtcggcccagagccacaagataacgcagccaagaacaagagacaccgccgagcgagcgaggcggggagaagcaggtccaggaccaggagaaaggaaaaggaagcccagctctctctagcctggagccgagaagccgaggtgaggtcgtggttggcctgggagcgaggaggaatttcgaggcgggaagaagcagagatgatttagcggtttggaagctggttgatgggtgcaattcgttttgtgctgctgtagggggcgaaggagcagcaaggcatggaggagcccgttccggctgatccccccaggattttctggaagtcaaggagttcaggttcaggtgtctgcttgtctcaattcatgttgctgcatacaaaatctcgctgatttcaattgcttcttcttcttctttctttcttttttttaacccccgaagaatcgtattctcgtggcttatccgtttctatgttgttgaaagatgctaatttcagctcagtcatctgcaaatttctctgtcgtaatacagttcatgcagcaatacagttagaatcacacctaaacaccattaatctcagctacttcgtttcggtccacaagcaacagcgctgaccagaaacatttctacctttttgtccatataagttttggtactgatgcccaaaatgtggcggtgagatatttcgtgtggggatagatgatagccagctcactcacgttatgtaactgcgctccgttcttttttatttgtcgctgtttagtttaaaaataagttaacagtaagacgtgaatcacgcacgcacccgtgctactgaactgctgttggttagcccgtttggtggttcacgagacgaccgtagcaatcccttgccaggtacaactacaagaagagctagcgattgcagcaagaaatcgtattcctagtaggcacgctttgcagcaagactagtgattgctaattagctagatttctgcgtgtctcttgtctgtttctgcccttccatcactgttcccctcctcctgcggttcagacgtggccaaagacttgtacgcgttctgcaaccgatgtagcgtcgtcctagagtttctaggcatggcaacagaaacaagcacgaaccgttctaaccgtctaggcatggtcacagacaagcagataaactacaatctttgtgtattatatgcaaattaaattatatgagtattttcgtagcccatgtccggacggcagcatggccgggtctcgtgtgggtcaaattaaattatatgtagcctttgtgtcttgtgtgggccggcttattattggaatgctacatctggttaatactactgaccataatgtgacgctgacagattagtttagggaaaaataaaccagccttggaaattgctctctatgttcgattcagtgtttcggccccttgttactttgcttctgtgtggggggctggtacatatacatatagcatacttgcaagacactgaagggctgtaaggaaccaaagaacccccagaacaaaaaaatgaaagcaagggctgtaaaaaaaatctcactatgaactgaatagaagcaagcatcccttggcctctccaaaagagctgttcacatatggcagccaaactcatcctcaccactcgctaacatattggttgtccaagtgaacgatcgtgctgtagagccaagggtcggtcacgcgtgcattagattttagggatccctagattttaactggggaattgcactggctcctgatctgactaacaatgtgtgtgttccagccaatggccggagcctgcaacaagagcctgacaaagacgctaccgaggaaactaacgagcaggctcaagaggaacccatgaagaccgacgacgcaacggacacagcagcagcagcagcagctacagctgagccgtacccgaaagctaacctatccgagaagcggaaggctctcttcgagcctctcgagccgatcaacggcaagcgcggcgctgctgagacgctgctcccaccgccggactttgagcccgcgtcgtaccccaaggggtggctggtgggcaagaaacgcaagctcgtcaacgtagacgtcgtggagagcatgcggaggattgcgatccaggaaatgaacagaaaggttcatgcataatcacatctttctagtggtcatgcaatgctgtttcttcactcgatcgtaaatgcatcgatgtgttcagttcaggttgacacatttgaaaaaaatatatcctcaaatgttgttggcttctgtttttaatctgtgataaagagtgagtatgcgttcatgtgtaaactgcaggcagttttgttgctgaacatgcatgcgtgcatcaaatgctgaccaatgttgttgctgtggacatggtgtggcacgcaggaccgtgagatcaatgggctgaacgagcagctagaggaagactcccgcgtgctggagcttctgcagaagcagctggctgacgagcgcaggaagcggacagagatcgagaaggagaactccatgctccatgagcaggtcaccatgctgatgaacatgctcgacgagaacgagggtttcgacgaggacggagaggccccgccgcccgattccttcgattaagcgttgttacagtactatatccgttttctttttcccgtcagtgtgaaatcatacgtctctaggtgctggtttcagagtatccgagagatatgggctagctgtgtagtaggatttcattggtggtcgtattccattacatggctttggcttctgtagataaagggtgcattgcatgtctgttgtactgtactgtacctactccttttctaggcttcaaaagtgtatgtgagaaactagcaacatgttatgtttgaatcgaagtgtatgtacatgttacttaaaattcttccttgctatgccaaaa

SEQ ID NO: 15 - protein, 211 aa, Zea mays
MEEPVPADPPRIFWKSRSSGSANGRSLQQEPDKDATEETNEQAQEEPMKTDDATDTAAAAAATAEPYPKANLSEKRKALFEPLEPINGKRGAAETLLPPPDFEPASYPKGWLVGKKRKLVNVDVVESMRRIAIQEMNRKDREINGLNEQLEEDSRVLELLQKQLADERRKRTEIEKENSMLHEQVTMLMNMLDENEGFDEDGEAPPPDSFD

SEQ ID NO: 16 - DNA, 2940 bp, Oryza sativa
  source 1..2940: mol_type = genomic DNA
gaaggcacgcgagacggtcaagaaacaaacgggagttgcttccaaggcgaaggcgacccggtgacccacctctcctctctcttctcgccgtcctagcaagtagcaaccctcctcagccaagaaccacaagataacgcaactcacaaggcacgcacccatagattgatagagagagggacagagagagagagagatagagctcaggttgcaagcagatagaacgggtccaggtagcttcgcaatcaagaagaagaagaagaggtgagattttgattttgattttgattttctctctgtttgtttttgctttggtgtggttcttgtttccccagtcgagagcctcaccccctcaagaggctcatggaggtgaggagaaatcaaaggccaagctgattttgtgtgatttgattctctctgctgcagtgaaggaggaggaggagcaagagcaagccatggaggagccggcctcggctgatcccccgcggattttctggaagtcgaggaggagatcagcctcaggtgctttgttaattacatgcttcattcaaatgtaaatcatgctgatttcgactcctgcttcttcttgctctgctcagatatgagatatccattccttctctcataatctcttgttgattaaatctcgctagcttcaaattcagtccctttcgaagcttctctgcattttctttcagttttaaaaaaattgtatgaaccatacaacactttgatttacggttttacacctaattactggtaatcttggctacttacaagttagtatcctcgaaatttcctgctgctaaacgtactgtagctggtagcatggaataatttctgagtgagatgtttcgtgggggattaaattattgccagctcactgaatcgatatataattattattccgtacacgttaatcacgcaccggtttggctggtccatttggtgcaagctcatgaggattaagacttagaggcgccttgataactaaactaagaggatgtggcctgcttaatttgcttgtctttaccgccaagattctgaaactgcacctgtcggtgctaggtagcttaccagtgctagtgcgaatatgcttgcagaaacaaatcatattcctctccgtaacttggtactgccttgctttgtggaatgagattttttattggtgcatctggctgctacttcttttgttgctcatgtatcctctatgatttcactgctcttttggtcaactcccaattaagttgcaactgcatctagataattttggtattgacaaagacatagacgaacttgcttggtcgcatacagtaattatggcctcacgtgcaataatttttcccggggtcagagtgtcagattaaatagcatgttgtcgaccttagcagttagcagtgttaaataaggttagggtgtcgttgcatgtggcaatattgaacctttttttttttttgaacatgtgttgttgaccagttagcttaggccttaggccaaagtaaatcaatcagtttttgctcttgaaaatgtaaggcttgtcaatgcatagaacttgcaggagataatttgtttaattgtgcatgttccaaatagttgctgtttttgtaccttgatactttgcttcatcaccaaggatggtctacatatgtcaatataaatacattgagagaccgttcgttggtcttgagctgatgtatgctaacaagttatcaggctgtcatgatagcagaacacactctgaaattaaagaacttccatataatcatgtagttataatgttcacctgtatgcattagattttagctagagaagtgcactgactcttgaatctgactaacaatatgtatgttccagccaatggccggagcttgcaacaagaacttaacaaagaggctgctgatgaacaactgaacaatcaggctcatgaagaggccatgaaaatagatgatgcaaatgcagtaagtactgacgacgatgttcatccagatccaaaagctaacttatctgagaagaggaaggcgctgtttgagcctttggaaccaatcaacggcaagcgcagttctgctgaaatgttgctcccaccaccagactttgagcccgcgtcatatcccaagggatggctggttggcaagaaacgcaagcttgtgaatgttgatgtggtggagagcatgaggaggatagcaatccaagaaatgaacagaaaggttcatgatctttttaatagtttgctaccgtaccacaataccacatactagcacaatatcgtgatgcatttggtatacttttttcctttttttttatcgatgatcaaggcttgaaaaaactaactttatcctcaatttacgacgtgtgttggtctagttaaacccaaagttgaattatatgcgattctatttgttgctcactgaagcatacattgactcctatattcatggaaatgctgtggcaggaccgtgagatcaatggcctgaatgaacagttggaagaagactcccgagtgcttgagcttctacaaaagcagctcgcagatgagcgtaagaagcgaacggagatagagaaggaaaattccatgcttcatgagcaggtatctatgctgatgaacatgctcgatgaaaatgaagcctttgatgaggagggagaagcaccaccacctgataccttataggcttagattaagtaatattatcaaggttccaagttctacacatcttcggataccagtttaagagtattcccagatgtctttatcttgtgtaaaattcaatttatcttattttattttatggcttgtgtgtagatgaaggggttctgtttgctgtacctatttgtttctaggctgcaagtgtatgcgagatgcttgtaatgtattctatttaaatgcaagtgtttacatgttataagagctcttgcaagactccttttccttgcatgagctcttttgct

SEQ ID NO: 17 - protein, 210 aa, Oryza sativa
MEEPASADPPRIFWKSRRRSASANGRSLQQELNKEAADEQLNNQAHEEAMKIDDANAVSTDDDVHPDPKANLSEKRKALFEPLEPINGKRSSAEMLLPPPDFEPASYPKGWLVGKKRKLVNVDVVESMRRIAIQEMNRKDREINGLNEQLEEDSRVLELLQKQLADERKKRTEIEKENSMLHEQVSMLMNMLDENEAFDEEGEAPPPDTL

SEQ ID NO: 18 - DNA, 4304 bp, Triticum aestivum
  source 1..4304: mol_type = genomic DNA
gtggcttccaaggccaccgtttttcctttctttctgctagtggcaccaacagcccgcccacgccacggcacaagcacagccagaaaccacgagataacgcggcgcacgcgaccaaaccgcaccgaggcagagagagcgagagattgggaggagctccggcaggcaggcagcaggaagtcgagccgaggagccaccggaggtgagctgagctcctgaccatttcgtccttactgacgcaggatttcggtagctgatgtatatttgcgctcttgtcttgggctgcagtgacctgccggccggggagcatggaggagccgtccatggccgacccgccgcggatcttctggaagtccaggaggaggccgtcgtcaggtaggggtgctctgctccttcttgctgcttcaaatcctttgagcaaacgtcttcaactcttgaatccatcctgatttgaaccgcttcgttttaaaaaagaagaggatattgttcctttacaaagaaaggagcctgtccgtccttcagccattccctcttctctcccacaaccgtattgccggtttcgccaaatttcagtccagatctcggcaaaggctcccctcatgctttctctctctctctctctctctctctctctctctctctctctctctctctctctcctgggaattaattttgaaatttgctcctgccatttctttcttgaaaattatcacgaagtcttacaccaattcgatttacagcccagaatctccctctgttcctcgattcttcgttagcttcctctgcctctgcctctgcctctgcaaaaattagtggcttcttcctttttgttcgtcggttctttctaggatgttcatccgtcttcgcacggcaccagacctgacggcctgaaacattccagcagtgagatattgcgtgaggaaatggattgacaattgccacctcacgtagacgaatcacgaatatacaactaccaatacgagtaagaaaatcgcagtttccgcccacacgttagtcacgcggctgcccggcgcaactgattcttcgatgtatatttataatcaattaatcaacggcctcgcgcaagcaaggtcgttcagagcttcagaccttggttagtttgggggtaatttctcacaaggggggtgggtgggtgctgtgctgctgtagtgccccaattgcctagccttgcttgccgttgccggcaagatctctgcgggccggcagctgcagcagctacccagtagtggtcgtggtcgtggtcgtgcgaatatgctcgcgccaagaaaccgtatccctttcagtaatttgctgttgttgggtttcacttttcagtaatttcacagcgctgctatgcacacgacaaaatcaagccgatgcttgcacgacgctatggttagaaccgtccatgcatagaagaaattgtagcccagccgctgatttactgtcgtccacaaatcgtccaaggaaacgtcgtccgtatagtagtttcgtttcagccccactcctctgaattctattagtattctgtcttgggcaatgttacgagatgctctccaggagcaggggaagcttggctgcgagggcagcagcgaacaaggctgtaatttcttctcagaaaaagagggctgcagttttggtaatacaactactagatgacagagggtgaatgtgatgggctgagatatctatggccttaattctctgacttagtagataatgccgattgtttattatggcgcaacccgaggctcgagagatgcgcgtgtttcgtgaccactcgcttattttagagttcatgtcagaatgttcagtagtaaataagttaatctaatgatgctactactgaccaaattaccgtgtctgaacctgccaatgttgaccagtaagctaccgtgtaagtaaatcagtttgctcttagtgtgtaaccaatgaacagataaaagggttaaattgtttccactatcctctccagagcttctgagaatattctttcagtagatcttgcagggaattccttgtattatacagtatatgtgttctaagctgtaagctgtccctgtctatcacaaccctttcttgctttgcttccttgtcaaggagagggcatacagcttgttgaagtacgcatccatgttccaaatggcagcaaaactcactctcacctatcatcactctacctgtctaccagtaatccactgaaaaaacttctagctgatcatattctagtgctaatggccatgtaaataaacaagaatcattttggtcgtgttgatatcaatgcagataggtggagggcgcgggtcccttcactagtattaaacaagaatcatttttggttgtgtttccttttcaagttattgatgtcaatgcacacccatgattgaaaccatatccccttcagtaacttgctgttgtgcaatgaccttttcagtcctcttactctgaattccactagtattctgttttgggcgaggcagcggaaaggctcttcaggaggagcagtaacaacgcggcaatttcttaggacgaaagaaaagggtgactgtgatagactgagatatctatggtccacattgtcttcgtataataccgattgtttacagcataatgtcaggctcgagacaggcgtgaccactcacgtttatttggagttgctgtcagaatgtttactttaattaggctggtctgatgatactgaccagataaactatttctgaacctgccaatgttcattgttatttatatagcttcaccattcatgccgaatggtctgaacctgccaatattgaccgtgttagtaaatcactgctcctagtgtataactgataaacggataaaaggataaattgtttccacttctatcctctccagagcttctgagaatagtctgttgatagatcttgcagggaattgcttgtattatacaatatgtctaagctgccgctgtctatccaagttccaaatggcagcaagactcactctgaccaattactccaccagttatccaccaaaaaaacttccggttgatcatattctaattcgagtgccaatggtcatgtatgtcagtcagtatatgtatgcactgcattttgctagggtaaatgtactaactactgacttactcagtctgacttaccaatgtgtatgttccagccaatggccggagcttgcaagcacaagaacataataacgaggccgctgccaccgaagaggcagcagcggacactcttccggctcaaggagaagccatgaagattgatgacgcaaatgcagcaagcactaccacagaggatgatgctcatcaggcagatccgatggctaacctatctgagaagcgaaaggcgctctttgagcccctggagccaatcaatggcaagcgcagcgctgacatgctgcttccgccaccggacttcgagcctacatcatatcccaagggatggctggttggtaagaagcgcaagctcgtcaatgtcgatgtcgtggagagcatgaggaggatagcgatcctggaaatgaacagaaaggttcatgttcttgctaattatttgccagcatatgctagcgtaatatcatgctggatatatgccatactgttttctgtggtaattgcatccatgatcaaggcctgaaatcaagcatgaaacactaactttaccattaacttatgatgacccatgcattgttctagtgcagctaaggtaattaggcatttttgttattgttgccaaatctgcatcataggttgatacatattatcatgtaaaatatctcgcaaattggcatggcaggaccgtgaaatcggcgggctgaatgaacaactagaggaggactcccgcgtgctggagcttctgcagaagcagctcacggacgagcgcaggaagcggtcggagatcgagaaggagaactccatgcttcaagagcaggtgaccatgctgatgaacatgcttgatgaaaacgaagccttcgacgaggaaggagaagaggcgccaccacccgactcaatcgattaagcatttccgacaactgcaggttcccctttttaagaaaaggcgtctgcagcacgtccgtctttgggtgccaatttgagagtatcccggaggtttctattggtctcttgtgtagaattcaaatattatttcgtttcatggtttgcatcgtgtaggcgaagggtgcatgttttattgttcctgttcgtatctaggtttgttgcagatgtatggagacatttgcgacgcattttatttgaaatcaagtgtgtgtatatggtattacgattattttgccagccactgctatttttttct

SEQ ID NO: 19 - DNA, 4101 bp, Triticum aestivum
  source 1..4101: mol_type = genomic DNA
gagtggcttccaaggccaccgtttttcctttctgctagtagcaccaacagcccgcccgcccacgccacggcacaagcacagccagaaaccaccagataacgcagcgcacgcggccaaaccgcaccgaggcagagcgagcgagcgagagattgggaggagctccggcaggcaggcagcgggaagtcgagccgaggagccaccggaggtgagctgagctcctggccatttcgtccgtgttagacgccggatttcttctatagctgatgtatatttgcgctcttctcttgagctgcagagacctgccggccggagagcatggaggagccgtccatggccgacccgccgcggatcttctggaagtccaggaggaggccgtcgtcaggtaggggcgctgcttcttgctgcttcaaatcctttgagcaaacctcttcaactcttgaatccattccatcctgatttaagctgcgcgcttttttctttaaaatacaagatattattcctttacaaagaaagtaacctgcccctcacctattccccacgcagccgtattgccgatttcggcaaatttcagcccagatctatgcttgttctttcctggggattaatcttgaaatttactcctgccgccgtttcttttttgaaatctatacaaatcgtacaccagttcgatttacagctcggaatctccccctgttcctcggctcttcattagcctcgtctgcctctgcagaaattagctccttcttttttgttcctcggttctttttagttaggggtgttcatccgttttcggacggcaccgaaacattccagcagtgagatattgcgtgaggaaatgggttgacgattgccaccccacggagacgaatatacaaccacccatacgagtaagaaaatcgcagtttccgcccacacgttagtcacgcgcgcggccgtgcaactgattctttgttgcatatttataattaattaatcaacggcctcgcgcaagcaaggccggccgttcagagcttcagaccttgtttagtttgggggtaatttctcacaaggcgggtgggtgagtgccccgcttgcttagccttgcttgccttcgccggcaagatctctgcagtgcaggcagctgtcagcaccgcaggccggcagctgcagctgcagctgctacccagtagaggtcgtggtcgtgcgaatatgctcgcagcaagaaaccatatccccttcagtaactttgctgctgttgggttgagcttttgaggccccctcctctcaattttactagtattctgccttgggcaatgcagcgagatgctctccaggagcaggggaagcttggctgtgagggcagaatccaacgaggctgtaatttcttctgagaaaaagagggctgcagttttggtaatacaactactagatgacagagggtgaatgtgataggctgagatatctatggcctcaattctctgacttcatagataacaccgattgtttattatggcgcaacccgaggctcgagagacgcgcgtgtttggtgaccactcgcgcttattttagagttcatgtcagaatgttacagtaagtaggttaatctatctaatgacactgaccaaattaccgtttctgaacctgccagtgttgaccagtaagctatcgtgtaagtaaatcaatgtttgctcttagtgtgtaacccatgaacagataaagagttaaactgtttccactatcctttccagagcttctgagtgtattctttctgtagatcttgcagggaattccttgtattatacagtatgtgttctaagctgtccctgtctatcagagccctttcttgctttgcttcctagcaaaggagagtgcatacagcttgttgaagtacacatccatgttcgaaatgtcagaaaaactcactctcacctatcatcactctgccagtaatccactgaagaagcctctagctgatctctgtggtcatgtaaataaacaagaatcattttggttgtgttgatattaatgcaaataggtggagggcgcgggtccttttatactatattaatcaagaaccatttttggtcgtgtttccttttcaagttattgatgtcaatgcacacccatgattgaaaccatatccccttcagtagttccctctgaacaccactggtatttctgtcttggcgaggcaatggaaaggctgtttaggaggagcagtaacaacgcggcaatttcttaggacaaaaagaagagggcgactgcaatagactgagatatccatggtccacattggcttcgtataataccgattgtttacagcataatgtcaggctcgagacaggcgtgaccactcacgtttatttggagttgctgtcagaatgttaatttaattaggccggtctgatgatactgaccagataaactatttctgaacctgccaatgttcattgttttttatatagcttcaccattcatgccgaatggtctgaacctgccaatgttgaccgtgttagtaaatcagtctgctcgtagtgtataactcatgaacagataataaaaggagaaactgtttccacttctatcctctccagagcttctaagattagtctgttaatagatcttgctgggaattgctttattatacagtatgcctaagctgtccctatctatgctttgcttccttgtcaaggagagtagatacagattaaagtacatccaagttccaaatggcagcaaaactcactctgacctattactgaattactccaccagttatccactgaaaaaacttccggctgatcatattctaattctaatgccaatggtcatgtatatcagtcagtatatatatgcactgcatttttgctgggctaagtgtactgactactgactcactcgatctgacttaacaatgtgtatgttccagccaatggccggagcttgcaagcacaagaacatagcaacgaggccgctgccaccgaagaggcagcagcgggcaatcttccggctcaaggagaagccatgaagattgatgacgcaaatgcagcaagcaccaccacagaggatgatgctcatcaggcagatccgatggctaacctatctgagaagcgaaaggcgctcttcgagcccctggagccgatcaatggcaagcgcagcgctgacatgctgcttccgccaccggacttcgagcctacatcgtatcccaagggatggctggttggtaagaagcgcaagctcgtcaatgtcgatgtggtggagagcatgaggaggatagcgatcctggaaatgaacagaaaggttcatgttcttgctaattatttgccaccacatgctagcataatatcatgctgggtatatgccataatgtttctctcgtaactgcatacatgatggaggcctgaaatcaagcattaaacactaactttatcgttaacttaaattgacctgtgcattgttctagtgcagctaaggtaattaggcatttttgttattgttgccaaatttgcatcataagttgacacatattatcatgtaaaatatctcgtaaaatggcgtggcaggaccgtgaaatcggcgggctcaatgaacagctagaggaggactcccgcgtgctggagcttctgcagaagcagctcacggacgagcgcaggaagcggtcggagatcgagaaggagaactccatgcttcaagagcaggtgtccatgctgatgagcatgcttgatgaaaacgaagccttcgacgaggaaggggaagaggtgccaccgcccgactccatcgattaagcatttccgacaactgcaggttcccctttttaagaaaaggcatccgcagcacgtccatctttgggtgccaatttgagagtatcccggaggtttctattggtctcttgtgtagaattcaatttatattatttcgtttcatggtttgcatcgtgtaggcgaagggtgcatgttttattgttcctgttcgtgtctaggtttgttgcagatgtatggagacatttgcgacgcattttatttgaaatgcaattgtgtgtatatggtattacgattattttgccagccactgcaattcttttttcatattttgaagtggccatggcatctgatctactagtgt

SEQ ID NO: 20 - DNA, 3914 bp, Triticum aestivum
  source 1..3914: mol_type = genomic DNA
taacgcggcgcacgcgaccaaacaagctacaccgaggtggggagagcgagagattgggagctccggcaggtagcaggaagttgagccaaggagccaccggaggtgagctgaggtcctgaccatttcgtccttgttagacgcgggatttcttccatagctgatgtgtatttgcggccggccggccgctcttgtcttggaccgcagagacctgccggccggggagcatggaggagccgtccatggccgacccgccgcggatcttctggaagtccaggaggaggccgtcgtcaggtaggagcgctgcttcttgctgctcaaaatcctttgagcaaacctcttaactcttgaatccgtcctgatttgaactgcgccctttaaaagaagaagaagatattgttgttcctttataaagaaaggaacctgtccgtccttcacccattccccatctatcccacaaccgtactgccggtttcggcaaatttcagtccagatctcggcaaaagctcccctcatgctttctctctctcctgggaattaattttgaagtttgctcctgccatttgttttttgaaaattatcacgaaatcttacaccaattcgatttttacagcccagaatctccttctgttcctcgattcttcgttagccgagcctcctctgcctctgcctctgcctctgcagaaattagtggcttcttcccttttgttcgtcggttctttctagggatgttcatccgtcttcgcacggcaccggacctgacggcctgaaacattccagcagtgagatattacgtgaggaaatgggttaacgattgccacctcacacggacgatatatacaactaccaatacgcgtaagaaaatcgcaatttcccgcatacgttaatcacgcatgcggccggcgcaactgattcttcgttgtatatttagaatcaattaatcaaaggcctcgcgcaagcaaggccggccgttcagagcttcagaccttggttagtttgggggtaatttctcacaaagggggtgggtgctgtgctgctgtagtgcaccgcttgcctagccttgcttgtcgtcgccggcaagatctctgcaggcagctgtcggcaccgcaggccggcagctgcagctgctaccctacccagtagtggtcgtggtcgtgcgaatatgctcgcggcaagaaaccatatccctttcagtaatttgctgttgttgggatgagcttttgaggccccctcctctgaatattactactagtattctgccttgggcaatgcagcgagatgctctccgggagcaggggaagcttggctgtgagggcagcagccaacaagtctgtaattttttctgagaaaaagagggctgcagttttggtaatacaactactagatgacagagagtgaatgcgataggctgagatatctatggccttaattctctgacctggtagataatgctgattgtttatttatggcgcaacccgaggctcgagagatgcgcgtgtttggtgaccactcgcgcttattttagagttcatgtcagaatgttacagtaagtaggttaatctaatggtactgaccaaattaccgtttctgaacctgccaatgttgaccagtagataatgccggagtaagtaaatcagtttgctgttagtgtctaaccaacgaacagataaaagggttaaattgtttccactatcctctccagagcttctgagaatattctttctgtagatcttgcagggaattccttgtattatacagtatgtgttctaagctgtccctgtctatcacagccctttcttgctttgcttccttgtcaaggagagtgcatacagcttgttgaagtacatccatgttccaaatgtcagaaaaactcactctcacctatcatcactccaccagtaatccactgaaaaaatttctagctgatcatattctagttccaatggccatgtaaataaacaagaatcattttgttcgtgttgatatcaatgcagataggtggagggcgcgggtccctttactagtattaaacaagaaccatttttggtcgtgtttccttttcaagtaattgatgtcaatgcacacccatgattgaaaccataccccctttagtaactccctctgaattccactggtattctgtcttggcgaggcaatggaaaagctcttcaggaggagcagtaacaacgcggcaattccttaggacaaaagaagaggacacctgtgatggactgagatatctatggtccacattggcttcgtataataccgattgtttacagcataacatgaggctcgagacaggcgtgaccagtcgcgtttatttggagttgctgtcagaatgtttactttaattaggccggtctgatgatactttctgaacctgccaatgctcattgttttttaatatagcttcaccattcatgccgaatggtccgaacctgccaatgttgaccgtgttagtaaatcagtctgctcgtattgtataactcatgaacagataataaaaagataaattgtttccacttctatcctctccagagcttctgagaatagtctattaacagatcttgcagggaattgcttgtattatacagtatgcctaagctgtccctatctatgctttgcttccttgtcaaggagagtagatacagattgaagtacatccaagttccaaatggcagcaaaactcactctgacctattactgaattactccaccagttgtccactgaaaaaacttccggctgatcatattctagttctagtgccaatggtcatgcatatcagtcggtatatatgtgcactgcatttttgctggggtaaatgtactgactacggactcactcaatctgacttaacaatgtgtatgttccagccaatggccggagcttgcaagcacaagaacatagcaacgaggccgttgccaccgaagaggcagcagcgggcaatcttccggctcaaggagaagccatgaagattgatgacgcaaatgcagcaagcactaccacagaggatgatgctcatcaggcagatccgatggctaacctatctgagaagcgaaaggcgctctttgagcccctggagccgatcaatggcaagcgcggcgctgacatgctgcttccgccaccggacttcgagcctacatcgtatcccaagggatggctggttggtaagaagcgcaagctcgtcaatgtcgatgtggtggaaagcatgaggaggatagcgatcctggaaatgaacagaaaggttcatgttcttgctaattatttaccaccacatgctggcataatatcatgctgggtatatgccatactgttttttctggtaactgcacacatgttcgaggcctgaaatcaagcatgaaacactaactttactattaacttatgatgacctgtgcattgttctagtgcagctaaggtaactaggcatttttttattgttgccaaatttgcatcataggttgatacatattatcatgtaaaatatctcgtaaaatgatgtggcaggaccgtgaaatcggcgggctcaatgaacagctagaggaggactcccgcgtgctggagcttctgcagaagcagctcacggacgagcgcaggaagcggtcggagatcgagaaggagaactccatgcttcaagagcaggtgtccatgctgatgagcatgcttgacgaaaacgaagcctttgacgaggaaggagaagaggcgccaccgcccgactccatcgattaagcatttccgacaactgcaggttcccctttttaagaaaaggcatccgcagcatgtccatctttgggtaccaatttgagagtatcccggaggtttctattggtctcttgtgtagaattcaatttatattatttcgtgtaggcgaagggtgcatgttttattgttcctgttcgtatctaggtttgtt

SEQ ID NO: 21 - protein, 292 aa, Triticum aestivum
VASKATVFPFFLLVAPTARPRHGTSTARNHEITRRTRPNRTEAERARDWEELRQAGSRKSSRGATGVTCRPGSMEEPSMADPPRIFWKSRRRPSSANGRSLQAQEHNNEAAATEEAAADTLPAQGEAMKIDDANAASTTTEDDAHQADPMANLSEKRKALFEPLEPINGKRSADMLLPPPDFEPTSYPKGWLVGKKRKLVNVDVVESMRRIAILEMNRKDREIGGLNEQLEEDSRVLELLQKQLTDERRKRSEIEKENSMLQEQVTMLMNMLDENEAFDEEGEEAPPPDSID

SEQ ID NO: 22 - protein, 219 aa, Triticum aestivum
MEEPSMADPPRIFWKSRRRPSSANGRSLQAQEHSNEAAATEEAAAGNLPAQGEAMKIDDANAASTTTEDDAHQADPMANLSEKRKALFEPLEPINGKRSADMLLPPPDFEPTSYPKGWLVGKKRKLVNVDVVESMRRIAILEMNRKDREIGGLNEQLEEDSRVLELLQKQLTDERRKRSEIEKENSMLQEQVSMLMSMLDENEAFDEEGEEVPPPDSID

SEQ ID NO: 23 - protein, 219 aa, Triticum aestivum
MEEPSMADPPRIFWKSRRRPSSANGRSLQAQEHSNEAVATEEAAAGNLPAQGEAMKIDDANAASTTTEDDAHQADPMANLSEKRKALFEPLEPINGKRGADMLLPPPDFEPTSYPKGWLVGKKRKLVNVDVVESMRRIAILEMNRKDREIGGLNEQLEEDSRVLELLQKQLTDERRKRSEIEKENSMLQEQVSMLMSMLDENEAFDEEGEEAPPPDSID

SEQ ID NO: 24 - DNA, 4239 bp, Hordeum vulgare
  source 1..4239: mol_type = genomic DNA
cctgtccgtccgtctgtctgacagtcagccacaagcgtgaacggcgtgagcaccgtggttcaccgggcgacagccagcgcgtcacgtcacgggcacggctgaaagccaccgtcaagggcgccaaggaaacgggagtggcttccaaggccaccgttcctttctttctcctcctgctagcagcaccacgcccacgcccacgccacggcacgagcacagccagaaaccaccagataacgcaccgcaccgcaccgcacgcgaccaaacaagctagaccgaggcggagagagcggcgagagattgggagctccggcaggcggcagccgggaatcgagccgaggagcccgccgaggtgagctgagctcctgaccatttccgtccgtccttcttgaccccggatttcttcagtaccagactagctgatgcgtgtttgccgctcttctcttgagctgctgcagcctgcagggggggcataggaacagattggaaggggcggagcgcatggaggagccgtccatggtcgacccgccgcggatcttctggaagtccaggaggaggccgtcgtcaggtaggggcgccgcttcttgccgcttcaaatcctttgaacaaacctctgaatccatcctgatttgaaccgcgcccttttatataaaaatacacatgagatagtgttcctcctttacaaagaaaggaacctgcgttcctcacccattcaccgtctctcccacacccgtgttgccggtttccgcaaacttcagtccagatctccgcaaaagctcccctcacgctttctctcctggggattaatcttgagatttgctcccgccgtttctttcttggaatttgcacagaatcgtacaccagttcgatttacagctcgggacctcctcctgttcctctgcagaaaaaccagcggcttcttcctttttcttcctcggttatttctagggatgttcatccgttcccgcagtccgcacggcgccggagcattccagcggtgagatattgcgtgaggaaacggattgacgaccgccaccccacgcagacgaatatactaccaccaatacgagtaagaaaaatcgcagtttccgcccaccacgttggtcacgcggccggccggctcaactgattcttcgttgcatgtttataattaattaatcaacggcgtcgcgcaagcaaaggtcgttcagagcttcagaccatggttagtttgggggtaatttctcacagagtgggtgggtaggtgggtgctgtgctgctgcagtgcccttgcttgccttcgccggcaagatctctgcaggtcgtgcgaatgtgctcgcgccaagaaacctatccccttcagtaactttgctgttgttgggatgagcttttgaggcccctcctcctctgaatattactagtattctgtcttggacaacgcagcgagatgctctccaggagcaggggaagcttggctgtgagggcagcggccaacgaggctgtagttttcctgagaaaaagagggctgcagttttggtaatactagtactagatgacagagggtgagtgcgataggctgagatatctatggccttaattctctgacttcgtagataatgccgattgtttatgtcgcgaccagaggctcgagagatgcgcgtgtttggtgaccactcgcgcttattttagagttcatgtcagaatgttacagcaagtaagttaatctaatggtactgaccaaattaccgtgtctgaacctgccaatgttgaccaagttagatcttgcagggaatttccttgtattgtacactatgtgttctaagctgttagctgtcgctatctatcacagccctttcttagcttcgcttccttgtcaaggagagtgcatacagcttgttgaagtacacatccaagttccaaatggcagcaaaactcactctcacctatcatcactctaccagtaatccactgaaaaaacttctagctgatcctattccagtgccaaaggtcatgtaaataaacaagaaacatttcgattgtgttgatattaatgcagataggtggagggcgcacccccctttactatattaaacaagaaccattttggtcatgtttccttttcaagttattgatgtcaatgtgcacccatgattgaaaccatacccccttcagtaacttgctgttgtgcaattaccttttcagtcctcttcctctgaattccactagtattctgttttgtgcgaggcagacgaaagtctcttcaggacgagcagtaacaacgcgggaatttcttaggacaaattgactgtgatagactgagatatctatggtccacattggcttcgtataatactgattgtttacagcataatctgaggctcgagacaggcgtgaccagtcacgtttatttggagttgctgtcagaatgttactttcattaggccggtctgatgatactgaccagataaattagtatttccaaacccaccagtgttctttgtttttatatatcttcaccattcatgccgaatgatctgaacctgccaatgttgaccgtgttagtataaaccgtttgctcgtagtgcataactcatgaacagataagaagataaattgtttctacttctatcctttccagagcttcttagaatagtctgttaatagatcttgtagggaattgcttgtactccctccgttcctaaannnaagtctttttagatattccactagaggactacatacggaacaaaatgattgaatctacactctaatgtatgtctnnntacatccgtatgtagttttttagtagaaactcttaaaagacttatatttaggaacggagggaatattatacaatatgtttaagctgttgctatctatgttttgcttccttgtcaaggagagtagatatagattgaattacatccaagttccaaatggcagcaaaactcgctgatctattactccaccagttatccaccaaaaaaacttgcagctgatcattttcaaattctagtgccaatggtcatgtatattcactgcatttcgctggggtaaatgtactgactagtgactcgctcaatctgacttaccaatgtgtatgttccagcaaatggccggagcttgcaagcacaagaacataacaacgaggctgctgccacagaagaggcagcagcagacaatcttccggctcaaggagaagccatgaagattgatgaagtaaatgcagcaagcactaccacagaggatgatgctcatcaggcagatccgatggctaacctatccgagaagcgaaaggcgctcttcgagcccctggagccaatcaacggcaagcgcagctccgctgacatgctgctcccaccaccggacttcgagcctgcgtcatatccaaagggatggctggttggtaagaagcgcaagctcgtcaatgtcgatgtggtggagagcatgaggaggatagctatcctggaaatgaacagaaaggttcatgttcttgctaattgtttgccaccaaatgctagcataatatcatgctaggtatatgccatactgtttttctctggtaactacatacatgaccgacgcctgaaataaagcatgaaacactaactttaccattaacttatgatgacctgtgcattgttccagtgcagccaggtaattaggcatttttattagagttgccaaatttgcatcataggttggtacatattatcatgtaaaatatctcgtaaaatggcatggcaggaccgtgaaatcggcgggctcaatgaacagctagaggaggactcccgcgtgctggagcttctgcagaagcagctcacggacgagcgcaggaagcggtcggagatcgagaaggagaactccatgcttcaagagcaggtgtccatgctgatgagcatgctcgacgaaaacgaagccttcgacgaggaaggagaagaggtgccaccgcctgacccatccttcgattaagcatttccgagaactgcaggttcccttttataagaaaaggcatctggagcacgtccatctttgggtaccaattagagagtatcccggaggtttctattgatctcttgtctagaattcaatttatattatttcgtttcatggtttgcattgtgtagacgaagggtgcatgttttattgttcctgttcgtatctaggtttgttgcagatgtatggagacatttgtgacactttttatttgaaatgcaagagtgtgtatatggtattctgatttttttttcatatttcgaagtc

SEQ ID NO: 25 - protein, 351 aa, Hordeum vulgare
CPSVCLTVSHKRERREHRGSPGDSQRVTSRARLKATVKGAKETGVASKATVPFFLLLLAAPRPRPRHGTSTARNHQITHRTAPHATKQARPRRRERREIGSSGRRQPGIEPRSPPSLQGGHRNRLEGAERMEEPSMVDPPRIFWKSRRRPSSANGRSLQAQEHNNEAAATEEAAADNLPAQGEAMKIDEVNAASTTTEDDAHQADPMANLSEKRKALFEPLEPINGKRSSADMLLPPPDFEPASYPKGWLVGKKRKLVNVDVVESMRRIAILEMNRKDREIGGLNEQLEEDSRVLELLQKQLTDERRKRSEIEKENSMLQEQVSMLMSMLDENEAFDEEGEEVPPPDPSFD

SEQ ID NO: 26 - protein, 345 aa, Hordeum vulgare
TVSHKRERREHRGSPGDSQRVTSRARLKATVKGAKETGVASKATVPFFLLLLAAPRPRPRHGTSTARNHQITHRTAPHATKQARPRRRERREIGSSGRRQPGIEPRSPPSLQGGHRNRLEGAERMEEPSMVDPPRIFWKSRRRPSSANGRSLQAQEHNNEAAATEEAAADNLPAQGEAMKIDEVNAASTTTEDDAHQADPMANLSEKRKALFEPLEPINGKRSSADMLLPPPDFEPASYPKGWLVGKKRKLVNVDVVESMRRIAILEMNRKDREIGGLNEQLEEDSRVLELLQKQLTDERRKRSEIEKENSMLQEQVSMLMSMLDENEAFDEEGEEVPPPDPSFD

SEQ ID NO: 27 - DNA, 1473 bp, Musa acuminata
  source 1..1473: mol_type = genomic DNA
gagagagaaagggaaaagggaaagcagaaacgggtcctcctcctcctcgtcttcctcgtgggtatctccctctttccagagagaattctactgcacacagaagagacgcaggtgacgattcgatccacacttgttccttgtgaatcagcttcagtgctcacctattgcttcttcttctgctcgcttgatcgaggtagtttggggaagggagcaggcggtgatgatggaaggcttctcgccggcttctcctccccggatcttttggaattcccgcaagagatcaggtgaagcaaagattctcatcactgtcttctcttctcttccccccaatctcatcggattccctctccaattttagtctattttatctatatttttcctaaatttcttggtcgagaaggaagagagaattattattgttgttggtagagagcagagatgatttcttgggtgatacgatacgtcacggatcagacagtgcaggtttcttaccggtgattgccgatttggggctgccgtgcctgttattcccgcatcttcgctttaccggcatcaccgggagtaagcagagggcacattgcctcgagcttgccactgtgtagaatctgctgatggcgcaggaagaagaagtactgacgtgtgatcggaatctgcttacagctactgcccggagcttggaagacgcagcagtgcgcgccgtcgctcgagcgaaggaaccgggtgaaacagcgaaagcccacccggctgcggctgacgagcaccgcccggaggaggaggaggagaaggtaggcaaagccgctttgtccgaacgtcggcaggcgctgttcgagccactggagcccagctcctacgggcgtcgcaccccggccgacgtcctgctccctccgccggacttcgatcccacctgctaccccaaggggtggctggtggggaagaagcggaagctcgtgaacgtcgacgtggtggagagcatgcggaggatcgcgatccaagagatgaacagaaaggtctgtagcttccacgcacgcatggtatttgcagaaatggcagaccgggattcacgggtgtgcgattggtgtgacaggacaaggagatcgacggactgaacgagcagctggaggaggacgcgcgctgcctggaacacctgcaggtgcagctactggaagagcggagcaaaagggtggaggcggagaggcagaacgccatgcttcaggaccaagtctcgatgctcatgaacgtgctggaagaaacccaggcagtagaagaggaggcctctggggatcactaatgcctccgacgataccattccttctaccttctactctatatggatcacattaaattcatatgttcaactaaattcatgtacgtgtgttgtgtgcattcacttgtaatgttgcagtctgcgaaaggtgtgaagatgtaattaacaaagcatatatacaaaagattagttttgctattcgatcaaaa

SEQ ID NO: 28 - protein, 204 aa, Musa acuminata
MMEGFSPASPPRIFWNSRKRSATARSLEDAAVRAVARAKEPGETAKAHPAAADEHRPEEEEEKVGKAALSERRQALFEPLEPSSYGRRTPADVLLPPPDFDPTCYPKGWLVGKKRKLVNVDVVESMRRIAIQEMNRKDKEIDGLNEQLEEDARCLEHLQVQLLEERSKRVEAERQNAMLQDQVSMLMNVLEETQAVEEEASGDH

SEQ ID NO: 29 - DNA, 3077 bp, Coffea canephora
  source 1..3077: mol_type = genomic DNA
gacaaatctaggccgtccaaagccattgacgattccgtcagccacctctctctttgggtgatgaatttgatgccaggaaacctggagtgctaatcctctctctctctctctcatttcccacatccgtccgtgttgatgattcaatattctctcacttcatcggcttgagttgtgtaataacaaccttcttcttctcgcctactccaactcctaacaaagcctactatttcctcaacagcaacagacttaaattagtactactactataattagcagctaaggtctgaagaggcagatataattactactactataaaaaaaaaaaaagatcttttctttccttgttatcttatgagtccataaaataaaaggaagaaatagcttttgatggtcagctcttgacttgtaagtcggataaggtacgaatgctatggaggaaccaaataagaaggtggagcagactttgatcaatggattctctcctgtttcttctgctcctgttttctggaaatccaggagaagggcaggttagctacccttttgattcttgtgcttaattatccttttctcttcgcatccttggggtcaaattttgttttgaatttgtggggtttaaggatcaacccatggtttgatgaggggttgcaggatgcaaatgactgtagaaccgtagatctcttcatgcaaaggctaagacttgggatccagaattgtttgctttcttgacatttgaagcttggagtatttttctgctttggttcttcttgtttgtcggctaaatcatttgcaaaactaatcccaacaattaactctgacaatttgacacagctgctccgagattaagcagcttagccctgaaccttatctctgcgactcctcctccctttttctttttcttttctttttttttgcccttttctggggttgggaacttgctgctgggatgtgtactctggacatgggcgatgattgtgaagtgggatcttcccatgtggatggggtgctgcggttgtgggttagggaagggaagcgtacagctgcaccaccaatacttggtctgactttgctcccacgtcacttcattactcatgattggctcgatttaggttggagttagctagcaaatcaacctcaaagaaaatactactattagaaaagaaaataaataaataaaaaagatgggagaaaatggattgtccatctacaatcctccccgtctgattggaatttaatgtttacccctaaagattatttttaaaaaaaaaaaattccttttagactatgaaatgaccacctcatgattagttggctttaaagttttgctgacgatttatttgagataattactgtagcactttttctgatgtgatgtgatgaatgtgagataaaaaggtgattgagaaaataaaaaggtgattgaaatttgtgaagcaaattattttatctgaaatcatgccaatccaaacaaacccacatttgatttttccgtcaccaagataagtatttttctcctccacagtttttccgctattaagattttacatttgattttaaaatcatctatacctaatgttaagaatctttttctactctgtgacatttttcaatggtgaaacttctgatcatagttaatgattgtaaacttgagatcttagttaagtcataatcgcaatttcaatcacttaatgtaatagctgtaatattttcaaaccagtatgagaagatcaaaattttgccaatgctaatttgcagtttgctcagtaaagtagagcctattaactggagacctgcaagcatttgactctggaatacctcttcagactaaaaactaaaccaaactaatactagttatttttaaacactctgagactaggttcacgtttacaagtttaacttcttcatagccttgtggacatagatttcaaataaaagggtgcctccttctagtcagagttttgccttcttacttactgcaaccctaatttgaaagcactaattcttgttacttactatagcatctatttagcagattatagaaggcagcaatcttgagctctttgtgattcccatcttgcttactgccttagtaaaaatattttgaaactaagcacattttttcctggagagattcctgctgaacgtttgcatcttcctgcagtcagcgtgaagtatttagacaaaccaacagaaaatgatgctgataaacctccagaaacacaggaaaatcccaccgctgaggcaatgcaggaggattcaacccctgttgttctatcagagaagaggaaggcactctttgaaccactggaacccatgacaaatataaatggtcgtagaccatccgctgaaatgttacttcccccaccggactttgatgcagcaacttatcccaaaggctggctgattggcaagaagaggaagcttgtgaatgttgatgttgtggaaagcatgcgcaggattgccgtccaggaaatgaatagaaaggtggtgttctcggtagcctctttgagtactagagcaaatattgctctttttactcgaaaacgccggttgtcctctcacaggatgtaacaactaattacattatttcgtttgcaggatagggagattgatggtctgaatgagcagttagaagaggatgctcgatgccttgagcatttgcaactccagctgctggaggaacggagcaagcgatctgaagttgagcgtcaaaatgcaatgctgcaaaaccaagttacaatgctcatggacatgttacaggagaatgacgacgtagatgatgatgaaggtggagaggagccttgattttttcgttctttcttcaatagtaggaactagtcatatggacttttcttctggggagtattgttttattttgcatatacggttggcacaatatttattttgtaattttgagacttatgcggtcatgtgtgtgtataattagttcacatatatttcacaactagcataaattgtatactgtaaatcttcttaatgaaagtcaaccagaacaactctgcgctttgagctctattttgcttgcagctgacttttcgcttgaccaatcgatcaaagac

SEQ ID NO: 30 - protein, 208 aa, Coffea canephora
MEEPNKKVEQTLINGFSPVSSAPVFWKSRRRAVSVKYLDKPTENDADKPPETQENPTAEAMQEDSTPVVLSEKRKALFEPLEPMTNINGRRPSAEMLLPPPDFDAATYPKGWLIGKKRKLVNVDVVESMRRIAVQEMNRKDREIDGLNEQLEEDARCLEHLQLQLLEERSKRSEVERQNAMLQNQVTMLMDMLQENDDVDDDEGGEEP

SEQ ID NO: 31 - DNA, 3792 bp, Vitis vinifera
  source 1..3792: mol_type = genomic DNA
gaaagctttacaacaaggaacaaaggaacaagaaaaagaaggaacaaggataattctgagaattccaacttgcccaactcacctcctcgcttcttctcttcatttctctctctctctctccccctctctccttcaatggaccttcccaagaagcctgacgggaaccttgatggcttctccacagtctcctcctccacaagggttttctggaattccagaaggagatcaggtgtgtactgctttttccctggatttttgtttctattgttctgttttcttcaggaattatgtttccttagggtttatctagaaaaaaaaaaattgtccaattgaatggtggcggtggtggtggtgttgattttttggggacttgggtttctgggaggtgggtttcagacaaatctagagatacccatgatcccatacctggataaaattgagtcaactgaacctctgggttgaacttattttcctgggaaattggactttttaggaactggtttttgggaaataattttcttatggatttagagattcccatctaccccatacctgtgtctgtactcccctttgttgtttgggttttctgggaaactgggtttttggaagcgatttccagaggaatttagagattccctttaacccacatctttaccaaaacattttccttgtaattctccttgatgggttctccaatttcttgattgggtttacagaaatatgtcttaaatcttgaaatttgtggttgcaaagaggcttggaagactgagaactataaacaatgacttggcttatactccatatttagttggtcttgttggcctacccatcactttctaccttagtagcactattatcatgactgttacttctgcttttctattttcttaaggcaaccaaaagggatgagtcatcattgtggccaaaaatcacagaaaagtatttcttactttctcgaaatactttacaaaattacttcttatagagacagtatacagatgaataagatattggagaggcatttcaaagggataatccaacatttttcaaagcaaaatgtacaaactagggtgtgtggatggaggaataatagaaaaaatagattcaaggtgtgtgttgagcattttagtcatatccattaagagattagtgttgaattaagaaaatttagaggttatttgtttttttaatttaagtttcagattacaagggtaaaaagggagaattacttttatataaaacaaaaactacttttttactctaaatttacctggtgttggttgttagggcggttagcctctcgtggtttgggttctcatggagagtcataaggacttcattatggaaggttcttattaaaaaaaattaatacaaaattgtcttagaaaaagtataaattcttgtttggatacattttttttttttttaaaaagaacaaaaattaataacaatttttatgttaaaagtcaaacttttatacaaaaagttactttaaaaaattttgaagtttgatatagtaattttttttttaatatcttatgtttttttaaatagttttgagagggtattatttttttaatgggttaatttcattcacctatcttgaagttttggctaaatatatttagccctccatagatttgaaatttcatggtagggaagatatttgatgaaatttcaaactaatgaatattgcttgtatttaagtaaaatcttacgggtgaatgaaattaattattttttaatagttcttttattgaatatagaaaaatatacatatccaaacatatatttgaaaaataaataattttaaaaatgatttaaatctttgtgtaatttcatttaagacttaagtgaaaaaaataaaaattactatttagatttcagaccaaaaaaaaggccttagatttgggctatgtgttaagactaccataaaatatggtctttagctaaaaatgaaaatgtggcacttagacgactcaaaatgaaaaattgggtcacaccctcgcataaagctatatagaaattgtctcatgttatatattagaaattaaagggtttgtttggtaattattttttaaaacaaggaggaaaacacatttaacgaccaatttttttaaaatagaaaacaaaatgttttcaaaaaacatttttagtttgtttcggttgtttgcttgtttcttgaggattgttttaaaaaataattatataaatatgaaaaatgattaaaaatgaaactctaggtataaaagttatttctaaaacctatttaaaaacatagaaaataagtttaaaacatttcgggttccaaataaatttttgttttcatgaaaaatcttttaaaaattattcttaaaaattgttttttaaaactattttagaaaacacttccgaatggttgcaagggaaccttagtttggtatgccatgaacacttcaaactagcagccaaggtatcccataaccatgagatcaaaacttcgttttcctatgtgatggggaaaggggaacattccatgataacttcttttaagttgttaatgatagaactctacaccaaccatttcccactttgacctttgccacactcaatgattcatcaatgcttttgtgcaccaccttttggaaagctactgaaaagctaataattaggagcatgggtgccatgaaatcattaaattcattcacatagaattagggcttgtttggattgtttgcagaaactgaatggcttttactgtgttttacactccgtttggatgatacaactgttttgtctccctacagaacataaaacacaattaagtcattcaattttcgtgttactttcaaatggcccgtgtatgttatgttctttctggcaggaagcgggcggaatttagaaaaggttgcagaagataccagtgataatacacccaaaaaacaggatgaatctccgcctgaagagacgatgcaggacatttctgttttatctgagcgtaggaaggctctttttgaaccattggaacctttaactgggtcacgacccttagccgaatccttgctgcctccacctgacttcgactctgcaaactatcctcgaggttggctgataggaaagaagaggaagcttgtgaatgtggatgttgttgagagcatgaggagaattgctgtccaggaaatgaatagaaaggtgctctgttcttaacacctcacttctcatccaaaaccaccatcttagtaatggaatgaatgaaccatcacttgattgtgcttacaggaccgggaaataaatggcttaaatgggcagttagaagacgatgcaaggtgcttggaacacctccaagtccagctcctgcaagaacgcagcaaacgtgcagaggtagaaagagagaacttgatgctgaaagatcagttgtctatgctgatgaacatgttgcaggaacaggaggcaatggaaaatgagagcacagaagagcattaaaattgttgtgttgctttgtctgtttaattcttttgtatatctattcgtgggttcggaaacgaagaaccaccatagaaccataccgtatatactaggattgccaatgtagtttcttggtgctacaagtagcttgcatttgttattgtttgtaattgagtctttaatatcttgttaaagtattaagtttgggtaaattgtatcttatctgtgtgtgtatatttgccaacaacaacaaccagctcaaacaaggctgtgttgttgagacaactcaaagtgaaaactcctatttgccagatgatataaaggatcatcatcttctttgttgtgtca

SEQ ID NO: 32 - protein, 201 aa, Vitis vinifera
MDLPKKPDGNLDGFSTVSSSTRVFWNSRRRSGSGRNLEKVAEDTSDNTPKKQDESPPEETMQDISVLSERRKALFEPLEPLTGSRPLAESLLPPPDFDSANYPRGWLIGKKRKLVNVDVVESMRRIAVQEMNRKDREINGLNGQLEDDARCLEHLQVQLLQERSKRAEVERENLMLKDQLSMLMNMLQEQEAMENESTEEH

SEQ ID NO: 33 - DNA, 951 bp, Solanum tuberosum
  source 1..951: mol_type = genomic DNA
atgactataagcccaatcaatacacagttcacacaattcatattttgtatattatacatttatcatgctaagaaaatacttcgcctagtagccggtgtgaagaacttggaaacacctcaaaagcaagaagagtctccagctgatgaaacacctcaaaagcaagaagagtctccagctgatgaaacacctcaaaagcaagaagagtctccagctgatgaaacacctcaaaagcaagaagagtctccagctgatgaaacacctcaaaagcaagaagagtctccagctgatgaaacacctcaaaagcaagaagagtctccagctgatgaaacacctcaaaagcaagaagagtctccagctgatgaaaagatgcaggaatcccagccctctactgaactctcagagcgtagaaaggcactttttgaaccattggaaccggttacaaatgcaaatggccgtaggccgtcagctgaaactttgctacccccaccagactttgatgctgcatgttaccccaaaggttggctggctggaaagagacggaagcttgtaaatgtggatgttgttgaaagtatgcgaagaatcgctctacaggaaatgaacagaaaggtgatgtcctcaaaattaccatttgtttgctttcttctaatctacatgttctgttttggctaacctctttaaatgtcttcaagttctcgtcttgctcagttcaaattcaacagaaacactaatcatatgacaatgctgcaggatcgtgaaatcgatggtctgaacgaacagttggaagcagatgctcattgcctggaacatctgcaaatacagctgctagaagaaagaagcaagcgtgccgatgtagagaggcaaaatgctatgttgcaaagccagataaatgtgcttatggacatgtatcaggataacgatgacattgatgatgacggtacagatgattcttaa

SEQ ID NO: 34 - protein, 269 aa, Solanum tuberosum
MTISPINTQFTQFIFCILYIYHAKKILRLVAGVKNLETPQKQEESPADETPQKQEESPADETPQKQEESPADETPQKQEESPADETPQKQEESPADETPQKQEESPADETPQKQEESPADEKMQESQPSTELSERRKALFEPLEPVTNANGRRPSAETLLPPPDFDAACYPKGWLAGKRRKLVNVDVVESMRRIALQEMNRKDREIDGLNEQLEADAHCLEHLQIQLLEERSKRADVERQNAMLQSQINVLMDMYQDNDDIDDDGTDDS

SEQ ID NO: 35 - DNA, 2722 bp, Solanum lycopersicum
  source 1..2722: mol_type = genomic DNA
gttgagagaaatcacaaaaacccaggtaccattttgtcctatgtggaaataataataataaaataaggtgtgtgggagatagataggaacacaaaacaagaaaccaaacaccagcatcaccgtgtaaaactaaaaaacaacaaaatcatgtccgttaaaaaattatgctttctctctctatgcttatttttcccaaccatatcttatttactttgtcaaacaaaaaaggggctcaagagttgggtaataaacgtttctttgccttgcttacacctacaacttacttcaactcttacgctatcaattctctctcttatctctttgtaccttataataaaaaagttctggtttttattttgtttttgttaaaaaaaactttatttatgtgtgtgtgttttttgaaatttgaaagttgattatggaggtaaggcagcagcagaagatggaaggatttcttgagggattttcacctgtttcttcaactcctgttttatggaagtctagaaaaagatctggtaatatttctttgttctttttctctgattttcaatttagtactagtattgcatgtagctacagtgatttattgaaatatggggttgattatttgtgctataactagatctatttctagaaatgattagaaaatacgcagcaaagctagaatttgaagtttcgattatagtcattttaagtcgttgagttctgaattaatggttttattagttgttgggtttcacagtttccggttaagttgaaagtagaggataattttgtccaatattagctagatttagtggcgaatttgccgacacgtcatttctagctaataaataagttcgattttcgaataaaaaacattttttttttttttgtaaatttatccgtagcttattaggtaaccattaataaagcatcgatttttagtgattttggttgtctttgtcatgatgagtgtgttttgattcattcattacattacatgtttcttctgcataattttacttatttgttaaggaatttgcctgtataagctaaacttgattaccactccaatattttatttttcaaagactaatctattattccacaccggatattgtgtagaaatagtgatttggccctgcattgttgactttgtattttttttaatgtacatgttctttttcccttaagcggactccttaatttatttggaaattcttcgagatggattagaatatgaaagatgacttgtggagctttagaaagactgattgaaaagaaaaaagatccttttctaagaaaggttacatataatatataattaaagacggtataatcattccataattacagaggtcgaaacaaatgtgtttagatagaatctcaaactcgaatctgaaaagtttaaatcttggatccacctttgctcgatagtgtttttgtgaatgctacatcaaatagcagacttgtttcttcactgatcaaggagaagatttgtagttagtgagctttttaattacacaagactggctcatgctatttgaacttgaaccagtcaacaattttcgttgagtcgaaggtctatcagaaacagtctctctacctcccaaggtgtaggggtaaggcttgcgtaaccctccccagaccccacttatggatttatattgggtatgttgtagttgttgaaatagtcaacaatttctgaacatcactaatattttgtttggagaacatacttctgatattttagtcctgtttaatgtcttgttccataaagataatagagtgatgactataagcccaatcaatacacagttcatacaattcatattttgtatatcatacatttatcatgctaaggaaatgcttcgcctagtagccggtgtgaagaacttggaaacgcctcaaaagcaagaagagtctccagctgatgaaacacctcaaaagcaagatgagtctccagctgatgaaaagatgcaggaatcgcagccctctactgaactttcagagcgtaggaaggcactctttgaaccattggagccggttacaaatgcaaatggccgtaggccatcagctgaaactttgctacccccaccagactttgatgctgcatgttaccccaaaggttggctggctggaaagagacggaagcttgtaaatgtggatgttgttgaaagtatgcgaagaatcgctctacaggaaatgaatagaaaggtaatgtcctcaaaattaccatttgtttactttcttctaatctacatgttttgttttggctaaagctcttaaaatgtcttgctcagtttaaattcaacagaaacactaaccatatgacaatgctgcaggatcgcgaaatcgatggtctgaatgaacagctagaagcagatgctcaatgcctggaacatctgcaaatacagctgctagaagaaagaagcaagcgtgctgatgtagagaggcaaaatgctatgttgcaaagccagataaatgtgcttatgaacatgtatcaggatgacgatgatattgatggtgacggtacagatgactcttaatcagtcattttctttattcttttgtagatttcgttagacaataataggacagatatagaagaaggttgttgtgctttcaagatgtaaaatatatatttgcgagtaccacctgtgtgttcgcaatattatttactgtttaaaagctgtgtaagacgttggtagttccttttatttgatccatcattcctcgc

SEQ ID NO: 36 - protein, 241 aa, Solanum lycopersicum
MSVKKLCFLSLCLFFPTISYLLCQTKKGLKSWVRQQQKMEGFLEGFSPVSSTPVLWKSRKRSAGVKNLETPQKQEESPADETPQKQDESPADEKMQESQPSTELSERRKALFEPLEPVTNANGRRPSAETLLPPPDFDAACYPKGWLAGKRRKLVNVDVVESMRRIALQEMNRKDREIDGLNEQLEADAQCLEHLQIQLLEERSKRADVERQNAMLQSQINVLMNMYQDDDDIDGDGTDDS

SEQ ID NO: 37 - DNA, 2780 bp, Manihot esculenta
  source 1..2780: mol_type = genomic DNA
atggaaaaaaagaaagagtacagtaataaagatggcttctttccagtctcttctcctagggtctcttggaaacctccaaggacatcaggtacttgtttctcttctctgtgtttgttttccaagaaaaagtaatacaaaagagaaaataaagggaggaaatgttgaaatcagaaggttttatgatattttttaactagaagagcatatataagagagctgcatctgggtatctgaagtgaagaattttcattgttaactgtttgggtttgaaaatctctactgaaattggataagtgtaccaattcatgaatctttagctagcttcgtcaaaagcaagatccttgaatgtgcttggagttaacgtgcaagttgtggattctgtcgccagagtcccaggggaagagacgacgatacctgagagagagagagagagagagagagagagaggtagaagaggtagaacagcaatttgctgttggttgctgttcagtctgtcaacctcaacattgtccatcctccatcttttcattcaattaaattaatttcaattttatttaattagtttttaagttttgaaaattaagattgttagtatatatttatcttttaactagaaaattaaattatttgaaaagaaataaattcataagtgatctgattttgttagtatttaattaattaaataattttttcgtcatttctacgtaaaataaataagggtaacatatgaaaataaatacattcattttttcaatcatcaacggtttcaaacaatataatttaaatgaacagaaaattactattagatttttaaaaattaattaagttatccatattttaaaatacttaattaaatcatttttatatcctataaattaaatataggtatttaaaattataggaattagatatataataaaaattataggaattaaataaaattaatatttaagatatttaataattcttttataaaaaaaaactaaaaaatttaattttatatgatatataaatatgaaaaattactatttaatttttatagtatatgagagtttctcacgttgatttttttattttaaaaagtatattaaaatatttataatattttaaaaaaattatttattagtatttctattgattttaatcattaaatattgtaaaaaaatttaaaatattactgatacaaaatgattaattaatatatttttttaaaatttgaaagatgagttaataaattttttaaaagtataaaaactgaatagtgaaataattaattgtaaaattaatgaatggactaattagtaggttttttaaaatataaaaaatattttaatatatccttttaaaattaagacactaagtaccgtatcataaaaattaagtaataattatttataaaaatattttaattaaataattttaaattaaaaataaattagtaaatttttaaaaatttaataataattttctgtaaataaatcgaagaagtatccaaatatatgattttcttataaagtgattggaattgattaattccttgaataaaatttaattatgttgcgttataagaatcatttcaaagagttgtgattatcttatttatattctaattaataccacttatccctttcattatgttcaatgtataaaaatatattttaaaagtttattattcttaatcagtttcaattaagtggtagcttttctaaatatttccagacagccaaattcaagaaggattctttttcaggctattagtctatatttatacacataatttcaatctaatttttatttaaatcagattcatacagatttaatatataaaaattattattgttatttattgtcatattacataattttatattttatttattttttatttgtataatatatctgatttagatttgtatcctattaagtcagacacacgtacatgcacccattttaattaatcattgtaacttaggcatttttgtttgttaaattttcatagcatcaacttttcaatgggtgcacttccatacaataaatttgcattttctccttctagtttgcaactgctggtgctgctgaaagcaagtaaacccattacaattcttatgctgttgtgcttgtaaatttttcatgtctaaaattgttggaacttgaatggtaactcctttccaacagctagcgggaggagtttatgcagtgtaactgctaatgaaactcccagcaaaatggaagaatcttccaatgatgaaaagatgcaggagccagatacacttcctgtgctttctgagaagcgaaaggctctctttgaaccattggaaccagtaaccaatatcaatggcaaacgaccatcagccgagtcccttcttcctccaccagattttgactcagcaagctatcccaaaggttggctaattggaaagaagcgaaagcttgttaacatagatgtcgtcgagagcatgaggaggattgccattcaggaaatgaacagaaaggtatttgcttcccattcattgcaggttgcatgtgcacaacgtgtatatatatatatatatataatcattggatgttcgtttcaggaccgggaaattaatggcctaaatgagcagttggaagaggatgcaaggtgtctagaacacctgcaactccagcttctgcaagaacgaagtaaacgtgccaatgttgagagagagaacgcaatgctgcaagaccaaatatccatgctgatgaacatgctagaggaaaatgaacaaatgggtgatgaaggccctgatgaaccttaa

SEQ ID NO: 38 - DNA, 4590 bp, Manihot esculenta
  source 1..4590: mol_type = genomic DNA
tgatggctttgacttgtttgtattgcatattttcttaaaaaattaaaatcaaaagttaaggaggagtatcgttattggaaaactgtcaactgtctgctcaactttaaatccttaggtcggaaataaagggtgtaacggagcagaagtcgtgccagaatcaccaaaggtgtctgttaaaaaaaattgttcataaaagaattaaggatggtggtgatggttttaaaatttaattttaactaagaatattaaaatatatattttttaataaataaaattataaaatatatcgatcataatatatatttataaattaatttactactaaataatttctcaactatttataaatatttaattaaatatataattattttaaattttaaatatttataaatattaaataatttatatggcggatgaatctaagtaggctgaagtagtgcaggcaggacagtggaagcatggaaattgcagctaactttttataaagagattccaaactccaagaaacttcctcacttcgagaaaaatccgtttatgctctaggggatatgctcccaacaatttctttttattttttatttttttttctataaaatattacattttatattttgtattttttaaaatcagcaaaaaaacagaaagacatttaaaaaaaaaaaaaaataacaaaaacaaggatggagttttacatagaaaaggcaagctaaatgggacccatacacccaactgctggcttaaaatcttcgacagaaaatccaaatcccaagcgttgagaagctttgatggtcccggtcaccgttctcatttccttgtagctgaagtctcccaaaactatcttctctctcagaaaatatcgatttttatgttggattcttgattattcaagctcctctgctatggaaaagaagaaagattacagtaataaggatgggaagaaggtgttggatgggcttttagatggcttctctccagtctctacgcctagaatcttttggaaatctcgaaggagatcaggtaatattttgtttgttttgattcaacttgctgtttctcttctctttctgtttgttttccgagaaaaaacaataacaaaggaatactagagaaaagagaatgttgaattcagcatggtttaatccaataaacccatgtctagggatctgatatgagtgaagaatattttcattttttctttttggattgggtttgtgagatttctcttcaaattggtcaattctacaatttttgaaactttagttagtagtatcaaaagcaagattatcatttgatttgcttaatttcttggaataatttcataatttcataagttgttaattgtgcttcaacaaatcgagggaaagaggcagcaatagctttgacatttttgttggttagagagagaacagtaattctatgactgtctgctagagtattttctttgctgttatatcaattttaatgttaggttagctcaccattataagtttaattttaatttggaaaaaaaataattttatttttttttaattttatccaaagattaagaaaacccattttttaattttcttgatttttcatttacgtttaaattaaaaattaaaaatagacaaattgagcatttcaatgcacagtgaaattcagtggtaagctgtctctgtcatattgaccatggaaggtctcgtagtgttatgctaaaatctctgcccctgcttcaatttttttcctgcatttatctatagatttttttggataattgtaattatttgaaataagatggacatggtgcaccctctttccaccatcaaatgaaaattttaactgattatccaagactctctctccattttattggttgatgattataataattaataattacttgataattataataattaataattaattaaagagagaaaataataattaatataaaaaaatacatttcaatgagaagatggagaatattagatggacacttaaagttagaaacttaaataactaattataattagaataaaaatgagtttgggataattttcggcagttatgtgaggttaaggtttcaattctcctagatgaaacaaatatcactgagagtaccctactctttaataagcggatccaacccggtgtggatacgacttagtttagtgggcatgttccttcttgtcctcaagaactctgagtcaaatagttacccttcaaattcggactagccgatcattataagccattggtccaaatgcttttttttttttgagaaaaaaaaaaaagaaaattgtttgccaattcaacaatgtccatcctgcagcaattttagttgacaaattctaatagctcttaccccttccaacttagcagttgagcttggtggcttgttttagcggtaacttgtcatgcaggaagaaacatgtctgtgatcatataaggcaggaaaagtagaagaatcaataatatgtgaaggaaagaagagtactgaatcaatgaaaccgtctgtttgtttggaaggattaacgggagaaaatgcagatgaggttgtggtggaatcattttatcatcaacggatcaataatgtatttttgtttaaattacagttttcctatcatttcacttgatagcttcttcaccttattcaacggatgcattttcatcccatgtattttgtatttgcatttctcctccagtggtactgctcaaagcagcatcatataaaggccacccattacatttcttatgctgttgttttgtaaacttgccctatctaaaattgttggaagtagaatggtaactcatttccaacagctagcgggaggaatttagacaaggtaacagacgatacagctaaagaaactcctagcaaacaggaagaaatttccaatgatgaagacatgcaggagcccaaagaacttccagaactctcagaacggcgaaaagctctctttgaaccattggaacctgtgacaaatatcaatggaaaacgaccttcagctgaatcccttctacctccacctgattttgactcagcaagctatcccaagggttggctaattggaaagaagcggaagcttgttaatgtagatgttgttgagagcatgagaaggattgctgttcaggaaatgaacagaaaggtattgattctcaaacatggattgtaggtttcacatgcataatacatacacaatcattggatatttttgtaggaccgagagattaatggcctaaatgagcagttggaagaggatgcgaggtgtttagaacacctgcaactccagcttctccaagaacgaagtaaacgtgctgaggtagagagagagaatgctatgttgcacgaccaaatatccatgctgatgaacatgatagaggaaaatgaacaaatgggcgatcaaggtgccacagatgagggccctgatgagccttaaaagatagctttgcttctcttttttctttatattttattcttttataggttggtttgaatgcatggatgtcctgatagtttgttggaagtcgtattaccttgtgcatgatggatgatgtttatagttttgagtatcgcatttgtaggcatatacatcaaaataatttgtccatttgtaaatcgcctgcttgcccaacaacatttttttttatcaattattctgtgtttatattgttcatgttttgctcatgacattggaaattaagtagttaaaaatgcatatcgagctttgttcgcaataatagagaaagaataaaaagaacaaaaaagttcaatgtcattctcgtaagatcagacaagacaataataaattaataaatactgcaaatttgcaatattgtggccaaactgaattattaaaatatcagaatagaggggcaaaagggcggatgctacattgaaaacccaatacgctcgagtctaattacgatgagttgggactacagaaagctgtataaagaaagcaccaccaaactccaggaataaacatgcgaggatccttcatcaatacaaaatttcaaaatccccaagcttctacgatttaaagtcactgcaaaacataatatccacagaagtcctgtccacgatcacttgaaaatgatgcaacacactggaccttcccctacatattatgcaaaaattgggggagggaggcaatccttgggagattaagcagtagctccccaactgaatccttccttgacatggacggtggctgtttgcagctggaaacgctattagactgatcctcggacactggaaaaccctccacaaatttattctggcaggtcgctgcgctgagggattcagttccatcaattctctcattaacgtctgcttcaagatcaatgcaacccttagcctgcaaattcagtgctgatccaggatctctctgcagtaaacaacaaagagaattgacccttgacatgaggcactgctcgtctgatgcagatgtaagttgcgtgtcactaagcaagtattgggtaatttcccccagaatctctctgttcatcgggtcgccatttgaaatataaggatttccagatatctgttctgaaatgcattgtccaaggtggttcactaggtcgctcattgacatggat

SEQ ID NO: 39 - protein, 202 aa, Manihot esculenta
MEKKKEYSNKDGFFPVSSPRVSWKPPRTSASGRSLCSVTANETPSKMEESSNDEKMQEPDTLPVLSEKRKALFEPLEPVTNINGKRPSAESLLPPPDFDSASYPKGWLIGKKRKLVNIDVVESMRRIAIQEMNRKDREINGLNEQLEEDARCLEHLQLQLLQERSKRANVERENAMLQDQISMLMNMLEENEQMGDEGPDEP

SEQ ID NO: 40 - protein, 220 aa, Manihot esculenta
MEKKKDYSNKDGKKVLDGLLDGFSPVSTPRIFWKSRRRSASGRNLDKVTDDTAKETPSKQEEISNDEDMQEPKELPELSERRKALFEPLEPVTNINGKRPSAESLLPPPDFDSASYPKGWLIGKKRKLVNVDVVESMRRIAVQEMNRKDREINGLNEQLEEDARCLEHLQLQLLQERSKRAEVERENAMLHDQISMLMNMIEENEQMGDQGATDEGPDEP

SEQ ID NO: 41 - DNA, 1050 bp, Brassica napus
  source 1..1050: mol_type = genomic DNA
atggagaaagggaatggatttgagggagggaataggaagaaaaagaaggagacagctaacgatggatttgtcggtggttttttccctgtctctaccaccaagatcgcgtggaagtcaagaaaaagatcaggttctcctctgattcttgttttccagtaatttttatctgtcccttcatttttatggtctgaaagattttaggctttaaacagaaacttatcaattgttaggagccatgcttgaaaattagctctctgtgaactgttctctcaaagtgtctctgttcagagatctagagtctagacaggtagcttttgttactggtctcttcacttcatctctctctgtcttaagcttggaacattaaaaggttttagctttagtttcggtttgatccggttatatgcacgtttggaatataaagcattagcaacttctattacagcatctgtgaatccagacaaagaatctgaagctgctatggaactcacaccagagaaagatgagacaacaacagcaatggaaactgagaaagttggagaaccaatgaccacaactcctgttctgtccgagaaaagaaaagctctgtttgagccactcgaacccattacaaacttgaacggaaagcgacctacagatgctgattccctcttgccaccgcctgatttcgagtctgcaaactatcctaaagggtggttgatcggtaagaagaggaagctggtgaatgtcgatgtggttgagagcatgagaagaatcgctgtccaagaaatgaacagaaaggtaaacataaaacaatggcagaataatctttgttcttgttggaaattttttgataaaatagagattgtgggacaggatcgagagatagatgggttaaacgagcagttagaagaggactcgcgttgcttagagcatctgcaacttcagctgctacaagagagaagcaagagaacagagattgaaagagagaacacaatgctgaaagagcaagttgatatgcttgtcaacatgatccaacaagacgaagaagaagtaccagaagaaccctag

SEQ ID NO: 42 - DNA, 893 bp, Brassica napus
  source 1..893: mol_type = genomic DNA
atggagaaaggagctggattcgagggagacaatatgaaaaagaagaagacagttggtgatggttttgtcggcggttttttccctgtctctaccaccaagatcgcgtggaagtcaaggaaaagatcaagtacttttctctctcctctgtgtctctctcctctgtttcttagttttctcacatctctcttagtctcggaatcaaaaggctttagctttgattttggtctgatcccattatatatgcattagcattaacaacttagattgcagcatctgtgaactcagacaaagcactggagactgctatggaggtcacaccagagaaggatgagtcaacaacaacagcaatggaaaccgataaagctggggaaccaatgaccaccacaacccctcctgttctgtccgagaaaagaaaagctctgtttgagccactcgaacccatcacaaacttgaacggaaagcgaccaacaacagatgctgattccctcttgccaccgccagatttcgagtctgcaaactatcctaaaggctggttgatcggtaagaagaggaagctggtgaatgttgatgtggttgagagcatgcgaagaatcgctgtccaagaaatgaaccgaaaggtaaaaaagactgttgttgtgtgtttcttttttcttgttggactattttgttctgattaaaagaggattgtgggacaggatcgagagatagatgggttaaacgagcagctagaagaagactcgcgctgcttagagcatctgcaactccagctgctacaagagagaagcaagagaacagagattgaaagagagaacacaatgttgaaagagcaagttgatatgcttgtcaacatgatacaccaagaagacgaagaagaagtagcagaagaaccataa

SEQ ID NO: 43 - DNA, 1043 bp, Brassica napus
  source 1..1043: mol_type = genomic DNA
atggagaaagggaatggatttgagggagagaatacgaaaaagaaggagcagacagctaatgatggatttgtcggtggttttttccctgtctctaccaccaagatcgcgtggaagtcaagaaaaagatcaggttctcctctgcttcttgttttctcgtaatttttatctgtcccttcatttttatggtctgaaagatttgaatattagctctctgtgaactgttatctcaaagtgctctgttcagagatctagacaggtagcttttgttacagtcttcaattgaactctctctctctctctctctctctctctctctctcaagcttggaacattaaaaggctttagcttttgattgaaaaaaaaaagaaggctttagctttagtttcggtctgatccggttatatgcgcgtttggaatataaagcattaacaacttctatttgcagcatctgtgaatccagacaaggcaccagaagctgctatggaactcacaccagagaaggatgagacaacaacagcaatggaaacagacaaagttggagaaccaatgaccacaactcctgttctgtccgagaaaagaaaggctctgtttgagccactcgaacccattactaacttgaacggaaagcgaccaacagatgctgattcgctcttgccaccgcctgatttcgagtctgcaaactatcctaaagggtggttgatcggtaagaagaggaagctggtgaatgttgatgtggttgagagcatgcgaagaatcgctgtccaagaaatgaacagaaaggtaactgattgatggtgtgtttcttttttcttgttggaaaaaatttttgattaaaagggattgtgggacaggatcgagagatagatgggttaaacgagcagctagaagaggactcgcgttgcttagagcatctgcaacttcagctgctacaagagagaagtaagagaacagagattgaaagagagaacacaatgttgaaagagcaagttgatatgcttgtcaacatgatacaacaagatgaagaagtaccagaagaaccctag

SEQ ID NO: 44 - DNA, 935 bp, Brassica napus
  source 1..935: mol_type = genomic DNA
atggagaaaggcgctagatttgagggagacaatacgaaaaagaagaagacagttggtgatggatttgtcggcggttttttccctgtctctaccaccaagatcgcgtggaaatcaagaaaaagatcaagtacttcttctctctctgtctcctttgtttctttgttttctcagattttttttgtcttttcattttatcgtctgaacgatttaggctgttaaagtcatgcttgaatacttagctctctctcggttaactgtttcatcaaaggctttttctctctgtctttagctttagttttagcattaacgacttagattccagcatctgtgaactcagacaaagcaccgggagatgctatggaggtcacaccagagaaggatgagtcaacaacaacaacagcaatggaaaccgataaagctggggaaacaatgaccaccacaacccctcctgttctgtccgagaaaagaaaagctctgtttgagccgctcgaacccatcacaaacttgaacggaaagcgaccaacaacagatgctgattccctcttgccaccgccagatttcgagtctgcaaactacccgaaaggctggttgatcggtaagaagaggaagctggtgaatgttgatgtggttgagagcatgcgaagaatcgctgtccaagaaatgaacagaaaggtaaaaaagactcttgttgtgtgtttcttttttcttgttggtaaattttgttagattaaaagaggattgtgggacaggatcgagagatagatgggttaaacgagcagctagaagaagactcgcgctgcttagagcatctgcaactccagctgctacaagagagaagcaagagaacggagattgaaagagagaacacaatgctgaaagagcaagttgatatgcttgtcaacatgatacaccaagaagaagaagaagaaccctag

SEQ ID NO: 45 - protein, 219 aa, Brassica napus
MEKGNGFEGGNRKKKKETANDGFVGGFFPVSTTKIAWKSRKRSASVNPDKESEAAMELTPEKDETTTAMETEKVGEPMTTTPVLSEKRKALFEPLEPITNLNGKRPTDADSLLPPPDFESANYPKGWLIGKKRKLVNVDVVESMRRIAVQEMNRKDREIDGLNEQLEEDSRCLEHLQLQLLQERSKRTEIERENTMLKEQVDMLVNMIQQDEEEVPEEP

SEQ ID NO: 46 - protein, 223 aa, Brassica napus
MEKGAGFEGDNMKKKKTVGDGFVGGFFPVSTTKIAWKSRKRSTSVNSDKALETAMEVTPEKDESTTTAMETDKAGEPMTTTTPPVLSEKRKALFEPLEPITNLNGKRPTTDADSLLPPPDFESANYPKGWLIGKKRKLVNVDVVESMRRIAVQEMNRKDREIDGLNEQLEEDSRCLEHLQLQLLQERSKRTEIERENTMLKEQVDMLVNMIHQEDEEEVAEEP

SEQ ID NO: 47 - protein, 218 aa, Brassica napus
MEKGNGFEGENTKKKEQTANDGFVGGFFPVSTTKIAWKSRKRSASVNPDKAPEAAMELTPEKDETTTAMETDKVGEPMTTTPVLSEKRKALFEPLEPITNLNGKRPTDADSLLPPPDFESANYPKGWLIGKKRKLVNVDVVESMRRIAVQEMNRKDREIDGLNEQLEEDSRCLEHLQLQLLQERSKRTEIERENTMLKEQVDMLVNMIQQDEEVPEEP

SEQ ID NO: 48 - protein, 220 aa, Brassica napus
MEKGARFEGDNTKKKKTVGDGFVGGFFPVSTTKIAWKSRKRSTSVNSDKAPGDAMEVTPEKDESTTTTAMETDKAGETMTTTTPPVLSEKRKALFEPLEPITNLNGKRPTTDADSLLPPPDFESANYPKGWLIGKKRKLVNVDVVESMRRIAVQEMNRKDREIDGLNEQLEEDSRCLEHLQLQLLQERSKRTEIERENTMLKEQVDMLVNMIHQEEEEEP

SEQ ID NO: 49 - DNA, 1074 bp, Brassica oleracea
  source 1..1074: mol_type = genomic DNA
atggagaaagggaatggatttgagggagggaataggaaggagaagacagctaatgatggatttgtcggtggttttttccctgtctctaccaccaagatcgcgtggaagtcaagaaaaagatcaggttctcctctgcttcttgttttctcgtaatttttatctgtcccttcatttttatggtctgaaagatttgaaaattagctctctgtgaactgttatctcaaagtgctctgttcagagatctagacaggtagcttttgttacagtcttcaattgaactctctttctctctctctctctctttctctctctctctctctctctctctctctctctctctctctctctcaagcttggaacattaaaaggctttagcttttgattgaaaaaaaaaaagaaggctttagctttagtttcggtctgatccggttatatgcgcgtttggaatataaagcattaacaacttctatttgcagcatctgtgaatccagacaaggcaccagaagctgctatggaactcacaccagagaaggatgagacaacaacagcaatggaaacagacaaagttggagaaccaatgaccacaactcctgttctgtccgagaaaagaaaggctctgtttgagccactcgaacccattactaacttgaacggaaagcgaccaacagatgctgattcgctcttgccaccgcctgatttcgagtctgcaaactatcctaaagggtggttgatcggtaagaagaggaagctggtgaatgttgatgtggttgagagcatgcgaagaatcgctgtccaagaaatgaacagaaaggtaactgattgatggtgtgtttcttttttcatgttggaaaaaaattttgattaaaagggattgtgggacaggatcgagagatagatgggttaaacgagcagctagaagaggactcgcgttgcttagagcatctgcaacttcagctgctacaagagagaagtaagagaacagagattgaaagagagaacacaatgttgaaagagcaagttgatatgcttgtcaacatgatacaacaagatgaagaagtaccagaagaaccctag

SEQ ID NO: 50 - DNA, 990 bp, Brassica oleracea
  source 1..990: mol_type = genomic DNA
atggagaaaggcgctagatttgagggagacaatacgaaaaagaagaagacagttggtgatggatttgtcggcggttttttccctgtctctaccaccaagatcgcgtggaaatcaagaaaaagatcaagtacttcttctctctctgtctcctttttttttttttttttttttttttttctctctgtctcctttgtttctttgttttctcagatttttttgtcttttcattttatcgtctgaacgatttgggctgttaaagtcatgcttgaatacttagctctctctctcggttaactgtttcatcaaaggctttttctctctgtctttagcttcagttttagcattaacgacttagattgcagcatctgtgaactcagacaaagcaccgggagatgctatggaggtcgcaccagagaaggatgagtcaacaacaacaacaacagcaatggaaaccgataaagctggggaaacaatgaccaccacaacccctcctgttctgtccgagaaaagaaaagctctgtttgagccgctcgaacccatcacaaacttgaacggaaagcgaccaacaacagatgctgattccctcttgccaccgccagatttcgagtctgcaaactacccgaaaggctggttgatcggtaagaagaggaagctggtgaatgttgatgtggttgagagcatgcgaagaatcgctgtccaagaaatgaacagaaaggtaaaaaagactcttgttgtgtgtttcttttttcttgttggtaaattttgttagattaaaagaggattgtgggacaggatcgagagatagatgggttaaacgagcagctagaagaagactcgcgctgcttagagcatctgcaactccagctgctaaaagagagaagcaagagaacggagattgaaagagagaacacaatgctgaaagagcaagttgatatgcttgtcaacatgatacaccaagaagacgaagaagaagtaccagaagaaccctag

SEQ ID NO: 51 - protein, 216 aa, Brassica oleracea
MEKGNGFEGGNRKEKTANDGFVGGFFPVSTTKIAWKSRKRSASVNPDKAPEAAMELTPEKDETTTAMETDKVGEPMTTTPVLSEKRKALFEPLEPITNLNGKRPTDADSLLPPPDFESANYPKGWLIGKKRKLVNVDVVESMRRIAVQEMNRKDREIDGLNEQLEEDSRCLEHLQLQLLQERSKRTEIERENTMLKEQVDMLVNMIQQDEEVPEEP

SEQ ID NO: 52 - protein, 225 aa, Brassica oleracea
MEKGARFEGDNTKKKKTVGDGFVGGFFPVSTTKIAWKSRKRSTSVNSDKAPGDAMEVAPEKDESTTTTTAMETDKAGETMTTTTPPVLSEKRKALFEPLEPITNLNGKRPTTDADSLLPPPDFESANYPKGWLIGKKRKLVNVDVVESMRRIAVQEMNRKDREIDGLNEQLEEDSRCLEHLQLQLLKERSKRTEIERENTMLKEQVDMLVNMIHQEDEEEVPEEP

SEQ ID NO: 53 - DNA, 1017 bp, Brassica carinata
  source 1..1017: mol_type = genomic DNA
atggagaaagggaatggatttgagggaggggataagaagaagaagaagaagacagctggtgatggatttgtcggcggttttttccctgtctctactaccaagatcgcgtggaagtcaagaaaaagatcaggttctcctctctctctcccttcctttttatggcctgaaagatttacgctttaaaagagaaacttatcaattgccttaagggcccatgcttgaaaattagctctctgtgaactgttatctcaaagtgcctctgtccagagatctagacaggtagcttcatttttagttatctctcagtctttaagcttggaacattaaaaggtttttttagctttggtttcggtctgatccgttcgttatatgtgcgtttggaatataaaatcattagcaacttggatttgcagcatctgtgaacccggacaaggcaccagaagctgctatggaggtcacaccagagaaggatgagacaacagcgatggaaaccgagaaagatggggaaccaatgaccacaactcctcctgttctgtccgagaaaagaaaagctctgtttgagccactcgaacccattacaaacttgaacggaaagcgacctacagatgctgattccctcttgccacctccagatttcgagtctgcaaactatcctaaaggctggttgatcggtaagaagaggaagctggtgaatgttgatgttgttgagagcatgcgaagaatcgctgtccaagaaatgaacagaaaggtaaaaacacaaaacaaaacacaatgcagttttttgctggaagtttttgattaaaaaggaatgtgggacaggatcgagagatagatgggttgaacgagcagctagaagaggactcacgttgcttagagcatctgcaacttcagctgctacaagagagaagcaagagaacagagattgaaagagagaatacaatgctgaaagagcaagtcgatatgcttgtcaacatgatacaacaagatgaggaagaagtagtagcagaagaaccatag

SEQ ID NO: 54 - DNA, 1045 bp, Brassica carinata
  source 1..1045: mol_type = genomic DNA
atggagaaagggaatggatttgagggagagaatacgaaaaagaaggagcagacagctaatgatggatttgtcggtggttttttccctgtctccaccaccaagatcgcgtggaagtcaagaaaaagatcaggttctcccctctctctctctcgcctcagtttcttgttttctcgaaattcttatctgtccattcattttcatggtctgaaagatttaggctttaaacagaaacttatcaattgttaagagccatgcctgaaaattagccctctgcgaacttatttctcaaagtgtctgtctacagtctagacaggtagcttttgttactggtcttcacttcatctctctctgtcttaatcttagaacattaaaaggttttagctttagtttcggtttgatccggttatatgtgcgtttggaagtaaaagcattaacaacttctatttgcagcatctgtgaataaggcaccagaagctgctatggaactcacaccagagaaggatgagacaacaacagcaatggaaaccgacaaagttggagaaccaatgaccacaactcctgttctgtccgagaaaagaaaggctctgtttgagccactcgaacccattactaacttgaacggaaagcgaccaacagatgctgattcgctcttgccaccgcctgatttcgagtctgcaaactatcctaaagggtggttgatcggtaagaagaggaagctggtgaatgttgatgtggttgagagcatgcgaagaatcgctgtccaagaaatgaacagaaaggtaaatgattgatggtgtgtttctttcttcttgttggaaaatttttttgattaaaagggattgtgggacaggatcgagagatagatgggttaaacgagcagctagaagaggactcgcgttgcttagagcatctgcaacttcagctgctacaagagagaagcaagagaacagagattgaaagagagaacacaatgttgaaagagcaagttgatatgcttgtcaacatgatacaacaagatgaagaagaagtaccagaagaaccctag

SEQ ID NO: 55 - DNA, 976 bp, Brassica carinata
  source 1..976: mol_type = genomic DNA
atggagaaaggcgctagatttgagggagacaatacgaaaaagaagaagacagttggtgatggatttgtcggcggttttttccctgtctctaccaccaagatcgcgtggaaatcaagaaaaagatcaagtacttcttctctctctgtctcctttttttttttttttctctgtctcctttgtttctttgttttctcagatttttttgtcttttcattttatcgtctgaacgatttgggctgttaaagtcatgcttgaatacttagctctctctctcggttaactgtttcatcaaaggctttttctctctgtctttagcttcagttttagcattaacgacttagattgcagcatctgtgaactcagacaaagcaccgggagatgctatggaggtcgcaccagagaaggatgagtcaacaacaacaacaacagcaatggaaaccgataaagctggggaaacaatgaccaccacaacccctcctgttctgtccgagaaaagaaaagctctgtttgagccgctcgaacccatcacaaacttgaacggaaagcgaccaacaacagatgctgattccctcttgccaccgccagatttcgagtctgcaaactacccgaaaggctggttgatcggtaagaagaggaagctggtgaatgttgatgtggttgagagcatgcgaagaatcgctgtccaagaaatgaacagaaaggtaaaaaagactcttgttgtgtgtttcttttttcttgttggtaaattttgttagattaaaagaggattgtgggacaggatcgagagatagatgggttaaacgagcagctagaagaagactcgcgctgcttagagcatctgcaactccagctgctaaaagagagaagcaagagaacggagattgaaagagagaacacaatgctgaaagagcaagttgatatgcttgtcaacatgatacaccaagaagacgaagaagaagtaccagaagaaccctag

SEQ ID NO: 56 - DNA, 939 bp, Brassica carinata
  source 1..939: mol_type = genomic DNA
atggagaaagaaggtgctggatttgagggagacaatatgaaaaagaagaagacagttggtgatggatttgtcggcggttctttccctgtctctaccaccaagatcgcgtggaaatcaaggaagagatcaagtacttcttctctctgtttctctctctcctcagtttcttgttttctctgtcctttcatttttttgtcggaaagatttgagcttttaggagaaacttgtcaattgttaaagccaccatgcttgaatatttagctctctatgtgaactgtttcatcgaagtctctgttacaaatttgttagcagcatctgtgaaccctgacaaggcaccggatgatgctatggaggtcacgccagagaaggatgagtcaacaacaacaacaatggaaaccgataaagctggggaatcaatgaccaccacaactcctcctgttctgtccgagaaaagaaaagctctgtttgagccactcgaacccattactaacttgaacggaaagcgaccaataacagatgctgattccctcttgccacccccagatttcgagtctgcaaactacccgaaaggctggttgatcggtaagaagaggaagctggtgaatgttgatgtcgttgagagcatgcgaagaatcgctgtccaagaaatgaaccgaaaggtaagaaaaggaagctgcttgtgtgtttctttgttctttgttgggaaattctgttctgattaaaagaggattgtggggacaggatcgagagatagatgggttgaacgagcagctagaagaggactcacgttgcttagagcatctgcaacttcagctgctacaagagagaagcaagagaacagagattgaaagagagaacacaatgttgaaagagcaagtcgacatgcttgtcaacatgatacaccaagaagacgaagaagaagtagcagatgaaccatag

SEQ ID NO: 57 - protein, 220 aa, Brassica carinata
MEKGNGFEGGDKKKKKKTAGDGFVGGFFPVSTTKIAWKSRKRSASVNPDKAPEAAMEVTPEKDETTAMETEKDGEPMTTTPPVLSEKRKALFEPLEPITNLNGKRPTDADSLLPPPDFESANYPKGWLIGKKRKLVNVDVVESMRRIAVQEMNRKDREIDGLNEQLEEDSRCLEHLQLQLLQERSKRTEIERENTMLKEQVDMLVNMIQQDEEEVVAEEP

SEQ ID NO: 58 - protein, 217 aa, Brassica carinata
MEKGNGFEGENTKKKEQTANDGFVGGFFPVSTTKIAWKSRKRSASVNKAPEAAMELTPEKDETTTAMETDKVGEPMTTTPVLSEKRKALFEPLEPITNLNGKRPTDADSLLPPPDFESANYPKGWLIGKKRKLVNVDVVESMRRIAVQEMNRKDREIDGLNEQLEEDSRCLEHLQLQLLQERSKRTEIERENTMLKEQVDMLVNMIQQDEEEVPEEP

SEQ ID NO: 59 - protein, 224 aa, Brassica carinata
MEKGARFEGDNTKKKKTVGDGFVGGFFPVSTTKIAWKSRKRSTSVNSDKAPGDAMEVAPEKDESTTTTTAMETDKAGETMTTTTPPVLSEKRKALFEPLEPITNLNGKRPTTDADSLLPPPDFESANYPKGWLIGKKRKLVNVDVVESMRRIAVQEMNRKDREIDGLNEQLEEDSRCLEHLQLQLLKERSKRTEIERENTMLKEQVDMLVNMIHQEDEEEVPEE

SEQ ID NO: 60 - protein, 224 aa, Brassica carinata
MEKEGAGFEGDNMKKKKTVGDGFVGGSFPVSTTKIAWKSRKRSTSVNPDKAPDDAMEVTPEKDESTTTTMETDKAGESMTTTTPPVLSEKRKALFEPLEPITNLNGKRPITDADSLLPPPDFESANYPKGWLIGKKRKLVNVDVVESMRRIAVQEMNRKDREIDGLNEQLEEDSRCLEHLQLQLLQERSKRTEIERENTMLKEQVDMLVNMIHQEDEEEVADEP

SEQ ID NO: 61 - DNA, 1050 bp, Brassica rapa; identical to SEQ ID NO: 41
  source 1..1050: mol_type = genomic DNA

SEQ ID NO: 62 - DNA, 898 bp, Brassica rapa
  source 1..898: mol_type = genomic DNA
atggagaaaggagctggattcgagggagacaatatgaaaaagaagaagacagttggtgatggttttgtcggcggttttttccctgtctctaccaccaagatcgcgtggaagtcaaggaaaagatcaagtacttttctctctctctgtgtctctctcctctgtttcttagttttctcacatctctcttagtctcggaatcaaaaggctttagctttgattttggtctgatcccattatatatatgcattagcattaacaacttagattgcagcatctgtgaactcagacaaagcactggagactgctatggaggtcacaccagagaaggatgagtcaacaacaacagcaatggaaaccgataaagctggggaaccaatgaccaccacaacccctcctgttctgtccgagaaaagaaaagctctgtttgagccactcgaacccatcaaaaacttaaacggaaagcgaccaacaacagatgctgattccctcttgccgcctccagatttcgagtctgcaaactatcctaaaggctggttgatcggtaagaagaggaagctggtgaatgttgatgtggttgagagcatgcgaagaatcgctgtccaagaaatgaaccgaaaggtaaaaaagactgttgttgtgtgtttcttttttcttctttgttggactattttgttctgattagaagaggattgtgggacaggatcgagagatagatgggttaaacgagcagctagaagaagactcgcgctgcttagagcatctgcaactccagctgctacaagagagaagcaagagaacagagattgaaagagagaacacaatgttgaaagagcaagttgatatgcttgtcaacatgatacaccaagaagacgaagaagaagtagcagaagaaccataa

SEQ ID NO: 63 - protein, 219 aa, Brassica rapa; identical to SEQ ID NO: 45

SEQ ID NO: 64 - protein, 223 aa, Brassica rapa
MEKGAGFEGDNMKKKKTVGDGFVGGFFPVSTTKIAWKSRKRSTSVNSDKALETAMEVTPEKDESTTTAMETDKAGEPMTTTTPPVLSEKRKALFEPLEPIKNLNGKRPTTDADSLLPPPDFESANYPKGWLIGKKRKLVNVDVVESMRRIAVQEMNRKDREIDGLNEQLEEDSRCLEHLQLQLLQERSKRTEIERENTMLKEQVDMLVNMIHQEDEEEVAEEP

SEQ ID NO: 65 - DNA, 5333 bp, Phaseolus vulgaris
  source 1..5333: mol_type = genomic DNA
gtaagttgtttgggagaaggaaaacgagacttttagatggtcggaagattaaggtaaaaaccaaacagcacctccaaaaaacaacacaacacaacacaaaacctttctctctctttctcttctctttgttttagtatgtgttgaaattctgaatttgaagcatatcttgttcttgaatggaaaacatgaagatgtccatagatgatgctttgaacgccttctctcccgtatccacagctaccatttactggaaatcccgaagaagaccaggtatatctatatgtttatctatacgtacatatatgtgaatgtgtaaaactctctttttcttaattaacttcacctatctttaatttactttgtctattacttagtgttgttccaaacatggtggtaattgttgcactttactttctcttctgtgccattttcatctcatgatgctcagatttcgaaatagaattcaatggttttgttcatttttgcatgggattttcggtatttacatgccctctgtcaattcttagttttttcacagaaaagaagatttttttgtgtgtatttacatgattgggaactgagggtagttccttttgatttcctttgtgctggaatggtttctgtgatttctgcaaaattggtcactgtttcagattgaggaagagtaaaatgggttttaacggttggtgtgacttttattatacattgctttgtttgttagggtaaagttcaacttttgtcccctagttccctagttttgctcatcccatttttttaaaataaaataataataattagatccttactttttcaaaaaataatattttttattaactaataattttttatttaaattgttttttatgattgttaaaaatttgtattaggtttgaagctcggttaaaataaaatgaaaaataaaacatacccaaattgaaaattaaatcaaaattactgatttttttttaccaccaaaaaactaaatgtgcttgtttgaaaatggaatattagaagtacggattcaacaagataaaaggatcaaaattgtattttatcccatttgttatcaatggcttaccaaactttggctctctcttgatatcaggatgtgataataattgggttgggatccaaatttatcttaataaaaaaattttaaaaaattattatgtagtttgttggctgattaataataaaagaaacaagagaattttgatgcaccttggtaaaagctttatttgtgatgatatagatattgatgatttattgcattctgtgaaggatagggaaaaagggaaataaaaaacgtatgtggctgttgagattatgtagtaattatgcagtcatcatcatatcattggtttcactgtaggacagctcaccctccaaccaaccctcttcacaataacacaatagccttaattatggtttccttgcatatctgaatttcaatttgatacctcttgttactgatgggacttctaagcttgtcaatattaccttttgtaaaaaaaaaatcttttgtcttcaatgtatttacgtgagcatttaaataagcatcttccttttggtatacgttctctaactatatcaaaggcaatccaaaagcaaggttggccaaatcttgactgaaaatcaagagaatttatccatccaaaagtataagtatatatatacagaaatgattatattatatatgtaataataagtttattaacttttataacaactattttgtaccaatagtgatttgagtttcattaagaataaaaaaaggttactttatactgtgaagaattgggtcagtaaaaatcttgatcaaagggtcctaccatgtatgaccaatattagactagtgttaatatgcatcgaatggaccgtctagtcttttgtctattgagccctgtaccaaccggtggaaccatctgacaactagtctgttttgttatgaggagtacggttaacgtgtcttccttgatagttttagatgtgtttcaagtttgtcaattataacagtatttgctttataaataggtaccttgaatagaaagtaactaagagttgtaacatagaattgtaatttgagtaagagtttagtaagagagaaattgttaagttacaatctctacgcattatagagagtgaattctctcataaaaataggttgaagttcattaatacttcaatctgtgtgagattttttcttattcctcaccttttattgtttaacatttacgaagtccctttgttatcaatattatttttattgtacacgttctaagtgaatttgttgagctgttttctaacaaactggtgcggtgaacgtgaaatcaatcatcatgactttcgcaaagcatgagatagagaaattcgttggtctaaatgacttcaaattgtggcaattgaagatgcgtactcttctggttcaacaaggcttcctcaaaacactggaaggtgaatccttcatgcattcatggctaagatagactagaaaacgttattaaagaacacttatagcacaattgttttaagccttggtgattaggtgttgaggcaagtcgtgaaggagaagaccacaacaggattatggatgaaattagtgaataactagacgaactcaaccagctaatccttgatttggagaacattgatgtgcaaattgatgatgaggatcaatcaagtgctattgttattgtgttcattacctaagatgcattatcaattcaaggaaaccttgttgtatggtagagagactctcttttttgagggggttcaggctggtctaagctctaaggagctgaatgagaagtttgaagttaaggtgtttggtgctgaagataacggagtagaccgtgtaccaataataatagagaaggtagaaggaggtcaaagtcgaggtcaaagaatagtgaaaatacatcttttataaaatgttaccattgtaaaaaaggaaggtcacacaaataagtattatcctcaaatttggtgatgtagctttggtgaaagaagtttatgaatcattggaggtcctcacggtatcaagtagtgttgataattgagtggataatggatttcaaatgtttattccattaacacctgagaatttgtggttcccagagtttacagaacctaaaagaggtttagttctccttggtgacaagaagccttgtaagataactaaaattggaaccatcaggtgtgatatgcatgatggaattgaaagagtgctggaggaagttaggtgtgatatgcattatggaattgaaagagtgcttgaggaagttaggtttgtaccttgcttgaaacgcaacttaatatcctttagtgagtttgagaaaaatgaatgtgtttaaaggaaagaggagagggttaaaggtgatgaggggatccatgatagtgatgaaacgtgtgagaaagaatgaattgtatgccttggaaggtgttgtagtgtttggctcagcgtctaaaccatcttatccaagactgaaatgtggcatagaaggttaggtcatgaagcaataaaggtttagttgagttgaagaagcaaggtttgtttaacaatgacaaaattgaattttgagttgaagctaacctttattttgtctattcggcgtgagagggtgtgcagagatcccacatcgactacggattaaagcatttcatagtatataagtaggtgtaaacttcacctcataaaccggttttgtgaggttaaactagcttatgagatcaggtttaaattcattatatattataaaaggctgatattgaactagagaatcttgtagatgacaaacaacaagcggatagtttcgtgtaaaatgagatctgtgaaattaggctctgttcaactaaccctgcccatgagaaataatatttgaaatgctaaatgccttgtccataaattcaattttatgagaactcactttgaggaaacttatttacaattggatatataacatacgatggagaggacactgtggtaacaggttttatctcgtaaatgctacttaactcaatgtaactgcatgttagttgccttgtctttatcggcttatatgttctgcaagcaatgttaaatcgtgaatcatttgataaaatcaatattttttttttatctctaaccactgtttcatgttgacaactataatctacaagaaattcatgtaatatagagatcaacaagatagttctgatcttgaactaccaaataatttctcggataacattcatctagtaattaatatcatatcattagatgcatttgttgagtgcaatgaacatgactactttgctaaatgatgagctgccaaaaacaaaaatggtaacttgttgcccacagctagcgggaggaatttagaggtatcagaagatactgctaatacaccacccagcaagcaggaagatactcctcctcctcctccttcttcttctagtgaggaggtgcagaacacaactccaatttctgagcgtcgaaaggccttgtttgaacctttagaacctataaagaatgttaatggccgacgaccctcggctgagtctttacttcctccccctgactttgagtctgcaaactatcctaagggctggctgattggaaagaagcggaagcttgttaatgtagatgttgttgaaagcatgcgaaggattgccatccaagaaatgaacagaaaggttccaagtttcctcagctccctttatttccaagctaagacaaaattattttcttacaggcctcaaactcaagccacttgctcactcacttttgctatttttgttgttgttgttgcaggacagggaaattgatggactaaatgaacaactggaggaggattcacgttgcctggagcacttgcaacttcagcttgtggatgaacgaagcaaacgtgctcgagttgaaagagagaatgcaatgcttgaagaacaagtgagcatgcttatgaacatgttacaagaagcagaacaaatgggagatgaaggcccagatgaaccttaatgtttatcattacacattttgtgtgcttgtgtgtatcaattttttgtgtgtatcaattttttgtgtgtaggttctgttcgtcatgtctagcatattggatgtctatgcagttattagagtgcttgtagtaatatctgggggcaaatagatcaaatcgcaatgagcaaactattcgtttgtctctaaaaaaaagttgtaattctttctagagactatgtggttgttaattcatatcttgttactctttcaaactataaaagagtattgtaatttatctacttgccaagtttataaagtggctcagttgaataaagatctcggttcaataagatcatag

SEQ ID NO: 66 - protein, 209 aa, Phaseolus vulgaris
MENMKMSIDDALNAFSPVSTATIYWKSRRRPASGRNLEVSEDTANTPPSKQEDTPPPPPSSSSEEVQNTTPISERRKALFEPLEPIKNVNGRRPSAESLLPPPDFESANYPKGWLIGKKRKLVNVDVVESMRRIAIQEMNRKDREIDGLNEQLEEDSRCLEHLQLQLVDERSKRARVERENAMLEEQVSMLMNMLQEAEQMGDEGPDEP

SEQ ID NO: 67 - DNA, 3405 bp, Glycine max
  source 1..3405: mol_type = genomic DNA
agagacaagaaaaacgagacctttagatggtcggaagatcaaaaggagaaagccaaacagcacctcctcagcaaattaacataaaaaacctctctttctctatttcttttattattgggtatgtcttgaagttcttctgaatttgaagcatatatttgtccttgaatggaaacacgtgctggaagtgatatgaagatggccatagatgatgctttgaacgccttctctcctgtttccacccccaggattttctggaaatcacgaaggagatcaggtatatattatactatacataccctcttaagtcttaacttcacctacctctactttctctttctactttatctgttacgtagtgttccaaaacatttggcaattgtgctatctttctcttatgtggcatttccatgtgatattgttcagatttggatgtcaaattcaatgtttttgcatggaattaattttcaatattgtgacatgccatctgacaattcttaattctttcaaatgttttttaactgggaattttgcaagatttggaactgaggcttcctttttctatttaacttccctttttctgggattgatttctgtaattcctgcaaaattgttcactgtttcagagagagagagagaggaagcgtaaacacaggttttaacggttggtgtgacttttatgttacgttgctctattttgttagggtcttgcagcaaataaagcaattaaaagataaaagtttctaatgcattttaaaattacagagaaacgtatttttacgcattcagtattttttttttcttaaccgctgcccggttagcatttggcaatttgctatcaatggcttaccgaactttggctctgtctcgttatcagtatgttttaatgattgggacccaaatttattctaaagataaaataaattggaagaaattatgatgtattttgttagctaattagtagctcataattatgagctaactctattatttttacctaataataataatagtaaaagcaacacgacaattttatgcatcttagtaaaagttttatttgtggtgatatagatgttgaagatttgcagcattttgtgaaggataggaaaaaagagaaaataaaaacgtatgtggctgttgagatagtgtaaccatcatcatatatcattggttacactgttggacagctcacccttcaaccaaccctcttcagtatataacactaacctttttgtaatccttttttaatgtgtgtatattaacattttaagtttacgtttggttgggcggtagaaaaaagaaaaaaaaacccaccaaaaatgcatgaaaatccaaaagtgatgaagagttgcggtaaccttgactctctttcacccaaccaaatcactgtaaataggcatcttccttttagtaaccgtactcaattatattaaaggaaatccaatatcacggattacctagccttcactgaaaatgaagtcaatttgtccatccaaaagaataggtttatctacatgattttgcgttgctaataagtgtccttaggatattagtttaagaattaaaaaaaaaaaaaatttattttgtgaatcataagaaaatgaaaaaaaaaatcatgagaaacataattttgtgcctccaaataaagatatttctactttaaatttcttaagaaatatacttaaggtattggttagtattttccttatctatatatgccatcatgccagccatgtgacttgttgacattggtatagtttggtgtataatggcacctatgaaattaggcttcaagcaggcggctatgtttaactaaccctgcccatgaattcattttgatgaccactctctcgaggaaacttgtcttcaaaaggatatagaatatactagggaggggacaacatactaaaagttttgatctcttaaatgctatttaccttggtgcaactccttattagttaccttgtctatgtaggcttatacattatttaagaaatgttagaacgtgattcatctgatcaaaatcgatattatatctcactaaccacagttttcatcttggcaactatgatagatgagaagttattaggaagttttaggccattactgtttgtggtaacaattaatgtctatgtgatatgtatttgagttttttaatttacaagaaagaactaatgatactctattacgcgtcacataaagattaattgaaactgtgatagtcttaaactttgcgatgtttactcattaacttaactatgtccgtcatgtagtaatcattggatacatttgttgagaacaatagatatgactactttgctaacaacttagagcagaaaaggttttccattttattttcctttgttgtgcaaatttactgtatctaaatgatgagctgccaaaaacaaaaatggtaacttgttccccacagctagcgggaggaatttagaggtatcagaagatactgctaataaaccacccagcaagcaggaagatactcctcctcctcctcctccaccttctagtgaggaggtgcagaacacgactccgatttctgagcgccgaaaggccttgtttgaaccgttagaacccataatgaatattaatggccgacgacccttggctgagtctttacttcctccccctgactttgagtctgcaaactatccaaagggctggttgattggcaagaagagaaagcttgttaatgtcgatgttgttgaaagcatgcgaaggattgccatccaagaaatgaacagaaaggttccaagtttcctcaacaccttcacttccaaacaaagacacaattatactgagccacctgctcattttgttgttgttgttgttgtaattgttgcttgcaggacagggaaattgatgggctaaatgaacagctggaggaggattcacggtgtctagagcacttgcaactccagcttgtggatgaaaaaagcaaacgtgctagagtggaaagagaaaatgcaatgcttcaagaacaagtgaacatgcttatgaacatgttacaagaagcagaacaaatgggagatgaaggccctgatgaaccttaaagtttattattatacccagtgtgtgtgcttgtgtgtattaaattctttttgtaggttttgttcgtcatgtctagttggctgcgcatgtcggatgtctctgcagttattaattagagtgtgcatatagtaatatttggggggaaatagatcaaaccgcaatgagcaaactattcgtttatctcaaaaaaaaaaaaaaattgtaaatcttctggtgactgtgtggttgttaatttattatatcttgttactcttttaagctataaaagagtattgtaatttagatactttccaagttgattcagtggctcagttaaataaagatcacagtcgacattatttt

SEQ ID NO: 68 - DNA, 3171 bp, Glycine max
  source 1..3171: mol_type = genomic DNA
acgagagctttagatggtgggaagatgaaggagaaaggcaaagagcacctccaaaaaaaacaataaccgtagcccacacctcctctcagcaaacatctctctttctctgtttcttttattatgttgtgttccttgggggtgctgatgtatgtgtgttgaagttctgaatttgaatggaaacacgtgctagtggtgatatgaagatggccatagatgatgctttgaatggcttctctcctgtctccacccctaggattttctggaaatcacgaaggagatcaggtatatattaagtcttaacttcacctacgttcctctattttctctctctactttatctattacattctgttccaaacaattttcgcaactgcactttactttctcttctgtgccatttggatttcaaattcaatgtttttgttcatttttgcatggaattttcaatattataacatgccctctgccaattcttaattctttcaaaaataaaaataaaaattatctctgtatttacaagatttggaactcagagtctgagactaaggctaattcctttttcaatttaacttcttttctgtaattcctgcaaatttgttactgtttcagatagaggaagcgtaaacacacaggttttaacggttgggtgtgacttttatattacgttggtttattttgttaggatgttgctaacaaataaagcatttaaaagataaaagtttctcttgtaaaaaaaaaaaaaggatataagtttctaatgcatttaaaattacagaaaatcgtatttttacacatttaatatttttttcttttattttcttaaccactgcctgcatagcatttgacaatttgttatcaatggcttgccgaactttggctctgtctcgttatcagtatcttatgatgattgggatccaaatttattataaaaaaaattggaagaaaatatgatgtattttgttagctaattagtagctcataattatgagctaactctattacttttacctaataataataataaaagcaacacgacaattctatgcatcttggtaaaagttttatttgtggtgatatagctagctgttgaagatttgttgcattttgtgaaggataggaaaaaaaaaagagagaaaaaaaaacgcatgtggctgttgagatagtgtagtcatcatcatatcatcggctacactgttggacagctcacccttcaaccaaccctcttcggtatgagtgtatgaccttaattttggtttccttgcatatgtgaatttcaacttgatgtccctcttgttacagatgggacatctaaacatttcaatattaccttttgtgtttctttttttaatgtgtgcattagcattgaagtgtatgattggttggactgtggagaaaagaaaaacccaccaaaaatgcatgaaaatccataagtgataaagatttgtggtaaccttgactctctttcacccaaccaaatacactaaataggcatcttccttttagtaaccgtgttcaattatattaaaggcaatccaatagcacggatgacctaaccttgactgaaaatgaagtcagtttgtccatctaaagaataggtttatctatatatgccattatgccagccgtatggcatgttgtgtattggtatagtttggtgtataatgaaacctatgaaattaggcttcaagcagccggctatgtttaactaacccttcccatgaattcagttttatgactactctcttggggaaacttgtcttcaaaaggatatagaatactagggagggtataacattataattttgatctcataaatgctatttaactcggtgtaactccttgttagttaccttgtttatgctggcttatacattatttaagaaatgttagaacgtgattcttctatttagaatcgatatttttttttttgaaggatgatcaaaatcgatattatatctcactaacaacagttttcatcttggcaactatgataaatgagcaattattaggaagtttcagactattacaggtctctggttacaattaatctctatgtaatatgtattcaagttttttaatttacaagaaagaactaataacactccattacgcgtcatgtaaagattaattgaaattgtgatggtcttaaactagctcataatttgcggtgtttactcattaactatatccgtcatgtagtaatcattggatgcatttgttgagtacaatggatatgactactttgcaaacaacttagagcaaaaaaggttttccattttatttttcctttgttgtgcaaatttactgtctaaatgagctgccaaaaacaaaaatggtaacttgttccccacagctagcgggaggaatttagaggtatcagaagatactgctaataaaccacccagcaagcaggaagatactcctccaccttctagtgaggaggtgcagaacacgactccgatttctgagcgccgaaaggctctgtttgaacctttagaacctataatgaatattaatggccgacgaccctcggccgagtctttacttcctcctcctgactttgagtctgcaaactatccgaagggctggctgattggcaagaagagaaaactcgttaatgtcgatgttgttgaaagcatgagaaggattgccatccaagaaatgaacagaaaggttacaacttacaagtttcctcaacaccttcacttccaaactaagacaaaattatactgagccacttgctcattttgttgttgctgttattgttgcttgcaggacagggaaattgatgggctgaatgaacagctggaggaggattcacggtgtctagagcacttgcaactccagcttgtggatgaaaaaagcaaacgcgctcgagtggaaagagaaaatgcaatgctgcaagaacaagtgaacatgcttatgaacatgttgcaagaagcagaacaaatgggagatgaaggcccagatgaaccttaaagtttattattataccgtgtgtgtgtgtgtgtgtgtttgcttgtgtgtattaaattctttttgtaggttttgttcgtcatgtctagttggctgcgcatgtcggatgtctctgcagttataaaaatagagtgcatatattaatatttgtggggaaatagatcaaaccgcaatgagcaaactattcgtttatat

SEQ ID NO: 69 - protein, 214 aa, Glycine max
METRAGSDMKMAIDDALNAFSPVSTPRIFWKSRRRSASGRNLEVSEDTANKPPSKQEDTPPPPPPPSSEEVQNTTPISERRKALFEPLEPIMNINGRRPLAESLLPPPDFESANYPKGWLIGKKRKLVNVDVVESMRRIAIQEMNRKDREIDGLNEQLEEDSRCLEHLQLQLVDEKSKRARVERENAMLQEQVNMLMNMLQEAEQMGDEGPDEP

SEQ ID NO: 70 - protein, 210 aa, Glycine max
METRASGDMKMAIDDALNGFSPVSTPRIFWKSRRRSASGRNLEVSEDTANKPPSKQEDTPPPSSEEVQNTTPISERRKALFEPLEPIMNINGRRPSAESLLPPPDFESANYPKGWLIGKKRKLVNVDVVESMRRIAIQEMNRKDREIDGLNEQLEEDSRCLEHLQLQLVDEKSKRARVERENAMLQEQVNMLMNMLQEAEQMGDEGPDEP

SEQ ID NO: 71 - DNA, 3141 bp, Pisum sativum
  source 1..3141: mol_type = genomic DNA
aataataatttctcaaggattatttctaagcatagaaataattttttattgaaaaaaaaaatagaccacgaaggagttagagacaggtccacatataaaaaaagagacaaaaccagtctctgacataaaaatttccacccaagtaaataaaatctggaccgttgaaaatccttatatctgaaaatcacggtcccatgacatcgacaattacaattttcagcatcttctttgtaaggttgttgtaaagaacaagaaaaaataaaaccaaacaaacaacacttacaaagaataaactctatttttcatgtcttcattttggagctgaattttgaagcaactatggtcatggatgatgatgctttgaatggattctctcctatttcaactcctatgatttcctggaaatctagaagaagatcaggtactctctctttttcttcttcaatttcaaattcattagcttaaattgtgaaaaatagctcaatttgtgtttcttattttgctatttcaatataatgttaactaatagtacaaatacttaataataacaatttgtgaatcactttgtcttttatggcttttacaaaatttcctctcacaaaccctaccatataattgaatattatttttctattatttgggggttttatttttttttttaaatttaacatgctaactggaaattcttcctgcaaattttatgtttgtgaacttgtacaattttgaaattttgtttttacttttcgatttaacaatttgtttttttttcctggaattgatttgtgtaatttctgcaaaaaaaatctgttagagagagagagggagaagcgtaaaacagtaggtaacagttggtgtgacttctacgttaagctgctatatttgctatgattggcttaccaaacagtatattctaaattttaagtatcataaaaaaatggggtgaaatttgtaagataaaatgtttgagctcattattactccctcatttgcatttttcatatctcaaaaataattgtctttttataatatcaatacagtatttattattattttcccactatcatattcctatttattaattttcactttattcaaccattttttatatacaattaatagaaatattctagtaaatgatattagttttatcatcaaaacaaacacatctaatcattttcttaagaaccgtgaattgttcaaattgaacacttttttatgagacggaaggagtagcttattattagctgatgtagagatgcattgagtgtacggcacagagacgacggcacgatattaatcaatgtagttatgtttaattacttttagtttttaaagttattaccgatgttaacaaagagtttgctgtggtaagtgtaagtgagctgatagttctagtctcaggctcgattcctccttgcacctcatatatgttgggcgcaggttcgaacctgcaatattgatatttgatatgctaggacacaggtccgaacacttcaatgtgttcaaacccgcaatgtctctgtgtcagtcttgtggccgatgtctgtttcggtgctttatagattttacttattaactagttttcttataactcggtttcttaagtctctgacctcaaccaccagaccaatcttatatagtaaataaaaattgatagtcttaacatgattgttagttttgtgatcatgaaaattgatgatgtattaatgcatgtggttgttgagatagtttagacattatcttatcctgtgttgagttattggacaaccaaccttggcctccacttccaactaaccctttttaatgtagcctctatttttggtttcttgcatatgtgacttttcaattttgatattactcttctttattattcatctaaccatgtgaacattaccctcttgagtaagtaaagtcgagtcaaagattgttttaatgagagctcaatcttggatattttctttcgattcaaaagtttattaactaaatgaattcaaccatttgattatggacgcaaatatttgttgaaagtgttgttttccttgcattacaaagttttactatctctaaatgagtagaaatgaatggtaacttgttcaccgcagctagcgggagggatttagaggtatcatctgaagacaatgctacaacaccacctggcaagccagaagatccatctcctaatgtggagatgcttgacacaacggaagtttctgagctttctgaacgtcgaaaggccttgtttgaaccattagaacctataaagaacatcaacggtcgacgaccctcggctgagtctttgcttcctccccctgactttgagtccgcaaactatccaaaggggtggctgataggaaagaaacgaaagcttgtcaatgttgacgttgttgaaaagatgcgcagaattgccgtccaagaaatgaacagaaaggttatattccaagtttcctctaagagtactaataataacacaatctaacagtctcttttcaacatatatttctatgttagttgaatttaatgaagactcgcatgaaaagagtgttactaacattattcgcatgaaactgaggctaatgcatttgacgacttttgttacaggacagggaaatagatggactaaacgaacaattagaggaggattcgcggtgcctggagcatttgcaagtgcaacttgtggacgaacgaagcaaacgctctcgactcgaaagagaaaacaatatgcttcaagaacaagtgaacatgcttatgaacatgatacaagaaactgagcaaatgggtgatgaagggcacgaaataggagatgaaggccaaaatgaaccgtgaagatgcattgttttatactatcggtgtgtgcatgctcatgattgttatatttgtttgtagattttctccaacttatgttattagaatgcatatagtagtagtaatattaatatcgggataatcaaatagtactggatataattttttatctcaaacacagaagtaaagtgttattttatttattttttaacagaaaccaaattactacttatagtaataatgaaatgctcaatacattttcgaatacaataggaaaattttgttgttttagtatgttgaatggctctggttaaattaataaacggataattgcagatt

SEQ ID NO: 72 - protein, 210 aa, Pisum sativum
MVMDDDALNGFSPISTPMISWKSRRRSASGRDLEVSSEDNATTPPGKPEDPSPNVEMLDTTEVSELSERRKALFEPLEPIKNINGRRPSAESLLPPPDFESANYPKGWLIGKKRKLVNVDVVEKMRRIAVQEMNRKDREIDGLNEQLEEDSRCLEHLQVQLVDERSKRSRLERENNMLQEQVNMLMNMIQETEQMGDEGHEIGDEGQNEP

SEQ ID NO: 73 - DNA, 3467 bp, Eucalyptus grandis
  source 1..3467: mol_type = genomic DNA
ggaaaaagcaaacaatttcctatcttctggctctctcctgctctgctctttctcggtaataccaaacaacgacaacaacaaggaacgagaatcgagacccggaagggagaagaccaggacgcagaacagcatccttgaaaagctcctcgctttcagacccctctctctctctctctttctgggtcggtgttggtttttgaggttgaagcttcggcttccgggagctgtggaggtttcttgagatggtccaggaagagaagccggacggcggcagcgctgcggtggatgggaatctgcccggtttctctccggcggcttcgagtcctcggattttctggaagtcccgcaagagatcaggtaacgagtctcgatccctcttccgcatcagtggtttgtccggcgatgcgcgcgcgcgtgagggtccgtgtgcttcgtagatagaagaaaaagtgcgaatcttttttggggtagctgcgtaagtctgaaaatttcctcgtgggtccgcgtttcttgagttgttttcgaagcgagggtgcttcatattcacgttctgcagaattacccttcatttctctgtcgcgcaattgcttatagattcagagagagagatagagagagagagagaggacttgttgcatatctaagtctttgctggtacgttacttaactgcgtttggttagctggcttaccagtcattctctctttctccctccctccctccctatctctctctctctctctctctttcattctctaattatttcaaatatcttttttttttgcttaattaaggccaccaatctctttctttggcccccgttgctccattcaagatggatggctccaaaagagtcttctacttattttattgatttcttccccttcggctacacctagttctcgatatttatttctttgagatgcgtggtctttgtatatttgcttaatgtttctggggttgtattttatatagggtgcgtggaaatggtccatcttttaaatttcggctcattttctcccgattggatccaatcaattgactatagacaactggggtttttttaattagacttcttgatccaagtccttatttttaagattctgtgccctcgtaagacaaatcatttgttcggaaagttgttagtctttttgttcacgcttttcgcagtgccctattgcgattttgtaaacgattgtatgcccttccgttaggtaagtttgtcggccgtgtctaactactaggaatttgtttttttcccttggagcagccataactatacagcacttgtttgaccgttgcgtttgagcaatacagtgtttatgctaggggacaatgccttaaaactttttctcgcttaatacggttctaaatcctaaaagtgtcttccattttatgttttaatcgatggagttgttgactacaagccaccctcctccttggcttttaagggtctgcatattcgtcgccaatggcataggtggaattacttgtgattcgtttgtgcatctttggcatccttatctgtattatagaagatcatggatgaagcaagatgtgactgctgtgggattcatgggattatatccgtttcggtgtcttataaacgaaccagtcttgtggtttgccaccagctttatgtttgttaaacgattggttcatcaagttactgtcattctttcaagaaagaagaaaatagaccagtgatgccttccattccttcagttttggtggctccaaaattcccttggagccccaaatttcggagctttggtcttcgtctcttgttcccttctgcttgaaaaacaattggtccatcgagttcctgtgctgtgtctcgtgttttactaggatgcatgagctgtttcgctcataaattgtttttgatagtcttacatcttggattgaattagtttaggcagagaatactaatttggttgctttggcgatgatgttggcttggcagccactatatgatcatgtctttcggtgtaaagatgtgaatatgaaactagacctcacttgggcacagttacagctttacgatgacctttctcaatgcatcaccttgaagattgtgcgtattaatatcactattgctcatacttttgattgaattgttctcaattcatggttcacttctttctcatttagaagtcaaaagaaagaaaaagaaggtatgcttttcacttgtttgcagctccaatattagaatacttggtactagaatcatttcttttccaaatttccaacagttggtggaaagttattgaacgaggtagcagatgctgctgataaacttcccgacaagcaggaagatgcaccgacagatgagaatatgcaagactcaacgcagacgcctccactatccgagcgtcggaaggctctgtttgagccattggagcctgtgggtagcgccaacagccgactgccatcgaatgagtctttgttgccaccacccgacttcgattctgcgagctatccacgaggctggctgatcgggaaaaggcggaagcttgtgaatgtcgatgtggttgaaagcatgcgaaggattgctgttcaggagatgaacagaaaggtgcttatgagcaaaaccacctatcctcaacaaatactaatctaatcccatttgttattagctctttagttaaatcttagaacccaaacatgatgcgtgcaggacagggaaattgatggcctgaatgagcagttggaggaggatgcgcgggttctcgagcatctgcaagtgcagctactcgatgaaaagagcaagcgctctgaggtcgagagagagaataagatgctgcaggaccaaatagcgatgttgatgaacatgttggacgaaaatgaatcgatggaagaggtccccgacgagccttagacatcgcatgttggtaaaaaactgttctttcgtttcctatttcattttgaaagagtctatatagatgaacgtacgaaaacagaaggcatagctggacctaataatatgcatgttctttgatatgttactttcctccgaaaatttctttttagagggttggagattccttgttatcgaggtagctgtgagtgtcattagctatctggtaaagggaaagaaaaaaaagaaaaaaaaaaagaaacaagtttggaagttaggtaatgccatgtaagtgcgagttcctatttgtaactgaaattgaacatagcgggtctgtaatacaaaagtctgttgatataaactctattgtccttcctttttgctgtaagttcttccatctgttcctctcgtggagatccggggactgacagaatcgacgctatttcctacccccctcccttttctctctctctctctctctctctgtggataatgatcagaatatgctcgcgcatcgttccatcaaccgtgtagctggtcaatcatgtcaggcagcttagatgagctcgccgatcgggaacactttgattttcaccgtatcatctccg

SEQ ID NO: 74 - DNA, 2314 bp, Eucalyptus grandis
  source 1..2314: mol_type = genomic DNA
ggttttggtgagagcagctggaactccaagaaagccgatgcggaagcaatctgctgccaccataaaaatccgttctctaggcgcttctgtatgatctctttcgtggagcacgagggggggtatttggatttcgttgctctgttctcttcagatggagcaagcgtctaaggacagcacgaacgggactctgcagggcttctcgcgagtgaccgatgctccagttctttggaaatctcaaaagagatcaggtatcgactgcccagacaacccaatttacttgactctgtttcttctctgtttctgaatatgggtttaagttgaagaaaactggtgattgattggtgcatgcttggtgggggggatttcatttagggactaactgtagcagaacccatctgggttttcaaatggggctgtgcatgatcgcggaagatagggtcttgtggaggactctattatagtttcacttgttttcctgcttgctgttcgctgaattatgctaagaccgtttgaacagtgcattgtcttgcaccttcatttgcttcctcaaaggagggtaatgatcttactcggtatataaaagtccatccgccctgaaaatggaagacaaaaagaacgtcttttgctgaattttttttctagttcacctcttattctgactctgtctgtcatgctgcgcaacttacgtttcattcttgcattttctctgattcaatctgccgtatgatagaggacaccgttgagtcactgacggccctgtgatttgagtgatcccaacgactcgagtgatatttcacatatgatgcaattcccctttgaattagtgcctcaacaaatctttgtcatgttaatagattatgagtgttctgcagttgcagctgccctgctacattgctcctttcgtctgatggaaacatcaatggatatgctaggagttgaatattcaataacttattggtgctcctccaatttcttagcgatgatttcatagtgatgttactctgagttcttttatcaaatttaggctatggctcaggatgagattgataagttgcaaaattggttgactactcatcacttgcacttaatattgttctccttttatgtgattcctcaatctaataatcgggaaaagtttgcccatttttaaactaaaactctggtgttcctaatgaaatacggatcccacccattttatttgtttgcaaatctcagtgaaccctgacctatcgtgtcattacatctcaagctgcacgatcttccattttaagcttcaatatctccctgagattctttgaaatctaaagaaagtaaagtccttttcttttcagacatctgaaagtgaaaggaagacattattcatccacgtttgcatgttctgagtcggattttttgtattttttaggtacggaataaatgttttgcccaagcatcatatctgttattattcctcttatgaaatttctgcttccttttgccgcacacagaagaacatatggtgttgatgcttggtaccacgaagtatacctgtaacaaacattatgggcactctatatgtttcttgatcctagttagaattgattctcaattacttgggattatggattctgtaatttgatatccacagcagatgcctggaatttagacaagaccatggcagacactgctgatgacacacctactaaacaagaagagaggaggatggaggagaaaacccaggattcgacaccactctctgttctttctgggaagcgcaaggctctgtttgagccattagaaccgataaatgatatcaacaatagaagactatcggctgaatccctgctcccaccaccagatttcgacactgcaagctatccacgcggctggctagttggaaagaagcgcaaactagttaatgtggatgttgttgaaagcatgagaagaattgccattcaagagatgaacagaaaggtgcaactcctatttatctcttaagtcatcctcagtctttcttgttcattatattagaaagtctgaaacagagaactaaggatcacgtgcttgcaatttctgtgtgcaggaccgggaaattgttggtctaaatgagcagctggaagaggactctcgggtactggaacaccttcagctacagctcctggaggaaaagaggaaacgtgtggaagtagagagggaaaatgcaatgctgcaggatcaaatatcgatgctgatgaatatgatacaggagaatgacccgatagatgaagaaaggcaaggcgagccataatcaatgagtctttgttgataaatagttttctcagttctgcataaatct

SEQ ID NO: 75 - protein, 212 aa, Eucalyptus grandis
MVQEEKPDGGSAAVDGNLPGFSPAASSPRIFWKSRKRSVGGKLLNEVADAADKLPDKQEDAPTDENMQDSTQTPPLSERRKALFEPLEPVGSANSRLPSNESLLPPPDFDSASYPRGWLIGKRRKLVNVDVVESMRRIAVQEMNRKDREIDGLNEQLEEDARVLEHLQVQLLDEKSKRSEVERENKMLQDQIAMLMNMLDENESMEEVPDEP

SEQ ID NO: 76 - protein, 208 aa, Eucalyptus grandis
MEQASKDSTNGTLQGFSRVTDAPVLWKSQKRSADAWNLDKTMADTADDTPTKQEERRMEEKTQDSTPLSVLSGKRKALFEPLEPINDINNRRLSAESLLPPPDFDTASYPRGWLVGKKRKLVNVDVVESMRRIAIQEMNRKDREIVGLNEQLEEDSRVLEHLQLQLLEEKRKRVEVERENAMLQDQISMLMNMIQENDPIDEERQGEP

SEQ ID NO: 77 - DNA, 3681 bp, Theobroma cacao
  source 1..3681: mol_type = genomic DNA
aggcaaagagacaactgttttgacgtaaaatcggtcacccaaattccaaatcttaaccgttgaaaaacccttgatgatggtccctcttcttccttgtgattacccacaatttatcttcttctccttcctctcccctttctagttaaaaccgcatctgaatcccaacaacaaaagcaaaaagctcaaaccaaaactcaactcgtagagaaacaaggacatacttttttttcatttgttcttttcgttctttagggagttttgggtgttccaggtttgaaaagaaagaataagtggatacctctctatatattttgatttgtttataattatttgttttcgtcaatggagaaagagaacaagaaggtagatgcagcagctttggaagggttttctcctgtcactacaactaggattttctggaaatccaggaagagatcaggtagtgtcagttctttgttttcactttctctgcttggtttctatggaaatgaagtaagcaaaagaaatggaaaagctatgaacatgtttaattcactccctttctatggctttttttttgtcttgcgtgatttgaccaaacacccttcaacccatcactcatgtcttaaaattcattcatctccttggtgtgaaaattatactatcaattaaggaagggaaggatagtcgacccagtttctatttgatcctcatttcgatttaagccattatcttttctttgtttcttcaagtttttgtttgagtgattagttaaggataacatattatggaccatattgtttatgacttgtagcaagtggttactttgctgctacgttaatttacctggtttggttaaaagctgattggttggcttacctctctgtctctcattagtatatctttttcttctaccatatatttatcatttcattttcctgtctattctgttcattttgatttttcttgttgatagtcttaaccagcacgttttccctgcctttttgttgatatgtctggattggctttgactttggacagctgcccaccatatttttttattgcttaatcatccagctaatcatctttaactattcccaattttaaatcatatcagttggtttgctaccaaaaaaagacttaagaaaataagcaaatacaactacctcttacaatttctttcactctagattttaactagacctatccgttggcatgagtctcacaacatgatgctgtaaaagggtattaccacagtagtcattgattttaatgataggcatcaattgagctcccttcatggtggcatcctttcaatgggtttagtaaaacagagaacagtaagattcttgtacccaacagtcacacctaattggctcaggtctccttttctaagtttgtttttgaataagttggaaaaggattttggaacttgatctttttttttcttttgaaggagagacaatgttactaaatcaaaatgatattttgtccttaattaatataaaagctttttcttggtttgaaaatgggttgaaatgagagacattttcatgtcaaatctgttcatgatggaaatgggagacttcccaccaaacttgtcatcattctaatcatttgccagcacatgatgatttattcatttgttttttttttttgtcccaaaaataatttttgcttttacgttcacttctgataattttgcaacttttttttcttctttctcttttgtttgtcatctttgcaactttcagtcagaccataaaaggaatatagttaaagaataaaaagaaatcgtctattcattggttctttacttgaaataattgcacttagttgaaaagttatggtttaaatttaaggatgaaggatagagtcacacaatgtggagagtagggagtagggacatgtgggatggatgttctaccgtcaatattacagactccctttcttaggagatctcaactcaagtggtacctaacttttcggtgggataacacaggcatcttcaatatgctcttaaaaattgttccttgtcataaaatctagctacaaacctcacgatgaaggcacaattgctaagtagaggacctaatgtacaacagtatataaatttacaacattgcgagtatgtttttgtttagcaacattaagttaccgtaaagaagcttggaactagaatatttaacttctttccgacagctagcgggaggaatttagacaaggtaacagaagagactgctaatatgacacccaccaaacaggaagaagaaactccagatcaagagaatgccccagatccaacaacagcttctgaactttctgagcgccggaaggctctctttgaaccactggaacccataaaaaatctcaatggccagcgcccatcagctgaatctttacttcccccaccagactttgatgctgcaatctatcccaagggctggctgattggaaagaagaggaagctggtaaatgttgatgttgttgagagcatgaggaggattgcagtccaggaaatgaacagaaaggttgcttcctagacttaacatctcttctacaaaacactagcttaagttcatgtacgtatcttatcagccagaggcttaataaatcaagatgctatacattttatccacaattagtaaatgacacattgcatcttgagttattgggtctgcaactgacctgataacgaagatgtatagaataagatcactgtgcacgcatataggcacaaattgcagggacggtgcaaggtaacagcaaagggttaattttgtaggaccgggaaattgatggcctaaatgagcagttggaagaagatgcccgatgcctagaacatctgcaacttcagcttttacaagagaaaagtaaaaggtcagacgtagagagagaaaatgcaatgcttcaagaacagatatccatgctgatgaacatgttgcaggagaacgaaagcatgggagacgaaggtccagatgaagcttaaagaaaaaaaaaattcatttgtagtttgtttattcttttgtagagttgtttgaaaagagtaagaaggcaggaatacatgcaaatatatacacatttgggagaaaataggtctagtgattgtagtttgtttggcctggtgagtagctttcttatgcttattattgcttgtaagttgtaagtgagtctcaaatcttatgccaaatttatctaaataaattgtttttatgttagttcttctcaccttaaaatgctttgtgtgcagcagcttgtgcacgccaaacctatttgtgccttacctatcaaattaaacttttaggtaaagatcattatccatagtaaaccttccttttttcattattactagagtatgcctgtgtgatatacgtaaattaatgtttattgaaatatatctatacatcaataatcatatggtgctcactttacgtaagcatttatgaagttatttgtcaactatatagaaaaggtcaaaagttgcataattgtttaagtgataagctgtttaagagttgtgaatgtagattgcaatatacaacttaagaacacataaaatacatgataagtgactttactcgatgattttaatgaccctaacatttgatctctatggaacttctttctcattagtgacaataagcattccatcttctataaaaccctagatctgataagtccttacattctcagacaacttga

SEQ ID NO: 78 - protein, 209 aa, Theobroma cacao
MEKENKKVDAAALEGFSPVTTTRIFWKSRKRSASGRNLDKVTEETANMTPTKQEEETPDQENAPDPTTASELSERRKALFEPLEPIKNLNGQRPSAESLLPPPDFDAAIYPKGWLIGKKRKLVNVDVVESMRRIAVQEMNRKDREIDGLNEQLEEDARCLEHLQLQLLQEKSKRSDVERENAMLQEQISMLMNMLQENESMGDEGPDEA

SEQ ID NO: 79 - DNA, 4300 bp, Gossypium hirsutum
  source 1..4300: mol_type = genomic DNA
ggattataacgagttgtatttgatcaattttgcaagtatttttttggttttcgttatagaataaataaaacaggtaaaatatttattataataataagttgtattttatcaattttgtaagtaatttttttttttggttttctttacagaatatatgaaacaggtaaaatatttatgaaaatagatgcgatagaaaattttctaggaaaatagatgttaaatgtttttaaatttttattggtaccaaaatataataaaaataaataaataatattttttaaattgatattaaaaatgtaaaaaaataattatagattgtttttgaaaggattatcccattttctaaccctaaaaaacctatgttcttaatttcaacatttgtggaattccaatatttaatttattaatcatgtgtatttatcctgcaaattggatttgaattataaaaattgcttcctatgcttaacaatgactttttcctatgaaaaggaatatatgaattattagagaaaacatggaagtccgtggctacacagttgagtcaatccggttcgaacatttattcgaaaaattagaagatttaaataaaaatataaatttaaaaaataaatttagataaaaaaataagattcatttaaaaaacatgtcagaccttgggtaatttttttttattcaagtttggctcaaatttacaaaaaaaaagcatactactgttttttaactattatattgtcacttcaatattatattactattattttttattattatttagatattgtataatttttattttattattataattacttgttatgtattgtaaagcagtctgaattgatgagagacgcggaaattatgtattgagcttcactggagctaccgaaaaagatatgattgggcccttgatcgaagtccaatatctatgatctaaagtaaagaaaggcctattgggtgatagaaagagaacggtcatgaaaaccgaatgatttctttttcttggggcgataaaaccaaatgaaatggtgttttaagtatgcgtgtctctgatccattcattttgtagtcatgtactctctttcgtctcttcgtttcaatcgctgcgtttacatttcaatttattatcctctttctttccttgtattctagtttaataataaaatccaaattcaacaacaaaagcaaaactcaaatttgttgagcaaaaaaaaaaaaaacagatatcattttgtttgctcttttcctatttttggacttttctgtatattcactgtttgagaagaaagaattggggcatctctctctctttagttagattttattaatggagaaagaagagaagaggaagaagatggaggttgattcagttccagcagcagctttggaagggttttcaccagtctctacaactaggattttctggaattccaggaaaagatctggtacttcctttttcacttttcttcccctttttctttgttaatttcattttaggaaaaaaaagaaaagagagagctatgaacatgtttaattcactttccttctgtcttttttttttccttctattttccatgttttgacttttcttccctgatttattttcatcttcaattgaactaaattcatttgacaaactccttgttttaaacaaccaaaagaaaaagaaaatataaaattgatgacattagaaattcagagtgttttgtttgattggtgccatgtagtggttactttgctgctacgttaatttgccgggttttgcgtgccttagcataatgatcaattcatcatctatatatttcattttcttgtctattatcctgatttgattatcttttaatttccaacacgttttccctaattttttgttgatgctttggcttcaatgctgctttttttttgtatgtttaatattgcagttggtttacgtttacttgaaaaaactgttaaaaagaaaataaattagaacaaccaccacttataactttcttgtgcccaccatttccacctaactgatttgaatctcattctctaatatattcatttatttatatttctttgaataggttggaaaacagaaatttgttttctctaattctgtatatcatgtgacaatcaagcacgttaaaatcaagctcttaactagtttaaaaatgggttgggttttgggcatgtatttcttttttaaattcggtccggtccggtctggttgtataaattataaaggatcaattttatgatttacatgatgaaagactttcatttatttttaaatcttgattgacatcatgtgataaaaatatatatatctcttctttcgaggaattaactattttatttacaaatttgggttaacctatgctgacctagattgtgtttttacacgtgggatcctgtctaggcataattttttagttgtattttttggtcaggtccggtttggacagacaaatttttataaaagaaaaagtggaaaggataaatctaaatatctgttttttaaattaataaaaggccttggaagaggtttgacgtcatacgaatggagacttcctattcaaatctatataagcttctaattatgacttcaagcatatgttccttgttctgaaaatatgagctatttattcccaataaacctataccatggtaaattaaatttcaaattagctatggtagcaatcaagttcatatgatttgcttaacatgataaaccttttctttttaatgtatatttggtggataaaaacctcgaatttagaagaagatgcagaagaagaagggtgtgtcatttagaaactgtttcaaataagtcttagccaagtgtggagattagatttatgttacgttcaagtactttttgatggttttcatgtatttcaagaaaaaacacacaagtatgactgttaaacaagcagtttttagcttcataaattatttctatcttcacaattaagttcagtgaattcctgttttagaagatcgagtaagcttaaagaagcttggaacttaactacaaatgaggtttaaatggcttcatgtttggtttagaaatgcatctaaaattagttggaattagaatgttttaacttctctccgacagctagcgggaggaatttagacaaggtaacagaagagactgctaatgtgacacccaccaaacaggaagaacaaactcttgatcaagacaatacaccagattccgctacctcgtctgaactttccgagcgtcggaaggctctctttgagccactggaacctattaaaaacatcaatggccggcaaccgtcagcagagtctttgcttcccccaccagacttcgatgctgcgagctatccaaagggctggctaatcggaaagaagaggaagctggtaaatgttgacgttgttgagagcatgcgaaggattgcagtccaggaaatgaatagaaaggtctcatgtcatatacttaagctcctctcaaaacactagcatctatcttatattacattgactccaataaaagtcagatatggatatgtctaacacggatctgaatatttgtaagataagggtattttaagaaaaatgaagagtccatatgacatcttgatttgtagagtccatgtctaaataagtgctagatacgagaacttgaaaaagaaaaaaaagaaaaaaagagcgtatgcagctgatatggtgagaaagttgtataggataatgagtagagacgatggaaggtaataacttgaaatggttaaaatatgcaggacagggaaattgatgggttgaatgagcagttggaagaagatgcgaggtgcttagaacatctgcaacttcagcttttacaagagaaaagtaaaagatcagaggtggagagagaaaacgcaatgcttcaagaacaggtatccatgctgatgaatatgttgcaggaaggtgaggaaggtccagatgatcatgaaccttgaaaactttttcatttaattgttcttttctttgtagagttagttgttggaaaattagtaaagaagagcatgcaggatatatatggcatgcaatctaccctccccacgatttaaatttgcacccacccacccacagttagtcgcgtctcgtttgttgcagaagacatgatgaatattattgcaatgtattgtattatgtatgaaaaagaaaatgtcaaagctgtaaaatagtcggctacttaggtagatatgatttaagtttgttttggcgtgttacgtgtatgccaaattatactaaataaattgtttatctgtttggatttgtacactgccactgcatgattgttggttaaata

SEQ ID NO: 80 - DNA, 3442 bp, Gossypium hirsutum
  source 1..3442: mol_type = genomic DNA
aaaccgaatgatttctttttcttggggcgataaaaccaaatgaaatggtgttttaagtatgcgtgtctctgatccattcattttgtagtcatgtactctctttcgtctcttcgtttcaatcgctgcgtttacatttcaatttattatcctctttctttccttgtattctagtttaataataaaatccaaattcaacaacaaaagcaaaactcaaatttgttgagcaaaaaaaaaaacagatatcattttgtttgctcttttcctatttttggacttttctgtgtattcacagtttgagaagaaagaattggggcatctctctctctttagttagattttattaatggagaaagaagagaagaagaagaagatggaggtagattcagctccagcagcagctttggaagggttttcaccagtctctacaactaggattttctggaattccaggaaaagatctggtacttcctttttcacttttcttccccttttgctttgttaatttcattttagaaaaaaagagaaaaagaaaaagagagagagctatgaacatgtttaattcactttccttctgtctttttctttttccttctattttccatgttttgacttttcttatcatcttcaattgaactaaattcatttgacaaactccttgttttaaacgaccaaaagaaaaagaaaatataaaattgatgaattcatggtattgatgacttcagaaattcagagtgttttgtttgattggtgccatgtagtggttactttgctgctacgttaatttgccgggttttgcgtgccttagcataatgatcaattcatcatctatatatttcattttcttgtctattatcctgatttgattatcttttaatttccaacacgttttccctaattttttgttgatgctttggcttcaatgctttttttttttaaatattgcagttggtttacgtttacttgaaaaaactgttaaaaagaaaataaattagaacaaccaccacttagaactttcttgtgcccaccatttccacctaactgatttgaatctctttctctaatttattcatttatttgtatttctttgaataggttggaaaacagaaatttgttttctctatttctgtatatcatgtgacaatcaagcacgttaaaattaagctcttaactagtttaaaaatgggttgggttttgggcatgtatttcttttttaaattcggtccggaaggattttaaatcttgattgacatcatgtgataaaaaatatatataggaattaattattttatttacaaatttgggttaacctatgctgacctagattgtgtttttacacgtgggatcctgtctaggcataattttctagttgtattttttggtcaggtccggtttagacagacaaatttttataaaagaaaaagtggaaaggataaaatctaaatatttgttttttaaattaataaaaggccttggaagacgtttgacgtcctaggaatggagacttcctaatcaaatctttagaagcttctaattatgacttcaagcatatgttccttgttctgaaaatatgagctatttgttcccaataaacctataccgtggtaaattaaatttcaaattagctatggtagcaatcaagtttatatgatttgcttaacatgataaaccttttctttataatgtatatttggaggataaaaacctcgaatttagaagaagatgaagggtgtgtcatttagaaactgtttcaaataagtcttagccaagtgtgtagattagatttatgttacgttcaagtaccttttgaaggttttcatgtatttcaagaaaaaacacacaagtacgactgttaaacaagcagtttttagcttcataaattatttctatcttcacaattaagttcagtgaattcctgttttagaagatccagtaagcttaaagaagcttggaacttaactacaaatgaggtttaaatggcttcatgtttggtttagaaatgcatctaaaattagttggaattagaatgttttaacttctctccgacagctagcgggaggaatttagacaaggtaacagaagagactgctaatgtgacacccaccaaacaggaagaacaaactcttgatcaagacaatacaccggattccgctacctcttctgaactttccgagcgtcggaaggctctctttgaaccactggaacctattaaaaacatcaatggccggcgaccatcagctgagtctttgcttcccccaccagacttcgatgctgcgagctatccaaagggctggctgattggaaagaagaggaagctggtaaatgttgacgttgttgagagcatgcggaggattgcagtccaggaaatgaatagaaaggtctcatgtcatatacttaacctcctctcaaaacactagcatctatcttatattaccttgactccaataaatgtcagatatggatatgtctaacacggatctgaatatttgtaagataagggtattttaagaaaaatgaagagtccatatgacatcttgatttgtagagtccatgtctaaataagtgctagatacgagaacttgaaaaagaaaaaaagaaaaaagagcgtatgcagctgatatggtgagaaagttgtataggataatgagtagagacgatggaaggtaataacttgaaatggttaaaatatgcaggacagggaaattgatgggttgaatgagcagttggaagaagatgcgaggtgcttagaacatctgcaacttcagcttttacaagagaaaagtaaaagatcagaggtggagagagaaaacgcaatgcttcaagaacaggtatccatgctgatgaatatgttgcaggaaggtgaggaaggtccagatgatcatgaaccttgaaaacattttcatttaattgttcttttctttgtagagttagttgtcggaaaattagtaaagaagagcatgcaggatatatatggcatgcaatctaccctccccacgatttaaatttgcacccacccacagttagtcgcgtctcgtttgttgcagaagacatgacgaatattattgcaatgtattatgtatgcaaaagaaaatgtcaaagctgtaaaatagtcggctacttaggtagatatgatttaagtttgttttggcgtggatgccaaattatactaaataaattatctgtttggatttttacactgcaactgcatgattgttggttaaataatcgcgttctttctcaactctggataagcttgtgaaacaaatttataagcctgcagagaaaaaggaatgggaatgggaattggaccataaccccataggcaaaacaagaaaaggaaaaacaaatttttcttatgaatgcataaaaagactaattgcttttgattgggaaattgagctcaaacatatgttttgtgaagagaatcgattagctaatcgaatga

SEQ ID NO: 81 - protein, 214 aa, Gossypium hirsutum
MEKEEKRKKMEVDSVPAAALEGFSPVSTTRIFWNSRKRSASGRNLDKVTEETANVTPTKQEEQTLDQDNTPDSATSSELSERRKALFEPLEPIKNINGRQPSAESLLPPPDFDAASYPKGWLIGKKRKLVNVDVVESMRRIAVQEMNRKDREIDGLNEQLEEDARCLEHLQLQLLQEKSKRSEVERENAMLQEQVSMLMNMLQEGEEGPDDHEP

SEQ ID NO: 82 - protein, 195 aa, Gossypium hirsutum
MEKEEKKKKMEVDSAPAAALEGFSPVSTTRIFWNSRKRSASGRNLDKVTEETANVTPTKQEEQTLDQDNTPDSATSSELSERRKALFEPLEPIKNINGRRPSAESLLPPPDFDAASYPKGWLIGKKRKLVNVDVVESMRRIAVQEMNRKDREIDGLNEQLEEDARCLEHLQLQLLQEKSKRSEVERENAMLQEQS

SEQ ID NO: 83 - DNA, 3235 bp, Gossypium raimondii
  source 1..3235: mol_type = genomic DNA
gatctaaagtaaagaaaggcccattttgggtgaaagaaagagaatggtcatgaaaaccgaatgatttctttttcttggggcgataaaaccaaatgaaatggtgttttaagtatgcgtgtgtctgatccattcattttgtagtcatgttctctctttcgtctcttcgtttcaatcgctgcgtttacatttcaatttattatcctctttctttccttgtattctagtttaataataaaatccaaattcaacaacaaaagcaaaactcaaatttgtcgagcaaaaaaaaaaaaaacagatatcattttgtttgctcttttcctatttttggacttttctgtgtattcacagtttgagacgaaagaattggggcatctctctctctttagttagatttattaatggagaaagaagagaagaagaagaagatggaggtagattcagctccagcagcagctttggaagggttttcaccagtctctacaactaggattttctggaattccaggaaaagatctggtacttcctttttcacttttcttccccttttgctttgttaatttcattttagaaaaaaagagaaaaagaaaaagagagagagctatgaacatgtttaattcactttccttctgtctttttctttttccttctattttccatgttttgacttttcttatcatcttcaattgaactaaattcatttgacaaactccttgttttgaacgaccaaaagaaaaagaaaatataaaattgatgaattcatggtattgatgactttagaaattcagagtgttttgtttgattggtgccatgtagtggttactttgctgctacgttaatttgccgggttttgcgtgccttagcataatgatcaattcatcatctatatatttcattttcttgtctattatcctgatttgattatcttttaatttccaacacgctttccctaattttttgttgatgctttggcttcaatgctttttttttttttgtatgtttaatattgcagttggtttacgtttacttgaaaaaactgttaaaaagaaaataaattagaacaaccaccacttagaactttcttgtgcccaccatttccacctaactgatttgaatctctttctctaatttattcatttatttatatttctttgaataggttggaaaacagaaatttgttttctctatttctgtatatcatgtgacaatcaagcacgttaaaattaagctcttaactagtttaaaaatgggttgggttttgggcatgtatttcttttttaaattcggtccggaaggattttaaatcttgattgacatcatgtgataaaatatatatatatatatatctcttctttcgaggaattaattattttatttacaaatttgggttaacctatgctgacctagattgtgtttttacacctgggatcctgtctaggcataattttctagttgtattttttggtcaggtccggtttagacagacaattttttataaaacaaaaagtggaaaggataaaatctaaatatttgtttttttgacgtcctaggaatggagacttcctaatcaaatctatagaagcttctaattatgacttcaagcatatgttcatatgagctatttgttcccaataaacctataccgtggtaaattaaaccttttctttttaatgtatatttggaggataaaaacctcgaatttagaggaagatgaagggtgtgtcatttagaaactgtttcaaataagtcttagccaagagtgtagattagatttatgttacgttcaagtaccttttgaaggttttcatgtatttcaagaaaaaacacacaagtacgactgttaaacaagcagtttttagcttcataaattatttctatcttcacaattaagttcagtgaattcctgttttagaagatcgagtaagcttaaagaagcttggaacttaactacaaatgaggtttaaatggcttcatgtttggtttagaaatgcatctaaaattagttggaattagaatgttttaacttctctccgacagctagcgggaggaatttagacaaggtaacagaagagactgctaatgtgacacccaccaaacaggaagaacaaactcttgatcaagacaatacaccggattccgctacctcttctgaactttccgagcgtcggaaggctctctttgaaccactggaacctattaaaaacatcaatggccggcgaccatcagctgagtctttgcttcccccaccagacttcgatgctgcgagctatccaaagggctggctgattggaaagaagaggaagctggtaaatgttgacgttgttgagagcatgcggaggattgcagtccaggaaatgaatagaaaggtctcatgtcatatacttaacctcctctcaaaacactagcatctatcttatattacattgactccaataaatgtcagatatggatatgtctaacacggatctgaatatttgtaagataagggtattttaagaaaaatgaagagtccatatgacatcttgatttgtagagtccatgtctaaataagtgctagatacgagaacttgaaaaagaaaaaaagaaaaaagagcgtatgcagctgatatggtgagaaagttgtataggataatgagtagagacgatggaaggtaataacttgaaatggttaaaatatgcaggacagggaaattgatgggttgaatgagcagttggaagaagatgcgaggtgcttagaacatctgcaacttcagcttttacaagagaaaagtaaaagatcagaggtggagagagaaaacgcaatgcttcaagaacaggtatccatgctgatgaatatgttgcaggaaggtgaggaaggtccagatgatcatgaaccttgaaaacattttcatttaattgttcttttctttgtagagttagttgtcggaaaattagtaaagaagggcatgcaggatatatatggcatgcaatctaccctccccacgatttaaatttgcacccacccacccacagttagtcgcgtctcgtttgttgcagaagacatgatgaatattattgcaatgtattatgtatgaaaaagaaaatgtcaaagctgtaaaatagtcggctacttaggtagatatgatttaagtttgttttggcgtggatgccaaattatactaaataaattgtttatctgtttggatttttacactgcaactgcatgattgttggttaaataatcgcgttctttctcaac

SEQ ID NO: 84 - protein, 214 aa, Gossypium raimondii
MEKEEKKKKMEVDSAPAAALEGFSPVSTTRIFWNSRKRSASGRNLDKVTEETANVTPTKQEEQTLDQDNTPDSATSSELSERRKALFEPLEPIKNINGRRPSAESLLPPPDFDAASYPKGWLIGKKRKLVNVDVVESMRRIAVQEMNRKDREIDGLNEQLEEDARCLEHLQLQLLQEKSKRSEVERENAMLQEQVSMLMNMLQEGEEGPDDHEP

SEQ ID NO: 85 - protein, 195 aa, Gossypium raimondii; identical to SEQ ID NO: 82

SEQ ID NO: 86 - protein, 194 aa, Gossypium raimondii
MEKEEKKKKMEVDSAPAAALEGFSPVSTTRIFWNSRKRSASGRNLDKVTEETANVTPTKQEEQTLDQDNTPDSATSSELSERRKALFEPLEPIKNINGRRPSAESLLPPPDFDAASYPKGWLIGKKRKLDREIDGLNEQLEEDARCLEHLQLQLLQEKSKRSEVERENAMLQEQVSMLMNMLQEGEEGPDDHEP

SEQ ID NO: 87 - DNA, 2216 bp, Lactuca sativa
  source 1..2216: mol_type = genomic DNA
cgccaaatcgcgttcgtccaatttcctcgatctcaccgtttaatattttctcatcggtgaacaacatatgtacgttatacaattcaacaactcagcctcagctcagacagaataaccagaataaattctctctcatctattgctgtttccatgtcttttcaaccgccaactgtgtgtacgtgaggtttttgagaagagatttggtggaattagttgaattgtgatcgatttttgttgattcgtagttgcgaattttgacggagtaatggatgacggaaagaagatggagaatagcgtcgttaatggcttctctccggtgtcttctactccagttttctggaaatctcggaagagatcaggtaattcgagtttgaatacgagtatgcgttttcgtgaatcattttaagcataattgagtaattttgtgattgatttctcttcttcttcttattgttgttgattcaattacgtacggtagtagatctgtatatccacatgttgtggcagtttgaatatttgatgatcatgatgttcggagcaaatttagatagggagtaggtggccgattttgcaaaatgttattgtaaaatgggtaaatagttttggaaaatttaattagaaatagattcatagttctagttttgacagatatcatctggttactgctgataattcagggttatgaattaaattgatttagcagtttctggttgcagcgagtgcgaagaatttgtacaaggacattgtagatgaaggtgataagacttcagagaagaaggaagagcaggtgacaacaacagatgaaaaaatggaagactcattatcaactccacccacagttctgtccgagaaacgtaaggctctttttgaacctttggagccaataatggatttgagtggtagaagaccttcagctgaatccttactccctccgccggactttgacactgccagttacccacgtggatggctaattgggaagaaacggaagcttgtaaatgtggatgttgttgaaagcatgcgtaggattgcagtacaggaaatgaacagaaaggtattgtacctttgcacgctttctttttataattggattttaatatatcattaaaagacactaatcctactcgactttaccccctttgcctttttagtctaaaactgtacttgaatataataaaaatcataacaatcctactgaagataaacagatagcaactcaccattttttctattgatatcccgtttatatgtgtgtatgtgtgggaaagaagagcaggccacatgtcggactttaaatgtggtccatttttgctattatgagatataaaaccttgtaccttgtgtatatttttataaaaatggttaaatgcaagaaacaatcacatatacacatacaagctagctcaaaaactatgttatttcaataacaataactatgcaagaaacaataactatattaaccttgtactaagatacgataagctacttttgcaataatcataaaaaataagcttgcttataaaacgccaacacagccttattaactagctatcataacattctactttcatttcctcctaatacaacatagtacttcggaaaaaaaatatccaattgtagcaacatcatcaaaatacaatataatttgcactgctataattgggtggacttttcaaaatataatgtccgaataaaaaatgatatgaaagtagactgctatgaggtaacattctgctttcgtttcatcctattacaacattgtactttgataaatttatcaattatagcaatttcatcaaaatacaatgcaatttgctttgcaataatttggtagatttaaaaaaataggatgtctgaataaatataatttgaaggtagaatgctataaccaggtaacattctaatcctattacaacatttactatgaacaatgtatcgtttatatatagatatatgctatggaatctaactgtgaatacaggacagagagattaacggacttaacgagcagttagaagaagatgcacgtgtccttgagcaccttcaactccaactgcttgatgaacgaagcaaacgcgcagatgttgagcgacagaatacaatgctgcagaaccaggtggatatgctcatgaatatgcttcaggagcctgaaaatatcgatgatgaagatggctcacaagaaccataagtaagtctgttccttttttttttttttt

SEQ ID NO: 88 - DNA, 2129 bp, Lactuca sativa
  source 1..2129: mol_type = genomic DNA
tactacctcctggtttttcgtaatatcgcaaaaaatcctgtgcatttcagtaaatttgacattttgtaatcctttgttgcaggaaagaaaaggtcccagaaatcagaatagaaggatagagtaatatgaaagcagacgaaaagagacaacaaaccaaacctcatccaccgtggagactcagtcgaccctacaatcatcaaatcctagccgtccaatttccataccactgatcctatcggcaccattaaaaataaaactcttgtgcgttaagcgacaactacacgatttacaagaacaacaactaacaacaaacaatataccagaagaaaacgaagcgaatctctctctttctatctttcgctttctcattcttccttttaaattttatctctgtgtatcgtattctgtgatttcagttttttgaagttataaacaacgagaagattggtgaagttgattgattggtgagtttgtaaacagaggagaaatggaagaaggtaagaaggaggtgcagagtattctcgttaatggcttctctccggtcacttctacgcctgttttctggaaatctcgcaagagagcaggtaatcaacgttttttttcgaagtttgtgtaattatttcacgattaatgagttttatgtgtaacgatataaactgttgctgatttaattgttaagagctgtagatctgtgttctttcatgttggaaatagttcgacattcatgatttttgaagcggatattattatgaatttaatgttactttgatcaaacgaaagaggaaaccggagtcgttaaggtcaaattttcatttcgaaaagtcaaaattatttataaaagttaataaaatttatagttgttcgtaagttccttaatacaattatgaacatttaataaacgatcaaaatattgcttttaatagatgaatacaactatacaaggagatacgcaattattttatgtgatttgatggccaacaggcaacaaattttgacttttcattgctgatattataatacatcaatttggaataggaaaaataatgttttaaaatataattacgtgttttttttttcttattgatttagcagctttatggttgcagctagtatgaagaatttgtacaaggacaatattaaagactcaactgaagataaagataaaataaacgagcacaataacgataacaataacaataaagatgattccattgatgagaaaatggaagaaacaagtatactttcagagaaacgtaaggctctgtttgaacctcttgaaccaataatggatttgaatgggagaagaccttcagctgaatccttacttcccccacccgactttgactctgccagttaccctcgcggatggctcattgggaagaaacgaaagcttgtaaacgttgacgttgttgaaagcatgcgcaggattgccgtacaagaaatgaacagaaaggtatacagtacatgacatgacaaaacaaattgtattgcattttttgacgtcagaggataaaattgcaatatttttgctccaacgtaatatgataaatatcatatgagatggatgtcataggacataatagcccaagaaaattgtacacactagacagactggtttagtcttcttcagttcagttcagtctaatctaacctagctcatttagttcagtacattctagtctagtccaacccaatctcatctattactagtccagcccaatctcatctattaagttcaatccaatccagtataagtctagtctcatccaagtgaaatatgaagatggattgattaattgcaggatagagagattgatgggctaaacgagcagttggaagaggattcgcgtgtgcttgaacatcttcagttgcagttactagatgaacgaagcaagcgtagtgatgttgagagacagaatgcaatgttgcagaatcaggttgatatgcttatgaatatgcttcaagaacatgagaacttggaagatgatgaaatcccacaagatccttagtttagtgtacttttattttttttgttatgatgatattatttcatttggcgttgtttgtgagtctgatataatatatacaaattacaagcatacgtgtcatccagaataactgaaataaat

SEQ ID NO: 89 - protein, 212 aa, Lactuca sativa
MDDGKKMENSVVNGFSPVSSTPVFWKSRKRSASAKNLYKDIVDEGDKTSEKKEEQVTTTDEKMEDSLSTPPTVLSEKRKALFEPLEPIMDLSGRRPSAESLLPPPDFDTASYPRGWLIGKKRKLVNVDVVESMRRIAVQEMNRKDREINGLNEQLEEDARVLEHLQLQLLDERSKRADVERQNTMLQNQVDMLMNMLQEPENIDDEDGSQEP

SEQ ID NO: 90 - protein, 216 aa, Lactuca sativa
MEEGKKEVQSILVNGFSPVTSTPVFWKSRKRAASMKNLYKDNIKDSTEDKDKINEHNNDNNNNKDDSIDEKMEETSILSEKRKALFEPLEPIMDLNGRRPSAESLLPPPDFDSASYPRGWLIGKKRKLVNVDVVESMRRIAVQEMNRKDREIDGLNEQLEEDSRVLEHLQLQLLDERSKRSDVERQNAMLQNQVDMLMNMLQEHENLEDDEIPQDP

SEQ ID NO: 91 - DNA, 528 bp, Carica papaya
  source 1..528: mol_type = genomic DNA
atgctgataccacccctgatgtgcctgttaaactggagctttctgatcgacgaaaggctctgtttgaaacctttagaacctctgggaaatattagtggtcgtggaactcagccgaatcctttactacctccaccagacttcgactctgctgcatacccgaaaggttggctcattggaaagaagcgaaagctagttaatgtggatgtggttgagagcatgcgcaggattgctattcaggagatgaacagaaaggtgaagatacacacatcaaggcattaacctaatcctgcattcttgcctaattgtagtttaaattttctgcaggatcgggaaatagatggtctaaatgagcagttagaagaggattcgaggtgcttacaacatttacagcttcagcttctgcaagaacgaagcaaaagtgcagatgtagaaagacaaaacaaaatgctgcaagagcaggtgtctatgcttatgaatatgttacaagaaccagtgatagtggaggatgaaggcacagatcaagcttaa

SEQ ID NO: 92 - protein, 151 aa, Carica papaya
MLIPPLMCLLNWSFLIDERLCLKPLEPLGNISGRGTQPNPLLPPPDFDSAAYPKGWLIGKKRKLVNVDVVESMRRIAIQEMNRKDREIDGLNEQLEEDSRCLQHLQLQLLQERSKSADVERQNKMLQEQVSMLMNMLQEPVIVEDEGTDQA

SEQ ID NO: 93 - DNA, 2992 bp, Ricinus communis
  source 1..2992: mol_type = genomic DNA
atgaagctttcaagaagtgcttctttaatggaaaaggataagaagtacgatagtaaacaagggaagaaggtcgatgatgggcttttgaatggattctctatatcctctactcctaatatctcctggaaatctagaaggagatcaggtagctagttcttactctttttcctttttgtttctttacttttttgtttgctttccgagaaagtaataatcaaagagaaaaagaaagaaagaaagaagctggctttctgatatttttcttgttacaaaatcatatatcaagagaacccacatcttgaaattttgattgaagttgaagatctaaattaaaatagccgactcttacccattttcataattggaataattaaggttttacgaattctgtattgagacaaagtaagagaataactttgacatctgttattgatatgaccagctgttattagggctgttaagaatgttatgacttgctgttagacagttactttgctgctacgttaattcttgaggttaggttgcttaccagtcactctctcctcattatcaccattcttatttttatatctccttttcctttttattttttcaaattctttttattcataatatattttcttatctttcatgaaaatcatgtcttttattattattattattattattattattattattattatgattattgttttgccactgatttcgtttctgctaaaattcatgtattgatgaaatttttatttacctatattttatcaagatttgttccactgacttttccacatgcattctttttttttttttttttaaaaaaaaagagaatgcaatatttagttttattaattttaattttttgtatttaatttaagttatttaatagattttcaagttgaatgcaaattatttaatgtgaacaaaaaaattgaaaaatctctgaatttctattattcccttcaataccgatgttccgacaaactaaaagagttcggaatagagatttttatgttccggtgcaattctaaggatgtaataatgaatttctgtttggaaactgtcggattctcccaaagcgtgatgacccctaaatgaaacatttcaatgccgtttaaaaagaacaaaatagaaaggaacatttcagtgacaatcatcatttgcatgtgagtagggcaatatcaatacgaatttttaatgcgaagtagttggacgagggaaagatgagtctttgaggaaataatataatttaaactcatttgatcactttcgtataagctttcaggaaactgtttcttaaaagaacagagttttcgtttgcaaattggtgtcattgaaactatgtcgcttttgggctatttggtcaactgctgctttgctttttctattcgaatggtctttttttcttttaattaatagagtctcccagtcaacagtgactctttaacattcttatttatttttacaactcttctttaagaaaagattgcaattatgtaatagtaatttcgagacagcaaattcaagtatgttttttctgtttctccttttctcatgatttcttccttttgttttattctaataagctttggtaaaagttttcagactccgtgcaaaattctcttacagttaatttgccctcagcttatgctttggtaactactatacacagttcagtgtctttaaatttttaaaggaagaagaagcaaacaatggctggctgtgtttccaattgacaatgaccctgaatcttcgtcactgacccgtagcttgtctgtagtattttctcctgcttttaattctaaccagcaactttatcacaataggaatgctctatagtctgtactattgaactctctgctccataatgtaccctaattttaattcctcgacattttggagatcataagttagtttactaattaacctagtaagcatgctctagtccgtcctgtcatgcagcaagaaacttgtcattgcatttgccaaagtaggaaagacagaatattgaagggagataattaaaaatcttctctttgattggaagaaaatttaaaggtggatgaaatgggaagaggtcgtaatggggggaatcttgctgtaagactcgattcagtggatagaatattcactagccctttaggcttaaaatcggataatacaggacgttggtgtactgaaaggaaaaatatggttgcatttcaattttagtatctgcaactttcccttcaaagcttttgatgcgtggagctgcagggagcaggaatacacccaacatcattgtattttcttatgctatcagtgtttctaagtttctcacgtgttctaaaatagttggaactagaatggtaacttctttccaacagctagtgcgaggaattctgacaaggtaacaaacgacactgctaatgaaacaccacccgacaaacaggaagaatcttacaatgacgaaaagatggaggagctaaatgcagttccagtgctttctgagaagcggaaggctctctttgaaccactggaacctgtaaacaatatcaatggccggcgatcatcagctgaatctctgctccccccaccagattttgatgccgcaagctatccaaaggggtggctgattggaaagaagcgtaagcttgtcaatgtagatgttgtcgagagcatgcgaaggattgctgttcaggaaatgaacagaaaggtaactttccatacacctgacatctcctaatcatgtatggttgcacgggcagaaaaaaccatcattgaatatttctttcaggaccgggagattgatggcctaaacgaacaattggaagaagacgcaaggtgtctagagcacctgcaagtacagcttctgcaggagcggagtaaaagagcagaggtagaaagagaaaataccatgctgcaagaccaagtaaccatgctgatgaacatgctgcaggacaacgagccaatgggtgatgaaggcgcaggagatgaaggtcctgatgaaccttaa

SEQ ID NO: 94 - protein, 230 aa, Ricinus communis
MKLSRSASLMEKDKKYDSKQGKKVDDGLLNGFSISSTPNISWKSRRRSASARNSDKVTNDTANETPPDKQEESYNDEKMEELNAVPVLSEKRKALFEPLEPVNNINGRRSSAESLLPPPDFDAASYPKGWLIGKKRKLVNVDVVESMRRIAVQEMNRKDREIDGLNEQLEEDARCLEHLQVQLLQERSKRAEVERENTMLQDQVTMLMNMLQDNEPMGDEGAGDEGPDEP

SEQ ID NO: 95 - DNA, 3626 bp, Citrus clementina
  source 1..3626: mol_type = genomic DNA
gttgttgatggtcccgccacgcttctgacaactaacagcacattttcacaaactcttaacacaacgatgctctccttacaagtcttggatttatcttcttcttcttctcttcaaaaaaacaaaaacaaaagcaaagcaaacctcaacttttgagctgaagaaagctaccagtggttgattttattaattttttttttattttttaagttttaatggaaaaaacgaattttcatcctgtcaagaagcagcatcagcagaggctgcacaaggttgatgatgcacctttgactggcttctcccctgtttctgctcctaggattttttggaggtctcgcaagagatcaggtagtagatgcaatttttttttttttacttttttctggggctttcagtttgtcagcttcttgtttgtttctcaggaaaattatgtgaaaatggtaaaatttgctaacttgaacttggtctgtggctgtttgcatgatttagcacatacccatttcatatttgatcaagtcctgctagaaattttatccttttttgcatgtttgtgaaagatctgtatttctcaaaaatgtgattttttaagcggtgtttattattaatctttttgaagctgaatcatttttttttcttttccttctttttcattcctcttggtttcttcatttatttaattattcttgtaaaagtttcttttgttggtggagaaggtggagagaataattttttgacttgccgttgctttgcccctaagctaattttactggatttggctggctaactagtctctgtcaatttcatgatttttatctgtttctttcattttactttaccttatttttcattttcttgtctattacctcaataatgatagggtccattctttttcctttttgtgcatctttagttttagcttttatgtgcattcatggttcaatttcctgggcagcagcagattgtttgttcattgtcttaattgctcttgtatgttttgacattgagcaagctgcattactttacaatttattgttcatctaactgtcatcaaactcagcagtttttatttattaataaaaatggaaacataagacggttggggttgattcttcttgttccctttacaatagatctaactaattaggctattcattagggacaatggtaggtagacagatataattgggctatataatcttcagaaacttatgaagattatatattgataaggcatagaatagaaaaataaactaatatgagttttgatccaaaggagagagctggagactttaatattttgcattattaagataaagtgctgcaattttgaccgagtagtgatattgacaatttcaccacaccaaacacatggggtgatccaaatagtagttgggtgaaaatttttgaaattgttctctctttcaattctattttttgttcttaccaataaaataaaataaaattcctgatgtagctggatgggatttgttgtgaaatacttaaaatagtataatatatatatatattaaggaatgcttgcatgcaggttttgcaaaacagggattagattagaacttaacctcccttgcctcacaaacatggaaaaccaaaagtatttctaataactgataaaaattaaacaaaactatgcaaaggcaacaaagctatatggagatgaagcaaaagagaattagagaacacttatcaatctttagatttcatgacatgcgttcaagttgaatgccaactttgagttagatgaatctacatatgttttatctgatcactgccaaatttccctaaatcttcaaaatttcatagtcttcatcatttcttcgattaattatgtattacattatacgatagtgattccaagcattacttgtttccctagaccaagaagggaaatagtttgcattacttgcaaactatttttgcctgcctatttgaatgatttaccattcggcatactcccagctagcctttcacgtgttgataagtctattgtttcacttagcgtatgctggagtttagaattaggtgttgagacgtatttttcagcatacaaataaacctagggaggccaccatatgtactcatacatgaggaaaagttgaatagctttaaatgttatacaaatcagagcaccttgtcccaatgtaaggttttgttgcttaacatattgtggattttgagtggcatcatacagtataatgtaaaaatattgtcaagggctccatcatatattcaaatccaaatggctccatgaggatatatgccttcgaagacattttaaaagtgaaaatgtttcagttgtagttacagcctatagatggccagttgtaattacagcctataggtgggtcaagttcttcggaacatccaaatccagctcctgcatttcaacgatcctctatgtcccaccacctcctctccctcgcattggaattttgcctgagatagattctgtgtccttgatgttttctgcatgctgaccagcatgatgacctgcttggttaagtgacgcttaaattattatgacatactttgctttttcttggaatatgcattgaagaaagtatttgcgagtgtaaccatatattgtctcaacattactatgttaagattggcaatatctgtagaagtgtttggaattagaaaagtatcttctttctaacagctagcgggaggaatttcgacgtaacaggagacagcgctaacgaaacgcccatcaataaggatgaaaacccagatcaagagatggaacagcagcaaactccagaacctgtcctcaccgagcgacgaaagtctctctttgaaccactggagcctaacaatggcaagcggaaatcagctgaatccttactacccccaccagactttgattctgccgcctatcccaagggttggctgattgggaagaagcgtaagttagtaaatgttgatgtcgttgagagtatgcgaaggattgccgtccaggaaataaatagaaaggtgctgttccaaacatgtcacctcctctcttaacatatgcgcacacaataacaaattatgaacctgtgaacacacacacaccctgcttgctgagagagccagaaaattgtattgcaacaaaaattcatggaatgaattacctagtgattaattttgcaggaccgggaaatcgatggactaaatgaacaactggaagaggatgcacgttgcctggagcatctgcaactccaacttctagaagagcggagcaaacgttcagaggttgagagagaaaacggaatgctgcaagaacagataaacatgctgatgaacatgttgcaggaaaatgagacaatgggggacgagggtgcagatgaaccttgagcatagtttgtttaatgtttgtttgtttattcttttgtacgttagttttgggaactgtagaaaggagtcacacatgcatacatatatatatatatatatatatatatgcctagctagtccaatagaattataggtatactaagttgccattatagcttgcttgatgcttcaagaccttgctcatgcttattactgtttgtaatgaactttcacaaattatatcaaactgatgtaattattatgcatcaaagaattctttatttgtgaatggt

SEQ ID NO: 96 - protein, 216 aa, Citrus clementina
MEKTNFHPVKKQHQQRLHKVDDAPLTGFSPVSAPRIFWRSRKRSASGRNFDVTGDSANETPINKDENPDQEMEQQQTPEPVLTERRKSLFEPLEPNNGKRKSAESLLPPPDFDSAAYPKGWLIGKKRKLVNVDVVESMRRIAVQEINRKDREIDGLNEQLEEDARCLEHLQLQLLEERSKRSEVERENGMLQEQINMLMNMLQENETMGDEGADEP

SEQ ID NO: 97 - DNA, 6733 bp, Citrus sinensis
  source 1..6733: mol_type = genomic DNA
tatactaccaccatatagtataataataaagccgcatgaaatctgtattaattattggagaagctctctcttttccaatacacatccactgatacacaaatacatatacatataatgataaacataaatcgccaaacaaataaacaacaaataaaataagcaaaagaaagaaaataaaaacatggaaaatgctgtgggccccacggaaaagacaaatgtagacgtaaaatcttccgaaggcaaaaccaaacgtaaaccgtagatgaaagttgttgatggtcccgccacgcttctgacaactaacagcacattttcacaaactcttaacacaacgatgctctccttacaagtcttggatttatcttcttcttcttctcttcaaaaaaacaaaaacaaaagcaaagcaaacctcaacttttgagctgaagaaagctaccagtggttgattttattaattttttttttattttttaagttttaatggaaaaaacgaattttcatcctgtcaagaagcagcatcagcagaggctgcacaaggttgatgatgcacctttgactggcttctcccctgtttctgctcctaggattttttggaggtctcgcaagagatcaggtagtagatgcaattttttttttaaacttttttctggggctttcagtttgtcagcttcttgtttgtttctcaggaaaattatgtgaaaatggtaaaatttgctaacttgaacttggtctgtggctgtttgcatgatttagcacatacccatttcatatttgatcaagtcctgctagaaattttatccttttttgcatgtttgtgaaagatctgtatttctcaaaaatgtgattttttaagcggtgtttattattaatctttttgaagctgaatcattttttttttcttttccttctttttcattcctcttggtttcttcatttatttaattattcttgtaaaagtttcttttgttggtggagaaggtggagagaataattttttgacttgccgttgctttgcccctaagctaattttactggatttggctggctaactagtctctgtcaatttcatgatttttatctgtttctttcattttactttaccttatttttcattttcttgtctattacctcaataatgatagggtccattctttttcctttttgtgcatctttagttttagcttttatgtgcattcatggttcaatttcctgggcggcagcagattgtttgttcattgtcttaattgctcttgtatattttgacattgagcaagctgcattactttacaatttattgttcatctaactgtcatcaaactcagcagtttttatttattaataaaaatggaaacataagacggttggggttgattcttcttgttccctttacaatagatctaactaattaggctattcattagggacaatggtaggtagacagatataattgggctatataatcttcagaaacttatgaagattatatattgataaggcatagaatagaaaaataaactaatatgagttttgatccaaaggagagagctggagactttaatattttgcattattaagataaagtgctgcaattttgaccgagtagtgatattgacaatttcaccacaccaaacacatggggtgatccaaatagtagttgggtgaaaatttttgaaattgttctctctttcaattctattttttgttcttaccaataaaataaaataaaattcctgatgtagctggatgggatttgttgtgaaatacttaaaatagtataatatatatatatattaaggaatgcttgcatgcaggttttgcaaaacagggattagattagaacttaacctcccttgcctcacaaacatggaaaaccaaaagtatttctaataactgataaaaattaaacaaaactatgcaaaggcaacaaagctatatggagatgaagcaaaagagaattagagaacacttatcaatctttagatttcatgacatgcgttcaagttgaatgccaactttgagttagatgaatctacatatgttttatctgatcactgccaaatttccctaaatcttcaaaatttcatagtcttcatcatttcttcgattaattatgtattacattatacaatagtgattccaagcattacttgtttccctagaccaagaagggaagtaggctaaactgatttgcaaactatttttgcctgcctatttgaatgatttaccattcggcatactcgcagctagcctttcacatgttgataagtctattgtttcacttagcgtatgctggagtttagaattaggttttgagacgtatttttcagcatacaaataaccctagggaggccaccatatgtactcatacatgaggaaaagttgaatagcgttaaatgttatacaaatcagagcaccttgtcccaatgtaaggttttgttgcttaacatattgtggattttgagtggcatcatacagtataatgtaaaaatattgtcaagggctccatcatatattcaaatccaaatggctccatgaggatatatgcgttcgaagacattttaaaagtgaaaatgtttcagttgtagttacagcctataggtggccagttgtaattacagcctataggtgggtcaagttcttcggaacatccaaatccagctcctgcatttcaacgatcctctatgtcccaccacctcctctccctcacattggaattttgcctcagatagattctgtgtccaccattgatgttttctgcatgctgaccagcatgatgacctgcttggttaagtgaagcttaaattattatgacatactttgctttttcttggaatatgcattgaagaaagtatttgcgagtgtaaccatatattgtctcaacattactatgttaagattggcaatatctgtagaagtgtttggaattagaatagtatcttctttctaacagctagcaggaggaatttcgacgtaacaggagacagcgctaacgaaatgcccatcaataaggatgaaaccccagatcaagagatggaacagcggcaaactccagaacctgtcctcaccgagcgacgaaagtctctctttgaaccactggagcctaacaatggcaagcggaaatcagctgaatccttactacccccaccagactttgattctgccgcctatcccaagggttggctgattgggaagaagcgtaagttagtaaatgttgatgtcgttgagagcatgcgaaggattgctgtccaggaaataaatagaaaggtgctgttccaaacatgtcacctcctctcttaacatatgcgcacacaataacaaattatgaacctgtgaacacacacacaccctgcttgctgagagagccagaaaattgtattgcaacaaaaattcatggaatgaattacctagtgattaattttgcaggaccgggaaatcgatggactaaatgaacaactggaagaggatgcacgttgcctggagcatctgcaactccaacttctagaagagcggagcaaacgttcagaggttgagagagaaaacggaatgctgcaagaacagataaacatgctgatgaacatgttgcaggaaaatgagacaatgggggacgagggtgcagatgaaccttgagcatagtttgtttaatcgtttgtttgtttattcttttgtacgttagttttgggaactgtagaaaggagtcacacatgcatatatatatatatatatatgcctagctagtccaatagaattataggtatactaagttgccattatagcttgcttgatgcttcaagaccttgctcatgcttattactgtttgtaatgaactttcacaaattatatcaaactgatgtaattattatgcatcaaagaattctttatttgtgaatggttctcttctaaacaatatttcacttatcagaggatgaaccacatcagtttttgtcagtctcatttttgtctcaggactttcataaccctgaaggtacctaaattttctctcaaaaaattacttgacacggactgtaatgatctcaggctttgatagcaagaatgtgtgaaaccatatctcattttgcaagtcccattcagaaggtacaatatatcctttttaagagttaccatgcaaatttactaatggcgacaatagcaaatcaattatctgaatatccatgcccaacaaaaaaggataaatccactgatcacaaaggctagaaagaagatttgattggaagaacagctggaaaagcattttattagtagatatatttacaagagtggctaaacctaaagcacgatacaaacagcaggtacacttatgtacatgtcgggactatccactaatatacatttccgaacacacaaacttcacaaaatcagggaacaacctgcaagtgtcatattcacataccgtaaagagtacctttggactgagaaaggatgagaacagcagaaaaagatcctgctatctttcttcattagaagctgagatgttgaacaaaaactggggaagagatgctatccttggaaggttgtgaaacagttcagcaattgagtccttcctcgacattcctggtgccggcttgcagccagaagtgtcactgggatcaccgttgggtccgcaaaaaccctttccaaccttgttttcacatgctgacacagagctagagttggtttctcggatattcccatcaccatgtatgttgataccttcattactctgagcctgtgtgttttgcgcaactgtagaatcctgcagaaggcagcatagtgaattgacccttgacatgagggacttctcgtcagaggccgctgtaaattgagcatcacttaacaaatattgggtaatctcatccagaatttcttttgcctgcagatcatcatcagaaatcatggaagtcccagacgtcctccgttccgaaatgcaattacctatgtgattcatcagatcactcattgatatagatggatgaaatccaggaatctttatctggtcccagtggcttaacatgttaggttccttagctctgctgctgctgatttctccaattccacaggtatcagttactgcaaagacagaaagaagttcaatcaaacacagtgacaagaggagttgccatagcaattattatcagaaatatgaaaactgctgcaggggatatcaagacaaaatctcggaagagtttaaaatagacacaaatatgaattaatttactaaggcgctaaagtggaagcgaaaaacatggtacaagaccaagcagtttttcttcttcagtggcaaaaagtccagatattaatgggtgggtgccatacttagccaaatatgtcattggtaagaataccaaacatttgaatccaaacaacgatcaccagttccaagacggtaggtaatatcaatccaaatacgtaattacatgtgcacttacattctatatttttctcccaaacacacaggttcccttgatggctagtacttatcctagctgataattaaagataactattctcacagaactagcatcccaaaagattctttggaaattttcaacactaatgaagtgaattcacacccaaatacttatacagaatcttatcctcaaaaaatcactgtgcaactaattagttagagttcactgttctccccgtcttttttatttttttttgagaatatttgttctatataaagaaaggcagacatattacatcatccttaacagataatactttcaaaccaaccaaactgcagattacaataataagagtcatacaagagaaaatccttttagttgatagcaacaaaagacgatgtcccagattactgatgatagctttgtgtgggatattttgcaataaaaacatattgttttgactactagaacgacatgcagaaatgctcttgatacatcaaatactcattgtaaggcataattaatccttttaatatgcatcagtttcttcataaatctcaatttgaggttcaattttaccagagctggtcgaaggtttgaaaaaatcttgttcaaaatttgaggacgatgactgaaccccagatggtgatgctgcatgctgcaaatcaaaagaaacaggtccctcttctctctttgaatggctggaaacatctggctcatcatatatagtaactttagattcaaaatatggagattctaacaaaatttctggttcttgactaagaaagttgagacgaggatcacactgcatcagcttttcaaaatgcttgcctaacatgccttgggggcacatcagaaaatgatgcctgtgacaattgaaacagcataatcagtacaaatttaacattataatggagtgctttcattcaaattttgacgcttgcatgacccagtgacacagcaaccctgaataataatcaaaataacaaggataacaaataaaatcaagatagtgacctgacggcaatgaaatgctttgaaataattaaataaatatataatcatggcagtaattatattataaaaacacactttcccatgacacctaattaccaatttgggcatctactaaaaattcataaatattgaatattgcatccaatgccactgatcacacatatttatacagtgaaataaaacatcagttaaaaaaaaggagagatagataaaataaacatatgtcatgagaaagcacataggctaacttgaagttcatatttattacctatggatactcgcttgtccaccagaaaaatctgatgttgcct

SEQ ID NO: 98 - protein, 207 aa, Citrus sinensis
MEKTNFHPVKKQHQQRLHKVDDAPLTGFSPVSAPRIFWRSRKRSGDSANEMPINKDETPDQEMEQRQTPEPVLTERRKSLFEPLEPNNGKRKSAESLLPPPDFDSAAYPKGWLIGKKRKLVNVDVVESMRRIAVQEINRKDREIDGLNEQLEEDARCLEHLQLQLLEERSKRSEVERENGMLQEQINMLMNMLQENETMGDEGADEP

SEQ ID NO: 99 - protein, 216 aa, Citrus sinensis
MEKTNFHPVKKQHQQRLHKVDDAPLTGFSPVSAPRIFWRSRKRSASRRNFDVTGDSANEMPINKDETPDQEMEQRQTPEPVLTERRKSLFEPLEPNNGKRKSAESLLPPPDFDSAAYPKGWLIGKKRKLVNVDVVESMRRIAVQEINRKDREIDGLNEQLEEDARCLEHLQLQLLEERSKRSEVERENGMLQEQINMLMNMLQENETMGDEGADEP

SEQ ID NO: 100 - DNA, 2870 bp, Miscanthus sinensis
  source 1..2870: mol_type = genomic DNA
atggttctggacgattcaatagtgctgaaacaacggaaacaatccggtagtagaccagccgaacgcagtgaaaaaccaagccaacgacgaccaggacgacacggccaagaaacgggagtgtcttccaaggcgaccgccccctcgcgcactccaaacagcacacatccatccgtcagcccggagccacaagataacgcaaccaacaagacacagcgagcgagcgagcgagcgagagggcggggagaaaagagtagagcgcgcggcgcggcaaccaggtccaggagaaaggaagcccagctagcctggagccaagaagccgaggtgagattttgattgacatggttgctgaggcctggaagcgaggaggaattcgaggcggaagaagcagagatttagcggctgaaagctgatgggtgcaatttgttttgtgctgctgctgcagggagcgagggagcagccaggcatggaggagcccgttccggctgacccccccaggattttctggaagtcaaggagatcaggtgcctgctgtctcaattcctgttcctgcatacaaaatcttgctgatttcaagtgctttttttttttgcccccaagaatcgtcttctcgtgacttacccctccttatctatttctctgttcttgaaaaatggctaatttcagctcagttctctgcaaatttctctgtaattctgcccaaaagaaagtaatacagacatatagttcatacagcaacataattagattcacaccaacactattaatctcggctactttgtttccctccacaagcaccggtttcttttttttctcgaccagaacattttcctttttgttcatacaagttttggtactgatgcccgggaatgtgccggtgagatatttcgtgtggggatgaatgatagccagctcactggcgtgacgtaccggcaggccagtactagttaacaattaacatagcacgttaatcacgcacccgtgctacttaactgctgttgataactaaccgcccatttggtggttcacgtgagcgtagctggtcatttcaatcccttgtcagctacaggtagagcagacgtctcagtctttgcttgtcttcaccgctaagatgtaagatcccaggcctgcagctgccagtgtggtgcttagtaatagtggtctcaggaatatgcttgcagccagaaatcatattcctagacaccctttgcagcaagagtaatttctgattttgctaccgtgggattagatttctgtgtgttttctttgtctgtttctgcctttcaattatttccccctctttgccgcggtgaagacaaggccaaagactagtagtatgcgatcggtgtagcgtcctagagtttctaggtatggcagcagacaagtatgaacaattctaaccgagtagccgtctaggcatggtcaagtatggaacaaacagataaactacaatctagtcgtatatgagtattttgtagcatatgtccagacggcagtatggtcgtgtctcatgtgggtcagattatgtagcgtcgtggaatgctaatcaggtcaatctgatgctacatctagttgatactgaccaatatgtgacgctgacagattaaaataaatctgccttggaaattactctctgacagacataaaaacgatgtcttagtcttcttttcagagcttgccgcattgttcatgaatagatctttatgttgaatacagtgtgttatttcggtcccttgttactttgcttctatgtgaaggatggtacatatacatatagcatacttgcaagacactgaagggatgtaaagaattaaagaaatccacaaaaaaaatgaaagcaagggctataaaatctcactaagaactgaataaaagcatcccttggcctctccataagctgttcacatgacagccaaatgcatcctcacaactcactaacttattggttgtcaaagtgaatgaacttccaactgatcatattgtagagccaatggtcatgtgtgcattagattttaactggggaagtgcactggctcttgatctgactaacaatatgtatgttccagccaatggccggagcttgcaacaagaacctgacaaagatgctagcgaagaaactaatgagcaggctcaagaggaacccatgaagaccgacgatgcaacagatacaacagctacagctgaggatgtacaaccaaacccaaaagctaacttatctgagaagcggaaggctctctttgagcctctcgagccgatcaacggcaagcgcagtgctgaaatactgcttccaccaccggactttgagcccgcatcatatccaaagggatggctggtgggcaagaaacgcaagctcgtcaatgtagatgttgtggagagcatgaggaggattgcaatccaagaaatgaacagaaaggtttataatctttctagtggtctgattctacatacctgcatgatatcatgcggcatgcaatgctatttttctagtaaatgcatcgatgatcaaactgaaaatcctgaaatgttagcttctgcttttatctgcgataagagtatcatgcttgtgtgccgcctaaggtaaactgtaggcaattttgttgctgaatgtgcatcaaagactgacaaatgttattactgtggaaactgtgtggcaggaccgtgagatcaatggactgaacgagcagttagaggaagactcccgtgtgctggagcttctacagaagcagcttgccgatgagcgcaagaagcgggcagagattgagaaggaaaattctatgcttcatgagcaggtgaccatgctgatgaacatgctggacgaaaatgagggttttgaagaggacggagaagctccgcagcccgattcctttgattaa

SEQ ID NO: 101 - protein, 321 aa, Miscanthus sinensis
MVLDDSIVLKQRKQSGSRPAERSEKPSQRRPGRHGQETGVSSKATAPSRTPNSTHPSVSPEPQDNATNKTQRASERARGRGEKSRARGAATRSRRKEAQLAWSQEAEGAREQPGMEEPVPADPPRIFWKSRRSANGRSLQQEPDKDASEETNEQAQEEPMKTDDATDTTATAEDVQPNPKANLSEKRKALFEPLEPINGKRSAEILLPPPDFEPASYPKGWLVGKKRKLVNVDVVESMRRIAIQEMNRKDREINGLNEQLEEDSRVLELLQKQLADERKKRAEIEKENSMLHEQVTMLMNMLDENEGFEEDGEAPQPDSFD

SEQ ID NO: 102 - DNA, 4120 bp, Secale cereale
  source 1..4120: mol_type = genomic DNA
caccaacagcccgcccgcccacgccacggcacaagcacagccagaaaccacgagataacgcagcgcacgcgaccaaaccacaccgaggcagagagagcgagcgagagattgggaggagcttcggcaggcaggcagcaggaagtcgagccgaggagctgccggaggtgagctgagctcctgcccatttcgtccttgccgacgccggatttcttgtatagctgacgtatatttgcggccggccggccggccgctcttctcgtgagctgcagagcatggaggagccgtccatggccgacccgccgcggatcttctggaagtccaggaggaggccgtcgtcaggtagggggcgccgcttcttgctgcttcaaatccttcctttgagcaaacctctccaactcttgaatccatccggatttgaactgcgctcttcaaaaaataaattagatactgttcctttgcaaagaaaggaacccgtccttcacccattccccatctctcccacaaatttcagtccagatctcggcaaaaaaaaccctcgtgctctctctcccggggattaattttgaaatttgagcgattcggtttacagctcggaatctccccctgttcctcggctcttcattagccccgtctgcctctgcagaaattagtctcttcatttttgttccccggttcttcttagttagggatcgtgttcatccgtcttcgcacggcacctcacggcctgaagcattcccagcagtgagatattgcgtgaggaaatggactgacgattgccgccgataccgagtaagaaaatcgcagtttccgcccacgcgttagtcacgcggccggccggcgcaactgattcttcgatgtacatattatttataatcaactaatcaacggcctcgcgcaagcaaggtcgttcagagcttcagaccttggttagtttgggggtaatttctcacaagggacgtgggtgggtgctgtgctgctgtagtgccccgcttgcttgccttcgccggcaagatctctgcaggcagctgtcggcgctgcaggccggcagctgcagctgctagccacagtagtggtcgtggtcgtgcgaagatgcttgcgccaagaaaccatatccccttcagtaactttgctgttgttgggatgagcttttgaggtcccctcctctgaatattactaccagtattctgtcttgggcaatgcagcgagatgctctgcaggggcaggggaagcttggctgtgagggcagcagccaacaaggctgtaatttcttctgaggaaaacagggctgcaatttgatactgcattactactagatgacagggcgaatgcgataggctgagatatctatggccttaattctctgacttcgtggataatgccgattgtttattatggcgcaacccgaggctcgagagatgcgcgtgttcggtgaccactcgcgcttattttagagttcatgtcagaatgttaagtaagtaggttaatctatctaatggtaccgaccaaattaccgtttctgaacctgccaatgttgaccagttagctgccgtgtaagtaggccagtttgctcttagtgtgtaaacaacaaacagataaaagagttaaactgtttccactatcctctccagagcttctgagaatattctttctgtagatcttgcagggaattccttgcattatacagtatgcgttctatgctgtcactatctatcacagccctgcatgcatcgttctgatgcagaggtctttcctcctttaaaaaaaaattaaaaaaaatctatcacagccctttcttgcttttcttccttgtcaaggagagtgcatacagcttgttgaagtacatccaagttccaaatggaagcaaaactcactctcacctatcatcactctaccagtaaccccctggaaaaacttctagctgatcatattctagtgccaatggccatgtaaataaacaagaatcattttggtcgtgttgatattaatgcaaataggtggacggcgtgggtcccttaactatattaaacaagaatcattttggtcgtgtttccttttcaagttattaatgtcaatgtgcattcatggctgaaaccatacccccttcagtaacttgctcttgtgcaatcaccttttcagtcctttctctctgaattccactagtattctgttttgggcgaggcaacggaaaggctcttacaggaggagcagtaacagcgcggcaatttcttatgacaaaagaagagagcgactttgatagaccgagatatctatggttcacattggcttcttataatacggattgtttacagcataacgtgaggctcgagacaggcgtgatcagtcacgtttatttggagttgctgtcagaatgttactttaattaggccggtctgatgatactgaccagaaaaactatttctgaacctgccaatgttcattgttttttatatagcttcatcattcatgccgaatggtctgaacctgccaatgttgaccgtgttagtaaatcattgcctcctagtgtataactgatgaacagataaaaggataaattgtttccacttctatcctctccagggcttctgagaatagtctgttaatagatcttgccggaaattgcttgtattatatagtatgtctaagctgttgctatctaccacaactctttcttactttgcttccttgtcaacgagagtagatacagattgaagtacgtccaagttccaaatggcagcaaaactcactttgaccttatcactccactagttatccactgaaaatacttcaggctgatcatattctaattctagtgccaatggtcatgtatatcagtcagtatatatatgcactgcattttgctggggtaaatgtactgactactgactcactcaatctgacttaccaatgtgtatgttccagccaatggccggagcttgcaagcacaagaacataataacgaggccgctgccaccgaagaggcagcagcggacattcttccggctcaaggagaagccatgaagattgatgacgcaaatgcagcaagcactaccacagaggatgatgctcaccaggcagatccgatggctaacctatctgagaagcgaaaggcgctcttcgagcccctggatccgatcaatggcaagcgcagcgctgacatgctgcttccgccaccggacttcgagcctacatcgtatcccaagggatggctggtcggtaagaagcgcaagcttgtcaatgtcgacgtggtggagagcatgaggaggatagcgatcctggaaatgaacagaaaggttcatgttcttgctaattatttgccaccacatgctaccataatatcatgctgggtatatgccatgctgttttttctggtaactgcacacatgatcgaagcctgaaatcaaacatgaaacactaactttactattaacttatgatgacctgcgcattgttctagggcagctaaggtaattaggcatttttgttattgttgccaattttgcatcataagttgacacatattatcatgtaaaatatcttgtaaaatggcgtggcaggaccgtgaaatcggtgggctcaacgaacagctagaggaggactcccgcgtgctggagcttctgcagaagcagctgacggatgagcgcaggaagcggtcggagatcgagaaggagaactccatgcttcaagagcaggtgtccatgctgatgagcatgcttgacgaaaacgaagccttcgacgaggaaggagaagaggcgccaccacccgactcctccttcgattaagcatttccgacaactgcaggttcccccttttaagaaaaggcatctggagcacgtccatctctggggtaccaatttgagagtatcccagaggtttctatgcatctcttgtgtagaattcaatttatattattacgtttcatggtttgcatcgtgtaggcgaagggtgcatgttttattgttcctgttcgtatctaggtttgttgcagatgtatggagacatttgcgacgcgttttatttgaaatgcaagtgtgtgtatatggtattacgattatttcgccatccgctgcatttctttcttcatatttcgaagtcgccatgacatctgatctacaaatgtgat

SEQ ID NO: 103 - DNA, 4272 bp, Secale cereale
  source 1..4272: mol_type = genomic DNA
aaaacgaaaacgcccctgtccgtccgtctgtcagtcagtcaagcgtgaacggcgtgagcaccgtggtttacgtcccgtccaccggacgacagccagtacgtactggtaccaggaagccagcgcgtcacgtcacgggcacggctgaaagccaccgtcgaggtcgccaaggaaacgggagcggcttccaaggccaccgtttttcctttctcctagcagcaccaacagcccgcccgcccacgccacggcacaagcacagccagaaaccacgagataacgcagcgcacgcgaccaaaccacaccgaggcagagagagcgagcgagagattgggaggagctccggcaggcaggcagcaggaagtcgagccgaggagctgccggaggtgagctgagctcctgcccatttcgtccttgccgacgccggatttcttgtatagctgacgtatatttgcggccggccggccggccgctcttctcgtgagctgcagagcatggaggagccgtccatggccgacccgccgcggatcttctggaagtccaggaggaggccgtcgtcaggtagggggcgccgcttcttgctgcttcaaatccttcctttgagcaaacctctccaactcttgaatccatccggatttgaactgcgctcttcaaaaaataaattagatactgttcctttgcaaagaaaggaacccgtccttcacccattccccatctctcccacaaatttcagtccagatctcggcaaaaacaaccctcgtgctctctctcccggggattaattttgaaatttgagcgattcggtttacagctcggaatctccccctgttcctcggctcttcattagccccgtctgcctctgcagaaattagtctcttcatttttgttccccggttcttcttagttagggatcgtgttcatccgtcttcgcacggcacctcacggcctgaagcattcccagcagtgagatattgcgtgaggaaatggactgacgattgccgccgataccgagtaagaaaatcgcagtttccgcccacgcgttagtcacgcggccggccggcgcaactgattcttcgatgtacatattatttataatcaactaatcaacggccttgcggtcgttcagacttcagaccttggttagtttggggggtaatttctccagtgtgggtgggtgctgtgctgctgtagtgccccgcttgcttgccttggccggcaagatctctgcaggcagctgtcggcgtagtttgccggcagctgcaggtgctacccagtagtggtcgtggttgtgcgaagatgcttgcgccaagaaaccatatcccattcagtaacttgctgttgttgggatgagcttttgaggccccctcctctgaatattactactagtattctgtcttggacaatgcagcgagatgctcctcaggagcaggggaagcttggctgtgagggtcgcagccaacaaggctgtaatttcttctgaggaaaacagggctgcaatttgatactgcattactactagatgacagagggtgaatgcgataggctgagatatctatggccttaattctctgacttcgtggataatgccgattgtttattatggcgcaacccgaggctcgagagatgcgcgtgttcggtgaccactcgcgcttattttagagttcatgtcagaatgttacagtaagtaggttaatctatctaatggtaccgaccaaattaccgtttctgaacctgctaatgttgaccagttagctgccgtgtaagtaggccagtttgctcttagtgtgtaaacaacaaacagataaaagagttaaactgtttccactatcctctccagagcttctgagaatattctttcagtagatctttcagggaattccttatattatacagtatgtgttctaagctgtcgctatctatcacagccctgcatgcatcgttctgatgcagaggtctttcctcctttaaaaaaaaaacaaaaaaaatctatcacagccctttcttgctttgcttccttgtcaaggagagtgcatactgcttgttgaagtacaaatccatgttccaaatggcagcaaaactcactctcacctatcatcactccaccagtaattcactgaaaaaacctctagctgatcatattctagtgccaatggtcatgtaaataaacaggaatcattttggtctgttgatattaatgcaaataggtggatggcgcgggtccctttactatattaaacaagaatcatttttggtcgtgtttccttttcaagttattaatgtcaacgtgcattcatggctgaaaccatacccccttcagtaacttgctcttgtgcaatcaccttttcagtcctttctctctgaattccactagtattctgttttgggcgaggcagcggaaaggctcttacaggaggagcagtaacagcgcggcaatttcttatgacaaaagaagagagcgactttgatagaccgagatatctatggttcacattggcttcttataatacggattgtttacagcataacgtgaggctcgagacaggcgtgatcagtcacgtttattcggagttgctgtcggaatgttactttaattgagaggccggtctgatgatactgaccagatatagtatttctgaacctgccaatgctcattgtttttttatatagcttcaccattcatgccgaatggtctgaacctgccaatgttgaccgtgttagtaaatcattgcctcctagtgtataactgatgaacagataaaaggataaattgtttccacttctatcctctccagggcttctgagaatagtctgttaatagatcttgccggaaattgcttgtattatatagtatgtctaagctgttgctatctaccacaactctttcttactttgcttccttgtcaacgagagtagatacagatttaagtacatccaggttccaaatggcagcaaaattcactctgacctatcactccaccaattatccactgaaaatacttcaggctgatcatattctaattctagtgccaatggtcatgtatatcagtcagtatatatatgcactgcattttgctggggtaaatgtactgactactgactcactcaatctgacttaacgatctgtatgttccagccaatggccggagcttgcaagcacaagaacataataacgaggccgctgccaccgaagaggcagcagcggacattcttccggctcaaggagaagccatgaagattgatgacgcaaatgcagcaagcactaccacagaggatgatgctcatcaggcagatccgatggctaacctatctgagaagcgaaaggcgctcttcgagcccctggagccgatcaatggcaagcgcagcgctgacatgctgcttccgccaccggacttcgagcctacatcgtatcccaagggatggctggtcggtaagaagcgcaagctcgtcaatgtcgatgtggtggagagcatgaggaggatagcgatcctggaaatgaacagaaaggttcatgttcttgctaattatttgccaccacatgctagcataatatcatgctgggtatatgccatactgttttcctctggtaactgcatacatgatcgaggcctgaaatcaagcatgaaacactaactttaccattaacttatgatgacctgtgcattgttctagtgcagctaaggtaattaggcatttttgttattgttgccaattttgcatcataagttgacacatattatcatgtaaaatatcttgtaaaatggcgtggcaggaccgtgaaatcggcgggctgaatgaacagctagaggaggactcccgcgtgctggagcttctgcagaagcagctcacggacgagcgcaggaagcggtcggagatcgagaaggagaactccatgctccaagagcaggtgtccatgctgatgagcatgcttgacgaaaacgaagccttcgacgaggaaggagaagaggtgccgccgccggactcctcctttgattaagcatttccgacaactgcaggttcccccttttaagaaaaggcatctggagcacgtccatctttggggtaccaatttgagagtagccccgaggtttctatgcatctcttgtgtagaattcaatttatattatttcgtttcatggtttgcatcgtgtaggcgaagggtgcatgttttattgttcctgttcgtatctaggtttgttgcagatgtatggagacatttgcgacgtgttttatttgaaatgcaagtgtgtgtatatggtattacgattatttcgccatccg

SEQ ID NO: 104 - protein, 220 aa, Secale cereale
MEEPSMADPPRIFWKSRRRPSSANGRSLQAQEHNNEAAATEEAAADILPAQGEAMKIDDANAASTTTEDDAHQADPMANLSEKRKALFEPLDPINGKRSADMLLPPPDFEPTSYPKGWLVGKKRKLVNVDVVESMRRIAILEMNRKDREIGGLNEQLEEDSRVLELLQKQLTDERRKRSEIEKENSMLQEQVSMLMSMLDENEAFDEEGEEAPPPDSSFD

SEQ ID NO: 105 - protein, 220 aa, Secale cereale
MEEPSMADPPRIFWKSRRRPSSANGRSLQAQEHNNEAAATEEAAADILPAQGEAMKIDDANAASTTTEDDAHQADPMANLSEKRKALFEPLEPINGKRSADMLLPPPDFEPTSYPKGWLVGKKRKLVNVDVVESMRRIAILEMNRKDREIGGLNEQLEEDSRVLELLQKQLTDERRKRSEIEKENSMLQEQVSMLMSMLDENEAFDEEGEEVPPPDSSFD

SEQ ID NO: 106 - DNA, 6957 bp, Beta vulgaris
  source 1..6957: mol_type = genomic DNA
atttgtgccacttccttaatctcaaccgtccatttctcagacaattctctgcaacaaacaaaaccccatatttcttatttttacgttttccaattcaactcccaacatattccaagaaaatggagtcagaaactcagcacttattaagataagagagagagagagaaaaataaaaactgcaacttctcaatttttaagaaacgaaacattcaaaatcaataaactttagcataaagcaataacaccccattttctgattttctatatctagctgaaactacaaaaaaaaaaaaacagtaagaagtataataaaaatgggagaagcagctaataattctgggagtggaagttcttttgatgggttttctcctgtttctgatactcgtgttttctggcaatctcgtaaaaagcgtggtaatttctctctctatctttgcttacgataatcaaaattagctcatctaattatatgttgtaggatttattagtttactactcttgaacgcatgtcaatgcaaagtttgagacatatgttttaaaattttatatttgtaaaaaatataaaaagtaaatattaataaaatacatattatgatgaatttaacaagatcgtacataagaaaccctccgcttgtgtgggaaacaaactatatatattcaaccaatacgacttactctatattagagtgtataatgaaaactgttttctttttactggaaaattacgactgtatatttagcttttacgactatatattagaaatattttgtttaaagatggttgtttgtttgatataattttatcatcttagagattaacaggcatgtatttagaaacgaaggaagtatatttgatggagtgttgatttgttgcttaatatgtgagaaatccctgtttatttttccaactaacaatagctttctctctctaaccactacgtaacgtcagagaaaatctttgggtaatttttgcaaggactttttttgcttccttttttcatacttctaccattttacgtcatagaggtagggttagatttatttttaaataaaatgaaatctttgaatattacatgtttactttatgaaaatgatttaaacaggtttttttttttttttttttgatttctgttaaattgaagtaatagacagatcattcgagttggtataacagtaagaaagtgaattccagctaatccgcttctagaagtttttggttgaagttaaatttcatatttcaaatgttggataattttagccatgcaagtaagcaataatgttgttaagttgctattgaggcattctttgaatttgatgaagtgatttattgatgaggattttatgtaacaataggaattgattatggcattatcctaaagacttgaaaacctttttgatgccaactaaaacaactagttttgttggtaaagtcttgtaggggtagtacctaggggctaggatacgggatcaaacccttctatatcggttcgtttaatactcgctaacacaaaaaaaggacttgattaactcggtccgtactaacccccccccccccaccccccccccccacccacccaaaaaaaatcgtcgtcttgctgaatactgcaaaatggtattatgaccaaattaatctttacaaatatgccttcaatgcacaatttccttacatattacatttcacatgtcttttcatcaaaatttccaatactaccacaaatatgttaattctatccatttcatgttgtgttttgctatggattggtatgtttaaggagcagataatgagataatagtgtatatatgaagtgaaataaattgggaaggagagaagttaattaagttcaaataatatgatttggtgggattacttatgttgaaatttgaaagttctattacttttgaagaggaaaatcaacttttcacttttgttgaattttcagtggccatgccacaaatctccaaagtttgtccttagtcgataggactacaatctagtgataatatggtgtatttatttttggtgcatcaggagaagaggctaccttgtaacaaaataggtttaagaagtatacagtataattaactatttaggggagggatattgtggtataaaaccaaatttttctgaattggaatctgtcccttgtattatactagtaagtgattgacaacttaccaaatggtagtggactgcaagcaactgttgtcaagtctatagagcttaatctttacacttgatgggtccttgatggctgtttggcatctttgcgagcttcttgtctcaacaagttttgtagtatttcttccaatgtttattggttgcaacatagggggatgcacgatattctagcagcccatgtgataggagagagatagagaatggagagatggaaaatgtgcccatgtgattaagagtgagaaatagagaacacaaatacttagataagtttgttgcaaccatttagaaaatatctaaaatacagaagtattgctgctaaataaacctactgaagtttaacgcaagtattactaaatggttttctagaggctctatttatttttaagattttgattctgtttttagaagatattttctgttagtaaggatttcatttcggttaggaggtctcatgtgcgaggggaggggaactatgttacccatcacctcgctagatgcattctctttggtactgactactgagcaacgttgggaatatcattgtccttcggatgtctcaccctacttatggactctatgcccatctcttgattaatgcatattttatgaccccttcaaaataaaaaaaggtttctgaagaaactcatgccattttgtttatcagcccacattgcccatctacaagagattggtagcaattaatcatttatcagtgtttctcggctatatggtggtctctttgcagaaagttttgcaagtttgtttcttgcctagatggttgatgtggcctttcctttccagatcaataattccattgttttttttttacttgccatcgttatttaataagttttacttgtatcgacaccctttgatttgaaaaatgaaaatacagatatttccacttggttttgtatgcatcgccaacaggcctgatcaatacgcataagagggtatgcagtatggtgtaagtctcctcagttcaggagttgtgtatattcccattagggtattgaccctctatatctatagggcaaaaatagcagccatataatcctataaagaaaaaagggctcagaccgctagtgacccacgacgcactaggccaaccttcttgcagccctttaacaaggctgaacagttatggcctgctatcaacccgcactagagtgagctgcccgcaagccaatagctaagcttatttgccaaatgtgagaccatgcattttgttttgctctttgtgataagtaaatcaagagcgtcaaaacttagagcttcttctcaaactgcttattttgtgcgtgggttaattattgattggacaattcttattaaagaagcctttccattccttttttatagtcgagtaactatgttccttgcttgaagcggctggcattcccctatgcagacaccagcaagttaattgtttattgcacccctttttgttgaaattggcattattacacaacgagcttggaagaaagagaagaataagtcataggaactattgttgattggttattaggagtttgacttgttctgcccaagtaaactgtgttacacatatgtggttcaaatttctcaaggttcacccttgttttttggttttaaactatctccttatgctatatggacttacccctcctcccctaaaatatctagtagggtttatatcttttcttcttcaaacgaaaatctgtaacttttttcgtatcatttcacttcttctttcttttgggctatggctgggggaggttaggacaagattgtcattacaaagtcgtgagcctttttcatcaaatctagaaaccatattctcaatcatgattcggaacgatttgcaatgaaaccatgtcccgactattaacgaccccctggaaattttttctcttagttcgagggagaaacatcaatgctagttttaactcacatatttcttggatctcagtcctaattctttggctcttgtctcatttacaaacttttgaccattaatttactaaaaacttagtttcaagattgtttctattactcatttctcaattgttttctcccataatcatgaaagatactattccaaagtcccatgcaaatcttcctactttttgatgttccatctaatgttctctaatatcgattcttgcagaacttctcttccattttgcttagaattcccctagtcttcacattttggcgcaacttcgtatttacttaactatgctaggttattttaatagtatcaagttttccataacattatttatcatccttttcaatctatgtttagtcataagtaatatttatctgggttgaaataacagttgaagtcaattacaagaatcaggttatgagaagagggagtttcttacctatgaactagcatagttgtttctccctcagacaaagagcattgtgaactgccaatgacttttgacttacagacttccaaacagttggctcttaaaaccaaagtgaggactgacaacattcttagtgggtcaaattgaagttaccaaaagcacttgtgtatctagcatatatggcttcatgtttgctgaaaattgctccttgaactcggagttaatcaagtagaaaagttgtagatgccgctctttcacttgctgctgctctcgtctcccgtctaggctctttccggcgcttttggggacggggccattttctaagagtaaaaaggcattcgaatagcgaaggagagaccagaagattgtatgtaggcactgcacttaaaatggattgatggctgtgtagtcctcattcagctggaaataggaaatcagtcccggcacgatcgatgcttagtctccttctacgcttcaaaaaaccacctacctaacctcttagaagagatgcaatagatagcggcaaccgctccgtggggtttggtaccgtcaccactacttttccatatcctttattcctttctagtttctcttttatagttttcctacggtttggccttctttccattctccttatatcctttttgataaagctcttgagtgtcgcaatactttaactactagaatgaatgtagcaaaaatgtgcttccagctgtctcacatttgtttggatccatgtgctgctagttatacgaaatcaaacttatataaaatgtttgctaggataaggtaatatttagagaagaaggtaaatcaagtgttccaattgggtcaactggaaattctgatgaataatgatgatgtttaaaccactcgcagcatgttaagggaggggtaatggaaatgtttactaggttcacattgctcttgaaaaatgcttgttgctttaagtgtactcaagctccaaaatgaattttatatgttttgtatgattaagattgatgcatgcttagtataataattggtaccatggtattagtttctgctataatttgttccacaagactagcttcttgtgacagctagctcactgaatgaggccaagccaagagatgagccaatgtttgaaacgcctccaaaacagggaaatccaacagaagagaataaactggactcaactcctccagatactgttctttcagagaaaaggaaggctctctttgaaccactagaacccattgataatatctcaagaaaacgaccctcaaacgagagcttacttcctcctccagactttgactcaacaatatatccaaagggctggttgataggtaaaaagaggaagctagtaaatgtcgatgttgttgagagcatgcggaggattgccatccaggaaatgaatcgcaaggtacctttctaaagtccccgcaaacccattcaccccttcccccccccccccccccaaacggtcctaaattactgatatgagaaaactctacaagagttgaatgtacaatacagtagaatgtagattgcttacacagttacatgtgaacgaagcaagacttaactcacttggtaagactcttacctcatacggagtcgtatgactcgtatcctagaggttaggggttcaagtcgtgccatgtgaagatgcttggggctgggaatagcaccttgccccccctactccaagtgcttgtcctgtaaatactggaccaagaaattgttgctccgtgagaattaaggtctggtgagggtcttccttactgtttagatgaaataatcttaattatgcatgagagaactcgtgctagaagagcatggtgcggtacaataagataaaggaatccattccccaacaaaatatatagataactttgataacctaactttcgtaagaaactatatttctcagagttgttgataggatagctatatgtgcaggatcgtgaaattgatggattaagtgaacaactggacgaggattcacgggttctagagcacctacaaattcagcttctagaagagaaaaggaagcgtactgatgttgagagagaaaatacaatgcttcaggatcaaattaacatgttgatgaacatgctgcaggaaaatgaagctgcaggcgaggagggtgcagatgagccttagttagtaggtctcaactcttgagcaagattataattcttttgtataggtttttcttgggttacagtagaaggtaagtggtgttaagttagttgctgcatggaatttactgttgtttgtttggttgctgcaattcgttttacaataaacaattgtactcttttagtatgtacaatgtatttgcagtaaatatctgcttccagaagacaatatactgttaatgtatggtctgcaagtgcaaataaacagctggtgtaaataattctt

SEQ ID NO: 107 - protein, 209 aa, Beta vulgaris
MGEAANNSGSGSSFDGFSPVSDTRVFWQSRKKRASSLNEAKPRDEPMFETPPKQGNPTEENKLDSTPPDTVLSEKRKALFEPLEPIDNISRKRPSNESLLPPPDFDSTIYPKGWLIGKKRKLVNVDVVESMRRIAIQEMNRKDREIDGLSEQLDEDSRVLEHLQIQLLEEKRKRTDVERENTMLQDQINMLMNMLQENEAAGEEGADEP

SEQ ID NO: 108 - DNA, 13189 bp, Sorghum bicolor
  source 1..13189: mol_type = genomic DNA
tttttttcccatttctacatttctgtcgaacaggaccctaccgcgccggaatcgcactgcttgtgccttttcctcctccacaatccgtcacgctctgcgcgccgccgtcgacctatcgaatggaggcggagcagcaaaagcagccccagcgcccgcgccgcaaggggcagaagcggaagttggaggacgaggcatccgccgccgccgccgccgccgccgccgccgcggtagccgccgccgcgtcctcgctcggcagcgcgggcgccgacgatgacaacgaggaggaggacggctcggcgggcacccccgagatctgctgccgccactcccacgcggcgctggcccgcgaggtccgcgtgcaggttgatgtcctcgtccgctgcgcctcttcgtggcgccacgccgaccgcgccgccgccaagcgcgccacccacgtcctcgctgagctcgccaaaaacggtaaccacccttcgccaaacctcactccggccgcgccgatccgtgcaaccgcatccttaccgagtggatctggtggttgtcaattgagcagaggaggttgtcaacgtgattgtagagggcggcgccgtggcggccttggtgtgccacctagaagagcctgctgtggcggcgccaacgcaggaggaacaacaactgcggccgtttgagcacgaggttgagaagggcgctgccttcgctctgggcctcctagctgtaaaggttttttcattaattccctaattgagttttagatgcacttttggtaccaatgcaattacttgtatcatcgacaaatttatgttctaaataggactgtgaattttcaagtttcctgtggcataggattacaaagtttaagaacttcaactatcccacatgttgtatacaataattcagaatgcctaaacctgtatcctcgtatatctgtatttcttgtaaaatactgtaagatccaatgcctttgaatagttagaattagaaaaacctaggaacttccaagtcctatatacttggtgcctttctagtcagtctctagtacccttcagaaaaatttaggaacctaagatatcctataatcgttctagttctgtaggaatcttttaatagttgtgctttgagcaattgatgatttactcttatgtacttttcatcaaattactattgctatggtcaataatcatttattctgtgttcactgtaacagcctgaacatcaacaacttatagttgatgctggtgcactacctcctctagtgaaactcttgaaaaggcagaaaaatactacaaattcgagggtggttaatagcgttatcaagagagcagctgatgcaattacaaatcttgcacatgagaatagcaacatcaaaactagcgtcaggtattgttttatgcctctttggtcatttgataacgttttccttcagaagttttcacttgctgagggttttgttttactgcagaatggaaggtggaatcccgccacttgttgaattgttagaatcgcaggatcttaaggtgcagagggcagctgcaggtgccttgcggactttagcctttaaaaatgatgaaaataaaactcaggtgagatatcaaaatcaatgaaggctataattgtgtttgattttgacatctgaacttgcatatgccttttacacatactcacgacatggtgaattcctgtaatgcagattgttcaatgcaatgctttgccaactttgatcttaatgctgcgatctgaagatgctgcaattcactatgaagcagtaagtccttgtgctattctccagttttgatatgaggcactgaatactctgatgtcaactccacttctctaagtgcactttctcacactgttgagatgtattgtttgattgattatgagcaggttaatgttgttacagataaatgatcatatcatttgaaattgtgccattctacaattttgcacaatccttaatcagcatttatcattgccgggccttgtgaaatataaaattttaatgctccattttgaaacttaatgctggatcataacactgtacatttagttggggaatttcatgctagaccgtgcttcatcctcgattacatggacaattttgaatgtatttccaaagttgaataaaaacttagttttgttggctgttagcagttactccctccgttccaaattgtaaggtgttttggcatttctagatacatagattttgctacgtatctatgtctaaatacatagtaaaatcaatgcatctagaaaaaccaaaatgtcttataatttggaacggagggagtaccttacagatattatgttgtcctacaacacatttatatcataggctttgcataatttattcaatatttcctgccatgtaagatactaagatgcagtttgattaatattttctgatcccgttgatgaattatgttaatttgctttcatgattaccctgaatttgtgcactgatattgatctattacatatagccaaccttagcgaaactactagcagtgcatttggcaactattggaaaggggcatgggaattggtggtgggagttgttggagcgaattatgagaatttgattttaaggcctaatcacttgtttggttcatttctaaactcttaccccccaaactctcattcccttgtaccaattacccccaaccaaacgtgctgtagaggttattgaattggcgaaggtaaacatcttgaatgcaatcaacacactttctgtttttttgtcaactggtgatagaccttaatggctgtattaagttagttcaggtgatctttgaggctgaaattgaagatttgaaaacttgcaatacacccaaataagtttgagggccagtggtgcagccatgcaggttaagctgtatcatggtgcatgtacatggatgcttgatgtattaaatgtttatttgaatgcctaaatgtgtggcaagtactgagacaacactagaaggctgaggctatttactactttgttcctgaaatatttcaaaaagtaatctgcacctgctacttgtaacatgtttgctaagtaaacttgattgtagaagcttatgcaaaacaaataaattgcatgaaactggtccgaggctctgagttacctccttatattgacttgctgttctatgctcttttatccgttgaataaacttctacatggtgcagggttacctttctgtactaacttccttatcaatccaacatgtttgctgatcaactttcatagaatatcagcacaatcttggatctaatctattcatgatttctttaactttattgcaatgcactctaatgactttcctcgactgacatgttaggttggtgtcattggaaatttggttcattcatcaccaaacatcaagaaggaggttcttaatgcaggggcactacaacctgtgattggattattaaggtatggtcatcatagggaagtgcagctttgtgaggtgcataaagaactttgtaattgtatatatttgttaggttctgctccaatactgatagcatagttgtgcatgtttttattgaattattatcactagcaaatatgcccgtgtgttgcaatgggaaaaagactttttgtataaaagaggagaaaatagtaaggttcttagcagaaatgcccgcgtgttgctattggaaaatactaattctttacatgagaaagggggaccaaaatagatgcatatctccaagtagaatacttattgcaaaggtactccttccattccaaaggaatgaatgtagacatgaaggctgcaacatggtgctctaagaactcaagctggtatgggcccaacctagtgttctaaataaggaataaaacattaagttttttgtatcctaaaacatcacgtgttctgaaacggagggagtaagatggaaaaaaggtaaataaatgtctcaaaaagttggtctgcttcaaggagatcagataagatcagagctaaattctcatccatgatgctgtgggtaagtttttagtgcaagttgagtgaatggcttggtaacaatcaacactgcgagtttctctacatatgcattacagagtagagtctgatattgataaagagctagctccttcgattttcatctgttagtagagccatcaagaatttccatgcacctacactggacctacttctaaaatctaggaaacatgccccttctaaaatatagttgcttgtgtgttgattcgactcaattagcatcgatatggtggctggttgattgagcaacacacatattcattgaggccaataaacacacatttattgaggccagtgttcaataattgaattagatgtgaatccgaagaaacacagatcgaaaaggagaagaattgcagacctcgccatcaggttccatgggagtggggttggctgtgctgcctacgactagatctcaacaccactcgttgatcgtggaggaagccaaacctctagagtcatggactccatggcccatgggcctccactgcgacatgacagatgcctggatccggtatcccaggttggagggggaggacggagcttccaatactgcgctatcgcaaggaaggcgaggggcatgctaagaagctctacgcttggccacagagccggtgccgtcttctcacaggtgttctccagatctcccaccggtggtcatgcttcatgactgtcgtggggctaacgaacgtgttgaaggaggtgtagcaggcaggcggattcgtgagccaagggcgtggtcttggacagttggacgaaattcatgatgcagcattggacgagatgggggaacatacgttcatgcgtagggagcgctggtggggcgatgaacgtatgaatgggcttggttgacggacaaaatcctgaggagagaaacttttgctctttaatactcccaattgtccaaaaagaatgtaattctctcttccctaggagtcatacaataaaaagtttgaccaaatatattatactaaaaaaatactaacatttatgatacaaaatatgtatcattagattaaaatatatttttatagtaaacctaaatggaaacataaatgttgatactattttctttgaacttagttaaacttaagaaagtttgacctgtttcaaatctggaatatacattctttttgggacggatggagtattaggtatagatatatactgcatcttctgttgagcatgccttacaaatgttctattagagcatctccaacagattacttatcctgcatcccctaaaagtctatataagtgatctgttattcgtagtgtagctttttcttctcctcccaacagattaccaatacctttaaagtggataggggagagggaatggatagggattttaagtagttacttaaaacttttaggtattggagataggatgagtaatctgttggagcaaccacaataccttgtattgcatatttttagtatcagggatgagataagtaatctgttggagatgctctaattttgaggacaccagtgtacatgaagatttaatgattaagccaaccaaaacaatgctgattattatatttgagcgtgggctaggccattcctagttctattcagatccttgtcattaccatggctttgtcttaaagagcgggggagtagattgaaccccgattgtccagaaaactcgctgaaaccagttcagtgaggtatccacatttggcgagggactggaattttgggtgggtggccttcttgttgggaaactgtaccaaccaagcgactggctcctttctcatctcgtattctagaataccatcttattcaaatttgtcattgttattcaagttttaaagggtgttctatgatttgctctacaccagcagctcacctcaagaatatctgcttgatgtatgaaacattgtttttttttcagctcatgttgtacagaaagccaaagagaggctgctttgttgctagggcaatttgcttcggccgactcagattgcaaggtgcttaataaatgtggaatacttattgtttacatgtcttcagtaaattttgcgaatctgctggtagattagtcaaaagtaaagaaagaatcgcacctgaatttgcatggttgtctcttccacacccctcagtttgtaacttacattgtgagcccttctaactttggacccattgtggcatcagcccaaatcaccgttagctacttagtttaattgatggtgctggtgtggcatcaaacatgggctattatactggactttttattttcatcgtcgcttcccttttcttttacattgatcaataaatcactgacatggatatgtagatgatgccatcaaattgactaatgatttgaccagtcaacaaaatatttgtttttgcatgagtcattatttatggtgtactcaactggtagccgtgtcttcttgtgaacagtcccttattgcagttaggcattatttatgaatgtgacactgtgactttcaataccttgtatatttggcaaatattagactatcaacccccccccccccccccccccccccccttttttttttcaagaagtatttattttgtattacttactgttccataatttgatggaatttagccatccatgttatttagttgtgattggaatgtatattgcacatgttttaaggttataggccaaaacctgtgtcaacatgccatggagagcaggtcccatgtttaatgctcatgtcaacacaatttgtatgttaaggtgatttgggccaatgttgcaaacagacctgaagtttagggggctagcaaagtaatttgcaagttgagggaagttggtgagagtgaggcaacaacacaactttaagggctagtggtgcaattctctcttttttcagaagtactggtgatttacatatgtaacatttaatttatgtgtactgtatgttgggatagaagtgaaataagtagtaaaacccatttctggccaagcacatcaggtgtgacagattctcattgctgggactgtctggcgccttttgagatgatgcctcatagggcctacatcctgctggccagtccatgcatgacctcgcttattctccttgttgctcttttccaactatgcctctgcatctcttattgttggtctgatctgggtgccacacaatcatgaatccagattggtgtgccatatggcagcctctgcaactgccctattcggctggcacacttatcttcttttgtctagttagtccatcctcaccctggtgtctgcacgtgccaagtcccagctctgcccttacctgcactgcgtcttcatcactgttcttggcaacaacacaccctggattctatgctcaagctgaacctagctcggctaccacatgcatttcaattgctccaccactcctggcttacaccacaccctaagccctcccacaccaataaatcattggataagatttaagttttttcagaagttagtttctttgttgcagaggtaggttttgctttattttttttagatgtttccttgggagatgggagaggacagccattgggaccacttgttgtctgtcctttgagtggatggatgcagaaggtagaaaaagaatgaacttaacaattgaatataatgttcagtataaggaaatctagaatgataaatctcataatctaaggaatgacacaaaagcaaaaagatataagatgttttctccagttaattcgtttctgaacttgatagattaatatatatttttgtttacaggtccatattgtgcaaagaggtgcagtccgtccactaattgaaatgctacagtcagctgatgtccaactccgggagatgtctgcttttgcacttggcaggcttgcccaggtttaatttttatttttaatctaacatatttttttaatgtttaaaggtactttactgttttctactctagagaatcagtgtaggcagtgaaataaaaaaccacagaaattttcttgctctcttacaaaatccacacaatgtataactttatcaaattagttcccttgctcctctgttgatgggaactatatgtggggactggggatgcaaagaccataatatgtttagggcaaaaccatagtgagtttgctggcaccacatggacagatttccagatatgctggcttatccagtccatcctagacatggacagatttccagatatgctggcttcatgtaatcatcatgttactggtgtctgcatgtgccaagtcccttgctttgcactgcatcttcaccacttattgtcaacaacacaccctgggtgctgctgtgttcaaggtactctggtaccacaagcatttcaattgctctgccaagtaattgaagttacacagctattctccatacgtcggagctcctagcccactgtactgtagcttccctgccatggtcgagctcgcttgcactgccattctcgttggtataggacatcactgcttcaatgagtgtgcggttgagcgcgctgaggtcccattgtcctagtgcgcaggcaatcagggcaagtctatgccggacccaccatttttgctgcagtcttctacctgccgtcaaccaccggattggcacgctcatggctgacccgctactggccgccatcggacaaattaaaaccattctcgggtggtgctggtagctcgtggtcccatccattgccgctgctgagtgctcccttggctgaatctgcccctccacaccatacttgtgcctatgttgatttggggaagaaagaagaggaaggagatgattcatgggacacatgagccttcgcgtctctgccatgcacccctgcgtccttatgtcgtgtcaccaggccttcgtcgagggccactgtcccctacgctcatgccgcttgccggcacatgcgctcactgccgcacactgccgctcagggaatggggcaaggagaatggagggaggaggggctaattgcaaatttcgtaccatgctgactgctgactccacatgccacatcagatctaagggccaaacgaaggggtatggacctactgtgaaccacataaagtttatggacccagaaatcaacttttagagttgatgggcctaacaaaaacccccacataagttaatggagtgcatttaattcttttttttttgtaagggaattatgtcttttagtttttgctccaccatatgctctgaccactaaccatgcctatcttagcagaacttttgagcatttgtaagtcctaaatgctaggtgacaacgtcctagcttagttatcctccctagtccaatgatgggtgcttggagcgttccctgtgactttggccccagctaatcgtcgattatgtgctaggagctggtctgctgtctgactattaaagacccactctgtcagtggtacattctagcagagtgataatatttgtgacgattgcaaccaaccaaacatcgtagcatatatttttcttgtgagattgtttggctagttttatacagagtgcaatgcagagtgaaccatttaaaaagttgacccagatactcacttgagagattatggacccagttgagtatctgggaaaagtttaacgatccaacgcattttcgctctttcatatcatataatgtaaggggaaatccccattcatctttaccttttacttatggttagtggggttgtttctttttctatctttctttcttttttgtttagttgcaactcgtaatctaatctaaggagtcttttatcaggacacacataaccaagcaggtattgcatataatggtggtttggcgcctttgttaaaacttcttgactcaaaaaatggatcgctgcaacataatgctgcatttgccctttatggagttgcagataatgaggtaatttacgattttttttttcacaaagtttgccatctctctcaaatctcccttttccacttttggttaataattccacactacatgttcctttgtaatgggattaactcatttttttatataaaatgtttatcttatatttcttatcttcattattttagaagcaaatcactgttctttcttataggactatgtatctgacttcattaaagttggaggtgtccaaaagttgcaagatggagaatttattgtccaggtacattggccttcattatatattggtcactttgttgtgaatgctttttattaagctattcttaatttcaggcaacaaaggactgtgtggcaaaaacattgaagaggttagaggagaagataaatggacgagtaagttctgcttgcaaggtttctgtatttcgttgtttgtgatgtgcttgactttagtatttatgaagcttgttcccatgtgatggtttacaggtgttgaaacacttgctttatttgatgcgagtaggagagaaatctgtgcaaaggcgtgttgctctggctcttgcacacctttgtgcccctgaagatcaaagaacaatttttattgataataatggtaaacaattttccaaccgctgaaaattgtaccttttcatttccattctactgtatggtgttcttcatgaatttaaattgtgggtcatccaggtctcgacttgcttcttgatcttctgatttccatgagctcaaaacatcaacaagatggctcagcagcattatacaaattggccaacaaagcagcagcactttctcccatggatgctgctcctccatccccaacacctcaggtatgcaaaagaattattaaatttaaatttactttgtattacgtatgctgtttgagttgcagtgactttatgagctgactgtaatatggttaaaaatagtatcacaatggcatgatcttcagtgtgctaggatgcacatgaatttattttgattaatcatcgtggaatggtgctttggttgaacaaggtatataagggcccaaacgagtccctcgtagtccaacctgttgtgaatgacagtgtgtacaacctgctggaggaaaataaatgttcctctggcataggttgttcattgcacttaacttgcagcagctggtgcctagcattactaaacatagtttcactacttggtggcagagagttagcaaaagagttagcaaagatcaaagaaaaggggttagcactctcatcatcttgggtccctggatgccctggaagcaggggaatgcgtgtgtgtttgagggagactctccagtgtccctactacacctagaaacctgaagttagaagctcatctctggacgcttgctggggcttccaagctacaggatcttgggctaagtcagttggaaacctgaagttagaagctcatctttgttgtaacccccttaccttggtcctagtaagaggggcttgtatggaccatttcttttccctatagtacaaagatatgcagctctcctgcatgtgcgataaaaaaatatcatgttgatagttttatactgcttggcattgtgttgaaaattatgaaagaatttagctatcatcggcatttttaacaagatttccaaacactgcctgtattttgctatcctaaataaagtcattgttgcattgtgggatttttccatcctattgtgctggtaatggctgaggcactggcaattgttactgaatttatatttcattgcaggtttatcttggtgagcaatacgtgaatagttcaacactttcagacgttactttcttggtagaaggttggtactatttcatgaccgtgatttcatcagtaggtactttaaataattattttctatcgtgtcccagataatcttaatcccttcttctacaggaaagcgcttttatgcacacagaattgctttgcttgcttcttcagatgcatttcgtgcaatgtttgatggcgggtacagggtgagttttgacttgccacaacataatgtacttttgctggttttagtctgttgatctctttccgtagttgatatattgctgctatatatagtatgttagttttgaacaaaccttgaatctcatgtctaattcaaaggtcattttcttaaccaggaaaaggatgcaagagacattgaaattccaaatatcaaatgggaggtctttgaactcatgatgaggttagtaagtcgttgacctcccttctcgtttggccacggttctgtttctgttgatgaatctgcaactatttttcctcttttatttttttatgccactgtatgctggattaaagtctgaaatcctctttggttttgcagatttatctatacagggtcagtgcaggttaccagtgaaattgcacaggatcttcttagagctgcggatcagtatctcttagaaggcctcaaacgcctatgtgaatatactattgcgaaggtgactagaaaacctactctctattccttgtttaaaccgcatattatatatattaatttgaatgccattatttgccttgtaggatgtgaatcttgataacgtatctgacatgtatgacttgtccgaagcctttcatgccgtgtcactgagacatacatgcatcttgtacattctggaacattttaacaagatctgcaccagagccgggtacattctcttgctaataacctttgatctgagaccagtacgatttcaagtaactcaaatattaacacgcaatcttggcatgcagttctccacagctgatccagcgtgtcattccagagctccgcaatttcctaaccaaggcactgagttcatcaagaagtccaagcccaagcgacaggaactcgcagatttgatttaagtcccaattcattgacaccgacgccgtcatctgaccaaagtttgctggagatcctgtacagtaacgtttctggctctgagcgttcgatggtatctattgtgtgtacatggtggccgggtccttcaaattaacatcagcagtgtaacaaacttttctaagatttagtagaggatatgggtaaagagaacctgtgtcttagtcatgcatcgagccatcgaccagcttacactgggataggctgtagttggatgttcctaattcgtcggtcccagctttgtttctgagtttagtgtttctttccagttcacagttcagtgtatgcccccatctgtttaatgtatgaagcttgagcaagttagaaattgacccccgtagtgataaagctgtccgttaatctcctagtgtggaaccaccgtctggatttaccgagacaacaatgtaacatcatagatgacattagatgcatgatccgct

SEQ ID NO: 109 - protein, 745 aa, Sorghum bicolor
MEAEQQKQPQRPRRKGQKRKLEDEASAAAAAAAAAAVAAAASSLGSAGADDDNEEEDGSAGTPEICCRHSHAALAREVRVQVDVLVRCASSWRHADRAAAKRATHVLAELAKNEEVVNVIVEGGAVAALVCHLEEPAVAAPTQEEQQLRPFEHEVEKGAAFALGLLAVKPEHQQLIVDAGALPPLVKLLKRQKNTTNSRVVNSVIKRAADAITNLAHENSNIKTSVRMEGGIPPLVELLESQDLKVQRAAAGALRTLAFKNDENKTQIVQCNALPTLILMLRSEDAAIHYEAVGVIGNLVHSSPNIKKEVLNAGALQPVIGLLSSCCTESQREAALLLGQFASADSDCKVHIVQRGAVRPLIEMLQSADVQLREMSAFALGRLAQDTHNQAGIAYNGGLAPLLKLLDSKNGSLQHNAAFALYGVADNEDYVSDFIKVGGVQKLQDGEFIVQATKDCVAKTLKRLEEKINGRVLKHLLYLMRVGEKSVQRRVALALAHLCAPEDQRTIFIDNNGLDLLLDLLISMSSKHQQDGSAALYKLANKAAALSPMDAAPPSPTPQVYLGEQYVNSSTLSDVTFLVEGKRFYAHRIALLASSDAFRAMFDGGYREKDARDIEIPNIKWEVFELMMRFIYTGSVQVTSEIAQDLLRAADQYLLEGLKRLCEYTIAKDVNLDNVSDMYDLSEAFHAVSLRHTCILYILEHFNKICTRAGSPQLIQRVIPELRNFLTKALSSSRSPSPSDRNSQI

SEQ ID NO: 110 - DNA, 16199 bp, Saccharum spontaneum
  source 1..16199: mol_type = genomic DNA
gtaccgcgccggaatcgcactgcttgttccttttcctcctccacaatccgtcacgctctgcgcgccgccgtcgacctatcgaatggaggcggagcagcaaaagcagcagccccagcgcccgcgccgcaaggggcagaagcggaagttggaggacgaggcatccgccgccgccgccgccgccgcggtagccgccgccgcgtcctcgctcggcagcgcgggcgccgacgatgacaacgaggaggaggacggctcggcgggcacccccgagatctgctgccgccactcccacgcagcgcttgcccgcgaggtccgcgcgcaggttgatgtcctcgtccgctgcgcctcttcgtggcgccacgccgaccgcgccgccgccaagcgcgccacccacgtcctcgctgaactcgccaaaaacggtaacctcccttcgccaaacctcactccggccgcgccgatccgtgcacccgcatccttaccgagtggatctggtggttgtcaattgagcagaggaggttgtcaacgtgattgtagagggcggcgccgtggcggccttggtgtgccacctagaagagcctgctgtggcggcgccaacgcaggaggaacaacaactgcggccgtttgagcatgaggttgagaagggcgctgccttcgctctgggcctcctagctgtaaaggttccttcactaattccctaattgagttgtagatgcacttttggtaccaatgcaattacttgtattatcgacgaatttatgttctaaatagggctgtgaattttcaagttcctgtggcaaaggattacaaactttaagaacttcaactatcccatgtatttatatactgtaattctgaaggcccaaacctcattctcatatatctgtatttcttgtaaaaaaactgtaagatcccatgccttttaatagttagaaaaacctaggaacttccaaatgctatatacttggtgtctttctagtcagtctctagtaccctttagaaaaacttaggaacctaagatatcataaccgctctagttctgtagtgtgttttgagcaattgatgctttactcttatgtactttcatcaagttactattgctatggtcaatttaatcatttattctgtgttcactgtaacagcctgaacatcaacaacttatagttgatgctggtgcactacctcctctagtgaaactcttgaaaaggcagaaaaatactacaaattcgagggtggttaatagcgttatcaagagagcagctgatgcaattacaaatcttgcacatgagaatagcaacatcaaaactagcgtcaggttttgttttatgcctctttgatcatttgataacgtttttcttgagaagttttcacttgctgagggttttgttttactgcagaatggaaggtgggatcccaccacttgttgaattgctagaatcgcaggatcttaaggtgcagagggcagctgcaggtgccttgcggactttagcctttaaaaatgatgaaaataaaactcaggtgagatatcaaaatcaatgaagactataattatgttagattttgacatctgaacttgcatatgccttttacacatattcacgacatggtaaattcctgtaatgcagattgttcaatgcaatgctttgccaactttgatcttaatgctgcgatctgaagatgctgcaattcactatgaagcagtaaggccttgtgctattctccagttttgattatgaggcagtgaatattctgatgtcaactccacttctctaagagcactttctcacactgttgagatgtattgtttgattgattatgagcaggttaatgttgttacagataaatatcatatcatttgaaattgtgccattctacaattttgcacaatccttaatcagcatttatcattgcaaggccttgtgaaatatacaattttaatgctccatcttgaaacttaatgctggatcacaacactgtatatttagtgggaaatttcatgctagaccatgtttcatcctcgattatatggacaattttgaattttgaatgtatttccaaagttgaatagaaacttaattttgttggctgttagcagttaccttacagatattatgttgtcctacaaaacatttatatcataggctttgcataatttatttaatatttccttccatgtaagacgcagtttgattaatattttctgatcccattgatgaaattatattaatttggattcatgattgcatgtagccaaccttagtgaaaccactagcagtgcgtttggcaactattgggaaggggcatgggaattggtggtgggagttgtagcgaattacgagaatttgatttttaggtccaatcacttgtttggttcattgagggaaataagacacggaaagaggttgtgtgtgtgtgtgtgtgtgtgtgtgtttttctgtgagaaagggaagtgattggtaggtgttggccctgtaaactcactttcccgtcccaccaaacaaacaaaagatttctaaactcttaccccccaaactcccattcccttgtaccaattacccccaaccaaacgtgccgtagaggttattgaactgactaaggtaaatatcttgaacgcacttttttttgactttttttttgtcaactggcgatagaccttaatggtagttcaggcgatctttgaggctgaaattgaagatttgaaaacttagcaatacacccaaataaatttgagggccagtggcgcagccgtgcaggttaagcctgtatcatggtgcatgtacatggatgcttgaagaattaaatgtttatttgaatgcataaatgtgcggcaagtactgagacaacactagaggctgaggctatttactacttggttcctgaaatgtttcaaaaagtaatctgctgctacttgtaacaggtttgctaagtaaacttgattgtagaagcttatgcaaaacaaataaattgcatgaaactggtctgaggctctgagttacctccttattttgacttgttgttcatccgttgaataaacttctacatggtgcaaggctacctttctgtactaacttccttatcaatccaacatgtttgctgataaactttcatagaatatcagcacaatcttggatctaatctattcatgatttctttaattttattgcaatgcactctaaccatttttctcgactgacatgttaggttggtgtcattggaaatttggttcattcatcaccaaacatcaagaaggaggttcttaatgcaggggcactgcaacctgtgattggattattaaggtatggtcatcatagggaagtgcagctttatgaggtgcataaagaactttataattgtatatatttgttaggttctgctccaatactgctagcatagttgtgcatgtttttttttaattattatcactagcaaacgtgccggaaccgtgacctcttttgtctctctttatgtccttttttgtgtctccctgtttctcgtctcttttgggtttcatctctagcctaccccaacttgcttgggacaaaaggctatgttgttgttgttgttgttgttgtattatcactagcaaatatgcccgtgctttgcaacgggaaaaaagagagtatggtccttagcagaaatgcccgcgcgttgctatggaaaatactaatcctttacatgagaatgggggaccaaaataaatgtatatctccaaagtagaatagtattgcaaatgtactccttccattccaaaggaatggatgtagacatgcagtgcaacatggtgttctaagaactcaagctggtatgggcccaacctagtgttctaagatctaaaacattaagttttctgggattatttttgaatcctaaaacatcacgtgttctgaaacggagggagtaagatggaaaaaaggtaaataaatttctcaaaaagttggtctgcttcaaggacatcagatgagatcagagttaaattctcatccatgattgatgattccttctggctccatagctgtgggtaagtttttagtgcaagttgagtaaatgtcatggtaacaatcaacactgccgagtttctctacatgtgcatgtacagaatacagtctgatattgataaggagctagctccttcgattttcatctgttagtagagacatcaagagtttccatgcacctacgctggacctacttctaaaatctaggaaacatgcctcttctaagatataggatatatggatcatctaggatacatggccctccctttttaaattataggacatatggaccattggccgctcttttttctctgaagctaaaaactgttcagttagtgtgggttagattgacttccttgtacattagttagtcgttaaacttgttagtcgttggattctcactcttggtagtagcagaatccttactctcatcgagagaggatgacactaggagttggggcaattttctggtttatttcttacacaaactcatacaatgttatgccaacctgaggggttggggatacatatttatagggctgctagccagccaagcatatactaagatgctgctaagatgctagtctaagatgctgtcctagatgctagtcaagatgctgtcctaaaatgcctgtcctaagatgctgtcctaagatgctaactgctgtcctaaaagcagtcaaggatgctgttacaaggacacaaggaccatgtgttgcagtcccacaaagaccaaccacacacggacttatttctgtcattctccccctaagtcttgtgtggcgccgtctaggaaactcggaccatcccaatcctggcgcaaagctcctggaacttcactcgcccaagggacttggtgagaaggtctgccagctgatcctgggtgttgatgtagccggccttgatgctcccctcgtccaagcagctccgaatgaagtggtacttgatgcggatgtgcttgctgcgctcatggaagacgggattctttgctaaggtcaaggcggacttgctgtccaccctaagctccaccgcttcagtgtctctgccgaggagatcaccaagtagtcgagcgagccagagcgcctgagtcgaagcggtggaagccgctatgtactcagcctcgcagctggacagggccaccacctgctgcttgaccgactgccagctaacaaggcacttgccgaggaagaagaggaccccgcttgtgctcttgctggtgtcgatgtcgcccgcgtggtcactgtcgctgtacccgacgaagtgtgtcgcgccaggacacctcgggtagtagagaccgtggtcgagagtccccgcaacatagcggatgatcctcttcacagcctgctggtgttccgttgtcggtcgttgcatgaaccgactaatgtagccgacggagaatgccaagtccggccgtgtgtgggcgaggtagcgaaggctccccacaagacgccggtactgcgtagcgtccacctcctccgtcgtgctgtcgcggctcagcttcagcctcctccatcggagtgagggctgggttgcagtcggtgagcctagctagctcagcgatgcgcttgacgtaggcggtctgttgaagcgtgatcccggagtcatcctggtgcacctcgattcccaggtagaaggagagagaccccagatcactcatctggaaggtggccttcatctcttccttgaatgccaccactccgcatccttggtgccggtgatcaccaagtcgtcgacgtagacacccaccagcagggcctttcctctgctgccccgccggtagatggccgcctcgtgcgggctttgctcgaagcccatcccctttagcgtggaatccagtttggcattccacaccctcggtgcctgccgcaagccatagagggccttgcgcaggcggagcaccttgccctccttgccggaaatcgcaaatcccggcggctgatgcacgtagacctcttccttcaagtcgccgttaaggaacgccgacttgacatccatgtgatggacacgccagccctcctgggcagctagcgcaaggagtcgcacggattccatccgtgcaacgggtgcgaaggcgtcgtcaaagtcgattccttcttgctggacgaagccgcgcgccaccagacgcgccttgtgcttgatcacctctctggtctcgtccttcttgagcttgaagacccacttgagagagatggcgtggtggccggctggaagatcggctagctcccacgtcttgttccgctcgacggcgtccatctccatctgcatcgcggcacgccatgccgcgtccctctccgcctcggtgaaggaacgaggctcgccattgtcctgtgcgaggtgcagctctgcctcaaagtcgtgctgcgccagtccagggaccggctgctcgccgaggaggttgtccacggtacggtaacgtagaggctcgccgccgtggtaggcgtcgatgcgatcctcgtcgttggacagcggagtggcgaactccactatgctcgtcgtgggtcgaagctgccggtgccgagcctgaagggttagggtccggtgtaggagagcgaggcatggccggcgtggccggcggtgttggtagcagactgccaaggaggcctgggacgccatcgctgcagcaaaataaaccagaaaattgccccaactcctagtgtcatcctctctcgatgagagtaaggattctgctactaccaagagtgagaatccagcgactaacaagtggtatcggagcatcaaggccggctacatcaacacccaggatcagctggcagaccttctcaccaagtcccttgggcgagtgaagttccaggagctttgcgtcaggattgggatggtccgagttccctagacggcgccacacaagacttagggggagaatgacagaaataagtccgtgtgtggctggtctttgtgggactgcaacacatggtccttgtgtccttgtaacagcatccttgactgcttttaggacagcagttagcatcttaggacaggcatcttaggacaacatcttgactagcatctaggacaacatcttagactagaatcttagcagcatcttagcatatgcttggctggcttgtagccctataaatatgtatccccaacccctcaggttggcatagcattgtatgagtttgtgtgagaaataaaccagaaaattgccccaactcctagtgtcatcctctctcgatgagagtaaggattctgctactaccaagagtgagaatccagcgactaacaaaactgttgtatgcccaaacaaccagaagagagttccatattgtttctcaggcatggaagttgcttgtgggttgattcaactcaattagcatcgatgtgatggctggttggttgagcaacacacatatttattgaggccaataaacacacatttattgaggccaatgttcaataattgaataagatgtgaatctgaagaaacacagatagaaaaggagaagaattgcagacctcgccatcaggttccgtcggagtgggttagcagctcggccgtgctgcccacgactcaacaccactcgttgatcgtggaggaagccaaacctctaaaagccatggacatggactccatggcccatgggcctccaccttaccacgacgtgtcggatgcctggatccggtatcccaggttggagggggaggatggagcttccaatactgcgctgtcgcaaggaaggcgaggggcatgctaagaagctctacgcttggccgcggagccggtgccgtcttctcacaggtgttttccagatctccacccacggggcaatcatgcttcatgtccgtcatggggccaatggccgtgtcgaaggaggtgtagcaggcaggcaggcggaggtgtgagccaagggtggggtcttggacagttggacgaaagtcagggtgcagcattggacgagacgggggaacatacgttcacgcggagggaccgctggtgaggcgatggatgtatgaatgggcttggctgacagacaaaatcctgaggagagaaacttttgctctttaacactcccactgtccaaaaagaatgtaattctctgttccctaggagtcaaacaatgtaaagtttgaccaaatctatactaaaaaaatactaacatttatgatacaaaatatgtatcattagattaactataaaatatatttttatagtaaacctaaatggaaacataaatgttgatactattttctttaaacttagttaaacctaagaaagtttgacctgtttcaaatctagaatatacattctttttgggacggaaggagtattaggtatagaatatatactgcatgctctgttgagcatgccttacaaatgttctattagtgcatctccaacagattacttatcctgcatcccctaaaagtctatctaggtgatctattatgtattattagtagtgtagctctttcttctcctctcccaacagattaccaatacttttaaagtggataggggagagggagtggatagggattttaagtagttaaaacttttaggtattggagataggatgagtaatctgttggagcaaccacaatcccttatattgcatatttttagtatcagggatgaagctttaatgattaagccaaccaaaacaatgctaattattatgttcgagcgtaggctaggccattcctagtccttctattcagatccttgtcatttttatattattctagagaaacacttgactatggctttgtcttaaagagggggagtattgaaccccggttgtccaaaaactcgctgaaaccggttcagtgaggtatccacatttggcgagggactggaattttgggtgagcggccttcttgttgggaaactgtaccaaccaagctactggctcctttctcatcttgtattctagaataccatctttttcaaatgagaaggttctttgtcattgttattcaagttttaaagggtgttctatgatttgctctacactggcaactcacctcaagaatatctgcttgatgtatgaaacattactttctttatttttttcagctcatgttgtacagaaagccaaagagaggctgctttgttgctagggcaatttgcttcggccgactcggattgcaaggtgcttaataaatatggaatacttattgtttacaagtcttcagtaaattttgcaaatccactggtaggttagtcaaaactaaagagagaatcgcaccactaatccctgaatttgcatggttgtctctcgcacacccctcaatttgtaacttacattgtgagcccttctaactttggacccattgtatcatctgcccaaattaccgtcagctacttagtttaattgatggtgctgatgtggcatcaaacataggctgttatactggactgtttattttcttttatcatcgcttccttcccttttcttttccattgatcaatacatcactgacatggatatgtagatgatgccatcgaattgactaattatttgaccagtcaacaaaatattttgttgtatgtgtcattatttatggtgtactcaactggtagccgtgtcttcttgtgaacaggcccttattgcagttaggcattatttatgaatgtgactttcaatacaatgtatatttggctaatattagactatcaatccccttctttttcaagtagtatttattttgtattattgttccataatttgatggattttttgtgtgattggaatgtatattgcacatgtcttaaggttataggccaaaacctgtgtcaacataccatggagagctggtcccatgtttaatgctcatgtcaacacaatttgttatgttaaggtgatttgggccaatgttgcaaacagacctgaagtttaggggggctagcaaagtaatttgcaagttgagggaagctggtgagagtgagacaacaacacaactttaagggctagtggtgcaattctctctttttcagaagtactggtgatttacatgtgtaacatttatgtgcactgtatgttgggatagaagtgaaattagtaaaccccatttctgaccaagcacatcaggtgtgacagattctcattgctgggaccgtctggctccttttgacatgatgcctcatagggcctacatgctgctggccagtccatgcatgacctcacttattctccttgttgcttttttctaactatgcctctgcatttcttattcttggtctgatctgggtgccacacaatcacgaatccagattggtgtgccatatggcagcctctgcaactgccctatccggtgctggcacacttatcttccttatccagtccatcctcacacggagtcatggacatgttctgcaaatatggtgggctcatgtttccggtttctgcacgtgccaagtccccagctctgccctacctgcattgcgtcttcatcactgtgcttggcaacaacacaccctgggttctatgctcaagctgaacctagctcggctaccacgcatttcaattgctcccccgctcctggcttacaccacaccctaagccctcccctaccaataaatcattggatataagatttaagtttttgtagaagttagtttctttgttgcagaggtaggttttgctttatttttttcgatgtttccttgggagatgggagagagggcagccattgggaccacttgtctgttctttgagtggagagatgcagaaggtagaaaaagaatgaactcaacaattgaatataatataaggaaatctagaatgataaatcttattatctaaggaatgaaataaaagcaaagagatataagatgttttctccagttaattcgtttctgaacttgatagattaatatatatgtttgtttacaggtccatattgtgcaaaggggtgcagtccgtccactaattgaaatgctacagtcagctgatgtccaactccgggagatgtctgcttttgcacttggcaggcttgcccaggtttactttttatttttaatatagcatactttttaatgtttataaggtgctttactgttttctactctagagaatcagtgtaggcagtgaaataaaaacaccacagaatttttcttgctctcttacaaaatccacacaacgtataactttatcaaattagttcccttgcagccttgctcctctgttgataggaactatatgtggggactggggatgcaaagatcataatatgtttagggcaaaaccatagtgagtttgctggcaccacataccttccttatccagtccatcctagacatgaacagattttcctaatatgcgggcttcatgttattggtgtctgcatgtgccaagtcccttgctctgcccttatctgcattgcatcttcaccactgtgattgtcaacaacacacccagggtgctgctgtattcgaggtacctctggtaccacacacagtccaattgctccgccaagtaattgaagttacgcagctattctccatatgttggctcaagagcccatatgttggttgcacagaattctgtcttttgtttttgagttaaatgcaccagaggtccattaacttgtgttggggtttgtccatcaactctaaaagttgattttcgaatccataaacttttaaaatggttcgccacaggtccatatcccttcatttggcccttagattctacttccgggtccataagcttttaaagtggttcaccacaggttcataccccccttcggttggcccttatatctgacgtggtatgcagccagcatggcatgaaatttgctgagcccatgcttatcctccgcctgtgctggcctcctttccactccctcaagcctggcatctgtgcctttgttctatctctgctccagtgctcgccaccaccattaccggtcaccgagctcccactaccgtgcctggcatctgtgcctctgctctatctctgctccagtgcttgccaccaccattaccggtcaccgagttcctgctaccgccgctgttccttgccttgtgcttcagctctgtcctagaaatgagctctactgagtccatctctgcctcctctaccctttgcgctcgttggacgcacaaacaccgtgttggagctcctagcccactgtactgcagctgccctgccatggtcgagctcgcttgcgctaccattcttgtcggtataggacatcaccacttcaatgagtgtgcggttgagtccgctgtggtcccaatcgtcctagtgtgcagtgcgcacgcatttagggcaagtctatgccggacccaccatctaccttctacctgccatcgaccgccggattggcacgctcgtggccgacccgctagtggcctccatcagacaaattgaaaccaccctcgggtgcgctggtagctcgtggtcccatccattgccgccgccgagtgctcccttggccgaatcggcccctccacgccatacttgtgcctatgttgatttggggaagaaagaagaggaaggagatgattcatgggacacatgtgccgtcgcgtctctgccatacgtccttgtggccctatgtcgcgtcacagggcctacgtcgcgtgccaccgccccctacgctcgtgccgcttaccggcacctgcgctcactgctgcacactgccgctcagggaatagagcaaggagaagggagggaggaggggctaattgcaaatttcatgccatgctggctgctgactccacatgccacatcagatctaagggccaaacgaaggggtatggacctacaatgaaccacttataaagtttatggacctaggaatcaacttttatagttgacgggcctaactgaaacccccgcataagttaatggagtgcatctaagtctgtttttttttgtaatattttggtttttgctccaacatatgctctgaccgctaaccatgcatatctaagcaaaacttttgaacatttgtaattcctaggttacaccatcctggcttgatccctagcttagttatcctagcccaatgatgggtgcttggagcattccctgtgactttggccctagctaatcgtcgattaggtgctaggagctggtctgccgtctgacaattaaagacccactttgtcagtggtacattctagcagagcgataatatttctggcaattgcaaccaaccaaacttcatagcatacagagtgcaatgtggagtgaaccagttaaaaagtagacccagatcctcacttgagagattatggacccagttgagtatctgggaaaagtttaacgatctaacgctttttcgctctttcatatcatataatgtaaggggaaatccccattcatcttttcctttcacttatgggttagtggggttgtttctttttctttctttctttctttctttcttagttgcaactcgtaatctaatctaaagagtcttttatcaggacacacataaccaaacaggtattgctcttgcttagttgcaactcgtaatctaatctaaagagtcttttatcaggacacacataaccaagcaggtattgcatataatggtggcttggtgcctttgttaaaacttcttgactcaaaaaatggatctctgcaacataatgctgcatttgccctttatggagtcgcagataatgaggtaatttacgatctttttttttcacaaggtttgccatatctctcaaatatcccttttccactattggttaataattccacactccatgttcctttgtaatgcgttaactcattttttataaaatgtttatcttatatttcttatcttcattatttctgaagcaaatcactgttcttccttataggactatgtatctgacttcattaaagtaggaggtgtccaaaagttgcaagatggagaatttattgtccaggtacattggccttcattgtatattggtcactttgttgtgaatgctttttattaagctattcttaatttcaggcaacaaaggactgtgtggcaaaaacattgaagaggttagaggagaagataaatggacgagtaagttctgcttgcaaggtttctgtatttcgttgtttgcaatgtgcttgactagtatatatgaagcttgttcccatgtgatggtttacaggtattgaaacacttgctttatttgatgcgagtaggagagaaatctgtgcaaaggcgtgttgctctggctcttgcacacctttgtgcccctgaagatcaaagaacaatttttattgataataatggtaaacaattttgcaaccactgaaaaattgtaccttttcatttccattctactgtatggtgttcttcatgaatttaaattctgggtcatccaggtctcgacttgcttcttgatcttctgatttccatgagctcaaaacatcaacaagatggctcagcagcattatacaaattggctaacaaagctgcagcactttctcccatggatgctgcccctccatccccaacacctcaggtatgcaaaagaattattaaatttaaatttactttggattacgtgtgctgtttgagttgcagtgactttatgagctgactgtggtatggttaaaaatagatcacaatggcatgatcttcagtgtgctaggatgcacatgaatttattttgattaatcattgtggaatggtgctttggttcaacaaggtatataaaggcccaaacgagtctcttgtagtccaacctgttgtgaatgatagtgcgtacaacctgctggaggaaaataaatgttcctctggcatgccatgaaaggtaaatgttggactgctgatcagcttgcaaaacatgatctgtctcatccagataaaagcctactctgtgatcacgaagaggaaacagtccagcacatccttacaacctgtgtctttgcaagacagttttggcataggttgttcattcttcattgcacttaactgcagcagctggtgcctagcattactaaacatagtttcactacttggtggcagagagctagcaaaagagttagcaaagatcaaagaaaaggggttaacaccctcatcatcttgggtccctggatgccctggaagcagaggaatgcgtgtgtttgagggagactctccagtgtccctactacacctagaaacctgaagttagaagctcatctctggatgcttgctggggcttccaagctacagggtctttggctaagtcagttagaaatctaggctagcttagttttctttgttgtaaccccccttaccttggtcctagtaagaggggtgcttgtatgtaccatttcttttccctataatacaaagatacgcagctctcctgcatgttcgataaaaaaaaatatcatgtcgatatttttatagtgcttggcattgtgttaaaaattgtggtcagaatttagctatcattggcatttttaacaagatttccaaacactgcctgtattttgctgtcctaaataaagtcattgtgacattgtgggatttttccatccaattgttctggtaatggctgaggcactggcaattgttactgaatttatatttcattgcaggtttatcttggtgagcaatacgtgaatagttcaacactttcagacgttactttcttggtagaaggttggtactatttcatgactgtgatttcatcagtagatactttaaataattcttttctatcgtgtcccagataatcttaatcccttcttctacaggaaagcgcttttatgcacacagaattgctttgcttgcttgttcagatgcattccgtgcaatgtttgatggcgggtacagggtgagttttgacttgccacaacataatgtgcttttgctggttttagtctgttgatctctttccatagttgatatattgctgctgtatatagtatgttagttttgaacaaaccaatctcatgtctaatttaaaggtcattttcttaaccaggaaaaggatgcaagagacattgaaattccaaatatcagatgggaggtctttgaactcatgatgaggttagtaagtcattgacctcccttctcgtttggccacagttctcattctgttgatgaatctgcaactatttttcctcttttcttttttatgccactgtatgctggattaaagtctgaaaccctctttggttttgcagatttatctatacagggtcagtgcaggttaccagtgaaattgcacaggatcttcttagagctgctgatcagtatctcttagaaggcctcaaacgcctatgtgaatatactattgcg

SEQ ID NO: 111 - protein, 622 aa, Saccharum spontaneum
MEAEQQKQQPQRPRRKGQKRKLEDEASAAAAAAAVAAAASSLGSAGADDDNEEEDGSAGTPEICCRHSHAALAREVRAQVDVLVRCASSWRHADRAAAKRATHVLAELAKNEEVVNVIVEGGAVAALVCHLEEPAVAAPTQEEQQLRPFEHEVEKGAAFALGLLAVKPEHQQLIVDAGALPPLVKLLKRQKNTTNSRVVNSVIKRAADAITNLAHENSNIKTSVRMEGGIPPLVELLESQDLKVQRAAAGALRTLAFKNDENKTQIVQCNALPTLILMLRSEDAAIHYEAVGVIGNLVHSSPNIKKEVLNAGALQPVIGLLSSCCTESQREAALLLGQFASADSDCKVHIVQRGAVRPLIEMLQSADVQLREMSAFALGRLAQDYVSDFIKVGGVQKLQDGEFIVQATKDCVAKTLKRLEEKINGRVLKHLLYLMRVGEKSVQRRVALALAHLCAPEDQRTIFIDNNGLDLLLDLLISMSSKHQQDGSAALYKLANKAAALSPMDAAPPSPTPQVYLGEQYVNSSTLSDVTFLVEGKRFYAHRIALLACSDAFRAMFDGGYREKDARDIEIPNIRWEVFELMMRFIYTGSVQVTSEIAQDLLRAADQYLLEGLKRLCEYTIA

SEQ ID NO: 112 - DNA, 12013 bp, Zea mays
  source 1..12013: mol_type = genomic DNA
ttgtttcttttttctaaaaaccaggagaggttattattaaaacatcggtcgtttaaataaaaagtgtttaattaaaaaaaaccattcattttttaatttctacttttctgtcgaacccgaccctaccgcgccggaatcatactccttgcgccttctccttcctcaatccgacacgctctccgcgccgccgtcgacctatcgaatggaggcggagcagcaaaagcagcagcgcccgcgccagcgcccgcgccgcaaggggcagaagcggaagttggaggacgaggcatccgccgccaccgccgccgccgcgtcctcgctcggcagtgcgggcgccgacgatgacaacgaggaggaggacggctcggcgggcacccccgagatctgccgccactcccacgcggcgcttgcgcgcgaggtccgcgcgcaggttgatgtcctcattcgctgcgcctcttcgtggcgccacgcagaccgcgccgccgccaagcgcgccacccacgtcctcgctgagctcgccaaaaacggtaaccttccttcgccaaacctcataccggccgcgccgatccgtgcacccgcatccttaccgagtggatctggtggttcttggtggttgtcaagagcagaggaggttgtcaacatgattgtagagggtggcgccgtggcggccttggtgtgccacctagaagagcctgctgtggcggcgcaaacgcaggaggaacaacaactgcggccgtttgagcttgaggttgagaagggcgctgccttcactctgggcctcctagctgtaaaggttccttcattgattccctaattgagttgtagatgcacttttggtaccaatgcaattacttgtatttttgacaagtttatgttctataaatagggctgtgaattttcaagtttcacttaacatataggattactaaggaagaacttcaatacgcacgcgcgcccatgcctgcccgcacgcatatatacaccttgggtgatggaccaacgatccatcacctgcacccaatgctgcagttggatcaaccagatatcgaagtgacatagtcggatgtgttcggtcgggtatgggtgatggactattggtttgtcaccctaggtgacaaataatgctcatatatagtagttctaaacacccaaatctgcatcctcatatatctgtatttcttgtaaaaaactgtaagatcccatgccttctaatagttaggaaaatttaggaacttccaagtgctacttggtgtctttctagtcagtctctagtaccctttagaaaaagagtaaagtacactgccggttccgaaacttgtagcgttgtgtcatcccggtccctaaactatcaaagtgtgcatccaggtccctaaacttatgaagtcatatcatcctgatccctgaactctcaacatgcacatttaggtccttgtacttgtatggttgtgtcatctgggtctctaaacttgtttttagtgtcatcaaaggttcaaactacttggacctgtgatgacactaaaaacaagttcatggacccggatgacacaactatagaagtataaggaccagaatgtgtaggttgagagcatggtttttaaagcggtaaggcgctccaaggcgttggaccaccgcctagacgcctaggcggcgcctaggcgacgcctaggcgaggtaggcgggcaaggcgcctaggcgtcagaccaccgcccggacgcctaggtgacgcctaggcgacgccttaaaaacagtggttgagagtttagggaccaggatgatataacttcacaagtttagggacctggatgcacatagagtttagggaccgagatgacacaacgctacaagtttagggaccaatagtgcactttactcttagaaaaacctagaacctaggatatcctgtttgctctagttctgtagggatcttttaatagttgtgttttgagcattgatgctttactggtgtgtacttttcatcaagttactaatgctaatttattatgtgtctcactttaacagcctgaacatcaacaatttatagttgatgctggtgcactacctcccctagtgaaacttttgaaaaggcagagaagtactacaaattcaaggatggttaatagcgttatcaagagagcagctgatgcaattaccaaccttgcacatgagaatagcaacatcaaaactagagtcaggttttgttttatgcctctttgatcatttggtaaccttttccttgagaacttttcacttgctgatggttttggtttaccgcagaatggaaggtggaatcccaccacttgttgaattgctagaatctcaggatcttaaggtgcagagggcagctgcaggggccttgcggactttagcctttaaaaatgatgaaaataaaactcaggtgagatatcaaattatcaaaatcaacgaaggctatatttatgttagattttgacatctgaacttgcatatgcttttacacatattcacaacatggtaagttcctgcaatgcagattgttcaatgcaatgctttgccaactttgatcttaatgctgcgatctgaagatgccgcaattcactatgaagcagtaaggccttgtgctattctccagttttgattatgaggcactgaatactctgatgtcaactcgacttctccaagagcactttctcacactgttgagatgtatgtttgatttattatgagcaggttaatgttgttacagataaattatcaaatcctttgaaatagtgccattctacggttttgcacaacccttaatcagcatatatcatcgcaaggccttatgaaatataaaatttcaatgctccatcttgaaacttaatgttggatcataacactgtatatttagttaggaaatttcatgctggatcatgttccatccttggtcacatggattttttttaatatatttccgtagtcgaataaaaacttaattttgttggctgttagcagttaccttacagatattatgttgttctacaacacatttatatcataggctttgcataatttgttcaatatatcgtgccatgtaagatgcaatttgattaatattttttgatcccatcgatgaagttatattaatttggattcatgattaccctgaatttgtgcactgatattgatctattgcatatagccaaccttagcgaaaccacaagcagtgtgtttggcaactattgggaaggggcatgggagttggtggtggggagttgttggaacaaattatcggaatttgatttttagttccaatcacttgttttggttcattgagggaaatgacacgtaatttaagaggaaattcatgtcccctgtttggtgtgtgtttgtaagaaagggaggtgattggtaggagttggcctactaactcactttccagtcccaccaaacaaacaaaagatttctgaactcaccccaaactcccattcatttgtaccaattacccccaaccaaaagtgctttactgctgtagaacttattgaattggctaagagaaatatcttgaatgcaatagaccttaatggctgtattaagctagttcaggcgatttttgaggctgaaattgaagatttgaaaacttagcaatatgcccaaataagtttgagggccagtgcatagttgggctggtttgggctagtcttttccttatctttatccttttctcgttattattattatcattgttgttgttgttgtgcaaatactttctcaaatattaacatttccctatttttttaatatatttaaggcgtcgcctcgccttacgctttatcgcttaaaagttaaaagggagtcactcgccttacctcgctttaccgctttaacaactatgggccagtggcgcagccgtgaaggttaagcctgtatcatggtgcacgtgcatggatgcttgaagaattaaatgtttattggaatgcataaatgtgtggcaagtactgaggcaacactagaggctgaggctatttactacttggttcttgaaatattaaaaaaagtaatctgcacctgctacttgtatgtttgctaagtaaacttgattttagaagcttacataaaacaaataaattgcatgaaactggtccaaggctttgagttacctccttatattgacttactgttctatgctcttttatccgttgaataaacttctacatggtgcaatgttacctttctgtactaacttagcaacccaacatgtttgctgataaactttcatagaatatcagatctaatttattcatgatttctttaattttattgcaagcactctaatcatttttctccactgacatgttaggttggtgtcattggaaatttggttcattcatcacctaacatcaagaaggaggttcttaatgcaggggcactgcaacctgtgattggattattaaggtatggtcatcaactcatcatagggaggtgcagctttatgaggtgcataaaaaacttcataattgttatatttgttaggtcctgctgcaatactggtagcatagttgtgcatgttttttttggattattatcactagcaaatatgcccgtgcgttggaacggaaaaaatagtttgtgcataaaagagtaaggttcttactccttagcagaaatgaccgtgcgttgctatggaaaatactaatactttacatgagaaaggaggatcaaaatagatatatctccaagtagaataactactgcaaagatactccttttgttccaaaatccttgatggtttaggatttaattaaggaataaatctctaaataaaaggaatggatgtagacatgcaggctgcaacatggtgttctaagaactcaagctagtatggggctatgggcccaacctagtgttctaagggcaaggcagacccagtgccggaggctcctacatgagtaaacacccgcccccaagatacggtgagactgcttcaaatccgtgccgtggtgactcagtgagataactctcacaactccaccttgcctgcccttcaacctagtgttctaaggactaaaacatttagttctctgggattatttttgaatcctaaaacatcaggtgttctgaaacggagggagtaagatggaaaaaagctaattttctcaaaaagttggcctgcttcaagggcatcagataagatcagagttaaattctcgtccatgattgctgattccttctggctctgtagctgtcggtaagttcttagtgcaagttgatcgaatggcttggtaacaatcaacaccaccgagtttctctacatatgcatgtacagaatacagtaaaccctactcagacccttctcatttttatagtattctagagaaactctcgaccatgactgtcttaaagagggggagtattgaacccctgttgtccaaaaaactcgctgaaaccagttcaatgaggtattcacatttggagagggactggaattttgggtggttggccttattgggaaactgtaccaaccaagctattggctcctttctcatcttgtattctagaataccatcttattcaaatgagaaggttctttgccattgctaatttgctattcaagttctaaatggtgttctatgacttgctctacactggcaactcaccccaaggatatctgcttgatgtatgaaacattgctttctttaattttttcagctcatgttgtacagaaagccaaagagaggctgctttgttgctagggcaatttgcttcagccgactcagattgcaaggtgcttaataaatatggacttatggagtaattattttttatatgtcttcagtaaattttgcaaatatactggtacgttagtcaaaactaaagagagaatcacaccaataatctctgagtttgcatagtctctctcccacatccctcattttgtaatttacactgtgagtcctaactttgcacttgttgtggcatcggccgatggcaccgttagctacttagcttaattgctggtgctgatgtagcatcaaacatgggctattatactggactgtttattttcttttattgtcgcttccttccatttttttccattgagcaatacatcactaacatggatatgtagatgatgccattaaattgactaattattttaccaccatcaccaccacaacaaaagctttttagtcccaagctagttgggtaggctagactttaaatcccaacagagctcacgagtcaaggttcgggcacatggatagctattttccatgcactcctattcaaggctaaatcattgggtgtattccatcctttgaagtctccttttagtgcctgcatggcggctggaggtggagggccaaccatggcggcgggaggcggtgagccggtggctgtgactaggggaggggagggagggagaaactctggctggataccatgttggaaagaaagaaaaccctagcctcttgagggcttgtttggttgcattgggattggaggggattgagggagattaaatttctttgtattcaattttgactagcaagggatttaatccccttcaatccattcctaaccgaaaagtcttgagtgggttgagtattgcatatattagaaaatagagttacatgggctgggccaagacctataacacttaggcagaatacaataatctaacaccttccttgggagatgggagagaggacagtcattgggaccacttgttctgtttgagtggagggatgcagaaggcaggaaaagattgaactcaacaattgaatatagtgtttagtataaggaaatctagactagaatgataaatctcattatctcaaggaatgacacaaaagaaaagagatagaagatattttatccagttaatttgtttctgaacttgatagattaatatattcgtttgtttacaggtccatattgtgcaaaggggtgcagtccgtccactaattgaaatgctacagtcggctgatgtccaactccgggagatgtctgcttttgcactcggcaggcttgcccaggtttattttttatttttaatatagcatatttttaatgtatataaggtactttactattttctactctagagattcagtgtaggcagtagaataaaaacaccacataatctcttacaaaattcacaccgtgtataactttatcaaattagttcccttgctcctctgttgatgggaagttgggaactgtatgtggggactggatgcaacataatatgtttagggcaaaccatagtgagtttgctttcaccacataccttccttattcggtccatcctagacatggacagattttccaaatatgctggcttcatgttaccggtgtctgcatgtgccaagtcccttgctctgcccttacctgcgttgcatcttcaccacatgtttgtcaactacacacccctagaaataaacttttagagttgacgggcctaacagaaacctcgcttaagttattggagtgcatttgactctgtttttttgtaagggaattatgtgtattggtttttgctccaccatatgctctgactgctaaccatgcctatcttagctaacatttgtaagtcctaaatactaggtgatatcgttctggcttgttccttagcttagctatccccctagcccaataatgggtgcttggggcgttccctgtgactttggccccagctaattgtcgattaggtgctaggagctggtctgctgtctgactattaaagatttaaagatccactttgtcagtggtacattctagcagagcgataatatttctgacaattgcaaccaaccaaacttggtagcatatattttccgtgtgagattgtttgcctagttttatataaagtgcaatgtgaaatgaaccatttaaaaagctgacccagatcctcacttgagagattatggactcagttgattatctgggaaaagtttaacaatccagcgcatttcattctttcatatcatataatgttagtgggattgtttcttttactttctttctttgcttagttgcaagctgcaacctgtaatctaatctaaagagtcttttctcaggacacacataaccaagcaggtattgcatataatggtggcttggtgcctttgtttaaactccttgactcaaaaaatggatctctgcaacataatgctgcatttgccctttatggagttgcagataatgaggtaatttactaatttttttcacaaggtttgccatatctctcaaatctcctttttccacaattggttaataattccacactccatgttcctttgtaatgggattatctcattttttataaaatgtttaccttatatttcttatcatcattatttctgaagcaaatcaatgttgtttcttataggactatgtatctgacttcattaaagtaggaggtgtccaaaagttgcaagatggggaatttattgtgcaggtacattggccttcattgtatattggtcactttgttgtgattgctttttattaaggtattcttaatttcaggcaacaaaggactgtgtggcaaaaacattgaaaaggttagaggagaagataaatggacgagtaagtgttttttgcaaggtttctgtattcgttgtttgcgatgtgcttgactattatttatgaagcttattcccatgtgatggtttacaggtgttgaaacacttgctttatttgatgcgagtaggagagcaatctgtgcaaaggcgtgttgctctggctctcgcacacctttgtgctcctgaagatcaaagggcaatttttattgataataatggtagcaattttgcaaccgctgaaaattgtaccttttcatttccattctactgtatggtgttcttcatgaattcaaattctgtgccatccaggtctcgacttgcttcttgatcttctgatttccatgagcccaaaacatcaacaagatggctcagcagcattatacaaattggccaacaaagctgcagcactttctcccatggatgctgcccctccatctccaacacctcaggtatgcaaaagaattattcaattcaaatttactttgtattctgtatgctgtttgagttgcagtgactttatgagctgactgtggtatggttaaaaatagtatcacaatggcatgaccttcagtgtgctaggatgcacatgaatttattttgattaatcattgtggaatagtgctttggttcaacaaggtatataagggcccaaacgagtctcttgtagtccaacctgttgtgaatgatagtgtgtacaacctgatggaggaaagtaaatgttcgtctggcttaccatgaaaggtaaatgctgtgttcatcatctgcctcatccagatagatgcctactctgtgatcaaggggtggaaacagtccagcacatccttacaacctttttcttttcaagacagttttggcataggttgttcattgcatttaacttgcagcagttggtgcctagcatgactaaacatagtttcagtacttggtggtggagagctagcaaagatcaaagcaaaggggttaacactaggggtggtaatggatcacgatccaaatgtttcttcacaataagttagggcccttaattaattttagttcaaaaatgaataagaatagtgcccgatcctaatccgattcgatccttgaaatgtatagtgtaaaatctagagcccattaccacccctagttaacatcctcatcattttgggtgtctgggtgctctggaagcagaggattacgtgagactctccagtgtccgtactacacctagaaacctgaagttagaagctcatctctggatgctagctggggcgttcaagctacagggtcttgggctaagtcggttggaaatctaggctagcatagttttgtttgttgtaatctcctttaccttgatcctagtaagaggggtgcttgtatgggcgttcaagctacagggtcttgggctaagttggatggaaatctaggctagcatagttttgtttgttgtaatttcctttaccttgatcctagtaagaggggtgcttgtatggaccatttcttttccctataatacaaagatacgccacatacggctccctgcatgttcgataaaaatggcatgccgatatttttatactgcttggcattgtgttgaaaattgtggacagaatttaggtagcattggcattttttacaagatttccaaacactgcctgtgttttgctatcctagataaagtcattgtgacattgtgagatttttccatccaattgttctggtaatggctgaggcactggcaattgttactgaatgtatatttcattgcaggtttatcttggtgagcaatacgtgaatagttcaacactttcagatgttactttcttggtagaaggttggtactatttcacgaccctgatttcatcagtagatactttaaataattcttttctatcatgtcctagataatcttaatcccttctacaggaaagcgcttttatgcacacagaattgctttgcttgcttcttcggatgcatttcgtgcaatgtttgatggcgggtatagggtgagttttgacttggcacaacataatgtgcttttgctggttttagtctgttgatctctttccgtagttgatatattgctgctgtatatagtatgttagttttgaacaggccttgaatctcatgtctaattcaaaggtcattttcttaaccaggaaaaggatgcaagagacattgaaattccaaatatcagatgggaggtctttgaactcatgatgaggtaagtcattgacctcccttctcttttggccacagttctctttctgttgatgatctgcaactattttttctcttttctttttttatgccactgtatgctggattgaagtctgaaatcctcttcggttttgcagatttatctatacagggtcagtgcagattaacagtgaaatttcacaggatcttcttagagctgctgatcagtatctcttagaaggactcaaacgcttatgtgaatatactattgcgaaggtgactagaaaagctactctctattccttgtttaaaccacatattagatattaatttgaatgccgttatttgccttgtaggatgtgaatctagataatgtatctgacatgtatgacttgtccgaagcctttcatgccgtgtcactgagacatacatgcatcttgtacattctggaacattttaacaagatctgcaccagagccgggtacgttctcttgataataacctttgatctgagaccggtacgatttcaagtagctcaaatcttagcatgcaatcttgccatgcagttctgcacagctgatccagcgtgttattccagagatccgcaattttctaaccaaggcactgaattcatcaagaagtccaagtccaagcgacaggaactcgcagacttgatgagtcccaattcattggcaccgacgccgtcatctgaccaaagttgctggagatcctgtacagtaaaatttctggcgctgagcgttcaatggtatctattttgggtacatggtggcgcggtccttgaaattaacatcagcaatgtaacaaaattttctaagatctagttgaggataaggataaggagaacatatctcgtactcatgcatcgaccagcttacactgggataggctatagttggatggtcctggccgtaattcgtcggtctcagctttgattgagtttagtgttgtttccactttccagttcacagttcagtgtatgcccgcatctgtttatttaaagtattaagcgtgaacaagttagacattaggacatgtacaatgatatcttgaggtgtctaaagggtttgcaaaaaaaattatggagccgtctctccgtgaagagacgccttctctgactcgtaacctaagtagcaatagatgcctcatttcttattgtacgaattcgtcgtatgttttttcattcggcgctgtataagtgtatttacttttgtatttattaatagactatatttataaacactattatataatagagtcttttagttgtc

SEQ ID NO: 113 - DNA, 20676 bp, Zea mays
  source 1..20676: mol_type = genomic DNA
gttttcgttcccacgcacattcatttttttcccttctcatttctacttttctatccaacacgaccctaccggctaccgcgccggaatcacactgcttgtgccttttcctcctcaacccgacacgctctccgcgccgtcgtcgaccaatcgaatggaggcggagcagcaaaagcagcagccccagcgcccgcgccgaaaggggctgaagcggaagctggaggacgaggcatccgccgccgtcgccgccgccgccacatccgcagcagcatccgccgccgccgcctcgctcggcagcgcgggcgccgacgatgacaacgaggaggaggacggctcggcgggcacccccgagatctgctgccgccactcccacgcggctcttgcccgcgaggtccgcgcgcaggttgatgccctcgtccgctgcgcctcctcgtggcgccacgccgaccgcgccgccgccaagcgcgccacccatgtcctcgccgagctcgccaaaaacggtaacctcccttttccaaacctcattccggccgcaccggtccgtgctcccgcatccttactgagtggatctggtggtcctcaattgaacagaggaggttgtcaacgtgattgtggagggcggtgccgtggcggccttggtgtgccacctagaagagcctgctgtggcggcgccaacgcaggaggaacaacaactgcggccgtttgagcatgaggttgagaagggcgctgccttcgctctgggcctcctagctgtaaaggtttctttattaattccctaatttagttgtagatgcactttggtaccaatgcaattacttgtatgaccgacgaatttatgttgtacatagtatgaattttcaagtttcctgtgacatgggaatatgggattacaatgtttatgagcttcaactatcccatatatgtacagtaattctgaacgcctgaacctgcatcgtcatatatctgtatttcttgcaagactgtaagatcctattccttttaatagttagagaattctagaaaattccaagtgctatctactttatactttgctctagtaccctttataaaaacttaagagcctaagaaatactaaaccctctagttctgtggggatctttaatagttgtgttttgagcattaatgctttattgttgtgtacttctcaccaagttactattaatcatttattttgtgtctcactgtaacagcctgaacatcaacaacttgtagttgatgctggtgcattacctcctctagtgaaactcttgaaaaggcagaaaaatactacaaattcgagggtggttaatagcgttatcaagagagcagctgatgcaattaccaatcttgcacatgagaatagcaacattaaaactagcgtcaggttttgttttatgcctctttgatcatttgataaccttttcctcgagaagttttcacttgctgatggttttgttgtactgcagaatggaaggtggaatcccaccacttgttcaattgctagaatcacaggatcttaaggtgcaaagagcagctgctggggccttgcgtactttagcctttaaaaatgatgaaaataaaactcaggtgacatatcaaaatcaatgaaggctatacttatgttagattttgacatctgaacttgcatatgctttttacacatattcatgacatggtaaattcctgtaatgcagattgttcaatgcaatgctttgccaactttgatcttaatgctgcgatctgaagatgctgcaattcactatgaagcagtaaggcctcgtgctattctccagttttgattatgaggcactgaatattctgatgtcaactccacttcactaagagcatttttcacactgttgagatgcatcttttgactgattacgagcaggctaatgttgttacagataaatgatcatatcctttgaaattgtgccattctacagttttgcacaatccttaagcagcattaattattgcaaggctttatgaaatataaaattttaatattccatcttgaaactttatgctggatcataacgctgtatatttacttgggaatttttcatgctggaccatgttccatcctcggtacatggaaaatttagaatgtatttctgaagttgaatagaaacttaatttcgttggctgttagcagttaccttacaaatattatgttgtcctagtgtcctacaacacatttatatcataggctctgcataatttattcaatatttcctgccatgtaagatgcagtttgattaatatttttctgattccatcaatgaaattatattaattttgattcatggctaccctgaatttttgcactgatattgatctgttgcatacagccaaccttagcgaaaccactagcagtgcgtttggcaactactgggaaggggcatgggaattggttgtgggagttgttggagcgaattgtgagaatttgttttttaggcccaaccagttgtttggttcaaataagatagggaatttaagaagaaattcatgtctgtttggcataattgctgcttgttgaaaaaaacagcttatttgagaagttggtgaaaagcaacttctgcttattgactgcttttagttcattctaagaagtagcttctgcttattgattgcttttagttcattctaagaagcagctgaactgataaccctacatgatcggcttccatgtgagctctcttctttcccctgcaaataccttggtctgcctctgtctttaaaaaaactgtccaaaaatcaggtgcaacccattattgacagagtggctgatcaattgtctgggtggaaaacggatctaatgacaagggctggcagaagagtacatgtccagtatgtgatgacatgcatgctcatttatttagccatggcagttgacatacccccaggatcactcaaagttattgacaagatcagaaaaggctttatctggcgcggaaggaaagatgtaagaggaggacattgtttagtggcttggggcagagtctgtagacctctcgaaattggcggtcttggtatttctagtctcaaaaaattgggatgggccttaagaatgagatggctgtggctgagcaaaacagaactggataaaccgtggtctcaatgcctatgcggttttccaaaaaaatgaaggccttcttttccactgccatgctcactgaaattgggaatggttcttcaaactcattttggcaagatcgttgggtccatggaaagaaaattgaagaccttgctcctcgactgcttgcagctgtgccaaataagattaagaacaacagaactgttcttgaggccttaacagatagaaaatggttaactgatattaaaggggccttgacagtaggagtttttgctgacctcctagatctctgggatgcacttcaaacaatccagctacatccagacatggaggacagacatattttcaggcttgctactgatgggaattactcagcaaaagcagccaatgagggtttcttcattgggtcaacccaagctgaacattgggaattaattttgaaaacttggtctcctcctaaatgtaaattcttcatatggcttgctgatttaagaagatgttggacagcagaccgtctagagaaaagaggtttaagccatcctgacaaatgtcctttgtgtgaccaagatcaagaaagcatagaccatatgattggtgggttgtgtctttgctaggaacttttggttccagctgctcggacaagtcaatctgcctggttttgctcctcagctgggggaagagagcactatgcagtggtggagtagaaccagtgagcagctgcaggggattgcaaaaaaaagggtttaattctttaatcaccctcgggctatggactctccggaaccatagaaatgggtgtgtctttgacagaattaaacccagcctggaggtagctataagaagagctgaagaagatattgatttatggacgtttgcgggggccaaacatctagctcttcttacagctcccattccaggtgtcttacatgggtctggtagagggagcagatgataacatcatagatgaagatgttgtctggtgctaggctggtgcgtcgggtctgtgtaggtggtggcctttttaggtgttccttcatggatgttttcatgtattctaagttgcggccaccatagagtgtcctttctttgtatttgtaattggtctatttttggaccctcctttctctcttaatttaatgatacacagctctcctgtgtgttcgagaaaaaaaagatgttgcagaagcgccctgtttggtacaacttttgcttaaatctgtaaagaagctgtaagatatgccaaacaatgtcccccctgtttggtgtgttttttgtgagaaagggaagtgattggccctctaaaaccacttttccgtctcaccaaacaaacaaaagattcctaaactcttaccctccaaccacccattcccttgtaccaattgttactaaccttgattaggcgagataattaccccctcgggtactgtagcatatatataggcagacaagagtatatgggctttatgggccttaacaccccctgtcaaactcaaggcggaagtggaggatttgaagcattgagtttgattagatgaaactgatgttgtgccctagtttgtgcttttgtgaagaaatctacaagctgtaattctgagggcacatagtgaagatcaatggtcttctgatgacaatgagatctagtgaatgatacatcaacaccaatgtgttttgtgagttcacgcttcactggatcatgacaaatttgtatagctccagtgttatcacagtgaagaagcgtaggcgagtcacaagaaacgcctagatcagccaagagccaacgaatccagataatctcagcagtagtagtagccagggctcgaagttctgcttcagtactagatctagacacaacaacttgcttcttagatttccaagcaacaggagatgatccaagaagaatacagtaaccagtgatggagcgacgatctataggatcactggcccaggtagcatcagagtaagcatgaagctgaagtggggaatttgagtcataaaataaacattgtgtttttgtcccccgtaaatatctaagcacacgaagtaagtgcccataatgaactgatgtaggagcagagacaaactgactcaagatgtgtactgcatgagcaatatctggcctggtgacagtaaggtaaactaagctgccaacaagatgtctatatcgagatggatcctccaaaggtgtcccatcagtcggacgaagagataagtgaagatccataggcgtggcaacagtgcgagtatcactaagaccagaacgatcaagaaggtcttgtatatacttggcctgagaaagataaataccattttgagtctgcaaaacctcaatgcccaagaaataactgagtgcccccaagtcagacatttgaaattccttactcagatatgccttcacatgagcaatatggtctggatcatcgcctgtaatcaacatgtcatcaacatatagtaatagtaatgtgcgtcctcgtgaagaaacatgaatgaacaatgcaggatcatgatcactagaatagaaaccacaagccttgatgacagaaacaaatctctcaaaccaagcacgaggagcttgtttaagaccatacaaggctcgacgtagacgacatacatgccctgatggaacctctatcccaagaggtggatgcatatagacttcctcatgtagatcaccatgaagaaaagcatttttgacatccatctgagagatagtccaagaagatgaggctgcaacagcaagtaaggctcggacagtagtcagatgggccacaggtgcaaaagtctcatcatagtcaataccctgagtctgttgaaaacctctagccacaagacgggctttatatcgctcaatagacccatcagatttggttttaaccttgaagacccatttgcacgtgataggtacaacaccagcaggtaacggaacaacatcccatgtacatgtgcgatgaagggcattcaattcatcagtcatagcaagctgccactcaggtataccagaagcctctttataagatgatggttcagcaatgactgcaccagcacggaaaaacccataacgttctggagctgcaatagtgccacggtcacgaagatgatacccctgattaaaaacaacatgagagtcatcattgttagtacaagtatcagcaacaggttcatcatcaggactggccatgggagtagagcgaggacgacgaatgtaagtctgagtgacaggtggtttggaagagtaagacggaggtggtgtggaagttgaaggtggtgtgatgggaatacgaacatttggggtagaggcagtatgcggtgatactgatgaattttcagaaatgggagggaggctcatgaaggaggtagactctgtgctatacaaggaagaatgagtggaagagttgtaaaagaagggtcgattttcattaaagctcatatctcgagaaatacgcatgcgacgagaagatgaatcataacatcgatagcctttatgttcagggctatatccaagaaaaacacactcaacagattgagcagtcaatttagtacgttcacgaggtgataatagaacataacacgtacatccaaaaactcgaaggtggtcatatcgtggaggagttccaaaaagaacttcaccaggtgttttgccagagagtttggatgatggttgtctattgatgaggtaaaccgcagtagaaactgcttcacccaaaaatgtgaagggacaaaagaagatatcaacaaagtgcgagcagtttctataatgtgacgatgtttgcgttcagccacaccattctgtgcatgggcaccagggcaagaaagctgggcaagagtaccctctaaagtcaaaaactggcgaaaattatcagataaatattcaccaccagaatcagaacgaaaggttttaatatgagtggaaaattgagtgtgagtcatgcgagcaaagtttttataaatagaaatcagctcagagcgacgtttcatgaaataaatccaagtgtaacgagaatgatcatcaataaaaatgacatagtatctatatccaccttttgacacaaaaggtgcaggaccccaaatatcagagtgaaccaaatcaaagggttcgacagaagaatcactagtaaaatatggaagttgtatttgttttccaagatgacaacccttacaatgaaaatcagactcaaccgaagtatgacctaagcaacctgactttattagagtagacaatctagatccacacaaatgacctagacgatgatgccactgggcaaaagacgcaacagaagcaagggtagctgaaagcacatgcgctggagatgtagccaaggaaggaagccgcaaagagtccaagatgtagaggcgaggggcagctctacggcgacggccagtcccaatcacttcccctgtgcgaaggtcctgtacaaaacaagatgagtcatcaaatccgacgaagcaattatgatccgtaatttgacctactgaaagaaggtccatagatagctcaggaacaaagaaaatattaggtactgtaaaatgtggatcacaaagagaacccttatgagtaatgtggcatacagtaccatcagctgtctgcactgaagcaccgtctgtgataggagtagtagaggccaactttgactgatcagatgtgacatgaaaggaggctcctgaatcaagtacccaggccgactctgaggtacaagcagacgaagtggcagcaacagcaactgagcctctagtagatggtcctggaccacgaccatgagcagcacgtcgggcacggaaatcagtcaacttctcagggaacttgataaagcaaagctcagatcgatgattggtcttgccacaatgatcacaaggcttaaaaacactcttaggtttctgggcagcagccaacacactgtgagtattactaccagtagaagacagagcattaagacgagtctcttcagccagtaaatcagacaacgccttagccattgtgagagtgtcagaatcctgaagtaaacgagcacgaagagaatcaaactcagcccgaacgcccataacaaatctgtaagtgaagaacttttcaataaacttatgagccggacacggatcaacagtacaagcaggcaccatagatatcaaagcactcatcaggcgatcaaaagctgagtagtactcatcaatactcatatcattttgctcaataacatgtgtctgctgcatgagagtgtgtaatagagcaccactgtcctgaacaaaacgctccttcaaatgagaccagatggctttaacagttttaaatttagacaaactcataatcatagatggtttgacgctgtttaccatagcagccatcactttaccatcattaagctgccatgttttgatatcagcagcattgcgacgatcatccgcaagaacaggtgccacatcagtcaaatgaaagagtaatccatgtcctctgagtgcagtctcaacacagaaagcccactccggataattttggccatcaagagtgatattggccacaatagcatttgtcgccatactgaattcaatgaaaatcagggaacaagagaccgaaaaccaaacaaaccagaggagccgcagctgacagcagcccgagtacgagttggcggaggtcctgagcgcggaagccgagttggacagcggctgctgtcctgatgactctgcccgcaatggcagcgaccggcgcagaagcaggaacggcgcagatccagatctgtggaggcgacagacgacacagaaatcgacggcgcagatctggttctgcagcccttgtggcgtgcagcaggcagacaactgcagaggtacggcaggaatcgacggcgcagatccggttccgcagcccttgcggcgtgcagcagttgcggcgtgcagcaggcagcaactgcagaggtgcggcagggcgcagaacccaggcgcagcaggcaaataggcaacaggtgggcggcggctgaggcagggcgcagtgcggcgcagcaggcaacaggtggaagacgcagcaggcagcaggcgggcggcggatgaggtgcggacggcggacggcacaagagctcagatccgcagctcgcgggactgaaggaaaaccgcgacggcgtggcagaggaagcgggaaccgcgatggcgcggcagaggaggcgggggaactgcgacggcggctgcgggtggcagatggaggccgcccagatccgccgcgacggcggcagaggaagcaggaaaggccggccgcgacggcggctgaggatggaaccgtgacggcggtagggcggacggctggaaggctggccgcgatgggcggacggcgcagcagcgacgcgatggcgccaaagaaaattgatcagggacggattagatgtaaaccctaaccctaacctcctctgataccatgttactaaccttgattaggcgagataattaccccctcgggtactgtagcatatatataggcagacaagagtatatgggctttatgggccttaacaccaattactaaccaaacatgccatacaggttattgaattggctaaggtaaatatcttgaacacactttctgttttttttgtcaactggcaacaaaccttaatggctgtattaagctagttcaggccattttgagtctgaaattttgaagatatgaaaactcaacaatacacccaatgacccaaataagtttgagggccagtggtgcggccatgcaggttaagcctatatcatggtccacatacatggatgcttgaagagttaaatgtttatttgaatgcataattgtgtggcaagtactgagacgacactagaggctgatgctatttactacctggttcctgaaatatttcaaaaagtagtctgcacctgctacttgtgacatgtttgctaagtaaacttgattgtagaagcttatgcaaaacaaataagttgaatgaaactcgtccgaggctctgagttacctccttatattgacttactgttctatgctcttttatccgtgaataaacttctacctggtgcaaggatacctttctgtactaacttccttagcaatccaacatgtttgcttccaagcacaatcttggatcgaatatattcacgatttctttaattttattggaatacactctaataattttttccactggcatgttaggttggtgtcattggaaatttggttcattcatcaccaaagatcaagaaggaggttcttaatgcaggggcactgcaacctgtgattggattattaaggtatggtcatcatagggaagtgcagttttatgaggtgcataaagaactttataattgtatttatttgttaggttctgttgttgagcagccttacaaatgttctaagcatctctaacagattactttcctacgtcccctaaagtctatataagtgatctcctattattagtagtatagctttttcttctctctcccagcagattaccaatacctttaaagtggataggggagagggagtggatagggattttaaatagttacttaaaacttttagatgttggatataggatgagtaatctgttggtgcaaccacaaccccttatattgcatatttttagtattagggatcaggtaagtaatattttggagatgttcaaattttcaggcaatgttttcaagtcgtctagtcgaacctagtcatatagctaccgaacaatcgatcagtcgcgattagtcgtcgactagatcgactaatcgagcctagtcgagctagtcgtccatatgtttctggagatatatagtatacagtaataggatatagtatatacaatttataatacacaataaaacaagcaccaagatggtgacttacctgcgtgtttgttgtccacaactccccattcccatggttattaaagcggtaaaacgataaaaggttaggaactacctttttaacatttaaacgttgaaacttgaaacgtcttttcagacttgagataaaacgacacactagaatatgttcatgctcataagttgagtatttgagttcacaaaacaaatagcataaaaggaaaaaagatcaagttcaaccacacaagtctatgcaactatgcaacatgcaagttacaacttgcatctagcatcagtaaccatcatccaactcatcaatatcaagagcatgagcatccctggaagtctggaacttgatggttgcagctgctagcgacgttggctgctagagctggcgggcggcatgccggcattagaggcggccggtgctgggggagggagaggggatggggcgctcgggtgctggaggaaggaagcgggcgctcggttgctgaaggcggcggtcggcgttggaggaaggaagcgggcgcttgggcgctggaggaggcggtctgcggtcggcgctattggggagtgtcgtggcggtggcggacctggcagcgctagaggagggaggagggggtggaggagaggagggagacacgtggcagtagatggccggagcgggcggcactgaaggagagaagggaggaggttgtcttgacctagttttttgggcctttgtgaggcccaacaaggtaaaaggtcctaaaacgtttaaacgatgccaaattgatgttaaaacacgtttaacggatgttctacgcggtttgtttaaaacgatcggacgttctaccctgtaatcacaatttatcgtttaaacgacgttttaataaccttgcccatttcttctccaaaactccatattcttgctgatttgttgctgaaataacaaaaaaattgaagtaataggtacgaaagtagctgcaaaaataggtgtaaagtcaatagcagcagttagcattaggaaaacacaacagctgtacaacaaacatagccaagaaaagttcactagtgcagcagtctgctagcaacattaatgcagtacaacactacactacaccatctaaaccaagttctcaagtccaataatgcaaaagtagcacaacaaatgaacaaagtagaaaacagctgctaggcccagcaagacagcaacacaagcggtggctgcagctgcgtccttgtgcggtggcggcggcaagacgggcgcccgcctggaacttgcaggcggggggcgacagcggctctgtcttcggctgggggcggtgccgcgtcttcagcggcggcgggtggcggctgcagctgcgtccttgtgcggcggcgggtggcggctgcacccttggtgaaggactgggggagcgcgagcaggtgtctggcgtctaggcttccagcactccaagcttttgtcttgtgcgtgttggccaaccctagaagcccacatttgcagcccacagatgcagcagcccagctccaatagaccatctacaaagacacgtccaatatggtcgtccccagttcaaatcggacgactagttgtgactaatcgtcgactaatcggacgactagttttctgatcgggattactagttttcggatcggactaatcacatcgatgggtctggtcggatgtagtctaccgattaggccgactagtcggacgacttgaaaacattgttttcaggacaccagtgtacatgaaactttaatgattaagccaaccaaaacaatgctaactattatatttgagcataggcttggccattcctagtcattcagacccttaccatttttatattattctagagaaacactcgatcatgggtttgtcttaaatagggggagattgaacctcggttgtacaaaaactcgatgaaaccagttcagtgaggtatccaccattgttttcaagtcggatgacttgctagtcgttctagctgaccgacttggacgattaatcgcgattaatcacgattagtcggacggcttgggcgatttatcgcgattggtccaaaccgacttgaacgattatcacgactatccacatttggtgagggactggaattttgggtgggtggccttcttgttgggaaactgtaccaaccaagctactggttttttcctatcttgtattctagaataccatcttattcaaatgataaggttctttgtcattgttatttgagttttaaagggtgttctatggcttgctgacttgctctacaccggcaactcacctcaagaatatctacatgatgtatgaaacattcatttctttattttttttcagctcatgttgtacagaaagccaaagagaggctgctttgttgctagggcaatttgcttcggccgactcggattgcaaggtgcttaataaatatggagtacttactgtttacaagtcctcagtaaattttgcaaatctactggtagtgaaaactaaagagagaatcgcaccactaatccctgaatttgcatgtttgtctctcccacacccctcaatttgtaacttatattgttagcccttctaactttggacccgttgtggcattggcccaaatcaccgttagctacttagcttaattgatggcgctgatgtggcatcagacatgggctattatactggactgtttgttttcttttatcgtcgcttcctttcctttttcttttccattgatcaatacatcactgacatggatgtgtagatggtgtcataaaatcgattaattatttgaccagtcaacaaaatattttgttttcgtatatgtcattatttatggtgtactcaattggtacccacttcttgtgaacaggcccttattgcaggtaggtattatttatgaatgtgactttcaataccatgtatatttagctaatattacttattgttccatagtttgatggaatttagccacccatattatttatttgtgactggaatgagtatcgcacatgtcttaaggttataggtcaaaacctgtgtcaacatgccatggagagcaggtcccatgtttaatgctcatgtcaacacaatttgttatgttaaggtgatttggcccaatgttgcaaacatacctgaactttagtggggctagcaaagtaatttgcaagttgcgagaagttgctgagagtgagacaacggcacaactttaagggctagtggtacaacctctctttttcaaaagtactggtgatttacatatgtaacatttaatttatgtgcactgtatattaggatagaggtgaaataattctggccaatcacattaggattgacagattataattgctgggactgtctggcgccttttgacatgatgcctcatagggcctacatgctgctggccagtccatgcatgatctcgcttattctccttgttgctcttttctaactacgcctctgcatttcttattcttcgtctgatctggctgccacaatcacgaatccatattggtgtgcatatggcagtctctgcaactgtcatatctggtgctgggaccacttatcttctttatctagtatatcctcacacggagtcatggtctcatggacatgttctccaaatacggtgggttcatgttcctggtgtctgcacgtgccaagtccccagatctgcccttacctgcattgcgtctatatcactgtgcttggcaacaacacaccctgggttctatgctcaagctgaacctagctcgtctaccacatgcatttcaattgctccaccactcctggcttacaccacaccctaagatttaagtttttttagaagttggcttctttgttgcagaggtatgttttgctttatttttttagatgtttccttgggaggtgggagggaggacagccataggaaccacttacggtttgttctttgagtggagggatgcagaaggtagaaaaagaatgaactcaacaattgaatataatgttcagtataaggaaatctagaatgataaatctcattatctcaaggaatgacacaaaagcaaagagacataagatgttttctccagttaattcatttctgaacttgatagataatatatatgttcgtttacaggtccatattgtgcaaaggggtgcagtctgtccactaattgaaatgctacagtcggctgatgtccaactccgggagatgtctgcttttgcacttggcaggcttgcccaggtttaattttcatttttaatatagcatcttttttaatgtttataaggtactttactgttctctactatagagaatcagtgtaggcagtgaaataaaaacaccacagtatttttgttgctctcttacattagtaaatcagttcccttgctcttctgttgatgtgaactacatgtggggactgcggatgcaaagatcataatatgtatagggcaaaaccatagttagtttgctggcaccacttaccttccttatccagtccatcctagacatggacatattttttaaatatgctggcttcatgttaccggtgtctgcatgtgccaagtcccttgctccgcccttacctccattgcatcttcaccactgtgattgtcaacgacaccataggtgctgctgtgttcgaggtacctctggaggcaccacacacattccaattgctccaccaagaagttacgtagctagtagctactcttcatataggaaaatgttcaagagcccatatgttgtctgtacataattctgccttttgtttttgagttaaatgcaccataggttcgttaacttaatgctgggttgtcagttaggtccatcaactctaaaagttgattttcgaatccataaacttgaaagtggttcacctcaggtccataccccttcgcccttagaatctacttctgggtctaacaacatcaaaatcttttagtcccaagcaagttagggtagactagagttgaaacccgaccaaaaccacaagtcaagtttacgccccaacagttttttttcgggtttcatctccattagaatggcttggtttaacattcgctcgccaagcctatcacaaccctctttctttaccaggcttgggacctgttatgttgagacaacataggcaaagtttaaaaaaatagttctacttctgggtccataaacttttaaagtggttcaccataggtctatactcctttgtttggcccttagatctgacacggtatgcgggtcagcagccagcatggcatgcttgccaagttagatctaagggccaaacaaaggggtatggacctgtggtgaaccacttaaaagtttttggacccggaagttgaatctaagggccaaatgaaagggtatggacttgcggtgaaccacttataaagtttatggacccacaaatcaacttttagagttgatggacctaacagaaaccctgctaagttaatggacctatagtgcatttaactcttctattttgtaagggaattttgtcttttttttttccctaccatatgctctgatcgctaaccacacctatcttagccaatcttctgaacctttgtaattcctaattgctaggtgacaccgtcctggcttgatccctagcttagttatcctttctagcccaacgataggtgcttggagtgttccctgtgacttttcccagctaatcatcgattaggtgctaggagttggtctactgtttgactattaaagacccactttgtcagtggtgcattttagcagagcgataatatttctgacaattgcaaccaaccaaacttcatggcatataatttccttgtgagattgtttggctagttttatacagagtggaatgtggagtgaaccacttaaaaagttgaccctgatcctcacctgagagattatggacccaattgagtatctgggaaaagttaaatgatctagcacattttgctctttcatatcatataatgtaaggggaaatcccattcgtttttccttttatttattggttagtggggttgttctttctttcctttttgcttagttgcaactcgtaatctaatctgaagtcttttctcaggacacacataaccaagcaggtattgcatataatggtggcttggtgcctttgttaaaacttcttgactcagaaaatggatctctgcaacataatgctgcatttgccctttatggagttgcagataatgaggtaatatacgatcttttttccacaaggtttgatatctctctcaaatctccctttttttactattggtcactccatgttcctttgtaacgggatcaactcattttttttaacaaaatgctgatcttatatttcttcattatttctgaagcaaatcactgttctttcttataggactatgtatctgacttcattaaagtaggaggtgtccaaaagttacaagatggagaatttattgtccaggtacattggccttcattgtatattgtgtcactctattgtgaatgctttttattaagctattattgttttcaggcaacaaaggactgtgtggcaaaaacattgaagaggttagaggagaagataaatggacgagtaagtttgctcgcaaggtttctgtatttagttgtttgcgatgtgcttgatagtatttatgaagattgttcccatgtcatggtttacaggtgttgaaacacttgctttatttgatgcgagtaggagagaaatctgtgcaaaggcgtgttgctctagctcttgcacacctttgtgcccctgaagatcaaagttcagtttttattgataataatggtaaacaattttgcaagcgctgaaaattgtacattttcatttccattctactgtatggtgttctttatgaatttaaattctgggtcatccaggtctcgacttgcttcttgatcttcttatttccatgagttcaaaacatcaacaagatggctcagcagcattatacaaattggccaacaaagctgcagcactttctcccatggatgctgcccctccatctccaacacctcaggcatgcaaaagaattattaaattcaaatttactttgtattatgtatgctgtttgagttccagtgactttatgagctgactgtggtatggttaaagtagtatcacaatgacacgatcttcagtgtgctaggatgtgcatgcaattattttgattaatcattgtggaatggtgctttggttcaataaggtatataagggcctaaattagtctgttgtagtccaacctgttgtgaataatagtgtgttcaacctgctggaggataataaatgttcttctggctttccatgaaaggtaaatgttgaactgagcttgctgcttgcaaaacttaatctgtctcatctggataaatgcctactctgtgatcaagaggaggaaacagtccagcacatccttataacctgtctttgcaagacagttttggcacaggttgttgattgcacttaacttggtggcggagagctagcaaaagagttagcaaagatcaaagaagaggggttaacactctcatcatcttggatgcatggatgctctgtaagcagagaaatgcatgtgtgtttgagggagactctcagtgtccgtccctacttacacctagaaacttgaagttagaagctcgtctatggacgctttctggggcttccaagctacagggtcttgggctaagtcggctggaaatctaggctaccttaattttctttgctgtaactcacttaccttggtcctagtaagagttgagcttgtttggaccacatttcttttccctataatacaaagatacacagctctcctacatgttcaataaaaaatatcatgtcaatatttttgtactgtttggcattgtgttgaaaattgttttcagaatttagctatcattgacattgtaacaaggtttccaaacactgcctgtattttgctatcctaaattaagtcattgtgactttgtcggatttttgcatccaattggtctggtaatggttgcggcactggcaattgttactgaatgtatatttcattgtaggtttatcttggtgagcaatacgtgaatagttcaacactttcagacgttactttcttggtagaaggttggtactatttcatgaccctgatttcatcagtataattcttttcaatcgtgtcccagataatcttaatcccttctacaggaaagcgattttatgcacacagaattgctttgcttgcttcttctgatgcatttcgtgcaatgtttgatggcgggtacagggtgagttttgacttgccacaacataatgtgcttttgctggttatagtctataggtgtaacctttttttattctagtcctataatataaggcgcgtgtgttatctttagacatgcgtacattgatgtagtagtataaagagaattaaatatatttttcagtctttgaactagaggtggttatgccttatatacttatatactgggactgagggagtatatttctgcatacaatatgttagttttgatcaaaccttgaatctcatgtctaattgaaagcatttcttaaccaggaaaaggatgcaagggacattgaaattcctaatatcagatgggacgtctttgaactcatgatgaggttagtaagtcattgacctcccttctcgtttgaccacagttctctttctgttgatgaatctgcaactaattttccccttttcttttttgtgccactgtatgctggattaaagtctgaaatcatctttggttttgcagatttatctatacagggtcagttcaggttaccagtgaaattgcacaggatcttcttagagctggtgatcagtatctcttagaaggcctcaaacgcctatgtgaatatactattgcgaaggtgattagaaaagttactatctattccttgtttaaaccgcaggtttgatattaatttaaatgccattatgtgcctttgtaggatgtgaatctagataacgtatctgacatgtatgacttgtccgaagcctttcatgccgtgtctctgagacatacgtgcatcttgtacattctggaacattttaacaagatctgcaccagagccgggtaccttctcttgctaattacttttgatctgaaagcagtgcgatttcaagtgactcaatttttaacacgcaatcttgccatgcagttctgcacagctgatccagcgtgttattccagagctccgcaatttcctaaccaaggcactgagttcatcaagaagcccaagtacaaccgacgacaggaacttgcagacttgattttgagtcccaattcattgacactgacaccgtcatctgaccaaagttgctggacatcctgtacagtgaagtttctggcgctgcgcatttgatggcatctgttgtggtacatggtggccggctcctcaaaattaacatcagcagcttaacaaacttttgtaagatttagtggaggatatgggtaaagagaacccgcgtcttagtcatgcctcgaccagcttacactgggataggctgtagttgtgaatggtcttggccgtaattcgtcggtctctgctttgtttctgagttgtgtttgtttcaagttcacagttcagtgtatgcctgcatatgtttaaagtatgaagcttgagcaagttagaaattagcccctgtagtgataaagctgtctgtgtagatccaccgattggagttaccgaaacaactatgtaacatcatagatgacattagatgcatgataattgctggtaaagcttggtcaaaatatgaggtagaaccactgatcatcacttaaatagattgcgaagca

SEQ ID NO: 114 - protein, 724 aa, Zea mays
MEAEQQKQQRPRQRPRRKGQKRKLEDEASAATAAAASSLGSAGADDDNEEEDGSAGTPEICRHSHAALAREVRAQVDVLIRCASSWRHADRAAAKRATHVLAELAKNEEVVNMIVEGGAVAALVCHLEEPAVAAQTQEEQQLRPFELEPEHQQFIVDAGALPPLVKLLKRQRSTTNSRMVNSVIKRAADAITNLAHENSNIKTRVRMEGGIPPLVELLESQDLKVQRAAAGALRTLAFKNDENKTQIVQCNALPTLILMLRSEDAAIHYEAVGVIGNLVHSSPNIKKEVLNAGALQPVIGLLSSCCTESQREAALLLGQFASADSDCKVHIVQRGAVRPLIEMLQSADVQLREMSAFALGRLAQDTHNQAGIAYNGGLVPLFKLLDSKNGSLQHNAAFALYGVADNEDYVSDFIKVGGVQKLQDGEFIVQATKDCVAKTLKRLEEKINGRVLKHLLYLMRVGEQSVQRRVALALAHLCAPEDQRAIFIDNNGLDLLLDLLISMSPKHQQDGSAALYKLANKAAALSPMDAAPPSPTPQVYLGEQYVNSSTLSDVTFLVEGKRFYAHRIALLASSDAFRAMFDGGYREKDARDIEIPNIRWEVFELMMRFIYTGSVQINSEISQDLLRAADQYLLEGLKRLCEYTIAKDVNLDNVSDMYDLSEAFHAVSLRHTCILYILEHFNKICTRAGSAQLIQRVIPEIRNFLTKALNSSRSPSPSDRNSQT

SEQ ID NO: 115 - protein, 748 aa, Zea mays
MEAEQQKQQPQRPRRKGLKRKLEDEASAAVAAAATSAAASAAAASLGSAGADDDNEEEDGSAGTPEICCRHSHAALAREVRAQVDALVRCASSWRHADRAAAKRATHVLAELAKNEEVVNVIVEGGAVAALVCHLEEPAVAAPTQEEQQLRPFEHEVEKGAAFALGLLAVKPEHQQLVVDAGALPPLVKLLKRQKNTTNSRVVNSVIKRAADAITNLAHENSNIKTSVRMEGGIPPLVQLLESQDLKVQRAAAGALRTLAFKNDENKTQIVQCNALPTLILMLRSEDAAIHYEAVGVIGNLVHSSPKIKKEVLNAGALQPVIGLLSSCCTESQREAALLLGQFASADSDCKVHIVQRGAVCPLIEMLQSADVQLREMSAFALGRLAQDTHNQAGIAYNGGLVPLLKLLDSENGSLQHNAAFALYGVADNEDYVSDFIKVGGVQKLQDGEFIVQATKDCVAKTLKRLEEKINGRVLKHLLYLMRVGEKSVQRRVALALAHLCAPEDQSSVFIDNNGLDLLLDLLISMSSKHQQDGSAALYKLANKAAALSPMDAAPPSPTPQVYLGEQYVNSSTLSDVTFLVEGKRFYAHRIALLASSDAFRAMFDGGYREKDARDIEIPNIRWDVFELMMRFIYTGSVQVTSEIAQDLLRAGDQYLLEGLKRLCEYTIAKDVNLDNVSDMYDLSEAFHAVSLRHTCILYILEHFNKICTRAGSAQLIQRVIPELRNFLTKALSSSRSPSTTDDRNLQT

SEQ ID NO: 116 - DNA, 9071 bp, Oryza sativa
  source 1..9071: mol_type = genomic DNA
aacccccctctaatggaggcggagcagcagcagcagccgccgcatcgcccgcgccgcaaggggcagaagaggaagttggaggacgaggccgcggcctccgcctcggccgcggcggcggcggcggcggccgccgccgccgccgccaccgcaaccccgtcgtcgctcgggagcgccggcgcagacgacgacaacgaggaggaggaggacggctcggccgggccggagatctgctgccgccactcccaggcggcgctggcccgcgaggtccgcacgcaggtcgacgccctccaccggtgcttctcctggcgccacgccgaccgcgccgccgccaagcgcgccacccacgtcctcgccgagctcgccaaaaacggtaaacgctccccccaccaccccgaaccctcgccgcaccgcaccgcgccgcgccgatccgtggttttccgcgccaggcttccgggcccgttcagctgaggcggatctggatgttgtgtttttcttcgcagaggaggttgtgaacgtgatcgtagagggcggcgccgtgcccgccctggtgtgccacctgaaggagccgcccgcggtggcggtgttgcaggaggagcagcagcctcggccgttcgagcacgaggtcgagaagggggctgccttcgctctcggcctcctagcagtaaaggttccctgttcgtgccgtactagtttttattcccatttcattgcaattattggtatttctttctcacctgagttatccaaatgtatcattccataataaaattaagagtagctttggatatgccatcgtctgccaaaatttaacccgagaacaactactgaacaagatagtaacacctaggaattcgtttagtagtttttatgtatacatgttccctatctccctttaagtgattcatggaaactggtgtttttgagcatgacctcagtaatatgtttttgatctaagttacttttgagaaatttagtcattaattacttaatgtgtttgcataacagcctgaacatcaacaacttatagttgacgccggtgccttaccactgctggtgaatcttctaaaaaggcacaaaaatgctacaaacttgcgggcagttaacagtgttatcaggagagcagctgatgcaatcaccaatctagctcatgaaaatagcaacatcaaaacttgtgtcaggtgttttttctatattttgttgatagtctgatgctccttcaactagggaactttttattgcttaatgatgtttttatattggtttactgcagaattgaaggcggaattccacctcttgttgaattgctagaatcacaggatctcaaggtgcagagagcagctgcaggggccttgcggacgctggctttcaaaaacgatgaaaacaaaagtcaggtgagatatcaaaatttcaaaataacgaggccaacattatgatatattttaacaccataatggtgcagttacatccatatttactcatactattttgtgtaattttccccttaatgcagattgttgattgcaatgcgttgccaactttgatattaatgcttcgatcagaggatgctgcgattcactacgaagcagtaagacactaggaatttattttttgtgaattatgaaccgcacttctctgggaactcttttatgttaaggttgatgctgactgatatgcattgattgattatgcggttagtgttgcaaattttctagttatcagcaatcttgagcagcagttatcctaatgtgttctagaacataaatttcgaagtgctcatccttcatggccagggccacaaaaatcactttgtgttctcccagaacaagcaaaccctgttttcttgtttactgcaacaatttttatttaaagttctttttgttgaattcgattcaggttttctactatatcggcctccaaacaacatatggcaacaaataacaacaaaatcaatcaactactccaaaataacataggggaactggcagctacagtgctactacagtcatggggaatttgtaacaagcgtgtgaccattattttgaaccctctctacaacttaacattgaatatagaactacgggtaatgtgttacatagagaaccatggactactaaacttgattgcttgaaatgaacctagtgcgctaacatattaaagagtataaacttgcatgacttggacaaagcataaacaagcatgctgaaaagtgaaaacttagcatgaaattggtcaaccgagccaattaggtccatccgcaggtttaatgaaggtaaaaatgtcatgttaggctgttggaccgataaaacaaatttaatacagaggtattgatgcttaagatccatatcatagttaatcatgtcagttttctacttttctggcacttgactggaggatgggcatatctaactaactggttctgtaagcaatttgaggggacctgccaatctaaaattgaaattcaagagcttttgttacagagatcaacaaatttgatggcctattgacctattccactgttttagaattattagtagccaaatacccgtgcacagtaacgatttagaataatttaccagaaattctaaacttgaaaaaaaaatcagttgaacatcaatctccaaataattcgatcacaaaccacatgtgcaaataatataattatcgagggaatattcttcaaccagtaaaaacatatatgtatgtatctatgcagagcacccacccgttgtcctggtgtgggatggcagagccaccaccactactaccatcattagcttcttttgtaatagtagagataagcatggtgaaaaaacatcaattactgcaaacagcctaacaatgctagttatacacttcattgtcttacatagtaacttgatcctgtgatatccacatagaacaagtaaatcgcatgattatggtcttgacactgactcttctccatcaagtatttctatcagtactatgtatattcatatagttatacacttcattgtcttacataggagtaacttgatcctgtgatatccacatagaacaagtaaattgcatgattatggtctcgacacttcctctactcttctccatcaagtatttctatcagtattatgtatattcatatcattttggcttttttgcaccttgcaaggcttcctgtctgtatgaagtcttctattgatacaacaagcaagttattgaactacacttatgtactatctttttataatgcatgccaataagtactctgttcacatgtcaggttggtgtcattggaaacttggttcattcatccccaaatatcaagaaagaggttctcaatgcaggggccctgcaacctgtaattgggttattaaggtatgatcgtcatatgcagtttaggatcatatttttaaactatctttgaaaataattgaatgcattagaaatattgtatgtatttgttgaaccctattgctgatgactcaaatgtaatatatttttttagctcagcatgagaacttttaacatttccaattactatggtagtaactgcttgcttcatggtacactccatacaattactttgaattgtacgcatgtttctgaatgatagttagcttacacctttactgctttaaattgagaatattaagttggctattatcttatggctgttcattttgcagttcctgttgtacggagagtcaaagagaggctgctttgttgctagggcagtttgcttcggctgattctgattgcaaggtacttgcttgttcttcgttcatttttagctggcttgtttctaattcttttctgatgagttaatgcagtggaggagcaaaaaacaagcttaaataagtttcccttgatataatattctggtgtgaaagagatgactgttctgttatgttttgctacttgctaaatattttatgtgcacaatagaaggtttaagcatggaattctagaatatatgaatgaaaagaagctgatgttttcttaccttttcgttgtttaacatcctgtgcatgtgtattccctacaggtccatattgtgcaaagaggtgcagtccgtccgctgattgaaatgctacagtcagctgatgtccaacttagagaaatgtctgcttttgcccttgggaggcttgcccaggtttgttagcttgttttactgtgtgtagtttagggacaaaacactgaaaaagaacaacactgacatgccacttagtaactttgctcctcttaattctaacaatggcagctgtatgttaggacacaattataacaataattttgaagaaattataatgagtcttcactcttgaatgaatagatataggctccttaccgtgtgttcttttgttattcgtcggcacagtagtgacttaacaacagtttaggtataatatatctgaatagctaaagtatcccagctcattctccatacaggcaaacttttcatactaacttttgagcacctgagagtcgtgcctttcaaatgttcattgcgcagagtatccactatcctgtgaagagtaacactggatattttctagacctgaatctgtgcatgtgggaatggtcctatagtgagggcaagatcccatttggtcattggctgattcttgcatagtaatgacttgaagtcacccatgcaaatacatctgtagaaccgagagaataatttctgtcacttgattatttgattatatttatgcaagggacaatccacatgcaatcatactaacatcttaggatggtgatactaacatattttggtctttgtaagccaaaagctccgcatatacccagatatcgcttcatgcgtaatgcaccagttgaaacatgtcaaaatgatcatcgatataacatgttggatatattattcttttgcctatcaattctactttgctctcagcagagcacattctgtatgttagtgatgaagtcagatatctgagacacagacctagttattttcttctcaaaaccctaggctgtaaagatattaaagaacttctataacatgcaccggtcaattcacagagaagttcatttgtttcccaggacacacataaccaagcaggcattgcatataatggtggtttggtgcctctactaaagcttctagactcaaaaaatggatctctgcaacataatgctgcatttgccctttacggagttgctgacaacgaggtaaataatgattattcaagcaaatggtaacccatttgtggatagcttgttttccactagtaggctaatgattcgatttcggaaaaggaaatgatctcttgctttattttttttttcaaaataaatgactatactcttcttattgtaggactatgtgtccgacttcattaaagttggaggtgtacaaaagttgcaagatggagaatttatcgtgcaggtatgccagccatcatattattgttggattactttcaatgtaacttgcaagtgagtttaattacgtaattttaaatttcaggccacaaaggattgtgtagctaagacccttaagaggttagaggagaagataaatggacgagtaagctgtgctcagtgcccaccagattttgcttttccatcgccacattctagcatttagcttattttgttcctgtatgaccgcaggtgttaaaacacttgctttatatgatgagagtaggagaaaaatctgtgcagaggcgggttgctctggccctggcacacctctgtgcgcctgaagatcaaagaacaatttttattgataataatggtatgagcaatttgaaatgcaccaaaatgtgctcctttgtattacttttgtgtaatgtttaccattgattaagttattaaattaattcaggccttgagttgcttcttgatcttctggtttcggtgagcctgaagcatcagctagatggttcagtagcactatacaaattggccaacaaagctgcagcactttctcccatggatgctgcacctccatctccaacaccacaggtagagaattggttcttaattcaacccaacctttccttgtttatgccaaaggctttatgagttgattgtggtgtgctatgtaaaaggttttcaatgtgatatggactgaactacgatgtggtaatgcccatgcattgattttattttgtataatcaatgcattaaaagggtttttttgttagaaataaacaaaacagtacatgtttaggggaaatttgtgtaatgcaacaaaactagctaattgttggctgacaatcttgtttgattagtattttgacaggaaattggaggtggatgtataatagctgtaaataaatatgcaacacagattcttggcttcttggttgtgcgaattatgtgatagctgcggaaaattgttgcaaaatattaactaaaggaacaatcctgtacattcatcgccaatatttcattaagaagcttagggttactaggatgtgaatattaatagctaagtttaatgctagttttaagttgaaaaaagaaacattagtttacataacttataacatactgtaacatttcagttgaaccacccaacagtttttcaaacttgtactatcttaagttaattttggagcagtctatgataatagttttttaagacctatgtgttatttgactcgtcagtagcggtaacattgcctttaatcatgttcttgttgccttacctcgaaatttaaaagtttttatcatgatattggtggtacaactgttgccatgaaattctagaagtatgattgactgatattccccatggctcgtgtaaactaaataatagaaacatctgtcataaatactgatataaatggtgcttcatctcgcaaattgcacaacagcctcgtcacactttcacacttatttatatacgtttcatcctagtcaacactatgcatgatttcccattcatgtcttttaagatgtgtgaccttcaggccatctgctttctgagcaaaccaagcatttatttcctttgttaggcttttgtaggacaaaacttttaggaacttcgtcagacatgaccaagttgttgcaagatttgaattcactcaggcagtatgtatgcatctgtgcatttctatggattatttttatcctcagccttcagagcatagcgcacatagaattcagatatactgccatctgaatttatatgccggatagtctgttcctaattagcagtcagtcctattaataaggtgttatctcagtaaaacctagtttgtgcaatgctggattcgaatatatcatttggagcaattggtccatcaacagtgctggcaatccctgatacttaatgtattttcttcattgtaggtttatcttggtgagcaatatgtgaacagttcgacactttcagatgttaccttcttggtggaaggttggtattttatctgtggacccagttgtcaccagaaagtcactttagatacttcgatcttttccatagaatccatgtaaatcatattcctgttgtctccaggaaagcgcttttatgcacatagaattgcattacttgcttcttcggatgcatttcgtgcaatgtttgatggcggatatagggtgagtcttgtgtagcatttcttttttcgtttggtacatgtggatttgtttcttagtgaaacaattcttgttgaggtatattttttcattttttaaagaacctcaatgtgtcttgactcgaatactatttttcttaaccaggaaaaggacgctagagacatagaaattccaaatatcagatggaatgtgtttgaactcatgatgaggtaagtcagctttgagttctcttcctccttgaccatggacgctttgcttctgtgcacatatctgtaattgttattattcttttctggtttgtgggcaaatgcctgctaaactagagtctgaatatcctacttggtatatgcagatttatctatacaggttcagtggaagtaactagcgatatctctcaggatcttcttagagctgctgatcagtatctattagaaggcctcaaacgtctgtgtgaatatacaattgcgcaggtaattaggattgttacctgtatgctatgctcaaaatgctggcttggtcttatttaatatatctgccttgcaggatgtgaatgtagacaacgtttctgacatgtatgacctatctgaagcttttcatgcaatgtcactcagacatacatgtgtcctatttatcttggagcagtttgaaaagatttgcgtcaaatctgggtacacttcctcacctagtgtcctgttcctaggtccaaatgtttgtgttatgtaactcattttgggtaacagaaatcatttgccatgccattttgcaatgcaggtcaagccagctgatccagcgtgtcatcccagagcttcgcaacttcttcgctaaggcgctaaggccaagccacaggaatgcgcagccatgagtccgtgccccttccacaatccttgacaccacccacacatctgacagtcgcttcgggagatcttgtacagctaaaagtttctttttctggcgttggacattggcattcgatggcaccaacaacattgtaacatccttttattcgattaaaacagagcccaaatcatggtaagagcatatggcttagccagccatgtctcggaccagcctaggctgggataggtttacttcgtttcgccttggcatagtcaccgagtttagggccactttcccagtccagagctccgtgtatgcccgtctctttgatgatgcagaggataagatcgatctgtgtattagtgctgtagttgcaatcagtttcgtctccttcgtgttgtttaacaatgcagaaatgctaatcagattggcgttttctcccaacttgtccctcgtcatggtccatgtatatactgctatgcagtagatgcatatggattgtattgcggtccagcctgacgtcggtagacggggacaaatacggtggcaggcgccgccatctcgtcagcggcttaatcggttgtctttgtcccactggatattcggcggaagaatagccggatttatttttctgccctgctctaataatttctgtatctctatttaaatttgtttgcttctgt

SEQ ID NO: 117 - protein, 745 aa, Oryza sativa
MEAEQQQQPPHRPRRKGQKRKLEDEAAASASAAAAAAAAAAAAATATPSSLGSAGADDDNEEEEDGSAGPEICCRHSQAALAREVRTQVDALHRCFSWRHADRAAAKRATHVLAELAKNEEVVNVIVEGGAVPALVCHLKEPPAVAVLQEEQQPRPFEHEVEKGAAFALGLLAVKPEHQQLIVDAGALPLLVNLLKRHKNATNLRAVNSVIRRAADAITNLAHENSNIKTCVRIEGGIPPLVELLESQDLKVQRAAAGALRTLAFKNDENKSQIVDCNALPTLILMLRSEDAAIHYEAVGVIGNLVHSSPNIKKEVLNAGALQPVIGLLSSCCTESQREAALLLGQFASADSDCKVHIVQRGAVRPLIEMLQSADVQLREMSAFALGRLAQDTHNQAGIAYNGGLVPLLKLLDSKNGSLQHNAAFALYGVADNEDYVSDFIKVGGVQKLQDGEFIVQATKDCVAKTLKRLEEKINGRVLKHLLYMMRVGEKSVQRRVALALAHLCAPEDQRTIFIDNNGLELLLDLLVSVSLKHQLDGSVALYKLANKAAALSPMDAAPPSPTPQVYLGEQYVNSSTLSDVTFLVEGKRFYAHRIALLASSDAFRAMFDGGYREKDARDIEIPNIRWNVFELMMRFIYTGSVEVTSDISQDLLRAADQYLLEGLKRLCEYTIAQDVNVDNVSDMYDLSEAFHAMSLRHTCVLFILEQFEKICVKSGSSQLIQRVIPELRNFFAKALRPSHRNAQP

SEQ ID NO: 118 - DNA, 9777 bp, Triticum aestivum
  source 1..9777: mol_type = genomic DNA
gaacgcggaataaaatccctatcgcgctggggcgcgcatactctttgcttctgcccttccctcctcctccgcctccgacaagttccccaccttcatcgccgtcgacccgctctaatggaggcggagcagcagaagccgcagcgcccgcggcgcaaggcgcagaagcgcaggattgacgacgaggccgccgcctcggccgccgccgccgccgccgccgtcttgtcgccgctcggcagcgccgatgccgacgacgacaacgaggacgacgagggctccgtcggccccgagatctgctgccgccagtcccaggtggcggtcgcccgcgaggtccgcacgcaggtcgacgccctccaccactgcttctcctggcgccacgccgaccgcgccaccgctaagcgcgccaccagcgtcctcgcggagctcgcgaaaaacggtaatcccccaaccctacgcccaccgtgccgatccgtactcttccccacccgtccaggcgccgttactgaggcggatctgcttgctgcttttgccgcagaggagatggtgaacgtaatcgtagagggcggcgccgtgccggcgttggtgtgccacctgaaggtgccccatatggcggcggcggtggaggaggagcagcagccgcggccgttcgagcacgaggtcgagaagggggctgccttcgctctcgggctcctagctgtaaaggttaattcgattagttttcctctttgcactttagctgagattttgcttacattccattgcaattgcttgaattgttcttataatcccaattttctgggccgtggccggctcatacatgaaacatcccatttcgtagcaaaatgcaagagagagaaaaataccattctcttcccttcccctaatctcttgtttatctgtaaatgtaacttcatacgccttcataagaatctaggtatacttgggttcaagcagaataggtttcaaccttgcctagttctctttaggcaatccataaatattattgttaacttttcttcaacatgactacttcattgttatgattttagctatgttactgtcagaatttagtcatttattactttttgtgttggtttaccagcctgaacatcaacaacttatagttgatgctggtgccctacccctgctggtgagtctcctaagaaggcataaaaatgctacaaattcgagggcagttaacagccttatcagaagagcagctgatgcaattaccaaccttgctcatgagaatagcaacatcaaaacttgtatcaggttttgttctatccactgcccactagccaatgctgcgtttccatgaaagttttctgtgcttgctgatggttttgttccactgcagaattgaaggcggaatcccacctctcgttgaattgctagaatcacaggatattaaggtgcagagggcagctgcaggggccttgaggactttggcgtttaaaaatgatgaaaacaaaaccctggtaagaatataagaaagtttaaattattgaaaccaacattaatgttagattttaacatcagactttcatccacattcacccatgtatattatttcctcacttctagatgttaaatcttccccttaactccttaatgcagatcgttgattgcaatgcattgccaacattaatcttaatgctgcggtcagaggatgctgcaattcactatgaagcagtaagatactgaatattcatatatgttcatcaaatacacttctttggttgaacccctctccatttttagtgcggcacttgtcatgtactccctccgtccgaaaatacttgtcggaggaatggatgcatctagacatattttagttctagatacattcgtttttatgcatttctgcgacaagtatttccggacggagggagtatctattacaggaaaacattgttctggttttgaaccttgccatttctcttgtttttctacaatcatgaataacagttatcctaaggcctcatggaatgtaaacttcaaaatgtattgtcttgattggcttaatggtgaaccgtagtactatatattgcttgggaaacttccaggtgaaagtttttgttcaagttgcaatgtaacttgggttagttggcacaagtggcacttaccttaacttatcattatactccatttacattacgagcaatgcaattatggtgcactatattgatattgatgtgcattagaacccaattccttaagtgtattgaactgttgtctcttattattattaaatattaaataaaggatagagtaattcctttgtctagagattctagtgctgcaataagggttcatattgtcattatgttaataaaaagtggttcagtggcatgttagcaaatcggtcgattacgaaaactagactttctgtctcttggacttcttattcttttgcttaggttcagccgaggtagtggacaaacagtggggaagaaatatggcgagaaatttcttgtgattgtgagcaagtagaattgcttgacttcaacaaacaaatggaagttctatctatcaatatctatggtcttgaccgtcatggttaacctccttccatattactccctacccccagggaagttgaatccccgctgcctccttgaaagagagatgccctgaaccactagacgatagcagtgaaaaattgagtgtacgcctaggcacgctcaagtgatgagcggaggcctaccgctttgcttttgtggtaagtggtgaaacaaagcgctcggacgcctagggttagacaaaggagggcaggggtgagagaaacagaggagagcaagacgaccttgcgccagggttagacaaaggagggcaggggtgagagaaacagagagcaagacgaccttgcgctgcaaggtgtggggctttattcctcggtctcaccacccatcttcttccccgacctagcgccgctggatcttgagctccccgcccccaaccttgccaccagtcctcccccctcttccccaatctcaagctcctccttgtctaggctggagcctggtgatttctctccaacctcaccgctgccagcttgcttcccttccctgagctcgagctcctcctcgtctcttcttccccaacatgcttgcgattttaggcttaatacatgacttacagaaagcttaatatatgtcctgcagctttatatgtttggtgcacacaacttactttttggagtgttacaaaagaaaagctattccacatcagccaattagaaatttggagcattaacacctttaacttaccaatggagttactaatcctgtggaatttatacaaagaaaatgatctgactatttgcttctatcagttacatatagatttatacttttgccaaatgcaaaggctgtcctcataaggttctcagcatacaacatatatcgtgacaattttgcatgaaatcaccctagttttatacttttgccacatgcaaaggctgtcctcataaaccagccatatgtatgatattgtttttgctgtgcatgccagtaagtactaaatacactctcttggcgtggcaggttggtgtcattggaaatttggtccattcatccccaaatatcaagaaagaggttcttaatgcgggggccttgcaacctgtaattgggctattaaggtatgatgatcatcatatgcagcttatgataattgttttaattgtatctgttaataattaaatgcatataacttactgtatttatttgttgagttctgctagagtactgctggaaattcaaattctatgtactttacttttagcgtacatgagcaatacacactcgattactgattacaccattgtgcatgtgttcctggatgcagattaattttgttgctttaaggtcaaaacaatatgtgattgtaatgatataatcttatgagatcttcaagtgtaagcttgcgtgtagcaaattatcttctaacccagattccatatccatatccatattgtaacacgagaagcggttttattgtagtcccaatcttagtatatgaaggcatggtattaccctgagtctgctctctagcttaaagaacctgtgtttcatcttttcttttgcagttcctgctgtacggaaagccaaagagaagctgctttgttgctagggcagtttgcttcggccgactctgagtgcaaggtgcttaaggatgcttcatttgttgttagctccatatttatttttatgatgagtgatgaagtggaagagtaaaaaataaaatgaagtacttttttcctatatactccctccgttcctaaatataagtctttttagagattccaatatagactacatacggagcaaaatgagtgaatctacactccaaaccacgtctatatgcatccgtatgtagtccatattgaaatctctaaaaagacttatattttggaacggagggagtaatactcgtgctacatatcattgattgattatgtctacctacttacttaatatgttgtttcgtacgataaagagttagccatggtgaatcaaaagagtacaaaattgttttttgagctatcctctctaaatatgcatgtatggggtttggcaggtccatattgtgcaacggggggcagtccgaccactaattgacatgctacagtcagctgatttccaactcagggagatgtcagcctttgcccttgggaggcttgcacaggttatatttctctctatactccccttgcacacaacaatatcaatctgattgcttatgtttgtcagcgggttgtactgcatgtattttagggaggtattgtagcagtgaaagagaaacaacaatgacaatccttactccccttcataaaatcacctgacatagtgacagagcactttctcaattttgttgcttccctttttctctatgttgattttacatcgggatgcggtgccccctcttagaaggattgacatgagagtgaccacaggttatgtttaatgtaccatcaataattgaagccatgcagctcattctctttatatgtgttaaatatccagactaactgttgagcatctgcctctcaaatgatgtctgtttagatttgtaccttttgtttgtgtatgcttcttcactgtatccattgtcctgcgacaagtaatcgtaacccagcatagtttagcacatctcttgaacatgcgcatttctgaatagtcctgaaggaaaagacaccattttctccctggcagattcttcggagtgaaatgcctgtttgacatgcatgatgaagtcaccccgttcaaatacaatcactatcagaattgatgaaattgcacaagagataacttctccgccagattatttgattagtttcgttcaaatacaaccagatcaatttaaactgcagcatcgcacacatgcagattgatatacagttttacagattcttgtacataaattgaaatacagttttacaaattaactaacatctttgatttacataagccaaaggctgaaacataagcccattgtcatatggtgtatcatgttggatatattattttttgcctaccaggtgtcatctggactccatgcagtacattgccacattctgtatttgttattgaacaagagtttagatattttagtgtcaggcacatgccaagttattcccttttcactgtctttctaagctgtaaacattccattcatgggattcgaaaataaaacagtattctattagttttagtgtgttatctctttgtttggagtgggcatgttttatttatttctttatcttgattaacctgtatggctaatttgacttttgtttcacaggatacacataaccaagcaggtattgcatacaatggtggcttgttacctttactaaagcttctcgactcaaaaaatggttctctgcaacataatgctgcgtttgctctttatggagttgccgacaatgaggtaattttttgttgttcaaaatatttgttcttggaagggaacggacttgtagtcatgttcatttctgttttatgtaagcttcttactttcatgtatccataataactttcttcttgtaggattatgtctctgacttcgttaaagtaggaggtgtccaaaagttgcaggatggcgaatttattgtccaggtatgtcaaccatcatagcatagattgatactttcttagtaaatttatacctgagtttggttaagcactttttttcaggctacaaaggactgtgtagctaagacattgaagaggctggaggagaagataaatggacgagtaagttctgctcactgtttcttttttcttttatttgccaagctgtggtatctactccaactgactcacgcgtgatctttaacaggtattaaaacacttggtttatctcatgagagtaggagaaaagtctgtgcagaggcgtgttgctctggctcttgcacacctctgtgcccctgaagatcagcgaacaatttttattgataataatggtatgaacaatttgacatcttaagtgttccttgtcccatttgtgttctgttctccatggattaaattctggcttaattcaggtctcgacttgcttcttgatcttctggtttcgggcagctcgaaacatcaacaggatggttcggtagcactatacaaattagccaacaaagctgcagcactctctccgatggatgctgcacctccatctccaacgccacaggttattagaaactaaaaaaagggtgatttgtctttactatgtagttatgctattgaagtgaataaggtcttcacagtgcttggaaaagagagttgtctaacaaaattgtcgtaaaaaaatatagttctagggatatatgctagtactccctccgttcggaattacttgtctcggatatggatgtatctacaactaaaatacatctagatacatccatttctgcgacaagtaattccgaacggagggagtattactttggagctattagcaagatctgaattaaatcaagatcatatgtgcacaaacttacttaaaatgttatttcctacaaatcgtgacatgtgcaacctgttggacacagatgttctgtcatgtaactttatactgcttagcagtctgttcttagtagttggcaggctttaccttgccctatcctggatattcttaatgaggtttccccataaatcaactcttaataccgatggattggtccatccataataagttactatactaaagcaggaaggctttggtttttctggtttttttgaattttttccaagcttctactattcatttacatccatgtcagtgaatagtaatagtgagcagtatcatgcataaacagcaccctgcatgaacagtaccaccactgaacagtgctccgaataatctgattttcccttttttttactttcaatggattaaaaatacgcacgttgtaaacaaaaactgggacttttttacacattatttctctcctccaccaccatcgcgtccatatatatagggttaagatttaggatttttctacacatcatttctctccactggcgtaccaacgcagagccgtctcagtcgtctcctgatcctttccggtgatggtgttgctgaggcacaaaacagtaggttggaacagtatatttgcataaataataattcatggggaaaataagttcttgaccgattactgcccatttttacaccacgacatcagcaaacagtttactaacacctgaacaaaaaccaaaacattatctgaataaacccagaatgctaaccagaacaataacaaaataaaccaagacaccaaccccgaataacctggaacacaaaaaccagtgaaacgggacaacagctgaataaaccaaaatttttaacccacccgaaccataaaccgaaacaataaccgagttgtaatctagaatagtacacctgaataaaccggagcaacatacgaaaaaatattaataggccagccggttttcttaatttgttaaataatttaatgttggttacgtgcctacactgatcatggggtaaagatagaattcgtgttctcctcttcattttattttatcgcttaatacatgttgttttcttgcttattttggtaaaatacagacagaaacgatcacgggcgcggcgtgcgccgcgcttcttcggcgctagttcttgctattgctattactaaatgtacttctgactgcaggtttatcttggggagcaatatgtgaacagttcgacactttcagatgtcaccttcttggtggaaggttcgtgacgtttctgcaccctgccttcacagaaactactttagataattgctttttttcattaggatcataataatcacctcccttgtgatccacaggaaaacgcttttatgcacacagaattgctctgcttgcttcttcagatgcattccgtgcaatgtttgatggtggatacagggttagtctcgacattacatgctattccttttttggttggaagatgtggatcttgtttgctagttgaacaatttctgtttacagaaactcactattttctcaaccaggaaaaggatgcaagagacatagaaattccaaatatcaggtgggatgtgtttgaactcatgatgaggttagtaaatcattgatcattcttgttccttggccatgtcccatgggtaaatctgcatgttagttcctcactctgaggggacaaggcctgcaattgaagtttggaaacatctttgttttgtgcagatttatctatacagggtcagtcgaagtaaccaatgagcttgctcaagatcttcttagagctgcagatcagtatctgttagaaggcctcaaacgcctatgtgaatatacaattgcgcaggtgatttcaggagcattacccccaagttctatgtttgaaccgctgccaactgggtctaattgattgtattgaatatcttgcaggatgttaatttagacaacgtctctgatatgtatgacttatccgaagcctttcatgccatgtcactgagacatacatgcgtcttgtttattttggagcagtttgataagatctgcaccagacccgggtgggtatcttaacctagggccaccacatttggtacataatgtaacacgcttcaagcaacgaaaaatccaaatccatctaactggtcatcttgcaaatgcagtttctctcagctaatccagcgcgtcatccctgagctccgcaacttcttcgctaaggcactaaggccaggccaccggagtgcgcaaccatgagccctgcccacattcgttgataacaccgccgccatctgacagatgctgctggaaatcttgtacagctgaagtttctggttctgggcattgggtactcactcggtggtaaggttaactattcaatctattatggtttgcatgatggccaggtcctcaatcgacacccagcaagaatgtaacatctcctattcgattgaacaatggtgatcatgctaagggaagtgtatggttatagagagacatgtggtttgcctagatgcagtcagaccggcctagtctgtgataggattagttggttggccttgaccggatttgtcgggtctcgccgtagttactgagttacttagggtcacttccagttcgcagttccgattatgtccgtgtatgttgtttggagatgttaagctcgagcggtgtaatgctgtagcatcaatctgtgttctccatgttaacaaccgtgctgatgttcaagactagtgttcagaactcgtgggctgtttcataccaaattcccatatatagcctttgctcaggttgtttg

SEQ ID NO: 119 - DNA, 11347 bp, Triticum aestivum
  source 1..11347: mol_type = genomic DNA
gcgctggggcgcgcatactctttgcttctgcccttccctcctcctccgcctccgacaagttccccaccttcatcgccgtcgacccgctctaatggaggcggagcagcagaagccgcagcgcccgcggcgcaaggcacagaagcgcaggattgacgacgaggccgccgcctcggccgccgcagccgcagccgccgccgccgccgccgccgcagcggccgccgccgtctcgtcgccgctcggcagcgccgatgccgacgacgacaacgaggacgacgagggctccgtcggccccgagatctgctgccgccagtcccaggcggcggtcgcccgcgaggtccgcacgcaggtcgacgccctccaccactgcttctcgtggcgccacgccgaccgcgccaccgccaagcgcgccactagcgtcctcgccgagctcgcgaaaaacggtaatcccccaaccctacgcccaccgtgccgatccgtactcttccccacccgtccaggcgccgttactgaggcggatctgcttgctgcttttgccgcagaggagatggtgaacgtaatcgtagagggcggcgccgtgccggcgttggtgtgccacctgaaggtgccccctatggcggcggcggtggaggaggagcagcagccgcggccgttcgagcacgaggtggagaagggggctgcctttgctctcgggctcctagccgtaaaggttaattcgattagttttcctctttgcactttagctgagattttgcttacattccattgcaattgcttgaattgttcttataatcccaattttctgggccgtggccggctcatacatgaaacatcccatttcgtagcaaaatgcaagaggaaaataaataccactctcttcccttcccctaatctcttgtctgtctgtaaatgtaacctcatacgccttcataagaatctaggtatacttgggttcaagcagaataggtttcaaccttgcctagttctctttaggcaatccataaatattattgttaacttttcttcaacgcgactacttcattgttatgattttagctatgttactctcagaatttagtcatttattactttttgtgttggtttaccagcctgaacatcaacaacttatagttgatgctggtgccctacccctgctggtgactctcctaagaaggcataaaaatgctacaaattcgagggcagttaacagccttatcagaagagcagctgatgcaattaccaaccttgctcatgagaatagcaacatcaaaacttgtatcaggttttattctatctaccactcactagtcaatgctgcgtttccatgaaagttttctgtgcttgctgatggttttgttgtactgcagaattgaaggcggaatcccacctctcgttgaattgctagaatcacaggatattaaggtgcagagggcagctgcaggggccttgaggactttggcgtttaaaaatgatgaaaacaaaaccctggtaagaatacaagaaagtttaagttaatgaaaccaacattaatgttactccctctgttcacttttataagaccttgaagacatttcagacaatgtgcaaaacagcttattttgagttgtctgaaacgacttacaaaagtgaacagagggagtagatattaacaccagactttcatcattcacccatatatattgtttccttacttctagatggtaaatcttccctttaactccttaatgcagatcgttgattgcaatgcactgccaacgttaatcttaatgctgcggtcagaggatgctgcaattcactatgaagcagtaagatactgaatattcatatattttcatcaaatatacttctttggttgaacccctcttcatttttagtgcggcacttgtcatgtatctattacaggaaaacattgttctggttttgaaccttgctatttctcttattttctacaatcttgaataacagttatcctaaggcctcaaaatgtattgtcttgattggcttaatggtgaaccttagtactatatattgcttgggaaacttccaggtcaaaatttctgttcaagttgcaatataacttaggttagtcggcacagcggcacttaccttaacttacttatcattatactccatttacattatgagcaatgcagttatggtgcactgtatcgatattgatgtgcatcagaacccaattccttcagtgtattgaattgttgtctcttattattattaaatattaaataaaggatagagtaattcctttgtctagagattctagagctgcaataagggctcatattgtcattatgttaatgaaaagtggttcagtggcatgttaacgaatctgtcgattacgaaaactagactttcagtctcttggacttcttattcttttgcttaggttcagccgaggtagtggacaaacagcggagaagaaatatggcgggggagaaatttcttgtgattgtgagcaagtagaattgcttgacttcaacaaacaaattgaagttctatctatcaatatctatggtcttgaccgtcatgattaacctcctttcataatactccctacccccagggaagttgaatccccgctgcctccttgaaagagagatgtcctgaaccactagacaatggcagtgaaaaattgagtgtacgcctaggcgcgcttaagtgatgagcggaggcctaccgctttgtttttgtggtaagcgttgaaacaaagcgctcggatgcctagggttagacaaaggagagcggggtgagagaaacagaggagagcaaggcgaccttgtgccgccagatgtggggctttcttcccgggcctcaccacccatcttcttccccgacctagcgctgctggacctcgagctcccgtccccgacctcgccgccagtcctctcccctcttccccaatctcgagctcctccttgtctaggctggagcctggtgatttctctccagcctcaccgctgccagcttgcttccccttccctgagctcgagctcctccttgtctcttcttccccaacatgcttgcgattttaggttttatacatgacttacatgttttgaaaattgatttttgggtgcccttgttcctgtccatatgacgtccgtacagaaagcttcagcacctaggcaccgcttaagccgccgctgaagctgtcattgcactaagcagaggcacaactctcgctcagtgcctagcgcttaaaaaataccttggacaataggcaacaaaagagttggtgctttgatacatcatttctgatgtccggaactgcagctatcggaagaaaagatgctgcctgatggagtgaacgaactagttcttacttctgtttggtgcgagatcccatggcggtagaggagagctttctttggaatagtctgacccagggagaatagagttattacaagtgagctaattagatcaaatctcatcaacatacattactttaggagaaactgagaggaacacagatatgagaaatcttaccccccaaatcaatgagaaacaggatctaaaaatattgtctattcatgatgattcggtttcaatcgataaggtagctggaccaatgtgatctactttgagtgtacctcaaggcagtgtgcctttaggggtcgtagtatctggtaaccagtctactcaaagaatgagtgggatcatcacatcattgctagaagactggtgtcatttcactcataaaaatgtgcaggatagctcagttggtagaaaaatgagtctcatataaaaataaagcaaaaaaaggataacgctttgtttggatgtccgtattggaacactccgtattgaattggactagaattccaattcggtgaggaaactgaaatggcacgaatacgaattcgactgtttggctgttcactgaattgacccttgaaatgcctctgaggtttcaataccaaatcttgtttggatgacaaactttggaattgcatagctacattagcatgaagattatatcttggtgtacatgactgaaaaattaaatctgctcacatgtgactataattgaatgaatatatagcagtaaaaaatagtaaatattctagaaatgaatcacaacaagacaaatggtcacacaacaagaagagaaagtacaggttatagtcacaaccaaagcatgcgtactcatcacggtagccatatgacccatactcaaaatcaacgagacagaatttctctgtaaaaaaggaagaaaataacgacatggtggagaaggaggtgctgaataggactgattgaatcagtggtaaggggagagggatgcaacacatggggatggggacgggatgggatgatggtcgccgcggccaccagatgggatggtggtcgccgtcaagtcgggatggggatggagactggtctccatggtggtcgccacgggagatggagacccggagcggagggatgcgggagggggcagagcaacggggaccgggattggggagggaagggacggaagggggaggacagagctgcgccgccgctgagcgccatggttggtcgccgccgccctagtaggccgccgtctttgcgagatcccctttcttctcttttcctgattgctggggtcgaaggggtaagttgcgggagatggacgattcagaggaaaacagagcgggagccctccgaatcatgggagtgagctttacgttggaggcaatacggcttggaaatggtctggcgtttccaatacgaattcagtgcgcaaccaaacatccgtattgatgtcagatgattagcaatttgatttcctgggcttcaatggggacatccaaacgcagtgtaatagaacttggtgagagctatacttgattgcacaaatgaacctagtgcatgatggcagcaagtatataagtatgccacagtggaattcctagaaaatcgtctgatgaactcgttctaagtcatagtgactcgtattgcagcaagtgcagaataagaaataaagctacacaaaacatgctgattatcagaaaaatgaattgcattagaggttgtcaggcttcctggctgtgtatctaggtgtttgggctttgaactaaacattagcctatcggagcttgcttaattgagctagttagatccattcgttggctaaatgatggaaaattaatttgacatggaagatgcttaattggtatgacaagcttgaggttcataattagtagaggcaaagcatccttataatccgtactgtgctctgccacaccagtttctgtcgcattactaaagataggcctagttagtgcaattgagcaagctgaggccttgagggagcctgcaattctgaaattgaagttaaggaccttaatgtcacaaatgggcttgtttgaggaactcatttttctgtcacattattgaagatgggcctaagtagtacaattaagcaagctgagaccttgatgaagtctgccaggctaaaattgacgttaagaaccttaatatcacaacctaactaggcaagtttgagcacctgtcctgtagctttatatatttgatgcgatgcacgcaacttactttttggagtgttacaaaagaagagctattccacatcagccaattggaaatttggaacattaacacctttaacttagcaatggagttactgatcctgtgaaatttatacaaagaaaatgatccgactatttgcttctatcaattacatatagatttctatatagatttatacttttgccaaatgcaaaggctgtcctcataaagttctctgtatacaacatattgtgacaattttgcatgaaatcaccctagtcgtggaactagccatatgtatgatattgtttttgctgtgcatgccagtaagtactaaatacactctgttggcgtggcaggttggtgtcattggaaatttggtccattcatccccaaatatcaagaaagaggttcttaatgcgggggccttgcaacctgtaattgggctattaaggtatgatgatcgtcatatgcagcttatgatgatagttttaattgtactccctccgtaaactaatataagagcgtttagataactattttagtgatctaaacgctcttatattagtttacagagggagtatctgttaataatgaaatgcatatttactgtatttatttgttgagttctgctagagtactgctggaaattcaaattctatatactttacttttagctgtacatgagcaatacacactcgattactgattacaccattgtgcatgtgttcctggatgcggattaattttgttgctttaaggtcaaaacaatatgtgattataatgatataatcttatgagattttcaagtgtaagcttgcgtgtagcaaattatcttctaacccagattccatatcatatccatattgtaacacgagaaactgttttattgtagtcccaatcttagtatatgaaggcatggttgccctgagtctgctctccagcttaaagaacctgtgcttcatcttttcttttgcagttcctgctgtacggaaagccaaagagaagctgctttgttgctagggcagtttgcttcggccgactctgagtgcaaggtgcttacggatgcttcatttgttgttagctccattttttttatgacgagtgatgaagtggaagagtaaaaaataaaatgaagtactttttcctatataatactcttgtgctacatatcattgattgattatgtctacctacttactaaatatgttgtttcgtacgataaagagttagccatggtgaatcaaaagagtacagaattattttttgagctatcctctctaaatatgcatgtatggggtttggcaggtccatattgtgcaacggggggcagtccgaccactaattgacatgctacagtcagctgacttccaactcagggagatgtcagcttttgcccttgggaggcttgcacaggttatatttctcattctatactccccttgcacacaacaatatcaatctgattgcttatgtttgtcagcgggttttactgcaagtattttggggacgcattgtagcagtgaaagagaaacaacaatgacaatccttacttcccttcataaatcacctgacatagtgacagagcactttctcaactttgctgcttccctttttctctatgttgattttacattgggatgcagtgtcccctcttagaaggattgacatgagagtgaccacaggttatgtttaatgtaccatcagtaattgaagccatgcagctcattctctttgtgtgtgttaaatatccagactaactgttgagcatctgcctctcaaatggtttctgttcagatttgtaccttttatttgtatatatgcttcttcgctgtatccattgtcccgcgacaagtaatcgtaacccagcatagttcagcatatctcttgaacatgcgcatttctgaatagtcctgaaggaaaatacaccattttctccctggcagattcttcgcagtgaaatgcctgtttgacatgcatgatgaagtcaccctgttcaaatacaatcactattagaattgacaaaattgtacaagagataacttctctgccagattatttgattaattttacttttacgtgagagataaaccctgttcaaatacaatcagatcaatttaaactgcagcattgcacacatacagattgatatacagttttacagattcttgtacataaattgaaatacagttttacaaattaaactaacatctttgatctacataagccaaaggctgaaacataagccccaatggtcattgtcatatggcatatcatgttggatatttttttttgcctaccaggtgtcatctggactccatgcagtacattgccacattctgtatttgttattccctccgttcctaaatataagtctttgtagagatttcactatggaccacatgcggatgtatgtagatgcattttagagtagattcactcattttgctccgtatgtagtccatagtggaatctctacaaagacttgtactccctccgttcctaaatataagtctttctagagatttcaatatggactacatacggaacaaaatgtatgaatctacattctaaactacgtctatatacatctgtatgtagtccatagtgaaatatctagaaagacctatatttaggaacggagggattagtaagcaagagtttagatattttagtgtcaggcacatgccaagttattcccttttcattgtctttctaagctgtaaacattccaatcatgggattggaaaatgaaacagtattctattagttttagtgtgttatctctttgtttggagtgggcatattttatttacttatttatcttgattaacctgtatggctaatttgaaagaaaatcttttctttcacaggacacacataaccaagcaggtattgcatacaatggtggcttgttgcctttactaaagcttcttgactcaaaaaatggttctctgcaacataatgctgcgtttgctctttatggagttgcggacaatgaggtaattttttattgttcaaaatattggtttctatttattatttcatatttgttcttcaaagggaacgaactcatgtagtcatgttccatttctgttttatgtaagcttcttactttcatgtatcaataataactttcttcttgtaggattatgtctctgacttcgttaaagtaggaggtgtccaaaagttgcaggatggcgaatttatcgtccaggtatgtcaaccatcatagcataggttggtactttcttagtaaatttatacctgagtcgggttaagcactttttttcaggctacaaaggactgtgtagctaagacattgaagaggctagaggagaagataaatggacgagtaagttttgctcactgtttcttttttcttttatttgccaagctgtggcatctactccagctgactcacgcgcgatctttaacaggtgttaaaacacttggtttatctcatgagagtaggagaaaagtctgtgcagaggcgtgttgctctggctctcgcacacctctgtgcccctgaagatcagcgaacaatttttattgataataatggtatgaacaatttgacatcttaagtgttccttgtttcatttgtgttttgttctccatggattaaattctggcttaattcaggtctcgacttgcttcttgatcttctggtttcggtcagctcgaaacatcaacaggatggttcggtagcactatacaaattagccaacaaagctgcagcactctctccgatggatgctgcacctccatctccaacgccacaggttagtagaaactaaaaaaaaggtgatttgtcttgactatgtagttatgctattgaagtgaataaggtcttcacagtgcttggaagagagatttgtctaacaaaattgtcgtaaaaaatatagttctagggatatatgctagtactactttggagctattagcaagatctgaattaaatcaagatcatatgtgcacaaactaacttaaaatgttatttcctacaaatcgtgacatctgcaacctgttctgtcatgtaattttatactgcttagcagtctgttcttagtagttggcaaggctttaccttgccctatcctggatattcttaatgagccataaatcaactcctaataccgatggattggtccatccataattctggctattgctattactaaatgtacttctggctgcaggtttatcttggagagcaatatgtgaacagttcgacactttcagatgtcaccttcttggtggaaggttcgtgacgtttctgcaccctgccttcacagaaactactttagataattgctgttttttcattaggaccataataatcacctcccttgtgatccgcaggaaaacgcttttatgcacacagaattgctttgcttgcttcttcagatgcattccgtgcaatgtttgatggtggatacagggttagtctcgacataacatgatattccttttttggttggaagctgtggatcttgtttgctagttgaacaatttctgtttacaagaaactcaccattttctcaaccaggaaaaggatgcaagagacatagaaattccaaatatcaggtgggacgtgtttgaactcatgatgaggttagtaaatcattgaccattcttgttccttggacattgcccatgggtaaatctgcatgttagttcctttctcttacgggacaaggcctgctgcctgcaattgaagtttgggaacatcttctttgttttgtgcagatttatctatacagggtcagtcgaagtaaccaacgagcttgctcaagatcttctgagagctgcagatcagtatctgttagaaggcctcaaacgcctatgtgaatatacaattgcgcaggtgatctcaggaacatcacccccaaagttctatgtttgaaccgctgccgactgggtctaattgattgtattgaatatcttgcaggatgttaatttagacaacgtctctgatatgtatgacttatccgaagcctttcatgccatgtcactgagacatacgtgcgtcttgtttattttggagcagtttgataagatctgcaccagacccgggtgggtatcttaatttagggccaccacattggtacataataatgtagcgctcttcaagcaacaaaaatcctaatccttctaactggccatcttgcaaatgcagtttctctcagctaatccagcgcgtcatccctgagctccgcaacttctttgctaaggcgctaaggccaagccaccggagtgcgcaaccatgagccctgccaacattcgttgataacaccgccaccacctgacagatgctgctggaaatcttgtacagctgaagtttctggttctgggcattgggtactcgctcggtggtaaggttaactattcaatctattatggtttcatgatggccaggtcctcaattgacaccaagcaagaatgtaacatcctcctgttcgattgaacaatggcgatcatgctaagggaagtgtatcgttatagagagacatgtggtttgcctagatgcagtcagaccggcctagtctgtgataggtttagttggttggccttgaccggatttgtcgggtctcgccgtagttactgagttacgtagggtcacttctgtttcgcagttccgattatgtccgtgtatcttgtttggagatgttaagcttgagcggtgtaatgctgtaacatcagtctgtgttctccatgttaacaaccgtgctgatgttcaagactagtgttcagaattcgtgggctgtttcatatcaaattcccatgtgaggttatattatagccttgctcaggttgt

SEQ ID NO: 120 - DNA, 10192 bp, Triticum aestivum
  source 1..10192: mol_type = genomic DNA
gcggaataaatccctatcgcgctggggcgcgcatactctttgcttctgcccttccctcctcctccgcctccgacaagttccccaccttcatcgccgtcgacccgctctaatggaggcggagcagcagaagccgcagcgcccgcggcgcaaggcgcagaagcgcaggattgacgacgaggccgccgcctcggccgccgcagccgcagccgccgccgccgccgccgccgcagcggctgccgccgtctcgtcgccgctcggcagcgccgatgccgacgacgacaacgaggacgacgaggtctccgtcggccccgagatctgctgccgccagtcccaggcggcggtcgcccgcgaggtccgcacgcaggtcgacgccctccaccactgcttctcgtggcgccacgccgaccgcgccaccgccaagcgcgccaccagcgtcctcgccgagctcgcgaaaaacggtaatcccccaaccctacgccgaccgtgccgatccgtactcttccccacccgttcaggcgccgttactgaggcggatctgcttgctgcttttgccgcagaggagatggtgaacgtaatcgtagagggcggcgccgtgccggcgttggtgtgccacctgaaggtgccccctatggcggcggcggtggaggaggagcagcagccgcggccgttcgagcacgaggtcgagaagggggctgccttcgctctcgggctcctagccgtaaaggttaattcgattagttttcctctttgcactttagctgattttgcttacattccattgcaattgcttgaattgttcttataatccaaattttctgggccttggcctgctcaaggctcatacaacctcccatttcgtagtaaaatgcaagagaaaaacaaataccactctcttcccttctcctaatctctcgtatgtctgtgaatgtaacttcatacgccttcataagaatctaggtatacttgggttcaagcagaataggtttcaaccttgcctagttctctttaggcaatccataaatattattgttaacttttcttcaacacgactacttcattgttatgattttagctatgttactctcagaatttagtcatttattactttttgtgttggtttaccagcctgaacatcaacaacttatagttgatgctggtgccctacccctgctggtgactctcctaagaaggcataaaaatgctacaaattcgagggcagttaacagccttatcagaagagcagctgatgcaattaccaaccttgctcacgagaatagcaacatcaaaacttgtatcaggttttgttctatctactgctcactagtcaatgctgcgtttccataaaagttttctgtgcttgctgatggttttgttgtactgcagaattgaaggcggaatcccacctctcgttgaattgctagaatcacaggatattaaggtgcagagggcagctgcaggggccttgaggactttggcgtttaaaaatgatgaaaacaaaaccctggtaagaatataagaaagtttaagttaatgaaaccaacattaatgttagattttaacatcagactttcatcattcacccatatatattatttccttacttctagatggtaaatcttccctttaactccttaatgcagatcgttgattgcaatgcattgccaacgttaatcttaatgctgcggtcagaggatgctgcaattcactatgaagcagtaagatactgaatattcatatattttcatcaaatacacttctttggttgaacccctcttcatttttagtgcagcacttgtcatgtatctattacaggaaaacattgttctgattttgaaccttgctatttctcttgttttctacaatcttgaataacagttatcctaaggcctcatggaatgtaaacttcaaaatgtattgtcttgattggcttaatggtgaaccgtagtactatatattgcttgggaaacttccaggtcaaaatttctgttcaagttggaatgtaacttaggttagtcggcacagcggcacttaccttaacttacttatcattatactccatttacattatgagcaatgcagttatggtgcactacatcgatattagaacccaattccttaagtgtattgaattgttgtctcttattattattaaatattaaataaaggatagagtaattcctttgtctagagattctagagctgcaataaggcctcatattgtcattatgttaataaaaagtggttcagtggcatgttaacgaatctgtcgattaggaaaactagactttctgtctcttggacttcttattaggttcagccgaggtagtggacaaacagcggggaagaaatatggcgggggagaaatttcttgtgattgtgagcaagtagaattgcttgacttcaacaaacaaatggaagttctatctatcaatatctatggtcttgaccgtcatgattaacctcctttcataatactccctacccccagggaagttgaatccccgccgcctccttgaaagagagatggcagtgaaaaattgagtgtacgcctaggcgcgcttaagtgatgagcgtaggcctaccgctttgtttttgtggtaagtgttgaaacaaagcgctcggacgcctagggttagacaaaggagagcggggtgagagaaacagaggagagcaaggcgaccttgcgccgccagatgtggggctttcttccccggcctcaccacccatcttcttccccgacctagcgccgctggacctcgagctccctgtccccgacctcgccgccagtcctcccccctcttccccaatctcgagctcctccttgtctaggctggagcctggtgatttctctccaacctcaccgctgccagcttgcttccccttccctgagctcgagctcctcctcgtctcttcttccccaacatgcttgcgattttaggcttaatacatgatttacatgttttgaaaattgttttttgggtgcccttgttcctgtccatatgacgtccgtacagaaagcttcagcgcctaggctccgcttaagccgccgctgaagctgccattgcactaagcggaggcacaactctggctcagtgcctagcgcttaaaaaaaaccttggacgataggcagcaaaagagttagtgctttgatacatcatttctgatgtccggaactgcagctatcggaagaaaagatgctgcctgaggaagtgaacgaactagttcttacttctgtttgatgcgagatcccatggcggtagaggaaagctttctttggaatagtctgacccagggagaatagagttattacaagtgagctaattagatcaagtctcatcaacatacattacttcaggagaaactgagaggaacacagatatgagaaatcttaccccccaaaacaatgagaaacaggatctaaaaacattgtctattcatgatgattcggtttcaatcgctaaggtagctggaccaatgtgatctaccaagagtgtacctcgaggcagtgtgcctttaggggtcgtagtatctggtaaccagtctactcaaagaatgagagtgggatcatcacatcattgctagaagactgggcgtcatttcactcacaaaaatgtgcaggatagctcagttggtagaaaaatgagtttagcgctgttaagaaaatcatataaaaataaagcaaaaaaaggataatagaacttggtgagagctatacttgattgcacaaatgaacctagtgcatgatggcagcaagtatataagtatgccacagtggaattgctagaaaatcgtctgatgaactcgttctaagtgatagcgactcgtattgcagcaagtgcagaataagaaataaagatacacaaaatatatttgcctaaccatgctgattatcagagaaataaattgcattagaggttgtcaggcttcctggctgtgtatctaggtgtttgggctttgaactaaacattagcctatcggggacttgcttaattgagctagttaggtccatccattggctaaatgatggaaaattaatttgacatggaagatgcttaattggtatgacagcttgaggttcataattagtagaggcaaaacatccttataatccgtactgtgctctgccacaccattttctgtcgcattactaaagataggcctagttagtgcaattgaccaagctgaggccttgagggagcctgcaattctgaaattgaagttaaggcccttaatgtcacaaatgggcttgtttgaggaactcatttttctgtcacattattgaagatgggcctaagtagtacaattaagcaagctgagaccttgatgaagtctgccaggctaaaattgacgttaagaaccttaatatcacaacccaactaggcacgtttgagcacctgtcctgcagctttatatgtttgatgtacacaaattactttttggagtgttacaaaagaagagctattccacatcagccaattagaaatttggagcattaacacctttaacttagcaatagagttactgatcctgtggaatttatacaaagaaaatgatctgactatttgcttctatcaattatatatagatttcgagatagatttatacttttgccaaatgcaaaggctgtcctcataaagttctctgtatacaacatatattgtgacaattttgcataaaaatcaccctagtcgtggaactagccatatgtatgatattgtttttgctgtgcatgccagtaagtactaaatacactctgttggcgtggcaggttggtgtcattggaaatttggtccattcatccccaaatatcaagaaagaggttcttaatgcgggggccttgcaacctgtaattgggctattaaggtatgatgatcgtcatatgcagcttatgatgatagttttaattgtatctgttaataatgaaatgcatataacttactgtatttatttattgagttctgctagagtactgctggaaattcaaattctatatactttacttttagctgtacatgagcaatacacactcgattactgattacaccattgtgcatgtgttcctgaatgcggattaattttgttgctttaaggtcaaaacaatatgtgattataatgatataatcttatgagattttcaagtgtaagcttgcgtgtagcaaattatcttctaacccagattccatatcatatccatattgtaacacgagaagctgttttattgtagtcccaatcttagtatatgaaggcatggtattaccccgggtctgctctccagcttaaagaacctgtgcttcatcttttcttttgcagttcctgctgtacggaaagccaaagagaagctgctttgttgctagggcagtttgcttcggccgactctgagtgcaaggtgcttaaggatgcttcatttgttgttagctccatatttttttatgacgagtgatgaagtggaagagtaaaaaataaaatgaagtactttttcctatataatactcttgtgctacatatcattgattgattatgtctacctacttactaaatatgttgtttcgtacgataaagagttagccatggtgaatcaaaagaatacagaattgttttttgagctatcctctctaaatatgcatgtatggggtttggcaggtccatattgtgcaacggggggcagtccgaccactaattgacatgctacagtcagctgacttccaactcagggagatgtcagcctttgcccttgggaggcttgcacaggttatatttctcattctatactccccttgcacacaacaatatcaatctgattgcttatgtttgtcagcgggttttactgcatgtattttagggacgcattgtagcagtgaaagagaaacaacaatgacaatccttacttcccttcataaaatcacctgacatagtgacagagcactttctcaactttgctgcttccctttttctctattttgattttacattgggatgcagtgtcccctcttagaaggattgacatgagagtgaccacaggttatgtttaatgtaccatcaataattgaagccatgcagctcattctctttatgtgtgttaaatatccagactaactgttgagcatctgcctctcaaatggtttctgttcagatttgtaccttttatttgtatatatgcttcttcgctgtatccattgtcccgcgacaagtaatcgtaacccagcatagttcagcatatctcttgaacatgcgcatttctgaatagtcctgaaggaaaagacaccattttctccctggcagattcttctgagtgaaatgcctgtttgacatgcatgatgaagtcaccctgttcaaatacaatcactattagaattgacgaaattgcacaagagataacttctccgccagattatttgattagttttacttttacgtgagagataaaccctgttcaaatacaatcagatcaatttaaactgcagcatcgcacacatacagattgatatacagttttacagattcttgtacataaattgaaatacagttttacaaattaaactaacgtctttgatctacataggtcaaaggctgaaacataagccccaatggtcattgtcatatggcgtatcatgttggatatattattttttgcctaccaggtgtcatctggactgtatttgttactccctccgtttctaaatataagtctttgtagagatttcactatggaccacacgaggatgtttgtagatgcattttagagtagattcactcattttgctccgtatgtagtccatagtggaatctctacaaagacttgtactccctccgttcctaaatataagcctttctagagatttcaatatggactacatacggagcaaaatgagtgaatctacattctaaactacgtctatatacatccgtatgtagtccatagtgaaatctctagaaagacctatatttaggaacggagggattagtaagcaagagtttagatattttagtgtcaggcacatgccaagttattcccttttcattgtctttctaagctgtaaacattccaatcatgggattggaaaatgaaacagtattctattagttttagtgtgttatctctttgtttggagtgggcatattttatttacttatttatcttgattaacctgtatggctaatttgaaagaaaatcttttgtttcacaggacacacataaccaagcaggtattgcatacaatggtggcttgttgcctttactaaagcttcttgactcaaaaaatggttctctgcaacataatgctgcgtttgctctttatggagttgcggacaatgaggtaattttttattgttcaaaatattggtttctatttattatttcatatttgttcttcaaagggaacgaactcatgtagtcatgttccatttctgttttatgtaagcttcttactttcatgtatcaataataactttcttcttgtaggattatgtctctgacttcgttaaagtaggaggtgtccaaaagttgcaggatggcgaatttatcgtccaggtatgtcaaccatcataccccctccgttccaaaatagatgacccaactttgtacaaagttagtacaaagttgggtcatctattttggaacggagggagtagcatagattggtactttcttagtaaatttatacctgagtctggttaagcactttttttcaggctacaaaggactgtgtagctaagacattgaagaggctagaggagaagataaatggacgagtaagttttgctcactgtttcttttttcttttatttgccaagctgtggcatctactccagctgacccacgcgcgatctttaacaggtattgaaacacttggtttatctcatgagagtaggagaaaagtctgtgcagaggcgtgttgctctggctcttgcacacctctgtgcccctgaagatcagcgaacaatttttattgataataatggtatgaatgatttgacatcttaagtgttccttgtctcctttgtgttttgttctccatggattaaattctggcttaattcaggtctcgacttgcttcttgatcttctggtttcggtcagctcgaaacatcaacaggatggttcggtagcactatacaaattagccaacaaagctgcagcactctctccgatggatgctgcacctccatctccaacgccacaggttagtggaaactaaaaaaagggtgatttgtctttactatgtagttgtgctattgaagtgaataagggcttcacagtgcttggaaaagagatttttctaacaaaattgtagtaaaaaaatatagttctagggatatatgctagtactactttggagctattagcaaaatctgaattaaatcaagatcttatgtgcacaaacttccttaaaatgttatttcctacaaatcttgacatgtgcaacctgttggacacagatgttctgtcatgtaactttatactgcttggcagtctgttcttagtagttggcaggctttaccttgccctatcctggatattcttaatgaggtttccccataaatcaactcctaatacagatggattggtccatccatcattctggctattgctattactaaatgtacttctggctgcaggtttatcttggagagcaatatgtgaacagttcgacactttcagatgtcaccttcttggtggaaggttcgtgacgtttctgcaccctgccttcacagaaactgctttagataatttctgttttttcattaggaccataataatcacctcccctgtgattcgcaggaaaacgcttttatgcacacagaattgctttgcttgcttcttcagatgcattccgtgcaatgtttgatggtggatacagggttagtctcgacataacatgatattccttttctggttggaagatgtggatcttgtttgctagttgaacaatttctgtttacaagaaactcactattttctcaaccaggaaaaggatgcaagagacatagaaattccaaatatcaggtgggacgtgtttgaactcatgatgaggttagtaaatcattgatcattcttgttccttggccatggtccatgggtaaatctgcatgttagttcctcactctgaggggacaaggcctgcaattgaagtttagaaacatcttctttgttttgtgcagatttatctatacagggacagtcgaagtaaccaacgagcttgctcaagatcttcttagagctgcagatcagtatctgttagaaggcctcaaacgcctatgtgaatatacaattgcgcaggtgatttcaggaacataacccccaagttctatgtttgaaccgctgccgactgggtctaattgattgtttggaatatcttgcaggatgttaatttagacaacgtctctgatatgtacgacttatccgaagcctttcatgccatgtcactgagacatacatgcgtcttgtttattttggagcagtttgataagatctgcaccagacccgggtgggtatcttaacttagggccaccacatttggtatattgtaacgtgcttccaagcaacaaaaatccaaatccatctaactgtccatcttgcaaatgcagtttctctcagctaatccagcgtgtcatccctgagctccgcaacttcttcgctaaggcgctaaggccaagccaccggagtgcgcaaccatgagccctgcccacattcgttgataacaccgccgccatctgacagatgctgctggaaatcttgtacagccgaagtttctggttctgggcattgggtactcgctcggtggtaaggttaactattcaatctattaggtcctcaatcgacacccagcaagaatgtaacatcctcctgttcgattgaacaatggcgatcatgctaagggaagtgtatggttatagagagacatgtggtttgcctagattcagtcagaccggcctagtctgtgatagattttagttggttggccttgaccggatttgtcgggtctcgccgtagttactgagttacttagggtcatttccagttcgcagttccgattatgtccgtgtatgtttggagatgttaagttcgaccgctgtaatgctgtaacatcaatctgtgttctccatgttaacaaccgtgctgatgttcaagactagtgttcagaactcgggctgtttcatatcaaattcccatatatagcctttgctcaggttgt

SEQ ID NO: 121 - protein, 730 aa, Triticum aestivum
MEAEQQKPQRPRRKAQKRRIDDEAAASAAAAAAAVLSPLGSADADDDNEDDEGSVGPEICCRQSQVAVAREVRTQVDALHHCFSWRHADRATAKRATSVLAELAKNEEMVNVIVEGGAVPALVCHLKVPHMAAAVEEEQQPRPFEHEVEKGAAFALGLLAVKPEHQQLIVDAGALPLLVSLLRRHKNATNSRAVNSLIRRAADAITNLAHENSNIKTCIRIEGGIPPLVELLESQDIKVQRAAAGALRTLAFKNDENKTLIVDCNALPTLILMLRSEDAAIHYEAVGVIGNLVHSSPNIKKEVLNAGALQPVIGLLSSCCTESQREAALLLGQFASADSECKVHIVQRGAVRPLIDMLQSADFQLREMSAFALGRLAQDTHNQAGIAYNGGLLPLLKLLDSKNGSLQHNAAFALYGVADNEDYVSDFVKVGGVQKLQDGEFIVQATKDCVAKTLKRLEEKINGRVLKHLVYLMRVGEKSVQRRVALALAHLCAPEDQRTIFIDNNGLDLLLDLLVSGSSKHQQDGSVALYKLANKAAALSPMDAAPPSPTPQVYLGEQYVNSSTLSDVTFLVEGKRFYAHRIALLASSDAFRAMFDGGYRDARDIEIPNIRWDVFELMMRFIYTGSVEVTNELAQDLLRAADQYLLEGLKRLCEYTIAQDVNLDNVSDMYDLSEAFHAMSLRHTCVLFILEQFDKICTRPGFSQLIQRVIPELRNFFAKALRPGHRSAQP

SEQ ID NO: 122 - protein, 742 aa, Triticum aestivum
MEAEQQKPQRPRRKAQKRRIDDEAAASAAAAAAAAAAAAAAAAAVSSPLGSADADDDNEDDEGSVGPEICCRQSQAAVAREVRTQVDALHHCFSWRHADRATAKRATSVLAELAKNEEMVNVIVEGGAVPALVCHLKVPPMAAAVEEEQQPRPFEHEVEKGAAFALGLLAVKPEHQQLIVDAGALPLLVTLLRRHKNATNSRAVNSLIRRAADAITNLAHENSNIKTCIRIEGGIPPLVELLESQDIKVQRAAAGALRTLAFKNDENKTLIVDCNALPTLILMLRSEDAAIHYEAVGVIGNLVHSSPNIKKEVLNAGALQPVIGLLSSCCTESQREAALLLGQFASADSECKVHIVQRGAVRPLIDMLQSADFQLREMSAFALGRLAQDTHNQAGIAYNGGLLPLLKLLDSKNGSLQHNAAFALYGVADNEDYVSDFVKVGGVQKLQDGEFIVQATKDCVAKTLKRLEEKINGRVLKHLVYLMRVGEKSVQRRVALALAHLCAPEDQRTIFIDNNGLDLLLDLLVSVSSKHQQDGSVALYKLANKAAALSPMDAAPPSPTPQVYLGEQYVNSSTLSDVTFLVEGKRFYAHRIALLASSDAFRAMFDGGYREKDARDIEIPNIRWDVFELMMRFIYTGSVEVTNELAQDLLRAADQYLLEGLKRLCEYTIAQDVNLDNVSDMYDLSEAFHAMSLRHTCVLFILEQFDKICTRPGFSQLIQRVIPELRNFFAKALRPSHRSAQP

SEQ ID NO: 123 - protein, 776 aa, Triticum aestivum
RNKSLSRWGAHTLCFCPSLLLRLRQVPHLHRRRPALMEAEQQKPQRPRRKAQKRRIDDEAAASAAAAAAAAAAAAAAAAAVSSPLGSADADDDNEDDEVSVGPEICCRQSQAAVAREVRTQVDALHHCFSWRHADRATAKRATSVLAELAKNEEMVNVIVEGGAVPALVCHLKVPPMAAAVEEEQQPRPFEHEVEKGAAFALGLLAVKPEHQQLIVDAGALPLLVTLLRRHKNATNSRAVNSLIRRAADAITNLAHENSNIKTCIRIEGGIPPLVELLESQDIKVQRAAAGALRTLAFKNDENKTLIVDCNALPTLILMLRSEDAAIHYEAVGVIGNLVHSSPNIKKEVLNAGALQPVIGLLSSCCTESQREAALLLGQFASADSECKVHIVQRGAVRPLIDMLQSADFQLREMSAFALGRLAQDTHNQAGIAYNGGLLPLLKLLDSKNGSLQHNAAFALYGVADNEDYVSDFVKVGGVQKLQDGEFIVQATKDCVAKTLKRLEEKINGRVLKHLVYLMRVGEKSVQRRVALALAHLCAPEDQRTIFIDNNGLDLLLDLLVSVSSKHQQDGSVALYKLANKAAALSPMDAAPPSPTPQVYLGEQYVNSSTLSDVTFLVEGKRFYAHRIALLASSDAFRAMFDGGYRDARDIEIPNIRWDVFELMMRFIYTGTVEVTNELAQDLLRAADQYLLEGLKRLCEYTIAQDVNLDNVSDMYDLSEAFHAMSLRHTCVLFILEQFDKICTRPGFSQLIQRVIPELRNFFAKALRPSHRSAQP

SEQ ID NO: 124 - DNA, 18402 bp, Hordeum vulgare
  source 1..18402: mol_type = genomic DNA
atggaggcggagcagcaaaagccgcagcgcccgcggcgcaaggcgcagaagcgcaggattgacgacgaggccgctgcctcggccgccgcagcggcagccgccgccgccgccgccgccgccgcggctgccgccgtctcgtcgccgctcggcagcgccgatgccgacgacgacaacgaggacgacgagggctccgtcggcaccgagatctgctgccgccagtcccaggcggcggtcgcccgcgaggtccgcacgcaagtcgacgccctccatcactgcttctcgtggcgccacgccgaccgcgccaccgccaagcgcgccaccagcgtcctcgcggagctcgccaaaaacggtaatcccccaaccctacgcagactgtaccgatccgtactctttcccacccgtctaagcgccgttactgaggcggatctgcttgctacttttgccgcagaggagatggtgaacgtaatcgtagagggcggcgccgtgccggcgttggtgtgccatctgaaggtgccccctatggaggcggcggtggaggaggagcagcagccgcggccgttcgagcacgaggtcgagaagggggctgccttcgctctcgggctcctagccgtaaaggttaattcgattagtttcctctttgcactttagctgagattttgcttacattccattgcaattgcttgaattgttcttacaagccaaaatttctgggccagaatgcaagaggaaaatacaaataccgctctcccccatttcccctaatctcttgtgtgtctgtaaatgtaacttcatacgccttcataagaatctaggtatacttggcttcaagcagaataggctacaaccttgcctagttctctttaggcaatccataaatgttatcattaacttttcttcaacacgactacttcattgttatgattttagctatgttgctctcagaatttagtcatttattactttgtgtgttggtttaccagcctgaatatcaacaacttatagttgatgctggagccctacccctgctggtgcatctcctaagaagccataaaaatgctacaaattcgagggcagttaacagccttatcagaagagctgctgatgcaattaccaaccttgctcatgagaatagcaacatcaaaacttgtatcaggttttgttctatccactgctcactagtcaatgctgcttttccatggaagttctctgtgcttgctgatggttttgttctactgcagaattgaaggcggaatcccacctcttgttgaattgctagaatcacaggatattaaggtgcagagggcagctgcaggggccttgaggactttggcgtttaaaaatgatgaaaacaaaaccctggtaagactataagaaagtttaaattaatgaaaccaacattaatgttagattttaacattagactttcatccacattcgcccatgtatattatttccttctagatggtaaatcttccccttaactccttaatgcagatcgttgattgcaatgcattgccaacgttaatcttaatgctgcggtcagaggatgctgcaattcactttgaagcagtaagatactgaatattcatatatttttcatcaaacgtacttctctggttgaacgcctcttcatttttagggcggcacttgtcatgcatctattacaggaaaacatagttctggttttgaaccttgctatttctcttgtttcctataatcttgaataacagttatcctaaggcctcatggaatttaaacttcaaaatgtattgtcttgattggcttagtggtgaaccgtagtactatatattgcttgggaaatttcgaggatagagtaattcctttttctagagattctggagctgtaaaagggcttgttgttattatgttaataaaaagtggttcaacggtttgttaacaatcggtcgattacgaaaactaggctttctttctcttggacctctttattcttttgcttaggttcagccgaggtagcggacaaatagaggggaagaaaatatgttgggggagaaatttcttttgattgtgagcaagtagaatagcttgaattcaacaaataaatggaatttctatctatcaatatctatggtcttggaccgtcatgattagcctcctttcataatactccgtacccccaggggagtcgaatccctgctgcatccttgaaagagggacgtcctgaaccactagacggtagcagtgaaaaattgggcgtacgcctaggcgcgcttaagtgctgagcggaggcctactgcttcgcttttgggttaagcgctgaaacagcgctcggacgcctagggttagacaaatgagagcggggtgagagaaaaagaggagagcaaggcgaccttgcgccgccagatgtggggctttcttccccgacctcaccactcatcttcttccttgacttaacgctgctggacctcgagctcctcttcccgccttctccgccagcccccccttcctggatctcgggctcctcctcgtcttggctggagtctgatggcttctcttccccaaccttgccgctgccagctttcttccccttccctgacttcgagctcctcgtctctccttccccgacacgcttccgattttaggcttaatacatgacttacatgctttgaattttttttgggtgcccttgttcctgtccatacgacgtccgtacagaacgcttaagcgcgcctaggcgccgcttaagctgtcattgcactaagcggaggcacaatgttcgctgaatgcccaacgcctaaaaaaccctttgatgataggcaacaaaagagttagtgctttgacacaacatttcttccagaactgcagctatctgaagaaaaaatgctgtctgcgaaagtgaacgaactagttatttcttctgttcgaggatatgagtagatagctgttggtgcgagatcccttggcggtagaggagagatttctttgcaatagtctgacccagggagaatagagttattacaaggctgagctaattagatcaaatctcatcaacgtacattactttaggagaaattgagaggacacagatatgagaaatcttaccctccaaaacaataagaagcaggatctaaaaacattgtttattggtgatgattcgggttcaatcgataagttagctgggccaatgtgatgtaccaagagtacctcgagttagtgtgcctcgaggtcgtagtatttggcaaccagtttaattaaagaatgagagtgggatcatcatgtcattactagaagactggtgtcatttcactcacaaaaagtgcaggatagctcagttggtagaaaaacgagttcaccacttctaagaaaatcatataaaaacaaagcaaaagccgggcaatagaacttggtgagagctatacttgattgcacaaatgaacctaatgcatgatggcagcaagtataggagcatgctgcagtggaattgctagaaaatcgtccgatgaactcgttctaagtgatagtgactcatattgcagcaagtgcagaataagaaatacaacaacaacaacaaccaagcctttcagtcccaaacaagttggggtaggctagagttgaaacccataagatctcgaagccaagtcatggctctggaacgtggatagctaacttccacgcacccctgtccatggctaagtctttgtcgatattccaaaccttcaggtctctcttaacggactcctcccatgtcaagtttggtctaccacgacccctcttaacattctcagcacgctttatccgtccgctatgcaccggcgcttccggtggcctccgttgaatatgtcaaaaccatctgagacgatgctggaccagcttctcttcaatcggtgctaccccaagtctctcgtatatcgtcattccgtacccgatccttccttgtgtggccacatatccatctcaacatgcgcatctctgctacacctaactgttggatatgtcgtctcttggttggccaacactccgcgccatacaacatcgcaggttggatagctgtcctataaaacctgccttttagcttttgtggcactcttgtcacagagtacgccagaagcttggcgccacttcatccacctagccttgattcggtggcccacgtcttcatcgatatcgccatccttctgcaacatggaccccaaatatcgaaacgtgtctctctccggtatcacctgcccaccaaggctaacctctccatcctcgtgcctagtagcactaaaactgcacctcatgtattcagttttagttctactaagcctaaaacctttcgattctagagtccgcctccataactctaactttctattaacccccgttcggctatcatcgactagcaccacatcatccgcaaagagcatacaccatgggatatctccttgtatatcccttgtgacctcatccatcaccaaatcaaaaagataagggctcaaagctgacccttnnnnnnnnnnnnnnnnnnnnnnnnnnnnnnnnnnnnnnnnnnnnnnnnnnnnnnnnnnnnnnnnnnnnnnnnnnnnnnnnnnnnnnnnnnnnnnnnnnnnnnnnnnnnnnnnnnnnnnnnnnnnnnnnnnnnnnnnnnnnnnnnnnnnnnnnnnnnnnnnnnnnnnnnnnnnnnnnnnnnnnnnnnnnnnnnnnnnnnnnnnnnnnnnnnnnnnnnnnnnnnnnnnnnnnnnnnnnnnnnnnnnnnnnnnnnnnnnnnnnnnnnnnnnnnnnnnnnnnnnnnnnnnnnnnnnnnnnnnnnnnnnnnnnnnnnnnnnnnnnnnnnnnnnnnnnnnnnnnnnnnnnnnnnnnnnnnnnnnnnnnnnnnnnnnnnnnnnnnnnnnnnnnnnnnnnnnnnnnnnnnnnnnnnnnnnnnnnnnnnnnnnnnnnnnnnnnnnnnnnnnnnnnnnnnnnnnnnnnnnnnngcaaagagcatacaccatgggatatctccttgtatatcccttgtgacctcatccatcaccaaatcaaaaagataagggctcaaagctgacccttggtgtagccctattctaatcggaaagtcatcggtgtcgccatcacttgttcgaacacttgtcacaacattatcatacatatccttgatgagggtaatgtactttattgggactttgtgtttctccaaggcccaccacatgacattccgaggtatcttatcataggccttctccaaatcaatgaacaccatatgaaggtccttcttttgctccctgtatctctccatcagctgtcgtaccaagaagatggcttccatggtagacctccgaggcatgaaaccaaattggtttttggtcatgcttgtcaaccttcttaagcggtgttcaatgactctctcccatagcttcatagtatggctcatcagcttgattccgcggtaattagtataactttgaacatcccccttgttcttaaagattggtactaaaatactccgcctccattcttcgggcatcttgtttgaccgaaaaatgaggttgaaaagcttagttagccatactattgctatgtctccaaggcctctccacacctcgatggggataccatcaggacccatcgccttgcctacttttatcctttttaacgcctccttaacctcacactcctggatacgtcgcacaaagcacatgctggtatcatcaaaggagtcgtctagctcaatggtagagctgtcaccctcttcattgtaaaggttgtcaaagtactcccgccatctacgcttgatcgcctcgtccttcacaagaagctgatcatctccgtccttgatgcatttgacttcgccgacatccctcgtcttcctctccctaatcttggccatcttatagatgtccctttcgccttccttagtgtttgaacgttggtagaggtcctcatatgcccgacctctcgcgtcactcaccgcccgctttgcaaccttcttcgccactttatacttctccatgttagctgcactcctgtctagatacaggcatctgaaacagtccttcttctccctaataaccttctggacctcatcgttccatcaccaggtgtccttagcttcccttttacttcccttggtcaccccaaactcctctacagtgaccttccgcaggaaggtcgccatactcgtccacatcaagtttgcatcgcctccttcttcccaagggccctccttaatgaccctctccctgaaagcctgggatgcctcccccttgagcttccaccacttcgttctagcgacttttgcgcgcttatcccgttggacacgaatcctaaagcggaagtcagcaaccacaagcttatgttgagggacaacactctctccaggtatcgctttacaatcaatgcaagcgcgcctgtcttctcttctagagaggacaaaatcaatctggctagagtgtagaccactactgaacgtcactagatgggattctctcttcctaaagagggtgttagctacaaccatgtcgtaggctagagcgaagctcaggacatcttctccttcttggttcctgatgccatagccaaagcccccatgcaccctttcaaaacctgtgttagatgtacccacatggccattgaggtctcctcctatgaagagcttctcaccaataggtaccctcctaaccaagtcctccaggccttcccagaactccttcttggtgctctcattgtggcctacttgcggggcatacgcgctgataacattgaggactaagtccccaactaccagcttgacaaggatcatccggtccccttgcctcttaacgtccacaactccatccctaaggctcttgttgaccaagatgcctactccattcttgtttgaagttgtccccgtgtaccacaacttgaagccggtatcctccacctccttcgccttttgtcccttccatttggtctcttggacacataggnnnnnnnnnnnnnnnnnnnnnnnnnnnnnnnnnnnnnnnnnnnnnnnnnnnnnnnnnnnnnnnnnnnnnnnnnnnnnnnnnnnnnnnnnnnnnnnnnnnnnnnnnnnnnnnnnnnnnnnnnnnnnnnnnnnnnnnnnnnnnnnnnnnnnnnnnnnnnnnnnnnnnnnnnnnnnnnnnnnnnnnnnnnnnnnnnnnnnnnnnnnnnnnnnnnnnnnnnnnnnnnnnnnnnnnnnnnnnnnnnnnnnnnnnnnnnnnnnnnnnnnnnnnnnnnnnnnnnnnnnnnnnnnnnnnnnnnnnnnnnnnnnnnnnnnnnnnnnnnnnnnnnnnnnnnnnnnnnnnnnnnnnnnnnnnnnnnnnnnnnnnnnnnncctaaggctcttgttgaccaagatgcctactccattcttgtttgaagttgtccccgtgtaccacaacttgaagccggtatcctccacctccttcgccttttgtcccttccatttggtctcttggacacataggacatcaacacgcctcctcaccgccgtatcaactagctcccgtaacttacccgtcagggaccctacgttccagctacctaagcgtatcctcctaggctcggctaacttccttaccctccgcactcgtcgagtcaaatgcgaagacccttgctcatttttcactacaccggggcgtcggtgcagcgcgccactaaggatgcggcgacccgacccttgctcacttatcaccgtatccagatcaagatacggcgcgccaccaagggggtgacggcccggcccttgcccatttgacaccacacccgggttccgatgtggcgcgttactaagagggttacgccccaacgagtttcctttgggtttcatctccataagagtggctgggtttttcacgttggctcgccacgcctatcacaaccctcctcctttacccgggcttgggaccggctatgctgagacaacatagaataagaaataaactacataaaatctatttgcctaactatgctaattatcagatttttttatttgcattagaggttgtcaggtttcctggtgtgtatttaggtgtttggagtttgaactaaacattagcatatcaggaacttgcttaattgagctagttaggtccatccattagctaaatgatggaaaattaatttgacatggaaggtgctgaattggtatgcgaagcttgagattcataattagtagaggcaaagcatccttatattcaatactgtactctgccacaccatttttctgtcacattactaatgataggcctaattagtgcaattgagcaagctgaggccttgagggagcctgcaattctgaaattgaagttaaggaccttaatgtcagaagtgggcatgtttgaggaactcatttttctgtcacagtattgaagatgggcctaagtagtaaagttaagcaagctgagaccttgatgaagtctgccaggctaaaatcgaagttaagaaccttaatgtcacaacccaactaggcaaagtttgagcacctgtcctgcagcatatatgtttgatacacgcaacttactttttgaagcgttacaaaagaaaagctattccgcagcagccaattgcaaatttggaacatgaacacctttaacttaccattggagttattgatccggtggaatttttgtaaagaaaatggtctgactatttgcctctatatttcactttactcctatcaattctatatagatttatacttttgacaaatgcaaaggctgcctgttatcatgacaatggtgcatgcaatcactgtagccgtggagctagccatacgtatgatattgtgtttgcagtgcatgccggtataagtactaaatactctctgttggtgtggtaggttggtgtcattggaaatttggttcattcatccccaaatatcaagaaagaggttcttaatgcgggggccttgcaacctgtaattgggttattaaggtatgatgatcgtcatatgcagcttatgatgatagttttacattgtatctgttaataattgaatgcatataacttactgtatttatttgttgagttctgctaaagtactgctggaaattcaaattctatatacttcactcttagctgtacatgagcatgcacactcgattactgatgacaccattgtgcatgtgttcctggatgctgattaattttgttgctttagggtcagaacaacatgttgattataatgatataatcttatgagattcaagtgtaagcttgcacgtagcaaattatcttctaacccagattccatatccttgtccatattgtaacacgagaagctgttttattgtagtcccaatcttagtatatggaggcatgatattgccctgagtctgctctccatcttattcaaagaatctgtgcttcatcttctcttttgcagttcctgctgtacagaaagccaaagagaagccgctttgttgctagggcagtttgcttcggccgactctgagtgcaaggtgcttaaggatgcttcatttgttgttaactacacatttttttatgatgagatgaagtggaagagtaaacaataaaatgaagtactttttcctatgtaatattcttgtgctacatatcattcatcattgattatgtgttacaaacataagacattgttatgtctacctacttactactccctccgttcctaaatataagaccttttagagattgcactataaactacatacggatgtatatagacatattttagagtgtacattcactcatttttctccgtatgtagtcttctagtgaaatctctaaaaggtcttatattttggaacggagggagtactaaatatgttgtttcatatgataaagagttagccatggtgaatcataagaatacaggatggtgcgttgagctatcctttctaaatatgcatatatggggtttgacaggtccatattgtgcaacggggtgcagtccgaccactaattgacatgctccagtcagccgactttcaactcagggagatgtcagcctttgcccttgggaggcttgcacaggttatatttctcattctatgctccccttgcactcaacaaaaccaatctgattgcttatgtttgtctgcgggttttactgcatgtattttaggtaggtattgtagcagtgaaagagaaacaacagtggcaatccttactcccattcataaaatcacctgacatagtgacaaagcactttctcaactttgctgcttcccttcttctctatgttgattttacattaggatgcaaagataagttttggagcgaaaaatcataattagtgtcccctcttaaaaggattgacataagattgaccacaagttatgtttaatgtatcatcaacaattgaagccgtgcagctcgttctctttatatgtgttagtgttaaatatccagacggacttttgaggagcccttgtctttttgatttggtgatggatgaggtcacaagggatatacaaggagatatcccatggtgtatgctctttgcggatgatgtggtgctagtcgatgatagccgaacgggggttaatagaaagttagagttatggaggcggactctagaatcgaaaggttttaggcttagtagaactaaaactgaatacatgaggtgcagttttagtgctactaggcacgaggatggagaggttagccttggtgggcaggtggtaccggagagagacacgtttcgatatttggggtccatgttgcagaaggatggcaatatcgatgaagacgtgggccaccgaatcaaggctgggtggatgaagtggcgccaagcttctggcgtactctgtgacaagagagtgccacaaaagctaaaaggcaggttttataggacagctatccgacctgcgatgttgtatggcgcggagtgttggccaaccaagagacgacatatccaacagttaggtgtagcagagatgcgcatgttgagatggatatgtggccacnnnnnnnnnnnnnnnnnnnnnnnnnnnnnnnnnnnnnnnnnnnnnnnnnnnnnnnnnnnnnnnnnnnnnnnnnnnnnnnnnnnnnnnnnnnnnnnnnnnnnnnnnnnnnnnnnnnnnnnnnnnnnnnnnnnnnnnnnnnnnnnnnnnnnnnnnnnnnnnnnnnnnnnnnnnnnnnnnnnnnnnnnnnnnnnnnnnnnnnnnnnnnnnnnnnnnnnnnnnnnnnnnnnnnnnnnnnnnnnnnnnnnnnnnnnnnnnnnnnnnnnnnnnnnnnnnnnnnnnnnnnnnnnnnnnnnnnnnnnnnnnnnnnnnnnnnnnnnnnnnnnnnnnnnnnnnnnnnnnnnnnnnnnnnnnnnnnnnnnnnnnnnnnnnnnnnnnnnnnnnnnnnnnnnnnnnnnnnnnnnnnnccaagcttctggcgtactctgtgacaagagagtgccacaaaagctaaaaggcaggttttataggacagctatccgacctgcgatgttgtatggcgcggagtgttggccaaccaagagacgacatatccaacagttaggtgtagcagagatgcgcatgttgagatggatatgtggccacacaaggaaggatcgggtacggaatgacgatatacgagagagacttggggtagcaccgattgaagagaagctggtccagcatcgtctcagatggtttggacatattcaacggaggccaccggaagcgccggtgcatagcggacggataaagcgtgctgagaatgttaagaggggtcgtggtagaccaaacttgacatgggaggagtccgttaagagagacctgaaggtttggaatatcgacaaagacttagccatggacaggggtgcgtggaagttagctatccacgttccagagccatgacttggcttcgagatcttatgggtttcaactctagcctaccccaacttgtttgggactgaaaggcttggttgttgttgttgttgttgttgtttgtatatgcttcttgactgtatccattgtcctgcgacaagtaattgtagcccagcatagtttagcaaatctcttcaatattcgcatttttgtatacactgaaggaaaagactccattttcttcctaacagtttcttgggagtgggaaacctgtttgacatgcatgatgaagtcactcatgcaatcactattagaatcgacgaaattgcacaagagacaacttctccgccagattatttgattagttttacttttacgtgagagataatccccattcaaatacaaccagatcaaattaaactgcagcattgcacacatgcagattgatatacagttttacagacttttgtacataaatcagaatacagttttaaaaattaaactactctctctgatccatgttaattgacgctagtttcaattaatatggattgtagggagtaacatctttgatctacataggtcccaatggtcattgtcatacgacatatcatgttggattttttttttgcctaccaggtgttatctggactccacgcagtacagtgccacattcagtattcgttagcgagcaagagtttagatatttcagtgtcagacacatgccaagttattcccttctcattgtcttcctaagctgcaaacatgtcaatcatgggataggaaaataaaacagtattcgattagttttagtgtgttacctctttgtttggagtgggcatgttttatttacttctttaccttaattaacctgtatggctaatttgagagaaaatcttttgtttcacaggacacacataaccaagcaggtattgcatacaatggtggcttgttgcctttactaaagcttcttgactcaaaaaatggttctctgcaacataatgccgcgtttgctctttacggagttgcggacaatgaggtagttcatgattattcaaaagttcggtttctacttattatttcatattttttcttaaaagcgaatgaactcatgtagtcatgttccatttctgttttatgtaagcttctcactttcatgtatccataataacttttttttataggattatgtctctgacttcgttaaagtaggaggtgtccaaaagttgcaggatggtgaatttattgtccaggtatgtcaaccatcatagcatagattggtactactttcttaataagtttatacctgagtttggttaagcaccttttttcaggctacaaaggactgtgtagctaagacactgaagaggctagaggagaagataaatggacgagtaagttctgctcactgtttcttttttcttttatttgccaagctgtggtatctactccagctgacttacacatgatctttaacaggtattaaaacacttggtttatctcatgagagtaggagaaaagtctgtgcagaggcgtgttgctctggctctcgcacacctctgtgcccctgaagatcaacgaacaatttttattgataataatggtatgaacaatttgacagcttaagtgttccttatcctgtgttttgttctccatggattaaattctggcttaattcaggtctcgacttgcttcttgatcttctggtttcggtcagctcgaaacatcaacaggatggttcggttgcactatacaaattagccaacaaagctgcagcactctctccgatggatgctgcacctccatctccaacgccacaggttagtagaaaataaaaacagggcgatttttggactacatacggagcaaaatgagtgaatctgcactttaaaatatgtctatatgcatccgtatatagtccatattgaaatttctacaaagacttatatttaggaacggagggagtagttatgctattgaagtgaacaaggtcttcacagtgcttagaaaagagatttgtctaacaaaattgtcctaaaaaattagagttctagggatatatgcaaatctgaagctattagcaagatctgaattaaatcaagagcatgtgtgcacaaacttccttaaaatgttatttcctacaaatcgtggcatgtgcaacctgttggacacagatattctgtcatatatctttactagcaaatatgcccgtgcgttgcaacggggaaaacaaatctttgcatgcgcgtagcagcccatccatgttgtcacttctccacttcatcaacatcgctggtggttgtcagtcatccaccaactaacgacgaccatgatcaatcccaaagtgagcttggtcatcatactttaacacaccattttgcaagcccctcctttgtcacattgtccaccaattcaaaatgaatgtggtcaattccatagtgatgagtttggtcattgcacaatagaatgtcatccccgtgagcacctcgctatactaacttattgtccgattgaagagaagctggtccagcatcgtctcagatggtttggacatattcaacggaggccatcggaagcgccggtgcatagcggacggataaagcgtgctgagaatgttaagaggggtcatggtagaccaaacttgacatgggaggagtccgttaagagagacctgaaggtttggaatatcgacaaagacttagccatggacaggggtgcgtggaagttagctatccatgttccagagccatgacttggtttcgagatcttatgggttttaactctagcctaccccaacttgtttgggactgaaaggcttggttgttgttgttggacaatgatggtgttcgttgtggtgcggagagtaatagaggacatgtggaggccgcaccatggctgcatcagtagaatcacaaggaccacatatactatatgaccaatctccctaggattggaggcctcacaatcaattgaggtctccaattggaatttgatcatccgattttgattgggtcaacaatttctcaaacccttttatttaattttttatacggtacaatatgcttcctaatttttaaatcttcacaattaattgaggcttcaatttagactttggtcacccgattttgactgggtcaacaatttctcaaagagctctcctatttaattattttagttctctatgctctgtaattttaaagcttttcattcgactgaggtattcaattttgaatttggtttacgattttgatcgggcccatgattttccaaatcaacgacaactggcctatagaaacatatcaacccctcacagactcctatcacccatacaaaagcgtcatcatgtgatactatagcatgaatatagtatatgcaaccaatgatgaaaaaatatttccacatgaacatgtattgattagcggataacacaaaatcacaccgtgaaagacccaccaaataactgcattataaataaacgtaaaacacactccatcgtctcccacaccggccaaactaaatactccatcagtttcaaaatataagggttattagttttttggaaagtcaaatttctttaatttttgaccaagttcagagccaaaaaatatcaacatccacaatattaaacaaaaaatatgaaaattcatttcatgatgaatctaataacaccgatttgatattatgaattttgatatatttctctataaaatttgatcaaacttaaaaaggtttgacttataaaaaaagtaatacaccatatattttgaaatagagtggctaaagaaatttaagaatcctcacaaattcaacggcgcagcaaagcgcgcacaacccttgtagtatccaaaccaatgttagatgcaaattgcgcttgtataattcacttaacggacaacataaatagagcatgtatgcaaatagctaggtcgctagttggttgccgaggttagattgatgttgtgattgttgggtcgactccaacccacacatcaattgtttagcagatttattttgagccaaattgtttagcagatggacattggtgaagcaaactgggctgctgaagaacaggttcatgttaggtccaacggagcgatagaccatacagcgagaaaacgaagaaacatatttggcggtcttaaggtcctacgcaaaacaaaaacacacgagacgaacgaacgaacattcgaaaaatcatacggaagaaacattcctccctttaattcccgcgtgttgcaattttgagttaaatgtacccagtcaattgaacaacatcctttaatattttttaaacacgtacgcccttgcatgcgtgggctgccataatgggccaatcgatgatgctcctttaatcaccctacaaccttcccgtgataccagtctccttcacgctacagtccctcctccacgtgatgtttgcatgcatggccccgtgatttattttcctttgtggcagcctcacaatcctgggatttacaattaatttcttgctcatatattatatatacccatacaacgcatacaacagtgcgtttgttccctctgcctattgatctttcaggtgccttgcagatttcaagtcataactgtatttaaattggtgtgtctagatgtgaagtaccgaggtggtgctatctttgatgtaaccatctctcaaaaatacgtaatggggggctagctcagttgtccgctcacatttgcagttgacctcacgtcgggagtttgatccctcatgcacgcacattatttttgcgccccctgccggacggtatcggttgtttgggcagtcgtttcagccgggtgggctgcggcttcagccgggccgtttgccacagcatggtcgattgatgggttgaggcccacgcgagtcacgaaaggaatttcagggaaacgtttagcgcggatgtacaatcagaatcctattacaatgtacggacgaaaagattagcccgacggtgaacgtgcagaagcagtagcccttctattattaattaggtaaagattattaattcgttaattgtttgggcggctttctgattctggaccggtatgtataaaaattgatgaaaaaggaggagcgatgtgggactatttaataagcaaacgactctaccttttatacacaaaattgttttagctaagttggtcattggcttccagcctatatgggtgggcttgagttcgatccctcacccaagcaaataaatttttgcctcctgcgcagcatgattttttgccacatatgggctggctaccatcacgtgcggcgtgttaaggcccacactggcgacacataaaaagaaaacatgcgtttgactgtgggtatattcttcaaaatatcaaggattttttttgtaaaacacgtatgacggactaagaatacctatttcttttattagtaggtatagaatagatagatactgcttggcagtcctgttcttagtagttgtcaggctttaccttgccctatcctgggtattcttaatgaggtttccccataaattaactcctattaccgatggattggtccatccatgattctggctattgctattactaaatatacttctgattgcaggtttatcttggagagcaatacgtgaacagttcgacactttcagatgtcaccttcttggtggaaggttcgtggcatttctgcaccctgccttcacagaaactactttagatagttgctgatttttcattaggaccataataatcacctcccttgtgatttgcaggaaaacttttttatgcacacagaattgctttgcttgcttcttcagatgcattccgtgcaatgtttgatggtggatacagggttagtctggacataacatgctattcctttttttggttggaagatgtggatcttgtttgctagttgaacaatttctgtttacaagaaactcactattttctcaaccaggaaaaggatgcaagagacatagaaattccaaatatcaggtgggacgtgtttgaactcatgatgaggttagtaaatcattgaccattcttgttccttggccatggtcaacgggtaaatccgcatgttagttcctttttctcttacgggacaagacctgcaattgaagtttggaaacatcttctttgttttgtgcagatttatctatacagggtcagtcgaagtaaccaacgagcttgctcaagatctcctcagagctgcagatcagtatctgttagaaggcctcaaacgcctatgtgaatatacaattgcgcaggtgatttcagggaacatggctcctaagttctatgttcgaactgctgctgactgggtctaatttattgtattcaatatcttgcaggatgttaatttagaaaacgtctctgatatgtatgacttatccgaagcctttcatgccatgtcactgagacatacatgtgtcttgtttattttggagcagtttgataagatctgcaccagacccgggttggtatctttaacttagggtcgccacatttggtacataatgtaacacacttcatcaagtgacagaaatccatctaactggccatcttgctgtgcagtttttctcagctgatccagcgtgtcatccctgagctccgcaacttctttgctaaggcgctaacgccaagccaccggagtgcgcaaccatga

SEQ ID NO: 125 - protein, 742 aa, Hordeum vulgare
MEAEQQKPQRPRRKAQKRRIDDEAAASAAAAAAAAAAAAAAAAAVSSPLGSADADDDNEDDEGSVGTEICCRQSQAAVAREVRTQVDALHHCFSWRHADRATAKRATSVLAELAKNEEMVNVIVEGGAVPALVCHLKVPPMEAAVEEEQQPRPFEHEVEKGAAFALGLLAVKPEYQQLIVDAGALPLLVHLLRSHKNATNSRAVNSLIRRAADAITNLAHENSNIKTCIRIEGGIPPLVELLESQDIKVQRAAAGALRTLAFKNDENKTLIVDCNALPTLILMLRSEDAAIHFEAVGVIGNLVHSSPNIKKEVLNAGALQPVIGLLSSCCTESQREAALLLGQFASADSECKVHIVQRGAVRPLIDMLQSADFQLREMSAFALGRLAQDTHNQAGIAYNGGLLPLLKLLDSKNGSLQHNAAFALYGVADNEDYVSDFVKVGGVQKLQDGEFIVQATKDCVAKTLKRLEEKINGRVLKHLVYLMRVGEKSVQRRVALALAHLCAPEDQRTIFIDNNGLDLLLDLLVSVSSKHQQDGSVALYKLANKAAALSPMDAAPPSPTPQVYLGEQYVNSSTLSDVTFLVEGKLFYAHRIALLASSDAFRAMFDGGYREKDARDIEIPNIRWDVFELMMRFIYTGSVEVTNELAQDLLRAADQYLLEGLKRLCEYTIAQDVNLENVSDMYDLSEAFHAMSLRHTCVLFILEQFDKICTRPGFSQLIQRVIPELRNFFAKALTPSHRSAQP

SEQ ID NO: 126 - DNA, 10123 bp, Musa acuminata
  source 1..10123: mol_type = genomic DNA
tctgtctctctcttttcacagtcgaattccttcatctctctgttctgtgtttccttgggaccgatggaggcggagcagcagcggccgcggagaaaggggcagaagcggaagctggaggaggacgtcgccgccgccgtttcgtcggcggcctcggtgccggcggcggaagagggggacgacggggaggcggaggatggaggggaggcgggcggggacgagatctgttgccatcggtcccagaagacgctcgcccgcgaggtcaggacccaggtcgaggtcctcgagcggagcttctcctggcgcctcatcgatcgcgccgccgcgaagcgcgccacccacatcctcgccgagctggctaagaatggtccgccgaaccctttcttcctttcaatcagtttgctcgtccgttgatgttgtgttgttctggttgctgtctgctttagggtttttatttcttattgatgcttgatgttgatagatctgtttgccgatcctttctgcagaggaggttgtgaatgtgattgtggaaggaggggcggtgcccgcccttgtaaagcatctggaggagccgccgcctctgctggcaagggaagggagtgccgccggaggagatcgccccttcgaacatgaggtcgaaaaagggagcgcttttgctctcggacttcttgcagtgaaggtatccacggtagcacttttttatactttttcatgtggacaggagacctggaagctcttacgatcttagttgagacaaattatgaggatgggacaagggtcctctttttaactgcgatctaatatatgtaaaaatgaagtcctgtttttaggtaagcaatgcaatttcagatgtttgcaaggtagggatatgtagattttcagtgttcgaacatgggttttgtagattttcaccggttcacttgctatagttatgtattcgatgttagttgattggctgcttgataagcttgtggttagtaatttcactgagttacacgttttgcatattaagagggaagataatatgagataaaattgttttcagtggttttttacatgccttctctttaaaagttggcatggttaacaatttatttttcatcttgtttgtgtcaatttgtttttagcgctctgttcttgaacttgtcctacatccttttgtatttgtggtaggaacttttcttaactcatccggtatcagtttataatccttagattgtcttctgatgctggtctttgtatcaacttctactctcttacatagactaaacattcttaacactatttgttgttaagttcaaacttctcttccattccaagatgcacattacaagtggcataggttgtaatttgaagatatttagaagtttagtggttttttttgttttgtcatcctgttatgaagattttgctgtatgcatttgtttttagcagaatcataatgtatttgcacaatttaatagttattcatgctttcacataattcaccaatattttgtgtcaactaatgtataacttctactgcttctttgatagattgcttcatagtatatgaatattattttcctcttgttggagttgttccattcttttcttgttgttgctctaagtgctttttaatgattttaacagcctgaacaccagcaacttatagttgatgcgggtgccttgcgtctgcttgttaatctgttaagaaggcacaaaaaaggttccaattgccgagcagttaatagtgttattaggagagcagctgatgcaataactaatcttgctcatgaaaatagcaatatcaaaacttatgtcaggttctttcgcacaaaacttagttttgcttttgaatatttagcatatcatctttttctgattgttgtctttaatgctttctagaattgaaggtggaattccaccgcttgttgaattgctggagtctacagacctgaaggtacagagagcagctgctggtgccctgcggactttggcattcaaaaatgatggtaacaagaaccaggtcattctgctaactgatttaaaatttatacttttaatttggaaatatttttgctgctatttcatttcaaattaaatttgcagattgtggaatgtaatgctcttcccacgctgattctcatgcttcgatcagaggatgctgccatccattatgaggcggtgagataatgcagatgaaacacatggcctgatatcttgcacatttagacaaatattttaatttatttgaatataatgcatttgattcgtgaagtctgctcgatctgcacctggattagttatgatgaattggatgcatgtaaggtgaatcctagtgcttttggaggatataaatgtttagagcattatcctatcagggttggcaactcaagcatgtttgttgggttgagcgctgttaatattcagatgatcttgaatgtgcttaaccccatcctgttgtacaagcaatcaagtaaattgaaaaggagatccatcaacgttatttattactatgttatagtttggacaccattagagtattgaagaaaagtatacctatactcaacaacaatgtaatctagttgcatactctttagtgccatctgcttcacactcttctccatttgttgttctatgatcttgataattttgtccctttttcctttctagttttggacttttattccctcctttgccaccaagtatctatcaactaatttacaatttccttccccgcttcacacttcctactcttgatgactctgtcaatgatagtgctacatatcagttgctgagaaggaagagcacttagcttatattgtggagggtgacattaggcttgcagtacctttcagatgatattactttctcttctaatgagagatggattcatgttgatccatgtctctcttgtgcctccctattctcccattgcttttcttgaaccagttggttccagcttccaatatgagtacaatcaatttattaaattgggtatttcagagctgcaccggtaatgcttaggttagaaaaatagtgattagtgtcaatcatgttttttcagttcagtacatctgagctgactggtccatgtcatagatgtgcaactatttttaatatacatataaacttttcacatcctgaactttcttaagtcataagtgtattgtaacttgacttgttgataacagtgtgtagcaaagtttgttaggtagaatcttataacttgcaatatagtaaattgcctaatcagtgatcaaacagtagttggaattcaaaacagtgacaaagtaatgaaggtcaacaatatctacaagagaatatcacacatctagataaccttcatgattcgatgagtcatcaagcaatgcctaatctttcaagtaggtagagggaagtcatgtaggtatttgaggtttatgtaatagcctccattataatcagttttggagaagtacaacatttttcagagtcatgattgtttacataattactgtggaaagcggcatacttgtagtctaaaacattgttacattgtaacatatagaggtgaatgatttaatagactcaacaagtgacactcccttaagttatgatggaagttcaaattgattaacaaattgtcatattggtgtctctgggaaggaacattttgctgaataatcttcctgaaatcatgatttagagatgcatcacttactggagacaagctgatgacaaagctatgaattagctcatgcaatgtgacaatcttctggggatgcagtacataatggaactgttgttcactgcaataatgctcatgcagctttacagacttacggtggacgattcatccagctttgaataaaaaaatacattgaattattattatctattccttggatgtcatgacaaactcatgttatctatattttaaaggtactcatgtttcttaattttttgagatttattctttttcaatgtccagctaaccagttgattttctcttgatattcaggtaggtgtaattgggaatctggttcattcatcacctaacataaagaaagaagttcttcttgcaggagctttacaacctgtaattggcttattaaggtatatctttggacttcattgccctgattaaggtagcatgactcatttgtcaataggtgattgtgaaacctcttttgttattttatcatttattattttcaatttgtgcttccttagttgttgtaagaatgtgatgaacaatcctgaactgcatcttaacttattcatttataagttggtgatttgactttcaataaaagctgctatgctggtaggattaaacttaattctagaacgagatcaggaaatctgaactttatatctgattgaaaataaaaggttatattatgatattttttgaaagaaaactaaagggtttcttttccttctgaaaaatcaagcttgtaattctctttcggtgtgaattttcaattaatttaagcagtgttctgagctggtgagggtcaacaaagatctaaagattagcttgtattttttatcattggtatggctggcaatgtgattgcagaaatagagttaaaaactaatgtaggttatggtaccactagtaggaaatggaggaagaagtgtcgcccacttcaagttggcctcctgattttgctgtggttaacattggaatgaacaacctagtgttctgtttctttaacaataagcttttctgcatttacttcaacagattagactctagctgtctgacttcccagaactgattcctttagaataaaaggatctttcggttgtttaacttttccctcctgcttctcctgatgaatatggaatagaaaaccatactgcattaaacagatgcatgggtgcagatttttgataaattttagcaatgtcatttacccataactgatcagccaagttatttgatttctcatttcaattagagaaatttgaagaatgataatgtgaattatgtgaagattgattgtgtgagttgtgtcttcttgaagtgcaaatgtagtcttgataggtaaatgctatgatgtatatgaccccaattcatctcaaattggacataatcaactccaactggattaggccagttcaaagctacccgctcagtttggcccgggtgattggcatagctagttcgatggtgttcagcatgctatgatgtatatgatgccaagttctttaattgacatctgtgggcgaatagttatcatatgtttaactgttatgctatttctgaacaagcaaaatgacctaaggtgtcatcattcatatcatttgggatttaactttcccaagtactcaacagaatcagatggcagtgacacactgccttttacactattgctacagatctttgactttagtttgcaagtgggaagatataattgtgtgataatgatggcaaaatatgcacttatgtgcttgataagtacgtacatcgtgttgtaatttcaaattagattcatcatagaatgtttgggttggttaaatacttctttctgcattcctttaaactgagcaagtaattaattacagttcatgctgcacggagagccaaagggaagcagctttattactagggcaatttgcttcagctgattcagattgcaaagtacttcattgaacgcttttcttctttgttctatctgaaggataatattgatatgggttaagttataatctcatccatgtacctgttctgctaccttgactttcttgcaggtgcacattgtacagaggggtgctgtacgaccactgattgagatgcttcagtccccagatattcaacttaaagagatgtctgcctttgctcttggcaggctggcccaggttattgatatatgttaccgttcaatctgatacctatcatatcttaatttttctattttactagtgtttattttaaagctagctccgttcatcattgctattcttgccattttttgttactatttctttgtatatggaagattcggataggctattatcaagaataactcattcagttatttcatttctcttttcatgtatgttcatgcttttgcagctttatgtgctttctttagcacacttatagttctaggttaaagcattaatttgaaaatttgaaatccatgagaaggaatgttcaggggaaaagaaagcttcctacttcagatagagcttccggacatatgacttgtaatatattgggtcatagcactgcttaccaatttgaagtttcaagaacactattgctatttagcaatgtggttcattgggccatggcttatttttgtttgggctgcgcctccattgtgcactttctagcattggatataccgaattgtagaatatttgtacccttactcactgtttcacaagtctagtttggtgtcaaatgagttgacaacaaatttaagttttttcctctgattctctgcttagattgatttttcatttatactttgaataattcttcattaaattcttagaaaaaaaggaggattaagtttaatctttctataacagatatttgccacattttgaaattattcgacatgctccttttaaatgctttctatgatcttttgtgcttgtagttaagataatatcctttggtcataaaaaacttctctttttcctgtttaataatttctctcgaatttgttctggctggatttgtttcttaagcttccatgtggtcaatagtacctaatttctggcgtgtctcaaagaccctttttctttataggactcacacaaccaagctggtattgtctacaatggtggtttggttcctctgctgaaacttcttgactcaaaaaatggatctctgcagcacaatgctgcatttgctctttatggaattgcagacaatgaggtgaatctacatcaaatgttcctttgttctgacttgattctctgttattttttataatgctagaagttcagataggcttactcttgtctttttttcaggataatgtttctgattttatcaaggtaggaggtgttcaaaagctccaagatggtgagttcattgtccaggtatgttgatgtgatgcttcagatcaatgctttcggttgtgagtgtcaatcttgttttgttttaaatcgtgcattaacaagatatataagttcaattgcaggcaacaaaggattgtgtagcaaagacattgaaaagattagaagagaagatcattggacgagtgggttttgtttcttaggtcctttgcattgtaaattgattgacaaacattgactttccaagttttaaatcatgtttacttctgatagtaacatcctgtaccttgcttttttgctctttcaggtattaatgcatttgctatatctgatgcgaatcggagagaaggttgttcaaaggcgtgtagcactggctcttgctcatctatgctcacctggggatcaaagaacaattttcgttgataacaatggtaactgttacatgtccagttatccgtatcgtcctttcaccactgatatccttttcatttctcttttgtactttaagaaaatatctttgtttgttaattaacaatttctcaatgtagggcttgatttacttctagatctactggggtctactaatctaaaacagcaacaagatggttcagttgctctttacaagttggctaacaaagccatgacactctcttctatggatgcagctcctccatcccccacacctcaggtttgttaaaacaggcattagttagctttgctacgagttttaatgattaaaatttgttccataatcatggagatacaaataaaaagggtcgggatttcaatgcttaaaacttgtatacttaaaaaataatcttttatttaaattgatggaattatcttctatatttgttgaatttcacagttgtcactatcaaggtattattaagcaaagaattattacttcacaaatatagcctttattctaatgggaaaatggttatttttatccaaaatatcatttcttctacaagaaatctgtgctacaaatgtaaaatatgattttggattataattggaatcataagaaaactaggtgataaatatattccttcaggtaagggatagacaactggcattttcatagctaaaaaggagttactaatgcagcattattgttcttatattagtgccatcatgtgtgtttgagttttcacactgagatggttgttgaaattaatgtgggtgcctttatctttttattttcctgatcacattgaggaaggaaagaaaattattcacatcgaatgtcatgattattattttaataatttaaagatcctggattctcagtattggtgttcttacactggacatcccggtgtacaaggattaacttcatattggaacttgttcatactacaatattgagaaatgcatgaattatgcaaaggtcctaaaagctaattaccagtttgtcagaagactcagaacagacagctgtatatatctatgaatatagaagcaactatatcttatcttggtgacatcctccttctaaagtgcctggtagaaaaacttcaattatgttgtttggatttgcttttgtgagaacagaatagtaacgtttgttattgtttccaatcaatgcattgtacgtgttactagtcatttgtttcctgcaggtttatctgggtgagcagtatgtgaatagctccacgctatcagatgttacctttctggttgaaggttgtagaatattcttactatgctgttattttccatcaaaaaatgtggataacctttaaaattttcataaagtttttcacatttcatttcccattcatgaggatgctatcagttatttgctacatattaaaatgttttcttttcctgttctcttccaggcaagcgcttctatgcacacagaattgctttgcttgcttcttcagatgcatttcgtgcaatgtttgatggtggatacagggtaaggaaactcttaattcttaccatgtttgtttttcctctataattaggctttactcacattcaggtggataaataattgttcttgcaaagttatggtatttacaagccccaagaatgtcagcgtatgatatgttcggaaactttttctactaaacaatgtcagagtatgaatgacgaaagttatattttttttaacaagtcgcttctggaaagagcaagatatcgtagtacctgttctggcctagtaagatctgattaaaaatgtcttacttttcctgatttgttacaggagaaggatgcaagagacattgagattcctaatataagatgggaggtttttgaattgatgatgaggcaagtgcagttactcttcatactaatgatgctttgtgttatggggtttgacatttgggtgttcgtttgcagatttatatacacaggatcagtcgaggttactactaatatcgcacaagacctactaagagctgcagatcagtatcttctggagggtcttaaacgcttatgtgaatatgctatcgcgcaggtgaatagatgatgtatttttccttcttttcggaaattttgttcagctagtaatagtagttatgtattaaagctgaaatattctttgcttatgcaggatgtcaacatagacaacatctctagcatgtatgaattgtcagaggcattccatgccatgtccctgaggcacacttgtgtgttgtttattttggagcaattcgacaaaataagcattcagccagggtactttctactctgctgtttcttcaaaatttcttaacttggtctacacgaactcaagccatgaccctaatggatttctgtaggcattcccatctgattcaacggatcatcccggagatccgcaactacttcgcaaaagcattgcgacctaatccaagaaactcctgatcctaactactcttttctgacaccatctttgctaactcatgctgctggggggactgtatacagtttggaaaagccttctgcatcgagtgatttctattttccaagagcaggtttggggaagaatgttctaagctttctggaacctgtatctcctttttcttggatgctgtttggtacggtacatcactagcatcggagttgaagctaatgacacttgaaatttccactcacttgttattacaaaaaaaaa

SEQ ID NO: 127 - protein, 726 aa, Musa acuminata
MEAEQQRPRRKGQKRKLEEDVAAAVSSAASVPAAEEGDDGEAEDGGEAGGDEICCHRSQKTLAREVRTQVEVLERSFSWRLIDRAAAKRATHILAELAKNEEVVNVIVEGGAVPALVKHLEEPPPLLAREGSAAGGDRPFEHEVEKGSAFALGLLAVKPEHQQLIVDAGALRLLVNLLRRHKKGSNCRAVNSVIRRAADAITNLAHENSNIKTYVRIEGGIPPLVELLESTDLKVQRAAAGALRTLAFKNDGNKNQIVECNALPTLILMLRSEDAAIHYEAVGVIGNLVHSSPNIKKEVLLAGALQPVIGLLSSCCTESQREAALLLGQFASADSDCKVHIVQRGAVRPLIEMLQSPDIQLKEMSAFALGRLAQDSHNQAGIVYNGGLVPLLKLLDSKNGSLQHNAAFALYGIADNEDNVSDFIKVGGVQKLQDGEFIVQATKDCVAKTLKRLEEKIIGRVLMHLLYLMRIGEKVVQRRVALALAHLCSPGDQRTIFVDNNGLDLLLDLLGSTNLKQQQDGSVALYKLANKAMTLSSMDAAPPSPTPQVYLGEQYVNSSTLSDVTFLVEGKRFYAHRIALLASSDAFRAMFDGGYREKDARDIEIPNIRWEVFELMMRFIYTGSVEVTTNIAQDLLRAADQYLLEGLKRLCEYAIAQDVNIDNISSMYELSEAFHAMSLRHTCVLFILEQFDKISIQPGHSHLIQRIIPEIRNYFAKALRPNPRNS

SEQ ID NO: 128 - DNA, 6778 bp, Coffea canephora
  source 1..6778: mol_type = genomic DNA
gttgtccgcccgatatagaggttgcgaaacggaagaacattttactcccacttcacactaaactcaaatttatttcccaaattgccctctcacacagaacacccactcccctgtctcgtttcacgcaccttttcacatcgtgttctctctcatcatcttcttcgtttctctctcctcacactctcgatggagaaccagagccaaagacgccatgaacaattaccatcaagttcagcagcgaggagaagcttgaagagaaagcttgacgaggatttcgaggacgatcgtaagatcgaagctctctcccctcccgacgctcaccaagatctcgtccgtgaggttcgcactcaagtgcagattctggacgctactttctcttcgatcgaggcagatcgagcctcctcgaagcgcgccattcagattctctctgaactcgccaagaacggtagcgccgaacctgctgatttcttgattttcgtttcatttcgttcttgtttaaacatgattactgaaagttttggcttttaggttaagatttcttgttcgtttgattcgtttgcgtattgatctttgaggatttgtgttgctacagaggagattgttaacgtgattgtggattgtggagcggttccggcgttggtgcggcatctccaggcgccgccgccgccagtgagagagggagacagtgcaccgagaccttacgagcatgaagtcgagaaaggaagtgcattcactctcggtcttcttgctattaaagtaggcgcagaacttttgctcttcatttatagtcggctatgcttgtattttccttgtgcaatcagtatgtaatctgtctttttacacgtagaaaaattaattacagcagcactaaaatttttagggaactaagtaagcgtaagctttatataataggagattttgtaattggtagttgaacgcagtaaaacttatgtccagcatctgagattttctaaccttttttggactagctctttggatggtcccagaaatttgattggtgtaatctccttcactatttgtagactttttatgagcttacgtacagtttaacaagaattggattatgcatcggtaaccagctcgcagaatttggcatctgagtacaaaatcctagtaatagtttcacttgtacttaatcaaagcaatgatggtgaaatggaaagtcgctctaacttatatcaaaagttcccagtgaccaagaattataatttaaattaactaattatccacggcaaatggttacattttgtaagtatgaggcatttgcttaatgcaataggctctattatggtaattgtattgctatttatctgttaagatgcttgtcatgttcttattctctgcattatttaaaattaatgttcaagtcaagaaacaaccctacaagatgagacaaaaccattaattaagaacaccttttgagacattcataaactttgcaattattattgctattatttttttatgcctttaatgaatttgctgctcaatgttgctttaatttacagccagagcatcaacaactcattgtagatgctggagccctgcctcatcttgtggaccttttaaagagacacagaagtggtcaaaactctagggcagtcaatggtgttattcggagggcagcagatgcaatcactaatttggctcatgagaatagcagtattaaaactcgtgttaggtatttcctttttcagtcggagatgcctgttaattctagtatgtcatcctgacttaatacttgtcaatcatatggttaggattgagggtggtatcccccctcttgtcgaattgctcgagttcattgacacaaaggtgcagagagcagctgctggagctctgcgaacacttgcatttaagaatgatgagaacaagaatcaggttgacgaatagtctggtttttataaatttatcttggcagtttttttttctttgcttaaagatttattttgaataattgcagattgtggaatgcaatgctctgcccacacttattttaatgcttcgatctgaggatgctgcgatccattatgaagcggttagtttccctgaaaaattcatggttatattgtgcttcaaatttggtatctccagatgttgaagtcatgccttagctggccactattgttaagatagcaaatcaatgccttcttcaggttggtgttattgggaatttggttcattcatcacctaacataaagaaagaagttcttcttgctggagctttgcaacctgttattggattacttaggttagtcatgatctttttttagtcagcatcattagcttcttttttactttttgtttttattttagaagattaaatttcctatctgattttcaaggccatggatgttatcctcttcaaggtttcactttctcactctcagtgtcgttgcttttgttatattttgactacagttcctgctgttcagagagccaaagagaagctgctttgctacttgggcaatttgctgcaacagattcagattgtaaggttgacaaaagaataaattccctatatagctagtagatgttctatcaattactctcttttaccactcccggttattctttagtttaagttcatgtacgagtttgcaggttcacattgttcagagaggtgctgtgaggccattgatcgacatgctgcaatctccagatcctcagttacgggaaatgtcagcctttgctctggggaggttggcacaggtagttgttgttgaagtttgtcttactacttgctccttggatgttcctttttctctgtagtgtctataagtttaatagttttcaatggttttgctaattgatgtttccctgcagattgtttcctcttttatattaagttacctgttgtagtttcctattcatccttcaaatcaatgcgcattacacgtcttctgtggaatggagtcagtttttgtgtgtttcctatgtctgtataattttggttggttatgttatgactactctttttgcaatgattgctaggttgatgtcaacttttctaagagtattgtcctttgacttcaaatattttatttcatttgttttggggtattaggatatgcacaaccaggctggaattgctcatagtggtggcataatgccattactgaagcttcttgattcaaaaaatggatctctgcaacataatgctgcatttgcactttatggacttgcagataatgaggtatttcggactttctatcagcccagctgaaattttgatttgttatttgaattgcttcttttacttttttcacctgctaagttatgtttaccacccttgtaggacaatgttgcagatcttattagggttggaggtgttcagaaacttcaagatggagaattcattgtgcaagtctgtaccaattttgcaatttacccactagattttctctctttctgaagtgattttacagttatatagcatgtcagctgaaagatttgaattggttttaactttcttgccttctgctgacatagaattcttttaaatgcagccaactagagattgtgtagcaaaaacgttgaagagattagaggagaagatccatgggcgagtgagtcctttttggtagagtccactttagatggtgatgtcaatttgaacaatctaatttccgattttaggtgtaaatggaattattgattactttcagaattttggctatctattggccaagccattgaatgtcatttacttgctgcaatggattttctaatttagaacagcttaatttacaaagtcaatgttgttgagaggtaacctgaataacactattatgtttagaacaatggggacaagttactattgatagttgggagtttattgcaagcattttggtcatgctttcataggaattagcatctgctttatttgttgttatgaatctgcccctcttgattactcctgttttaattggttatatataactctgcaggtattgagccatttgttgtatttgatgcgtgttggagagaaggttgtacaacgacgcattgctttggcccttgcccatctttgttctccagatgatcagagaacaatttttattgataacaatggtaattatctgttccaaaagctttgtaaaattgttcatatagacttttgagagtccatttttattcttttatatgcaggtcttgagctgcttttggagcttcttgaatcgacgaacttcaaacaccaacgtgatgcctctgttgctctgtacaaattggctagcaaagctagcacactttctcctgttgatgctgctcctccatcaccgataccccaggtgagttgtggtggtttatttatccctgccagtttcagctcatggactcaccaatagctcaattgacattgcttagcttgttggaatttctgaaggctatatctctcctgtgctgtttctatgtctccttgtggtgatggaaaaaccagtgtcatttcagtaattgatgtttgtgtgttattaatataaaattctgatgcctctattgaactgtcacaaaaagaggatctaccagtggtgttgatgaggccctctggattatccctttcaatattgatgaaactgttttgtttcaatattgtataaagttctgtacaatcactgaagcactaaagttcatgcttataccttgtcatcgattctgaaaaggatttgatttcctatctaatagtgtgaagttgcaaactctaaatagttcaccattctgtctgggtgagatttgacaatttagccaatcatgttgtcatttgttgttgcaggtgtatttgggagagcagtatgtaaataattctacgttgtctgatgtcacattcttaattgaaggtaagctaacatgctgtgcctctggtgctttttaaatatgttcttgttaatcagtttttctgattgctgttgtcttcacttgttagggaaacggttttatgctcatagaatttgcttgcttgcttcttctgatgctttcagagcgatgtttgatggtggttaccgggtgagtttaatactagtttgaaaatttatttgttttgcaattttgtttgttgaaatgccgaagtcatgccaaaaccgttttaaatacaatgttgaaacatattcctgttggttgctcaacaacggctcttttggatgtctgagcatagatttggtcattggaatctgtgcaagctatctagatatgtattgacacatgatttgtccttcaggttgattcgctgaaaattattttaacagtgttcttaatggtgttgtaggagagagatgccaaagatatagagattcctaatattagatgggatgtttttgagttgatgatgaggtgtgtctttctttagcaaaatttttcagcttctctttaagttgaaggaaactatgaatttgcaaaatgctatatatgcttacattctctgttgcaggtacatatacactggatcagtcaatgtcaatttggatgtggcacaggatcttctgagagctgctgatcagtatcttctggagggcctcaaacgattatgtgaatattcaattgctcaagtaagttcaatttacaagaggaatatctctcttgggcctgtcatatattaggtctgatggtttcttcttgtgtttggaaggatatctcggtggaaaatgtttctttgatgtttgagctatcagaggcattcaatgctatgtcattacagcatgcttgtatactgtttatcctcgagaactttgacaaattaagtctcatgccatggtatggtactatcgcctcctctctctgactcttccggtaaagaatgcttgatagatttattaccataaaaagttaattaaaaaaattgaaagaaactgaaaagtgcttggttcctgcaagtcttacttaggagtgtcttcgaagtggttggcttgaagttgtcaccacttggaggttttgctactggattgcgtgttgggtcttgaactgattgcatcatgctctgctgtcaacgatagacactgcaaactaatcaaaatgaaactacagaaaataagtggcacaaaggccttcactattgccttttcaatctataagcaaatgttgatgccttatgggtttcaggttttttgagctgcaggtattcgcatctgatccaacgcattttaccagagacacggcagtacttcttaaaggcgcttatccggcctacccaagctgaattacggagatagatattgggccagttttgttctttgacttagttgtgttgacagagaaaaagaatgtacagatggaataggtgaaagcaaccattgattctcttgatctggatgcatcggcatttcatggttgaatgcaatctccagaatttgactgattcattatcactgcacaattggcagttgtgaagtctctcagatagaagtgcacagctgagggaagcagaggagccttcaaacagaactgtatttggttaatgtgaagaatgtacctcgcacaagctgaatagccaaatgcattttgtacctgaaaaaaagctatatatatatatattaaaaaaaaagcagaatggtttggtaacttcatgggtgttgtccaataaattaacaactgtgtgattgacaagctgaattggctcttatttttaaatatttaaatgtgaatacgatttgcgaaaggattagaagggctaattttttagattatatgtaaaagaaaaatatcgcacaaatgtatgtatgacagggaggttttctaagcaagaatgaattttgcagggttctttgat

SEQ ID NO: 129 - protein, 712 aa, Coffea canephora
MENQSQRRHEQLPSSSAARRSLKRKLDEDFEDDRKIEALSPPDAHQDLVREVRTQVQILDATFSSIEADRASSKRAIQILSELAKNEEIVNVIVDCGAVPALVRHLQAPPPPVREGDSAPRPYEHEVEKGSAFTLGLLAIKPEHQQLIVDAGALPHLVDLLKRHRSGQNSRAVNGVIRRAADAITNLAHENSSIKTRVRIEGGIPPLVELLEFIDTKVQRAAAGALRTLAFKNDENKNQIVECNALPTLILMLRSEDAAIHYEAVGVIGNLVHSSPNIKKEVLLAGALQPVIGLLSSCCSESQREAALLLGQFAATDSDCKVHIVQRGAVRPLIDMLQSPDPQLREMSAFALGRLAQDMHNQAGIAHSGGIMPLLKLLDSKNGSLQHNAAFALYGLADNEDNVADLIRVGGVQKLQDGEFIVQPTRDCVAKTLKRLEEKIHGRVLSHLLYLMRVGEKVVQRRIALALAHLCSPDDQRTIFIDNNGLELLLELLESTNFKHQRDASVALYKLASKASTLSPVDAAPPSPIPQVYLGEQYVNNSTLSDVTFLIEGKRFYAHRICLLASSDAFRAMFDGGYRERDAKDIEIPNIRWDVFELMMRYIYTGSVNVNLDVAQDLLRAADQYLLEGLKRLCEYSIAQDISVENVSLMFELSEAFNAMSLQHACILFILENFDKLSLMPWYSHLIQRILPETRQYFLKALIRPTQAELRR

SEQ ID NO: 130 - DNA, 7590 bp, Vitis vinifera
  source 1..7590: mol_type = genomic DNA
atggaaaaggttggagtagcgtctgcaaggaaaagcctgaagcgaaagctcgaagaggagttcgaagaggatggcagattggatgctctctcacaaccccacgcgcttcgcgaactggtgcgcgaggtcggcgtgcatgtcagcgttctcaactctgctatttcttcgtccgaagccgatcgatccgctgctaagcgcgccgttcatgttctgaccgagcttgcaaagaacggtgatgaaccgcttgattacttctctattcgtgttgttagagtttggtgccgtttggtttctgagaaaacggagggaaaggggggaaaaaggaaatttaacttttcggggtgtttcgtcttgattttacaatgaatattcacttaagctgagtttgttagttgcattgggttaaattggttggagggttatgttttattggattcttcgtatcagtttcgtcatttttcgttatattttgttgctttattaatatatcgggtatagttattgggttctggtcgggatttaggatcctttctattttgagaaagtagacgaaaataaatgaaaagagatttagaatcttatgaatgaaattccaatttcaggttctcatttatctatatgtttccttgatagtcatctgtagaattaggttttaaatttgataattcgtgtccttgcagatgaaattgcgaatgtgattgttgattgtcaagttgtgccggctctggttgggcatcttcagtcacctccacccttggtagaaggtgacagcagcccgattccatttgagcatgaggtcgagaaagggtgtgcccttgcactcggactccttgctgtaaaggtaataaacttcgctcatagttagtcttgattaatttaattccaagttttttcattttgttgttatattctgtttggccagatactttttccagtttcataggacaaacacttagcaaaactggtcctttactcatattgattgttttgtcgagcagccagagcatcaacaactcattgtcgatgcaggggctctgcctcatcttgtggaactcctaaagaggcataggtctggttataaaactcgggctgtcaatagtgttgtaaggagagcagccgatgcaataacaaacctagctcatgagaacagtaacatcaaaacccgtgtcaggtttgcttccttgcatgcgttttagttgccacaagtacaccgtcgtgcctttttgtgacagatttagttctatactcaggattgaaggtggtatcccgccccttgttgagttgcttaaattcattgacacaaaggttcagaaagcagctgcaggagctttgcgaaccctcgcatttaaaaatgatgaaaataaaaatcaggttattgacttttccttgttcagaatcctattgggatcataactattgttagtgacatgaaattacacttttgcagattgtggaatgcaatgctttacctatgcttattctaatgctcagatctgaggacacaggtgtacactatgaagcggttagctctcatcataagattttaattggaacttttgctttgattatcttgggaatcttgttcctgtactttgcattgtcttcagtattagctgattgttttggagtctatcagattggtgtgattgggaatctggttcactcatcccccaacataaagaaagacgtcctttttgctggagctttacaacctgttattgagttgctcaggtattgctgattatttcattatgttattcttccagtttctatgactgcttcttagaggggtttttttttttttttttttgttttgttttgttttttttgtttttttgttttttgtttttttctctgtttgttatatggttgaaattcctttctaattgtctgcaaatcgtccatgaagtttacacagaattcattttttcttggtgcctttctcttttccaaatttcaagtgtaattttgatgacaggtccagctgttctgagagccaaagagaggcagctttgttacttgggcaatttgctgctgctgattcagattgcaaggtggattaaataatatttcctcatttcccttgaattgtaaaacttctatgtcaatactcaaggagaaatgccataataactgatccattgattttgtcctcatatccctcttttagtatcatgaatttttttttcccatattttttttattgagtgatgttccaacatgaggttcatgcaggcacacattgtacagagaggtgctgtccaaccattaattgatatgctccagtctcctgatgtgcagcttagggaaatgtcagcttttgctctagggaggttggcacaggttattacttctctgatttcatcatgcagtgcttaaacagatatacagatgtaattgtaacacaattttagctatcatattgttggctgatctcattttttcagttattgtcactgctttcattttcttttttatgaaatatgaatagcattctccttgggtgctgctttagataaggattactagtctttacatgcagtatgagaagcctctttctcttgttccttgtcttttggttgtgctaataaccttcagacgggtttttgatgtatgaatggacacttgaatgcatttcagtcttagagttcatacttgtggctgcttgctattatactgatgtttttggattctcttcagtgtccatcatagcaaatcccgaatgtgcaggcaattagattttccctttcttgggataatgtaatgcaacatttaagtttatgtcatttgtgggtgtggcagtggtagctcctcgtgaggtaaccacttgatgttggcttgtgatcatgttattcacaaacttgaaattttcttatatttttctttatcttcttttaagttttaacatttaaatgcttgtgcaagtaatgtaaatggttgccaatacaagcttaaatttctattttttttccctactattgaagtacttgattacagagactgatattttcctttattggtgcttaataatgactgaagaaaatttgatccttatggaaatctgctggcatagttgaaaaaattcaacaaaggatttttcttggtttactaaaaggttatcatttttaggaccaccacaaccaagctggaattgctcataatggaggtatggtgccattgttgaagcttcttgattcaagaaatggatctcttcaacacaatgctgcatttgctctgtatggtcttgcagataatgaggtattataacactcatgggatcattattcaatctgtagttgtgtttgtttttctcaagttactcatcttaaaatgggaatgtagtggaactaatttaaagtttcttctgtaggataatgttgcagaccttgtcagagtaggaggtgttcaaaaacttcaagagggggtattcaatgcccaagtatgctacatgcttacttcattttacagtttacttaaattgctgcttctaggttcttgatttttaattttctcctcaaagctgaatagagttgaaaaatcatcactccctcccccgtctcccttttttcctgtttaatcatagtttctcagttgtctgctgatgtacttgcagccaactaaggattgtgtggcaaagacattgaaaagattagaggagaagattcatggacgagtgagttttcctttatgggctagacttctttggttttttttcatccagttcttttgcatttgttgccagttagctacctcccttacacaacaagtttattcattggcttattaagatttattatatattttcttggggcaagtgctaaaacttcagaaataaacttgtgctatcttatcaggcttgaattctttctccttgatgtcaaattggtttttggcattacttggtgttgataattactgtttctttattgctttatttaacaggtaatgaaccatctattatatctaatgagggtagcagagaagtctgtacaaagacgagttgttctggctcttgctcatctgtgttcccttgaacatcaaaaaattatttttattgatggccatggtataaatcactatgccaactcttttggtctgcattttgtcttgtacagaagtttattctaattattcagtgagtctggattctgattttgtaatgattgtggcttatatgcaaaatgttttgcaggattagagttgctgttggagcttcttgaatctacaagcgtgaagcaccaacaagatgcttcagtggcattgtacaagttggctaacaaagctacttcactctgtgtcgtggatgcagctcctctatcaccaacaccccaggtatcttttctccttgtttcttatttgtttgtggtaggtgcattcttgtgttcaagttgaggccatagggtagcatgacatgcagtcctgaactgaaataaaaaaagatatttagtttttaattaaatgtttgtgatttgaattaattcatggaattatttcttgttctgttaattgaattctcaattaatgtctcatgcaaaatattaaagatcttttttccattgtctggcaaaagactatgtggagtctgcagatgagttgattttttcttttaattgctcgaaattcttgctgtcctgtaacactcacagttgttctgagcgtcttatggtacttaagtttgtattaatatgggctacaatatgtttgggattcctatatcccaaatgatgttttggttggcaacacagatattggttcattactttgggttgttgcagtcatctttattttaaagctacaatatttatattgatttgtcgtagtagtttgacttacagttcttatggtcgtgaaccaaaattaactattttagtttatagtttcgccagccataaatttgtccaagattagtcacagtgattttatttccctgtcatttttaatggaaattgtccaactattgattgtagcatgatggtgataatgcacattggacctccatgttggttatggaagtactgaaatttctttcctttgttcagtccagcgactttggttgagaagcaatacttttattatttatttggtgtttgtgagttttgagtggtttcaaaacttctgcatctactctttcctggagggtctgaagtgttgatatcttctctcaatttcagttcacgtaaatctttttgatcagtgttctaaaagtacacagaagaaggttttcactatggctctttcctttccccctcccatcatttttgtgcccgctgatgttacatgctgttgtgtttctcttcccctcaatgttttgaaaatgatcatttgttatgaatacttgtttcttccctcctaaaacagagaagtagacttcctttttgttgtctgtttagaggttcatttatgtggatggtcattacctcattatttctgtcaagagcattaaatcagtattacttgaaaagaatggttagcaaatcatctctgttgttttactccaatgatcttattcttttggatgttaaaggactcgaacaatttttaggttttctattaagcctttcaattttgttgcaggtgtatttgggtgagcagtatgtaaacaattcgacactctctgatgttacattcctagttgaaggtagtcaacttgttatcacttccaaattttgttgtttgtatttttgttatgtactgcaatccctacttaaaatccatgcagcattggggtgatcccaaacactctcagtgcccatttcagcttggctcaagcggccttgagtattgtctaagcaaaagaagtgaaataaagagtcaaaagtagacaacatttaaggaaagcaagtgtagtgacagtaaaagttttggtgtacagtctagctttcaatttggagattttgacacattagggacttaagatccccatggctaagaattagactgagcttgtacagtaaagcttccaagcattactgcactcactcttttcaagtgttttatttcttaggctctttattttgctttgcctagagggtatctaagggtgctctagtgtggctgatattggcacttgagactgctaggttatgctatttaaaaaaaataatatttgaatctttaatctatgttctttatcacattaaatttattgtgctttccttttaccagggaaacggttctatgctcacagaatttgtctacttgcttcttctgatgcgtttcgtgctatgtttgatggaggttaccgggtcagcatctactgcctttaaagcactctttttggtccaatgttgatgcttttgtgattttgccccaactttacctctcccccaccttttattttcttgaagatcatgaaaaaatgcaaaaaactagaatacaaatatctgtgttttgtgtgggagacttccctcttccattacatgggtccttaagtcagtaagctgtttctactattaaagaaagccatcaaacttgtgcaatccattgggcccctacttgggcagcaacaatcctgtgagccataatgtagaaaagggagatgacttaatgaagatttggcttattatttatgttagttttgaatatcaattgcaggagaaggatgctcaagacatagagatccccaatattagatgggatgtctttgagttgatgatgaggtcagaatttctagatttgccatgttattaaaaaggaaaaggcattgattgttccccacaatatgctgatgtttcactgtttctattttttatcttatgcttgcagatacatatacacaggatcagtggatgtcaatttagatattgcacaggatcttctcagagctgctgatcagtatcttttagaaggacttaagcgtctctgtgaatatgcaattgcacaggtgagctaagaaatcagttggataactgccttttcattttgtagaacacgtattggtctaaaacctactcattatcttcttcaggacatttctgtggaaaatgtttcgctcatgtatgagttatcagaggcctttaacgcaatgacactgagacatacttgcatcctgtatattttggagcactttgagaaattgactgttaagccatggtatgttcttctgagccactaatacctccacagatttattgaatgaagtcaaacatagactgttgctctgttttaaagcctatttctctcttacaacttaatagaacatccagggattttttacatttgaaatctattcatttcctcaatatctgtcaaacaaattcaatgaagacatgagtttcctccacagatattctccaagcacacttcagtatgcccgttacattattcctcttgtagtaccctagtaccatgttcattccccatcagttttggaccatcaattcttaaatcaaatcaaacctatggtgatcaacattataaaagtttgactggagggctttcaccactctgcaggatcttaatatctaattattatgtacaaaaaaatgcaggtactctcgtctgatccaatgtatattaccagaaatccgcaaattcttcagagaagcacttaccaagccggtcgaaccagtcctgaccttgtcgacatga

SEQ ID NO: 131 - DNA, 16008 bp, Vitis vinifera
  source 1..16008: mol_type = genomic DNA
ggctcgcttcttgtatctgatgtctcatctctgagcggacctcaggtctcaatcctttgccttgatggagcttcagaagcgccaagatcagggccagcccgagaggaaggggcaaaaacggaaactggaggaagaattcgaagaggagcgggagatctccgtggcgccgtccggcgaggcgcaccaggcgttatcctgcgaggtcagtgcgcaggttaatatcctcaacacaaccttttcgtggaaagaagccgatcgagccgccgctaagagagccactcacgtactcgccgagcttgctaagaacggtactctcaaaacatcccgatctgcttttagtttgcttcaatttctagggttttgttcttgttcttgttcttgttcttgtacttggtaggagaataatctcctcaatttctgtttgcagaggaagttgtgaatgtaatcgtcgacggtggggctgttccggcactggtgaagcatctgcaggcaccgccttccagcgatggcgaccatgaccagaggcccttcgagcacgaggttgagaaagggagtgcttttgctctgggtctccttgctgtaaaggtcatttgattatctttctgtttccttaattttgtgtatttatggagtgatttttgttggaaatttgtgtgataaacagatttttctatggcaatattcttattttatttcagttgtgccaacaaatgatattgtctgcagttcagaatttgtcaagatttgtgcaacttgtttagaaacttaggaaaattggtatttctgaattatgcattatacactgagagggttgaactattatatgaaaattgcagaactggaactgtaaggcaggtagttttagtccacttatcctatagcttgcatgtcttagtagccatgcatttgctctatgccttcttatttctagcagtaataagttggtatatgtttaagtgacatcttaagaagtgttttatgtaatcaatagtcatacagagatggaattttaagataaatgagtgttgataagctgaattgtcttctttttagtaagaatgcttctgtgattgtgttttatatgttgtatttgttttgacgttttaattgaagtcagataagactcagattatgttctcttgattgggaaagttattctgtttattcgttcatttatcattcaacatcttttgctttattggcaattttgaacaatttaaactcattatttttcagtcctgggaaggaaaatatgaaatgcgaggatcatcattgtcatggtagggctatttatcaaaaaaaaaaaaaaaaaatcattgtcatggtaggactacctaaacatttcatgaagtgggtcacaccgtcacacaagacctacttttatgctatatggttttgggaaggactgctgtactattggtttaaattccttgacatagattagggtggatcctcagtccgcaatctgcatgctatcttttggaagaaccaacttagcttaaagctgtaaacctttttgagcctgttttctgccaatagttgtggtttttggtttttaaaaattatttcctcagtccacaatcttcatgctgtcttttggaagaaccagcttagcttaaagctgtatgtctttttgagcctgttttctgccaattgtcatagtttttggtttttaaaacattttttaaaatttttttataggtaaataaggatacatatatttttttttgtaggtaaagaaaagatctattgaaaaaagacgccaaaagagcgactcaaggtatacaatacctatacacctaccgccaaactggccaaaaaagtacaagtgaacaagcgcccacggtaaaaaaacaaccttaactagagcccaaccaaccaataaaactaactaaagtttataaacaactttgcctctgaccaaaaggaaaaaacaaaaaagtatatatatatatatatatatatatacatacacacacacacgcacacacacacacacacataattgcaagatgaagtatagaacaatatataatatatttcatgaaagttactaaaggtaaaagaggcaaatagatatcaaatttcagtacaatatgtgtgtaaacattaaatattggagttttgatgaaatcaacctggcaaaataagaaattttatatcaaaaccaacttaacaaattataattttttttttttgataggtaaataagagattgtattagaaaagcctagaagaggcgaaaaaagtacacacgaagtatacaagcaagcaacgcccaagaagttaggcaaaaagaaagaagaaaacctttctcctatctagacaaaagccactctataaaatcaaataaggacaaagaatgatcccctctaaatacaccctaccccaattcacaaaagtgtacaaaaaagaaagttttaaagcttggtcggaatgttcagtgtcattgaacactctttcatttctttccttccataaggtccacattaaacataggggggcagccctccaagccttttcctttctcttactcacaaatgcaccatgtagaaattttaatttatagattcatcattgacttcattaaaaaaaaaacttttgctagatgttattgccctaaaactttcaagctttgacatgttctcaaacaataaaaaaagtaactgtgagcaattgagcatgttcaattataaacaaccaagtaaggtgaggttgtttttttgtgtgcctgctcgccttgctttggccttttggtgcccttgtatgcatcacgtgtatgtatatttgttaggacatatgtctctgggtgacatgtttggagttttgttctgactttatgaattcatcatttctccccttctccccactcccgaacacagacacacacctctaacacaaagaaacttcccattcagacatgaaagtgaaaaaaagaaacccatttttaattttaagaaagggaagaaagagagtgccatgaaactctaaaagctacaaatagattttttttcttttaactacagtatgggcaaaatgaaacaaaagaaagtttctgaaatcttattttaatttagtgttttttttaaacaggagtataataatcctttttaagataaaagttgaagttgaattttccgttaacctttaaaacattgtcaaatcaaatgcatgcattttctatctattgtgcattgtaagatacatttaagatattgcatcagtggtatgtttgtttcacattaaaaatatattgtatcatatgtgaactattatgtgctttaacttttgacaattattctgtcagttgagcttccatatattgttcatgtccaaacaaaaagaagtcaagccagcctgtttatgatctgtttactggtttttgggttccctaagcagcctctagattagtcgtgggtagaaaatctggtgaaactggcccttaatttttatttatttatttatttatattttaaatgagggtttaacaaattgtttacttgtaagaaatttgaaatctaaaaactacaagtattaggaatatagagtggcaattggaatgatctagaagtacaaaaaacattttattatgcttactcaatggaaagaaggtattaaagaaatgctatcatcatcttcgtctatctattcaggactgagaagttagaggaattttatttttatatctttctaataatgatgctaaaagggtttgtagtccccttttttgggtgggtttatattcaagccgttttagggattgggctagcacagagagaacttatccgaaagtttcttgcactcttgttgtattaataacaaccatgaatactaaagtgaaaagcttctttttggattagttattatatttcttttcaagactaagaatttggtcttcgatgctttcccaataacaacaatcacagttcaggtaaaagccttcatttttttctgggtttctactcttctccaattttaattcctgaaatgaccatgaagtttcattctgcttgtttgtgttacatatgtttgaggcaatttgttgtgagcatcaatagccaatatttctgtaggctggcgatttagagcatgccaccatttttttatgctgttgctagattggatgtccaagacaagttccacttattagatctagtcaattgttattctcattcttcctctaccttgcatgtttcctcatgaatttgaaaggctgtagcttattgaatacatttacctttacatttaattgctgagcccattgattttattgtcttctgaattaacagccagagcatcagcaactcatagttgataatggtgctttgtctcatctagtggatcttttaaagaggcacagagatggttctaactctcgagctgtcaatagtgtcattcgaagagcagccgatgctgtcactaaccttgctcatgagaatagcagtattaaaaccagagtcaggtttgcttatttgcttagtacttcaacttcaactttctgatttagcagtattttatcattctgataatctgattggacatgcaggatggaaggcgggataccaccccttgttcagttacttgaatttgctgatacaaaggtgcaacgggcagctgctggggcactgagaaccctggcatttaaaaatgatgaaaataaaaatcaggtaattgccttctgtggagagttggacctttatggcactaattcagctcagaaattgatatggatattttgattttgcagattgtagaatgtaatgctctccctaccctgattctaatgcttcgatctgaggatgctgctatacattatgaagcagtaagatgtcattggatatggactttgcatttgtgaccagtctattgtttgtgcttacaattagccaattatcatgaattccaggttggtgtaattggaaatttggtacactcttcgccaaacataaagaaagaagtgcttttggctggagctttacagcctgttataggattacttaggtatgaaagaatcttgaattcttgtcattattatggagtctttgcacttggtttggtagtgcatgttcaattgttattaatcgtctgttattttaattgttcaccacaagttttctgtgaagaattttgttttcttgttgtatttcctaagttgtctcattgatgtcagttcgtgctgctctgagagccaaagggaggcagctttgttacttggacaatttgctgcaactgattcagattgcaaggtggagtcatgttcttgtatatgttcttacatatatattgctttttttattattttatttatcttcgctagagccctggacttttcccatatgcttgtttgttgcaaacaagatggaggaaataacaagaaaaaattgaatttcctgctctttggggttggattgtttgttcaataattcctggtattgttctcttatcctgtcttgttggcagtttatcagtgtgctatcatttttatgttcatgtgtttgggatgaatacaatacagaatggtcctttggcttcattcaatggaccttcatatatacgttattgtttcttctttttcttcttctacctcttttctttggtttttattttttcttaaagatgttagattcttgcaggtgcatattgcacagagaggtgctgtgcgacctttgattgagatgcttcaatctgcagatgtacagctgagggaaatgtcagcctttgcattggggagattggcacaggttatactccttgaattcttttatttccttttcaaattacaattgacaaataatactgatggcataaaatgcttactatattatactgagtagtctgtttctttcaagtaatctttgcaggatttatcacaataagtttgtgttatcaattatcatgttctgtgaatttctatccctcctttatagccttatgtttcattgcttgtttaggtgaaggataaaacaaacttttgggtttcaagcactgatgagaaaacatcccaaattttgtgcaaaggggaaaataaccttctaaaagaaaatataaaaggctccaatcaaaaagaggagggggggcagtgcacaccccaagtacacaggaaagaggaaaataacctagaactaacagcaacaaagaaaggaaacagaagtcccggagcacagaaccattatttaaattctaaagggttttaacagaccttcatttgatatattttattttgaaaaacaaaaaatgaaagaaattaaaaaaaaaaattgagaacttgggaatgtacacctaagtattgtttggaattaatatttgtttggttcttgggtgaaagcttgggcaagcctctatattaagagatcacatatatgagcatttgaatggaaaaggaagccctactacatcagctggtagagagttctatactttcttgtctatatcatgagtcttcactgccctttgtccttccataaattactggacctcatggtgtgccccatttctagagtccatcagagctggttgacagtctaaaatgccttttgatagtttttttatttagttgtatcagttcatgaaagattttatttgtgaaattttccttaagtaactttgttcttgttttagacagacgctaaacctcattacgtcggtttattctgtcttgaattgaagttccaggattcaacctttgcttcctctggtaccaaggtttaggataaatagtccaaggactgaaccaagttctacaacaaccctattttgttgaggatatgaatagcttgagcatcctagtttgtgattacagctgttactatgaagtgattgggctttatgatctagcacctatgtcaggagcagaacaactttgctgatacttgctaaatgttggactgtccatcagggaactagagatcattgttcatctcctcaaactagcatggatattctatatgatagaatttgtttatcttatatgcccttgatttttgcagccctctggggaaaaaagtttttaaaaagaaaaaggtaacacgccatacaatattgacatgttacatgagatattttgtggattatcttgaccttcatagccttccaatatcttcaaaacgtgccaccccaatgttaactggtttggcctgtgggatggttaaagtccctttatttatttatttagtttttgaaatttgccagttgccatgtgcatattggttggagtgccctgcattttgttttgtccgtgtgcttcttgttatattttttttgatacacatgtttgattacgcatctctttgtctttgattgttattggtgttgattgttatcatcttttctaagaaaaacttttaattcataggagatcaagggccattctgaaaccagccttgagaatgaagatgccaggcaatgcactggcaatagtcttgggtggataccaaaaccatgcaagtgccaccctgtgagaaaagctctagcaggagctatcaccttgtcagtatctgctagcactctgagattgcaaaatcttaatttcattgccaggataggaaaaaactttggcatatctccataggcttaaaatatgatacataaaatactgatggagttggcaaactcactatcattgaagacttgatgaggaattcttaattcacctcgatgctgtttctctttcctccttgggaaagaaattaaagaagttagtcatgcataaactatgaagagttgaatccatgcctgtatgactctcaatataattcatttgttaggctcacttctgggagatgcacttgaattttcgtttgcttcattatatttcatgaattaccactcatatcatgtcactgagaatctgatgataaattttgtagtggataataacctggttcataatagatattataaccataatgctgaatcagtggcatacctggatctacttctttgatattacagatgtggcctgtgctgcttcttactctctttaatttttatattttgcagctgcatctatcctaaatttgctcactgtgatgtttgtatacatttgttagctgtagttatctatggctttaaagagaaatttctgttttgtcaggacacacacaatcaagccggtattgctcataatggcggtctagtcccattattgaagcttcttgattcaaaaaatggatcactgcaacataatgctgcatttgcactttatggccttgcagataatgaggtatatgtcttcattgactttatccaaaaggaattcatttaaaactacttcaatagaattttgttaaatttatttgtttatttccctccaaaggacaatgtatctgattttatcaaggtgggaggggttcagaagctgcaggatggagaatttattgttcaagtaagcttctctcctagtttacttttaataagtatctgttatttctaggtttatcaagttatcaattactataaaagcttgagtctttgtaggttgtgattgttgcatcttaaagttaccaactagccttaaaagcttaagttgttatgtaatgggtcaactatgtatatcatgccaatttgcactgggagtaaagttcaacacttgtctcatgaacagctttctttgggcttgcatgtgggctcgataaatagggaaaataaacaaaagtgaggtttgaaaacctgacctcctttgaactaagacccttataccatgtcaaactatcaatttgacccaaagccaagttatgcttgcgctgaaaccctaacatccgccattaccaatgttaaggtttataatgtaattgcaggcaacaaaagattgtgtagccaagacattgaaaagattagaggaaaagattcatggaagagtaagttgtttcttatcaatattactgtctaggtattgatgtctctcatgattttctatgttgaattgttgggatggttagtcattaattttcacttacaggttttgaaccatttgttatatctgatgcgtgtatctgagaaggctgttcaaagacgagttgctttagctcttgctcatctttgttctgcagatgatcagaggacaatcttcattgataacaatggtatgccattttttttctctaatatcaaatataatcagtaagccctaccctttcattattttgagatctatctagcccttcatttgttccttttttgggttttatttgggcacacaaaagtcattttatttattattgtcatgccagtgtcatgttatttgaacaccatttccgtgcaggattggagttgcttcttgggcttcttggttcttcaagcccaaagcagcaacttgatggttctgtggctctctacaaattggccaacaaagccatgactctctctcctgtggatgcagctcctccttctcccacaccccaggtgagcatcctttcaaaagctggtgtaattttttttttttgccttgtcatgatctagatttttttcaagtgttttatgcacataatcatggcagatataagtgtgaaagaatgcttcaatttactaaaacaaatcatgctaggatttaggattgtggatttaagtagtttattcgtgtgatttagatgtatctattaaatatctggggttccaaggcgttgaggggcttatcttcttgtttacatgaatgatgataatatatgtaaaattgctcagataatgtactcagaatcttttatttgaggttcttctctggcatctcttgattggaacaagagtcagaagcagcttgggatgttgtcatttaatgcttttttcttgccttttctttccaatagacagagacaaataaagaagtaaatcaataagttccaaagagagcttgcccttgatgcctaactcaagtggtaaagggatggggggaggtttcaggttcaagtcccaatggggacaaaatttacctaatgaaaaaaaaaaaaaagaggtgccaaagagagtggcacaacctaggtatatggcaagtatgcataaagcaccaaagcaaaaaggaagtagaaagagaaaggattcctcacacctgctggaaagtctaaacacaaataaaatttacaaaaggcttttttcccattccctacagattacacaaactgaggattaatgagcatactttccagtttcaagtttgctataaacaacaaattaagcaaattggtgtcctagtccatacgtcgctttcctttatgaacaaatctatcttacttgtgcttcttgaacaagcaaaccccaattggatagaatcataaccctccctctcagttggtctgaagggagaattttccccaaacccctctatgcatgaaagagacattaaaattcagaatcaaagccttaggggtaggatttttactgtgaaacgagcatctttggttagcttccatattggtttatcttccctaaacatgagcagcacccacttttgaatacaagggtagaaccattctgccatctctaactccccatcatggaagcttctgatgaatgtcaggaatctatggtccttatcagctcccatttttcaattttctgccactgtaacttcttgattcactgtgatggagaatagatcagaaaagtggctaagaggaatctatccattctaaatctcacatcaaaatttatttttaactatcctccttacacatctgacacaaaagaagaaaaatgtctcatccttttccaatggctttctaccaagccctgaatatatttctcctcttcccacaccagagccgcaactaccatgtcccttgtcaaacttccccacaataaccttactccacagcctatttttattacaacagatcttcatagccactctcacctgataaaaacttatttaggatggagaaactttgaatacccaaaccagctttctccttggagaaaacacagttgcctagttgaccagatgccattttacttcgaaaatcaggattcttatttttcacagaagtctttttaaatttctctaacctaacttgaaccaaaactagtataggacatgaaatatactggcaagctagggaagatgctcttaaccagtgtaggtctttctcataatatgtggatgatgtattgtgaaattaaatgagatttatgattgtttttccttattcttaagaaatcatatgccaattgatgttgtgttatgctgtgagtgagtgcatgctgcatatcctatgcggcctcacctggtatcacttggtgataccctgtgatatttggatgaattctccggcaggctgttaaaagaatccaacttgaaatttctgcctccaaagcatggtttgaaatgtcggaaaatttcggcgaaatatcaccaaaatttcacttatcgaagaggctcgacacgatattccacattgataatcagttgacagaattttctgtgatttttttggaatatcgccgatatttcggtaattatcggtatttttattgatattgtgggagatttcctgatatttcggtgagtggtcaacacagtcagctgaaacaaggggattcgaacttgaacataggccacaaggcttgggttgaaccttggcttccactggaccaacttcacatttgtaaatatatattgaatttaaatatgttaaagtttattatttaaaaaaaaaaattataattattttattttgaattttatttaattgattaataaaaatataaaaaccaactttataattttcttaactagtttttttttttaaatatatatatattatttatgtgataattaaatattaaaaaaaatcatatatcaatcatcatttattttacattattgaatgcatttgaataaaataaattatagttttaatattcaatatatcatcatttatctcattaatcctattttaaaaaattacaatcacttcacttttaatttttttatatttatctttttaattttgaatgtctttattttaaaatattaaaaatataaatttattaaaaaaactaaaatataaaaaaatagtaatgaagttctaatattttataaattaaaattgatttgataagatgaataataaattatatattaagaccgatatatgattgcttatcgatatatttctctttaaccatacttatgtttacacttacaaaataactttaacatttgtatttttatttattttattattttttagagttttttcaaatatttccgtcaattttgaataattttcacctcaccgatatttttgtcaaaatatccattaatatttctttgatatttccgatatatccataaaatccaaatatcgatatattcgtgtttaccaatatttcaaaccatgctccagagcagatgtttttggtagtcaagataaatactaagcctcgagggtggatgctagtatggcaaaccttctagttcacctaaggtggttccgattttatggcattacatcctagtggctgatgcatgcttgagtcaagtgctgggtcaagagatttctaatggtcttgatgtgttttaatattgtggcacaatgatcctgctgttggatgctggaatggttttatgggctctgcttgatggtcagagtataggcccactaagggagatgcctgccgttgttaggatgagggcaatgccagttgcttcagcctatttgtgtaggtcttccactctctctggagcatagttgctgaatgctgtatcatactgtggttcctgttaggtcctcacatgtgctaagtttcttatacaaggatacacagggaagaaggcttctattggtttggattgattatctttgaaatttgggagtggtcagtatttggatttagtgatgccttggttgctgtaacttacctaggaaggcaatattctattgacatacacggaacagctcatgtctctttccaccctagcgatataaagcaactgagagcataccaaagtttgaaaataattacttcataaccttagttccttagtgaagctttagctcttatgtaaacattttgaattattgtaacatgcatcatattacttaccaaagtaagacttagagtcaaaggctttttttggtgattgtaaagccaacaacagaataaatccagggtcttttgtttgcttgctgtacatgtagaaataaggagttcatgtcttactaccattccttggaactcaaatttttaaatgtttgacctttgttcttggagggccattctaatttgtaaccttttgttctttcaactttttagttctagagacgccttttttttcctctaacatagttcaagattcctttgttttctctgtgagacctcctctttgaaatatctaaagctagaagttaaaattgcacaccatttatcatcatttctttgctggtaaaacagaagttacatacttcaaagaacatccttttattctaaattgcttgttttcttaaattagtcctgtgttttgttttaagtgatttatttatttttttacatgatggtatggttagggaataagaagtctattttctagttttgattattttttacccttatttttttcccactggtatttcaagtatttgaaagtctcttactttaaaagcttgcattggtatgaaaattaggttcctgtgatgacaagcagttcttactgcaggtctatttgggagagcaatatgtaaacagtgctacattgtccgatgttacctttctagttggaggttgtaaatcactatttcttcatcatataaattctgcttatgtaaatccagatactttcatggctgtactggctcaagttcttttaccataaatcgtctctttgaatgctcagttgcttttaattttcccacttcaggtaaaaggttctatgctcaccgaatttgccttttggcatcttcagatgcattccgtgcaatgtttgatggtggttatcgggtgagtatttgtatagtattctttgtctaatgatttttgtagtttcttttctatatttttccttctcttcctttacactatagactgggaatctttactaactcgctggtaatttatcaggtgagtttttgtgtagtgtactttgtttgatgatttttggagtttgtgttctatactttccttttcttcttttgcactgtagactgagaatcttttctaattctattatttggaacgaaaaaaataagaaaatacgtttgacaatcagaaaaccgttttctattttttgttcttaaaaccaaaaaacatgatatttttagagaacattttttagttgtttttagttctttttacttgttttctgaataccgttttaaaaaataattatataaatatggagaatgattaaaaataaatcactacatataaaagttatctttaaaatatatttaaaaacatagaaaataagttaaaaacatttcaagttttcaaacagacgcttgttttataaaacatcataaaacaattttcaaaaagtctggcaaaactgttttaaaaaacagttaacaaacaaaactttagagaacagctttcaaaaatagttttcgaaaaagttatcaaacaggacctaatattctctatgcctatgtataagtaaaaattggagccatagattagagcatagaaaggttgtaactaagtatttgcatgtatgttgataagcacatttgaattaattccttgcatgacaggagaaggatgcaagagatatagagatcccgaatatcagatgggaggtttttgagttgatgatgaggttagacaatttcttagtccagtatcagagtctctttcttctcagtgagctttgcttatttgccagcattctgtatttgggcagatttatatacactggatctgtagaaattacattggatattgcacaagatctcctcagagctgctgatcagtatctcttggagggactaaagcgtctctgtgagtataccattgcccaggtgagttaaggaggttgattttttggtatgaattcctttactgctttaaatcagaaggtggacacctgctgactctttaatttttcatcttcaaggatatatcactggaaaatgtttcaagtatgtatgaactttcagaagccttccatgctatttcattaagacacacatgcatcctgtttatcttggagcagttcagtaaactgagttctaggcccgggtatgtggtgctctctctctctctctctctctctccctctccctctccctctccctatccatctatccatccatttgtaactgccttttctactaatagcttattaaggaagaagttgtaaatacttttggagttgtacgaattctcaatggaggcaattgcttggaagcctaaatatttgtcttataaaaatctttagctagcttctgatatatgaaaaataagattgaaaaatgcggttgcttgtttgaagcatacttacaagtcccttgaaaactgggatgatgctccttaacgaatgttggatgattacctggaaaaattttgaaaaatgttttggtgctgtgtcattttcctcattgatagattttctgaatgaaaataaatatgtggtaagggggctaggttctgaatgatatgttattcataatccaaagttccatgtggcttgtaaatcctgccaattctatgtgcacagtcatgaaccttacctatgaaaaaaaaaaagtggtcatgaaccatgataatataaagctgcactattacaactttgcatcatcattttggaccaattattgcatcttacatttattacaactttgattggaaaaatgatgctgtattttttttttttttgatgattttattttaatagaatgagaaaagaaaatgcatatatattgatgcatgatctctctatctaaactcatgtctattgtgagctgagattttctgttcaaaatttgtaggcattctcatctgatccaacgaataattccagagatccgcacctactttgctaaagcacttaccaagcctaacccacataattcgaggctataa

SEQ ID NO: 132 - protein, 713 aa, Vitis vinifera
MEKVGVASARKSLKRKLEEEFEEDGRLDALSQPHALRELVREVGVHVSVLNSAISSSEADRSAAKRAVHVLTELAKNDEIANVIVDCQVVPALVGHLQSPPPLVEGDSSPIPFEHEVEKGCALALGLLAVKPEHQQLIVDAGALPHLVELLKRHRSGYKTRAVNSVVRRAADAITNLAHENSNIKTRVRIEGGIPPLVELLKFIDTKVQKAAAGALRTLAFKNDENKNQIVECNALPMLILMLRSEDTGVHYEAIGVIGNLVHSSPNIKKDVLFAGALQPVIELLRSSCSESQREAALLLGQFAAADSDCKAHIVQRGAVQPLIDMLQSPDVQLREMSAFALGRLAQFMSFVGVADHHNQAGIAHNGGMVPLLKLLDSRNGSLQHNAAFALYGLADNEDNVADLVRVGGVQKLQEGVFNAQPTKDCVAKTLKRLEEKIHGRVMNHLLYLMRVAEKSVQRRVVLALAHLCSLEHQKIIFIDGHGLELLLELLESTSVKHQQDASVALYKLANKATSLCVVDAAPLSPTPQVYLGEQYVNNSTLSDVTFLVEGRKRFYAHRICLLASSDAFRAMFDGGYREKDAQDIEIPNIRWDVFELMMRYIYTGSVDVNLDIAQDLLRAADQYLLEGLKRLCEYAIAQDISVENVSLMYELSEAFNAMTLRHTCILYILEHFEKLTVKPWYSRLIQCILPEIRKFFREALTKPVEPVLTLST

SEQ ID NO: 133 - protein, 705 aa, Vitis vinifera
MELQKRQDQGQPERKGQKRKLEEEFEEEREISVAPSGEAHQALSCEVSAQVNILNTTFSWKEADRAAAKRATHVLAELAKNEEVVNVIVDGGAVPALVKHLQAPPSSDGDHDQRPFEHEVEKGSAFALGLLAVKPEHQQLIVDNGALSHLVDLLKRHRDGSNSRAVNSVIRRAADAVTNLAHENSSIKTRVRMEGGIPPLVQLLEFADTKVQRAAAGALRTLAFKNDENKNQIVECNALPTLILMLRSEDAAIHYEAVGVIGNLVHSSPNIKKEVLLAGALQPVIGLLSSCCSESQREAALLLGQFAATDSDCKVHIAQRGAVRPLIEMLQSADVQLREMSAFALGRLAQDTHNQAGIAHNGGLVPLLKLLDSKNGSLQHNAAFALYGLADNEDNVSDFIKVGGVQKLQDGEFIVQATKDCVAKTLKRLEEKIHGRVLNHLLYLMRVSEKAVQRRVALALAHLCSADDQRTIFIDNNGLELLLGLLGSSSPKQQLDGSVALYKLANKAMTLSPVDAAPPSPTPQVYLGEQYVNSATLSDVTFLVGGKRFYAHRICLLASSDAFRAMFDGGYREKDARDIEIPNIRWEVFELMMRFIYTGSVEITLDIAQDLLRAADQYLLEGLKRLCEYTIAQDISLENVSSMYELSEAFHAISLRHTCILFILEQFSKLSSRPGHSHLIQRIIPEIRTYFAKALTKPNPHNSRL

SEQ ID NO: 134 - DNA, 7737 bp, Solanum tuberosum
  source 1..7737: mol_type = genomic DNA
atggagaaccagaagcttaccgagcgttcgtcaagttctgcgaggaggagcttgaagagaaagctagaggaagatctccaagacgatcgtaaggtttctccttctctatcttcggaagatggtcatcaagatctggaacgtgaagttcgtacacaggtggagattcttgagtcatctttttcttcatccgagtcagatcgagcctcttccaaacgcgctatacatgttctctctgaatttgccaaaaacggtaactgatttgcatttcattttccagtggatcagaattttagatgttcacgctgagagttttcttgttttttgtttaatcggtttggaagtgttattaggttttgatatttgaggatttgtgttttgtagaggaaattgtgaacgtaattgtagattgcggcgctgttccggctttggtgcagcatctacaggcgccgcctcatgtaaatgaaggtgaaggtagtcacatgccatacgaacatgaggttgagaaaggaagtgcttttacgcttgggcttcttgctataaaagtaagcattcagttcgttttttggatatgtgttagttttctctgcgtataatcagtacatgtactgtaaaataaaactagttacttccagcagatgattgtatgaattatctcatacttctggtgaaaagatcttgcttgtgcagcaggagctatgtattaaatggaataagttactgtaaatgggattttcattttgctgtattcttgaacacttatttaattaatttgtgcattcctttgcggcaagtgaagaagacacaagtttcatttagcaagggcatttaccaagtgtgtctctaggtgatcattgaggaactatcaatatgacttttctggtagcggtggatctacagtagcgggtgtgggttacggggaactcagtaacttcttctgaaaccctacaattatattgaaaattcttttaaatatataactatattttctgaaatccattaacaactagaaggctagttccgtggcaaatagaggaacgattgaaccgcaccagcgctagtgtgtgcaggtatgaatccccctgagatcagttttactaaaacctaaaatatctttgttgggaaccataaacttaacatccaggatttgcctttgactttacgtatctcttagactctgaagttatctattaacaagaaagggtaatagaatgctgatctcttaaagattattttgtgtgcaaatcaaataaaaggtattaacgcacagtagataatttccaattaggaacatgtgcagatctaaattaattgcaatcaatctaagttgagtgctttgagtttaattgtctggtattactagatttatgttctacttgaaaaagaagcttccagaattgttctgtcgatcaggtttcatggcatatagataattttccatcatcacaacctcaactaactcatacacttggatcatttgcgttttcattgatgtactttcttaaatttttgtctctcataatcctactgaaaagaactttgcttctcctctacttaattcggtatagtccttactttttgcatctatccgaggagtagagatttactctctttctatattttaaacttatgtctgacagccggagcaccaacaactgattgttgatgctggagctttgcctcatcttgttaatttgctgaagaggcatagagatgctcagaactctcgcgcagtcaatggtgttattcggcgcgcagctgatgcagtcacaaatcttgctcatgaaaacagtagcatcaaaactcgtgttaggttagtttattcttatctggaaacattgttattacaatatctatggaaataagaaccctttttcttacttcatctgtattttgtgactatagggttgaaggtggcatccctccacttgttgagttgcttgagtttgttgattcaaaggtgcagagagcagctgcaggatccttacgaacgttagcatttaagaatgatgaaaacaaaaatcaggttaatggcttacaaaatttatcttgaatatctctgtggtcacgtcttctatttatgttaatttgtgtgaattgattgcagattgtggaatgcagtgcactccccactcttatactaatgcttcggtctgaagatactgctatacactatgaagcggtgagacatcattcaatgtcatgctgaactagcacatatatatagtaatgattgataatacctaggatattggctattcttcatgtggtagtcatccccagaactaattaaattgtgggtggcaggttggagtcattggaaatctggtgcactcgtcaccaaatatcaagaaagaagttcttcttgcaggagctttacaacctgtaattgggttgcttaggtatactcaactctcataacttttgatcatatgaacatttctggtctgtagtaggacctatgtagttatatgctccctcttcttttgctcaactataaatcttgtatgccagttcctcctgttcagagagccaaagggaagctgctttactgctaggacaatttgcagcaactgattcagactgtaaggttgattaaaataataagctctattattgtcttaaatggtgaaactctttagttaagtagcattactgagctacttaaatcattttttacacatagtttaatctgtttgaaactcttgcagattcatattgttcaaagaggtgcagttccaccattaattgagatgcttcaatctccagatgctcaacttagagaaatgtcggcctttgccctaggaaggttggcgcaggtaattcctcttggatgatatcttgagtagcgcaagttttcttatacgtttcatgataagctttccattcccttgtctactagtagcagttggtctattggttgtctgatgaaatcttgctattccagaatttcttttccgacattcatatgttctttgggatgatccatcacaaacttgtatttgatgatttctgatattgtttttcaagtgtgatctctttaatatgtattgtctacgttctataaagaaaatcgtatttcttgactgttaaggaatggaaaggaagtgaagcatgttgtgattggtgtccccattgggctattggttattcagctgctgcaaaaggtttttattttaaaatgttcgtttctgaaaattatttctagatgagcaacagttttttcacatagttgatatgatacctacctcgggggtatgttgaggagtctctaaggcttcatttgtttgtacttaatgaaagtctgaatttgaaccgtttagatgtggaaaaacaaacaatcttaatcattcaatcttcaaatctaaagacaacatctcaatctttcatatgtggagtcagatttagacgcgttaatcttaatgaaaataaatgaggcctaagagaataagagattggttcttttgggcacaaaacttgattgaaggacaatagtaatgatttcccagtttggaagtttaatctacccaaacttagtggaagctatagtgctgactctgagcaaaatcataaagtgtggtttgaagggtattattttcattacttagtcttttgaagctgctcaatctcttgtgatttatagtttctactgaagatcttcagatttgtaatatttcttcatcagtagctctgttttagatgtagataattatatgtgccttgctatctcacaattttttggttcatgttttacaatcacataataacagttctgaagagtaagactgattgaatctttaatagccctagcaaaatggaatatcaagatgctgtgatgtttctaattctttggtacatgagtattttaattttttactctctttggagctcttatttaacttcagatgtgatgattgatggtgcaagaacatttccttttcttcttccttctcatagtactttatttgatttgaggatttagtacgacattgtgaccgggtgttagtggttccatgatgttcaggacacacacaatcaggctggtattgctcactgtggtggaattatcccattgttgaagctccttgattcaaaaaatggatcattacaacataatgctgcatttgctctttatgggcttgctgataatgaggtgttgcatgtcatcagatcatatatgctttgattataattaattttatgcacttacatgcttctttagacttactgtgactttctgctataggacaatgtagctgatcttataaaggtcggaggtgttcaaaagcttcaggatggagaatttattgtccaagtatgatctcttgatgtcgtttcttttagattttatgttttctctcaaggataagtacctttgttgctttaaatgagtttgcattattctctttttacatattgccctaagttctaaattgagttcctgactatgcagccaactagagattgtgtggcgaagacattgaagagattagaagagaagatccatggtcgagtgagtttctattttttaaattttttgtttttgtcttcggatgacacgaatgcagcttacctcccttctccacattttgatttttcttttcttaaatttcttttgttaaatcttattaggttatttgtgagtacaatatgtaatatctttctccttctttggtagatattgggccatctgttatatttgatgcgtattggggagaaggttattcagagacgagttgcattagcccttgcccatctttgcgcaccagatgaccaaaagattattttcattgataacagtggtatatgtttgatttaaacttgagattgctttttaatacgttctggttaggcagtgacaataacatcctgtttgtttatgcacttgtaggattagaattgcttttggagctctttgactcaacaaacttgaaacacaaaagagatggctctgcagctttatgcaaattggctaataaagctagctcactttcacaagtcgatgctgctcctccatccccagtgcctcaggtttgtttatcttagtctccattctgattgcactactaagattcttcaaatttttgctttgagcaggatttagtttgactattagttggtttgtgttaaatttctccacttctgtacatgtagtactttagtttgactattagtactaatttagtgcactatataactcccatgaacagaccaggccttaacggttactaaattggtgcgctatatgtagaaaatgtcaactttattttggtcagttgtctttttgtccatcatttagtaaagggaggtaacaaccctctgaagtttataaaatatagctatgcaaatttaatatgtttggtcatttttcttcttgtttctaaatttacatgttcatgcctatagaccaatttctaaaaaaaattcaaggcagtgtgctatgcagactcaagactttgacctcctacctccaccccccaaatagttagccaagactagaaacttgtagtgcgctaatgatgttcttaccataggcagacaccactttcttggtcttttctgcctgagctggagctttagactctttgagagatatattagtgattgggcaacctctcttggcaaagaatggttttcctcatagagagggggagtaaggggttttctgctgagtcagaaaatgttgtttgtagagtctctttctgttcaggtcttgaatcatttgatttgggaaaatccaacaatgttgattggtaaaaattgaagacatgaaaagtagccccggagcatgtgctccaattttgtgtcgtttttgcctctaggtttatgtgttaagtaggacgtgaagtgaggctaggacgattcttctattttgaggatgtagataatgagaggaacttttgatgaatttggaagaatatgcatttttgatgaaatcttgttattttaccaccctatattggttattaggtgctgattgtgttgaccattttctgttccttatttgactgattgtatccattcttccatttatattttatctcaattgataatgcagcttattccatcctgatgttgtacctcgttccctcattttttctcttataatttcttttaaatccaggtctatctgggtgaacagtatgtaaataattctacactgtctgatgtaacatttttagttgagggtaagagtggttctattttttaataatgtgactctcttccccttttcctttttaatgttctactaacttttttgttcattcttctaccaggcaaacggttttatgcccataggatttgtttactagcttcttctgatgcatttcgagctatgtttgatggtggctaccgggtgagttatagtctgccttttatgttctatatttattcatttcctaatatgatccattgtaaaaatctctcgccaagttttaagttgacatcttgctaagtgtaagggtagaggagcagaccattatccattgagttttgaatcttgcacctcatatcttttattttatcttctttttgtttgtgtttgctacttcaaagttttcattttctattattgtcttcttcttttgtataaatgtaactcttgctgctttgatttatgtcttactctcctttatagtttgtgtcaaaaaaatgccttactttcctttgattcatgtctttaagaccacaagattcaagggcattttggtacattacatgcatgatgcatctttagtttaagaccataagattcagaagtcatcattttaaaaactttgtacccagtcgaatcaagacacaatgaagtgggggggagttatgagaaccaagatagtgtatgcatggccattgcaaaaggagtcagcccaacatatttgtttgaattttgtcagcgtatctggggttatcttgatacttttgtttctaatagtttgtagtaaatgtattgcaggagagagatgccaaagacatagaaatcccaaatatcagatgggacgtttttgagttgatgatgaggtagaatgatctttaattaccattttacatcctcggttcagatcctggaagtcaatcttgcagttttaaggactaatctttcttgcttgcaggtacatatacacaggatctgttgatgttaatttggatgttgcacaggatcttctaagagctgcagaccagtatctattagagggccttaaacgtctttgcgagtatgccattgcacaggtgagtgctgagatcttttgggagtttggggggttttcctgtcacatttatgctctaatgatgttgtcttttctaggatatatctgtggaaagtgtctctctcatgtttgagttgtcggaggcatttaacgctttgacgttacgtaatgcttgcattctattcattttggaaaagtttgaccaattaagtgtcatgccatggtatgtcctggacttttctatccttaattacattatatttttatgggtttggtgcatggggaatcaagctggatatccttttatttaatttatttgatgtgtgaaattgtgaagcatgtcattgaagtgaagatttccaaaaattatatatgaactgattaagaatgtggattttctcttgaatgtgtattgacgtgatgcgatctcctatgcaggtattcacatttgattcaacgtgtattacctgaaactcgaagttactttgtaagggcacttaccagggctattcaagctgacatgcgggtctag

SEQ ID NO: 135 - DNA, 22184 bp, Solanum tuberosum
  source 1..22184: mol_type = genomic DNA
atggagaaccaagcaaaacggagcaaacaatcttcgagttccgggaggagaagcttgaagagaaagctcgaaggagattttgaagacgatcgtaaagtttcttctccgttttctcatgatgatgatgatgctcatcaagatctcgctcccgaggttcggacgcaagtggagattctcgaatctactttctcttcgacggaagcagatcgtgcctctgccaagcgtgctattcatgttctctctgagctagctaagaacggtaactcaatatctcgtttctagcggatcagaaaatttcatgtacatttctatctatcgggagttaattcaactaatttcccaagttaaactctactggatttattcaacaattttttttttcttaaaaaatacaagttagatatccaaaaacagcacgataagtaatgtattagaacattacaaatgttagtcaaagttcttatagagtgctgaatgtcctgggaagtacatgcagagagttgaattggtttatttcaatcaatttgggcctgaaagttgggttttgatatttgaggatttttgtgttgcagaggaaattgtgaatgtggttgtagactgtggtgctgtcccagctttggtgaagcatcttcaagtgccatcccttgggagtgaaggagatggtggacagatgccgtatgagcatgaggtcgagaaaggaagtgcttttacgcttgggcttctagccataaaagttagtataaatcacatttattctcttaagagttgagcacatatgagaaggcaattttcgttattagggcagatgattcttcgaattactccgtactatccacactttagcatacactggagcttgcttacacaataggactacatgaacttgcttatacaataggagctatgttttgttattgaatgcattccacgttaattggtactttaattttatctgtatattgcatgtaccatttgtgcactctcttgccactgtgaagaagatgaacaatttcgctaataaggactgttaccaaaatgattaaatactagtgtttcctaccaatttttgtctctcaacagtaacttctagtctaccctgtaaggcccttcattggttcataatttagatggaggtgttttaaactgtttctgtttcttgacagccggagcaccagcaacttattgttgatgctgaagctctacctcatcttgtagatctgttgaaaaggcataaaactgcacaaaattctcgtgctgtcaatggtgttatccggagagcagctgatgcaatcactaatcttgcccatgaaaatagtagcatcaaaactcgtgttaggttagcttatttgttctctaaaatttggtcactacagcaaatcaaaagaaaacttatattcacacttcatctctattttgtatgtgaaggattgagggcggtattcctccacttgttgaattgcttgagttcgttgatgcaaaggtgcaaagagcagctgcaggagcgttgcgaactttggcatttaaaaatgatgagaacaaaaatcaggctagtggctttaatctttattctgatttataaaaagtatctctgaatttcttgtgttatctgttctattagaataatttctctgatttgatttcagattgttgaatgcaatgcactccctactcttattctaatgctacgttctgaagatactgcaatacactatgaagcggttaggcatcattctgcaagttcatattactagctctttttttgtttttatatataattaggtataaagtcacagccatgcttcaagtggtagacataataaaattgtgggatgtcaggttggagtcattggaaatttggtgcactcatcaccaaatatcaaaaaggacgttcttcttgctggagctttacaacctgtcattgggttacttaggtagtgttggatcttataatttttgagtggctggtcatgtacaacttctgttccatagatgcttatcatttgcagattccatctaatggacgtagacatgctactatttggtttgttcttttcctcgatggcttctgaaataagcccttttatatgatagttcctcctgtccggaaagccaaagggaagcagctttattgcttggacaatttgcagcaaccgactcagactgcaaggttgatgatgctactgtactctattaatgtcctaaagagtagtaaaattattgatttattggcatttaaagcaacttagtctgatttatgcttgaattttttttctgatggttttgcagattcacattgtgcaaagaggtgctgtaccgccactgattgagatgcttcaatctctggatgctcaacttagggaaatgtcagcctttgcccttggaaggttggcacaggtgacttgaaatccttacagagcttctttagggtactttgttttcttgtggttataaagtaattcttctgttctgttagtagttgtcccctgggccactatttctctgagtactctttaagtttaccattcagatttattttctggcattacttgtgttgatagttgatgatcatggacttacctttcacgattattgaggttgttttcaagtatgatatgtgcctgtgacatctttgcactgtcttacccccttttccaatcaaaccttataccaaagaatattattgtagtattggttccaattagaccatgtttttctaattatttgcgagcttatgattcaagaatttactttcttatttacttgtatgtcggatgattaattggcatggcttgtcccttgatggagtggaatgattacataagattcatatgggttacccctttaggattgaggttttgttgattgattgaagtttgacttgtatacttggatgatagatcctggatgggaacttgattacttgtttttagtttgttttcatgtattaaagatgctggattatcttatatattgacttgcccacttttttaacattacttgttacgtaggaataacataaatgaataaaacaaggaatcatgcttgtgagtagtggttcctttgcaccattgtgcagtttccatgagtggtttcaattcaaaactgacttgttttcctttcatggtatacatgtatggacaattaacagttaaattcactatcttgttgttactcatcaaaaaacaataaatgctgtattgctgttcaagtggaccttatttcatgtgaaatattatatgcacatggatagggttccctaaagtagtttaaattgttgttgcttggcatttacaccttttctattgggcagttacattttatcataattttcttaagggataatgctaacgttgtgattatatcataatagtgcgtgaagggtcaaagcttggagctctttttttttcctcttaattatagtgcagtacgactggaaagtgccatggcactgggttgttcttttctttctttctcagtcaattagcgacaactcagtccaaaactatttaggctttgctatatgaattttttctatactagctcattacattccaatactcaataatctacatgttgaatatataattaaataaatagaagtggggtctctgaaacaacttaagcttttggatgaactagaaatacacttcatgatatcagggcagaaccttgggtttgagtctcatcgccacccatttaaaaaaagaagtatattcacctgcttgactcatgacaaaagaatcatccttgcatgtacagaggcatgttgaagacataattaagtacatagaaatgtgctctatctgacagtttaggagttcatgtgatttgagaattctctacatgcattctagttgattggatttattggttccctgatgttcaggacacacacaatcaggctggtattgctcattgcggtggtatagtcccattattgaagcttcttgattcaaaaaatggatcgttgcaacataatgctgcatttgctctttatgggcttgctgataacgaggtgtaacaacttatccaaacaataatgttattataaccagattttgtacttttaaatttgtaatgacgtgttacatctcatctgattcgggtgcaacttttcgctataggataatgttacagatcttgtaaaggttggaggtgttcaaaagcttcaggatggagaatttattgtccaagtattattctttttttcttcccgtgatcattattttgtgccaaattttacttaaaggagaaataatttcatagaattatgatgcttttctcattattcttaagtctttgtcatgacccttgatattgttcactcatttttcagccaactagagattgtgttgcgaagacattgaaaagattggaagagaagattcatggacgggtgagtttctatttgttgcaaggaatttgttgatgcatactttatttgttggcagtgaagcacatgatgcaatgagtacatttcttttgctaatgaatgccaagttaattttgtttttaaaagctacgaaacgtggtgtatcccccattgtccagttccttcttgtcccttcaatatggtaaatttctttgttaagtcttataggttactgatggttatatctcaaacctttttgccctcttttgaaggtattaggccatttgttgtatttgatgcgtgttggggaaaaggttattcaaagacgagttgctctggtgcttgcccatctttgttcaccagatgaccaaaagatgatatttatcgataatggtggtatgtgatctgtacctatactcagactcagtttttctcggtgtgctggttaggctgtgacagtttatccactatgtggactatgttcttgtaggattggaattgcttttagagcttctagtatcaacaaacttgaagcaccaaagagatggttctgtagctttatgcaagttggctaacaaagccagctcactttcacccgttgatgcagctcctccatctcctacacctcaggtttgctccgcagtttaatgctcatactctggcaaagtttttgttcaggtttttggttcttaagttctaacatgagtaatactagtctcttagtcactaatgggtttttatttagtttttcactgttacatggtgcttctcatatcaagttaacactaagctatgtgcatattatcatcaagcatttcgaagatgcacgctgaaccgtctgatgttcaaatttaatcattgattgtgataatttgtgaagcttttaccatttactttataaacatatgtcaaatcaagttttgctagtgttacctcaagacttgaaagttataatgtagctgtcctgcaaatttaatacaatgtctactttaccaaccatttgaattactccataaaaactcgggtcgtacagtttcttcccatattgtggttcagtttgcttctcacattgtgacccttcttgtgttatatgctgctgtttataccaactttattatgataaaacatctatttagagtatgatatgccttttatttgttcttggcatctgttatgctgatgaggggtagaagaccttagaaccctctcttgatatgctaaatttgcttcactgagcgttatttttttggttctgggagggtgtgtataccaagacttggtattcctgtcgatctcttattcaggtctatatcattgtcaattgttctatggtcttagtaatacaaaacagttgagttctgaaagcttcactcactgacccttaattgctggcatgcttggtgtatcctgagaatcaattaggcaatatgagggcttttcttatcccttcattttgaggatttagcttttgggagcaactcgtcttcactttggtgatcgtttgaggagggtttacatgttgacagattccataggctgttttcgccacagtttacttgatgttcactttctttaccaattaataatgttgtctgagctttccatgtttgttagtttgtatgtccgctttctgtcttttctttctcaattgacttataggttgttcataaccattcatggtgcagtaattagacactgtatttgatcctatattacatctcttttccttattttctccttgtgcatttctttttgcaggtctatttgggtgagcaatacgtaaataattctacgctatctgatgtgacatttttagttgaaggtagcagcagttttgtgattcaaatattgtcatcttctctatatcatggtgtatcttaatgatttttgtggtccttcaccaggcaaacggttttatgcccacagaatttgtttacttgcttcttctgatgcatttcgagcaatgtttgatggtggctacagggtaagtagaatagttggcataaagatttattgcttttacttttagatttattggtttctaaattgatcattagcaacacaagaggaaagctgtttttgctcccgaaactgattaccttacccttttgacaaatttagattgactatcagacagtcttgcaaaattgctaaaaggcaaacatcttcatttgaaatgttacaagcatatgtgtcatgtgacgtggctgaatgcacaaatatggagtacaaaactctgatgatctgttatctatttattgcaggagagagacgccaaagatatagagattcccaacattccatggaatgtttttgagttgatgatgaggtgcactgctgttcaatctctgtcacatctgggatacaaatcaatctagcaatattgaagagaggaatgtttatgtttgcaggtacatatacacgggatctgttgatgttaatatggatgttgcacaggatcttctaagggctgctgatcaatatcttctcgagggccttaagcgtctgtgcgaatatgcaattgcccaggtgagtgctggggaccttcctgtcttagaggaggatttatgtcgggtttctcctgatagtttcttatcttcggtaggatatctcagtggaaaatgtctctctgatgtttgagttatcagaggctttcaatgcattgtcattaagaaatgcttgcattgtcttcacattggagaagttcgacaaattaagtgtcatgccatggtatgtccagattcctatccttttgcttcatcatttcttggaagaaaaaaagacacgctaaacaaacatgtaattgtgtattaacacactgtaatcttgttacatgtaggtattcacaattgattcaacgtatattacctgagacacgtgcgtactttgttagggcgctgaccaggccaattcaagctgacctctgatgtagagattttggttcatttttactttgattaaatgtagaatatgatgtaaattgtacaggaagtggattttattccactcgttcttctctaattgcaagagttatgtgtaacttctcatcacttgcaattccatatttgttgtgacgtttaatgtagcgtatgaagtccagttgcgacgccagccatgcttctaaatctctacaacaagcttacaaataaattaccggttttacgaagatgtatagatttaaattatccacaatattattgggatctcatctatattgttttttcttagttgagggtctatcagaaatagtttctaccttcaagtaggggtgaggtgtgcttacactcaattctctctatactttactttgtgggatatgggaatacaccatccaactttcatactttagataatccctatctatttgctagatgtaaatgtccttgacaacttggtccatcacgttctattttgagacagcataatcaagtcgagtataaaatacatacattaattagttgtctcacatagattatgatatgtagaattggtttccctgtatagtttcggaattcatatgatacaccattactgagttgagtcaacttttaagattgagttaggtttaaattttttatttctttacatgatgagacccatttaaattcttgattcagatttttttttcgttgcttgttctttttaggacaattctttagtgaatgatcactttttgtttcttgtgcaatttacccggggggataaattacctcattgctggcatgtgagatataaattgatattccttatggcttgtatgatccttagaccaattctcattttatgatcagttatgtttaaaaatttagcgaggctcaacgttcatttaatcattttttttttctttttctatctacatatgagccaataataaggactgaaaaaaccttctatcataaatggattttttcttaatcttaaatataggtgattgcaatctcaacaccctaaacgagccgaccaaaatttggtatggaaattggacctctattcagttgccaggcccagaccattagagaagtgaactgaatctccaccgaaaatgggccaagtccaaggagtaatggcctaatggccgttttttttaagggcaaattacagaaatcacatacttttaaggcaaaattacaatttatcccttaaaaatttataattacagaaatccctcaaactgatacaataatataagcgctgatacattaatctgatgcgcgagatacattaatcgttaagtaagatacattacattttatacatgatacactaatctgatatacattttatacatgatacactaatctgatgcgcgagatacaataatataagcgctaatacattaatctgatgtgcgagatacactaatctgatgcacaaaaatgagggattttggaaatttgtaaaacttataggggataacgataataagtaaactaaaaagtggatttctgtaaaaaaaaaaatttgggtaaactgtgaaagattacgttagacaatcaatatttacacttaacagagcactcataggatccgaatcagaactagagtgttaatcatctccaacctcatactcagtaaaaaccaattagttacaaatttctgaattatataactatatttcctagagccttttactagttctatcctttctataatctcctttgttaatctgtgtaacaactaactctgtatttacatttaatcaatttttaagtgttttcagtttcttgtcttccccaaaattgtagttgccagttcctttatggattgtcgtcaatttctcctttttatccatattgaacatggataacaccttctttctctgaactcaccattgtgattgttgttatccacatacattttaaaaaaaataaatagatgcagctaggactcctcattcacacaaacaacatatttgttcattctctcctttatcaatagttatcttgatttgccagccagagtagaaatctttgtctagatagtaaaatagagctcaacatatcaacgtcctttactctctccaagttgatttaataaaaagagcactaatttttctataaccatagatagtttaattttaaaactcttatttggccttagcaactatgacacaaatataatgacatgtttaagataatagatttcaaaagatcttcttttctttagtgacggagctaggaatttcaggaagagggtccaaacattaaataacaaaagttctttttaaaaaggggaaaatattgttcaaagtgagatttgaacatgtgagcactgactcattaaagatgtcgaaacatacattcaagacatcttaaaccactaggctataacaacctattatgtcaagggtgtccaaaatatgttatttaatcacttcgtatataattttacttgtatatgcggtatttttttccgaccaagggtgtccaattggacacccttgcatacatgtgcctacgccactgcttttcttcacgaatttagtaaccaataaaatagtttcacataaaatgaacatgtcaaataatacacatattaataatatttatttaatttaaatctttcttatatcaaataaaactccacaattggcaggcatgaaacacttacaaaaaatgaatatttttaatatgcatccaaatgatattcatgaatcaaaaagcctagaagatgaaattcttgccttccacaccactaaaagtgaaaacaaaaaagcgtaaagaaaatagaagaagaaaaaacactatggaagaaaagaattactctatcctttttggttaaaactataaagtactcctagtataaaatacactcaaaccatggtaaataaaaaataaacaatggcttctctgcgttttccattcttgttttctcagccccacaagactccgtcttcagccacttcagatgctccatctcgatccttctccaccgtcgctgtcgccctcgcgtccggcggttcagccctcgctgccgccggagcgatcattgccataactcaaagccccaaaaatccgtttctggaaaatgctatgaatttcctactttccaatttctcacctaacaaaaatcattcatcccctttgtggggttctgtttctctagcagataactcagctccggtcactgaatccagggccggaatggcatttccgtcaattctgaaagatactcagcgactccttggaattgggctgcgtaaaaaggcggtttttggattgaaaaacattgatgtctatgcttatggtaccaaattgtcactgcaatttacttaattgtttttgctctttatcgatttatgtttctgtctcttctgcaaatgttgttatattgtagttgaggttcttaatttttatgatccttgtgtggagcaccaaatgctcaaatatataaaatgaattccaattctatggcaataggaagttatggaggaaatgttgtctcacttatccttccatactagtaattgtagcattacattttttttctccagattttattccttttttattttcaagatgtattttgtcgtggcttcttcacttctgttattcttttcccgagctgctttgttatgttttttcttgatctaagggcatatggaaaacaatctctctactttccaagctagggataaggtctgagtacacactacactcccagtcagaactcaattcatgctttaccatttatagcagttcatgtgggatcgtgggcttatcaattgttaacagcttgtgtaggcttatcaactcatgcttactgtacatgttattaagtttttgaagcaacataatacagtttcttgcaccgtcagtgccagtggtggtgccaggaagttatacaagggattcaaaaaaataataggattctcatacatgagatttgaacataggtcttaaagtaattgtgttacccctttgccactttactagaattttgccttctatctaggggattcaatagtatcaaggggtttcaatagtgaaataataccaatatagaattcatttttgctctatttgttcaatgtaaattttttaacgaggggaagttaattgaatctcctttctacaacttagctccgtccctggtcagtgcataaaaattaaacctgtggtggtatcatatttgagaatctcatcgtcatctctattggaccttcctttatatgatcaggggggatatgcattataacactctttgtctccttttggaagtttgaatctgcatttcaaagtaaaagtgatgtttactttaaatatggcctttatctaatgtgatatcaatatggcattctctaggtgtgtatgctgatgatgttgatgtaaagaagtgtctggctgagaagcatggacggcactctgtttctgaactgcagcaaaaggaagagttgagaaatcatctcatggaaaacgatatacgcatgactgttaggcttcaaatagtctatggcagactaagcattaattctgtgcgcagtgctttcgaagaatctgttggcagcagattacataagtttggaggatatgataacaaggaattgctccaaaggtaattccttagcctcatattattcatatcttattcaaccttttttggaataattaccatatcaccacagggaaacaagcctgccaaagctggatgaagcacttcatttgtttgcactctaaattattatgttttatatgtattctggaaccttactcaagttgcctttcaaatatgatgccttgcgatatcatagtgtttaacattattgctggactcttttgcccaactgtgatcaattatctctcagctacatacgtaacatcttttcttgaatagagttattgagctgcgaacaggttaacccacaagattttttttggaaatggaaaatttattgtttctcaatccttaaactattattgcctccttcctatctatctatatatcatatatatatatataaaggagaatgttagacttgcttatgtggcatgcctctaagggctagaaaactatttatcttttttgtggtttttttgtattttttatttatctttcaaattttctcctttataatttgaaggcacaatcattattattattcaattaaatgaacaatgaatatgtgtaaatattcggttactgatctttcagactttcacatcctacgtttttcatattcccataaaattaaatacacatttactgttctcctacaaatacaaactgaggtgttgggtcttcattaccatttttttttcatttttcatttcatgtatcccaaccaccatttagttatttcttttagaatatgatattgtgtgcagattcttttgagaatttttcataccggctaacttagttacattttttaacatatcttatgataatatttattattctttatactttgattattgtattatatattttgctatctttattgtttctttactctagaatattttatcaagctttttatattattttgttatgatttctttcatttcgctgtttttttcttgatatatttttccttgagtagaagtctatagaaaacatctctacctccaaaagtaaggtaaagacactctaccctcccccatattatttcatgttcatgtgctaattattttaattcccaattaaagtgaataattatattagtacgtataaatgtatctcctcaattttttcattcatctgtcactacaatttttcagtcttgcaattttcctcttaggcctaatagtagtctatgatttatattttttttggttttattatctctatatgtgtatatgatggagtgttagttgtctatgtagattatcttattcaattttgtatgatctgcgagtgtattgtatattacgcacataagtgatctattttattaaagtggtgttgtaagctactaattcttgataggaagctaaaggaagaaataaaatcacaaaaaaaattatgttttaatttctttgttttctttattcttaattttgacatttttaatttagagtatattaatttggcttgaattttattatattgttggtagtaacttaaatttgattgacatgtaatatgtattcaatattagtattatttgatggacatgaatgggattgcttatttacttaccatcatcacacctttctaattctactcttatacatttataattaaaactttttttattcatagacaaatttattatttacttattcaccatattgtgactaatggaaagcctctagcaataagaataaattaacttttgttcttttttgcatttgcttcttttcaaaataaatctgcccaacaatctttttcaacctctttaattatatcatttatatgtttttcttaaatatttttaaaaataattctcattaatcttgattcttaattaatctcattaatttcttcttaactatctttagaatggtgacgtttcgaaaatgaagggtagtgcaggaagggtagaggaccattcatgtacccctatttactacttcatattagtacgtataaataacaacaaaattcaataaagaccttcatcttctccacatcatgcccctcttatacattgctatatatcatatggtgcttgtttttgtcagatgttcaataccttttgattgagaagagattataccatcacgttgttactttcacttaatgcttacatgaagattttactgaccacttctctttgatagtaataacttcacattcgactaaaatatgaaaaagatagagcatatgaagattttatccttattttataagatatatattttatttgaaatatctaatatttgactccaaataatttgtcacaatatttcaaattttaacgacgagacacgaataaaattttacttttttttaaacaagtcacgatattcttgtgttagccaacaaataaccttatttgtattgccctcaccttttttatcaccttattttaaagcccaatattctcaactttcgtctttcttctgtaattttttatttattactagctcaattggacatccatttgttcctatagttatttatttaaaatatttaatatttattttatatgttttaaaattatggtcttaaagaggtgatatagacaatacttcttttaaattggaaattacatttattatttcttttttaaaatctacctactaatagaatatttttaaaatacatttactactattaaagtaaattttaatgaaattatttatgaccgcgcgaagcgcggtttagtttactagtatatatataaaggagaatgttagacatgctgatgtggcatgcttctaagggctagaaagctatttatcttttttttgtggtttttttggccatttttcaaattttaaaatacaaaaaattcacctaaatattaaagatagtcacatttaattctttctttatcaatagtcctatttaatctattttatcattaaatgctattattttcttttccttaatatttctcatttttttctttttagtattttaatttcttccctaatgatatttatatcatttctttaaatcaccttttcccccttttagttcctttttacttctttttttaatttatccaattcaagaaacttatatttctataaaatataaagtcttttttaaaaaaaataattaaattacgattttgttttccttaagtcacttctcttcctttccttgttctttttttacttttttatttatttattcaattcaagaaatttatatctctatttagtaaaggtatttcttttatcttttttatttatttttttccttctttatttacttttaaagtttcacctccataacttatatctattaaacttctattcttaataatataattaatttcatgacttttaagttttcatattcataaccccccaactattaaattataaaatttaagatactttatgatatttctccatttttgtcaatataaattcacaagttttttgtttcatgaaattactactcaagattatttttatatttcattgttctttgtagtattattctattatcaaatccatgtgttaacttgacacgatgaagaagactcttgaatgttgattaatttgacaaaaaaggtgtcggccaagagctcaaaaaagtgggcacttattttgtattcttatttgtttagatgcaaattagttattgtaactttgtgtgtaataatattaactactgaccaatgttcaacaatattattgtacaaaaactatttttgtttttttttaaattcctctattttgtccatataaaatcataatttttatttcatgaaactcctactcaagattatcctttttatttcatatttgaagtcgtgttttccatgttttgttattgtagtaaaggtagactcaataaagaggacacttagatattgatcagttagtaagagggagtgttgacaagagctcaaaaattgtgcattgattcattaatatttttttaaaaatctattttcttatgattaaggtcctaatgaaggaatgtgcattgtgttctttctatgtaatttcttagtttggaaggtaagagcattcgaaaattaattaccgtaactttgtcttatgctaattattatcaaggttcaaacactattattgatagcttagagaatttgaatatatatcaaatattgaaatacggcttttttatgatatttttttacagtacaaagaaccatttatgtttcttatgattaagatcctaaggaagatgtgtttttgttactataaaaagttactattaagtaggatagaggaaggaaccctcaggggttggcctactggcaattgacttgagccttggggtttgctccctttcaaggtctcaagttcgaaacccactgggtgcaaacaatttctgagggccatcggactgggtaaaacctgaattaaccgtggtgcacttgcgggaaactccttgccgagggcctgtgcacccccgggattagtcggggctcaaagagactcggacacccggtgcaaatcaaaaaaaagtggatagaggaaggaaaagagaaaaagaagaaaaaattaataaaatagaaaacaaatactacaataaaggatagaggcaaaattaaaaatatgaatatttatttagataatgatgaaaaataagaggaaaaataacaacaatgaatgaataaaattgacacctctctttggccaagaatattgttattattataataataataaaaagaattgtgttagttactatttctgcattcatttttattctttattgtaaaaatctgaatgtctataaataaagacattgtaagactcttctgaaatgatcacattagagtttgaaaaattgtgcattaatttcgtattttcttcttccttttcttaataattaagatcataagaatgatgttgcattatttatttatttatattctctccataattttatttgttttatattttatacagattttttattatcgtaagtttataattatttttggtccaaagtaacaacttatgactttgttggaagtcatataattactgaccaaacatttctctttatgaaatcacttatacgtctggatatatattatatttatgcacatattataaatatttcttctatctatattatattttcataagttccctagttcttatataaccaaaaatgtcttttgcaactgtaggttcacttcccagtttaaagatgaaattaaattacctcggggatctatcattgaactctccagagatcatgactacatactccacacaacaagtaagatgatttatttctgttgacagtattttggaaatgaacagctcaaagttctgtcttttttccactttttctacaatattgatatttcgatctgatacgaatcttttgaagtgaagactctcaatctctcagtgtatacgcctacgagacgtgcatgtgtgtctgtgtgttttgagaaaaaataaaatgttatagctatcacttgctcaaattattgaagagctattgaatggatacataaaacattaatttcttttagtcatttccctaataaggttggctttcgaagcagtatgttagaggctacaatgaagagaaattacttcaagtgagcgctatacaagaacaataccataaatatcctaattgcactgtcagttggcacattttatacccttacatttcctttgtgggaagtggctaaacattttcctgaatttggttacagaagtcatgctggaaattatgcttgtgtagtattacaccaatcaaccatccctattctcttttatacagatatagattttctggtctttaccagcttcactgtctataaaaccaaaaaaataaaataaaaattgttatatgttagctgttgaaaatattgttatatgttagctgttgaaaatattcttcaccaagatactagtgatgatttttattatcagcctgttagctcttgaaaatatgcttccgcaaaatactagtgatgatttttattaccaatggctgatacacctgtcacagtgactaataaataagttaaagacattccatattaaaaaaaagacttaagttaaacagcatcgaagtattggttgagatttgttttacatgcattttaggtaagaaactgatgagctagttaatttcccgtcagttccatagaccatagaagaataactaaaatatttgttggttttctttaaattcacaatatattagtttctgatcttttttctttctagttgtttgcttaaagtttgctctagcatcaatcacttagatgaagcttaggttctgtttatttttcttttgtagttgatggaaaggaagtgggaagcatacaaagcaaactcttatgcagatcaatcctagacctatatattggcgatgagtcatttgatcacaaagccaacgaagatgtcgagtcgaacttggcttctctacttcacaagtagctacttctttagcataaagagaattttatcaacacgaggaattgagttgtggtgatattggctagtttcaactgttgccccccctcagaagttctacataactcatgttaggttctattggttggatgattctctttaaatagttgaagtagagatttaatctcttgcaaactgaacttagatctatgttatatgctgatgagtggttttctctactcctgtaatattttgctttgaaatttttatagcataattggcttggtcaccaaatttgttttatttacctcattgaaatgtatcttggagtgtttactactaaggttggagaacaacttagataaccttagtagtgtttactgctaaggtttcttattatcatcttcttgttgtttacatttgttgctagtgtctctttttcactgtttatccagccatggtctttcggaaacaacttctctaccttctcaaaggtaaggtctgcgtacactctaccactctaccctcctcccaagaccccacttgtggtattacactggttttttttttttgctactaaggttattttgcctggagttagcacgatgcagatacaatttttcccaaagaaattctttggagagacagatttttttctttcttaattgaagttatatccagtcacactgaaataagtattacacttagcatagctttcttagagcatgcaacacattctactcatacaattagctcaattcatgcacaaattgtgagtgctactggactcccagatcagccttggctctttattcactcaaacatcatggtgcattcagcagcagaagtctgctgaacagttatatactgatagttcatgcaaaagtgctgctacaacatcccttgagttctaagtaactccttttgaatttccagaacacctattgtttttctgttttggaggtcaagtcatgatcttcacaaaggaagccgtgtttctcttctcgatgatggttgttttttatttattcagcacaaccgtgattggcggcacagtgtacaatgttggtgattccggcagttggaatggagacaatgttgacttccatatgcgggcttctagtagaactttccaggttggtgacactcttggtaagtccaactagtcgatcaactgggatctagtatgagaaaatcaaatgcttcacaattcgaacagtgtataaaataaattagtaattggctaacgttatgtgaagttgtctcccttgttggaaaaatactacaatattgatactgtacaaaaaatacaaaataactacactggagcttgcttatacaataggagctattttttgttattgactacatgaacttgcttatacaataggagctatgttttgttattgaatgcattccacgttaattggtactttaatattctctgtatattgcatgtaccatttggtctatttgtgcacttacttgccactgtgaagaagatgaacaatttcattaataagggctgttaccaaaatgattggatactagtgtttcctaccaattctgtctctcaacaggaacgtcaagtctatcctgtaaggcccttagtcatttatgggtttttatttaattttcactgttacatttggtgcttcttgcatcaagttaatactaagctatgttcgtataatcatcaagcattttgaagatatacggtgaactgtctgatgttcaaatttaatcattgattgtgatgatttatgaagcttttaccatttactttataaacatatgtcaaaccaagttttgctagtgttacctctagagtcgagacttgaaagttataatgtagctgttatgcaaattttatacaatgtctactttaccaaccatttgaattactgcataaaaactctggtcgtgcagtttcttcccatcttgtggttcagtttgcttctcacgttgtgacagcttcttgtgttatatgctgctgtttataccacatctataatgagaaaagcatctatttagagtatgatataccttttatttgttcttggatggtatctgttatgctgatgaggggtagaagaccttagaaccctctcttgatatgctaaatttgcttcactgagcgatatttttttggttctgagagggtgtgtataccaagacttggtcttcctgttgatctcttattcaggtctataaccttgtcaatcttttatggtcttagtaatacaaaacagttgagttctgaaaactccactcactgacccttaattgctggcatgattggtgtattctgagaatcaattaggcaatatgagggctttgcttatccctacatttaaggatttagattttggtagtaactcgtcttcactttggtgagtgttcgaggagggttcgcatgttgacaaattccataggctgttttcgccacagtttacttgatgttcactttcttcaccaatcaataatgttgtctgcttttcatgttttttagtttgtatgtccgctttctgtcttttctttctcaattgacttagaggttgttcatgaccattcatggtgcagtaattagacaatgtatttgatcctatattacatctcttttccttattttctcctagtgcatttctttatgcaggtctatttgggtgagcagtatgtaaataattctacgctatctgatgtgacatttttagttgaaggtagcagcagttttgtgattcaaatattgtcatcttcttcatatcatggtgtatcttaatgattttttggtccttcaccaggcaaagggttttatgcccacagaattgcttactttcttcttatgatgcatttcgagtaatgtttgatggtggctacagggtaagtagaatagttggcataaagatttattgcttttacttttaggtttgttggtttctaaattgatcattagcaacacaagaggaaagctgtttttgctcccaaaatttgtcttctactgcttacctttcccttttgacaaatttagatcgactatcaaatggtctttgcaaaattgctaaatggcaaacatctttctttgaaatgttgcaagtgtgatgtggctgaatgcacaaatatggagtacaaaactctgatgatctgttatctatttattgcaggagagagacgccaaagatatagagattcccaacattccatgggatgtttttgagttgatgatgaggtgcactgctgtttaatctctgtcacatctgggatacaaatcaatctagcaatattgaagagaggaatgtttattgtttgcaggtacatatacacgggatctgttgatgttaatatggatgttgcacaggatcttctaagggctgctgatcaatatcttcttaagggccttaagcatctgtgtgagtatgcaattgcacaggtgagtgctggggacctttctgtcttaggggaggatttatgtcaggtttctcctgataatttcttatcttctgtaggatatctcagtacaaaaatgtctctctgatgtttgagttatcggaggctttcaatgcatttgtcattaagaaatgctttcattgtcttcagattggagaagtttgacaagttaagtgtcatgccatggtatgtccaggttcctatccttttgcttcatcatttcttggaagaaaaacagacatcctaaacaaatatgtaattgtgttttaacacactattgtcttgttacatgtaggtattcacaattgattcaacgtttaatacctgagacacgtgcgtactttgttagggtgctgagcaggccaattcaagctgacctctga

SEQ ID NO: 136 - protein, 708 aa, Solanum tuberosum
MENQKLTERSSSSARRSLKRKLEEDLQDDRKVSPSLSSEDGHQDLEREVRTQVEILESSFSSSESDRASSKRAIHVLSEFAKNEEIVNVIVDCGAVPALVQHLQAPPHVNEGEGSHMPYEHEVEKGSAFTLGLLAIKPEHQQLIVDAGALPHLVNLLKRHRDAQNSRAVNGVIRRAADAVTNLAHENSSIKTRVRVEGGIPPLVELLEFVDSKVQRAAAGSLRTLAFKNDENKNQIVECSALPTLILMLRSEDTAIHYEAVGVIGNLVHSSPNIKKEVLLAGALQPVIGLLSSSCSESQREAALLLGQFAATDSDCKIHIVQRGAVPPLIEMLQSPDAQLREMSAFALGRLAQDTHNQAGIAHCGGIIPLLKLLDSKNGSLQHNAAFALYGLADNEDNVADLIKVGGVQKLQDGEFIVQPTRDCVAKTLKRLEEKIHGRILGHLLYLMRIGEKVIQRRVALALAHLCAPDDQKIIFIDNSGLELLLELFDSTNLKHKRDGSAALCKLANKASSLSQVDAAPPSPVPQVYLGEQYVNNSTLSDVTFLVEGKRFYAHRICLLASSDAFRAMFDGGYRERDAKDIEIPNIRWDVFELMMRYIYTGSVDVNLDVAQDLLRAADQYLLEGLKRLCEYAIAQDISVESVSLMFELSEAFNALTLRNACILFILEKFDQLSVMPWYSHLIQRVLPETRSYFVRALTRAIQADMRV

SEQ ID NO: 137 - protein, 709 aa, Solanum tuberosum
MENQAKRSKQSSSSGRRSLKRKLEGDFEDDRKVSSPFSHDDDDAHQDLAPEVRTQVEILESTFSSTEADRASAKRAIHVLSELAKNEEIVNVVVDCGAVPALVKHLQVPSLGSEGDGGQMPYEHEVEKGSAFTLGLLAIKPEHQQLIVDAEALPHLVDLLKRHKTAQNSRAVNGVIRRAADAITNLAHENSSIKTRVRIEGGIPPLVELLEFVDAKVQRAAAGALRTLAFKNDENKNQIVECNALPTLILMLRSEDTAIHYEAVGVIGNLVHSSPNIKKDVLLAGALQPVIGLLSSSCPESQREAALLLGQFAATDSDCKIHIVQRGAVPPLIEMLQSLDAQLREMSAFALGRLAQDTHNQAGIAHCGGIVPLLKLLDSKNGSLQHNAAFALYGLADNEDNVTDLVKVGGVQKLQDGEFIVQPTRDCVAKTLKRLEEKIHGRVLGHLLYLMRVGEKVIQRRVALVLAHLCSPDDQKMIFIDNGGLELLLELLVSTNLKHQRDGSVALCKLANKASSLSPVDAAPPSPTPQVYLGEQYVNNSTLSDVTFLVEGKRFYAHRICLLASSDAFRAMFDGGYRERDAKDIEIPNIPWNVFELMMRYIYTGSVDVNMDVAQDLLRAADQYLLEGLKRLCEYAIAQDISVENVSLMFELSEAFNALSLRNACIVFTLEKFDKLSVMPWYSQLIQRLIPETRAYFVRVLSRPIQADL

SEQ ID NO: 138 - DNA, 8623 bp, Solanum lycopersicum
  source 1..8623: mol_type = genomic DNA
gtatcacaccttttctcctcttcctcatttcctctctcccatggagaaccagaaacttaccgagcgttcctcaagttctgcgaggaggagcttgaagagaaagttagaggaagatctccaagacgatcgtaaggtttctccttctatatcttccgaagatggtcatcaagatctggaacgtgaagttcgtacacaggtcgagattcttgagtcatctttttcttcatctgagtcagatcgagcctcttccaaacgcgctatacatgttctctctgaatttgctaaaaacggtaaccgatttgcatttcattttatactggatcagaattttaggtgttcatgccgagagttttcttgctttttctttaatcgttttgggagtggtattaggttttgatatttgaggatttgtgttttgtagaggaaattgtgaacgtaattgtagattgtggcgctgttccggctttggtgcagcatctacaggcgccgcctcttgtaagtgaaggtgaaggtagtcacatcccatacgaacacgaggttgagaaaggaagtgcttttacgcttggacttcttgctataaaagtaagcatccagttcgttttttttttgtttttttttgtttgatatttgttagttttctctgcgtattataagtacaggtactgtaaaataaactagttacttcatgcatatgattgcatgaattatctcatatttctggtgaaacgatcttgcttgtgcgcaggggctatgtattaaatggaataagttactgtaaatgggattttcattttgctgttttcttgaacacttgtttaatttgttcgtgcattcctttgcggcaagtgaagaagacacaagttttatttagcaatggcatttaccaagtgtgtttctaggtgatcattgaggaactatcagtatgactttactggtagcggcggatctacagtagcggctgtgggttcctgagaactcagtaacttcttccgaaaccctataattatattgaaaattcttttaaatatataacaactagaagcctagttccatggcaaatagaggaacgattgaaccgcaccagcgccagtgtgcgcaggtatggatcccccaagatcagtgttactaaaacataaaatatctatcccataaacttaacatcctggatcagtgttgtgaaaggtgatcgcttcgtcgccaatggcaagaggcaaggcgaggcgacccttcatcgccttttagctttgtggtgaggcgatcttcaaaaggcgatggtatgacgacaaaaggctagaggcaaggggcgagaaaggctagaaaggtgtcaccttttgtattttcttaaaaaaaaagcgaccaatctagggttttgaaagttaaaaggtaattttaggatttttgactagactccttcggcaactacccaggcttttccggtgactccaaagtctaaccaatacatatttcttctttttttgagaaagttaacataatacatatttcttcttttcttcttcagacttgagtcacttctacctttgttttgacttttgttcttttctttctcattcaagttctagacttttagtatgtactatctatttttactttttgaattgaaaaaattgctaatatgttattgtttggttatttacatatgcaataaaatatttacatatgcaataaaatattttaattttttggtattaaatggtgccgcacttcaaaaaggagagcgcctcgccgttcgcctcgcctcgtggcaaggcagacccttgtcgacttttatcgcctttcgacgtccaaaacaatatcctggatatgcctttgactttacgtatctcttagactctgaagttatctattaacaagaaagggtaatagaatgctgatctcttaaagattattttgtgtgcaaatcaaaataaaaggtattaatgcacagtagataatttccaatttggaacatgtgcagatctaaattaattgcaatcaatgtgagtgctttgagtttaattgtctggtattactagatttatgttctacttgaaaaagaagcttccagaattgttctttcgatgagatttcatggcatatagataattttccatcatcacaatctcaactaactcatacgcttggatcgtttgcgtttttattgatgtactttctgaaatttttgtctctcataatcctgctgaaaagaaccttgcttctcctctacttcattcgttactttctgcttccatcagaggagtagatatttactctctttctatgttttgaacttatgtctgacagccggagcaccaacaactgattgttgatgctggagctttgcctcatcttgttaatttgctgaagaggcatagagatgctcagaattctcgagcagtcaatggtgttattcggcgcgcagctgatgcagtaacaaatcttgctcatgaaaacagtagcatcaaaactcgtgttaggttagtttattcttatctggaaacattgttatcacaatatctatggaaataagacctctttttcttacttcatcagttcatctgtattttatgattatagggttgaaggtggcatccctccacttgttgagttgcttgagtttgttgattcaaaggtgcagagagcagctgcaggatccttacgaacgttagcatttaagaatgatgaaaacaaaaatcaggtgaatggcttacaaaatttatcttgaatatctctatggtcacgtcttctatttaagttaatttatgtgaattgattgcagattgtggaatgcagtgcactccctactcttatactaatgcttcggtctgaagatactgctatacactatgaagcggtgagacatcattcaatgtcatgctgaactagcatatatagagtaatgattgataatacctaggatattggctatttttcgtgtagtagtcatccccagaacttaaattgtgggtggcaggttggagtcattggtaatctggtacactcgtcaccaaatatcaagaaagaagttcttcttgcaggagctttacaacctgtaatcgggttgcttaggtatactcaactcttatatcttttgagcaatctgatcatatgaatatttcgagtctgtagtaggacctatgtagttgtatgctccctcttcttttgatcaactataaatcttgtatgccagttcctcctgttcagagagccaaagggaagctgctttactgctaggacaatttgcagcaactgattcagactgtaaggttgattaaaataataagctctgttactgtcttaaatggtgaaactctttagttaagtagcattaccgagctactttaatcattttttgcacatagtttaatctgtttgaaactcttgcagattcatattgttcaaagaggtgcagttccaccattaattgagatgcttcaatctccagatgctcaacttagggaaatgtcggcctttgctttaggaaggttggcgcaggtaatttctcttggatgatatcttgagtagctttccattcccttgtctactagtagcagttggtctattggttgtctgataaaatcttgctattcaagaatttcttttccgacactcatatgttctttgggatgatccatcacaaacttgtatttgatgatttctgatattgtttttcaagcgtgatccctttaatatgtattgtctacattctataaagaaaatcttatttcttgactgtaaagaatggaaaggaagtgaagcatgttgtgattggtgtccccattgggctattggttatttagctgctgcaaaagtctttattttaaaatgtttgtttctgacaattatttctaaatgagcaaccgttttttcacatagttgatatgatacctacctcggggtatgttcaggaatctctaaggcctcatttgttcgtacttaatgaaagtctgattttgaaccatttagatgtggtaaaacaaacaatcttaatcattcaatcttgaaatctaaagacaacatctcaatctttcatatctggagtcagatttagacgctttaatcttaatgaaaataaatgaggcctaagagaataagagattggttcttttgggcacaaaacttgattgaaggacaatagtaatgattttccagtttggaagtttaatctacctaaacttagtggaagctatagtgctgactctgagcaaaatcaaagtggggtttgaagggtattattttcatcacttagtctttgcagctgctcaatctcttgtgatttatagtttctactgatggtctcggatttgtaatattttctcatcagtagctctgttttagatgtagatagattatatgtgccttgttatctcacaattttttggttcatgttttacagtcgcacaataacagttgtgaagagtaagactgattgaatgttattaaaaaaaaatttgttataaaaaaaaagagtaagactgattgaatctttaattgccctagcaaattggaatatcaagatgctgtgatgtttctaatgtttggtacatgagtatattaactctactctctttggagctctaatttaacttcagatgtgatgattgatggtgcaagaacatttcctttgctcatagtacttaatttgatttgaggatttagtacgacaatgtgaccgggtgttagtgattccatgatgttcaggacacacacaatcaggctggtattgctcactgtggtggaattatcccattgttgaagctccttgattcaaaaaatggatcattacaacataatgctgcattcgctctttatgggcttgctgataatgaggtgttgcatgtcatcagatcatatatgccttgattataattaatttcatgcacttacatgcttctttagacttactgtgactttgtgctataggacaatgttgctgatcttataaaggtcggaggtgttcaaaagctccaggatggagaatttattgtccaagtatgatctcttgatgtcttttcttttggatttttatgttttttctcaaggataagtacctttgttgctttaaatgagtttgcatcattctctttttacatattgccctaagttctaaattgagttcctgactatgcagccaactagagattgtgtggcgaagacattgaagagattagaagagaagatccatggtcgagtgagtttctatttcttaaattatttgttttcgtcttcagatgacatgaatgcaacttacctcccttctccacaatttgatttttcttttatgttatttcttttgttaaatcttattaggttatttgtgagtacaatatgtaatatctttctccttctttggtagatattgggccatctgttatatttgatgcgtattggggagaaggttattcagagacgagttgctttagcccttgcccatctttgcgcaccagatgaccaaaagatcattttcattgataacagtggtatatgtttgatttgaacttaagattgctttttaatacgttctggtgaggcagtgacaataactttctgtttgtttatgcacttgtaggattagaattgcttttggagctctttgactcaacaaacttgaaacacaaaagagatggctctgcagctttatgcaaattggctaataaagctagctcactttcacaagtcgatgctgctcctccttccccagtacctcaggtttgtttatcttagtctccattctgattgcactactaagattcttcaaatatttgctttgagttagttttgactattagttggtttgtttaaatttctccacttctgtacatgtagtgcttagtcaggttgtcatcatttgacgagtctggaacctatatgatggacaaaaagacacaattgaccaaaataaagttgaaattttctacatatagcgtactaatttagtgcactatatgactcccatgaacagaccaggccttaaaggttactaaattggtgcgttatatgttgaaaatgtcaaactttattttggtcaattgtgtctttttgttccatcatttagtaaagggaggtaaaactctctgaagtttataaaatatagctatgcaaatttaatatgtttggtcatttttcttcttgtttctaaatttaaatgatcatgcctatagaccaatttctaaaaaaaaattcaaggcagtgtgctatgcagactcaaaaatttgacctcctacctccaccccccaaatagttatccaagactagaaacttgtagtgcgctaatgatgtttttacaataggcagacaccactttcttggtctttgctgcctgagctggagctttagactgtttgagagatatattaggtattgggcaacctctcttggcaaagaatggttttcctcatagagagggggagtaaggggttttcttttgaatcagaaaatgttgtttgtagagtctctttctgttcaggtcttcaatcatttgatttgggaaaatccaacaatgttgatatgtaaaaattgaatacatgaaaattagccctggagcatgtgctcaaattgtgtcgtttctgcctctaggtttatgtgttaagtaggacatgaagtgaggctagggcggttcttctattttgaggatgtagataatgagaggaacttttgatgaatctggaagaatacgagtgctttacattttttatgaaagcttatttttttaccaccctatattggctattaggtgctgatggcgttgaccattttctgttccttatttggctgattgtatccattcttccgttcatattttatctcaattgatgatgcagcttattccatcctgatgttgtatctcgtcgcctcatttttttctcttctaatttcttttaaatccaggtctatctgggcgaacaatatgtaaataattctacactatctgatgtaacatttttagttgagggtaagagtggttctattttttaataatgtgactctcttccccttttcctttttaatgctctactaacttttttgttcattcttctaccaggcaaacggttttatgcccataggatttgtttactagcttcttctgatgcatttcgagctatgtttgatggtggctaccgggtgagttatagtctgccttttatgttctatatttattcatttccgtaaatgctatgatccattgtaaagatctctctccaattttaaagttgacatcttgcttaagtgtaagggtagaggagcaggccattatccattgagttttgaaccttgcacctaatatgttttattttatcttctttttgtttgtgtttgctagccagtttatcaaccaaacaaagagtaagcctgttattgcttcaaagttttcattttcttttattgtcttcttttctatagatgtaactcttgctgctttgatttgtcttactctcctttttagtttgtgtcaaaagaacgccttactaccctttgttcatgtctttaattccacaagattcaagggcattttggtacattacatgcatgtgtatctttagtttaagaccataagattcagaagtcatcattttaaaaactttgtacccagtcaaattaagatacaatgaagtggcggggggggggggggggggtttatgagaaccaagatagtgtatgcatggccattgcaggaggagtcagcccaacatttttggttgaattttgtcagcgtatctggggttatgttgatacttttgtttctaatagtttgtagtaaacgcattgcaggagagagatgccaaagacatcgaaatcccaaatatccgatgggacgtttttgagttgatgatgaggtagtgatctttaattaccattttacatcctcagtatagatcctgtaagtcaatcttgcagttttaagaactatctttcttgcttgcaggtacatatacacaggatctgttgatgttaatttggatgttgcacaagatcttctaagagctgcagaccagtatctattagagggccttaaacgtctttgcgagtatgccatcgcacaagtgagtgctgagctcttttgggagtttggggggttttcctgtcacatttatgctctaatgatttttttcttttctaggatatatctgtggaaagtgtctctctcatgttcgaattgtcagaggcatttaacgctttgactttgcgtaatgcttgcattctattcattttggaaaagtttgaccaattaagtgttatgccatggtatgtcctggacttttctatccttaattacattatttttatgggcttttggtgcatggggaatcaagcttggatgtcctatttaatttatttgatgtgaaaaattgtggagcatgtcattgatccaaaaaatgatacatgaactgattgagaatgtggattttctctaacatgatgcggtctcccatgcaggtattcgcatttgattcaacgtgtattacctgaaactcgaagttactttgaaagggtgcttaccagggctattcaaaatgacatgcgagtctagatgtttcagattcagttttgtttttttattaattgtaaccgggggaaggtagtatgtacaggagtggttactattgtaatagtctcaaaatgagcg

SEQ ID NO: 139 - DNA, 7521 bp, Solanum lycopersicum
  source 1..7521: mol_type = genomic DNA
atggagaaccaagcaaagcggagcaaacaatcttcaagttccgggaggagaagcttgaagagaaagctcgaaggagattttgaagacgatcgtaaagtttcttctcatgatgatgatgctcatcaagatctcgcttctgaggttcgaacgcaggtggagattctcgattctactttctcttcgacggaagcagatcgtgcctctgccaagactgctattcatgttctctgcgagttagcgaagaacggtaactcaatatctcgtttctagccgatttcatctacatttctgtttatcgggagttaattcaactaatttcccaagttaaactctactggatttattcaaaaaaaattttcttcttcttaaaaaatacaagttagtcagtcttatagagtgctgaatgtacatgcagagagtttgatttcaatcagtttgggcctggaagttgggttttgatatttttgaggatttttctgttgcagaggaaattgtgaatgtggttgtagactgtggtgctgtcccagctttggtgaagcatcttcaagtgccatcccttgggaatcaaggagatggtgggcagatgccgtatgagcatgaggtcgagaaaggaagtgcttttacgcttggccttctagccataaaagtcagtataaatcatatttattctcttgagagttaagcacaactgagaagacaattttcgctattagggcagatgatttctttgaattactctgcactatccacactttagcatatactggagcttgcttatacaataggagctattttttgttattgactacatgaacttgcttgcacagttggagttatgttttttcattgaatgcattccacgttaattggtactttaatttcatctgtatattgcatcatgcatgtaccatttggtctacttgtgcactctcttgccactttcctaccaatttttgtttctcaataggaacttctagtctatcatgtaaggcccttcattgattcataatttagatgcaggtgttttaaactgtttctgtttctcgacagccggagcaccagcaacttattgttgatgctggagctctacctcatcttgtggatctgctgaaaagacataaaactctgcaaaattctcgtgctgtcaatggtgttatccggagagcagctgatgcaatcactaatcttgcccatgaaaatagtagcatcaaaactcgtgttaggttagcttatttgtcctctaaaattttggtcactacatcaaatcaaaagaagacatatattcacacttcatctctattttgtatgtgaaggattgtgggtggtattcctccacttgttgaattgcttgagttcgttgatgcaaaggtgcaaagagcagctgcaggagcgttgcgaactttggcttttaaaaatgacgagaacaaaaatcaggctagtagccttaatctttattccgatttctagaatgtatctctgaatttcttgtcttatctgttctattagaataatttctctgatttgatttcagattgttgaatgcaatgcactccctactcttattctaatgctgcgatccgaagatactgcaatacactatgaagcggttaggcatcattctgcaagttcatattactagctctttttttttttatatatatatatttaattatgtataaagtcacagccatgcttcaagtggtagacatagtgaaattgtgggatgtcaggttggagtcattggaaatttggtgcactcatcaccaaatatcaaaaaggacgttcttcttgctggagctttacaacccgttattgggttacttaggtagtgttggatcttataatttttgagtggctggtcatgtaaaacttctgttccgtagatgcttatcatttgcagattccatctaatggatgtagacatgctactatttggtttgttcttttcctcttgattgcttctgaaataagccctttttgtatgatagttcctcctgtccggaaagccaaagggaagcagctttattacttggacaatttgcagcaaccgactccgactgcaaggttgatgatgctactgtactctattaatggcctaagagtagtatatttatcgatttattggcatttaaagcaacataatctgatttctggttgaaatttttttctgatggttttgcagattcacattgtgcaaagaggtgccgtaccgccactgattgagatgcttcaatctctggatgctcaacttagggaaatgtcagcctttgcccttggaaggttggcacaggtgacttgaaatccttacagattttctttagggtactttgttttcttgtggttatcaagtaattcttttgttctgttagtagttattccctgggccactatttctctgagtattctgtaagtttaccattaagatttattttctggcattacttgtgtcgatagttgatgatcatggacatatctttcgcgattattgaggttgttttcaagtatgatatgtgctcgtgacatctttgtcatgactcatggtcttatccccctttccaatcaaaccttatactaaagaatataattgtattattggttccaatcagaccatgtttttctaattattctgcgagcttagaattcaagaatttactttcttatttacttgcatgtcggatgattaattggcatggcttgtctcttgatggagtgaaatgattacataagattcatatgggttactcctttaggattgaggttttgttgattgattgaagtttgacttgtatacttggattatagatcttggatgggaacttgattacttgtttttagtttgttttcatgtattaaagatgctggattatcttatatattgacttgcccaccttttaaaaataacttgttacgtaggaataacataaatgataaaacaaggaatcatgcttgtgagtagtggttcctttgcaccattgtgcagtttcatgagtggtttcaatttaaaactgacttgtttttcctttcacggtatacatgtatggacaattaaatgttaaatacactatcttatttttactcatcaaataacaataaatgctgtcttgctgttcaattgctcctcatttcatgtcttgaaatattatatgcacacggatagggctccctaaagtagtttaaattgttgatgtttggcatttacaccttttctattgggcagtaacattttatcataattttcttaagggataatgcttgcgttttgattatatcataatagtgtgtgaagggtcaaagctcggagctctttttccgtggaaagtgccagggcatagggttgttcttttctttctttctcaggcaattagctaaacttcagtccaaaactatttaagctttgctatatgaattttttctatactagctcattacatttcaatactcaataatctacatgttaaatatataattaaataaatagaagtggggtctctcaagcaacttaagcttttggttgaaatagaaatacacttcatgatatcagggcagaaccttgggtttgagtctcatcgccacccattttttaaaaaaaagtatattcacctgcttgactcatgacaaaagaatcattcttgcatgtaaagtggcatgctggtgacataattaattgcatagagatgtgctctatctaatagttttggagttcatatgatttgagaattctctacatacattctagttgattggatttactggttccctgatgttcaggacactcacaatcaggctggtattgctcattgtggtggaatagtcccattattgaagcttctagaatcaaaaaatggatcgttgcaacataatgctgcatttgctctttatgggcttgctgataacgaggtgttacaacatatccaaacaataatgttattataaccagatttttgtactacgacgtgttacatctcatctgacgcaggtgcaactttctgctataggataatgttacagatcttgtaaaggttggaggtgttcaaaagcttcaggatggagaatttattgtccaagtattattctttttttcttcccgtgattgttattttgtgccaaatattacttaaaggaaaaatgatttcatacagtatgatgcttttctcattattcttagttctttgtcatggcccttgatattgttcactcattttttagccaactagagattgtgttgcgaagacattgaaaagattggaagagaagattcatggacgggtgagtttctatttgttgcaaggaatttgttgatgcatactttatttgtttgcagtgaagcacatgatgcaattttgtgtatgaagaactcagtgagtacatttcttttgttaacgaatgccaagttattttatttcttagctacgaaatgtggtgtatcccccattgtccagttcattcttgtcccttcaataaggtaaatttctttgttaagtcttataggttactgatagttatatctcaaaccagtttgccctcttttgaaggtattaggccatttattgtatttgatgcatgttggggaaaaggttattcaaagacgagttgctcttgtgcttgcccatctttgttcaccagatgaccaaaagatgatatttattgataatggtggtatgtgatctgtacctatactcagaatgaattttcctcggtgtgttggttaggctgtgacagttaatccactatgtggactatgttcttgtaggattggaattgcttttagagcttctagaatcaacaaacttgaagcaccaaagagatggttctgtagctttatgcaagttggctaacaaagccagctcactttcacccgttgatgcagcccctccatctcctacacctcaggtttgctccgcagtttaatgctcatactctggcaaagtttttgttcaggtttttggttcttaagttctaacatgagtaatactagtctcttggtcatttatgggtctttatttagttttgcactgttacatggtgcttctcataccaagttaacactaagctgtgtttgtattctcatcgagtatttcgaagatgcacgctgaaccgtctgatgttcaaatttaatcattgattgtgataatttgtgaagcttttaccatttactttatgaacacttgtcaaaccaagttgtgctagtgttacctcaagacttgaaagttataatgtagctgtcctgcaaatttaatacaatgtcaactttaccaaccatttgaattactgcataaaaactctgggcgtacagtttcttaccatattgtagttcagtttgcttctcacattgtgacccttgtgttatatgctgctgtttataccaagtttattatgaaaaagcatctttttagagtatgatatgccttttatttgttcttggcatctgttatgctgatgaggggtagaagaccttagaaccctctcttgatatgctaaatttgcttcactgagcattatttttttggttctgggagggtgtgtataccaagactggtattcctgtcaatctcttaatctagcctataacattgtcaattgttctatggtcttagtaatacaaaacagttgagttctgaaaacttcacttgctgacccttaatcgctggcatgcttggtgtattctgagaatcaattaggcaatatgagggcttttcttatccctacattttgaggatttagattttgtgagtaactcgtcttcactttggtgatcgtttgaggagggtttacatgttgacagattccataggctgttttcaccacagtttacttgatgttcactttcttcaccaattaacaatgttgtctgagcttttcatgtttgttagtttgtatgtctgctttctgtcttttctttctcaattgacttgtaggtggttcataaccattcatggtgcagtaattagacaatgtatttgatcctatattacatctcttttcgttattttctccttgtgcatttctttatgcaggtctatctgggtgagctgtatgtaaataattctacgctatctgatgtgacatttttagtcgaaggtagcagcagttttgtgattcaaatcttgtcatctttttcatatcatggtgtatcttaatgattttttggtccttcaccaggcaaacggttttatgcccacagaatttgtttacttgcttcttctgatgcatttcgcgcaatgtttgatggtggctacagggtaagtagaatagttggcataaagatttattgcttttacttttaggttattggtttctaaattgatcattagcaacacaagatgaaagctggttttgctcccaaattttgtcttctactgcttacctttccctttagacaaatttagattgactatcaaatgatttttgcaaaattgctaaaaggcaaacatctttatttgaaatgttacaagcatatgtgtcatgacaaatatggcgtacaaaactctgattacctttccctttagacaaatttatattgactatcaaatgatttttgcaaaattgcttaaaggcaaatatctttatttgaaatgttacaagcatatttgtcatgtgacatgactgaatgcacaaatgtggagtacaaaactctgatgatctgttatatatttattgcaggagagagatgccaaagatatagagattcccaacattccatgggatgtttttgagttgatgatgaggtgcgctgctgtttaatctctgtcacatctgggatacaaatcaatctagtaatattgaagacaggaacgtttattgtttgcaggtacatatacacgggatctgttgatgttaatatgggtgttgcaaaggatcttctaagggttgctgatcaatatcttcttgagggccttaagcgtctgtgcgagtatgcaattgcccaggtgagtgctggggacctttctgtcttagaggaggatttatgtctggtttctcctaatagtttcttatctttggtaggatatctcagtggaaaatgtctctctgatgtttgagttatcagaggctttcaatgcattgtcattaagaaatgcttgcattgtattcacattggagaagttcgacaaattaagtgtcatgccatggtgtgtccagattcctatccttttgcttcatcatttcttggaataaaaaagacacgcttaacaaacatgaattgtgtattaacacactgtaatcttgttacatgtaggtattcgcaattgattcaacttatattacctgagacacgtgcgtactttgctagggtgctgagcaggccaattcaagctgacctctgatttaggttcatttttattctttgattagatgtagtatatgatgtaaattgtacaggaagtgggttttattccactcgtctctaattgcaagagttatgtgtcatttctcatcgcttgcaattccatatttgttgtgacgtttaatgtagcgtatgaagttcagttgcaacgcctgccatgcttctaaaactctttcacc

SEQ ID NO: 140 - protein, 708 aa, Solanum lycopersicum
MENQKLTERSSSSARRSLKRKLEEDLQDDRKVSPSISSEDGHQDLEREVRTQVEILESSFSSSESDRASSKRAIHVLSEFAKNEEIVNVIVDCGAVPALVQHLQAPPLVSEGEGSHIPYEHEVEKGSAFTLGLLAIKPEHQQLIVDAGALPHLVNLLKRHRDAQNSRAVNGVIRRAADAVTNLAHENSSIKTRVRVEGGIPPLVELLEFVDSKVQRAAAGSLRTLAFKNDENKNQIVECSALPTLILMLRSEDTAIHYEAVGVIGNLVHSSPNIKKEVLLAGALQPVIGLLSSSCSESQREAALLLGQFAATDSDCKIHIVQRGAVPPLIEMLQSPDAQLREMSAFALGRLAQDTHNQAGIAHCGGIIPLLKLLDSKNGSLQHNAAFALYGLADNEDNVADLIKVGGVQKLQDGEFIVQPTRDCVAKTLKRLEEKIHGRILGHLLYLMRIGEKVIQRRVALALAHLCAPDDQKIIFIDNSGLELLLELFDSTNLKHKRDGSAALCKLANKASSLSQVDAAPPSPVPQVYLGEQYVNNSTLSDVTFLVEGKRFYAHRICLLASSDAFRAMFDGGYRERDAKDIEIPNIRWDVFELMMRYIYTGSVDVNLDVAQDLLRAADQYLLEGLKRLCEYAIAQDISVESVSLMFELSEAFNALTLRNACILFILEKFDQLSVMPWYSHLIQRVLPETRSYFERVLTRAIQNDMRV

SEQ ID NO: 141 - protein, 734 aa, Solanum lycopersicum
MENQAKRSKQSSSSGRRSLKRKLEGDFEDDRKVSSHDDDAHQDLASEVRTQVEILDSTFSSTEADRASAKTAIHVLCELAKNEEIVNVVVDCGAVPALVKHLQVPSLGNQGDGGQMPYEHEVEKGSAFTLGLLAIKPEHQQLIVDAGALPHLVDLLKRHKTLQNSRAVNGVIRRAADAITNLAHENSSIKTRVRIVGGIPPLVELLEFVDAKIVECNALPTLILMLRSEDTAIHYEAVGVIGNLVHSSPNIKKDVLLAGALQPVIGLLRHATIWFVLFLLIASEISPFCMIVPPVRKAKGKQLYYLDNLQQPTPTARLMMLLYSINGLRVIHIVQRGAVPPLIEMLQSLDAQLREMSAFALGRLAQDTHNQAGIAHCGGIVPLLKLLESKNGSLQHNAAFALYGLADNEDNVTDLVKVGGVQKLQDGEFIVQPTRDCVAKTLKRLEEKIHGRVSFYLLQGIFCPLLKVLGHLLYLMHVGEKVIQRRVALVLAHLCSPDDQKMIFIDNGGLELLLELLESTNLKHQRDGSVALCKLANKASSLSPVDAAPPSPTPQVYLGELYVNNSTLSDVTFLVEGKRFYAHRICLLASSDAFRAMFDGGYRERDAKDIEIPNIPWDVFELMMRYIYTGSVDVNMGVAKDLLRVADQYLLEGLKRLCEYAIAQDISVENVSLMFELSEAFNALSLRNACIVFTLEKFDKLSVMPWYSQLIQLILPETRAYFARVLSRPIQADL

SEQ ID NO: 142 - protein, 719 aa, Solanum lycopersicum
MENQAKRSKQSSSSGRRSLKRKLEGDFEDDRKVSSHDDDAHQDLASEVRTQVEILDSTFSSTEADRASAKTAIHVLCELAKNEEIVNVVVDCGAVPALVKHLQVPSLGNQGDGGQMPYEHEVEKGSAFTLGLLAIKPEHQQLIVDAGALPHLVDLLKRHKTLQNSRAVNGVIRRAADAITNLAHENSSIKTRVRIVGGIPPLVELLEFVDAKIVECNALPTLILMLRSEDTAIHYEAVGVIGNLVHSSPNIKKDVLLAGALQPVIGLLRHATIWFVLFLLIASEISPFCMIVPPVRKAKGKQLYYLDNLQQPTPTARLMMLLYSINGLRVIHIVQRGAVPPLIEMLQSLDAQLREMSAFALGRLAQDTHNQAGIAHCGGIVPLLKLLESKNGSLQHNAAFALYGLADNEDNVTDLVKVGGVQKLQDGEFIVQPTRDCVAKTLKRLEEKIHGRVLGHLLYLMHVGEKVIQRRVALVLAHLCSPDDQKMIFIDNGGLELLLELLESTNLKHQRDGSVALCKLANKASSLSPVDAAPPSPTPQVYLGELYVNNSTLSDVTFLVEGKRFYAHRICLLASSDAFRAMFDGGYRERDAKDIEIPNIPWDVFELMMRYIYTGSVDVNMGVAKDLLRVADQYLLEGLKRLCEYAIAQDISVENVSLMFELSEAFNALSLRNACIVFTLEKFDKLSVMPWYSQLIQLILPETRAYFARVLSRPIQADL

SEQ ID NO: 143 - DNA, 9386 bp, Manihot esculenta
  source 1..9386: mol_type = genomic DNA
ggcgggattgcgagttctgacgttctagccaatggaaagcaggtgcattggttcagttttcaaccttccagaaccggaaaataacgtggcccgtttaaatccgacacattcaatttccccaccggtaaagaaaacagaagaatagaaaaaggaacgagaggaaatcacaaaagttacacaaagcttgctaaaaaaattttccttataattcccaaaatgcccttgatctatggatctctcaatctattcgaattccttttcctttctgtttagcctctatttctgtcggtccatctcattctccgtgcgttactgttcttgatggagcctcagaggagccaacaagatcagggtctcccggagaggaagggacagaagcgcaaattggaggaagaaatcgaagaggagcaacgagagatctcgccggcggccacctttggcgatgcgcgccaagctcttttacatgaggttgctgcgcaggtaaatatccttaactcgaccttctcttggaacgaggccgatcgggcagctgtcaaacgagccactcacgtccttgcagagttcgctaaaaacggtaattcctccccctatcttgttcctctctttcatttttttagtccacggattctactttcggttctgaagtcaagatctctctttatgctaagtgttcttttgcatggttgcttgcaaattgaggaagtgttttgttcgttgatcgttgtttttcagaggaattggtgaacgtaattgttgaaggaggcgcagttccagctctagtaaagcatcttcaagcgccccagtcaggtgaagctgaccgtaattcaaagccgtttgagcacgaggtggagaaggggagtgctttcgcgctaggactgcttgctgtgaaggttactatttatatgttcttttcgtgcctacttttgtatttttacgcctagatactcgtttcatagcatcttagtttcgaggttcagtttctgtccagcgaagttcaagtattataggaagatgcttcctgttcaacagtgagtcagttatgctacggtgttatccatctgtaaattatagtccagttaaattttgcagaaaggaaattttcatatttgcatgaaatcgatgttttaggggtaactgtattttttagatgtgacaagaaatcttttatgcattgcagagaatggaacagttgttttattgtatgaagtatctggtttccagtaatctgcgatcatttctttgtttttaaatttgcaagaatatttcatgaataatacacacctaaaacagtgacactgctattccaaaaataaagctaagaaaggcaatcgaaggttgaatatcaaacataattttgttgagaaatactctaaacttgatctgatttaaaatctgcttttcccccatccctgaatattattattttttttccatcttgactttcaacagccggagcatcagcaactcatagttgacgcaggggcactgtcacttcttgtggacttattgaagaggcataaggatggttctatttctcgggcagtgaatagtgtaattagaagggcagctgatgctatcaccaatttagctcatgagaacagtagcattaagactcgtgttaggtttgctcattttagtggtaattttatttgaatttctgaatttggcactatgttcttcttattttcagtgtcattgggtatgcaggatggaaggtggaattcctcctctagttgagttgcttgaattcactgatacaaaggtgcaaagagcagctgctggggcactacgaaccctggcttttaagaatgatgagaataaaaagcaggtgataaatatggtcttggaggttgggcctataaggttggctttaatattagtaaaatgatagaaactctttgattttgcagattgttgaatgtaatgctcttcccaccctcattctaatgctacgatctgaggatgctgctatacactatgaagcagtatgccatgcaacattagttttaaattttgtattgatgtcgacttctatttttgcacttgacattaccatcgtcatgaaaaaattttgattctcacaggttggtgtgattggaaatctggtgcattcatccccaaacataaaaaaagaagtccttgctgctggtgctttgcaacctgttattggcttacttaggtttgtctaaatcttgtgttctaggcacccttgagctacctctctacttgttttggcagcatgcgaagattgtcattctttgaaattcattgatattttgtttttctaaactacttatcttcctttgcttgagtgaagattttctaagaaaaattaattctctgtaatttatcatgatttcttggaaatagctcctgctgttctgagagccagagagaggctgctttattactcggacaatttgctgcaacagattcggattgcaaggtatgctcgaccttttaagctaattcatgagaagattggaaaggcagaaaagcattttctagtttcaaagtttttgtttccagctgtccatttagaatataaacaagaaagtcaagttttttactttgatggatgacttgagactcaatccttcctccaaaaaaaaagggaaagcattttgttaaaaatgtgaattctttttaggttcacattgttcaaaggggtgcagttcaacctttgatagagatgcttcagtcccctgatttgcagctgagggaaatgtcagcatttgcactggggaggttggcacaggttaccatttctttctttctggttcatacttaatttacattaaatttagatttcctaatgacattgtgaaatgggtgttgccttcataccagtgaatagttagttattagctctaaggtttttagtggttagaaaagataatacattttgaaaaggaaaaattttaataaatataaaattttgtattttaagcattagataggaattcaaatgtatttttaacaatttagcttcaatgtagcgtttacacatgcatttcagcacttcctcactaacttgaccaattgaattgaattctgattagatggttcttttggcttttgattttattttttttatcgcaggattcgcataatcaagctggtatagctcataatggtggtttggtgccattactgaagcttttggattcaaaaaatggatctcttcaacataatgctgcatttgcgctatatggtcttgcagataacgaggtgtgctgtaggttatgaattcttatgaactttaggaccaaaatcccagaataattttgcaagtgagcctgtctaacttcatacgatcttatgttctctcatttttttcatataggataacatgtccgattttattagggtgggaggtgtccagaagctgcaggatggagagtttattgttcaagtatgttcattaatcatttcattggttagcagagctgttattattagtctcttttatatgcctatgctgctgattgtatatttgctttcactacatggtagcttgaaatcacaaattcatgtaggaaccgaaatgtttaccagttcattgctcttcttgctgacctaccgtgattaatatgcaattaacaatcacgcctgcaggcaacaaaagattgtgtctcaaagactttgaagagattagaggaaaagattcatggacgagtaacccctcactctctcattttattatctcttgcaatatctagtttacggaaagcataattttttttttcttttttccccctttgaatttaatatccaaccctttaaatttgtaacttatatatttattcttgtaggttttaaaccatttattatatctaatgcgtgtagcagagaaggctgtccaacgacgtgttgctttagctcttgcgcatctttgttccccagatgatcagagaacgatattcattgataacaatggcatgtcacattctttgtaatgatgccagttttaactttacaaccgagaaaaaacaattattagtttggaaaagtgtttgttgacttcagatgatcatgccggtatgagaatgctgataatttatctaatgcaggattggagttacttctcgggcttcttggctctacaaacctgaagcaacagattgatggagctgtagctctctacaagttggcaaataaagctatggctctctctcctgtggatgcagctcccccttctccaacaccacaggtggtttgctgtctaaaaccacttggacttaatctattcagttgcttatgacgtgacatcctaaacttgagctgaatgtatttgaggttgttggccgatataatggaagaacacaaatatttattataaaaggtttttggtttaacaatttattattttgttatcacttgaacttgtttcctgttcttgtgtcttgagtgtagattttgatggatgaaaatatcaaagaaacaaaatggttgtggggttggtgtgtaacaatttgttatttatcatttttacttgtcctttgctttaactttcaaaatatgaaaggatgtaattttaaaattttaatttgcatctggaatttcatgcctatgataatctgtctttttctgcaggtatatttaggggagcagtatgtaaacaatgctacattatctgatgtaacctttttggtcgaaggttgtaaataaaaagttttagatggttaccttctgtggaattcttattttgcagatcctgctagtattttggattttttgtcatgaattcttacaaaagcacattatttgtgtgctgtaggtagaaggttctatgcccatagaatttgcctacttgcttcttcagatgcatttcgtgcgatgtttgatggaggttaccgggtaagtttgtgcttcagtcatggtttagtttacattcatcaaacatcttcccttgggcctttatttaagagttcaggcccaaagagtgaaacagaaggttgcttttttttttgtctgccaaagtactctgcaaagtgaattcattcgactggataatatattgaatttggttcagataattacagagatcattattcatcttgttattgtaaacccagagtggtcttcttgatggatttgtagtttaagcaagacttatgcacaagtagggggtgaggagaaagattgttgggatgacatcatatgtgacacttacattttattaattgttcttggcatttgtcacaggagaaggatgcaagggacattgaaattccaaacattagatgggaggtttttgagttgatgatgaggtttgataaattgcatagtccttagtttcttgaagaagtctctccaaattgattatttagtgggttttgttttctacagattcatatacacaggatcaatagatatttcattagatattgcacaagatctcctgagggccgctgatcaatatcttttggagggccttaagcgactctgtgaatataccatagcacaggtgagctataaaggcttatttaagtatgtacttgaaaatgcataactggctattgttaaatatggttactgttttttgtccaactctctcaggatatatcactggaaaatgttgcaagcatgtatgaactttcagaatctttccatgctatttcactgaggcacacatgcattttgtttatcttggagcagtttgataaattgaatgctaagcccaggtacatgcccctctcaatctgccattttcctgttcccttagaacctttggatgtgaataaatatttcaaaaattcaggtagtaccttaagtgtaaacagttctctaatatacttgcacatatttatgtgtagaaaatggcaaattttaggataatcaatcaatcatttcacattgtaattgctaaatgcttcttgcttccctacgtgatatgtatgtttggaaaatgttagtttttccttcggtggaatgagaaatatataatttgttttcttggtggaaatttatattgcatgctggaattgcaggcattcccatttgatccagcgtattgtacctgagattcggaattactttgccaaagcacttaccaaagctaacccacataatttgcggctgtagattgctggtctttgattctcgatgtctaactagataacattgtacagagagtggtagatgttctaattgatgtcgagccatttgaaagtcctaataggttggttaatatggctccataatcttccctggtaccagattgctactaaatgtgtatgcaactgtaacattgtttccattttcttggatgttgatgggctatgttcttcaccaacattattgttgttgcatgtactgatgcattttgtaactctttaatgagttgacgtttggtgagagagcaagagttgattccctgaaaatttggggcagagcttcaggtttgtaatgctccctctcaaggacttcggtggcttaatatgttatagcgctttagacattgctctttatgtgaagagactaggaagttgcaataaaaatatatatgtgtatatcattgatcctttttcaaattgtaaattttctgcaggcgctgttgcatgatctttttcatttacgaacatggaaattgttaatcagactgtcattgtgtattgattaccacttgtgtaggtcgggtcaaaagggacagcaattaattgtttgttttcacattttctgttgatgctattttgacacaaacgtgacctggccgctggtctaagccagtttgccttaatcacccgttctggtttaattgggttaggtagaatcgggcagaaggttcatttggtcttattttttattcggtttgattcatccaatttaagtctgattttgatcaaatctagccacatatgttttttgaactttttttttttttgaaaaagggaaacgagattctttggtctgaatcagattggtttataacgttcttcattttcatttcacttgtgtttataagcctgatgggagaatcttccttttgttttgtcattttcatcaattatcccattaaaaaagatggaatttttagttgtagaacgaatttcgtgttgtctcccgttgtcctttttcgattctaatgtttaattttttggtttttgaatataaaatgcatattagcaatatgtctcatattttaatttcctttcataagatgttttattgaaatcaatctttatggagtattaaatgtgtattattaaattaaactattagttttttttttcttttttctgaaagaatataaatacgttgatatgcatatatcaatttaaagctgtatatttgtgaagttaaaaattgtcttggatatcataagaactggttcaatttaatagaacatttgaacattgatctgaagtttttatgataatgaggaatgccaagtagaatgtaagaagaaaaatagccaggtgttgtaagccttttatttggggctttttgcattttcatgttaaaaaaaaaaaaaatttctcaaatctcagtaagaacaaatttttttcccaaatcagggtgaaaattaacttagaatttaccgcacacttaaaatatagtaagaaaaaataaattttataaaaaattacattaccgcacttttgcagtgcggtaatgtaagaaaaattatttaaaaaaaaaattcattgaagtgcggtaatggatttgaagtttaaattttaatttttatttaattaattattatattatatttttattaatttaatttatttaattatatattaaatttatataaatataattataaaaattatattaatattaattattttaagttatttattattttaagttatttataatataatattatatttattttattaattatataatttaattaattatctattaaatttatataaatataattataaaaattatattaatattaattttaattattttaaattatttataatataatattatatttattttattaattatgatattatcagatttagagaagggtttcagtatgtatggataagcttgctagagagggaggcgcctatccctttattttttttccttttatcccctaatgacttgtagtgacctttttaatacagtaccacctgtcctattatactggtccatgcgtatggatgtttcagaggtcctcttcatgtcagacggccatttaatttttttcggtacacaagtgggcaggactgcgaagtgactgggcctgttatttttcctcttgtcatatcaccgaatcgagtaagagcttgttgggcttgggcttctggatgacccggcctatcattcatgttgaaatttagtctgaatctaccggacaggtctgctgagaggcgttctgaacttgaaatctgatatgctcttatgggccttaactcggcccaaagagtacgagactcgacggttatcaaattatataatttaattaattatatattaaatttatataaatatagttataaaattatattaatattattataaatattaattattttaatttatttataatataacattatattttttatatttatcattttattttattatttttatttttataaaatttctaaacaattataacgctaacaccacctacaaaaaaaaacttcagactttttactatttcaaaataaaaaaattattctaaaatctattattatttcaaaaattaaatatttataaattaattgtaataaaaataataattaattatattatattataaataaattaaaataattaatatttataataatattaatatagttttataattatattaattaatataaatttaatatataattaattaaattatataattaataaaataaatataatattatattataaataatttaaaataataaataatttaaaataattaatattaatataatttttataattatatttatataaatttaatatataattaaataaattaaattaataaaataaaatataataattaattaaataaaaattaaaatttaaacttcaactgcattacggcactgcggtaatgaatttttttttaaattaattttttttatattaccgcacaatgaaatgcgataatgtaattttttataaaagttattttttttactgcactctaagagtgcggtaggctctaccgcactctaagagtgcggtaggctctaccgcagtttaaaagtgcggtagagtcaactttcactttgattttagaaaaaaaaaatttcagaccaagatttgagaaatttttttttttaatttgaaaatacaaaaagcccttgtatttgagtacgaaatagttgcatctttgtgattacatgttacgagaacatttaggtgccggattttgaatcctagaagccaactta

SEQ ID NO: 144 - DNA, 6845 bp, Manihot esculenta
  source 1..6845: mol_type = genomic DNA
aatggcgcgcacttgcaatttaaaatttcataactgtccaaaggcgggaaggcaaccgcgcagcaataataaaattggaaacggaagtggcggtctttcttcccacacctaattcttcacccaacaataaaaagaaaaagaaaaatttacatttttttggtgaaattaattaacccacatcttatttcattcctccaatttcacggagaacaaaaggcacgccacggtctttcccaaattaccctctttcttcttcctcccatccatggatcaaccatcaatcgctgcaagaaagagcttgaagcggaagctagagcacgactcccttgaaggtagagatgatcgcaagttccgggctgccgaagccgaagctgaacctgatacaactggtcaagatctggctcttgaaatccaagcccatgtggatatccttaactcgaccttttcttctttagaagccgatcgcgccgctgccaagcgcgcttctcacttcctttctcagctcgccaagaacggtaaccttccctctttatctctttgtttatgtgatgttattcgtttctgaaatatcagcgcatgcttgcttgtgcgggttttggctgaaaaatgttttcagtgttagtcgacgttttccttttagctttgcctttcctggttgattagatagcagtttaattaatcattctatttatggccttttctttttaagcttagggtttataggtttccctaacttacgttttgcagaggaaatcgtgaatttgatcgtggattgtggcgctgtgccggcgctggtgatgcatcttatggcgccacctcctttgagaggtgaaagtactccaaaacagtacgaacatgaggtggagaaagaaagtgcattcgcacttggacttatcgctgtgaaggtaattggtcaagagactgactattcttttttaatttttcattgctcgttgcataacctgttcagttgacctaatatctttctgttatcgttgattttggtcctttaaagacttagaactatcatttacatgtctcttgtttgcttgtgggaaaaacataactaggagtgtgtagaatttagttcaatattctttaatcatttaaaggaccaaacataactatattgcagacacttcccttaagtgatgcgtagattaccttttctctaattacttcctaatcttgctctctctctctctctctctctctctctctctctcttctctactgtttaattaatagcctgagcatcaacaactcatagtagatgctggagctctgtcccatcttgtggaccttttgaggaggcataagagcagtagtaattctcgagcaatcaatggtgttatcagaagggcagctgatgcaatcactaaccttgctcatgagaataatgtcattaaaacatgtgtcaggttaatttacctttttataacaattatcaagtcttacattggttaattttttaatcccccttctaacaattgagatacatccaggattgaaggtggcatcccacctcttgttgaactgcttgagtttgttgatgtaaaggtgcagagagcagctgcaggggcactgcggacccttgcatttaaaaatgatgaaaacaaaaatcaggtatagtgttttcagtctctctctctctctcttaattatttatttgggaggggaggtgcttcttggggtttctatgagcagtatcagtgacgtgaaacacaaatttgcagattgtgcaatgcaatgctctacccactcttatactaatgcttcaatcagaggatcctactgtccactgtgaagcggttggttctaaactcaggttatccatagatcagggttttcttcttctagtttgttctgcattacacattggctgactttccaagagattgccaggttggtgttattggaaatctggttcactcatctcccaacataaagaaagaagttcttcttgctggagctttacaaccagtgattggattgcttaggtaaaagtgaattttcattctatccaatttttgcgctggagaatcatgcttttgttaacttttatctttaacccttttttatcatgctataattatccacctcaagttatttgcctctctttctcttataataaatattctactcacatacaagtttgacagctccagctgttcagaaagccaaagagaagcagcattgttactgggacaatttgctgccgctgattcagattgcaaggtacatttcatatcatttatggttttaaggcttgaatcatggaactcacttgttaatgctataggaatgcactaactggtgtgccaatcctagataggtgcaaatgcaaacatatattagtggcatgtttgtggctttattctgttttaattgttataagaatgatgttcaagcaggtgcatatagttcaaagaggagctgtccggccattaattgatatgctagagtctccagatgcacaaattaaagaaatgtcagcgtttgcactggggagattggcacaggttatttttttatcttttacctattgcatggccatgattcataaaatgtgcatgtgcaaacaaacacgtctgcagtttctactttcgtgaaagggagacagagcagtgatgggcattaaacactggctgacttttatatggtattggcatttttttgctgaaaaaattcttcagcatattataaacagattctgctgtatgtaatggtttttaccatttatgaaaggaaattgatgttaacatcttcttagatgttctcaatctttacacctttggaaaaggatttctgcatctttttctcccttgcaactattgttgcatctttctcatctttttttaaaaattttttttattctgttcttctttgaggggaaaaagtgcttgattgagggaaaaaaattccagatggtacattaaaagacaattttatttgtcattgtttttttacattttcaaatgttttgaatgattcatagcatgttatgtaagttatatttgcttcttgtttcttattttttttcttgtatgtatgtatatatatatatatatatatatatatatatatatatatatatatatatatatatatatattttaattttaggaaatgcataaccaagctggcattgcccatagtggtggcatagtgccattgcttaagcttcttgaatcaaagaatggatctttgcagcataatgctgcttttgccctatatggccttgcggataatgaggtatagttaagtttgttgcatcatttcctaatttcattgcattgcagcttgccagttactcttaaaactataattgctgtattgtttcaataggataatgttgcagagcttgtgaaggttggtggttttcagaaactccaagatggagaattcattgttcaagtatgtcttttgatgtgttttttttttataaagatttgagtggctacttcttggtgctttagctaatgctcatttatttgactgatagatttggaagatgttgctgtcttcctgtctgatattgctcattttattaatgttgcttagcccttattgttattatgtgatacttgcaggccacaaaggattgtgttgataaaacattgaaaagactagaggagaaagttcatgggcaagtgagtcgtctcactggcacctctgatcatctatgttttgtttagtgatttgtgtgttcttgctatgctgctggcttatatttatttattgaacccaaaacattggttttttgggcacaattgcatattgattcattttatgtttttcccatcaggtactgaaccacctcttatatttgatgcgggttgcagagaaatctgttcagggacaaattgctttagctcttgctcatctctgtgctcctgatgatcgcaaagctatttttcttgataacaatggtagaaattctggatctgctagtgatgctttcattcctttagatgatacattttaattctttagttgcttgcttttacatgtttgtgattttgctccagggttagagttgctgctggggcttcttgagtctggaaaccagatgcagcaacatgctggtgctgcagctttgtacaagctggccgccaaaaccacttcagtctcactgttggatgctgctcccctatcaccaacaccacaggtaaatttcttttatagtattattttttatatgtataatgttagttttcttttcttagaatgcttttaggcgtaggactgtattatatgcagtattattgaagttgcacttacttttccaatgggataatgttctgaatgagagttcattttttttacataattgtctgtgaggccattattagagttgttatttcaatctttatgtttggctcagttttcagccatcaattgatcttctggtgtttcagtgatttagtaagctcttatattgattgtaaagacagcaactggaaaattaatttcattatttgatattcgcactgcaggtatatttgggtgagcaatttgttaacaatcccacgctgtctgatgttacattcttggttgaaggtaataaataatctgtgttaacttaatgttctttatgccatgaaaaatttcaatacatgtgttgatgcagtacttactgactgcatggttgtgatattattttacaaggtaaacgattctatgctcatagaatttgcctccttgcttcttcggatgctttccgtgcaatgtttgatgggggttacagggtgagaatttatttcttctgaaaccttgcttttgttgtatgctttgtaatgaatttgcatgtttgttgttttgttagtgatctttactatcttgtccctaaaatatgcattggcagaattcaaaacactaatcagagttccttaactatcaagtttgataagttatttatcattaatgaactgcccatttataaggggatgcaactttaactgatctgagttttcctgctctgttatcatgtgtctattatgcaccggctaaaagaaatttgcaattttagaggtaaatagtttacaaatttctgttttatttcttattaaaacaaaaatgcaggagagggatgctaaagatgtagagatcccaaatattagatgggatgtttttgagttgatgatgaggtgagcattattgattttccttggtaggtacgcaaataaatcttccttctgctttctggtagcatgctgatttgagttgtttccttctaggttcatatacacaggatctgtggatgttgatattgaggttgcacaggatcttcttagagctgctgatcagtatcttctggaaggtcttaaacttctctgcgagtatactattgcacaggttagctaatttgtcttgatatttaccctttaattacgcaattaacattaaggttggtctgatgaattattgttgtctaatttcaaggatatttctgtggaaaatgtctcacttatgtacgagttatcagagggctttaatgctaggtcattgatggaagcttgcatactgtttatatttgagcaatttgacaaactcagttccaagccatggtatgtcatttccttccaatttgtctctatcctttccgtgttatgtcttgaaggataataactgatagttacagacatgcaaattagattggtaaaagatgttttgctattttcttataatttctgacatttcaggtaatgttttgatatttgaattttatattttatcacgctttttgcccttgtttgattctgtcatcagacgtaagcagttgaatgagttcagtgcctctaattctcaatatttgggcttgatgcatgtcctattcgggccacttctgcattatccactattcgtcgacttaaattggctgcgaaggttccgaatttaatgccttgtaatttgcaggtgttctcatttaatccaacacattttgcccgaggtacgagattactttactaaagcacttaccaagcccatccaagctaacttgaagcaagtgtagatgattcgtctagttctgatctttaactaaccacgctgaaagttgagggatgtacagaaattctggagttgagctaatgtggctaatcttcgtgtaagcatggtgtggaacccaagtaaatcaaatggcacaattttttaagcaaccattcattgaagcaatctttcgtatatggtgcttaggcaatgttaacccctggttttgtcattgctctgtgtaagtaactaatatacacgtagctaagttctggaaacaatgttgggctactttttttcttatggctaattggctaagttttgtttgatagggacacaatttaacctgtaattaatagtgagattttgtatttattctactgaattttacgtaatttctgaaaaatccatgaggttttatttgtatatgatcttcgtgctaggataaatgtctaagatatttgttttacaacagaaagaaaattcgtaatattgtcatatgggattcgactatgaaatggttatgaaagaaaaaagaatatgtagctgatcatcactctggaatatgcaacaaaaaggactgaaataaaccaaatccatctcaaaagcccacggtagccaatcacaatcagaccaagccagtaatgaagaggtgagagaatagcaatcaattttgtaaccataatgaaaatcacaaagctggagagtaggatatatggtcctgatgaggaaattgcagggcctaacacagaaaaatgggacaacataacaatgtttgaaaatgcaagcaagcgaggaagcttgccatcttttctaatgttcaaactgaagtgatcgacatataattgcatctc

SEQ ID NO: 145 - DNA, 7296 bp, Manihot esculenta
  source 1..7296: mol_type = genomic DNA
ttgcatccactcaccttagagtgcgcgtgttagcatatcgcatagttgtccacattttttccggcgggaatgtaagttagacgtttcccccaaatgaaaagcaggtgaggcgtgtaggtgtagcttcagttttcacccttccagttctaaaaccagaaaatccgatacattcaattttcccaccggagaagaaaacaaaagaaaatcgagaaagttactcttcagcttgcctttttttttcccccacctaaattcccataatgcccccggtctctcaatctttcaatctattcgacaaaattcccgtttctgtttagcctctttctgtcggtctatctcaatctccgcgcgttccagctgttgatggagccgcagaggagccaagatcagagtctctccgagaggaagggacagaagcggaaactggaggaagagatagaagagaagcagcgagagatctcagctgcggtccccttcggcgatgcgcgtgaagcacttttatacgaggtgactgcgcaggtaaatatccttaactcgaccttctcttggaacgaggccgatcgggcagctgccaagcgcgccactcacgtccttgcagagttcgccaaaaacggtaattcctccacctctctcgtcctatatatttcatttcttgaaccgacagactgtacttttctgaaatcaagatctctctttatgttttagtgttcttttgcatgtgttgcttatagattgaaaagtgttgtttttggtggtcattgttttccagaggaattagtgaacgtaattgttgaaggaggtgcagttccagctcttatcaagcatcttcaagcgccttacacgaatgaagctgaccgtaatccgaaaccgtttgagcacgaggtggaaaaggggagtgctttcgctctaggactgcttgccgtcaaggtcactacttctatgttcttttcctgcctatttttatatttaagatttacatgttttagtagcatctttagttttgaggtttcagttcctgtccagcgaagttcaatcatgcttggaagttacctccatttcaacagttatgctatggtcttagttatatatataaatttaaatagagaattttctacatagagaatttcatgcggacttgatatattgtggatagtctttgtaattttttagatgcggctacaaatctgatatgccttctattgaataaaacagtcagtatccttcccattgttccgttgcatgaaagttctagttgcctgtggtatgcgttcatctcttgtttttaacatttgcaagaatattatatgaataatatgcacctataagcacaaccatgacaatgtgatctgaaaaatgaagctaagacatgcaaacaacggtggcatatcaagcatatatattttttaagaaatgctctggacgtgatctaattaaaattttatttttcctccatactaaacgctaattctgcttttacatctttcctgtcaacagccagagcatcagcaactcatagttgatgctggcgctctgtcacttcttgtggacctgttgaagaggcacaaggatggttctagttctcgggcagtaaatagtgtaattagaagggcagctgatgctatcaccaatctagctcatgagaacagcagcattaagacacgtgttaggtttgctcattctggtggtaattttgtttcgatttctgattgaacactgttctcttcttatcttcattataattggtcttacagggtggaaggtgggattcctcctctggttgagttgcttgaattcactgacacaaaggtgcaaagggctgctgctggggcactacgcactctggctttcaagaatgatgagaataaaaagcaggtgataaaccttgatttggaagttggacttataaggttgagtctagtatcagtaaacaagactttgattctgcagattgttgaatgtaatgctcttcccaccctcattctaatgctacggtccgaggatgctgctatacactatgaagctgtatgtcatgtgatgtgaattttgaatttttcatttatgtggaattttattgtcatgaaaaaaacaatctcattcgaaaacgtcaatttcttcaggttggtgtgataggaaatctggtgcattcatccccaagtataaagaaagaagtacttgctgctggtgctctgcaacctgttattggcttacttaggtttgtcaaatcctgttttttttttttttggcacccttgaaatgcctttccatttgttttgaccgcgcgtggacattgttcattctttaaattttttgtgcatatttatgttttaatgccagttatattattttcctcatttgaagattttttttaaaaaaaacttattttgcaatttatcatttatttcacggaagcagttcctgctgctctgagagccagagggaggctgctttgttacttggacaatttgctgcaacagactccgattgcaaggtagagttaaacttgccttgttttcctttccttgagggaattatgcactttctacagctattgttgacaaaaaagaatgaagaaataaatactatccattatttctagtttctaagtatttgtttccagcagtttatgttataaacaaaagagtttacttttttatatcgatggatggattgataactcaatcacccttgccctgccagaaaaaaaaaaaaaaagaagaagaagaaaacatacacaccaccaccaacaacaaccaccttttctgctttagattaaaagcatgatgttttttaggttcacattgtacaaaggggtgcagttcaacctttgatagagatgcttcagtctccagatgtacagctgagagaaatgtcagcctttgcactggggaggttggcacaggttatattctctctctgatgcattcttcattttcatcaaaggttagagatcctaatgagattatgaaacagctacagccttcttgcctgtggatatttatttatttagctgaataaatgatatggaaatgacacagaggaggaaagtagtatggatattttttttgcaagttttgaatattgatattcaattggtcgcaaataaagctgaacgatcaatttagctgaccccaacttgcttgggattaagtcttaattgttgctattgttgattataaaagatattaatttttgaaaaggaaaaatttgagaaaatgtattttgtatatttgctttgcatagatgtaaaagcatgtttctttgccattttagcttacccatgtaggctttacacataaattgtgcatttctgtacttcctcactacattggccaattcagctgaattctggttggatggttctttttagcttgaagttttcttttttgcttgcaggactcgcataatcaagctggtatagctcataatggtggtttagtgccactactgaagcttctggattcaaaaaatggatctcttcaacataatgctgcatttgccctatatggtcttgccgacaatgaggtaagctataggttatgagttccgatgaatgcaaggaccctaatcccagaatatatttgagagttagccttttaacttgatacagtcttattgttcattcatttttcctataggataatgtgtccgattttattagggtgggaggtgtccagaagctgcaggatggggaatttattgttcaagtatgttcattaattatttcatcgtttataatctcaacagtttaatatagctgttatgattagtctcctttatgtgcctaatccatgttgctgattctattttgctttaactacatggtagcttgaaagcatgaattcatgcaggaacctagatgtttaccagttcatgctctttttctggaccttccacgaacaattaacgattaataatcacacttgcaggcaacaaaagattgtgtatcaaagactttgaaaagattagaggagaagattcacggacgagtgagttttctctctttatccttttattggctctcgcaatatctagtcctctctctctctcctcttttattatctctaactatattttgtctgttgaaactgtcatggtgtttttccttttaccaaatcagggttaaccctatatttgtgttctatacatttcttctgtaggttctaaaccatttgttatatctaatgcgtgtagcagagaaagctgtccaacgacgtgttgctttagctcttgcacatctttgttccccagatgatcagagaaccatattcattgataacaatggcatgccatattcttcctagttctccctgttttcaaatttaaaatagaaaaatgaaatcattggattggaatagtgtttatcaacttaagatgatcatgctggtgagcgattgctgatctttctaatgcaggattggagttgctgcttggtctcctaggctctacaagcccaaagcaacaaattgatggcgctgtcgctctctacaggttggcaaataaagcaatgtctctctcccctgtggatgcagccccaccttctccaacaccacaggcgagtttgctatccaacaccactaggtttattttattcagtttttttatgatgtgacatcataaattcaagttgaatgttaatatataaatccacatatttgaagaaagcagatatttattgtaataaggtccttggtttaccaatttattatttgtgatcataattatcccttgaactttgttccatccttaggtttttaggcaaggatataggtggacgaaatttcaaaaaataaaaacagttggagatttggtataacaatttattagtattatttgcttgttctgtgttgacttctaaatgtgacaaggatgcatactttttttcctttttgttatgttattttgaaagtcatgcatatgataacatctttcttcatgcaggtatatttgggggagcagtatgtaaacaattctactttgtctgatgttacctttctggtcgaaggttgtaaatgaaaattatttgatagttaccttctgtgaatttttgtcttgtagcctgctagtatattagatttgttagcatgaactctctcttacgaaatcatattatttgtgctctgcaggtagacggttctgtgcccatagaatttgcctgcttgcttcttcagatgcatttcgtgcaatgtttgatggaggctacctggtgagtaagcttgtcagaatgtcagtcgtgatttcatcaaacattccccttgggcccttttttagggtcaaggcccagaaagggggcaacagatggttgcttttttattttcttgcaactctggagtctgaattgaatccagtgggataatatactgactgacctttgtttcagataattacagaggttactatgcatttagttgttgccaaccccagagttggtcttctttatgactttgttgtttaagcagtacttgaaggaggaggaagatggttgggatgacattcatatcatatgtgctatatgcattttttttgtctgaaaaaatttttcttggcatgtgtcacaggagaaggatgcaagggatattgacattccaaacattagatgggaggtttttgagttgatgatgaggtttgatgaattgcaaatttcatggtttcttaaacaagtctcttcagattgtttatttaataggttttattttcaacagattcatttacacaggatcaatagatatttcattagatattgcacaagatctgctaagggctgcagatcagtatcttttggaggggcttaagagactctgtgaatatacaatagcacaggtgagctttgaaggcttgtccacgtgtgaatgtgatctgcttccgaacttaaaatgaaaatctaatgactgtttctctctctctctcaggatatatcactggaaaatgttgcgagcatgtatgaactttcagaagcttttcatgctatttcgttgaggcacacatgcattttgtttatcttggagcattttgataaattgaatgctaagcccaggtaacatgtccctcttaatccattattttcctgttctctttaatactccttcctgtccgtgagttggtactactaatgttaaggccaagtggtaccttaagtgctagcaatcccctaatacatacatgaaaaatgacaaaatttaggatcaaccattccttctacgtcactagttatacggttttaacatcctttgtgagatttctgagtgagaaacagtgcaatagttctgtaagatcctaaagaaatctcactccctttgtagaatgagaaattatggtggtggaaatttattttgtgtgctgaaatttgcaggcactcccatttgatccagcgtattatacctgagattcggaattactttgccaaagcacttaccaaaattaacccacgtaacttgcggttgtagattgctggtatttgattcttgatctctaactagataacattgtacagattggtagatctcatcgatgtcaagccatttgaaggttcttataggatggttaatatggctcataatcttccccaataccagagtgctgttccacgtgtatacattgtaacattgtttccattttcttgaatgttgatcggcatgttcttcaccgacattattgttgccatgtattgttatgtattctgtgtaagagttgatttctctggggcagaatttcaggtccaaaatctaaacctcattaacggctcgtgtggtttaatatgtttagtgctagctttgtgtgaagatagccacacccaaaaagaaaagaaaaaaccttactttttaaataatactatttttgaaggtgacgttccctagcattcccattcccaaattggattgaacatttttcattacagaagcaaaattttttggtgttttagatctgtttgatactgaatttcaattgaaaaaagaagttttagaactataatcttatatgttcgttgaaagaaaattaaaaaattaagaagttgttttattattttaacattcttataatcagaatacgttcatatatggtaaattaattttaaatactttatatatttttttgaaaaatataactaatatcaactgtgatgggagcgtcccgcggaattttcgtctagtggtttctagatcggttccaaataaaaacaaatttgccagttttccttcttcataggttattattttattttattttattttatttttgtcctgaacggcgaacaaggcatgggggacaatctacgccagtttttcaactcagagagaatgg

SEQ ID NO: 146 - protein, 708 aa, Manihot esculenta
MEPQRSQQDQGLPERKGQKRKLEEEIEEEQREISPAATFGDARQALLHEVAAQVNILNSTFSWNEADRAAVKRATHVLAEFAKNEELVNVIVEGGAVPALVKHLQAPQSGEADRNSKPFEHEVEKGSAFALGLLAVKPEHQQLIVDAGALSLLVDLLKRHKDGSISRAVNSVIRRAADAITNLAHENSSIKTRVRMEGGIPPLVELLEFTDTKVQRAAAGALRTLAFKNDENKKQIVECNALPTLILMLRSEDAAIHYEAVGVIGNLVHSSPNIKKEVLAAGALQPVIGLLSSCCSESQREAALLLGQFAATDSDCKVHIVQRGAVQPLIEMLQSPDLQLREMSAFALGRLAQDSHNQAGIAHNGGLVPLLKLLDSKNGSLQHNAAFALYGLADNEDNMSDFIRVGGVQKLQDGEFIVQATKDCVSKTLKRLEEKIHGRVLNHLLYLMRVAEKAVQRRVALALAHLCSPDDQRTIFIDNNGLELLLGLLGSTNLKQQIDGAVALYKLANKAMALSPVDAAPPSPTPQVYLGEQYVNNATLSDVTFLVEGRRFYAHRICLLASSDAFRAMFDGGYREKDARDIEIPNIRWEVFELMMRFIYTGSIDISLDIAQDLLRAADQYLLEGLKRLCEYTIAQDISLENVASMYELSESFHAISLRHTCILFILEQFDKLNAKPRHSHLIQRIVPEIRNYFAKALTKANPHNLRL

SEQ ID NO: 147 - protein, 692 aa, Manihot esculenta
MDQPSIAARKSLKRKLEHDSLEGRDDRKFRAAEAEAEPDTTGQDLALEIQAHVDILNSTFSSLEADRAAAKRASHFLSQLAKNEEIVNLIVDCGAVPALVMHLMAPPPLRGESTPKQYEHEVEKESAFALGLIAVKPEHQQLIVDAGALSHLVDLLRRHKSSSNSRAINGVIRRAADAITNLAHENNVIKTCVRIEGGIPPLVELLEFVDVKVQRAAAGALRTLAFKNDENKNQIVQCNALPTLILMLQSEDPTVHCEAVGVIGNLVHSSPNIKKEVLLAGALQPVIGLLSSSCSESQREAALLLGQFAAADSDCKVHIVQRGAVRPLIDMLESPDAQIKEMSAFALGRLAQEMHNQAGIAHSGGIVPLLKLLESKNGSLQHNAAFALYGLADNEDNVAELVKVGGFQKLQDGEFIVQATKDCVDKTLKRLEEKVHGQVLNHLLYLMRVAEKSVQGQIALALAHLCAPDDRKAIFLDNNGLELLLGLLESGNQMQQHAGAAALYKLAAKTTSVSLLDAAPLSPTPQVYLGEQFVNNPTLSDVTFLVEGKRFYAHRICLLASSDAFRAMFDGGYRERDAKDVEIPNIRWDVFELMMRFIYTGSVDVDIEVAQDLLRAADQYLLEGLKLLCEYTIAQDISVENVSLMYELSEGFNARSLMEACILFIFEQFDKLSSKPWCSHLIQHILPEKFWS

SEQ ID NO: 148 - protein, 707 aa, Manihot esculenta
MEPQRSQDQSLSERKGQKRKLEEEIEEKQREISAAVPFGDAREALLYEVTAQVNILNSTFSWNEADRAAAKRATHVLAEFAKNEELVNVIVEGGAVPALIKHLQAPYTNEADRNPKPFEHEVEKGSAFALGLLAVKPEHQQLIVDAGALSLLVDLLKRHKDGSSSRAVNSVIRRAADAITNLAHENSSIKTRVRVEGGIPPLVELLEFTDTKVQRAAAGALRTLAFKNDENKKQIVECNALPTLILMLRSEDAAIHYEAVGVIGNLVHSSPSIKKEVLAAGALQPVIGLLSSCCSESQREAALLLGQFAATDSDCKVHIVQRGAVQPLIEMLQSPDVQLREMSAFALGRLAQDSHNQAGIAHNGGLVPLLKLLDSKNGSLQHNAAFALYGLADNEDNVSDFIRVGGVQKLQDGEFIVQATKDCVSKTLKRLEEKIHGRVLNHLLYLMRVAEKAVQRRVALALAHLCSPDDQRTIFIDNNGLELLLGLLGSTSPKQQIDGAVALYRLANKAMSLSPVDAAPPSPTPQVYLGEQYVNNSTLSDVTFLVEGRRFCAHRICLLASSDAFRAMFDGGYLEKDARDIDIPNIRWEVFELMMRFIYTGSIDISLDIAQDLLRAADQYLLEGLKRLCEYTIAQDISLENVASMYELSEAFHAISLRHTCILFILEHFDKLNAKPRHSHLIQRIIPEIRNYFAKALTKINPRNLRL

SEQ ID NO: 149 - DNA, 3846 bp, Brassica napus
  source 1..3846: mol_type = genomic DNA
atggagagtcaacagaagcgccagcgaacaacacgcctcgccggaagaaacttgaggcgaaagctgtcccgggagacagacgcgtcgtcgtcgatagtcatgcagattacggaggtcgtagacgaagaagcagatctcgtcgtcgcgatccgccgccacgtcgaggttttgaactccagcttctcagatcgcgaagctgtcaaagaagctgctgctgctatctcctctctcgctaaaatcggtacactagtctccgcgattatgttgaaatgtctagtccttagtttccgaacggctttggattgctcaatctcgtgttagatctgattgaatcgatacagattttgaattccacttgtcaatcgatttgtgattctttgggatcagttttatattatgtatctgtttgtatagacgaaaacgtggagatgatggtggagaatggagttatccctgctttggttaggtatctagaatcgccgtggtctttggcgatcaatccaaacgttcctaaatcgtgcgatcataagctggagaaagactgtgctgtttcccttggacttatcgctgctattcaggtaactcaatctttcaactgtggatgaggagttgtgaatctctcagtttctgtttattaatgttagttttatttgttacatagcctggttaccagcagctcattgtggatgctggggccatagttcccactgtgaagttgttgaagagacgaggggtttgtcttgggtgcatggaagctaacgctgttattaggagagctgctgatatcatcactaatattgctcatgacaatccaaggattaaaacaaatataaggtattgtttgttgtttgatgatcattataggttttggtcatgcctatgcttacaccttttgtaaaacttttttttttcagggttgaaggtggcattccaccacttgttgagcttttaaattttccggatgtcaaagtccagagggctgctgcaggggccttgcgaacagtttcatttagaaatgatgataacaagaaccaagtatgttttgatgtgatgatgctttcttttgtttgatatgagaggcttgattcttacattaaaagcaaaattgtgtagattgtggagttgaatgctttgcccacgcttgtattgatgcttcagtcagaagatccttctatgcatggcgaagcggtaggttcttaccttgctttagatggctgcagttggttcgctttgtttctactaatatagactatggatttttttttcagattggggcaattggaaatcttgtccactcatctcctgacatcaagaaagacgttatccgtgctggtgccttacaaccagtgatcagtttacttaggtatgctttttattgtttttctacttagacatttgcttctgaaatttttgtaatatgtttagtaactttttgctatctgctacagctccacttgtttagagacacagagagaagcagcattactaataggtcaatttgcttcgcctgattcagattgcaaggtatgagctagtctctttcatcgcatgctgtagtaataatcttaacatatgcatgctttagtaataatcttaacatatgctcaatcaaactcaggagagaacttattaaacatagctggcaaaatgataatgcaggtgcacattgcccagagaggtgccattacaccattgattaagatgcttgagtcatcagatgagcaggtcatggaaatgtcagcttttgctcttggtcgtttggctcaggtacttatctttttgaattagcatgtgaatgttttcgttgcttctggaatctggttcgttatcaacgattgttaaatcataccttttatgtgataaaaatagtaatcctaaatttgcttggtacatatcttaatacgccggtatattctcaatgcaatgttgcaggacacacacaatcaagctggcattggacaaagaggaggcatcatctcactactaaatcttcttgatgtgaatactggatctgtgcaacacaacgctgcatttgctttgtatggccttgcagataacgaggtaaactaagttcacagtgaataattttgaaacagctgtcttttagtaactatacataccattgagtacctaaacaagatttttgtaaacaggaaaatctagcagacttcattaaggctggaggtattcaaaggcttcaagatgacaacttcactgttcaagtatgcttttgactgcttatgttgcaaaaccaatctataacatttccaaattctgatttatattcttctgtctgcagccgactagggattgtgttgtgaggacactgaagaggctagagaacaaggttcatggacctgtgagtatctatttctgttagtcctactggttcttatttaagtatggctttggttttagacccctgatgtcaaacccttctttcaggtactgaaccaattattatatctgatgagaaccactgagaagcctatacaaatgcgaattgctttggctcttgcacatctttgtgaccctaaagatggaaaattaattttcattgataacaacggtgagaatctcatttttcagaatttatatatttctgttgggttttactgtttctgatcaatatacgtattactaatgtaggagtagagtttctgttggagcttctatacttgtcaggcatgaaacagcagaaatatagttcaagggctttatttgaattagctagaaaagctacttcctttgcgccagaggactcagctccttcctcacccacccaacgggtaagaaaacttcattttttttttcaagtttaaaaactacttgtgatttgtggtcttgacttgtgattgattgtattactgaaggtttttttgggtgcggagttcgtgaacaaccctactttgtccgatgtcacattcctagtcgatggtacaacatttaatcccattctatgtttctgttaattctacctgcggataacactttctaattgaatgtttccatggcgtattatcaggtaaacaattctatgctcacaagatttgcttggtagcttcctctgatatattccgtgcaatgtttgacggcctttacaaggtaagcctctgaataaatgatttgcatcatatatatagaaatcactcaactaacttgagaattggttttaggaacggaacgcccaaaacgtggagattccaaatataacatgggaagtgtttgagcttatgatgaggtaaagttctataaaatcaaacgtttgaatattaccaaacttaaaataaagaatcttagcatgaaaacacaaaatgtgcagattcatatacacaggaagaattgacatcaccaaacatttggctcaagagctgcttgttgcagctgatcagtatcttatcgaaggcctcaagcgcctttgtgagtacacaatcgcacaggtataatatataagcaaaaacctaggtcttattcttttgcaagttagagcgactactaaatggagtttaccaaatgttggtgcaggacatctgtgtggataacataccgttaatgtatgacttagctgatacattcaacgcttcagccttaagacgagcatgtactctcttcgttcttgagcattacactaagctcagctctgaaacatggtatgccatcaaattcattataattttgttttggaagttctagctttggtccccttttataactcaaataatgtttaattttattcttctgtaacgcaggtttcccatgtttatcaagaaaattatacctgaaatccggacatacatcacagatattctcacacggccagtccaagctagctcaaccgttgtataa

SEQ ID NO: 150 - DNA, 3828 bp, Brassica napus
  source 1..3828: mol_type = genomic DNA
atggagagccaacagaagcgccagcgaacaacacgcctccccggaaggaacttgaagcgaaagctgtcccgggatacagacgcggcgtcgtcgatagtcatgcagattacggaggtcgaagacgaagaagcagatttcgtcgcctcgatccgccgccacgtggaggttttgaactccggcttctcagatcgcgaagccgttaaagaagctgctgctgctatctcctctctcgctaaaatcggtacactagtccttcgtttttaatcctcgactccgcgattatgttgaaatggcttctccttagtttcggagcggctttggattgctcaatctattgctagatctgattgaatctatacagattttgaattctacttgtcaattgggattagttttatattctgtatctgtttgtatagatgaaaacgtggagatgatggtggagaatggagtcatccctgctttggttagatatctagaatcgccgtggtctttggcgatcaatccaaacgttcctaaatcgtgcgagcataagctggagaaagattgtgctgtttcccttggacttatcgctgctattcaggttaactcaaacttttaaaatgtggatgaggagttgtgaatctctcagtttctgtttattaatgttagatttatttgttgaatagcctggttaccagcagctcattgtggatgctggggccatagttcccactgtgaagttgttgaagagacgcgggatttgtcttgggtgcatggaagctaacgctgttattaggagagctgctgatatcatcactaatatcgctcatgacaatccaaggattaaaacaaatataaggtatggtttgttgtttgataatcctaatggttttggtcatgcctatgcttacaccttttgtattttcagggttgaaggtggcattccaccacttgttgagcttttaaattttccggatgtcaaagtccagagggctgctgcaggggccttgcgaacagtttcatttagaaatgatgagaacaagaaccaagtatgttttgacgtgatgatgctttcttttgtttgagcttatgagaggcttgattcttacattaaaagcaactgtgtagattgtggagttgaatgctttgccaacgcttgtgttgatgcttcagtcagaagatccttctatgcatggcgaagcggtatgttcttaccttgctttaagtagttgcaattggtttgctttgttcctactaatatattatggaatttttcagattggggcgattggaaatcttgtccactcatctcctgacatcaagaaagaggttatccgtgctggtgccttacaaccagtgatcagtttacttaggtatgctatttattgtttttctacttagatatttgcttctgaaattttgtaatatgtttagtaacttattgctatctgctacagctccacttgcttagagacacagagagaagcagcattactaataggtcaatttgcttcgcctgattcagattgcaaggtatgagctagtctctgttatcacatgattcttgacatatgctcagtcaaattcagtttcttttgacaatattaaaagatggatgcaaactagagagaacttattaaacatagctggcaaaatgataatgcaggtgcacattgctcagagaggtgccattacaccattgattaagatgcttgagtcatcggatgagcaggtcatggaaatgtcagcttttgctcttggtcgtttggctcaggtactttttttttttgaattagcatgtgaatgtctttgttggttctggagtctgattgttaaaacagaccttttatgtgataagaacaattgcaattttatttttgcttggtacatatcttaataccttggcatatcctcaatgttttaaatgttgcaggacacacacaatcaagctggcataggacaaagaggaggcatcatctcactactaaatcttcttgatgtgaatactggatctgtgcaacacaatgctgcctttgctttatatggccttgcagataacgaggtaaactaagctcatgattaataattttcgatacatctatactttttgttaactatacataataccatgagtacctaaataaattttccataattaggaaaatatagcagatttcatcaaggctggaggtattcaaaggcttcaagatgataacttcacagttcaagtatgcatttgactgcttacgtttgcaaaaccaatctataacatttccaaaatctgatttatattcttctatttgcagccgactagggattgtgtggtgaggacattgaagaggctagagaacaaggttcaaggaccggtgagtacctatttctgttagacctactggttcttagttaaagtatgacattggttttagacccctgatgtcaaacccttctttcaggtactgaaccaattattatatgtgatgagaaccactgagaaccctatacaaatgcgaattgctttggcacttgcacatctctgtgaccctaaagatggaaaattaattttcattgataacaatggtgataatctcatttttcagaatttatatatttttgttgggttttactgtttctgatcaatatacgtattactaatgcaggagtagagtttctgctggagcttctatacttgtcaggcatgaaacagcagaaatatagttcaagagctttatttgaattagctagaaaagctacttcctttgcgccagaggactcagctccttcctcacccacccaacgggtaagaaaacttcatttttttttcaagtttaaaaactacttgtgattcgtggtcttgacttgtgattaattgcattactgaaggtgtttttgggtgcggagttcgtgaacaaccctactttgtctgatgtcacattcctagtcgatggtacaacatttaatcccattctatgtttctgttaattctacctgtggataacactttctaattgagtgtttccatggcatattatcaggtaaacaattctatgctcacaagatttgcttggtagcttcctctgatatattccgtgcaatgtttgacgggctttacaaggtaagcttctgaataaatgatttgcatcatatatagatagaaatcactcaactaacttgagaattggttttaggaacggaacgcccaaaacgtggagattccaaatataacatgggaagtgtttgagcttatgatgaggtaaagttctataaaatcaaacatttgaatattaccaaacttgagataaagaatcttagcatgaaacacaaaatgtgcagattcatatacacaggaagaattgacatcaccaaacatttggctcgagatctgcttgttgcagctgatcagtaccttatcgaaggcctcaagcgcctttgtgagtacacaatcgcacaggtatgtatacgcaaaaacctaggtggtcttattcttttgcaagttagagcgactactaaatggagtttaccaaatgttggtgcaggacatctgtgtggataacataccgttaatgtatgacttagctgatacattcaacgcttcagccgtaagacgagcatgcactctctacgttcttgaacattacactaagctcagctctgaaacatggtacgccatcaaattcattataattttgttttggaaattctagctttggtccctttttataactcaaataatgttttattttattcttcaggtttcccatgtttatcaagaaaattattcctgaaatccggacatacatcacagatattctcacacggccagtccaagctagctcaaccgttgtataa

SEQ ID NO: 151 - DNA, 3890 bp, Brassica napus
  source 1..3890: mol_type = genomic DNA
atgaaaatctccaaatcgctcaaaatccaccgccgaatctcctcctcgtcagcgatctctaaccatccacctatggaggagaatcatcacaagcgccagcgaacagctcgcgtcgtcgccggaagaacctcaaagcgaaagctcggccgagagacgtacgcggtttcgataatcacgcagatcaccgagaccgaggaagaagaaacagatctcgccgtcgcgatccgccgccacgtggaggttctgaactccagcttctcagatgcggacgatgtcaaaggagctgctgctgctctctcctccctcgctaaaactggtaccgtactccttagagtagatcgttttgtgttacagctgtctgaatcgatgccgatctgtgattctactttgcgattgaattgttctagctcagattaggcgagatctagattgattatggattgattttggattcgtaactctttgtattagacgaaaacgtggagatgatggtggagaatggagcgatccctgcgttggttagaaacttggaatcgccgtggtctttggcaatcagcgggaacgttcccaagtcttgtgatcataagctagagaaagattgtgctgtttcacttggacttattgctgctaatcaggtaacacttgtgaatatcatttactgcttcttgcactgatgcttttactaatgttagctttatatgtttaacagcctgcttaccagcagctaattgtagatgctggggttatagctccaactgtgaagttgttgaagagaagaggggtttgtattgggtgcatggaagctaatgctgttcttaggagagcagctgatatcatcactaatattgctcatgacaatccaaggattaaaactaatataaggtacggtttagtgtttgatgatccttgtgctttttggtcttggctaagttgttttcacttgacagggttgaaggtggcattccacctcttgttgagcttttggattttccggatgttaaagtacagagggctgctgctggggccttgcgtacggtttcttttagaaatgatgagaacaagaaccaagtatgttttgcttttgatgatgcttttttttttttttgagcttatgttaggcatggttcttacattatactctcataaatgtagattgtggagttgaatgctttgcccacgcttgtattgatgcttcagtcagaagatccttctgtgcatggcgaatcggttggttcttttatcttgctttagatttttggaattggtttgttttgtttagttcctgctaatataatattgaaatatcagattggggcaattggaaatcttgtccactcatctcctgacatcaagaaagaggttatccgcgctggtgccttgcaaccagtaatccgtctacttaggtatgcttattttctttattctgtttttctgtttctgctgaaatagatgtttactcttgatattgtgaaacatcttttgtaactgtttctgtttgctatgatatctgctacagctcaacttgcttggagacacagagagaagcagcattgttgattggtcaatttgccgcgcctgattcagactgcaaggtataagtttgcctctttcttgacgttgttgtgctctaatctgaatatatgctcactcaaactctatgttttgacgatatcaaaaggatggattcagagtaaagaaaacgtactaaaacataaatggcaatatgattatgcaggtgcacattgcccagagaggtgcaattacaccattaattaagatgcttgagtcatcagatgagcaggtcacagaaatggcagcgtttgctcttggtcgtttggctcaggtagttatgtttttgaataagcatgtgaatctttttgacgctttgtgtcataagaacaatggttgtaatttgtttgcttagagcataacttaattcgcatacatcaatgctttgaatgtcgcaggacacacacaatcaggctgggattgggcaaagaggaggcattatttcactactaaatcttcttgatgtgaaaactggatctgtgcaacacaacgctgcctttgctttgtatggccttgcagataatgaggtaaactaatctcataatgaatcgttttcaatacatctatactttttgctaactataaataacaatggttaattaatttttcgtaaacaggaaaatgtagcagatttcataaagactggaggtattcaaaagcttcaagatgacaacttcaccgttcaagtatgcatttcgctgcttatgtttgcaagaacaatatataggctttccaaattctaaattgcaagtcttctctttgcagccgactagggactgtgtggtgaggacattgaagaggctagagaacaagattcaaggacctgtgagtacctatctgttagaccttcttgttcttataagtatggctttggttctagagtcccttaatgtcatactcttctttcaggtactaaaccaactattatatctaattaaaaccactgagaagaatatacaaatgcgaattgctttggctcttgcacatctttgtgaccctaaagatggaaaattaattttcatcgataacagtggtaaatattctcatctcaaaattcatcaatttttcttttcttgtcgatttttttctgttcctgatcaatcgactattacatatgctatgttatacaggaattgagtttttgttggagcctctatacatctcaagcatgaaacagcagaagtatagcgcaagagctttattcgaattagctacaaaagctacatcctttgcaccagaggactcagcaccttcctcacccacacaacgggtaagaactcttcattacttctttcaattataaaaatataatttctgatttgaggtcttgacttgttattgattataatactgaaggcgtttttgggtgaggaattcgtgaacaaccctactttgtccgatgtcacattcctgatcgatggtaaaacatttaatcccttcgatgtttatgttaaatctacctgtgataacactttttaaactgagtaattccatggcatatattaggtaaacaattctttgctcataagatttgcttggtagcttcctctgatatatttcgtgcaatgtttgatggcctttacaaggtaaccttctgaataaatcattgtggtacccatttcatgatacaaagtatcaatcaactaacttgagaattggttttaggaacgaaacgcccaaaatgtggagatcccaaatataagctgggaagtgtttgagcttatgatgaggtaaagttctattaaatcaaaaccataataataagctaagaatctaaagcatgaaatgcaatggtgcagattcatatacacaagaaaaatcaacatcacaaaatacttggctcaagaactgcttgtagcagctgatcagtatcttctcgatggtctcaagcggctttgtgagtacacaatcgctcaggtaaatactcaaaaccaacttcttattcttctccttgtcagagtggcttgtctatgtgtataactaaatggacttctctaatggttggtgcaggacatctgtgtggaaaacataccgttcatgtacgacttagcagatacattcaatgcgtcagccttaagacgagcttgcactctcttcgttcttgagcattacactaagctcagctctgaattgtggtatgcaaaaacaaatcattacatcattaatacattttttttggaatcaaccttatctcttacttaatcaggttttatgttcttttttttttacgcaggtttcccatgttcataaagaaaattatacctgaaatcaggagttacatcactgatattctcggacggccagtccaagctagcagctag

SEQ ID NO: 152 - DNA, 7064 bp, Brassica napus
  source 1..7064: mol_type = genomic DNA
atggagcaacaacaaccggagaggcgagaaggccgaagcttccccgagcgcaagggacagaagagaaagctagaggaaggagcagccgccgccgcagaggatcgagagatctccgcctcaaccaccaccgacggcggcggcgatgcgattctcaacgaaatcgctgctcaagtctccgttctaaactccgccttctcatggcaagaatccgatcgcgctgcggcgaaacgcgccactcaagtcctcgccgagctcgctaaaaacggtagaagatcagcttctttctttttttttttctgcggtttcttcatatatattttttttgttgattcgtgacttagttagtaaccaccgtttgttcagcagaggatttagtgaacgtgattgttgatggaggagctgttccagctcttatgacgcatctacaagcgcccccgtacatcgacggagacttggctcagaagccgtttgaacatgaggttgagaaggggagcgcctttgctcttggtctacttgcaattaaggtttagttactttacaaagcagttgtctttttatgttattttgctccaagtctagttttttcttaaggattatagtatagtgtttgtgatctcgttgtggaattgactgcttacagccagagtatcagaagctgatagtggacaaaggtgctttacctcatctcgtcaatctgttgaagagaagcaaagatggttctacttcccgtgctgtaaatagtgttatcagacgagcggctgatgccatcaccaatcttgctcatgagaacagcagcatcaagactcgtgttaggtcagcttatttaggtggtttgaaagatttgtttttcggtacaactgtcctcatgacttcaagttcttgacaagcaggctcgaaggcggtattccacctctcgttgatttgcttgagttttctgattcaaaggttcagcgagcagcagcaggggcgttgagaacccttgcgtttaaaaacgatgataacaagaaccaggtaaatgtttctgtcttacagcttctatttcagtttttcggtggagcattattcattgtttttttgtgcagattgtcgattgcagtgctcttcccacgctcattctaatgttaggatcagaggatgctgctatacattatgaagcggttaggaatcttttactgggacgagagttttcataatcaactgttttgctagttgctactcaaacatcaacatgacattgacactgaaataacgagttgagtcacgcttttaggttggagttatcggcaatctagtacattcttctccaaacattaaaaaagaggttctttctgctggggcgttgcaacctgtcattggtcttctcaggtgtgtggaactcgccgttttaattacatggttaagcatagagttgttactgttaaccctaggttcattctcatcattttttttgaatttgtctattgcagttcatgttgccctgagagtcaaagagaggcggctttattacttggacagtttgcgtcgactgattccgattgtaaggtactatttcatcccgggttttctatcctcagttcgtttgccattaccccaaagtctaaactctttctgtttggttatactaggcgtaagttgtttgttgctattgatatttgtagaatattcgtttccaattcgtgttatctatcattttccctgatttatgtgtctttttcattcttcacctcattttcaaaaatataactttgcaggtgcacattgtgcaaaggggtgctgtccgtcctttgattgagatgcttcagtcacctgacgtgcagttgaaagaaatgtcggcctttgcactgggtagattggcgcaggttcttgtttcagtcatttgttattttcagtttataaagttgaggcattcttttttggcgttgtaaacttgcaacttcgctctgtagacttataaccatttgagttatattaaataacattaccgatatgtcttttaatgtctagcgtaccctttctcgcaggattctcacaatcaagctggtattgcccatagtggtggtttaggacctttgttgaagcttcttgattcaagaaatggatccctgcaacacaacgcggcatttgctctctatggccttgccgataatgaggtgtgttgtatgctaccttccgtatgtattaattaggaatgcaaaaaaaatatttaaacctcattaaatgggttattgatccatttttgtcccctaggataatgtatcagattttatcagggtgggaggtatccagaagctacaggatggagagtttatagttcaggtatgtatagcgttgttaccctttcactactttctagaatcatatcgtcttattccttgtatcggctagatactgaagattctttgcagctttagtagtctttgttttactctttgggtgttataatttacactgctttttaggcaactaaagattgtgtctccaaaacactgaagagattggaggagaagattcatggaagagtaagtaaaattatacctgtctttaaacttgctctttccacatctggtgactaaaacatacacatgcacggtttgtggtgaaactgctatatcctggtctagctctgtcgaagtttagtatttctctatccaaccattgagacacttgttctttggttttcctttgcaggttcttagacatctgttgtacctaatgcgcatttctgaaaagtctatccaaagacgggttgctctcgctcttgctcatctctgttcaccagaagatcagagaaccatattcatagatgaaaatggcatgtgacaacttttttgaatttattatgtttagactttgacgtgttatccattgttgttaagatgttctttgtgcaaaaagttttatatcgagtttgtcttttgacagggttggagttgctacttggtcttcttggttctacgaacactaaacagcaacttgatggcgctgcagcattgtacaaattagcaaataaatctatggcactttctccagttgaagctgctcccccttctccaacacaaagggtgagctcccgtcttacttcagtcctccaatacataacttgtggaagtctcattgcagtattctttttgtgtatttgtgacaggtttatctcggagagcagtatgtaaatagtgccacgctgtctgatgtaacttttctagtcgaaggtaatcatcatattaatcaggaagttgcagcagtcttgttcgctccaaagtccatatgtaaaccagaaaaatcatactgcaggaaggagattctatgcacacagaatttgtctcctggcatcttcagatgcatttcgcgcaatgtttgatggtggttacagagtaagttagctattatttttgggtgaccaaatccttttcaatatgttcttgcggaggaaatgaaaaaatatcatttactagctatgatgacgatgacatattggttttggctgctctgcttctctttcaaaaggaatatatggatagttatgtttcttgtgtgcaaattgaatatctcactcagtttgtgtttcgtttataccacaggaaaaggacgctagagatattgagattcctaatatcaagtgggaggtttttgagttaatgatgaggtatgacgagcttgcaggcttctttattgtgagaactcttaacatacatgtaaatatgtaattgactcacttggattgtgattcccaggtttatatacactggatccgtcgacataacaattgagatatcacaagatcttctaagagcagcggatcagtatctattggaggggctaaagcggctctgtgaatacacaattgctcaggtgagccagaatacttgcaatttcaagtgatgtggtttgcataataattgtcgaaatctaacacagttttgcttataaatgaaaggatataacgttggaaaacataggaggcatgtacgatctctcagaagcattccacgcaatgtcgctgaggcaagcttgtatcctgttcatcctggagcatttcgataaactgagcacaatgcatgggtaatataaataagctctgtctctctctctctctctttttttttcagactatctctctatttggcatttatctgaaacagagcgaatgaaaaatggcaggcaaaaccagctggtacagcgaacaataccagagataagagagtacttttgtagagctctaacaaagtctactacaaacctgcaaggcctgaggctgtaagaagaagaagactggtacctaactagggaggtaagtagacaaggaatatcatatagagagagaaagctcggtattagtaagaggtctttatggtcttgtcctatcctgagtcgttttagcaaatttgctgtgcgtttggttcattgtattttgtatcaaattctcttctggtcacaatcgcgtcttaaaaagagatcgccactttgtatccaaaacaccattatggtgaaacttcctctattcaattcaagatccacggaccacggtccaacgatcctgtgttagaagaaaatatacactgtgatgatggaatatggtagtgacaaatcagttcttgactaaatgattaatcagagaggaaaaataataatatttgttaatttttaatattatttgaggaaccgacgacatatacagtaataatatcccgttttggctttacaactaaataattgaaagaaatggcttgccattaggttattataaaatagcaactctaatatttttggagtttctgccggcagatatattttttttattatttcagaatgatagaaaatgaaaggtatataattataaataattttttttgaatatactcaaagaaaaaaataaaataaatcaaaatgttctcttacaaacaccaaattacaagcaccaaaagaagaaagaaaaaaattacaagtaccaaagtgaatgctttaatgctttatggtcacgacgtataattattattttatatattctttttgcctgaatgcttttttttatgattcagcgggaggggagatttaatttaaaggagctccggtgagaaaccctagcaccctctcatttcgagattcagccactgctcatcgctcaggtacgcttttgcttttgatctcctcagattttcgcgattagatgcgtcttctggaaactatccactatgcaatgcgatctccgatctttttacaatcactcttcgtaatctcctctgttatagatttatgcaaagtagtgatttattttatttattattagattcgaatctgatgatccttcaatcaaagccttctgctcgctacagtgtgattttgaattgaaaaatcattcctttgggctcaaagttatagtctttgtttgactacagttacaaccattgagcctcctcctctgattcttgaatgtgtgtgtttgtgcagtgatggctgatacactcgattcccgacctcacacattctccatcaaactctggccaccgagtctacccacaaggcaagctctcatcgagcgcatgaccaacaacctctcttccaaaaccattttcaccgacaagtttggcagcttaaccaaagaccaggccatggagaacgccaagaggatcgaggacgttgctttctccaccgctaacctacagttcgagagggagcctgacggtgacggcggctcagctgtgcagctctacgccaaagaatgcagtaagatgattttagaagtcctcaagaaaggccctgtttgtaaggctgaacaagtatcttctgcttctccttgtaaggaaactgttttcgatatttcgaaagacaaaagagcttttattgaggccgaggaggctgaggagcttctcaaaccgttgaaggagcctgggaatgtttacactaagatatgctttagcaataggagtttcgggttaggagctgcacgtgtcgctgagcctatcttggcctctctgaaagaccagcttaaggttgttgacttgtcggacttcgtcgctgggagacccgaggttgaagctcttgaggttatgaatatattctctagtgccctggatggtagtgttctctcgtctctcaacttatcagacaacgcgttgggtgagaagggtgttagagcgttcgggacgctcttgaaatctctgagctctttggaggagctttatctgatgaacgatggtatctctaaagaagctgcacaagctgtctccgagttgattccttcaacggagaagttgagggtcttgcattttcataacaacatgactggagatgaaggagcggttgcgatctcagaggttgtcaagcgttctccgctgctggagaatttcagatgttcttcaacaagagttggtgaaggaggaggtattgctttgtccgaagcacttgagaattgtactcttatggagaaactcgatctgagggataatatgtttggcacagaagctggagtttctctgagcaagactctttcaaggttcgaacatttggctgaggtttacttgagttatctaaacctagaggacgaaggtgccatagccatagcaaacgctctcaaggactctgctgcgcccattgaggttcttgagatggcgggaaatgacataacggttgaagccgcttcagctattgcggcctgtgtggcggcgaaacaggatctgaacaagttgaatttgtctgagaatgagctgaaagatgaggggtgtgtccagattgcaaagagtgtggaagaggagcatttgaaactgcaatacattgacatgagcaacaattacataagaagagctggagcacgggccttggctcaggttgttatcaagaaagaaggtttcaagttgctgaacatcgacgggaatatcatatcagaggaaggcattgaggaagttaaagagatattgaagaaaaccccggaggtacttggagcattggacgagaatgatcctgatggagaagaggaagaagatgatgaggaagatgaagagaaggaaggtgaagggaatgatgagttggaatcgaagctgaagaagcttgaagttaatgaggatgattaa

SEQ ID NO: 153 - DNA, 3925 bp, Brassica napus
  source 1..3925: mol_type = genomic DNA
atggagcaacaaagaggaagccggagctttccggagcgcaagggacagaagaggaaactagaggaaggaccacccgcagaggatccacagatctcttcctcaaccaccaccgacgcagcccctcacgctgcgcttctcagcgaagtcgctgctcaagtctccgttctaaactccgccttctcctggaaagaatccgatcgcgccgccgcaaagcgcgcagctcaagtcctggctgagctcgccaaaaacggtgaacatcagtctcctatagcttcacttttcttcggtttcttattatctcttagcgaaccttcgatgttcagcagatgatttagtgagcgtgattgtcgacggaggtgctgttcctgctctcacgacgcatctacagcccccgccgtactgtgaaggagacttagctcacaagccgtttgaacatgaggtcgagaaaggaagcgcctttgcgcttggtcttctcgcaattaaggttttggtcccaagtttagttttttaaagcaacttttggtaataaagtttctatgtttatattcggaggggactatgtacagtttgtgtgatcacgttgtggaattgattacttacagccagagtatcagaacctgatagtagacaaaggagctttacctcatctcgtggatctcttgaagagaagcaaagattcctccacttctcgagcccttaatagtgttattagaagagcggctgatgccattactaatctagctcacgagaacagcagcatcaagacccgtgtcaggtcagcttatttttctaagtggtttcctccttttcagtacaactatcctcctgactttttgacaaaacaggctagaaggcggtattccacctctcgtggagttgcttgagtattctgattccaaggttcagcgagcagcagcaggggcgttgcgaacgcttgcgtttaaaaacgatgataacaagaacctggtaagtattgctgtcttatagcttctacttagatttttggacggagtgtgttttgattgtctacttttgcagatagttgaatgcaatgctcttcccacgctcattctaatgcttggatcagaggatgctgctatacattacgaagcggttaggattcttttactgcgtcgagagttttcataatcaactcttttgctacttatctgagtcatgcttttaggttggagttataggcaatctagttcattcgtctccgaacattaaaaaagaggttatttcttctggggcgttgcaacctgtcattggtcttctcaggtatgtggaaactcgtcattttgatttaaatggttaagcatagagttgttactgttaaccttagtgacgttcttgttgtttcttgtattttgtctatttcagctcatgttgccctgagagccaaagagaggcggctttattacttggacagtttgcctctactgattctgattgtaaggtactatttcatctctatcctcagttcgtttgctatccaccaaagcataaactctttctgcttggttgtactaggtgtaagctgttttttcttctgttgattttcaggttcacattgttcaaaggggtgctgttcgtcctttgattgaaatgcttcagtcagcggatgttcagttgaaggagatgtcggcctttgcactgggaagattggcccaggttcctcttttaaacctttgttagtttgagccgctgtaaaattgtaacctcgctctttaggcttaaaaccaatgagctatattaaaattacaaaactgttatgtcttttaattctctagcatactctttgtcgcaggattcccacaaccaagccggtattgctcatagtggtggtttagaacctttattgaagcttctcagttcaagaaatggatccttgcaacacaatgctgcctttgctctttatggccttgccgataatgaggtgcgttgaatgctgctaccttccgtatatgttataattaggatgcaaaattccttattaaattggttattgatccccatttttctccccgtaggataatgtgtcgggttttatcagggtgggaggtgtccaaaagctacaggatgaagagtttattgttcaagtatgtgaatcatatcgtcatttttcttttagtggctatatactgaaatttcttagcagctgtatttgttttactctctcgttggatgtttctaatgtacaatgtttcttaggcaactaaagattgtgtctccaaaacattgaagaggttggaggagaagattcatggaagagtaagtaaaattttacctgtctttaaacttgttacttccatctctggtgattaaaaaaatacacaaatgcacggtttgtagtaaaactgatgtatcctggtctagtgtctgaaactttgtttaagtttagtatttctctatggaacctttgaaacttatgtgctttggatttcctttgtaggttctaaggcatctgttgtaccaaatgcgcatttctgagaagtctatccaaagacgagttgctctcgctcttgctcatttctgttcaccggaagatcagagaaccgtattcatagatgagaatggcatgtgacagatttttttgaatttatgatgttaagacttttaacgctttaaccattaagtttaaatgttctttctgcaattctttttatattgagctgtcttttgacagggttggagttgctacttggtcttcttggttctacaaacactaagcagcaactcgatggcgctgcagcattgtacagattagcaaataaatccatggcactttctccagttgatgctgctcctccttccccaacacaaagggtgagtcaccttcttgcttcagttctccattacgtaagttgtggaagtctcagtgcatcattctgtttatctttttgtgacaggtttatctcggagagcaatatgtaaatagtgcaacgctgtctgatgtaacttttctagtcgaaggtaatcatattactcagaaaattgcagcagtcttgttagctccaaacaccatatgtaaaacagaaaagatcatactgcaggaaggagattctatgcacacagaatttgtctgctggcttcttcagatgcatttcgcgcaatgtttgatggtggttaccgagtaagtgaactattatgttctttttgaaaaacatctactagctataatgactattatctatgaaactctgcttctctgtcaaaggaatacatggataattatgtaaacatgtctcattcagtttgtgcttcgtttataccataggaaaaagacgctagagatattgagattccgaatattaaatgggaggtttttgagttaatgatgaggtatgacgagtttctacaagcttctagactgagaactttcgtcatatacatgtaactaactcacacttgaactgtgatcttcaggtttatatacactggatcagtcgacataacaattgagatatcacaagatcttctgagagcagcggatcagtatctcttggagggtctgaagcgactctgtgaatacacaattgctcaggtgagtcagaacaatggaaaatgatgtggtttgcattataattctggaaatctaacacggttgcttatgaatgaaaggatataacgttggaaaacataggaagcatgtacgatctctcagaagcattccacgcgatgtcgctgaggcaagcttgtatattgttcatcctggagcatttcgaaaaactgagttcaatgcatgggtaatatgaagtacctctctcttactctcacagtctttggcctatatatctgaaacatagtggatgaaaaatgcaggcagaacgagctggtgcagcgaacaataccagagataagagagtacttctgtagagctctaacaaaatctactacaaacctgcaaagcctgaggttgtag

SEQ ID NO: 154 - DNA, 3020 bp, Brassica napus
  source 1..3020: mol_type = genomic DNA
atggagcaacaacgagaaagccggagctttccagagcgcaagggacagaagaggaaacttgaggaaggaccacccgccgccgcagaggatccacagatctctccctcaaccaccaccgacgctgcgcttctcagcgaagtcgctgctcaagtctccgttctaaactccgccttctcctggaaagaatccgatcgcgccgccgcaaagcgcgcagctcaagtcctcggtgaacatcagtctcgactctcctatctcgcttcagttttcatatcttttagtgaaccttcgatgttcaagcagaggatttggtgaacgtgattgtcgacggaggtgctgttcctgctctcacgacgcatctacagcccccgccgtgcagcgacggagacttagctcacaagccgttcgaacacgaggtcgaaaaaggaagcgcctttgcgcttggtcttctcgcaattaaggttttggtcccaagtttagttttttaaaggcaacttttggtaataaagtttcatatttttaattaccgaggggactatgtgatcacgttgtgggattgactgcttttacagccagagtaccagaacctgatagtagacaaaggcgctttacctcatctcgtgagtctcttgaagagaaacaaagagggccccacttctcgtgctgttaatagtgttgttagaagagccatcaccaatctagctcatgagaacagcagcatcaagactcgtgtcaggtcagcttatttatttaagtgatttaagatttgttttcagtgcaactctcctcgtgactgttcagttgttgacaaagcaggttagaaggcggtattccacctctcgtggagttgcttgagtattctgattccaaggttcagcgagcagcggcaggggcgttgagataacaagaacctggtagaaattgctatctttcagcttctacttagatttttggacggagcgtgttttgattgcctacttttgcagatagttgaatgcaatgctcttcccacgctcattctaatgctaggatcagaggatgctgctatacattacgaagcggttaggattcttttcctggtcgagagttttcacaattaactgtttgactacttatctgagtcatgcttataggttggagttataggcaatctagtacattcgtctccaaacattaaaaaagaggttatttcttctggggcgttgcaacctgtcattggtcttctcaggtgtgtggaaactcgccattttaatttacatggttaagcatttagttgttactgttaaccttagggtcattcttgttgtttattgaatttgtctctttcagctcctgttgccctgagagtcaaagagaggccgctttattacttggacagtttgcctctactgattctgattgtaaggtactatttcatctctatcctcagttcgtttgctatccaccaaagcataaactctttctgtttggctgtactaggtgtaagctgtttgtttctgttgattttcaggttcacattgttcaaaggggtgctgttcgtcctttgattgaaatgcttcagtcaccgtatgttcagttgaaggagatgtcggcctttgcactgggaagattggcccaggttcctcttttaagcctttgttagtttgagcgctgtaaaattgtaacttcgctctttaggcttaaaaccatttagttgtattaaaattacaaaactgttatgtcttttaattttctagcatactctttcttgcaggattcccacaatcaagccggtatagctcatagtggtggtttagaacctttattgaagcttctcagttcaagaaatggatccttgcaacacaacgcagcatttgctctttatggtcttgccgataatgaggtgcgttgaatgctaccttccgtatatgttataattaggatgcaaaatttctctatggaacctttgaaaattacgtgctttggatttcctttgtaggttctgaggcatctgttgtacctaatgcgcatttctgaaaagtctatccaaagacgacttgctctcgctcttgctcatttctgttcaccagaagatcagagaaccatattcatagatgagaatggcatgtggcagcttttttgaatttattatgttaaagactttttaacacgtcaggcattcagtttagatgttcgttctacaaaaaagttttatattgagatttcttttgacagggttggagttgctacttggtcttcttggttccacaaacactaagcagcaacttgatggtgctgcagcattgtacaagttagcaaataaatctatggcactttctccagttgatgctgctgctccttctccaacacaaagagtgggttcccttcttacttcagctctccattacataagttgtggaagtctcaatgcatcattctgtttgtctttttgtgacaggtttatctcggagagcaatatgtaaataatgctacgctttatgatgtaacttttctagtcgaaggtaatcatattaatcaggaagttgcagcagtcttgttagcgtcaaactccatatgtaagatagaataaatcatactgcaggaaggagattctatgcacacagaatctgtctgctggcatcttcagatgcattccgcgcaatgtttgatggtggttacagagtaagtgaactattatgttctttttgaggaaatatagaaaaacatctactagctataatgactattatctatgtaaacatgtctcattgagtttgtatttcgtttatacaacaggaaaaagacgctagagatattgagattccgaatattaaatgggaggtgtttgagttaatgatgaggtatgacgagcttacacaggcttctgactgagaactttcttcctaaaaatgtaattgactcacacttgaactgtggtactcaggtttatacactggatcagtcgacataacaatagagatatcacaagatcttctgagagcagcggatcagtatctcttggagggtctgaagcgactctgtga

SEQ ID NO: 155 - protein, 707 aa, Brassica napus
MESQQKRQRTTRLAGRNLRRKLSRETDASSSIVMQITEVVDEEADLVVAIRRHVEVLNSSFSDREAVKEAAAAISSLAKIDENVEMMVENGVIPALVRYLESPWSLAINPNVPKSCDHKLEKDCAVSLGLIAAIQPGYQQLIVDAGAIVPTVKLLKRRGVCLGCMEANAVIRRAADIITNIAHDNPRIKTNIRVEGGIPPLVELLNFPDVKVQRAAAGALRTVSFRNDDNKNQIVELNALPTLVLMLQSEDPSMHGEAIGAIGNLVHSSPDIKKDVIRAGALQPVISLLSSTCLETQREAALLIGQFASPDSDCKVHIAQRGAITPLIKMLESSDEQVMEMSAFALGRLAQDTHNQAGIGQRGGIISLLNLLDVNTGSVQHNAAFALYGLADNEENLADFIKAGGIQRLQDDNFTVQPTRDCVVRTLKRLENKVHGPVLNQLLYLMRTTEKPIQMRIALALAHLCDPKDGKLIFIDNNGVEFLLELLYLSGMKQQKYSSRALFELARKATSFAPEDSAPSSPTQRVFLGAEFVNNPTLSDVTFLVDGKQFYAHKICLVASSDIFRAMFDGLYKERNAQNVEIPNITWEVFELMMRFIYTGRIDITKHLAQELLVAADQYLIEGLKRLCEYTIAQDICVDNIPLMYDLADTFNASALRRACTLFVLEHYTKLSSETWFPMFIKKIIPEIRTYITDILTRPVQASSTVV

SEQ ID NO: 156 - protein, 755 aa, Brassica napus
MESQQKRQRTTRLPGRNLKRKLSRDTDAASSIVMQITEVEDEEADFVASIRRHVEVLNSGFSDREAVKEAAAAISSLAKIDENVEMMVENGVIPALVRYLESPWSLAINPNVPKSCEHKLEKDCAVSLGLIAAIQPGYQQLIVDAGAIVPTVKLLKRRGICLGCMEANAVIRRAADIITNIAHDNPRIKTNIRYGLLFDNPNGFGHAYAYTFCIFRVEGGIPPLVELLNFPDVKVQRAAAGALRTVSFRNDENKNQIVELNALPTLVLMLQSEDPSMHGEAVCSYLALSSCNWFALFLLIYYGIFQIGAIGNLVHSSPDIKKEVIRAGALQPVISLLSSTCLETQREAALLIGQFASPDSDCKVHIAQRGAITPLIKMLESSDEQVMEMSAFALGRLAQDTHNQAGIGQRGGIISLLNLLDVNTGSVQHNAAFALYGLADNEENIADFIKAGGIQRLQDDNFTVQPTRDCVVRTLKRLENKVQGPVLNQLLYVMRTTENPIQMRIALALAHLCDPKDGKLIFIDNNGVEFLLELLYLSGMKQQKYSSRALFELARKATSFAPEDSAPSSPTQRVFLGAEFVNNPTLSDVTFLVDGKQFYAHKICLVASSDIFRAMFDGLYKERNAQNVEIPNITWEVFELMMRFIYTGRIDITKHLARDLLVAADQYLIEGLKRLCEYTIAQDICVDNIPLMYDLADTFNASAVRRACTLYVLEHYTKLSSETWFPMFIKKIIPEIRTYITDILTRPVQASSTVV

SEQ ID NO: 157 - protein, 729 aa, Brassica napus
MKISKSLKIHRRISSSSAISNHPPMEENHHKRQRTARVVAGRTSKRKLGRETYAVSIITQITETEEEETDLAVAIRRHVEVLNSSFSDADDVKGAAAALSSLAKTDENVEMMVENGAIPALVRNLESPWSLAISGNVPKSCDHKLEKDCAVSLGLIAANQPAYQQLIVDAGVIAPTVKLLKRRGVCIGCMEANAVLRRAADIITNIAHDNPRIKTNIRVEGGIPPLVELLDFPDVKVQRAAAGALRTVSFRNDENKNQIVELNALPTLVLMLQSEDPSVHGESIGAIGNLVHSSPDIKKEVIRAGALQPVIRLLSSTCLETQREAALLIGQFAAPDSDCKVHIAQRGAITPLIKMLESSDEQVTEMAAFALGRLAQDTHNQAGIGQRGGIISLLNLLDVKTGSVQHNAAFALYGLADNEENVADFIKTGGIQKLQDDNFTVQPTRDCVVRTLKRLENKIQGPVLNQLLYLIKTTEKNIQMRIALALAHLCDPKDGKLIFIDNSGIEFLLEPLYISSMKQQKYSARALFELATKATSFAPEDSAPSSPTQRAFLGEEFVNNPTLSDVTFLIDGKQFFAHKICLVASSDIFRAMFDGLYKERNAQNVEIPNISWEVFELMMRFIYTRKINITKYLAQELLVAADQYLLDGLKRLCEYTIAQDICVENIPFMYDLADTFNASALRRACTLFVLEHYTKLSSELWFPMFIKKIIPEIRSYITDILGRPVQASS

SEQ ID NO: 158 - protein, 756 aa, Brassica napus
MKISKSLKLHRSNPPSNLLLVRRPSSISNLPPMENNLKRQRTTRVAGRSSKRGRETYAVSIITQITEIEEEETDLVVAISRHVDVLNSSFSDAGDVKGAAAALSSLAKTDENVEMMVENGAIPALVRNLESPWSLAISGNVAKSCDHKLEKDCAVSLGLIAANQPAYQQLIVDAGVIAPTVKLLKRRGVCIGCMEANAVLRRAADIITNIAHDNPRIKTNIRYGLVFDDPYAFFGLGYKLFSLDRVEGGIPPLVELLDFPDVKVQRAAAGALRTVSFRNDENKNQIVELNALPTLVLMLQSEDPSVHGESIGAIGNLVHSSPDIKKDVIRAGALQPVIGLLSSPCLETQREAALLIGQFAAPDSDCKVHIAQRGAITPLIKMLESSDEQVTEMAAFALGRLAQDTHNQAGIGQRGGIISLLNLLDVKTGSVQHNAAFALYGLADNEENVADFIKTGGIQKLQDDNFTVQPTRDCVVRTLKRLENKIHGPVLNQLLYLMKTTEKNIQMRIALALAHLCDPKDGKLIFIDNSGMEFLLEPLYISSMKQQKYSARALFELATKATSFAPEDSAPSSPTQRAFLGEEFVNNPTLSDVTFLIDGKQFFAHKICLVASSDIFRAMFDGLYKERNAQNVEIPNISWEVFELMMRFIYTGKINITKYLAQDLLVAADQYLLEGLKRLCEYTIAQDICVENIPFMYDLADTFNASALRRACTLFVLEHYTKLSSELWFPMFIKKIIPEIRSYITDILRRPVQASS

SEQ ID NO: 159 - protein, 1266 aa, Brassica napus
MEQQQPERREGRSFPERKGQKRKLEEGAAAAAEDREISASTTTDGGGDAILNEIAAQVSVLNSAFSWQESDRAAAKRATQVLAELAKNAEDLVNVIVDGGAVPALMTHLQAPPYIDGDLAQKPFEHEVEKGSAFALGLLAIKPEYQKLIVDKGALPHLVNLLKRSKDGSTSRAVNSVIRRAADAITNLAHENSSIKTRVSRLEGGIPPLVDLLEFSDSKVQRAAAGALRTLAFKNDDNKNQIVDCSALPTLILMLGSEDAAIHYEAVGVIGNLVHSSPNIKKEVLSAGALQPVIGLLSSCCPESQREAALLLGQFASTDSDCKVHIVQRGAVRPLIEMLQSPDVQLKEMSAFALGRLAQDSHNQAGIAHSGGLGPLLKLLDSRNGSLQHNAAFALYGLADNEDNVSDFIRVGGIQKLQDGEFIVQATKDCVSKTLKRLEEKIHGRVLRHLLYLMRISEKSIQRRVALALAHLWLELLLGLLGSTNTKQQLDGAAALYKLANKSMALSPVEAAPPSPTQRVYLGEQYVNSATLSDVTFLVEGRRFYAHRICLLASSDAFRAMFDGGYREKDARDIEIPNIKWEVFELMMRFIYTGSVDITIEISQDLLRAADQYLLEGLKRLCEYTIAQDITLENIGGMYDLSEAFHAMSLRQACILFILEHFDKLSTMHGQNQLVQRTIPEIREYFCRALTKSTTNLQGLRLFSRLDASSGNYPLCNAISDLFTITLLMADTLDSRPHTFSIKLWPPSLPTRQALIERMTNNLSSKTIFTDKFGSLTKDQAMENAKRIEDVAFSTANLQFEREPDGDGGSAVQLYAKECSKMILEVLKKGPVCKAEQVSSASPCKETVFDISKDKRAFIEAEEAEELLKPLKEPGNVYTKICFSNRSFGLGAARVAEPILASLKDQLKVVDLSDFVAGRPEVEALEVMNIFSSALDGSVLSSLNLSDNALGEKGVRAFGTLLKSLSSLEELYLMNDGISKEAAQAVSELIPSTEKLRVLHFHNNMTGDEGAVAISEVVKRSPLLENFRCSSTRVGEGGGIALSEALENCTLMEKLDLRDNMFGTEAGVSLSKTLSRFEHLAEVYLSYLNLEDEGAIAIANALKDSAAPIEVLEMAGNDITVEAASAIAACVAAKQDLNKLNLSENELKDEGCVQIAKSVEEEHLKLQYIDMSNNYIRRAGARALAQVVIKKEGFKLLNIDGNIISEEGIEEVKEILKKTPEVLGALDENDPDGEEEEDDEEDEEKEGEGNDELESKLKKLEVNEDD

SEQ ID NO: 160 - protein, 716 aa, Brassica napus
MEQQRGSRSFPERKGQKRKLEEGPPAEDPQISSSTTTDAAPHAALLSEVAAQVSVLNSAFSWKESDRAAAKRAAQVLAELAKNADDLVSVIVDGGAVPALTTHLQPPPYCEGDLAHKPFEHEVEKGSAFALGLLAIKPEYQNLIVDKGALPHLVDLLKRSKDSSTSRALNSVIRRAADAITNLAHENSSIKTRVRLEGGIPPLVELLEYSDSKVQRAAAGALRTLAFKNDDNKNLIVECNALPTLILMLGSEDAAIHYEAVGVIGNLVHSSPNIKKEVISSGALQPVIGLLSSCCPESQREAALLLGQFASTDSDCKVHIVQRGAVRPLIEMLQSADVQLKEMSAFALGRLAQDSHNQAGIAHSGGLEPLLKLLSSRNGSLQHNAAFALYGLADNEDNVSGFIRVGGVQKLQDEEFIVQATKDCVSKTLKRLEEKIHGRVLRHLLYQMRISEKSIQRRVALALAHFCSPEDQRTVFIDENGICLLTGLELLLGLLGSTNTKQQLDGAAALYRLANKSMALSPVDAAPPSPTQRVYLGEQYVNSATLSDVTFLVEGRRFYAHRICLLASSDAFRAMFDGGYREKDARDIEIPNIKWEVFELMMRFIYTGSVDITIEISQDLLRAADQYLLEGLKRLCEYTIAQDITLENIGSMYDLSEAFHAMSLRQACILFILEHFEKLSSMHGQNELVQRTIPEIREYFCRALTKSTTNLQSLRL

SEQ ID NO: 161 - protein, 554 aa, Brassica napus
MEQQRESRSFPERKGQKRKLEEGPPAAAEDPQISPSTTTDAALLSEVAAQVSVLNSAFSWKESDRAAAKRAAQVLAEDLVNVIVDGGAVPALTTHLQPPPCSDGDLAHKPFEHEVEKGSAFALGLLAIKPEYQNLIVDKGALPHLVSLLKRNKEGPTSRAVNSVVRRAITNLAHENSSIKTRVSRLEGGIPPLVELLEYSDSKIVECNALPTLILMLGSEDAAIHYEAVGVIGNLVHSSPNIKKEVISSGALQPVIGLLSSCCPESQREAALLLGQFASTDSDCKVHIVQRGAVRPLIEMLQSPYVQLKEMSAFALGRLAQDSHNQAGIAHSGGLEPLLKLLSSRNGSLQHNAAFALYGLADNEVLRHLLYLMRISEKSIQRRLALALAHFCSPEDQRTIFIDENGLELLLGLLGSTNTKQQLDGAAALYKLANKSMALSPVDAAAPSPTQRVYLGEQYVNNATLYDVTFLVEGRRFYAHRICLLASSDAFRAMFDGGYREKDARDIEIPNIKWEVFELMMRFIHWISRHNNRDITRSSESSGSVSLGGSEATL

SEQ ID NO: 162 - DNA, 3878 bp, Brassica oleracea
  source 1..3878: mol_type = genomic DNA
atgaaaatctccaagtcgctcaaaatccaccgtcgaatctcctcctcgtcagcgatctcagaccatccacctatggaggagaatcatcacaagcgccagcgaacagcacgcgtcgtcgccggaagaacctcgaagcgaaagctcggccgagagacgtacgcggtttcgataatcacgcagatcaccgagatcgaggaagaagaaacagatctcgccgtcgcgatccgccgccacgtggaggttctgaactccagcttctcagatgcgggagatgtcaaaggagctgctgctgctctctcctccctcgctaaaactggtaccgtactccttagagtagatcgttttgttgttacagctgtttgaatcgatgccgatctgtgattctactttgcgattgaattgttctagctcagattaggcgagatctagattgattatggattgattttggattcgtaactctttgtgttagacgaaaacgtggagatgatggtggagaacggagcgatccctgcgttggttagaaacttggaatcgccgtggtctttggcaatcagcgggaacgttcccaagtcttgtgatcataagctagagaaagattgtgctgtttcacttggacttattgctgctaatcaggtaacacttgtgaatatcatttactgcttcttgcactgatgcttttactaatgttagctttatttgttaaatagcctggttaccagcagctaattgtagatgctggggttatagctccaactgtgaagttgttgaagagaagaggagtttgtattgggtgcatggaagctaatgctgttcttaggagagcagctgatatcgtcactaacattgctcatgacaatccaaggattaaaactaatataaggtacggtttagtgtttgatgatccttatgctttttggtcttggctaagttgttttcacttgacagggttgaaggtggcattgcaccacttgttgagcttttggattttccggatgttaaagtacagagggctgctgctggggccttgcgtacggtttcttttagaaatgatgagaacaagaaccaagtatgttttgcttttgatgatgctttgtttgagcttatgagaggcatgtttcttatataaagagcatctgtgtagattgtggagttgaatgctttgcccacgcttgtattgatgcttcagtcagaagatccttctgtgcatggcgaatcggttggttcttttatcttgctttagatttttggaattggtttgttttgtttagttccttctaatataatattgagatatcagattggggcaattggaaatcttgtccactcatctcctgacatcaagaaagaggttatccgcgctggtgccttgcaaccagtaatccgtctacttaggtatgcttattttctttattctgtttttctgtttctgctgaaatagatgtttactcttgatattgtgaaacatttttgtaactgtttctgttcgctatatctgctgcagctcaacttgcttggagacacagagagaagcagcattgttgattggtcaatttgccgcgcctgattcagactgcaaggtataagtttgcctctttcttgacgttgttatgctctaatctgaatatatgctcactcaaactctttgttttgacgatatcaaaaggatggattcagagtaaagaaaacgtactaaaacataaatggcaatatgattatgcaggtgcacattgcccagagaggtgcaattacaccattaattaagatgcttgagtcatcagatgagcaggtcacagaaatggcagcgtttgctcttgggcgtttggctcaggtagttatgtttttgaataagcatgtgaatctttttgacgctttgtgtcataagaacaatggttgtaatttgtttgcttggagcataacttagttcgcatacatcaatgctttgaatgtcgcaggacacacacaatcaggctgggattgggcaaagaggaggcattatttcactactaaatcttcttgatgtgaaaactggatctgtgcaacacaacgctgcctttgctttgtatggccttgcagataatgaggtaaactaatctcataatgaatcgttttcaatacatctatactttttgctaactataaataacaatggttaattaatttttcgtaaacaggaaaatgtagcagatttcataaagactggaggtattcaaaagcttcaagatgacaacttcaccgttcaagtatgcatttcgctgcttatgtttgcaagaacaatatataggctttccaaattctaaattgcaagtcttctctttgcagccgactagggactgtgtggtgaggacattgaagaggctagagaacaagattcaaggacctgtgagtacctatctgttagaccttcttgttcttataagtatggccttggttctagagtcccttaatgtcatactcttctttcaggtactaaaccaactattatatctaatgaaaaccactgagaagaatatacaaatgcgaattgctttggctcttgcacatctttgtgaccctaaagatggaaaattaattttcatcgataacagtggtaaatattctcatctcaaaattcatcaatttttcttttcttgtcgatttttttctgttcctgatcaatcgactattacatatgctatgttatacaggaattgagtttttgttggagcctctatacatctcaagcatgaaacagcagaagtatagcgcaagagctttattcgaattagctacaaaagctacatcctttgcaccagaggactcagcaccttcctcacccacacaacgggtaagaactcttcattacttctttcaattataaaaatataatttctgatttgaggtcttgacttgttattgattataatactgaaggcgtttttgggtgaggaattcgtgaacaaccctactttgtccgatgtcacattcctgatcgatggtaaaacatttaatcccttcgatgtttatgttaaatctacctgtgataacactttttaaactgagtaattccatggcatatattaggtaaacaattctttgctcataagatttgcttggtagcttcctctgatatatttcgtgcaatgtttgatggcctttacaaggtaaccttctgaataaatcattgtggtacccatttcatgatacaaagtatcaatcaactaacttgagaattggttttaggaacgaaacgcccaaaatgtggagatcccaaatataagctgggaagtgtttgagcttatgatgaggtaaagttctattaaatcaaaaccataataataagctaagaatctaaagcatgaaatgcaatggtgcagattcatatacacaggaaaaatcaacatcacaaaatacttggctcaagaactgcttgtagcagctgatcagtatcttctcgatggtctcaagcggctttgtgagtacacaatcgctcaggtaaatactcaaaaccaactttttattcttctccttgtcagagtggcttgtctatgtgtataactaaatggacttctctaatggttggtgcaggacatctgtgtggaaaacataccgttcatgtacgacttagcagatactttcaatgcgtcagccttaagacgagcttgcactctcttcgttcttgagcattacactaagctcagctctgaattgtggtatgcaaaaacaaatcattacatcattaatacattttttttggaatcaaccttatctcttacttaatcaggttttatgttcttttttttttacgcaggtttcccatgttcataaagaaaattatacctgaaatcaagagttacatcactgatattctcggacggccagtccaagctagcagctag

SEQ ID NO: 163 - DNA, 7057 bp, Brassica oleracea
  source 1..7057: mol_type = genomic DNA
atggagcaacaacaaccggagaggcgagaaggccgaagcttccccgagcgcaagggacagaagagaaagctagaggaaggagcagccgccgccgcagaggatcgagagatctccgcctcaaccaccaccgacggcggcggcgatgcgattctcaacgaaatcgctgctcaagtctccgttctaaactccgccttctcatggcaagaatccgatcgcgctgcggcgaaacgcgccactcaagtcctcgccgagctcgctaaaaacggtagaagatcagcttctttctttttttttttctgcggtttcttcatatatattttttttgttgattcgtgacttagttagtaaccaccgtttgttcagcagaggatttagtgaacgtgattgttgatggaggagctgttccagctcttatgacgcatctacaagcgcccccgtacatcgacggagacttggctcagaagccgtttgaacatgaggttgagaaggggagcgcctttgctcttggtctacttgcaattaaggtttagttactttacaaagcagttgtctttttatgttattttgctccaagtctagttttttcttaaggattatagtatagtgtttgtgatctcgttgtggaattgactgcttacagccagagtatcagaagctgatagtggacaaaggtgctttacctcatctcgtcaatctgttgaagagaagcaaagatggttctacttcccgtgctgtaaatagtgttatcagacgagcggctgatgccatcaccaatcttgctcatgagaacagcagcatcaagactcgtgttaggtcagcttatttaggtggtttgaaagatttgtttttcggtacaactgtcctcatgacttcaagttcttgacaagcaggctcgaaggcggtattccacctctcgttgatttgcttgagttttctgattcaaaggttcagcgagcagcagcaggggcgttgagaacccttgcgtttaaaaacgatgataacaagaaccaggtaaatgtttctgtcttacagcttctatttcagtttttcggtggagcattattcattgtttttttgtgcagattgtcgattgcagtgctcttcccacgctcattctaatgttaggatcagaggatgctgctatacattatgaagcggttaggaatcttttactgggacgagagttttcataatcaactgttttgctagttgctactcaaacatcaacatgacattgacactgaaataacgagttgagtcacgcttttaggttggagttatcggcaatctagtacattcttctccaaacattaaaaaagaggttctttctgctggggcgttgcaacctgtcattggtcttctcaggtgtgtggaactcgccgttttaattacatggttaagcatagagttgttactgttaaccctaggttcattctcatcattttttttgaatttgtctattgcagttcatgttgccctgagagtcaaagagaggcggctttattacttggacagtttgcgtcgactgattccgattgtaaggtactatttcatcccgggttttctatcctcagttcgtttgccattaccccaaagtctaaactctttctgtttggttatactaggcgtaagttgtttgttgctattgatatttgtagaatattcgtttccaattcgtgttatctatcattttccctgatttatgtgtctttttcattcttcacctcattttcaaaaatataactttgcaggtgcacattgtgcaaaggggtgctgtccgtcctttgattgagatgcttcagtcacctgacgtgcagttgaaagaaatgtcggcctttgcactgggtagattggcgcaggttcttgtttcagtcatttgttattttcagtttataaagttgaggcattcttttttggcgttgtaaacttgcaacttcgctctgtagacttataaccatttgagttatattaaataacattaccgatatgtcttttaatgtctagcgtaccctttctcgcaggattctcacaatcaagctggtattgcccatagtggtggtttaggacctttgttgaagcttcttgattcaagaaatggatccctgcaacacaacgcggcatttgctctctatggccttgccgataatgaggtgtgttgtatgctaccttccgtatgtattaattaggaatgcaaaaaaaaaatatttaaacctcattaaatgggttattgatccatttttgtcccctaggataatgtatcagattttatcagggtgggaggtatccagaagctacaggatggagagtttatagttcaggtatgtatagcgttgttaccctttcactactttctagaatcatatcgtcttattccttgtatcggctagatactgaagattctttgcagctttagtagtctttgttttactctttgggtgttataatttacactgctttttaggcaactaaagattgtgtctccaaaacactgaagagattggaggagaagattcatggaagagtaagtaaaattatacctgtctttaaacttgctctttccacatctggtgactaaaacatacacatgcacggtttgtggtgaaactgctatatcctggtctagctctgtcgaagtttagtatttctctatccaaccattgagacacttgttctttggttttcctttgcaggttcttagacatctgttgtacctaatgcgcatttctgaaaagtctatccaaagacgggttgctctcgctcttgctcatctctgttcaccagaagatcagagaaccatattcatagatgaaaatggcatgtgacaacttttttgaatttattatgtttagactttgacgtgttatccattgttgttaagatgttctttgtgcaaaaagttttatatcgagtttgtcttttgacagggttggagttgctacttggtcttcttggttctacgaacactaaacagcaacttgatggcgctgcagcattgtacaaattagcaaataaatctatggcactttctccagttgaagctgctcccccttctccaacacaaagggtgagctcccgtcttacttcagtcctccaatacataacttgtggaagtctcattgcagtattctttttgtgtatttgtgacaggtttatctcggagagcagtatgtaaatagtgccacgctgtctgatgtaacttttctagtcgaaggtaatcatcatattaatcaggaagttgcagcagtcttgttcgctccaaagtccatatgtaaaccagaaaaatcatactgcaggaaggagattctatgcacacagaatttgtctcctggcatcttcagatgcatttcgcgcaatgtttgatggtggttacagagtaagttagctattatttttgggtgaccaaatccttttcaatatgttcttgcggaggaaatgaaaaaatatcatttactagctatgatgacgatgacatattggttttggctgctctgcttctctttcaaaaggaatatatggatagttatgtttcttgtgtgcaaattgaatatctcactcagtttgtgtttcgtttataccacaggaaaaggacgctagagatattgagattcctaatatcaagtgggaggtttttgagttaatgatgaggtatgacgagcttgcaggcttctttattgtgagaactcttaacatacatgtaaatatgtaattgactcacttggattgtgattcccaggtttatatacactggatccgtcgacataacaattgagatatcacaagatcttctaagagcagcggatcagtatctattggaggggctaaagcggctctgtgaatacacaattgctcaggtgagccagaatacttgcaatttcaagtgatgtggtttgcataataattgtcgaaatctaacacagttttgcttataaatgaaaggatataacgttggaaaacataggaggcatgtacgatctctcagaagcattccacgcaatgtcgctgaggcaagcttgtatcctgttcatcctggagcatttcgataaactgagcacaatgcatgggtaatataaataagctctgtctctctctctctctctttttttttcagactatctctctatttggcatttatctgaaacagagcgaatgaaaaatggcaggcaaaaccagctggtacagcgaacaataccagagataagagagtacttttgtagagctctaacaaagtctactacaaacctgcaaggcctgaggctgtaagaagaagaagactggtacctaactagggaggtaagtagacaaggaatatcatatagagagagaaagctcggtattagtaagaggtctttatggtcttgtcctatcctgagtcgttttagcaaatttgctgtgcgtttggttcattgtattttgtatcaaattctcttctggtcacaatcgcgtcttaaaaagagatcgccactttgtatccaaaacaccattatggtgaaacttcctctattcaattcaagatccacggaccacggtccaacgatcctgtgttagaagaaaatatacactgtgatgatggaatatggtagtgacaaatcagttcttgactaaatgattaatcagagaggaaaaataataatatttgttaatttttaatattatttgaggaaccgacgacatatacagtaataatatcccgttttggctttacaactaaataattgaaagaaatggcttgccattaggttattataaaatagcaactctaatatttttggagtttctgccggcagatatattttttttattatttcagaatgatagaaaatgaaaggtatataattataaataattttttttgaatatactcaaagaaaaaaataaaataaatcaaaatgttctcttacaaacaccaaattacaagcaccaaaagaagaaagaaaaaaattacaagtaccaaagtgaatgctttaatgctttatggtcacgacgtataattattattttatatattctttttgcctgaatgcttttttttatgattcagcgggaggggagatttaatttaaaggagctccggtgagaaaccctagcaccctctcatttcgagattcagccactgctcatcgctcaggtacgcttttgcttttgatctcctcagattttcgcgattagatgcgtcttctggaaactatccactatgcaatgcgatctccgatctttttacaatcactcttcgtaatctcctctgttatagatttatgcaaagtagtgatttattttatttattattagattcgaatctgatgatccttcaatcaaagccttctgctcgctacagtgtgatttttattgacaaaatcattcctttcgtctcaaagtaatagtctttgtacaaccatagagcctcctcctctgattcttgaatgtgtgtgtttgtgcagtgatggctgatatacttgattcccgacctcacacattctccatcaaactctggccaccgagtctacccacaaggcaagctctcatcgagcgcatgaccaacaacctctcttccaaaaccattttcaccgacaagtttggcagcttaaccaaagaccaggccatggagaacgccaagaggatcgaggacgttgctttctccaccgctaacctacagttcgagagggagcctgacggtgacggcggctcagctgtgcagctctacgccaaagaatgcagtaagatgattttagaagtcctcaagaaaggccctgtttgtaaggctgaacaagtatcttctgcttctccttgtaaggaaactgttttcgatatttcgaaagacaaaagagcttttattgaggccgaggaggctgaggagcttctcaaaccgttgaaggagcctgggaatgtttacactaagatatgctttagcaataggagtttcgggttaggagctgcacgtgtcgctgagcctatcttggcctctctgaaagaccagcttaaggttgttgacttgtcggacttcgtcgctgggagacctgaggttgaagctcttgaggttatgaatatattctctagtgccctggaaggtagtgttctctcgtctctcaacttatcagacaacgcgttgggtgagaagggtgttagagcgttcgggacgctcttgaaatctctgagctctttggaggagctttatctgatgaacgatggtatctctaaagaagctgcgcaagctgtctccgagttgattccttcaacggagaagttgagggtcttgcattttcataacaacatgactggagatgaaggagcggttgcgatctcagaggttgtgaagcgttcaccgctgctggagaatttcagatgttcttcaacaagagttggtgaaggaggaggtattgctttgtcggaagcgcttgagaattgtactcttatggagaaactcgatctgagggataatatgtttggcacagaagctggagtttctctgagcaagactctttcaaggttcaaacatttggctgaggtttacttgagttatctaaacttagaggacgaaggtgccatagccatagcaaacgctctcaaggactctgctgcgcccattgaggttcttgaaatggcgggaaatgacataacggttgaagccgcttcagctattgcggcctgtgtagaggcgaaacaggatctgaacaagttgaatttgtctgagaatgagctgaaagatgaggggtgtctccagattgcaaagagtgtggaagaggagcatttgaaactgcaatacattgacatgagcaacaattacataagaagagctggagcacgggccttggctcaggttgttgttaagaaagaaggtttcaagttgttgaacatcgatgggaatatcatatcagaggaaggcattgaggaagttaaagagatattaaagaaaacaccggaggtacttggagcactggacgataatgatcctgatggagaagaagaggaagaagatgatgaggaagatgaagagaaggaaggtgaagagaataatgagttggaatcaaagctgaagaagcttgaagttaatgaggatgattga

SEQ ID NO: 164 - protein, 729 aa, Brassica oleracea
MKISKSLKIHRRISSSSAISDHPPMEENHHKRQRTARVVAGRTSKRKLGRETYAVSIITQITEIEEEETDLAVAIRRHVEVLNSSFSDAGDVKGAAAALSSLAKTDENVEMMVENGAIPALVRNLESPWSLAISGNVPKSCDHKLEKDCAVSLGLIAANQPGYQQLIVDAGVIAPTVKLLKRRGVCIGCMEANAVLRRAADIVTNIAHDNPRIKTNIRVEGGIAPLVELLDFPDVKVQRAAAGALRTVSFRNDENKNQIVELNALPTLVLMLQSEDPSVHGESIGAIGNLVHSSPDIKKEVIRAGALQPVIRLLSSTCLETQREAALLIGQFAAPDSDCKVHIAQRGAITPLIKMLESSDEQVTEMAAFALGRLAQDTHNQAGIGQRGGIISLLNLLDVKTGSVQHNAAFALYGLADNEENVADFIKTGGIQKLQDDNFTVQPTRDCVVRTLKRLENKIQGPVLNQLLYLMKTTEKNIQMRIALALAHLCDPKDGKLIFIDNSGIEFLLEPLYISSMKQQKYSARALFELATKATSFAPEDSAPSSPTQRAFLGEEFVNNPTLSDVTFLIDGKQFFAHKICLVASSDIFRAMFDGLYKERNAQNVEIPNISWEVFELMMRFIYTGKINITKYLAQELLVAADQYLLDGLKRLCEYTIAQDICVENIPFMYDLADTFNASALRRACTLFVLEHYTKLSSELWFPMFIKKIIPEIKSYITDILGRPVQASS

SEQ ID NO: 165 - protein, 1267 aa, Brassica oleracea
MEQQQPERREGRSFPERKGQKRKLEEGAAAAAEDREISASTTTDGGGDAILNEIAAQVSVLNSAFSWQESDRAAAKRATQVLAELAKNAEDLVNVIVDGGAVPALMTHLQAPPYIDGDLAQKPFEHEVEKGSAFALGLLAIKPEYQKLIVDKGALPHLVNLLKRSKDGSTSRAVNSVIRRAADAITNLAHENSSIKTRVSRLEGGIPPLVDLLEFSDSKVQRAAAGALRTLAFKNDDNKNQIVDCSALPTLILMLGSEDAAIHYEAVGVIGNLVHSSPNIKKEVLSAGALQPVIGLLSSCCPESQREAALLLGQFASTDSDCKVHIVQRGAVRPLIEMLQSPDVQLKEMSAFALGRLAQDSHNQAGIAHSGGLGPLLKLLDSRNGSLQHNAAFALYGLADNEDNVSDFIRVGGIQKLQDGEFIVQATKDCVSKTLKRLEEKIHGRVLRHLLYLMRISEKSIQRRVALALAHLWLELLLGLLGSTNTKQQLDGAAALYKLANKSMALSPVEAAPPSPTQRVYLGEQYVNSATLSDVTFLVEGRRFYAHRICLLASSDAFRAMFDGGYREKDARDIEIPNIKWEVFELMMRFIYTGSVDITIEISQDLLRAADQYLLEGLKRLCEYTIAQDITLENIGGMYDLSEAFHAMSLRQACILFILEHFDKLSTMHGQNQLVQRTIPEIREYFCRALTKSTTNLQGLRLFSRLDASSGNYPLCNAISDLFTITLLMADILDSRPHTFSIKLWPPSLPTRQALIERMTNNLSSKTIFTDKFGSLTKDQAMENAKRIEDVAFSTANLQFEREPDGDGGSAVQLYAKECSKMILEVLKKGPVCKAEQVSSASPCKETVFDISKDKRAFIEAEEAEELLKPLKEPGNVYTKICFSNRSFGLGAARVAEPILASLKDQLKVVDLSDFVAGRPEVEALEVMNIFSSALEGSVLSSLNLSDNALGEKGVRAFGTLLKSLSSLEELYLMNDGISKEAAQAVSELIPSTEKLRVLHFHNNMTGDEGAVAISEVVKRSPLLENFRCSSTRVGEGGGIALSEALENCTLMEKLDLRDNMFGTEAGVSLSKTLSRFKHLAEVYLSYLNLEDEGAIAIANALKDSAAPIEVLEMAGNDITVEAASAIAACVEAKQDLNKLNLSENELKDEGCLQIAKSVEEEHLKLQYIDMSNNYIRRAGARALAQVVVKKEGFKLLNIDGNIISEEGIEEVKEILKKTPEVLGALDDNDPDGEEEEEDDEEDEEKEGEENNELESKLKKLEVNEDD

SEQ ID NO: 166 - DNA, 12836 bp, Brassica carinata
  source 1..12836: mol_type = genomic DNA
atggagcaacaacgagaaagccggagctttccagagcgcaagggacagaagaggaaacttgaggaaggaccacccgccgccgcagaggatccacagatctctccctcaaccaccaccgacgctgcgcttctcagcgaagtcgctgctcaagtctccgttctaaactccgccttctcctggaaagaatccgatcgcgccgccgcaaagcgcgcagctcaagtcctcggtgaacatcagtctcgactctcctatctcgcttcagttttcatatcttttagtgaaccttcgatgttcaagcagaggatttggtgaacgtgattgtcgacggaggtgctgttcctgctctcacggcgcatctacagcccccgccgtgcagcgacggagacttagctcacaagccgttcgaacacgaggtcgaaaaaggaagcgcctttgcgcttggtcttctcgcaattaaggttttggtcccaagtttagttttttaaaggcaacttttggtaataaagtttctatttttaattaccgaggggactatgtgatcacgttgtgggattgactgcttttacagccagagtaccagaacctgatagtagacaaaggcgctttacctcatctcgtgagtctcttgaagagaaacaaagagggccccacttctcgtgctgttaatagtgttgttagaagagccatcaccaatctagctcatgagaacagcagcatcaagactcgtgtcaggtcagcttatttatttaagtgatttaagatttgttttcagtgcaactctcctcgtgactgttcagttgttgacaaagcaggttagaaggcggtattccacctctcgtggagttgcttgagtattctgattccaaggttcagcgagcagcggcagggcgttgagataacaagaacctggtagaaattgctatctttcagcttctacttagattttggacggagcgtgttttgattgcctacttttgcagatagttgaatgcaatgctcttcccacgctcattctaatgctaggatcagaggatgctgctatacattacgaagcggtttggattcttttactgcgtcgagagttttcataatcaactgttttaccacttatctgagtcatgcttatacgttggagttataggcaatctagtacattcgtctccaaacattaaaaaagaggttatttcttctggggcgttgcaacctgtcattggtcttctcaggtgtgtggaaactcgccattttaatttacatggttaagcatttagttgttactgttaaccttagggtcattcttgttgtttattgaatttgtctctttcagctcctgttgccctgagagtcaaagagaggccgctttattacttggacagtttgcctctactgattctgattgtaaggtactatttcatctctatcctcagttcgtttgctatccaccaaagcataaactctttctgtttggctgtactaggtgtaagctgtttgtttctgttgattttcaggttcacattgttcaaaggggtgctgttcgtcctttgattgaaatgcttcagtcaccgtatgttcagttgaaggagatgtcggcctttgcactgggaagattggcccaggttcctcttttaagcctttgttagtttgagcgctgtaaaattgtaacttcgctctttaggctagttgtattaaaattacaaaactgtttatgtcttttaattttctagcatactctttcttgcaggattcccacaatcaagccggtatagctcatagtggtggtttagaacctttattgaagcttctcagttcaagaaatggatccttgcaacacaatgctgcattcgctctttatggccttgccgataatgaggtgcgttgaatgctgctaccttccgtataaattatacattaggatgcaaaaaattttaggtggtgaaccttattaaattggttattgatccccatttttctccccgtaggataatgtgtcgggttttatcagggtgggaggtgtccaaaagctacaggatgaagagtttattgttcaagtatgtgaatcatatcgtcatttttcttatattggctatatactgaatttcttagcagctttatttgtatttgttttactctctcgttggatgtttctaatgtacaatgtttgttaggcaactaaagattgtgtctccaaaacattgaagaggttggaggagaagattcatggaagagtaagtaaaattatacctgtctttaaacttgttacttccatctctggtgattaaaacatacacaaatgcgcggattgtagtaaaactgatgtattggtctagtgtctgaaactttgtttaagtttagtatttctctatggaacctttgaaacttatgtgctttggatttcctttgtaggttctaaggcatctgttgtacctaatgcgcatttctgaaaagtctatccaaagacgggtcgctctcgctcttgctcatttctgttcaccggaagaccagagaaccatattcatagatgagaaaggcatgtgacagcgtttctgaatttattatgttaagacttttaacgtattaaccattaagtttagatgttctttctgcaattttttttatattgagctgtcttttgacagggttggagttgctacttggtcttcttggttctacaaacactaagcagcaactcgatggtactgcagcattgtacagattagcaaataaatccatggcactttctccagttgatgctgctcctcgttccccaacacaaagggtgagtcaccttcttgcttcagttctccattacgtaagttgtggaagtctcagtgcatcattctgtttatctttttgtgacaggtttatctcggagagcaatatgtaaatagtgcaacgctgtctgatgtaacttttctagtcgaaggtaatcatattactcagaaaattgcagcagtcttgttagctccaaacaccatatgtaaaacagaaaagatcatactgcaggaaggagattctatgcacacagaatttatctgctgggttcttcagatgcatttcgcgcaatgtttgatggtggttacagagtaagtgaactattatgttctttttgaaaaacatctactagctttaatgactattatctatgaagctttgcttctctgtcaaaggaatacatggataattatgtaaacatgtctcattcagtttgtgcttcgtttataccacaggaaaaagacgctagagatattgagattccgaatattaaatgggaggtttttgagttaatgatgaggtatgacgagtttctacaagcttctagaatgagaactttcgtcatatacatgtaactaactcacacttgaactgtgatcttcaggtttatatacactggatcagtcgacataacaattgagatatcacaagatcgtctgagagcagcggatcagtatctcttggaaggcctaaagcgactctgtgaatacacaattgctcaggtgaggccgactaattgcaatgaaaagtgatgtggtttgcataataattaacatttgtttatggatgaaaggatataacgttggaaaacatagaaagcatgtatgatctctcggaagcattccatgcgttgtcgctgaggcaagcttgtatcttgttcatcctggagcatttcgaaaaactgagttcaatgcatgggtaatatgaagtacctctctcttactctcagtctttggcctatatatctgaaacatagtggatgaaaaatgcaggcagaacgagctggtgcagcgaacaataccagagataagagagtacttctgtagagctctaacaaaatctactacaaacctgcaaagcctgaggttgtagaatgtggaggaagaagaaggctgcacctaactagagaggcaagtagacaaggactatctatatagagagagagagccgctattagagttggtctttaccatcctgtcctatcttgatttgttttagtaattttctgtgcgtttggttcagtcttagccattgtattgtattattaatctcttctgataacagtcggtcttcaaagaaagcgccacttttgtatccaaaacaccatattatggtgaaacttccattattcaatccactgtccaacaatcctgtgtcagaagcaaatatacttttgtgtaggtttgttgacctgtcgatgatgagatatgtatattggtggtgactaatgacttattttctgatgactaatcatataatcacaagtgagaaaaatgaatattattgagactcgaatttataatcataagtgatttaatccccaaagtaaacgctctcaaggagtctgcttcccccattaaagctcttgagatggcagcaggtaatgacataacagttgaagcagcttcagctctcacagcttgtgtaaaagcgaaacaagatctgaacaagtttaacttgtctgcgaatgagctgaaagatgaggaatgtgtccgacttcagttagttcttctgttctaaacccatttcattcaatagtgatggagtgtgtaaatgtaataatactcatgtgtcatgtctctcccacttgctcatacatactttccagaaacatgttaaattgtttgtggaataagatcaatatcagtgaagcaatgctactgaagaaagaagatacccaaaaaattgcatttgatagataaaaagcttatcttaatgtattaattaactgagaaaacaaagcaaagaactttcaataatccaaatccctcaagcaaaacaacaatactaaaaacagagttgcagaaatcaaaacctcaaatttcaatttcacacaacaataaaacatcaacatcagatcctcctaccctcctggtagtagcagtgacagtcttcatcgcactaacatcaacattcaaaggaagcggaggcttcttgttctccttcttcatgctcctcagagaatacctcggcgccgtcgtctcaaccatcgtcgtcttcttcttaaccgttcctctcctcttagtcgtcataggctcgactccgagattgtaaggagttcctttcaccacagaatcatctcctcctttcttcctcctcagcctctcgttcctcctggcggaatactcatcgtagaacctccctctctcgaacaccggagacacctccgagttcgcagccatgtgctccagactcgaggctctggatttcacttcttcttgagcgaactctttctccaccatcttcgccatcgcgtggatctcgcttgagatcgatgagtactcgatcgggagcttcgactccagatccggcttctggagcttcgcgagttctggtggtgttcggagaatcgatgatgaagaggagtttgagaggacttggcgtgatcggagacggaggggggatttgggaagcggtggtttcaggtaagaagttctcatcctcgacatcgtctttgtttgaacacgagagtttcaaagagacagacagggaagtgagagattttgtctgatttattatcctttttggaggagcgctccctaacggttatatttgtcttgatccgacggctaagattgctccaaaattcaaattggaaaaaaaaaaaaaaatccgggtctatttatgttgaagcgtttttgtaacattaagcattaattagataacttaccttgttgtgaggattcgccttgaattaaagataaaagtttaggaatgttaaaatatatggttaccaagaaggcaagaagactagactactagataaaatctaggtgactttaagtctttcatcttgtgaatgaatctgttgaagagaaataaatatggtcttatcgttatatggattttgatattaaaactagagctgacatttctatgtaaattttcaaggttctaaaaatcggtataagcaaatcgtctacctaagcggcaactcggttaaaacccaatttctactaatttaaattggtttaaatcgatctaaatttatctaaatatgttaattaagcaataatactattataaatctacaaatttatctttttctgttttgtatattgaattttgataattcatcatactaattttataattaaacataaaaagtaaaatatggcatataaatctataatatatatcaaatatatcaataatttgctaatgcctaggcttcaactatatccctaataatccatctagtcgatagtcctctataaagtttcagctgagtcaaacacataagttgacaataagagtcttcgatgttatccacattttcattcttggacagtttgactcagctgaaacttattgcaatgtcatattaataataatatttttattttttattttttatcttttactttgaaaatataatataacttgacaatattttgtttccttttataaaagatatcaaatttgaaataacataatctagggggtgaacccaagaataagtctattttaaatgcgttttgcatgttaatatcatataatctttcatcttccgtaggttcttaattattctttcttacagctctgtaacttgtctgcttcttctgtttgtccatgtggtcttacctctctctctctctttgtatataaattctcatcattaccttctaactcttcacttctctctctctctctctctctctctctctctctctcaacgtccgttacgtttgtaccatcatggtatcagaggaaacatcgacaatggcggatgctaacatgcttttcatgatggagtcgccactgtcaggacctcgcatttccttctccgccgacttgtcatcatcagacagcgagggagattacatctgcatcaacccgaagaatctcttaccgggaaaacaagaacaagacaagagctcatcaaaagccggagactttgagtttctatcgaatactcaaacaatgctcaccgccgacgagttgttctccgaaggaaagtttcttcctttccggcacgtcaagcattcagagaagcttcaaaacgttacattgaaaacaaaagccgaagaacaagaacaagaacaagaaaagaagacggtgaagtagtgaaagaggagactgttaataacagcaacagaggaagctggtttcttgacgacgacccttctcctcgtccaccaaagtgcactgtgctgtggaaagagcttttgcggctaaagaaacagaggaacaacgcgaaggcatcgtctctctcgccgtcgtcttcttcgagctcgacttcgtcttcttccagctcgatcggggacgcggtgaagaaggaggagagagagagaggtaagaaagggttagagaggacgagatctctgactatgaggataagaccaatgattcatgttccaccttccaagcctcctctgtttcctctttcctctaaggcttcacaaaaacaaagtagagagacgaacttgatgatggaaattgtattgtgattagatggattgtgtgttttgttgagcttttgtgattgagatctgatgtgtgttgacattgtataaatgtgaatgacattttcataccctaacacaataaaatattcatcattaaataaactcattagtatgattttcgtctcattatattgaaagtgtttgtcttgttgtatttctgtctgtttgtatctaagccaaagatcaaatattttgggttagactcttgatgtttgttagtttaggggttaagatgtgagaaagtgagagatagacaaaagagttaaatgcaaaaactaatggaaaaaaaggcaatacaggagagtacagtgatgtgcagatgttttgttgtttagatcctttttctctcaagcaagaatccaccaagtgactctgctcaacttttataagtacatggttcactcttctgaaactctagcctcacgttttaaaaccaaaaaccatactaatccctatacatcatttcataatatccaattcagtttgatcatttatgacttccaattattatatatcgctgctgggctgtgttctatcatttcacaacgatatagagatacaacaaagaatggattacaaaacttaaggatataagtaacttacctaataagtgtgcatgtaagtcacaagtactgaagaagtgtgcatattaaacagttcaagatgagctgatataacttcgataggatatggttttgtgacttacctaagatcagatatatgtttagtaacatcaatggtcttccaagactaaagtaacgtagtagcaacatgcatgtcgatataccataaagacgaattagtggcatgtctatattcttaatcatggcactaattcgtctttgatctaatttaagattatacaactacatacggctgaagattgatatagtacttactgttttttttttgtcatagtggtatgtctcattacgccaatgtggcttgccatgtttatataactttttaaaatacatgttattcatagaaacatgaatattacttgtgtgaataataacaacattgcaagtaacatgtatataccagctagcagcacatacatcactacatagaaatgcttcctttctccctcttaaattgaagaactcatatatagtcatatactcatgtcattttgatattttattcaacactttcaaacacgtctcactttgtggcagaccccattcagtccaaaagccttctacttgtttcttttcttataaaataatcacaaaaccatattaataaagaaaatgaaatttagcaaaagtgcacacacaacctagactacctagtttccttttcgtcctgggaatgtgattatctttccgatacacaggcgtagtttagcacatactcatttccggtatcgagcgcaaattagcttcatgcggcaagaaaacattcaaaattacacatgagtaaatacccaaagcaccctgttctctattctgccttgattgatttcaaaaacgcttcttcttcttcttcttcgcatcgtctttctctcacgaacttggtgtacgatggagcaacaacgagaaagccggagctttccagagcgcaagggacagaagaggaaacttgaggaaggaccacccgccgccgcagaggatccacagatctctccctcaaccaccaccgacgctgcgcttctcagcgaagtcgctgctcaagtctccgttctaaactccgccttctcctggaaagaatccgatcgcgccgccgcaaagcgcgcagctcaagtcctcggtgaacatcagtctcgactctcctatctcgcttcagttttcatatcttttagtgaaccttcgatgttcaagcagaggatttggtgaacgtgattgtcgacggaggtgctgttcctgctcacggcgcatctacagcccccgccgtgcagcgacggagacttagctcacaagccgttcgaacacgaggtcgaaaaggaagcgcctttgcgcttggtcttctcgcaattaaggttttggtcccaagtttagtttttaaaggcaacttttggtaataaagtttctatttttaattaccgagggactatgtgatcacgttgtgggattgactgcttttacagccagagtaccagaacctgatagtagacaaaggcgctttacctcatctcgtgagtctcttgaagagaaacaaagagggccccacttctcgtgctgttaatagtgttgttagaagagccatcaccaatctagctcatgagaacagcagcatcaagactcgtgtcaggtcagcttatttatttaagtgatttaagatttgttttcagtgcaactctcctcgtgactgttcagttgttgacaaagcaggttagaaggcggtattccacctctcgtggagttgcttgagtattctgattccaaggttcagcgagcagcggcaggggcgttgagataacaagaacctggtagaaattgctatctttcagcttctacttagatttttggacggagcgtgttttgattgcctacttttgcagatagttgaatgcaatgctcttcccacgctcattctaatgctaggatcagaggatgctgctatacattacgaagcggtttggattcttttactgcgtcgagagttttcataatcaactgttttaccacttatctgagtcatgcttatacgttggagttataggcaatctagtacattcgtctccaaacattaaaaaagaggttatttcttctggggcgttgcaacctgtcattggtcttctcaggtgtgtggaaactcgccattttaatttacatggttaagcatttagttgttactgttaaccttagggtcattcttgttgtttattgaatttgtctctttcagctcctgttgccctgagagtcaaagagaggccgctttattacttggacagtttgcctctactgattctgattgtaaggtactatttcatctctatcctcagttcgtttgctatccaccaaagcataaactctttctgtttggctgtactaggtgtaagctgtttgtttctgttgattttcaggttcacattgttcaaaggggtgctgttcgtcctttgattgaaatgcttcagtcaccgtatgttcagttgaaggagatgtcggcctttgcactgggaagattggcccaggttcctcttttaagcctttgttagtttgagcgctgtaaaattgtaacttcgctctttaggctagttgtattaaaattacaaaactgtttatgtcttttaattttctagcatactctttcttgcaggattcccacaatcaagccggtatagctcatagtggtggtttagaacctttattgaagcttctcagttcaagaaatggatccttgcaacacaatgctgcattcgctctttatggccttgccgataatgaggtgcgttgaatgctgctaccttccgtataaattatacattaggatgcaaaaaattttaggtggtgaaccttattaaattggttattgatccccatttttctccccgtaggataatgtgtcgggttttatcagggtgggaggtgtccaaaagctacaggatgaagagtttattgttcaagtatgtgaatcatatcgtcatttttcttatattggctatatactgaatttcttagcagctttatttgtatttgttttactctctcgttggatgtttctaatgtacaatgtttgttaggcaactaaagattgtgtctccaaaacattgaagaggttggaggagaagattcatggaagagtaagtaaaattatacctgtctttaaacttgttacttccatctctggtgattaaaacatacacaaatgcgcggattgtagtaaaactgatgtattggtctagtgtctgaaactttgtttaagtttagtatttctctatggaacctttgaaacttatgtgctttggatttcctttgtaggttctaaggcatctgttgtacctaatgcgcatttctgaaaagtctatccaaagacgggtcgctctcgctcttgctcatttctgttcaccggaagaccagagaaccatattcatagatgagaaaggcatgtgacagcgtttctgaatttattatgttaagacttttaacgtattaaccattaagtttagatgttctttctgcaattttttatattgagctgtcttttgacagggttggagttgctacttggtcttcttggttctacaaacactaagcagcaactcgatggtactgcagcattgtacagattagcaaataaatccatggcactttctccagttgatgctgctcctcgttccccaacacaaagggtgagtcaccttcttgcttcagttctccattacgtaagttgtggaagtctcagtgcatcattctgtttatcttttgtgacaggtttatctcgagagcaatatgtaaatagtgcaacgctgtctgatgtaacttttctagtcgaaggtaatcatattactcagaaaattgcagcagtcttgttagctccaaacaccatatgtaaaacagaaaagatcatactgcaggaaggagattctatgcacacagaatttatctgctgggttcttcagatgcatttcgcgcaatgtttgatggtggttacagagtaagtgaactattatgttcttttgaaaaacatctactagctttaatgactattatctatgaagctttgcttctctgtcaaaggaatacatggataattatgtaaacatgtctcattcagtttgtgcttcgtttataccacaggaaaaagacgctagagatattgagattccgaatattaaatgggaggtttttgagttaatgatgaggtatgacgagtttctacaagcttctagaatgagaactttcgtcatatacatgtaactaactcacacttgaactgtgatcttcaggtttatatacactggatcagtcgacataacaattgagatatcacaagatcgtctgagagcagcggatcagtatctcttggaaggcctaaagcgactctgtgaatacacaattgctcaggtgaggccgactaattgcaatgaaaagtgatgtggtttgcataataattaacatttgtttatggatgaaaggatataacgttggaaaacatagaaagcatgtatgatctctcggaagcattccatgcgttgtcgctgaggcaagcttgtatcttgttcatcctggagcatttcgaaaactgagttcaatgcatgggtaatatgaagtacctctcttactctcagtctttggcctatatatctgaaacatagtggatgaaaaatgcaggcagaacgagctggtgcagcgaacaataccagagataagagagtacttctgtagagctctaacaaaatctactacaaacctgcaaagcctgaggttgtag

SEQ ID NO: 167 - DNA, 41668 bp, Brassica carinata
  source 1..41668: mol_type = genomic DNA
atggagcaacaacaaccggagaggcgagaaggccgaagcttccccgagcgcaagggacagaagagaaagctcgaggaaggagcagccgcctcctcagaagatcgagagatctccaccgacggcggcggcgatgcgattctcaacgaaatcgccgctcaagtatccgttctaaactccgccttctcatggcaggaatccgatcgcgctgcggcgaaacgcgccactcaagtcctctccgagcttgctaaaaacggtgagtgatcagcttcacttttctgcggtttcttcatatttttcttgatccatgacttagtaaccaccgttgttcagcagaggatttagtgaacgtgattgttgatggaggagctgttccggctctcatgacgcatctacaggcgccgccgtacatcgacggagacgtggctcaaaggccgtttgaacacgaggttgagaagggaagcgcctttgcgcttggtctactcgcaattaaggttttgatcctcatgtgattgtatagtgtgttagcttgtttgaaaacagttgctttttatgttatttttgctccaagtctagaagtgctttgtgatctcgttttgaaattgtctgattacagccagagtatcagaagctgatagttgaccagggggctttacctcatcttgtgaatctgttgaagagaaacaaagatggttctacttcccgagctgttaatagtgttatcagaagagctgctgatgccatcaccaatcttgctcatgagaacagcagcatcaagacccgtgttaggtcagcttctttaggtgttctcctgtcaagatttgtttttcgggatctcatgacttcaagtttttgataagcaggctcgaaggcggtattccacctctcgttgatttgcttgaattctctgattcgaaggttcagcgagcagcagcaggggcattgagaacccttgcgtttaaaaacgatgataacaagaaccaggtaaatatttctgtcttacagcttctatttcggttttcggtggagcatgattctttgttttttttgtgcagattgtcgaatgcaatgctcttcccacgctcattctaatgttaggatctgaagatgctgctatacattatgaagcggttaggaatcttttactgggtcgaaagttttcataaatcaactgttttgctagttgctacttaaacagctacacgagattaacactgaaataaccagttgaatcacacttttaggttggagttataggcaatctagtacattcgtctccaaacattaaaaaggaggttctttctgctggggcgttgcaacctgtcattggtcttctcaggtgtgtggaaactccacgttttgatttacatggttaagcatagagttgttactgttaaccttaggttcattctcgtcatttcatttctcctatttgtctatttcagttcatgttgccctgagagccaaagagaggcagctttattacttggacagtttgcctcgactgattctgattgtaaggtactatttcatcccgggttttctttcctcagttcgtttgccattacccaaattctaaactctttctgtttggttatactagttgttatctatttgttgctattgattttggtagaatatacattcccaattcttgctatctatcattttccctgatttatagttgtctttttcatttttcacctcgtattcaaaaatatacattgcaggtgcacattgtgcaaaagggtgctgtccgtcctttgattgagatgcttcagtcacaggacgttcggttgaaagaaatgtcggcctttgcactgggtagattggcgcaggttgttgtttcaaacattgttattttcagtttataaagttgaggcattcctatttggcgttgtaaactggcaacttcgctctttagacttacaagagttatactaaataacattaccgttatgtatttaattttctagcgtaccctttctcacaggattctcacaaccaagctggtattgcccatagtggtggtttagaacctttattgaagcttctggattcaagaaatggatccctgcaacacaatgcggcatttgctctctatggccttgccgataatgaggtgtgttgtctgcttccttccgtatgtattaatcaggatgcaaaaatttatttaaacctcactaaatgggttattgatccatttttgtcccctaggataatgtgtccgattttatcagggtgggaggtatccagaagctacaggatggagagtttatagttcaggtatgtacagcgctgttaccctctctctactttccagaatcatatcgtcgtattccttttatcggctagatactgaagattcttagcagctttaatagtatttgttttactctttgggtgtttataatatacactgtttttaggcaactaaagattgtgtctccaaaacactgaagagattggaggagaagatttaaagaaatgcttccttcttctatcatatatcatctttgatattttattcacacttttaaacacgtctcttttgtggcagaccaccaaaaagtccaaaagcctacttacttgttttctttttctttataaatatcaaaaatattaatgagttaaccatgttgaaagaaaataaaaatctagcagcaaaagtgcacaagtacaaccttgattcctttcgtcgtgggattaatttttcaatgttccggcacactgaaagccttcagtcaaaaaaatggtcctaaaaaacatttcgaagatagagaaaacaaacaataaaaatgtagataaattacacgaattttgaaattttattttccctgaaaaaactaaaagtaaattaaaaaaagggctaattggcgtaatagccatatttcagagggaaatcaagagaatagacatgattttgacataatttactcactgttttttgtcttcattccacccggttatacccttctaagtaataggtacctggttccttcacataaagtaaataacgtggtgattttgtgtcctatagtaacaatgagagaatttaggaagcgcgtggaatgaaaatcaaaggaaggaaaatatgcagagagaaaattagatgaaaatcgtaagtgtgaaagaaacaacgttaaacaaacggagaatccaaaaatcatatttccatactatatattttagatagaatagtagaaatacaaatatagttccaattcaaagagcatctacataatatagcgacagttgaagtcaaatattgcataaataaactgatgcacttactcagtcacgctaaattggaaatagaccacaagtttacaagcatgaattgtttaagttaaagaactcgatagtataccatcttctgtttcctaaaattgtaaagaacacaaggtcacaatcagaagtttaccatcttatgtttccttaataagactggaaagaactttaatttctatttaacaactactaatacacataatagaagatacaaatttatataaggtagaattatttgatatggtaacatatccatatcatttatacagttgtacgcaaatcaaacagaacgtactggtggttgggttatacaacagaagatagaaattgagaataagaagaataaggtacaatataggtttcggcatgtgtaatagacggggacgtggaagtcgggcagcaaaaaccgaaaagttggaatgaaacagcatgttatgaaggatccattttatattagggtagattccattttacctgactaaaatagaatagcttcactgtttataatttactaatataatcacgaacaaagacggtgaagtatgcggttggggagaggcgatgatgtagttagtgcaataaatttacaattgtgggttacagctcttccgtattaaagagtaggggaaagccacataacaaggtagatttactgaagttattttaactgtggaaaggtaaacgagtggtggaaattagcaccactgatcttaaatggtgaagtgaaagcaaaccataaatggtgtattccatataataatcaatgtaatctacgtgaagacactcagaagcaacaaagtgaaggaagttaaagattcactgctttgaagcaagaaagaggtaagttcgtgtgagaatattctaataaaccgagtttcataggaaaattactcttttgtgatagaataatactattctgaatatgtaatggactaaattttgaaatataaatggatttccacttaaaactaactgcagatgaatagcgaagataaggttttactggttgttggagcttgggtcagtgacagacataaaagatgggtgttcgaaacaaaccattccctcataggtgagcactacattagcctctacagtggtatgaacatgtctgatttagttagaggagtaagagaggagatagatccaacttatgaaggagtgaaattgaaactatcttatcaatacccggaatggatttcagctgatggtggaggtcttgaaatgccacaatacataacagaagacacagaagtgggagcatccatcgaacttagacaatcaatagaggcagttaatttacttgtctcgattatcagtcccaaggcgcatgacgagggggccgcttcatatataaatgacacaatggatggacgtcacacaatggatagacgtcaccgagagagagagaggatggtgggatagaagatgatgactggcatgaatttgcgatggctgagactcctatgaccactcctgatacgaagtgttatgcaggcgcgaaggatctcaaaattcttgatgctattccagccgaaatgagtggtatagcatatacatcaagatatgctattctatttccaatacgtggagtcgaaatccgagatcccgagcataaatttcgacaacgcattcagtctgagcctgatgtagcgatgcagaaggggaagaaaaaaatgaggattgaaacaacctcgcattaacggactcgactcgatgatgatatggttatgcccgccgtaacaaccgctgatctatcgggaaaagggaagaggcctatgtgggaacgtctaatatttggcattgcaggcattccaaaccgatctgaagaagataatgatagcagacgaaccacattagtaggtcaatctaacccagcacctgaaggtctcgatatggtcaatgacccacatcttcctgacttagttgacagagagaaaccccccaacggacagtacaccaaatatcgggtagtgtgcttagattactaaatggaatagaataactgcatatatacatatatatattaccagatttggattctaattttactcactgtatccatttgtaggtggagaatttaaaatatcagatgtccatattgagggagatgagatatttgttgggggaggcttaaattcaaatatcaatttcaacacctttactgctacgacgctgtttgtgaaggtaacaattatctaagtgtatcgaatttatggactttgcctaaatatagaaaagtaaagagcttattattaatgaggagtagaacggtttggtaacattaggttatattggctccatgaagaatgctatgcaaaatagtttcaaataatatataaactaacttcatcgtggtacaaacttgcagaactcggaaacggcatcttcaatccggcggcgcatgcgttgtggcctttacgggtacaacaaggcatcttgtcggatcccaatgtaataacaacggaaccgtcagtggcatcagaagggagggtgaagcaatattttggaaactttgagacataagcgggagccattgcaatatatgcaattggcagtagaaaaaacttggacggggaactgatgcattttgttgctaaatacacacataagtgtagaaatgccatttatgagtgtatttgtgatgtagatagtaagccatatgtagaacgtgtttgttgttcggaaaaccctatgaccttctattttggttatatgaaatgatgccaatgttaccttcgataatatatatgcatttataaggtgaattaacatttacaaggtttatgacgtgattgattatattccatatatattatgttatatacatgtctattttgtgattcattatattccatacagtatatgttatgttatatacatgcgaactactattccatgtaacataaaccttgttaattatatactacctgcatagtatatcctgcatatatttaactaatataatgggagattggagacaagtatttacaatcctaatgagccagataaaacaaacggagatgatgatagaaggttgaaagttatcactaaacccaagttgggaaatattaaccctcattcatgggaggcaatatcagtcataaattacatcttcttctctgtgtataagaattcatactatgttacttggaactatgattttgtaggaaataggaatataatgggggatttgtaaattagaattgacagtaaacactaaacccaagcttgggaaatataaaccctcattcatgacaaccaataccattcataaattagaccatagtatgtgtatataataatacaaactatgttacttggaatacttttatactatcaggggacatcattgatttacatagcatataggagacaagaggaaatttaatcgtgttgttaacaaaattaaacagaagataaactgaccaataggaccatatggaatagaatacgtaacataccaaatagtatagtaatgcggactgtgtaccaatttaagaagttaaatttactaaaccaaataccgagcgaccaataggatccgttaacccgatacttgaacccgagagttacatacttattcagataccgagacaccaaaatacccaattctctaaaatcaaaatattaaccataaatcctctttcggcgtctcgaattacaacgccaggaagttcaagtaatgcatctgggcatcgagtaagcggaagtgcttctcggcgaggtgggccggatagcgggaatacccaaagatgttggtgtggaactgaaattgtatctctgatgtccaattccgaccataatccttatagaagatacttttcgatgtacatgctgcagcgaaaaaggtatattcttctgtagttatgcataagtctgactgttttggcatattgattttgatatgaataggccttaagtgacttatcttttatgttctgattgatgatgtagcttaagaatgataaccgttttcaagtggattgatgatgaggttttgttaggcgaagtcagtcgattcaattgaagattggaaaatgaagaccaactgaaggagatggcaaaaacagagagtattttggctgaaagagttcagattaaggtggaagaggtgataattgatcaggtggaacaagtattggaagaaggcaaagcgagcatgaagaaaatgatgctattaggactagtcggatgcataatattgggagtagtaatggggaaggtttattgaaaatggttggcttggtgtgtgtgtagctgtaatcccatatgaaaacctttcaatcttcatgtattttaatgttattgtaaaactaatgttgctgttatgtagtaatgatattgtagagcgttactatggtaaacaatgaaggataaatggaatacaaatctaggggatgagtaagagatcagttgtttgtgaaacttaaacccaagtttgggtattgtaaaccctaatccattggcaatccgttggaaccccacattaccttcatgtacatattaaatgagacaagttaaagtagtgcttagaatatgtctgctatgttatgtggaacaaatagaaatgaaatacagaaaaccttatgcagtcagtgatgtgtgcggttggggagcaatcattatgcgattagataaagggacattaatcggtgacagctgttccatatgatagagtatgaagaagccatgtaatgggttgcagttaccaatataatttcactgtacaaattcaaataagtggtggaagttaaaactctatccataaatggtgtgttccatttatttaccactgtaatccatcgaagaattctgaaaaacaagaagctgaatgaagcagtagttaatctttgagaggaacatgtgtgaagtaaaatccacatgccatactattaggaacatgtatgtatattgctcatgaccaacatgaaatacaaagtcaatgagattggtaataaaacatttgatcgtaaatactaaaccaagttaggaaaatataaaccccgatacatagggaacccaaatcttctggaaatagaaactgcatgagcacattgaatatgcactggtaaatgtatgtacaatctaatgcgattatgttattccatataattgtgctatctatatattattgtaaatgttccattccatgtaccatatattatgttatttggatacaaatctaatggggagtggtacatgatattaaacacctaacacaaattgatagcgtctagtacatatgaaagagtaggaggatgcccgtccacctcattaacaaagatattttccccttaaatttaaacaatgagtataaggtaatgattaccaaaggcctatgtgtatacggttcgaagactttattccatgggaacagtactatttaaaatgtaagcatgtgtatagtaaatcaagaattgagcttcaaagataatacacaagatattatataaaagataatacacaataaacaacctagttaggaaaatataaacttacaaaccgagaacccaattccaaatctagcagcaagggactgcaaagcatagtatttccattccatatacactgaatgaaatgaaatagagaaccactaaattgatctactagtgttatctagaagcggcgtgtgtggtagaagaggtgacggcatgcaatggaataaatggctatcagttgtttacaccattccatttgagagaatagggaaaaacacgtattgagttggagttaccaagatattttccttgtatacattcaaacaagtggctcacgttaaaacattttatccataaaaggtttattccatttattactactgtaactccatctcaacaattccaaaaagaaggtgaatgaaggagcgtagttaatgggaagaaacaaccaggtaacttgtcctcagaatcttgtaattaatggggtttcagatgaaacaagcactcagacctgtaattaatgatgttttcagataaagcttgtttgttagaataacatcatgtagatagtgtaatggaatagctattcacatatagtaattatctgtaacttattactgcagatggcgagtcaagatagagttttactggttgtcggttgtgggtccgtgaccaatacgagcaatgggtttcgaacggacatatgtaaccaacttcgagacacatccgactctataccggggatgacattgtgagttagttacagccgttaagggcgacttcaagtaacaactaaagggtggcgctgaaactatcttaccaataccggagtgggtttcattcggcgatcctgagctgagtctgcctcaatacataacagatgacatagaactgcggggattcatcgagatgagaagagccatagaggaggttaatctgtttgtctcgttagttagccacacgctgcgggactaccattggcgggaccgcagctgatataaatccaaaatggcagcattgaatcacacaatgggcgaatcatggcatgactttgcctatcagagacccactgacatttcctcgaaacacagccgaatgcaaacaaaatgtcatagaagtccggatggttctatttccgtcaaccagatggaatggacaaaattggaggtcgtgctattccattctttacaggtggaatagaaatcgagaaacctaaccacatagtcttagaagtccgtatgcagctacggacaagggaagaacaaaatgcctatggattcatccacgagacagactcagatgatgatatggtggtccctgtcttgcaagcggcggttgatatagcacgagggcgaacatgccagtgtgtaggcgttttatttgggattccagacccagttcaagaccaatgatagcccagcaagttcaggcgaaggtgaagagttgccacctgatggcgaatacggggaagatttgatcaagctactacgacatgctgagcgacccatataatccggctctgcttggtgggatgctcctccggttttcagcccagaatcaggtgacttagaacctcgttgtccattattattaaaatagtatggaaaatatatactaaatatagtatatcgtataactaactcataacttcaccttgtaccaatataggtgtcgagtcgctgctagctgatgttcattctgagggagatgagatatttgttggcagtcttcaagtctaaagcggactgcaaaataaagctagccatacatgcaataaacagaaagttccatttcaagaccacccgatctatcgtccctgcttgtgattgaatgtgttgggaatcatgtccatggtgcgtttatcgatgctattagatgctactggtaacttccaggtccgacaagctagtctaactcaccgtgcactgttggcgagcgcggaactttcacaaatagccaaacaagtcataggagagattacaatcgctttgttggaattaagaaaggacccgactgcagttataagaaaaatactgcttgatgaattccatgtgaatgtatcatattggaaagcttggcgcaaagggaactagccatggaacaggcaatggggacaatggcgagggctactcactgattcctgcatatctgggacttcgcaagcctcaagcgaaggaccctttgctttatcgagcaaaagcgatgactcagaagggggaccgctttaaatactgctttgttgcatatggagcttctgtagcagaggtgcgcctacatgaggaaagtatgcgtcgttggcggcacttcaatgaaagtatggtggatgcctcttatcgcagtggcacaaggcggaaattttcaaatatttcggctgcttgcagttgttgacagcgaaaatgataatgcgtgggagtggttttcagaagctcagcacatttgtcgcggactgcccaacttcgtctttatctcggacagacatgctatatatacacaggcctgcgtaaggtaaaaattacaaacaaaaccactatatacttgcattatattttttctatgtattaaatggtatagcaacatgttgcgtaagtgtacaaagcacacgcatggcgtgtgtggtccatctttggtgcaatattcaagtcctcataaggcagacttggaaacctaatgtctgctgcagctttcgggcattcactatccgcgaatttaataggctgttcatacagatccgagaattaacctgcatgtgctgcatatcttgtggatataggtttgtactattatattttctattatatgttataccatttatagtagtgatatatagatttctattccatttccatatgcatttgacaccatggcttcataacagggtttgagcacggacaagagcacatttcaggtcaagatacaatataatggactctacatggctgagtcatggaatggccattaaggaggcaagagacccactgatcatgatgctcggtatatacgttacaagcgtgatggggtggttagcgttgcggccataaaactaacaaagaaggaccttgacaccaagcgtcgtaaacttgttgaagaaaactatgacctatctactgccttagctgtgtgacataagtgagctagagttccagtacaagacccaacggagagtgtttcactgttaacttagcgttgggagctgttaggtgtagagagtatagcaattggaatccctgtccccatgctctggctgcgggatcgaaggttcgcgttctcatcaggcaaatggttgcaccagcgtttgggtcccaacatggagacaaggatttgctggaaaaatttacccagttccttcagttggtgggtgcttaagtaggttcttctaccacagccgagctccttctccctgcagtccatgagccatgtggcagtccaaggaaggttaagcataaagtctgtggagagttcaaggtaacatactccataatgaaatatcttagatttggttatgaaggatatcatagtgaaagtggaataggttatgaatgctaaatgatggaatggtatttcaatgtggttcacatagaatggatactaactaccttataaaataacttgcagaagtcagggcaatcatcatcaaacagcgaaatcgcccgttgtggcggactaggcacagggcatcttaccatctatataaaaagtaagcggagccgaatggcatcgaggcagtagaagcaatattttgggaaatgggtaatataagcaaaagccattgtcatctacggacttggctattatataatctgcaatggggagatgttggttttgctcacaaatacacaaatatatgcactcggtgacatatatgggtgtattgtgatattataatatgtcatatataacccttaagcacaaacaatgtgtgttgttgtaatgaagacccatatgccttctattttctgtaatataaaatgattgttggggtcaaaatgggtcaatagccaatcgtcaccgaaagtcctcgaaagaaagccagcggcgatcaaattcaagcggtgaagtcgctcgatagctccgcggaaggcttcgtccactcccatctgggccagcggcggggttctggcccatcaatgcgatcgtctcgcgatctcgggcaatgacagcatcctggtccttgaaatccatgtctggattgtccgagatctacatgagtcttcagtaaaactttcgattgtttaaagattcatcttttaacatataaaacttcgaaccatattgctctcatcccgacgacggaaaatctgaagatctaagtccatctcaaaatccgataccggaatcgttggaaacaattatcaccgagatctacgactagagaccctcccaacttcgaaagatttccgcaaacaagcgtgagggaaagatcgaacaaacccacaggacggcaggcggcctggcaccaaccgcagcggggccttgagctaagcggcgacaccggctggcgccggtgcggcagcaggacccagccagctggcctgcggcggcacccgacctggcgccggcaccagcggagccaggctggcctagcgaccagcaccgacctggcgcccggcgacagcagagacagcagactggcctagcgccagcggcaccgacctaagcgccgcggctgggagacagccaggctggcctggcgccagtgacctgtgaagacaggtcggcctggcgccagcggacagcgggcagggctggcctagcgccagcggcaccgacctggcgccaggcgtacccagcggagagccaggcttcctggcgccagcggcaccatccgcagcgggcgacctggcgcggcggcaccaaatccagcaggcgacctgcgctggcggcaccacgtcgctgagcggcctggcgcccggcggcaccgacctggcgcccggcggcaccgtccgcagcgggcggcctggcgccggcaccaacctggcgcccgtttccacgtcgtgtagatgcgactggtgtcggtcccgaccctcgtcggtctcgttctatcgtgccggttcgatcccatcttagcttgttggatcaatcacgcaagtttggtatgatcacggttattctagaagcgtcacttcctcgactaaacaaggaattgaggttcgccggaaactccgagaccttcaaagactgtcgcttcgaaaaatcataaaagcgctaagcggcccagcagccaaaagcgatacgtcgattttcgaaaggaggataactatgacggtttatctttatcctcacataagagataaatgtcaagtttccataagagataaatatcaagtttcggaagataaaagaattccagaagataaatgtcaagtttcgataaacacaaagatgggcgaaaatggaaaaagccgactcagtccagcgagatgagaccgtcataggaggagtatataaagagagcttggaacaagaagcaaacaagatcacaaagcgtcgagcacttgagcaacttagcattcttttcattttccttggcggtgcgactcaactaggatagacaagcgtcagactagcgaactaccgacagctctcgtagccaaggctcttacctgttgttcacgctcaagcggattggaataaaatcttttgctctattctttttcttacgatttttgttcgtttcatattttctttgtcgaactgattgtgtaaattaatgcgacccggccggatatcagggaccgaggcttggttcacttggctttcctccaaatcaacttaatttgtggttaatttcggttcccacagtttggctagaaggagggttacggatctatctatctccatgcgcacgctcgatcatgtcagccggcgccaccaggatcagcggggctaggcggaacaccgtcgatgccaagctgaaagactccagctggaggcggtccacagtcactgctgatgcaaacactgaagctcaagcagatgaaggaactatttacctccgtgaggcgggcggaacaacggagacaagctgataacctgcgctcgccaaaaagtcgacaccttagctgcgaggagcaagttgcgtagcggatccaccaaggcgcggcaggcggcggaaattcgacggatctcggaagcgcgagaaagatgcccgaagagcccactcagaggaagcggcaaagacagcaagcgacctcgcagaaccttccactccggctgcggaaacaaaagcggcgtcggcgcgtccgatctagatgtcagcgaccgtcggatccttccgatgaaagcgctgacatccaccagaagaaccgaagccagtccgcttcggccggtatcgccgataggcccatggcgaagagaggaagaagaactcctggatgggcaggaaagaacttcgcggaagatcaaacttcggatctatcacgaccagcgtcgacaggttgaggagaggcgcggcaatagcgagatccatgatccgtgaatctctcaaaaagaggtggctgaagtggcggtaaaatcgccagatccatcgaggaccagttccacccgagatcgatagacttccgaggaaacgcggaagacaccgttcaccactttcggatccgcgaaccgcatctcagacccaggaagatcaaaatcgatctatatgatgcagccggatctaaagtcgcacctgcagtcctagatcgcaatgggtgatgcaaactcgggcgagcggtgacggggcatgagtcattgtcttcttaaaccgagcacctccaaggtgctcgctcagtggttctcggctcaaaggaactccatgggaagcttccgccaactggcctcggcgtttctcaaacagtactccatgttcatggatagaagcgtcggcgtggatctatggagtctagctcagaaggaaggcgagtcactccagcgacttcatcgcgaaggttcaaactggtgatggccagtagcgggcatcagcgacaatgtcatgtcggcgccctgagaaaaactctctggtacaaagtcggagttcacgaagtggatactactggaaaacgcggacaatccaggatactctcccaagacaacagacttcatcatcatggaagaagagatgaagcttatcgccagaagcacggaccgcgaaaacgcgtccaagaaaccctctcgtattacgacaaatcgtccatcacgaaggggaaggcgtccaaagccgagcataacttcatgtcaacttcgggcagggcaaaacctccgggaaacctggaccaggaaccagtacaaggataactcctactgcgagttccacgagaccagagccactccctgcgaactgcaaggttctcggcccggcttcgccgccaaaactcctcaccggcgagctatcaaaggtcaagagtataaaggacttgctcctggactccgaccagcccaaagactaacaaaactacctccgaagacgccgcgaccgaaaccaatcaggggaaagcggaagaagacagggcgaccaaagggaacaacagcggtcgcccgagtaaacatgatcattggaggatcacagttctgggactctcgtctcatcgataaaagcctacaggcggcgagaccagttccaactggttcccggacagcgatgttctaaccacacaatgcgctttgaggaacaggcagtccgaatcgacaaacctcactcgcgaccctttggtatcgacctggtcatccaggatctgaagtcggcgcgttcaccgtcgatgcggaagccggtccgcgtcatcttcagcgacaccctctacaggatgaagatcccacttgggaagttgtccctgagccaaaaccgttggcggggttcgagcgtcactaccatgaccctcggaaaattaaactccgatcatggcgatggaagttacaaagatcgtcgaggagtttgcagtgatcgacaacccgacatctacagcgccatcatgggaaccccatggatcgactccatgaaggcagtaccgtgtttgttgttcggaaaaccctatgaccttctattttggttatatgaaatgatgccaatgttaccttctgataatatatgtctgttataaggtgaattaacatttacaaggtttatgacgtgattgattatattccatatatattatgttatatacatgtctattttgtgattcattatattccatacagtatatgttatgttatatacatgcgaactactattccatgtaacataaaccttgttaattatatactacctgcatagtatatcctgcatatatttaactaatataatgggagattggagacaagtatttacaatcctaatgagccagataaaacaaacggagatgatgatagaacagttgaaagttatcactaaacccaagttaggggaatgtatacccttggaaataagtaaccgaccccaaacctttttgaaattaaatacacttgtcataataggggagacatgtatttgcacacttcatgaaagtaagccatatttagaatgtatatatttagctgcaaacgtaaatgcagatatgacatatatggatgtttgttatgtagaaaataagccatatgtagaatgtgtttgttgtttggaacacccaaaaacctcctttttggagaaatgaaatgatgtcattattaacttatgataatatatgtttgtagatgggtacgaaacactttcaaagctaactgtactaatgatgctattccacttggacaaacaaggttgttttaatattttcatgttacaacaccccatgattgttaaacaagaatctctaaaatattatttgagaagtcagtttcttatgtgtcgcgttcacgttaattctcaagatggttgattacactgatacttttaatgaattacaaatattacatttaagtattattattgattttttttagttaatttcctctttaaattttccaaataatatatatatatataataaaaaggaaatatttataaagtttaaaaacgaaaatatatgtatatacattatgatttcattaaaaaggaaagttcacaaaatagaaatatttcatttaaaaatatttttcaataaacataaaataaacaataataaaatatttctttatatctatattttcttagatgaaaatatatatttgcatataatgtaatttcataaaattcagataatcttgatattagaaaaagaaatattatttcttttaaaaataattttaaacaaaacaaatatatatatatatatatatatattcaaagtaatagaaatatttttttacatatctatctattttcttagatgattacatgaaataattaattatcattaattgatatatgttttattgactaaaataagtttataattaatattactgaaatatcttatctattttttttcatatatttatttgactataatatctttcaattacaacgaaaatctataaattatagtttaattatataatatgatttttaaaatataatcacacagttcttctcaactgcttatttttaagagatattaaaaaataaaaaattaacaataaacatcttttgatcaaataattaaaaaaaaagtaaaataacataacactatatattttaacgaggtagatatattatattttatcattactaaaattattttttcataatactaaattttcttttaaatttatgtttctatgtttgtcgaacttaataagaatataattaaaataccaagcaaatctgaattctcattttaatattatttaaaacaaatttcagtttaccgtttaataaatctaaggcataaaattatttagaatctataaaataatttaattattgtaaatactgatatgtgttcataagcttccaaaaatgtattagttacttatttatgtgactttctattgatcatctctttattttctgatgttttttaaaagagatcaacatataatttggtaaatattatgaaactacatgcacatttaaacgataaataaaattaatttgattttacttaattatactaaatataattatacttcagtttgaatttgaaagaatatatgtaactcaatatactcacaacatgagtgactcgacaaatcaaacttatatctaaatcaagatttaattacaataaaaaagaataaattttataataaaatttattttataaatttaaattatagaataaatcaaaacgtattaacaaatgaaaataaaatattaaccaactgttataatttagttcttttgtaaaatttatatatttgcatgagactgtagaatattatcgttttacaaatttacgtaatttggaataagacaatctattttatttttatttcattctaagtacaatatatcttaagttatacataatcttactcaaatatatttacatatctaagacaacaaccaacgtaaatgcaaaaaaaaaccataattttaatatatttaaaataaaaatattgtagttgaatttagagaaatagatacaatctaatatacccaaatgataactaaatcaagtgtaaaaataataaaccgactaactataatatatataaaatcatacatgtatttaaagtaataatgtattactaatataaattatgcatataaattataaaataatttaaaattaaaaataaataacagtcaattattttagattatatatattataaatatttgtatccgtgcatgagcacgggaaaatcacctagttggtagtaaacgctaaacccaagtttgggaaatataaaccctcatccatgggaagcaataccaatcataaattacatcttcttatgtgtgtttaagaattcatactatgttacttgggggtatgattctgtaggaaatataaatataatgggagatttgtaaattagaattgacagtaaatgtgggaaccgaaattcacactgtcgattttagttgatttggaggaaagccaagtgaacctagccttccctgaaggtcccggttatctgctgggccacgcacgacgcaatcaatacgacggaaagataacaaaacggaatataaaaatcgtaagaaaaaagatagagcaaaagatcttatttccgaatttgcgtttaagcgtgaacaacaggaaagagatcggctacaagagctgtcgatgagttcgctagtccagccacctatatctaacctagttgagtcgcaactcgctagtaaaaacggaaaaagtgcctaagttactctaagtgctatgttgctctctaaaagttctcgtcttgctcctcgcccctagctctccttatatactcctcttaggacggtctattcctcctttgggccgattctatcatgaatcaggcttcttccgttttcgtcggtcttcatgtttatcgaaacttgacatttatcttgacatctcacagacatagtatcgttatcacgagatcccaaaacatgtctcttataaactacacctaaaagcttcgctaaaaagtagcatctggaccagcgacaaaaagagttaggatctggtgactaccgcatccttccctctacacttggcgaaagtataaatcaaaacaaaaggcgaaatctcgcaaattttcatattcataaaagccgcaaagacggcaggattcaaagccaccagcggccagtcccaaaacatgagaatgcaacctccaacggtcgcaggataaaattactaaaagcggccaccacggccggaaattcaattcatagaaggaagtcaacgttgagaaatccggatgcagaaatcccaaatgaactagcaggctggtccacttcttcattcacacctcgagcattcccaccattctcggtgttctcatcagctccgacctccaccgtatcctcggaaacctcgataggttcccatagtctccggactctttcttctacggaggaaccaaggactcagcatgagcacactcgccatgaaatccttcatttcagcgatctcgaatcgaagagaaatctgggttctgagacttgtaaagattcgaccgaacctcggcactttcaaatcaccaacaaactcctgagcttctttaaagcattgaaactcagcagcaaacgattcgccgtcttgccacctcgctgcgaccatccttcttcctctcctttcgcccgtcacgagccggcgtgaagctcagcttgccagcgttctgtgccttcacctcttgacggaaccgaaaagctctcgcccacttctgtggtcttgaagttagcaatcctggatttgcggaaacttcgagtcaagcctcgctaaacactcttagtccctgcatgaaactcaagatcagcaagcatgcttatatacggattcaaacgcaaggttaaagaagttcgaagggccaaacctcgttgacacgttgggagccctcggcaaaaacccgttgtttctcctcatcctccagcgactcatcagtagtaaactccggaggaaggccatcaaagaagttgataggtggaaaaccgccggctccatcttttcgttggaacaaaactaggttttctccccagcggtgaagggttttccgagccttccccatcatcgatttccttcccctacgagacctctgtctgcgcctcgaaggaaccacggtaacaggttggtcgtgcggcgaacagaacccggaccgataaaggttaaccgcatctcggatccgctcgagggtgaaggatttccagaaaagcggcctttgtgaagatctctcttggccagcgttaccaggcaaatcttgcggtagggttgttcctacaaagcgaaaattttgtcaaagacacgccagaaaaagtgagatagataacagaattttcgtcatattacctcggttaaagttccatgcccgctgaaatagatggaggcagctctcctcgacagacttcgccatctatttgaacagaaagcatcctgccacgatttgggattgagtagtccctgaatcacggccatatccttcttaggcagcatggaatagtaaccgtcactcccgtcggccgagtaccccaagacgccgaaatcatcgggaccaagatcaatcccaagttaagtagctagcaattagtacgccaagccaactctccaaggcaggaacgctgagttggttgatcgaaagttcaagcggtgaagcgcatctaacaatggcaccaggaattgggaaccacatacggcgataaagcttaagtaacatgtaaagaaatcttgcggaggattccttgcactctcgttaccagcggaatcaaatttgactcttcagaacctggtaaaatctcgaagaaccttgagatatttgacagaaacttcggcgcaaaaggagcacgggctgcctcgaggcctcttgaacagggatctctggcagtgtaggaggccgaacctacaagggctcgtatcgcattcctcttttcctcctcgaccgactcctctgctaccgttacatgagcaggagagtcatccgaggatgaatgggaagaagagtttctctttgaggatcttgaagacattgttcttaaagagagaaaggattcttgagagagagagtaaaaaccttgtgatgaagtaagaatgagatttcttactccatataaagaaggtaaaatcactatttacccgatttttgtgacgattacatctcaacaccttcccacggctatacgaaagagatcggctacaagagctgtcgatgagttcgctagtccagccacctatatctaacctagttgagtcgcaactcgctagtaaaaacggaaaaagtgcctaagttactctaagtgctatgttgctctctaaaagttctcgtcttgctcctcgcccctagctctccttatatactcctcttaggacggtctattcctcctttgggccgattctatcgcgaatcaggcttcttccgttttcgtcggtcttcatgtttatcaggaaacttgacatttatcttcaagaaacttgacatttatcttcgggaaacttgacatttatctctttatgtaaagataaacatgggccgtcacgtccatttcgactttatctcctggaaagttgtaagtgggccgcttggtcgagtttgggccttctaagccgttgtttcgtccgtgaacattgtacgttttcgctagagactagcctgccatggtgcttgttttgctgaaagaaccacaactcctcgtatagtctagatgactggtgttctttagaataaccgtgatcgttttatacgatgaatcaaaatccattcaaacttttgatggtcttccgaagccttcccgatttttttcgaccagaacaaaatggggttctcaggtttcatgtcttcgaggagtttgatcagtgagtcttcgagcaaagatataaaatgtagagttggactagttgtcgagacagttttgcggggagaaggtcgcacttgtcgagtaatccgtatgcgggcgcccaggacttggacatggacgctggcgccggcgtgattccttcgctcgtttcgggttagctgcgggggcgttctgatcttttcgcagtttgaactcggctagatagcagagtctcgatcgcttcgactcccgacatctacggttccggttgagtcgggaatttgatgccgaggtgatatgtggacggtattgccttcatggagttgatccaaggggttcccatgattgcattgtagatggccgggttatcgactactgcgaactcgatgatctttgtaacttccttagccatgaccgggagtttgatgctccctagggtcatggaggtgacgcccgaaaacccagtcaaaggttttggcgctgggatgactttcccaagtgggatgttcatcctatagagggtgtcgcggaagatgatgttgacagtacttcctgtatcaacaaggatgtggccgacttcgaaatcctggatcaccaggtcgataaccagaggatcgcaatgaggtttgtcgattctgacagtttcttgttcctcgaaaacaatcgtgtggttgggaatatcgctatccggaagccagttggaacttgtctcgattttccgaccgtaggccttgatcgacgagactgagtcttgatagaactgcgaccctccgataatcatatttaccctctggcgactgctgctgttcccctggtcgtcctatctccttccacgcttctcaaccgattgactttcaggcgcgtggtcctcggagacagtcttgtcggtttttgggcggtcggactccaggagcaaatcttttatactcttaaccttcgacagttcgccagcgaggagttttgcggccagcctggcgccgagaaccttgcagttcgcggtggaatgacctcgggtgtcatggaactcgcagtaggaattatccttgtattggttcctggtccaggtatttccggagtttttgccctgtgcctagttgatggcgtagttatgttcgccttggacgtcttccccttcgtgatggacgtacttgtcgttacgagagggtttcttctttgaggaggttttctgcggtccatgcatttgcgataggactctcatctcttcctccatgacgatgaagtctgttgccttgtggagggtatcctggatcgtccgtggtttctccagcaatatccactttcggaactttgacttgtactagagagttttcttcgtatgccgatcgcgactttgtcgttgatacccgccactcgccatcactagtttgaaccttctcatgaagtcgcaagtgattcagattcctttgagccagactccaaaaagtctacgtcagaagtctctctatccataaacatggaatactgcttgagaaatgccgaggctagttggcggaaacttccgatggagtttcttttgagctgagagaaccattcgagcgcggcgtccctgagattctcgacaaagagaaggcagtgaccggcgtctcgttcacgctccggaaatttgcatcttcccatcacgatctggaaggactgcaagtgtgcctttggatctgtggtactgtcgtagacgggaattatgatcttcccagagttcgagacgcgagtttctgtgatccgagcggtgaacggcgtttttcgtgcttcctcgacaagtctatcgatctcgggagcggcactagttgcctggtgaatctgtgatctcaccgcatttacctcggccactgtttttgcgagagactcgcggagatcgtggatttcgctatcgctacctgcattcttccgagcctgtcggtgctggttgcgatggatccgagtttgatcctccgccagttcttcctgttccatccagtagaggtcttcttcctcttctgtcatgggtttttcgaaggacaccgtctgtcggacagactgacttcaggtccttctatgatgaacgtgggcgttatcgtccgaatgatcggatcggtcgctaatgtccaggttgacctgttcgacgtcgttttcgacgttgtccccatagggaggtggaagattctccgtagtcggttgcgcacccggttggagaggttcgtcggggttttggcctgaggaagccttgtccgcacgtgcagcttgatcgcccggagtcttgaaatcgagtcttttgccgctgcgggctcttgtgatccctcgcggggccttgctcttggccttcgccgttaaggtttccacctgttttgcgagagaggtcacgggttttccttgttcgtccgcctgtttctgagcggaggcgaacatttctttcatttggtcttgtatcgtggagtcagcggtgaccgttggtacgtttccagctggagtgttggttgcgtcggcatcgacgggagttccgtcgtgcgtttgcaggttgtcagtgttggtcgccatattagaccgagcgtgtgtggttgcgagtgagatagatccgtacccaccccctctctctagcgctaaactttgggaaccgaaatttacactatcgattttatttgatttggaggaaagccaagtgaacctagccttccctgaaggtcccggttatctgctgggccacacacgacacaatcaataggacggaaagataacaaaacggaatataaaaatcataagaaaaaagatagagcaaaagatcttatttccgaatttgcgtttaagcgtgaacaacatgaaagagatcggctacaagagctgtcgatgagttcgctagtccagccacctgtatctaacctagttgagtcgcaactcgctagtaaaaacggaaaaaagtgcctaagttgctctaagtactatgttgctctctaaaagttctcctcttgctcctcgctccaagctctccttatatactcctcttaggacggtctattcctcttttgggccgaatctatcgcgaatcgggcttcttccattttcttcggtcttcatgtttatcgggaaacttgacatttatcttcaagaaacttgacatttatcttcggaaaacttgacaattatctctttatgtaaagataaacatgggccgtcacgtccatttcgacttgatctcctgaaaagtcgtaagtgggccgctttgtcgcgtttgggccttctgggccgttgtttcgtccgtgaacattttacgttttcgcgagagactagcctgccatggtgtttgttttgctgaaagaaccccaactcctcgtatagtctagatgactggtgttctgtagaataaccgtgatcgttttatacgatgaatcgaaatccattcgaacttttggtggtctttcaagccttccgatttatttcaccgtaacgaaatgggattctcgtgtttcatgtcttcgaggagtttgatcggtgagccttcgagcaaagatataaaatgtagagttggactagttgtcgagacagttttgcggggagaaggtcgcacctgtcgggtagtccgtatgcgggcgcccaggacttggacatggacgctggcgccggcgccggtgccagcacgggcgaagccgggcgccggtgccagcatgggcgaagccgggcgccggtgccagcatgggcgaagccgggcgcctggcgccggtgccagcatgggcgaagccgggcgcctggcgccggtgccagcatgggcgaagccgggcgccggtgccagcacgggcgaagccgggcgccggtgccagcacgggcgaagccgggcgccggtgccagcatgggcgaagccggcgccggcgccgggctggggccgcccccgctggtgtccgggactacgatgcgatcatcccctccgatgattccttccgaggactttcgggtgttgattgcgtctttgaccgattttgaccccaacagtaaacactaaacccaagcttggaaaatataaaccctcatccatgacaatcaataccattcacaaattaaaccatactatgtgtacataattatacaaactatgttacttggagatacttttatactatgcaaaacatcattgatttacatagaatataggggacaagagggaaatttaatacgtgtcgttaacaaatttaacagaagataaattgatcaataacagaccatatagaatagattacgtaacatatcaaatagtatagtaatgcgggctgtgtacccaattaaccgaagataaatttactaaaccaaagacccgacctgatcaataggattacgttaacccgataactaacccgagagttacatacttattcagaaacccgagacaccaaaatacccaattctctaaaatcaaaaataataaccctaaatgcactttcacggtgtctcccgaattacaatgccagaaagttcaagtaatgcatctggagcatcgtgtcgcggatgtgcttctattcgacgaggtagaaggataacgggaatatccaaaagatgttggtatggaactgaaattgtacctctgatgtccaattccgaccataatccttacagaagatactttcgatgtgcacatgctgcagcgaaaaaggtctattcttctgtcgttatgcataagtctgactgttttggcatattgattttgagatgaataggctttaagtgacttatcttttatgttgtgattgatgatgtagcttaagaatgataaccacgttttcaagttgattgatgaggttttgttagacgaagtcgagtcgatgcaattgaagattggaaagcatgaagaccaactgaaggagatggcaaaaacagagagtattttggctaaaagagttcaaattatggtggaagagatgataattgattaggtggaacaagtattggaagaaggcaaagcgagcatgaagtaaatgatggtattaggactggtcggatgcataatattgggagtagtaatggggaaggttttttgaaaatggttcggcttggtgtgtttagctgtaattccatatcaaaacctttcaatcttcatgtattttaatgttattgtaaaaccttatgttgctgttatgtagtaatgatattgtaagaacatagtatggcaaacaatgaatcataaatggaatacaaatctaggggatgaataagagatcagttgattgtgaatactaaatccaatttcggggattgtaaaccctaatccattggcaatccattggaaccccacattatcccttcatgtacagtctaaatgagacaagttaaagtagtgcttagaatatgtctgctatgttatgtggaacagatagaatgaaatatagaaaaccttatgcagtcgaagtgacgtgtgcggttgggaaggcaatgacgtatgcgattggataaagggacatcagttggtgacagctattccatttgatagagtatgaagaagccacataatgggttgcagttaccaatatattttcactatacaaattcaaataagtagtggaagttaaacactctatccataaatggtgtgttccatttatttaccactgtaagtccatctgaaaaattctgaaaaacaagaagctgaatgaagcagtgtagttaaagctgagaggaacatgtgtgaaattaaatccacatgctatactattgggaacatgtatttatattcttcatgaccaacatgaaatacaaagccaatgagattggtaatagaacacttgatagtaaatactaaacgaagttagggaaatataaaccccaatacatagggaactaaaatcttctggaaatataaacctcatgaccacatggaatatgcagtgggaaacgtatgtacaatctaatgcgattgtgttattccatataattgtgctatgtatatattattgtaactggttccattccatataccgtatattatgtaatttggatacaaatctaatgggggagtggtaaaattacacttgacattaaacacctaacacaaattgatgacgtctagtacatatgaaagagtaggaggatgccacgtacacctctccattaaccaagatattttcaccttctaaatttaaacaatgagtataaggtaatgattaccaaaggcgtatgtgtatagggttccgagaagacttttattccatgggaacggtactatttaaaatgtaaccatgtgtatagtaaatcaagaattgagcttcaaagataatacacaagatatgatatacaaagataatacacaataaacaacccaagttaggaaaatataaacgtacaaacttcgagaacccaaattttaatgaaattaaatcattgttaatacctcatatatgaacaccaaacgtacaaacttcgagaacccaattccaaatctaaacagcgagggactgcaaagcatagcatttccattccatatacactgaatgaaatcgaaatagagaaccactaaattgatctattacccgtgttatctagaagcttgacatgtgtggtagaagaggtgacgacgcatgcaatggaataaatggctattagttgtttacacctattccatttgagagaatagggaaaaacacgtatttagttggagttaccaagatattttcactgtatacattcaaacaagtggcctacgttaaaacattttatccataaaaggtttattccatttatttactactgtaactccatctcatcaattccaaaaaagaagaaggtgaatgaaacaacgtagttaatactggaaggaaacaaccaggtaacttgtcctcagaatactgccattaatggggtttcagataaaacaagcactcagactactgtaattaatgatgttttagataaagcttgtttgttagaataacatcatgtagatagtgtaatggaatagctgttgagatatagtaattatactgtaacttattactgcagatgacgagtcaagatagagttttactggttgtcggttcgtgggtccgtgaccaatacgagcaatgggttttcgaaccggacatatgtaaccaactccagcactacatccgactctataccaggatgacattgcgtgagttagttacagctgttagggagcgactacaagtaaccactaaaggagtgacgctgaaactatcttaccaatacccggagtggatttcattcgacgaccctgagttgagtcttcctcgatacataacggatgacatagaactgcggggatttatcgagatgagaagagccatagaggaggttaatctgtttatctcgttagttagccacactgtgggactaccatttgcgcgggacacagctgatataaatccaaaaatggcagcacgggtgaatcacacaatggacgaatcatggcatgactttgccctatcagagaccccactgacatttcctcaaacacagccgaatgcaaacacaaatgtcatagaagtcccagagggttctatttcacgtcaaccagctggaatggacactattagaggtcgtgctattctattccctaccggtggaatagaaatacgagagcctgaccacactatttgtcttagaagtccacgtattgcagctacggacaaggggacgaacaaaattcctatggattcatccactgagacatactcagatgatgatatggtggtccctgtcttgcaaacgtcggttgatatagcacgaggagagaacatgccagtgcgtatgcatttaatattttggattccagacccagttcaagaccctaatgatagcccatcaagttcagatgaaggtgaagagttgccacctgatgacggaatacattggggaagatttgatcaagctctacacgacatgcagaacgacccatataatccggctctgcttggtcaggatgctcctccggctttcaacgcgcgcccagaatcaggtgagttagacgtcgttgtccatattattctaaatagaatggaacatatattctaattataatatatggtataactaactcataacttcaccttgtaccaatataggtgtcgactccgcactacctgatgttcattacgagggagatgagatatttgttggccgagtcttcaagtctaaagcggactgcaaaataaagctggccatacatgcaataaacagaaagttccatttataaaccacccgatctaataccttgctgcttgtgattgaatgtgttggcgaatcatgtccatggcgcgtttatgcgatgctgttagatgctactggtaacttctaagtccgacaagctagtctaactcacacgtgcactgtcgacaaacgccggaactttcacagactagccacaacacaagtcatagaagagattctacagtcccgctttgttggaattaagaagggacccactactgcagttataaggaaaatactgcttgatgaattccatgtgaatgtatcatattggaaagcttggcgcgcaagggaactagccatagaacaagcaatgaggacaatggccgggagctactcactgattcctgcatatctgggactgctgcaagcctcaaacgaagggaccctttgctttatcgagcaaaacgatgacccaaaggggggggacacgctttaaatactgctttgttgcatatggagcttcagcagggtacgtctacatgaggaaagtagtcgtcgttgacggcacttcaatgaaagggaagtatggtggatgcctcttatccgcagtgacacaagacggaaattttcaaatatttccgtttgcttttgcagttgttgacagcgaaaacgataatgcgtgggagtggtttttccagaagctgagcacatttgtcaccgactgccccgaactcgtctttatctcggacagacatgctagcatatacacagacatgcgtaaggtacaaattgcaaacaaaaccactatatacttccattatattttattctatgtattaaatggtatagcaacgtgttgagtaggtgtacaaagaagcacaccacgcagcgtgtgtggtccatctttggcgcaatattcaagtcctctataagacgccgagacttggaaacctaatgtatgctgcagctcgcgcattcactatcacgaaatttaataggctgttcaaacagatccagagaattaaccctgcatgtgctgcatttcttgtggatataggtttgtactattatattttctaatatatgttatatcatttccaatagtgatatatagatttctattccatttccatatgcatttgacaccaacggcttcatcacagggtttacgcactagacgagagcacatttcaaaggtcaaagatacaatataatggactctaacatagctgagtcatggaatgacgccattaaggagacaagagagtacccactgatcatgatgctcgagtatatacgtacaactgtgatggggtggttggcgttgcgacgcgcaaaagctaacaacgagaagggatcattgacaccaaacgtgcgtaaacttgttgaagaaaactatgacctatcaattgccttagctgagcgtgacataagtgagctagagctccaagtgcaagaccctaccggagagtgtttcaccgttaactttgtcgttgggagctgctcttatagagagtatgacgaaattggaatcccctgtccccatgctctagctgcaggatcgaaggttgtgttcccatcagacgcaatggttgcaccagcgtatcgggtcccaagatggagacaaggatttgctggaaaaatttacccagttccttcagttggtgggtcgcaagtaggttcttctaccacagccgaactccttccccctgcagtccgcaggccatctggccgtccaagaaaggttcgcataaagtctcgtggggagttcaaggtaacagactccataatgaaatatcttagctttggttatgaaggataggatagtgaaattggaataggtaatgagtgttaaatgatggaatggtatttgaatgtgattcacatagaatggatactaaataccttatgaaataaccttgcagaagtcagggcagtcatcatgaaacaggaaatgcgtccgttgtggccggactgggcaccaacagagcatcttgccgcaatcctatataaaaaaaataagcggaaggagatggcatcagaaggcagtagaagcaatattttgggaaatgggtaatataagcaaaagccattgtcatctacagacttggcgtattatataatcttgaatggggagatattgcttttgggaacaaatacacaaatatatgcactcggtgacatatatgggtgtatttgtgatgtacatagtatgtcatatatagcccccttaagcacaaacaatgtgtgttgttgtaatgaagatccgtatgccttctcttttgtgtaatataaaatgatgccaatcttacttttaattaaatatgtttgctgtagtctaagtacgtaattactaatacatacaaggcactcgaataggaaacaatttctatttaggaactaactattcctgtgtaggaactaactattccatctcatatagtaataatctatttcatatatgttccataactcgagtcgttaatgtcaagtaatggagcaaccatgacctaatctgactgtcagatacagtaataggacaacaacatctgaattaaagagaaagatgccaatggttggtttgttgaaaaattcaatttaaagagtcacaccggactccaaataagcatataatgtaggagttgaaatctttcattcacgatgcaatagaggcgaatggcaactgtggggctgtgtatcacatggaattacaggtgtacgtgatggtaactacgaaagtaagtggaatagcataagagtaaacggaatagtaaatgagagaacgaaacagtattccaatcaaacaaggtaagcaggacaataaaacagaattcatccttggagtcgagtatagaaacataagaaagcgagacaagtttaacatttttgttgcttaacctagaaaaaaaatggatagcagaaaacaacagacatagaacggaaatagtagcgtctactgagcaggaggaagtgacacgggcggagacatgtgcagtgcttgaatggcgtaattctcggaagcggtgcgcgcctgttctttagtaaattgcacaatattcacatccttgccaatggcgtgcagctctaataacataagcgccaccaccgccgaacaacctattcaatagaacaacattagtacttaaaacactgataattacaaggagatgaaactgaaacctggagactaacctgggtgctccacaagagaaggaatctccaacctcgagacagtcatgggctcgaaattacgtttttgcgcatggttagtcatacagtaccgaccgatcaggtgcggcaacataatagaggctggtgttatcactgaactgatgtcaaactcagatggacaaccggtattgccttcaacaacatacaacacccacatagtcaaatcaacaataactccaacccagtggcttttcttgattagcaccggtatgtggagaaaatcaacttgcgtgaaccactgcaggcggtagagaaacgatgtcctcaatgatggggagaacgcgaaagcaacctttgttgaacaagcattaaagtcggcgaagtcactcaggaggtcagaaaaaaatgatgcatcgaggaagtcaaatctagacggtggcaaaccatccttgcgcttgcgtatgaaggcgaccacacgatcaattgcctatcacattacaaagtaaagattacgttagaagtttacatgactctgcctgttggaaacatatagtaaaccgtaagtaaggaccttctcagaagcaacccggctgcagtcaaaaagaggcagtaacgtgccaagatcgaaagcaggaactttggcagcggattgattcctgcacattaattcaaacaccacagtaaacttaaatatttcaagcaactaaatttcatgtagtatggaaagaaaaatatgagagagagcgtatgtacaacttacttggcatccttcattgcctggaggaatgcagcgcgtttaacaggatttggtgggagaaatggtgtaaaacccccaatgaaacaagtgtttttcgtaattgtaaaagttgggttaccaacggatgcaaccaccttctccttctccttctccttctccttctccttctccttctcctttggaccacgacgagcgcgtttgacagtttcttgcttacggggtacttcacccggcgtatatttgtctggaaagtgacgctcccgtttgctataccgtctgaagccgtccagtggtccatctgcagtgaccttcaccgcacgaccagcctagtaagtattaattacgttagcgactatatatgtacttgtacaaaataatagagtaaggataggtagacctttgttgggtttagcgttgattttttaatcacgacttcatcccctttggtcgctaccgaccctccgacatcatcctacactgtaaacatcttagaactaaaggctggaaagtggaatgtaatatttcagttttatctctctaccatgttttcggatcctaattcggattttggtttggtttggttcggatcctagttcggattttggttcggttaggttcggattataaccaaactccaaagaactaagctcataagtcccgttcggatatttttgtataacaattctgatttggtttcagtttttccgatttgggtttaggtaagtacttcgggttgagataaaaacgcccagacctaactcaaactatgttgcagcacaggaaaaagaagtatagtcttgtttaagcaaacttgaacgctattaaggaattcgagatgagatatagtataactttgatcggatggttttgcgacttgtctaaaaatcaaatactggtttctgaggaagattccttgaaatttggcccgttatagaatattaaagcaatagtctataacacagggaacaaacatatgatgtatatattatataacacaatgttgatggtctcttctgggactaataaacgtagcagtaacaggcatgaccatataaataatataacgacggataaattgcatgacttggattataaatagttacatatggctgaggattgataaaaaaaatctcttatcatgtacaacactggattcaggcaaagttgatgtcctcatattgacagcaatccttcatgtaggagaagttttggagattgccatatgtaaatacatcaatagatttcacaacatattgatattaaaaaaactaatgaaattggaaagaaaaacagcactgaggtctgaacgcaagccactgaattcattcgaggtcacttgctactttggaaattttgaaccatatcatctaaatttatgcaagtttataaactgaagtagcttgcctattgggaatggaaacaaaattgcaagtaacatgagatgtattgtcataagcgttccaaaaaaaaaaaattgcaagtaacatgtatatggacaccagctagcatcacacacatctttaaattcgccgacttagacctcacctataataatattatttattttgatctcatatagagaataaccacatctaagtcttggactaacaacaacagatttaagatactttacattatggtaccgagagaaaaacatgctattaagttccatatttcataatgagctatgaataatgtaagtaaacatctttcactttccctactttgtaatcactttttcctttgtttcaccaaagttagaaaagcttgctcgtgcctccgaagttttcattccatgtggtcgcctctataaagaaatggctaatcttatcttgtttaaatttaaagaaatgcttctttcttctatcatatatcatctttgatattttattcacacttttaaacacgtctcgtttgtggcagaccaccaaaaagtccaaaagcctacttccctgttttctttttctttataaatatcaaaaatattaatgagttaaccatgttgaaagaaaataaaaatctagcagcaaaagtgcacaagtacaaccttgattccttacgtcgtgggattaatttttcaatgttccggtacactgaaagccttcagtaaaaaaaatggtcctaaaaaacatttcgaagatagagaaaacaaacaataaaaaatgtcctttaacaaaaaaaaaaaatgtagataaattacacgaatttgaaatttattttccctgaaaaaactaaaagtaaattaaataaaagcattttttcctaaatgccgagactacccctgatctctttttctgtctggattgatttcaaaacgctccttcttctctgatctcctcctctcttctcctctcctcgcatcggtctgtgtctagcgagaactcgtgaaacgatggagcaacaacaaccggagaggcgagaaggccgaagcttccccgagcgcaagggacagaagagaaagctcgaggaaggagcagccgcctcctcagaagatcgagagatctccaccgacggcggcggcgatgcgattctcaacgaaatcgccgctcaagtatccgttctaaactccgccttctcatggcaggaatccgatcgcgctgcggcgaaacgcgccactcaagtcctctccgagcttgctaaaaacggtgagtgatcagcttcacttttctgcggtttcttcatatttttcttgatccatgacttagtaaccaccgttgttcagcagaggatttagtgaacgtgattgttgatggaggagctgttccggctctcatgacgcatctacaggcgccgccgtacatcgacggagacgtggctcaaaggccgtttgaacatgaggttgagaagggaagcgcctttgcgcttggtctactcgcaattaaggttttgatcctcatgtacttgtatagtgtgttagcttgtttgaaaacagtttctttttatgttatttttgctccaagtctagaagcgctttgtgatctcgttgtgaaattgtctgcttacagccagagtatcagaagctgatagttgacaagggggctttacctcatcttgtgaatctgttgaagagaaacaaagatggttctacttcccgagctgttaatagtgttatcagacgagctgctgatgccatcaccaatcttgctcatgagaacagcagcatcaagacccgtgttaggtcagcttatttaagtgacttcttcctgttaagatttttttcgttttcagtacaactgtcctcatgacttccagttcttgacaagcaggctcgaaggcggtattccacctctcgttgatttgcttgaattctctgattcaaaggttcagcgagcagcagcaggggcattacgaacccttgcgtttaaaaacgatgataacaagaaccaggtaaatatttctgtcttacaggttctaattcggttttcggtggagcatgattctttgtttttttgtgcagattgtcgaatgcaatgctcttcccacgctcattctaatgttaggatctgaagatgctgctatacattatgaagcggttaggaatcttttactgggtcgagagttttcataaatcaactgttttgctagttgctacttaaacagctacacgagatttaacactgaaataaccagttgaatcacacttttaggttggagttataggcaatctagtacattcgtctccaaacattaaaaaggaggttctttctgctggggcgttgcaacctgtcattggtcttctcaggtgtgtggaaactccacgttttgatttacatggttaagcatagagttgttactgttaaccttaggttcattctcgtcatttcatttctcgtatttgtctatttcagttcatgttgccctgagagccaaagagaggcagctttattacttggacaatttgcctcgactgattctgatagtaaggtactatttcatcccgggttttctatcctcagttcgtttgccatcccccaaattctaaactctttctgtttggttatactagttgtaatctgtttgttgctattgattttggtagaatatacattcccaattcttgctatctatcattttccctgatttatagttgtctttttcatttttcacctcgtgttcaaaaatatacatcgcaggtgcacattgtgcaaaggggtgctgtccgtcctttgattgagatgcttcagtcacaggacgttcagttgaaagaaatgtcggcctttgcactgggtagattggcgcaggttgttgtttcaaacattgttattttcagtttataaagttgaggcattcctatttggcgttgtaaacttgcaacttcgctctttagacttactaaataacattaccgatatgtctttaattttctagcgtaccctttctcacaggattctcacaaccaagctggtattgcccatagtggtggtttaggacctttattgaagcttctggattcaagaaatggatccctgcaacacaatgcggcatttactctctatggccttgccgataatgaggtgtgttgtctgcttccttccgtatgtattaatcaggatgcaaaaatttatttaaacctcactaaatgggttattgatccatttttgtcccctaggataatgtgtccgactttatcagggtgggaggtatccagatgctacaggatggagagtttatagttcaagtatgtatagcgttgttacccttctctactttccagaatcatattgtcgtattccttttatcggctggatactgaagattcttagcagctttaatagtatttgttttactctttgggtgtttataatatacactgttttttaggcaactaaagattgtgtctccaaaacactgaagcgattggaggagaagattcatggaagagtaagtgaaattatgcctgtctttaaacttgttctttccatatcttgtgactaaaacacacacatgtggtgaaactgctatattctctattcaacctttgagacttttgttctttgattttcctttgtaggttcttagacatcttttgtacttaatgcggatttctgagaagtctatccaaagacgagttgctctcgctcttgctcatctatgttcaccagaagatcagagaaccatattcatagatgaaaatggcatgtgacaattgaatatattatgtttagacttctgggtgttatccatttctgttaagatgttctttgtgcaaaaagttttatatcgagttgtcttttgacaggattggaattgctacttggtcttcttggttctacgaacactaagcagcaactagatggtgctgcagcattgtacaaattagcaaataaatctatggcactctctccagttgatgctgctccaccttctccaacacaaagggtgagtttccctcttgcttcggttctccagtatataagctgtggaagtttcatttgcattgttctgtttgttttgttatgacaggtttatctaggcgagcaatatgtaaataatgctacgctgtctgatgtaacttttctagtcgaaggtaatcatattaatcaggaagttgcagcagtcttgttagctccaaactccatatgtaaaccagaaaaatcatactgcaggaaggagattctatgcacacagaatttgtctgctggcatcttcagatgcatttcgtgcaatgttcgatggtggttacagagtaagtgagctattatttttggttggctgaccaatactttttcaatatgttcttgcggaggaaatgaaaaaaatatcatttattagctacggtgactatgacctatgggtttaggctgctctgcttctctgtaaaagaaatatatggatagtaatgtttattgtgcgcaaattgaattatctcattcagtttgtgtttcgtttatgccacaggaaaaggacgctagagatattgagattcctaatatcaaatggaaggtttttgagttaatgatgaggtatgacgaggagcttctaaatgtttctagactgtgggactcttaatatacgtgataattgacttacgcttggattgcgatgctcaggtttatatacactggatccgtcgacataacaattgagatatcacaagatcttctaagagcagcggatcagtatctcttggaggggctaaagcggctctgtgaatacacaattgctcaggtgaaccagaataactgcagtgtacagtgatttagtttgaataatagtaatcgaaatctaacacgggttgcttatgaatgaaaggatataacattggaaaacataggaggaatgtacgatctctcagaagcattccacgcaatgtcgctgaggcaagcttgtatcctgttcatcctggagcatttcgataaactgagcacaatgcatgggtaaatataaataagctcaatctctctcactctatttggcatttatctaaaacagagtgtgaatgaaaaatgcaggcagaaccagttggtgcagcgaacaataccagagataagagagtacttttgtagagctctaacaaagtctacgacaaatctgcaaagcctgaggctgtaa

SEQ ID NO: 168 - DNA, 4260 bp, Brassica carinata
  source 1..4260: mol_type = genomic DNA
atggagcaacaacaaccggagaggcgagaaggccgaagcttccccgagcgcaagggacagaagagaaagctagaggaaggagcagccgccgccgcagaggatcgagagatctccgcctcaaccaccaccgacggcggcggcgatgcgattctcaacgaaatcgctgctcaagtctccgttctaaactccgccttctcatggcaagaatccgatcgcgctgcggcgaaacgcgccactcaagtcctcgccgagctcgctaaaaacggtagaagatcagcttctttctttttttttttctgcggtttcttcatatatattttttttgttgattcgtgacttagttagtaaccaccgtttgttcagcagaggatttagtgaacgtgattgttgatggaggagctgttccagctcttatgacgcatctacaagcgcccccgtacatcgacggagacttggctcagaagccgtttgaacatgaggttgagaaggggagcgcctttgctcttggtctacttgcaattaaggtttagttactttacaaagcagttgtctttttatgttattttgctccaagtctagttttttcttaaggattatagtatagtgtttgtgatctcgttgtggaattgactgcttacagccagagtatcagaagctgatagtggacaaaggtgctttacctcatctcgtcaatctgttgaagagaagcaaagatggttctacttcccgtgctgtaaatagtgttatcagacgagcggctgatgccatcaccaatcttgctcatgagaacagcagcatcaagactcgtgttaggtcagcttatttaggtggtttgaaagatttgtttttcggtacaactgtcctcatgacttcaagttcttgacaagcaggctcgaaggcggtattccacctctcgttgatttgcttgagttttctgattcaaaggttcagcgagcagcagcaggggcgttgagaacccttgcgtttaaaaacgatgataacaagaaccaggtaaatgtttctgtcttacagcttctatttcagtttttcggtggagcattattcattgtttttttgtgcagattgtcgattgcagtgctcttcccacgctcattctaatgttaggatcagaggatgctgctatacattatgaagcggttaggaatcttttactgggacgagagttttcataatcaactgttttgctagttgctactcaaacatcaacatgacattgacactgaaataacgagttgagtcacgcttttaggttggagttatcggcaatctagtacattcttctccaaacattaaaaaagaggttctttctgctggggcgttgcaacctgtcattggtcttctcaggtgtgtggaactcgccgttttaattacatggttaagcatagagttgttactgttaaccctaggttcattctcatcattttttttgaatttgtctattgcagttcatgttgccctgagagtcaaagagaggcggctttattacttggacagtttgcgtcgactgattccgattgtaaggtactatttcatcccgggttttctatcctcagttcgtttgccattaccccaaagtctaaactctttctgtttggttatactaggcgtaagttgtttgttgctattgatatttgtagaatattcgtttccaattcgtgttatctatcattttccctgatttatgtgtctttttcattcttcacctcattttcaaaaatataactttgcaggtgcacattgtgcaaaggggtgctgtccgtcctttgattgagatgcttcagtcacctgacgtgcagttgaaagaaatgtcggcctttgcactgggtagattggcgcaggttcttgtttcagtcatttgttattttcagtttataaagttgaggcattcttttttggcgttgtaaacttgcaacttcgctctgtagacttataaccatttgagttatattaaataacattaccgatatgtcttttaatgtctagcgtaccctttctcgcaggattctcacaatcaagctggtattgcccatagtggtggtttaggacctttgttgaagcttcttgattcaagaaatggatccctgcaacacaacgcggcatttgctctctatggccttgccgataatgaggtgtgttgtatgctaccttccgtatgtattaattaggaatgcaaaaaaaaaatatttaaacctcattaaatgggttattgatccatttttgtcccctaggataatgtatcagattttatcagggtgggaggtatccagaagctacaggatggagagtttatagttcaggtatgtatagcgttgttaccctttcactactttctagaatcatatcgtcttattccttgtatcggctagatactgaagattctttgcagctttagtagtctttgttttactctttgggtgttataatttacactgctttttaggcaactaaagattgtgtctccaaaacactgaagagattggaggagaagattcatggaagagtaagtaaaattatacctgtctttaaacttgctctttccacatctggtgactaaaacatacacatgcacggtttgtggtgaaactgctatatcctggtctagctctgtcgaagtttagtatttctctatccaaccattgagacacttgttctttggttttcctttgcaggttcttagacatctgttgtacctaatgcgcatttctgaaaagtctatccaaagacgggttgctctcgctcttgctcatctctgttcaccagaagatcagagaaccatattcatagatgaaaatggcatgtgacaacttttttgaatttattatgtttagactttgacgtgttatccattgttgttaagatgttctttgtgcaaaaagttttatatcgagtttgtcttttgacagggttggagttgctacttggtcttcttggttctacgaacactaaacagcaacttgatggcgctgcagcattgtacaaattagcaaataaatctatggcactttctccagttgaagctgctcccccttctccaacacaaagggtgagctcccgtcttacttcagtcctccaatacataacttgtggaagtctcattgcagtattctttttgtgtatttgtgacaggtttatctcggagagcagtatgtaaatagtgccacgctgtctgatgtaacttttctagtcgaaggtaatcatcatattaatcaggaagttgcagcagtcttgttcgctccaaagtccatatgtaaaccagaaaaatcatactgcaggaaggagattctatgcacacagaatttgtctcctggcatcttcagatgcatttcgcgcaatgtttgatggtggttacagagtaagttagctattatttttgggtgaccaaatccttttcaatatgttcttgcggaggaaatgaaaaaatatcatttactagctatgatgacgatgacatattggttttggctgctctgcttctctttcaaaaggaatatatggatagttatgtttcttgtgtgcaaattgaatatctcactcagtttgtgtttcgtttataccacaggaaaaggacgctagagatattgagattcctaatatcaagtgggaggtttttgagttaatgatgaggtatgacgagcttgcaggcttctttattgtgagaactcttaacatacatgtaaatatgtaattgactcacttggattgtgattcccaggtttatatacactggatccgtcgacataacaattgagatatcacaagatcttctaagagcagcggatcagtatctattggaggggctaaagcggctctgtgaatacacaattgctcaggtgagccagaatacttgcaatttcaagtgatgtggtttgcataataattgtcgaaatctaacacagttttgcttataaatgaaaggatataacgttggaaaacataggaggcatgtacgatctctcagaagcattccacgcaatgtcgctgaggcaagcttgtatcctgttcatcctggagcatttcgataaactgagcacaatgcatgggtaatataaataagctctgtctctctctctctctctttttttttcagactatctctctatttggcatttatctgaaacagagcgaatgaaaaatggcaggcaaaaccagctggtacagcgaacaataccagagataagagagtacttttgtagagctctaacaaagtctactacaaacctgcaaggcctgaggctgtaa

SEQ ID NO: 169 - DNA, 3904 bp, Brassica carinata
  source 1..3904: mol_type = genomic DNA
atgaaaatctccaaatcgttcaaagtccaccgctcaaatccaccgtcgaatcttctcctcatccgtcctccgccagcgatctcaaaccatccacctatggagaagaacaacccgaagcgccagcgagcaacacgcgtctccggaagaatctcgaagcgaaagctcggcctggaggcatatgccgtttcgataatcacacagattacagaggttcaagacgaagaaacagatctaaccatcgcgatccgccgccacgtcgaggttctaaactccagcttctcagatgctgaatctgtcaaaggagctgctgccgctctctcctccctggcaaaaactggtactagttcttagactagatcgaattcgtatagcactcatcggcttgttaaaattgctcgatcttgtgttatagttgtttgaatcgattcagatctttgattctacttagcgattgatttgttatagctcatattaggcgagatctatattgttttcggcttaattttagtttcgtacttgtttgtattagacgaaaacgtggagatgatggtggaaaacggagcgatccctgctttggttagatacttggaatcgccgtggtcttcggcaatcagcgggaacgttcccaagtcttgcgatcataagctagagaaagactgtgctgtttcccttggccttattgctgctattcaggtaacacttgtgaatatcatttactgcttcttgcactgatgcttttactaatgttagctttatctgttacatagcctggttaccagcagcttatcgtagatgctggggccattgttccagctgtgaagttgttgaagagacgagggatttgtattgggtgcatggaagctaatgctgttattaggagagcagctgatatcatcactaatattgctcatgacaatccaaggataaaagctaatataaggtacggttttagtggttgataatcattatggttttggtttttggtcttgacatctttttaataactcttcgcagggttgaaggtggtattccaccacttgttgagctgttaaattttccggatgttaaagtacagagggctgctgcaggggccttgcgtacagtttcatttagaaatgatgagaacaagaaccaagtatgtgtttgctacgatggtgctttgttttgctttgtttgagaggcatgtttcttacatagaaagcatttttgtagattgtggagttgaatgctttgcctactcttgtgttgatgcttcagtcagaagatccatctgtgcatggcgaagcggttggttctttatcttgctttagattttttggaattggtttgctttgtttagttccttctaatttactattgaaatatcagattggggcaattggaaatcttgtccactcatctcctgacatcaagaaagaggttatccgcgctggtgccttacaaccagtaatcggtctacttaggtaggcttatttattctgctttactacttttgctgcagtagatgtttactacacatcttttgtaactgtttgctatgctatctgctacagctcaacttgtttggagacacagagagaagcagcactattaataggccaatttgcagcgcccgattcagactgcaaggtatacatttgtctctttcttgacgttgttgtgctctaatctgaatatatgctcactcaaactctttgttttgacgatatcaaaaggatggattcagagtaaagaaaacgtactaaaacataactggcaatatgatcatgcaggtgcacattgcacagagaggtgccattacaccattaattaagatgctcgattcatcagatgagcaggtcatggaaatggcagcttttgctcttggtcgtttggctcaggtagttatattttttgattatgcatgtgaacctttttgacgctttgtgtcataagaacaatggttgtaatttgtttgcttggagcataacttaattcgcatacatcaatgttttgaatgtcgcaggacacacacaatcaagctggcattggacaaagaggaggcatcatctcactactaaatctccttgatgtgaaaactggatctgtgcaacacaacgctgcctttgctttgtatggccttgcagataatgaggtaaactaagctcataatgaatagttttcaatacagctataatttttgctaactatacatatcatgggtacttaagtattttttccgtaattaggaaaatgtagcagatttcataaaggcagggggtattcaaaagcttcaagatgacaacttcactgttcaagtatgcatttgcctgcttatgtttgcaaaaccaacaaataggattcccaaattctaaattgcagttcttgtatttgcagccgactagggactgtgtggtgaggacattgaagaggctagagaacaagattcatggacctgtgagtatctatatgttcgaccttctggttcttagttaagtctggccttggtttctagtcccttgatgtcatactcttcttccaggtactaaaccaactattatatctaatgaaaaccactgagaagactatacaactgcgaattgctttggctcttgcacatctctgtgaccctaaagatggaaaattaattttcatcgataacaatggtactaatctcatctcaaaatttatcaatttttctttttgttgattttttttccctgatcaatagactttatgctgttatgcaggaatagagtttttgttggagcttctatacttaccaagcatgaagcagcagaagtctagttcaagagctttattcgaattagctacaaaagctacatcctttgcaccagaagactcagctccttcctcacccacacaacgggtaagaaatcttcatttcttcttttaaattataaaatatgatatctgttttgaggtcttgacttgttatttgttttaatactgaaggcgtttttgggtgaggagttcgtgaacaaccctactttatccgatgtcacattcctaatcgatggtacaacttttgagcccatcaatgttattgctaaatctacctgtgataacacttttttaaaccgagtgtttccatggcatataataggtaaacaattctatgctcacaagatttgcttggtagcttcctctgatatatttcgtgcaatgtttgatggcctttacaaggtaaccttctgaactaatgactgtggtacccatttcatcatacaaatcaactaacttgagaattggttttaggaacgaaacgcccaaaatgtggagatcccaaatataagctgggaagtgtttgagcttatgatgaggtaaacttctataagatcaaacatgtcgaatctttaccataataaaaagctaaaaatctaaagcatgaaatgcaatgtgatgcagattcatatacacaggaaaaatcaacatcacaaaacatttagctcaggatctgcttgtagcagctgatcagtatctgctcgatggcctcaaacggctttgtgagtacacaatcgcgcaggtaaatacacaaaaccaacgtacttatgtgacttatctctgtgtataactaaattagactttacaaatggttggtgcaggacatatgtgtggataacataccattcatgtacgacttagcagatacattcaatgcttcagccttaagacgagcatgcactctcttcgttcttgagcattacactaagctcagctttgaactgtggtatgcaaaaacatcattacatcatttatacaattttagaattaaaacttctctcttacttgttcttctttttttaaacgcaggtttcccatgttcataaagaaaattatacctgaaatccggagttacatcactgatattctcagacggccagtccaagctagcagcagctag

SEQ ID NO: 170 - DNA, 3887 bp, Brassica carinata
  source 1..3887: mol_type = genomic DNA
atgaaaatctccaagtcgctcaaaatccaccgtcgaatctcctcctcgtcagcgatctcaaaccatccacctatggaggagaatcatcacaagcgccagcgaacagctcgcgtcgtcgccggaagaacctcgaagcgaaagctcggccgagagacgtacgcggtttcgataatcacgcagatcaccgagatcgaggaagaagaaacagatctcgccgtcgcgatccgccgccacgtgggggttctgaactccagcttctcagatgcgggagatgtcaaaggagctgctgctgctctctcctccctcgctaaaactggtaccgtactccttagagtagatcgttttgttgttacagctgtttgaatcgatgccgatctgtgattctactttgcgattgaattgttctagctcagattaggcgagatctagattgattatggattgattttggattcgtaactctttgtgttagacgaaaacgtggagatgatggtggagaacggagcgatccctgcgttggttagaaacttggaatcgccgtggtctttggcaatcagcgggaacgttcccaagtcttgtgatcataagctagagaaagattgtgctgtttcacttggacttattgctgctaatcaggtaacacttgtgaatatcatttactgcttcttgcactgatgcttttactaatgttagctttatttgttaaatagcctggttaccagcagctaattgtagatgctggggttatagctccaactgtgaagttgttgaagagaagaggagtttgtattgggtgcatggaagctaatgctgttcttaggagagcagctgatatcgtcactaatattgctcatgacaatccaaggattaaaaataatataaggtacggtttagtgtttgatgatccttatgctttttggtcttggctaagttgttttcgcttgacagggttgaaggtggcattccaccacttgttgagcttttagattttccggatgttaaagtacagagggctgctgctggggccttgcgtacggtttcttttagaaatgatgagaacaagaaccaagtatgtgtttgctacgatggtgctttgtttttgcttttgtttgagaggcatgtttcttatataaagagcatctgtgtagattgtggagttgaatgctttgcccacgcttgtattgatgcttcagtcagaagatccttctgtgcatggcgaagcggttggttcttttatcttgctttagatttttggaattggtttgttttgtttagttccttctaatataatattgaaatatcagattggggcaattggaaatcttgtccattcatctcctgacatcaagaaagaggttatccgcgctggtgccttgcaaccagtaatccgtctacttaggtatgcttattttctttattctgtttttctgtttctgctgaaatagatgtttactcttgatattgtgaaacatcttttgtaactgtttctgttcgctatgatatctgctacagctcaacttgcttggagacacagagagaagcagcattgttgattggtcaatttgccgcgcctgattcagactgcaaggtataagtttgcctctttcttgacgttgttgtgctctaatctgaatatatgctcactcaaactctttgttttgacgatatcaaaaggatggattcagagtaaagaaaacgtactaaaacataaatggcaatatgattatgcaggtgcacattgcccagagaggtgcaattacaccattaattaagatgcttgagtcatcagatgagcaggtcacagaaatggcagcgtttgctcttgggcgtttggctcaggtagttatgtttttgaataagcatgtgaatctttttgacgctttgtgtcataagaacaatggttgtaatttgtttgcttggagcataacttaattcgcatacatcaatgctttgaatgtcgcaggacacacacaatcaggctgggattgggcaaagaggaggcattatttcactactaaatcttcttgatgtgaaaactggatctgtgcaacacaacgctgcctttgctttgtatggccttgcagataatgaggtaaactaatctcataatgaatcgttttcaatacatctatactttttgctaactataaataacaatggttaattaattttttcttaaacaggaaaatgtagcagatttcataaagactggaggtattcaaaagcttcaagatgacaacttcaccgttcaagtatgcatttcgttgcttatgtttgcaagaacaatatataggctttccaaattctaaattgcaagtcttctctttgcagccgactagggactgtgtggtgaggacattgaagaggctagagaacaagattcaaggacctgtgagtacctatctgttagaccttcttgttcttataagtatggccttggttctagagtcccttaatgtcatactcttctttcaggtactaaaccaactattatatctaattaaaaccactgagaagaatatacaaatgcgaattgctttggctcttgcacatctttgtgaccctaaagatggaaaattaattttcatcgataacagtggtaaatattctcatctcaaaattcatcaatttttcttttcttgtcgatttttttctgttcctgatcaatcgactattacatatgctatgttatacaggaattgagtttttgttggagcctctatacatctcaagcatgaaacagcataagtatagcgcaagagctttattcgaattagctacaaaagctacatcctttgcaccagaggactcagcaccttcctcacccacacaacgggtaagaactcttcattacttctttcaattataaaaatataatttctgatttgaggtcttgacttgttattgattataatactgaaggcgtttttgggtgaggaattcgtgaacaaccctactttgtccgatgtcacattcctgatcgatggtaaaacatttaatcccttcgatgtttatgttaaatctacctgtgataacactttttaaactgagtaattccatggcatatattaggtaaacaattctttgctcataagatttgcttggtagcttcctctgatatatttcgtgcaatgtttgatggcctttacaaggtaaccttctgaataaatcattgtggtacccatttcatgatacaaagtatcaatcaactaacttgagaattggttttaggaacgaaacgcccaaaatgtggagatcccaaatataagctgggaagtgtttgagcttatgatgaggtaaagttctattaaatcaaaaccataataataagctaagaatctaaagcatgaaatgcaatggtgcagattcatatacacaggaaaaatcaacatcacaaaatacttggctcaagaactgcttgtagcagctgatcagtatcttctcgatggtctcaagcggctttgtgagtacacaatcgctcaggtaaatactcaaaaccaactttttattcttctccttgtcagagtggcttgtctatgtgtataactaaatggacttctctaatggttggtgcaggacatctgtgtggaaaacataccgttcatgtacgacttagcagatactttcaatgcgtcagccttaagacgagcttgcactctcttcgttcttgagcattacactaagctcagctctgaattgtggtatgcaaaaacaaatcattacatcattaatacattttttttggaatcaaccttatctcttacttaatcaggttttatgttcttttttttttacgcaggtttcccatgttcataaagaaaattatacctgaaatcaggagttacatcactgatattctcggacggccagtccaagctagcagctag

SEQ ID NO: 171 - protein, 700 aa, Brassica carinata
MEQQRESRSFPERKGQKRKLEEGPPAAAEDPQISPSTTTDAALLSEVAAQVSVLNSAFSWKESDRAAAKRAAQVLGEHQSRLSYLASDLVNVIVDGGAVPALTAHLQPPPCSDGDLAHKPFEHEVEKGSAFALGLLAIKPEYQNLIVDKGALPHLVSLLKRNKEGPTSRAVNSVVRRAITNLAHENSSIKTRVSRLEGGIPPLVELLEYSDSKVQRAAAGPCFDCLLLQIVECNALPTLILMLGSEDAAIHYEASCLYVGVIGNLVHSSPNIKKEVISSGALQPVIGLLSSCCPESQREAALLLGQFASTDSDCKVHIVQRGAVRPLIEMLQSPYVQLKEMSAFALGRLAQDSHNQAGIAHSGGLEPLLKLLSSRNGSLQHNAAFALYGLADNEDNVSGFIRVGGVQKLQDEEFIVQATKDCVSKTLKRLEEKIHGRVLRHLLYLMRISEKSIQRRVALALAHFCSPEDQRTIFIDEKGLELLLGLLGSTNTKQQLDGTAALYRLANKSMALSPVDAAPRSPTQRVYLGEQYVNSATLSDVTFLVEGRRFYAHRIYLLGSSDAFRAMFDGGYREKDARDIEIPNIKWEVFELMMRFIYTGSVDITIEISQDRLRAADQYLLEGLKRLCEYTIAQDITLENIESMYDLSEAFHALSLRQACILFILEHFEKLSSMHGQNELVQRTIPEIREYFCRALTKST

SEQ ID NO: 172 - protein, 711 aa, Brassica carinata
MEQQQPERREGRSFPERKGQKRKLEEGAAASSEDREISTDGGGDAILNEIAAQVSVLNSAFSWQESDRAAAKRATQVLSELAKNAEDLVNVIVDGGAVPALMTHLQAPPYIDGDVAQRPFEHEVEKGSAFALGLLAIKPEYQKLIVDKGALPHLVNLLKRNKDGSTSRAVNSVIRRAADAITNLAHENSSIKTRVRLEGGIPPLVDLLEFSDSKVQRAAAGALRTLAFKNDDNKNQIVECNALPTLILMLGSEDAAIHYEAVGVIGNLVHSSPNIKKEVLSAGALQPVIGLLSSCCPESQREAALLLGQFASTDSDSKVHIVQRGAVRPLIEMLQSQDVQLKEMSAFALGRLAQDSHNQAGIAHSGGLGPLLKLLDSRNGSLQHNAAFTLYGLADNEDNVSDFIRVGGIQMLQDGEFIVQATKDCVSKTLKRLEEKIHGRVLRHLLYLMRISEKSIQRRVALALAHLCSPEDQRTIFIDENGLELLLGLLGSTNTKQQLDGAAALYKLANKSMALSPVDAAPPSPTQRVYLGEQYVNNATLSDVTFLVEGRRFYAHRICLLASSDAFRAMFDGGYREKDARDIEIPNIKWKVFELMMRFIYTGSVDITIEISQDLLRAADQYLLEGLKRLCEYTIAQDITLENIGGMYDLSEAFHAMSLRQACILFILEHFDKLSTMHGQNQLVQRTIPEIREYFCRALTKSTTNLQSLRL

SEQ ID NO: 173 - protein, 715 aa, Brassica carinata
MEQQQPERREGRSFPERKGQKRKLEEGAAAAAEDREISASTTTDGGGDAILNEIAAQVSVLNSAFSWQESDRAAAKRATQVLAELAKNAEDLVNVIVDGGAVPALMTHLQAPPYIDGDLAQKPFEHEVEKGSAFALGLLAIKPEYQKLIVDKGALPHLVNLLKRSKDGSTSRAVNSVIRRAADAITNLAHENSSIKTRVRLEGGIPPLVDLLEFSDSKVQRAAAGALRTLAFKNDDNKNQIVDCSALPTLILMLGSEDAAIHYEAVGVIGNLVHSSPNIKKEVLSAGALQPVIGLLSSCCPESQREAALLLGQFASTDSDCKVHIVQRGAVRPLIEMLQSPDVQLKEMSAFALGRLAQDSHNQAGIAHSGGLGPLLKLLDSRNGSLQHNAAFALYGLADNEDNVSDFIRVGGIQKLQDGEFIVQATKDCVSKTLKRLEEKIHGRVLRHLLYLMRISEKSIQRRVALALAHLCSPEDQRTIFIDENGLELLLGLLGSTNTKQQLDGAAALYKLANKSMALSPVEAAPPSPTQRVYLGEQYVNSATLSDVTFLVEGRRFYAHRICLLASSDAFRAMFDGGYREKDARDIEIPNIKWEVFELMMRFIYTGSVDITIEISQDLLRAADQYLLEGLKRLCEYTIAQDITLENIGGMYDLSEAFHAMSLRQACILFILEHFDKLSTMHGQNQLVQRTIPEIREYFCRALTKSTTNLQGLRL

SEQ ID NO: 174 - protein, 737 aa, Brassica carinata
MKISKSFKVHRSNPPSNLLLIRPPPAISNHPPMEKNNPKRQRATRVSGRISKRKLGLEAYAVSIITQITEVQDEETDLTIAIRRHVEVLNSSFSDAESVKGAAAALSSLAKTDENVEMMVENGAIPALVRYLESPWSSAISGNVPKSCDHKLEKDCAVSLGLIAAIQPGYQQLIVDAGAIVPAVKLLKRRGICIGCMEANAVIRRAADIITNIAHDNPRIKANIRVEGGIPPLVELLNFPDVKVQRAAAGALRTVSFRNDENKNQIVELNALPTLVLMLQSEDPSVHGEAIGAIGNLVHSSPDIKKEVIRAGALQPVIGLLSSTCLETQREAALLIGQFAAPDSDCKVHIAQRGAITPLIKMLDSSDEQVMEMAAFALGRLAQDTHNQAGIGQRGGIISLLNLLDVKTGSVQHNAAFALYGLADNEENVADFIKAGGIQKLQDDNFTVQPTRDCVVRTLKRLENKIHGPVLNQLLYLMKTTEKTIQLRIALALAHLCDPKDGKLIFIDNNGIEFLLELLYLPSMKQQKSSSRALFELATKATSFAPEDSAPSSPTQRAFLGEEFVNNPTLSDVTFLIDGKQFYAHKICLVASSDIFRAMFDGLYKERNAQNVEIPNISWEVFELMMRFIYTGKINITKHLAQDLLVAADQYLLDGLKRLCEYTIAQDICVDNIPFMYDLADTFNASALRRACTLFVLEHYTKLSFELWFPMFIKKIIPEIRSYITDILRRPVQASSS

SEQ ID NO: 175 - protein, 729 aa, Brassica carinata
MKISKSLKIHRRISSSSAISNHPPMEENHHKRQRTARVVAGRTSKRKLGRETYAVSIITQITEIEEEETDLAVAIRRHVGVLNSSFSDAGDVKGAAAALSSLAKTDENVEMMVENGAIPALVRNLESPWSLAISGNVPKSCDHKLEKDCAVSLGLIAANQPGYQQLIVDAGVIAPTVKLLKRRGVCIGCMEANAVLRRAADIVTNIAHDNPRIKNNIRVEGGIPPLVELLDFPDVKVQRAAAGALRTVSFRNDENKNQIVELNALPTLVLMLQSEDPSVHGEAIGAIGNLVHSSPDIKKEVIRAGALQPVIRLLSSTCLETQREAALLIGQFAAPDSDCKVHIAQRGAITPLIKMLESSDEQVTEMAAFALGRLAQDTHNQAGIGQRGGIISLLNLLDVKTGSVQHNAAFALYGLADNEENVADFIKTGGIQKLQDDNFTVQPTRDCVVRTLKRLENKIQGPVLNQLLYLIKTTEKNIQMRIALALAHLCDPKDGKLIFIDNSGIEFLLEPLYISSMKQHKYSARALFELATKATSFAPEDSAPSSPTQRAFLGEEFVNNPTLSDVTFLIDGKQFFAHKICLVASSDIFRAMFDGLYKERNAQNVEIPNISWEVFELMMRFIYTGKINITKYLAQELLVAADQYLLDGLKRLCEYTIAQDICVENIPFMYDLADTFNASALRRACTLFVLEHYTKLSSELWFPMFIKKIIPEIRSYITDILGRPVQASS

SEQ ID NO: 176 - DNA, 3863 bp, Brassica rapa
  source 1..3863: mol_type = genomic DNA
atgaaaatctccaaatcgctcaaactccaccgctccaatccaccgtcgaatctcctcctcgtccgtcgtccgtcatcgatctcaaaccttccacctatggagaacaatcttaagcgccagcgaacaacacgcgtcgccggaagaagctccaagcgcggccgggagacgtacgcggtttcgataatcactcagatcaccgagatcgaggaagaagaaacagatctcgtcgtcgcgatcagccgccacgtggatgttcttaactccagcttctcagatgcgggagatgtcaaaggagctgctgctgctctctcctccctcgctaaaactggtaccgtaactgtttgaatcgatgcagatctgtgattctacttagcgattgatttgttctagctcagattaggcgagatctagattgttttttgattcgtaactgtttgtattagacgaaaacgtggagatgatggtggagaacggagcgattcccgctttggttagaaacttggaatcgccatggtctttagcaatcagcgggaacgttgccaagtcttgtgatcataagctggagaaagattgtgctgtttcacttggactcattgctgctaatcaggtaacacttgtgaatatcatttactgcttcttgcactgatgttttttactaacgttagctttatctgttaaatagcctgcttaccagcagctaattgtagatgctggggttatagctccgactgtgaagttgttgaagagaagaggggtttgtattgggtgcatggaagctaatgctgttcttaggagagcagctgatatcatcactaatattgctcatgataatccaaggattaaaactaatataaggtacggtttagtgtttgatgatccttatgctttttttggtcttggctataagttgttttcacttgacagggttgaaggtggcattccaccacttgttgagcttttggattttccggatgttaaggtacagagggcggctgctggggccttgcgtacagtttcttttagaaatgatgagaacaagaaccaagtatgttttgcttttgatgatgctttgtttgagcttatgagaggcatgtttcttacataaaaaaacatttgtgtagattgtggagttgaacgctttgcccacgcttgtattgatgcttcagtcagaagatccttctgtgcatggcgaatcggttggttcttttatcttgctttggatttttggaattggtttgctatgtttagttccttctaatatactattgaaatatcagattggggcaattggaaatcttgtccactcatctcctgacatcaagaaagatgttatccgcgctggtgccttgcaaccagtaatcggtctacttaggtatgcttattttctttattctgtttttctacttctgctgaaaatagatgtttactcttgatgttgtgaaacatcttttgtaactgtttctgcttgctatgatatctgctacagctcaccttgcttggagacacagagagaagcagcattgttaattggtcaatttgctgcgcctgattcagactgcaaggtataagtttgtctctttcttgacattgttgtgctctaatctgaatatatgctcactcaaactcttttgttttgacgatatcaaaaggatggattcagagtaaagaaaacgtactaaaacataaatggcaatatgattatgcaggtgcacattgcccagagaggtgccattacaccattaattaagatgcttgagtcatcagatgagcaggtcacggaaatggcagcgtttgctcttggtcgtttggcccaggtagttatgtttttgaataagcatgtgaatctttttgacgctttgtgtcataagaacaatggttgtaatttgtttgcttagagcataacttaattcgcatatatcaatgctttgaatgtcgcaggacacacacaatcaggctgggattgggcaaagaggaggcattatttcactattaaatcttcttgatgtgaaaactggatctgtgcaacacaacgctgcctttgctttgtatggccttgcagataatgaggtaaactaatctcataatgaatcgttttcaatacatctacactttttgctaactataaataacaatggttaattaatttttcgtaaacaggaaaatgtagcagatttcataaagactggaggtattcaaaagcttcaagacgacaacttcaccgttcaagtatgcatttcgctgcttatgtttgcaaaaacaatattataggctttccaaattctaaattgcaagtcttctctttgcagccgactagggactgtgttgtgaggacattgaagaggctagagaacaagattcatggacctgtgagtacctatctgttagaccgtctggttcttataagtatggccttggttctagagtcccttaatgtcatactcttctttcaggtactaaaccaactattatatctaatgaaaaccactgagaagaatatacaaatgcgaattgctttggctcttgcacatctttgtgaccctaaagatggaaaattaattttcatcgataacagtggtaatattctcatctcaaaattcatcagtttttcttttcttgtcgatttttttctgttcctgatcaatcgactattatttatgctatgttatacaggaatggagtttttgttggagcctctatacatctcaagcatgaaacagcagaagtatagcgcaagagctttattcgaattagctacaaaagctacatcctttgcaccagaggactcagctccttcctcacccacacagcgggtaagaaattttcattacttctttcaattataaaaatataatttctgatttgaggtcttgacttgttattggctgtaatactgaaggcgtttttgggtgaggaattcgtgaacaaccctactttgtccgatgtcacattcctgatcgatggtaaaacatttaatcccttctatgtttatgttaaatctacctgtgatcacactttttactgagtgtttgcatggcatatattaggtaaacaattctttgctcacaagatttgcttggtagcttcctctgatatatttcgtgcaatgtttgatggcctttacaaggtaaccttcttaataaattattgtgctacccatttcatgatacaaagtatcaatcaactaacttgagaattggttttaggaacgcaacgcccaaaatgtggagatcccaaatataagctgggaagtgtttgagcttatgatgaggtaaagttctataaactcaaacattttgaatacttaccattataataagctaagaatctaaagcataaaatgcaatggtgcagattcatatacacaggaaaaatcaacatcacaaaatacttggctcaagatctgcttgtagcagctgatcagtatcttctcgaaggtctcaagcggctttgtgagtacacaatcgcgcaggtaaatacacaaaaccaacttcttattcttctccttgtcagagtggcttgtctatgtgtataactaaatggactcctctaatgttggtgcaggacatctgtgtggaaaacataccgttcatgtacgacttagcagatacattcaatgcgtcagccttaagacgagcatgcactctcttcgttcttgagcattacactaagctcagctctgaactgtggtatgcaaaaacaatcattacatcatttatacaatgaaataacgtttcttttacttaatcaggttttatgttcttattttcttacgcaggtttcccatgttcataaagaaaataataccagaaatccggagctacatcactgatattctcagacggccagtccaagctagcagctag

SEQ ID NO: 177 - DNA, 3924 bp, Brassica rapa
  source 1..3924: mol_type = genomic DNA
atggagcaacaaagaggaagccggagctttccagagcgcaagggacagaagaggaaactagaggaaggaccacccgcagaggatccacagatctctccctcaaccaccaccgacgcagccccccacgctgcgcttctcagcgaagtcgctgctcaagtctccgttctaaactccgccttctcctggaaagaatccgatcgcgccgccgcaaagcgcgcagctcaagtcctgtctgagctcgccaaaaacggtgaacatcagtctcctatagcttcacttttcttcggtttcttattatctcttagtgaccttcgatgttcagcagatgatttagtgagcgtgattgtcgacggaggtgctgttcctgctctcacgacgcatctacagcccccgccgtactgtgaaggagacttagctcaaaagccgtttgaacatgaggtcgagaaaggaagcgcctttgcgcttggtcttctcgcaattaaggttttggtcccaagtttagttttttaaagcaacttttggtaataaagattctatttttatattcggaggggactatgtgtagtttgtgtggtcacgttgtgggattgattacttacagccagagtatcagaacctgatagtagacaaaggagctttacctcatctcgtggatctcttgaagagaagcaaagattcctccacttctcgagcccttaatagtgttattagaagagcggctgatgccattactaatctagctcacgagaacagcagcatcaagacccgtgtcaggtcagcttatttttctaagtggtttcctccttttcagtacaactatcctcctgactttttgacaaaacaggctagaaggcggtattccacctctcgtggagttgcttgagtattctgattccaaggttcagcgagcagcagcaggggcgttgcgaacgcttgcgtttaaaaacgatgataacaagaacctggtaagtattgctgtcttatagcttctacttagatttttggacggagtgtgttttgattgtctacttttgcagatagttgaatgcaatgctcttcccacgctcattctaatgcttggatcagaggatgctgctatacattacgaagcggttaggattcttttactgcgtcgagagttttcataatcaactcttttgctacttatctgagtcatgcttttaggttggagttataggcaatctagttcattcgtctccgaacattaaaaaagaggttatttcttctggggcgttgcaacctgtcattggtcttctcaggtatgtggaaactcgtcattttgatttaaatggttaagcatagagttgttactgttaaccttagtgacgttcttgttgtttcttgtattttgtctatttcagctcatgttgccctgagagccaaagagaggcggctttattacttggacagtttgcctctactgattctgattgtaaggtactatttcatctctatcctcagttcgtttgctatccaccaaagcataaactctttctgcttggttgtactaggtgtaagctgttttttcttctgttgattttcaggttcacattgttcaaaggggtgctgttcgtcctttgattgaaatgcttcagtcagcggatgttcagttgaaggagatgtcggcctttgcactgggaagattggcccaggttcctcttttaaacctttgttagtttgagccgctgtaaaattgtaacctcgctctttaggcttaaaaccaatgagctatattaaaattacaaaactgttatgtcttttaattctctagcatactctttgtcgcaggattcccacaaccaagccggtattgctcatagtggtggtttagaacctttattgaagcttctcagttcaagaaatggatccttgcaacacaatgctgcctttgctctttatggccttgccgataatgaggtgcgttgaatgctgctaccttccgtatatgttataattaggatgcaaaattccttattaaattggttattgatccccatttttctccccgtaggataatgtgtcgggttttatcagggtgggaggtgtccaaaagctacaggatgaagagtttattgttcaagtatgtgaatcatatcgtcatttttcttttagtggctatatactgaaatttcttagcagctgtatttgttttactctctcgttggatgtttctaatgtacaatgtttcttaggcaactaaagattgtgtctccaaaacattgaagaggttggaggagaagattcatggaagagtaagtaaaattttacctgtctttaaacttgttacttccatctctggtgattaaaaaaatacacaaatgcacggtttgtagtaaaactgatgtatcctggtctagtgtctgaaactttgtttaagtttagtatttctctatggaacctttgaaacttatgtgctttggatttcctttgtaggttctaaggcatctgttgtaccaaatgcgcatttctgagaagtctatccaaagacgagttgctctcgctcttgctcatttctgttcaccggaagatcagagaaccgtattcatagatgagaatggcatgtgacagatttttttgaatttatgatgttaagacttttaacgctttaaccattaagtttaaatgttctttctgcaattctttttatattgagctgtcttttgacagggttggagttgctacttggtcttcttggttctacaaacactaagcagcaactcgatggcgctgcagcattgtacagattagcaaataaatccatggcactttctccagttgatgctgctcctccttccccaacacaaagggtgagtcaccttcttgcttcagttctccattacgtaagttgtggaagtctcagtgcatcattctgtttatctttttgtgacaggtttatctcggagagcaatatgtaaatagtgcaacgctgtctgatgtaacttttctagtcgaaggtaatcatattactcagaaaattgcagcagtcttgttagctccaaacaccatatgtaaaacagaaaagatcatactgcaggaaggagattctatgcacacagaatttgtctgctggcttcttcagatgcatttcgcgcaatgtttgatggtggttaccgagtaagtgaactattatgttctttttgaaaaacatctactagctataatgactattatctatgaaactctgcttctctgtcaaaggaatacatggataattatgtaaacatgtctcattcagtttgtgcttcgtttataccataggaaaaagacgctagagatattgagattccgaatattaaatgggaggtttttgagttaatgatgaggtatgacgagtttctacaagcttctagactgagaactttcgtcatatacatgtaactaactcacacttgaactgtgatcttcaggtttatatacactggatcagtcgacataacaattgagatatcacaagatcttctgagagcagcggatcagtatctcttggagggtctgaagcgactctgtgaatacacaattgctcaggtgagtcagaacaatggaaaatgatgtggtttgcattataattctggaaatctaacacggttgcttatgaatgaaaggatataacgttggaaaacataggaagcatgtacgatctctcagaagcattccacgcgatgtcgctgaggcaagcttgtatattgttcatcctggagcatttcgaaaaactgagttcaatgcatgggtaatatgaagtacctctctcttactctcacagtctttggcctatatatctgaaacatagtggatgaaaaatgcaggcagaacgagctggtgcagcgaacaataccagagataagagagtacttctgtagagctctaacaaaatctactacaaacctgcaaagcctgaggttgtag

SEQ ID NO: 178 - DNA, 7030 bp, Brassica rapa
  source 1..7030: mol_type = genomic DNA
atggagcaacaacaaccggagaggcgagaaggccgaagcttccccgagcgcaagggacagaagagaaagctagaggaaggagcagccgccgccgcagaggatcgagagatctccgcctcaaccaccaccgacggcggcggcgatgcgattctcaacgaaatcgctgctcaagtctccgttctaaactccgccttctcatggcaagagtccgatcgcgctgcggcgaaacgcgccactcaagtcctcgccgagctcgctaaaaacggtagaagatcagcttcttttttttgttctgcggtttcttcatatatatttttttgttgattcgtgacttagttagtaaccaccgtttgttcagcagaggatttagtgaacgtgattgttgatggaggagctgttccagctcttatgacgcatctacaagcgccgccgtacatcgacggagacttggctcagaagccgtttgaacatgaggttgagaaggggagcgcctttgctcttggtctacttgcaattaaggtttagttacttgtatagtgtgttagtttgttatgttattttgctccaagtctagttttgattatagtatagtgtttgtgatctcgttgtggaattgactgcttttacagccagagtatcagaagctgatagtggacaaaggtgctttacctcatctcgtgaatctgttgaagagaagcaaagatggttctacttcccgagctgttaatagtgttatcagaagagcggctgatgccatcaccaatcttgctcacgagaacagcagcatcaagactcgtgttaggtcagcttatttaggtggtttccaaagatttggttttttttttggtacaactgtcctcatgacttcaagttacttgacaagcaggctcgaaggcggtattccacctctcgttgatttgcttgagttttctgattcaaaggttcagcgagcagcagcaggggcgttgagaacacttgcgtttaaaaacgatgataacaagaaccaggtaaatgtttctgtcttagagcttctatttcagttttttcggtggagcatgattcattgttttttgtgcagattgtcgaatgcagtgctcttcccaagctcattctaatgttaggatcagaggatgctgctatacattatgaagcggttaggaatcttttactgggacgagagttttcataatcaactgttttgctagttgctactcaaacatctacatgagattcacactgaaataacgagttgagtcacgcttttaggttggagttatcggcaatctagtacattcttctccaaacattaaaaaagaggttctttctgctggggcgttgcaacctgtcattggtcttctcaggtgtgtggaactcgccgttttaattacatggttaagcatagagttgttactgttaaccctaggttcattctcatcattttttgaatttgtctattccagttcatgttgccctgagagtcaaagagaggcggctttattacttggacagtttgcgtcgactgattccgattgtaaggtactatttcattccgggttttctatcctcagttcgtttgccattaccccaaagtctaaactctttctgtttggttatactaggcgtaagttgtttgttgctattgatatttgtagaatattcgtttccaattactgttatctatcattttccctgatttatgtgtctttttcattcttcacctcattttcaaaaatataactttgcaggtgcacattgtgcaaaggggtgctgtccgtcctttgattgagatgcttcagtcacctgacgtgcagttgaaagaaatgtcggcctttgcactgggtagattggcgcaggttcttgtttcaatcatttgttattttcagtttataaagttcaggcattcttttttttggcgttgtaaacttgcaactccgctctttagacttacaaccatttgagttatattaaataacattaccgatatgtcttttaatttctagcgtaccctttctcgcaggattctcacaatcaagctggtattgcccatagtggtggtttaggacctttgttgaagcttcttgattcaagaaatggatccctgcaacacaacgcggcatttgctctctatggccttgccgataatgaggtgtgttgtatgctaccttccgtatgtattaattaggaatgcaaaaaaatatatttaaacctcattaaatgggttattgatccatttttgtcccctaggataatgtatcagattttatcagggtgggaggtatccagaagctacaggatggagagtttatagttcaggtatatatagcgtttttaccctttcactactttctagaatcatatcgtcttattccttgtatcggctagatactgaagattctttgcagctttagtagtctttgttttactctttgggtgtttataatttacactgctttttaggcaactaaagattgtgtctccaaaacactgaagagattggaggagaagattcatggaagagtaagtaaaattatacctgtctttaaacttgctctttccacatctggtgactaaaacatacacatgcacggtttgtggtgaaactgctatatcctggtctagctctgtcgaagtttagcatttctctatccaaccatttagacacttgttctttggttttcctttgcaggttcttagacatctgttgtacctaatgcgcatttctgaaaagtctatccaaagacgggttgctcttgctcttgctcatctctgttcaccagaagatcagagaaccatattcatagatgaaaatggcatgtgacaacttttttgaatttattaatgtctagatttttgacgtgttattcatttatgttaagatgttctttgtgcaaaaagttttatatcgagttgtcttttgacagggttggagttgctacttggtcttcttggttctacgaacactaaacagcaacttgatggcgctgcagcattgtacaaattagcaaataaatctatggcactttctccagttgatgctgctcccccttctccaacacaaagggtgagttcccttcttacttcagtcctccagtacataacttgtggaagtctcattgcagtattctttttgtgtatttgtgacaggtttatctcggagagcagtatgtaaatagtgccacgctgtctgatgtaacttttctagtcgaaggtaatcatcatattaatcaggaagttgcagcagtcttgttcgctccaaagtccaaatgtaaaccagaaaaatcatactgcaggaaggagattctatgcacacagaatatgtctcctggcatcttcagatgcatttcgcgcaatgtttgatggtggttacagagtaagttagctattattttttgggtgaccaatccttttcaatatgttcttgcggaggaaatgaaaaaatatcatttactagctatgatgacgatgacatattggttttggctgctctgcttctctttcaaaagaggaatatatggatagttatgtttcttgtgtgcaaattgaatatctcaggaaaaggacgctagagatattgagattcctaatatcaagtgggaggtttttgagttaatgatgaggtatgacgagcttctacgtgtttcttgactgtgggaactccttaacatacatgtaaaaatgtaattgactcacacttggattgtaattcccaggtttatatacactggatccgtcgacataacaattgagatatcacaagatcttctaagagcagcggatcagtatctattggaggggctaaagcggctctgtgaatacacaattgctcaggtgagccaggagacttgcaatttcaagtgatttggtttgcataataattgtcgaaatctaacagagttttgcttataaatgaaaggatataacgttggaaaacataggaggcatgtacgatctctcagaagcattccatgcaatgtcgctgaggcaagcttgtatcctgttcatcctggagcatttcgataaactgagcacaatgcatgggtaatataaataagctctctctctctctctctttttcagactacctctctctctctctctctatttggcatttatctgaaacaaagcgaatgaaaaatggcaggcaaaaccagctggtacagcgaacaataccagagataagagagtacttttgtagagctctaacaaagtctacgacaaacctgcaaggcctgaggctgtaagaagaagaagaatggtacctaactagagaggtaagtagacaaggaatatcatatagagagagaaagctcgctattagtaagaggtcttttatggtcttgtcctatcctgagtcgttttagtaaaatttgctgtgcgtttggttaattgtattttgtatcaaattctcttctgatcacaatcgcgtcttaaaaagagatcgccactttgtatccagaacaccaatatggtgaaactttcactattcaattcaagatccacggtccaacgatcctgtgttagaagcaaaaatacacactgtgatgattacatatggtattgactaatcgctacttgtctaaatgattaatcagatgacccaagacaggaaaatgaataatatttgttaatttttaatattatttgaggaaccgacgacatatacagtaataatattaatatcccgttttggctttacaactaaataattgaaagaaatggctgccattaggttattataaaaaaaaatagcaactctaatatttttggtgtttctgccggcagatatattttttttttaatttcagaatgtatatagaaaatgaaaggtatatagttataaattttattttttgaatatactcaaagagaaaaataaaataaatcaaaatgttctctttaccaacaccaaaagaagaaaaaggatttacaagtaccaaagtgaatgctttaatgctttatggtcacgacgtataattattattttatattctttttgcctgaatgcttttttatgattcagcgggagggagagggagaggagatttaatttaaaggagctccggtgagaaaccctagcaccctctcatttcgagattcacccactcctcatcgctcaggtacgctcttgcttctgatctcctcagattagatagatgcctcttctggaaactatccactatgcaatgcgatctccgatctttttaatcccctttattatagatttatgcaaagtagtgatttatttattattagattcgaatctcatgatccttcaatcaaatcaaagtctttctgctgctcgctacagtgtgattttgaattgaaaaatcattcctttcgtctcaaagttatagtctttgtttgattacagttaacaaccattgagccttgaatgtgtgtttgtgcagtgatggctgatacacttgattcccgacctcacacattctccatcaaactctggccaccgagtctacccacaaggcaagctctcatcgagcgcatgaccaacaacctctcttccaaaaccattttcaccgacaagtttggcagcttaaccaaagaccaggccatggagaacgccaagaggatcgaggacattgccttctccaccgcaaaccaacagttcgagagggagcctgacggtgacggcggctcagctgttcagctctacgccaaagaatgcagtaagatgattttagaagttctcaagaaaggccccgttgctaagactgaagaagtatcttctgcttctccttgtaaggaaactgttttcgatatttcgaaagacaagagggattttattgaggcagaggaggctgaggagcttctcaaaccgttgaaggagcctgggaatggttacactaagatatgctttagtaacaggagtttcgggttgggagctgcacgtgtcgctgagcctatcttggcctctctgaaagaccagcttaaggttgttgacttgtcggacttcgtcgctgggagacctgaggttgaagctcttgaggttatgaatatattctctagtgccctggaagggagcgttctctcgtctctcaacttatcagacaacgcgttgggtgagaagggcgttagagcgtttgggacgctcttgaaatctctgagctctttggaagagttgtatctgatgaacgatggtatctctaaagaagctgcacaagctgtctctgagttgattccttcaacggagaatctgagggtcttgcattttcataacaacatgacgggtgatgaaggagcggttgcgatctcagaggttgtgaagcgttcaccgctgctggagaatttcagatgttcttcaacaagagttggtgaaggaggaggtattgctttgtcggaagcacttgagaattgtactcgtatggagaaactcgatctgagggataatatgtttggcacagaagctggagtttctctgagcaagactctttcaaggttcgatcatttggctgaggtttacttgagttatctaaacttagaggacgaaggtgccatagccatagcaaacgctctcaaggactctgctgctcccattgaggttcttgagatggcgggaaatgacataacggttgaagccgcttcagctatagcagcctgtgtagcggcgaaacaggatctgaacaagttgaatttgtctgagaatgagctgaaagatgaggggtgtgtccagattgcaaagagtgtggaagaggatcatttgaaactgcaatacatagatatgagcaacaattacatcagaagagctggagcacgggccttggctcaggttgttgctaagaaagaaggcttcaagttgttgaacatcgacgggaatatcatatcagaggaaggcattgaggaagttaaagagatgttgaagaaaaccccggaggtacttggagcattggacgagaatgatcctgatggagaagaagaggaagaagatgatgaggaagatgaagagaaggaaggagaagggaataatgagttggaatcaaagctgaagaagcttgaagttaatgaggatgattaa

SEQ ID NO: 179 - DNA, 3844 bp, Brassica rapa
  source 1..3844: mol_type = genomic DNA
atggagagtcaacagaagcgccagcgaacaacacgcctcgccggaagaaacttgaggcgaaagctgtcccgggagacagacgcgtcgtcgtcgatagtcatgcagattacggaggtcgtagacgaagaagcaaatctcgtcgtcgcgatccgccgccacctcgaggttttgaactccggcttctcagatcgcgaagctgtcaaagaagctgctgctgctatctcctctctcgctaaaatcggtacactagtctccgcgattatgttgaaatggctagtccttagtttccgaacggctttggattgctcaatctcgtgttagatctgattgaatcgatacagattttgaattccacttgtcaattgatttttagattagttttatattctgtaactgtttgtatagatgaaaacgtggagatgatggtggagaatggagtcatccctgctttggttagatatctagaatcaccgtggtctttggcgattaatccaaacgttcccaagtcttgtgatcataagctggagaaagactgtgctgtttcccttggacttattgctgctattcaggtaactcaatctttcaactgtggatgagaagttgtgaatctcagtttctgtttattaatgttagttttatttgttacatagcctggttaccagcagctaattgtggatgctggggctatagttcccactgtgaagttgttgaagagacgaggggtttgtcttgggtgcatggaagctaacgctgttattaggagagctgctgatatcatcactaatattgctcatgacaatccaaggattaaaacaaatataaggtattgtttgttgtttgatgatccttataggttttggtcatgcctatgcttacaccttttgtaaaactttttttttcagggttgaaggtggcattccaccacttgttgagcttttaaattttccggatgtcaaagtacagagggctgctgcaggggccttgcgtacagtttcatttagaaatgatgataacaagaaccaagtatgttttgatgtgatgatgctttgttttgtttgagcttatgagaggcttgattcttacattaaaagaaaattgtgtagattgtggagttgaatgctttgccaacgcttgtattgatgcttcagtcagaagatccttctatgcatggcgaagcggtaggttcttaccttgctttagatggctgcagttggttcgctttgttcctactaatatacactatggatttttttttcagattggggcaattggaaatcttgtccactcatctcctgacatcaagaaagacgttatccgtgctggtgccttacaaccagtgatcagtttacttaggtatgctttttattgtttttctacttagacatttgcttctgaaatttttgtaatatgtttagtaactttttgctatctgctacagctccacttgtttagagacacagagagaagcagcattactaataggtcaatttgcttcgcctgattcagattgcaaggtatgggctagtctctttcatcgcatgatgtagtgtaatcttaacatatgctcagtcaaactcagtttcttttgacaatataaaaagattgatgcaaactagacagaacatgttaaacatacctggcaaaatgataatgcaggtgcacattgcccagagaggtgccattacaccattgattaagatgcttgagtcatcagatgagcaggtcatggaaatgtcagcttttgctcttggtcgtttggctcaggtacttatctttttgaattagcatgtgaatgttttcgttgcttctggaatctggttcgctatcaatgattgttaaatcataccttttatgtgataaaaatagcaatcctaattttgcttggtacatatcttaatacgccggtatattctcaatgcaatgttgcaggacacacacaatcaagctggcattggacaaagaggaggcatcatctcactactaaatcttcttgatgtgaatactggatctgtgcaacacaacgctgcatttgctttgtatggccttgcagataacgaggtaaactaagttcacagtgaataattttgaaacagctatgtcttttagtaactatacataccattgagtacctaaccaagatttttgtaaacaggaaaatctagcagatttcattaaggctggaggtattcaaaggcttcaagatgacaacttcaccgttcaagtatgcttttgactgcttatgttgcaaaaccaatctataacatttccaaattctgatttatattcttctgtctgcagccgactagggattgtgttgtgaggacactgaagaggctagagaacaaggttcatggacctgtgagtatctatttctgttagacctactggttcttatttaagtatggctttggttttagacccctgatgtcaaacccttctttcaggtactgaaccaattattatatctgatgagaaccactgagaagcctatacaaatgcgaattgctttggctcttgcacatctttgtgaccctaaagatggaaaattaattttcattgataacaacggtgagaatctcatttttcagaatttatatatttctgttgggttttactgtttctgatcaatatacgtattactaatgtaggagtagagtttctgttggagcttctatacttgtcaggcatgaaacagcagaaatatagttcaagagctttatttgaattagctagaaaagctacttcctttgcgccagaggactcagctccttcctcacccacccaacgggtaagaaaacttcatttttttttcaagtttaaaaactacttgtgatttgtggtcttgacttgtgattgactgtattactgaaggtgtttctgggtgcggagttcgtgaacaaccctactttgtctgatgtcacattcctagtcgatggtacaacatttaatcccattctatgtttctgttaattctacctgcggataacactttctaattgagtgtttccatggcgtattatcaggtaaacaattctatgctcacaagatttgcttggtagcttcctctgatatattccgtgcaatgtttgacggcctttacaaggtaagcttctgaataaatgatttgcatcatatagatagaaatcactcaactaacttgagaattggttttaggaacggaacgcccaaaacgtggagattccaaatataacatgggaagtgtttgagcttatgatgaggtaaagttctataaaatcaaacgtttgaatattaccaaacttaaaataaagaatcttagcatgaaaacacaaaatgtgcagattcatatacacaggaagaattgacatcaccaaacatttggctcaagagctgcttgttgcagctgatcagtatcttatcgaaggcctcaagcgcctttgtgagtacacaatcgcacaggtataatatataagcaaaaacctaggtcttattcttttgcaagttagagcgactactaaatggagtttaccaaatgttggtgcaggacatctgtgtggataacataccgttaatgtatgacttagctgatacattcaacgcttcagccttaagacgagcatgtactctcttcgttcttgagcattacactaagctcagctctgaaacatggtatgccatcaaattcattataattttgttttggaagttctagctttggtccccttttataactcaaataatgtttaattttattcttctgtaacgcaggtttcccatgtttatcaagaaaattatacctgaaatccggacatacatcacagatattctcacacggccagtccaagctagctcaaccgttgtataa

SEQ ID NO: 180 - protein, 733 aa, Brassica rapa
MKISKSLKLHRSNPPSNLLLVRRPSSISNLPPMENNLKRQRTTRVAGRSSKRGRETYAVSIITQITEIEEEETDLVVAISRHVDVLNSSFSDAGDVKGAAAALSSLAKTDENVEMMVENGAIPALVRNLESPWSLAISGNVAKSCDHKLEKDCAVSLGLIAANQPAYQQLIVDAGVIAPTVKLLKRRGVCIGCMEANAVLRRAADIITNIAHDNPRIKTNIRVEGGIPPLVELLDFPDVKVQRAAAGALRTVSFRNDENKNQIVELNALPTLVLMLQSEDPSVHGESIGAIGNLVHSSPDIKKDVIRAGALQPVIGLLSSPCLETQREAALLIGQFAAPDSDCKVHIAQRGAITPLIKMLESSDEQVTEMAAFALGRLAQDTHNQAGIGQRGGIISLLNLLDVKTGSVQHNAAFALYGLADNEENVADFIKTGGIQKLQDDNFTVQPTRDCVVRTLKRLENKIHGPVLNQLLYLMKTTEKNIQMRIALALAHLCDPKDGKLIFIDNSGMEFLLEPLYISSMKQQKYSARALFELATKATSFAPEDSAPSSPTQRAFLGEEFVNNPTLSDVTFLIDGKQFFAHKICLVASSDIFRAMFDGLYKERNAQNVEIPNISWEVFELMMRFIYTGKINITKYLAQDLLVAADQYLLEGLKRLCEYTIAQDICVENIPFMYDLADTFNASALRRACTLFVLEHYTKLSSELWFPMFIKKIIPEIRSYITDILRRPVQASS

SEQ ID NO: 181 - protein, 716 aa, Brassica rapa
MEQQRGSRSFPERKGQKRKLEEGPPAEDPQISPSTTTDAAPHAALLSEVAAQVSVLNSAFSWKESDRAAAKRAAQVLSELAKNADDLVSVIVDGGAVPALTTHLQPPPYCEGDLAQKPFEHEVEKGSAFALGLLAIKPEYQNLIVDKGALPHLVDLLKRSKDSSTSRALNSVIRRAADAITNLAHENSSIKTRVRLEGGIPPLVELLEYSDSKVQRAAAGALRTLAFKNDDNKNLIVECNALPTLILMLGSEDAAIHYEAVGVIGNLVHSSPNIKKEVISSGALQPVIGLLSSCCPESQREAALLLGQFASTDSDCKVHIVQRGAVRPLIEMLQSADVQLKEMSAFALGRLAQDSHNQAGIAHSGGLEPLLKLLSSRNGSLQHNAAFALYGLADNEDNVSGFIRVGGVQKLQDEEFIVQATKDCVSKTLKRLEEKIHGRVLRHLLYQMRISEKSIQRRVALALAHFCSPEDQRTVFIDENGICLLTGLELLLGLLGSTNTKQQLDGAAALYRLANKSMALSPVDAAPPSPTQRVYLGEQYVNSATLSDVTFLVEGRRFYAHRICLLASSDAFRAMFDGGYREKDARDIEIPNIKWEVFELMMRFIYTGSVDITIEISQDLLRAADQYLLEGLKRLCEYTIAQDITLENIGSMYDLSEAFHAMSLRQACILFILEHFEKLSSMHGQNELVQRTIPEIREYFCRALTKSTTNLQSLRL

SEQ ID NO: 182 - protein, 1296 aa, Brassica rapa
MEQQQPERREGRSFPERKGQKRKLEEGAAAAAEDREISASTTTDGGGDAILNEIAAQVSVLNSAFSWQESDRAAAKRATQVLAELAKNAEDLVNVIVDGGAVPALMTHLQAPPYIDGDLAQKPFEHEVEKGSAFALGLLAIKPEYQKLIVDKGALPHLVNLLKRSKDGSTSRAVNSVIRRAADAITNLAHENSSIKTRVSRLEGGIPPLVDLLEFSDSKVQRAAAGALRTLAFKNDDNKNQIVECSALPKLILMLGSEDAAIHYEAVGVIGNLVHSSPNIKKEVLSAGALQPVIGLLSSCCPESQREAALLLGQFASTDSDCKVHIVQRGAVRPLIEMLQSPDVQLKEMSAFALGRLAQDSHNQAGIAHSGGLGPLLKLLDSRNGSLQHNAAFALYGLADNEDNVSDFIRVGGIQKLQDGEFIVQATKDCVSKTLKRLEEKIHGRVLRHLLYLMRISEKSIQRRVALALAHLCSPEDQRTIFIDENGIFISSCLLTGLELLLGLLGSTNTKQQLDGAAALYKLANKSMALSPVDAAPPSPTQRVYLGEQYVNSATLSDVTFLVEGRRFYAHRICLLASSDAFRAMFDGGYREKDARDIEIPNIKWEVFELMMRFIYTGSVDITIEISQDLLRAADQYLLEGLKRLCEYTIAQDITLENIGGMYDLSEAFHAMSLRQACILFILEHFDKLSTMHGQNQLVQRTIPEIREYFCRALTKSTTNLQGLRLSFMIDASSGNYPLCNAISDLFNPLYYRFMQMMADTLDSRPHTFSIKLWPPSLPTRQALIERMTNNLSSKTIFTDKFGSLTKDQAMENAKRIEDIAFSTANQQFEREPDGDGGSAVQLYAKECSKMILEVLKKGPVAKTEEVSSASPCKETVFDISKDKRDFIEAEEAEELLKPLKEPGNGYTKICFSNRSFGLGAARVAEPILASLKDQLKVVDLSDFVAGRPEVEALEVMNIFSSALEGSVLSSLNLSDNALGEKGVRAFGTLLKSLSSLEELYLMNDGISKEAAQAVSELIPSTENLRVLHFHNNMTGDEGAVAISEVVKRSPLLENFRCSSTRVGEGGGIALSEALENCTRMEKLDLRDNMFGTEAGVSLSKTLSRFDHLAEVYLSYLNLEDEGAIAIANALKDSAAPIEVLEMAGNDITVEAASAIAACVAAKQDLNKLNLSENELKDEGCVQIAKSVEEDHLKLQYIDMSNNYIRRAGARALAQVVAKKEGFKLLNIDGNIISEEGIEEVKEMLKKTPEVLGALDENDPDGEEEEEDDEEDEEKEGEGNNELESKLKKLEVNEDD

SEQ ID NO: 183 - protein, 707 aa, Brassica rapa
MESQQKRQRTTRLAGRNLRRKLSRETDASSSIVMQITEVVDEEANLVVAIRRHLEVLNSGFSDREAVKEAAAAISSLAKIDENVEMMVENGVIPALVRYLESPWSLAINPNVPKSCDHKLEKDCAVSLGLIAAIQPGYQQLIVDAGAIVPTVKLLKRRGVCLGCMEANAVIRRAADIITNIAHDNPRIKTNIRVEGGIPPLVELLNFPDVKVQRAAAGALRTVSFRNDDNKNQIVELNALPTLVLMLQSEDPSMHGEAIGAIGNLVHSSPDIKKDVIRAGALQPVISLLSSTCLETQREAALLIGQFASPDSDCKVHIAQRGAITPLIKMLESSDEQVMEMSAFALGRLAQDTHNQAGIGQRGGIISLLNLLDVNTGSVQHNAAFALYGLADNEENLADFIKAGGIQRLQDDNFTVQPTRDCVVRTLKRLENKVHGPVLNQLLYLMRTTEKPIQMRIALALAHLCDPKDGKLIFIDNNGVEFLLELLYLSGMKQQKYSSRALFELARKATSFAPEDSAPSSPTQRVFLGAEFVNNPTLSDVTFLVDGKQFYAHKICLVASSDIFRAMFDGLYKERNAQNVEIPNITWEVFELMMRFIYTGRIDITKHLAQELLVAADQYLIEGLKRLCEYTIAQDICVDNIPLMYDLADTFNASALRRACTLFVLEHYTKLSSETWFPMFIKKIIPEIRTYITDILTRPVQASSTVV

SEQ ID NO: 184 - DNA, 4641 bp, Phaseolus vulgaris
  source 1..4641: mol_type = genomic DNA
cagatttccctccaattttgttcccatcttctaccctctgttttccttttattctttttatctcttctcaagattctatggaaaaccctaacactgtatcaagaggcttgaagcgtaaacctgaaggagatctaagccagaaccaatcagatttcaaggctcaatgcctctcgtcaaagttccgtaagaagattttacgtcaggtttctcttcttaattctactacctcggatcctcttacacttcagaaagccattcacaacctctccgtacttgcagaagatggtaccttttttttcttttgctaactgctttgatccgtgtctgtgctgttactgaattttttttttcattgcctcttctcttaaccagaggatcttgtggatactgtgcttgattgtggtgttgttcctgctctggtgaggcattttaaactgccagatgcacgaaatgatgataatagtaatataggtaaagactctagtgacagagttatcgatcatgaggagtgtgagatggccaaaggatgtgctctcattatcgagcttctcgcagtcaaagtaagtaaattatactatttttttcctctttagtaattaagcggtgtattatatagaatgatttgaagttagataatggaatatttgtttgttaatattttttgtcataggtttatgtgctaaagaaaaatgacttatttctaacataataaatgtagaaattattattgatttcctgatgttttaatatatgtagttttctattgaatatagaatgtcaatgcatcaacacaagggtatttatttttagttagttcttttaagataatataacatttagattctgatttttttttatttttatcttgaaacagcaagagtatcaggacctcatagtaggtgctggagccttgccttgtctagtagaatctttaaagaagcacaagatctgtactatttctcagccactcattaatcttctaaagagagcagctgatgcaataacgagcttagctcatgaaaatagtgatatcaagacttgtgttaggtatttctcttttttttggtactttcagtaatatatattttacaactgtatttattatacttatatatacctatggtatacgcaggagagaaggtggtatacctcctctggttgaattgcttgaatttggtgatattaaagtacagagagcagctgcacggaccttaagaactcttgcatttaaaaatgatggcaataaaaatcaggtagttatcttcctgcattcaattgatgtgataaatttggttgtcttggttgtttacaagataaaaaaattgcagatagttgaatgcgatgcattacctactcttgtactaatgcttggatcagaggattctaaattacattctgaggcggtaagatgcttgtattactttatatgattaatgtatttggtagtctgttgcttgcagagttctacactactaacgcaacttaattaacgcttgttgtagattggtgtgattggaaatctggttcactcttcgccaaatattaagaaagatgttcttttagctggtgctttacaacctgtcatttgttcacttaggtatagttgtacttcagtcttgggttttcctgttagaaatccatagacgaatgatctgtttattaaacattattgttatttgctgaaagtgagtcattactttattattagtatttagtaatttggtacttttccttctgagtaatcttcgctagtctataatttcagttctagttcctattgttcggagagcagaagagaagcagcccttttacttggtcagtttgccacaacagattcagattgcaaggtggattaagtagttttgcaaacttttaatatgatttatcagtcagttataaagtctacttgttgactttcgtattttgtggttcatacaggttcatattgcccaacgaggggctattccaccattggttgatatgctgaagtcttctgatgccgagcttcaggaaatgtcgtcttttgcacttgggaggttggcacaggtgattattagtagcaacaaacatttagccattttcttataaaaagcaatttagaattgaagaatccaaattgaatttactttgccattttctatcataatctattatttttgctcatgtcgttcaaactttaggactcgcataaccaagctggtattgctcaaagtggaggtatagagccattacttaaacttctcgactcaaagaagacgcctgtccaacaaaatgttgtttttgccctctatggtctttctgataatgaggtgaagttaatctccttcttttctccgccaacaatgtttgttttcctttaggaatcattgatgcttagtgataatatgatatgctgtcgctgatgtaacaactttttatgataggacaatgttgtttgtattattaaggctgatggttttcaaagactgaaggctggaaatttcaaaaatcaagtatgttcattcattcttctgtgataaaagtgataaatttgcacacaactctctcatcaactgtgtcttgtgattgtcacttaactggcagcaaactgtagagtgtgccatgaagacgttaaaaagattggaggaaaagactcaagggcgagtgagttttcttacaaactctttgcgcggtgacttgtaatgttttccatttgttttaatgttactggattggatacgttttttttttatatctattcctctttggcaggtgttgaaacagctaatacgtcttatgtgctaccctgaagaagtggttcaaagacgtgtagctattgctcttgcatatttatgttctcctcgtgatagtaaaactatattcattgacaacagaggtaaataattgttctctgcattttttttaatttctcactcacagtattgtacacgtattcattctgtacggctctaaattttcaggattaaatttgctgctggacatgcttaaatctccaaacgtaaggcagatgagtgatgcttcggctgcgcttcacaaattggctgccaaagcccattcttccgttgtctccctttttgaacttcctcctccgtcaccaagtcctcaggtacttttctcttcacaagcgggcttaacacatcataaatgcattatttgaattagaatagttatcgtctttaaagttaaatatctgatattttgctgtccatatgctgaggggtgaaaatgggatgttgacgttttctttctctcaatatttttgttaacgaataatatttctgtaggtgtacttgggcgaggaatatgtaaacaatccaaaactttctgacattacattcctggttgaaggtggagtatctgctgttaaattttctccagctattaattttgtttagtttctatgcacactgatttcgatatatgtactaatttactttttttttctttctttcaggtagaaccttttatgctcatagagattgtttagtttcttcagacatatttcgcgccatgtttgatggcagttatagggtaagcattaatcagttgttattgtgctttattttcaagtcctcatttttttatttgttgtggaatggtgtaaaagaatttcatcctttcttgtaaaaaggtcacataccagctgtaacaattaaaatacgaccaggggatctgtggaactgaaatcgtcagttaggtgaaaatatccatattaatgtaatgtcttgcaaattgtggtgcaggagagggaagcaaaaaatgtagtgattccaaatataaagtgggatgtctttgaattgatgatgaggtgcattttcagccatcttttccttttgttttggtaatatcacaactaattttacgttgaaacttctagatttatatatactggaacggtagatgtcagtttggatatggctcaggatctcctcagagcggcagatcagtatcttctggacggtctcaagcgtatttgtgaatatgctattattcaggtacaccaaaactctgttttgctcttatgaatgtttttctaatggcttaatttcatctcaaggctaaccaacttaattttataggaaatatcagtggaaaatgttgtaatactgtacaaggtggctgaagatttcaatgctacttcattaagacatgcatgcatactgtttatgttggagaaatttgatgtactgagatctgaaccatggtatgtttccatttttacaacctgtacagtacttccattctttaccatgtttatatagagggggtgagtaactttcatttcattcatcattctattatatcttgttttcattttttcaatatgcaggtattgttccctggtacatcacattcttccaaatatatgcatgttcttctctactttacttgttaagtctcatccagttgacttgtgaggattcctagattgaaccatgaaggaggaaaggcgaaaatgtacagagctgtaaatgttagttggatatagaaagctcagatcattctttttttagggtatgaagtggggaatagtgattctgttgagtaacttttaatttatcatttttacagtacatgacttcaccttaatgaaaccttcgtaatgatcttgtctttaaggatctcctattgaaaggtggc

SEQ ID NO: 185 - DNA, 9168 bp, Phaseolus vulgaris
  source 1..9168: mol_type = genomic DNA
tctcttccgcgcctcgtttctaacactttgggttgcgtctcccaaagacagagggaccttctccttcttcttcctcttctccttcttttctcgtccatggaccttcacgcgcgaccagatcactgcctcccggagaggaaaggtcagaagaggaagctggaggaggatttcgaagacgaccgacagatctccgcgcctcccaccggccacgctcgggacgccctcctctccgacgtcaaggaacaggtcatcgtcctcgattccaccttctcatggaaggaatccgatcgtgctgccgccaagcgcgccacgcacgcccttgccgatctcgcaaaaaacggtaaatctattcgtcctctggcttccttcgttttcgttttcttctttcgcggaattcggttcttcgctgctttcgtccgttgcaccgcacgcgcttcattcggcgcttgtctttgtttgcagaggaagtggtgaacgtgattgttgaaggaggcgccattcctgctctggttaaacatcttaaagcgcctcctctagtcggaagcgacctgttgcagaggccaatgccgtttgagcacgaggtcgagaaaggaagtgctttcgcgcttggacttctcgcagtcaaggtaattttacttctcctctacggtgactgttagttaggaattattgcaacttagcttcttcatgccttgaaattgacaagctctgaagtctatataattcaaggttttaattccacgtctgttatttgtattgtgatatagattttacgttgagttcgcttactagtgatagttatctccttttttaaaacgttgtttatgccaaaaattgttttatcttatcgttttcaccaaacggcgtgagcgattctttttaggatggtatagttgatactgtatagtagaaggaagctttgaagataatgcatgatggtctaatgtgtggtgtgaaaatgccttctgcagccggagcaccagcagctcatcgttgacagtggtgctctaaaacatctcgttgatcttttgaaaagacatgaaaacggcttaacatctcgtgccattaatagtctaattcgtagggctgcagacgcgattactaatcttgctcatgagaacagcagtattaagactcgtgtcaggtatgcttcttcgagtactaccatgcaattgaaatttaatttggaatggtttattcttatgattatctggagttaatgtgtaggatcgaaggtgggattccaccgcttgttcatttacttgaatttgcggatacaaaggtgcaaagagcagctgctggtgcattgagaacccttgctttcaaaaatgatgaaaataaaaatcaggttagtggtctttagggaatgttttgggaatttaaattgacttacatatgatacgagtaagtcacgtaacgtaacataatgacatgtagatcgttgaatgcaatgcccttccaactctgattctaatgcttcgttcagaagatgctgctattcattatgaagcggtattacttgtgcaaccttaattcttaagttaaattttgcaatagtgttgactttggtctttgtactgatcttactgggaacttgcaatgaattttattgaattacaggttggtgtgattggaaatctggtccactcttcccctaatataaagaaagaagttcttcttgctggggccctacaaccggtcattggattacttaggtatattcttacttcgcaccctggaaaactacgctcatctcccttcccccatgtttcaaccctgcacttaatttgtttcactattataactcaaagttccttttttcattccaataattttccgtagtatatattactgaaaaagatgtctttctatcaacctattctaattctaatactgtatgatgaaacagctcctgttgctctgaaagccagagggaagcagccttgttacttggacagtttgcagcaactgattcagactgcaaggtaagcattaactttagtttttctaataactccatgattaaactgaatcgtgagggagagagagaaaggcataaaggaaaaatcctaacacctgtttttatgtttgtttattggatggtgaaaaaagtgatgtgaacaattttatgcatggatttttagtttggattctgaaaagtgctcaagcatttggggaaccaaccctttgaaagctagccattaaggagggagagtcaaacacttaaatacctccttgagcatcctatactacttgttgcaaactaaggcatctcataatatccaaattcctatcatagcactgcccctaagagctgaccagttagtactctctgtctgtagccctttccaggatatcggcaactagctctaataccaattgataagtacccatgttcttgggaaactgatgtgatttggaaaataaaaataaatgtgtattttctttttgtgaataaacttgttatccttagtatttgtatattctctgtttttgcttatctaatggagtttgagtggcacaaagggttgttctaattcctatcactatcttgatttttttatattattgaatctgtttcttttccatggcatccgcaaaattgaagatcacattttatataaaaattcttcaaagaatcgtttcaagaattcatccaaaagtttttccttgaagcttgagtggaaagatccttccaacccaggcaagcctccctgggttttcatcagaaacccacctcaaaagctagctattaaggtgggagaaccaaacacgtaaatacttgatcaagcatctcatactgacttaggcacctcctaatatgctagttcccatgagattctttctttaacttatttctgaatagggtggctcagtgggtgttaactcatcaactctttgtgtattatatatctctgtttttagttttacctttcgtattgtttgattttgtaggttcacattgttcagaggggtgctgtccgacctctgatagagatgcttcagtcccctgatgttcagctaaaagaaatgtctgcctttgcattggggagattggcccaggttatttcttttcccttgtcttttccatgtcagagttcaaatatgtaagttaagaggcatgatttaatgttacatttcctatttatagtttttaatcggtaatggtaacatatatattatacaaatttccatgtgtaagtattatagattatatactcggcaatggagttaattttaagttcgtcattttagtttaaaatcgttaacgtaaactctgtgcatttccatgtcttaagttttgtattaatgtcttatctcagaacataaaagtcatctttctaatatgttgtattacttacagctttataaaaaagtgttatgcactttttctgagtatgttgaatcactgtttccctttaacaccataacctgtagatattcaattttaattttcaggacacgcataatcaagctggtattgcacacaatggtggcttgattcccttactgaagcttcttgactcaaaaaatgggtctttgcaacataatgctgcttttgctctttatggccttgcagataatgaggtaaaataaactctacgagttctaataaaatatctttcttgactgtagtaaagcttattacttgaagttaaagtaaaataactgttccttttttatattttttactttgtcccataggataatgtggccgattttattagggtaggtggaattcagagactgcaggatggagagtttattgttcaagtaagtttgccttgttgataccaattctgtttctcggtttctcggtttcatggtttttgcatttgccctttgttgcctatatcaatgggagttcagtgctttatataattgcatacaaattttatgttcttaggcacacactaagagataaggaattggtttctcttgcaggcaactaaggattgtgttgcaaagacattgaaaagattagaagagaagattcacgggcgagtaagcaccacttcacattcacttgttctttggtacattttactgaaattagcttggaaatggtagggatgctactactgtattaattattaattctacaacaatctagccttatcccaccagtttgaattctacatgttgttcagatctgtaacgtattaattttgcctttgtaggtgctgaaccatttgttatatctcatgcgagtttcagagaaggcttttcaaagacgagttgctttggctcttgctcacctttgttccgctgatgaccagagaaaaatatttatagaacaccatggtatgcatcttaataaaatattttgctttagtttgatgtatattttttttaaaaaaaaattaaaacctttttctgtgtttttttttgccttttctattctatatgaatccaagcatctgtccatgcaggtttggagttgcttatggggcttcttggctcttattataactctaagcaacaacttgatggagctgtggctttatgcaagttggccaataaaggcacgactctgtctccagtagatgctgcacccccatctcccacaccccaggtaggcatatataattgttggcttgttctcatccttcatagcatcattgctaaatgattgattgccttttccaagtattttgatttgatctgtgttttatttatatatgatgcttttaggtttatttttctttcctgtccttttcatgatgatatatgaaaaaaatttcctctttgttttgatttttttccttgttatatttacaagatcactgtgtacacaccaacatgcataataaggcaggtattaacagtgtggctaattaatttttcaaatcctacatgataagtaagcaaggacatttgtaagcttaactgttagcagggatgtaatcctcaagcttaactgataaaacaccctgcttagaggctggtcctaccctatttaagctattgggcatggatgactgggctgaattgacccaataatccatcatgccctctcatgaccctttgtgcatataattttcactcttttagaggatctctgtccttgaacgtggagataattggaaacttgttaaacctgtaatttgaatctgtatgaattatgaaaccaaatgattgactaagaacacttactactctgccaaaagctttagttgttgggattggcacaactcttgacatataaaaccctgcataacacatgggctcttgcctgtttagccattgggcatggacccacaacccttagcacgtatcaaaaccaacaagattgttatttaaattttcatctcacctcttctcatatagtagtcaatggttttctggtttgcattttattttgacatgtgatatctcttggtcatgcttacctgtatcatgatttgcaatacttaagctgcacttgtttgctggtagtgggttgagaagggaaatgaccacaaccctaaagttaaacgacaacttactgcattcatttctttcatgctaggaccttttatatttcacttccaagatttttactttgggccataagttatctgttggaccttttattcattaggacttcctaatctctttttataaaaatatagaggaaaaaaacagaagtaacatctagatacgttataatcgaattttattttctaatttaaactgagatattttctaaccatgatatttggaaactaaaatacatgttattttgaaacttatatgttgctttgttagctatttaacttcacaatgctgcacacacattatttttatatgtttctgtatgttaaatgtctgtccgagctatgttttatcagtgatcatgaatctaccaattcactacttgaaaaattttgtttcacgatttgtatcccaagtcaactaccatatcttggtgtttaaaattgattcagatattggggatagtgtctagttataaatatatggtctgtttaattagttagtatctgcttctgtggatccaataatctgtagtacttgcatatgcctaaaaagcctaatgcactcattgactgcttactttctgtcttgtcttgattattctgtatccgtaaggtatttttgtaagttttaatgcctgtgatgctagacttttcttcttgcaggtctatttgggagagcagtatgtaaacaatgctaccttgtccgatgttacatttttggttgaaggttgatgttttttcattaacactgttttcttaaagctgttgcttggagaacaattcacctagaatgcagtgctgttgtagctgcagtttgcatttgtagataacctggtattttccatactttgctgcaggcaaacgattttatgctcacagaatttgtctgcttgcatcttcagacgcattccgtgctatgtttgatggtggttatagggtgagtatatattgatcttaagtgtatcatatgtctctcactgttaatagactatcgggcaaaaaaagaaaactgttattggctccacgatatcatgataagcatcatgtataatctatcatttggttagtaaatgtagctgttggatattttagacatggtaccctgtgcctattcttggatctaaataatcatggtaactaggcaattaggatacttgtatctaataactcatttcttaaccttattatataatagcactccctgctgtctaaattgacagattcaattatgtctcttgttttcttttcctctcattctcaacaatagcaatacaaaattacatttcatatctcagcacaataattgtgatacgctagtctattattgtatgtcaggagaaggaggcacgggacatagagattccaaacattagatgggaggtttttgagctgatgatgaggtcaaataaattctgcattcacgtgctttatgaaagttgtgctgtgaaaacttgtaataattgtgaacaacttaattcgtattgtctttaatcttttctccagatttatatacactggatcagttgagatcactcttgacattgcccaagatctcctccgagcagccgatcaatatcttttagaaggactcaagagactctgcgagtacacaattgcgcaggtcagctaagagaattttggttcacacataaatacacatagtctttacacttgtccttgtgctctactattagactggaaagtgaatttctcttatttgatgttttggtccaggatatatcacttgagagcgtatcaagtatgtatgaactttctgaagcatttaatgctatatcgttgaggcacacatgcatcctttttatcttggaacacttcgataaattgagtggaaagccagggtacgtatctgatccctctacaatgtgtacagatgtctgtaataagtaaacaaaatctaaatggaataaatgtctgaatcatcttttataagctggaggttttatgtcagttgtatctactttctatttctctttattttccttgtagttttggcaggcttgtgtcaacctaaaaggagttaagatattgaaaatttgaatctacttaaaattcttttacatgactaaataaaaaattcttttacatgacttgatttcatttctctttccattttaataaagctctatttcatttagaaagcatgctttcgtgttatttttattagtattcatttgcgaaatgaagttgacgttttatatatagttatcaaaaatatgaaaagctgtgggcttacccttttttcagagggcgggttgtgatttttgttcaacatgttgctgatctttctttctttcttttttctgcaagttgctatattcttaggtttgtttgctttttgacaaatatgatggtcagggatcttaaactttgttacacaatagatgccgacctttggtttgaaattaattgaataattaagctttggccggataaataaatcacagatatgatgaatgcatttcattttacatttctatgttctgtctttctaaccttttagaatttcttttgtaccaattatttgcagacactcccacctgattcagcgtataatacctgagattcagaattactttggtaaagcccttacaaagggcatttcctacaatcagccgtagaatttactgttctatttgacatctaaccagttgcaatgtacataatgtggtcgatgttaattgaacctgcgaaggaagtctcctggattgagtgcagcatggcttaaaaaatatttaacatcaggtcgtgtacgttcttttctgattcagtgtaagtccttctaggctctacctgtaatgtcattctcgtagatgtagcaaatgaccttcacgaacattgttttttctcgtgcaatattgtgatggttatgatttgatagtgttcattttctcatttgtttaggcattataattgctgtatttctgagagtagtataggttgcccaagcacctcatgtttatatgacaattaaatatttgtctgtaatgtgctgatgattaattgcaaatacatgtagctttaacgcaaattaattgcaaaatgcaaatacgtcgcaaatgcgtcattggatactcagttactcgtttgaccatgataaaattgaattcagtgctgcttataaaattgactgtatattcaatgaagtgaccatgctgtatggaatgaaagacacctatatccaaatgaaaaccctctcacaaatcagtggacaaccaaaatcggctaaacagcttatgatgatggtctaagagaatcttttataatatagtgatgtactttgaccaatcaaaacatatgaaatgaaaattgaatgtgtcgtctttgtctggatgtatcagaacttctggtgagtttttctgtgggcagatggaaggtcttgttgaaaaggggctttgattgttatttttgaagacaaataaaagcattgaactgctttttccttgggcatcatgtgttaccatcgaggaaaaagaatcccctcaagtcactcccaacggtgtactttcacttggaatgggccaatcggctgaactcaagtctttttattatacttgtttcatgattagagtagactgcacgtgcatgagataggtatgtcttctgctttggagggtttgtatgccagtatccgtcaaacatgagttatggatatactaacttaattcac

SEQ ID NO: 186 - DNA, 4066 bp, Phaseolus vulgaris
  source 1..4066: mol_type = genomic DNA
atggattccagtgccagacaaagcttgaagcgcaagttagcggaagaggtgaaggattctctctgcaagcgagttcccccaactttcacttccattattcttaagactctctttctcctcaactctttcgatcacgttcttctcaacaaactcatcaccattcttgtcaaactctgcaaaacaacgaagcatggtacatatttttctctcacccttttacgtaaacatgctgacatgaacaccctttttcgccttctcaccaaatttcctttctttcgcagaaatccatgacgattttattgatattttggtgaataacggtgctgtccaggctctggtgaggatacttcacctaccggaaaaggttgtggaagattacagtgacagacttatccaggctcgtctcctccaactgaaaaaagggtgcgcgttcatccttggaactcttgccaaaaaggtaattaactaactttctgctgttaaaagaaaaatcagaaatttcatttttttttcttgttgtgttaataacgaagcatcttaactttttgtctttatcatccagtcggtttatcagcaacttatcatagatgctggagccttcttgtatcttctgcgcttgttaaagagccacaagacgattcccaaatctccatcagttcctggttttctgaggagagtggttgatgcaatatccaagcttgcttacaaaaataacaaagttaaaatgcttataaggtttttgtcttcttcttttcttttctatttttaaagatatgttttctttaattattgtattcactgtgcttgtataaaattttccatcatgtttagaaaggaagatggcatcgctcctctgattgaattgctcgaattcaaggtgaaaaaggtgcaggtcgcggttacaaatgccttaggaacattggcatttgataatgctcacactgtaactaaggtacttgaatttagtaaattggtttgatgaaggtttatgtggttacaagattgaaaattgcttgcagatggttgaatgcaacgcattacccagtcttgtactaatgcttcaatcagaggattctgtaacacaattcacgacggtaatatgattttattatatgtattttgcatagttctaaactactagcaccagcatcttaattagcactgttttgtaggtgcaactgattaaaataatggtagacacttcaccgcatattggaagagaagttctaaaagctggagctttaacacctgtcatctgtttacttaggtaaaacattatactttggtggtggttttctgtaagaaaatcatagaagaatgatatgtttattgaacattttagtagtttgttccccgagtagactttcaatgtttgtaatttcaatgacagttcctccttttcggagagccaagcattagcagcccttctacttggtcactttctcgggactgattctgatttgaaggtgatttattttgtgttgcatacttgtaatatggtaaatctgagtcatgagtcattaaaccctgttattaagttgcctactttgcttgtgtttcatgcatgcaggttcatatttcccaaagaggggctattccaccattagttcacatgcttcagtcccaaaatactaaccttcggaaagcatcagcttttgtacttgtgatattagcacaggtgattattactagcaagtaccaaccatcatttggccctatgcttacataagcaatacaattcaaactgatttcttttatcatcattttctaccataaccataaaccttttttgcatgaacaattcaaatggtaggactcacataatcaagttagtattgctcatagtggaggtatagagcctatgctcaatctttttcaatcggacaatccaacagttcaacaatatgctgctcgtgttctctattctcttgctgataatgaggtgaagttagctccccttgttctttattttggtcaactttgtatgttgcccttcagaaacaacattgatgtgcattgatattgtcataacataaaatgttttgtatgtgtgataggacattgttgcaaacattattaaagttggcgggtttgaaaagctaaaggatttacatttcaccgaggaagtatgttgatttactcgtctttgtaattgaagaaataaattttcatttcaacgtatttactcctatttcttcctcttgatagatatttgtaataaatgcttgctaacagaacacttttctctccccaaatttccttgtgatttgcagcctatcagcgagtttgtagcaatcacgttgttaagattagaacgacacatgcaagggcgagtaagttttcttgataattttgtctcaatgaaaatcatagatgacaatcataatctgtttaaactttgcttattcctttttggcagacattgaaatacctaatccatcttatgtgttctgcggaagaaagggttagaaatcatgtagttattgctcttgctcatttatgttctcctccagatcatgaaactgtatttattcacaatgaaggtaataaacgttctataaagttttgtttcctaatttctcactcactttattcggagtgcattttcaaacaagatgctgctaaatcttcaggattagagttgctgctgaatattcttcaatctcaatgcacaatacagaagcgcaaggcttcaatggcgctaagcatgttggctagtagagccaatttcatttcctctctcattcagactatttctccatcaccaacttcccaggttttttttcactctttatgtgtttccttgccacgtttgtttactttgatttgttttccttattcattgaatcatttgtcttaccctattgtctttgaaatcgaattgtttttactgccttcacagtaatgatgttgttgcttttgatgtagatggacttgggcgaggaatctatcaacaatccaaagctttctgatatcacattcctggttgaaggtggagcatctactgctgttaatttcggttaatgcacactgatttcaatatatatactgatttactgcgttttgcttcattcaggaaaaatattttatgctaataaagatcgtttagtttcttcaagtgtatttcagaccatgtttgaggcagagtattttgtaagcattacttaatcaaaattgtttgtcctttccttctcaatgaatttattaccttaaacacactatgcaaatatctcaatcaaatagaaactaatgctgtaattggttgtccattcacttgctatcttcaaactaatccacaacaataatttgcaattagaaagggacatgtacagaacttaagacttatgaatgtgttatgatgtgtggtgcaggaaaaggaaaccaaacaagcagtgattccaaatattaaatgggatgtctttaaattaatgatgaggtacattttctgctatccccttctttcgtgcttctgtaacatcaaaattggtcttctgtttgacctggttttggttgacacttgcagatttatatacactggaacagtagatgtcaaattggatgacgctaaagacctcctaagagctgcagatcaatatcttcttcaagaccttaagcttatttgtgaacgtgttattgctaaagtacactaaaaactgtttttcacttttcatttcttttgtttttgtagaaagctttttcagtgaactccatgactcatcaaccttttctttcagagtatttcaccagaaaatgtttcgctattgttggatctctcagaagatttcagtgctaatacattgaaaaatgcatgcatactgtatatgctagagaagtttgatagattgcattcaaaacgatggtatgttccttttttactacttcaacttgaatggcatcaaaattaaccttcatcaatcatttgatcatgtttgtgttcttcatcttttcaacctgcaggtattataccatgcttcatcgcattgtaccagacatagatactctcttctcaactttacttattatggatcaaagcaatgaagatgcttctgttgcatacttgtattaa

SEQ ID NO: 187 - DNA, 9091 bp, Phaseolus vulgaris
  source 1..9091: mol_type = genomic DNA
tcaaatctccaattgcatttctcaccctctcttttctttctcgcaccagacagagcaaacactctgttctcagaaccttcctttgctttttctctcgttcatggagctccagaggcgccaggatcagagtctctcccagcggaaggggcagaagcggaagctcgacgatgaacatcacgacgaggggcagatctcggcggcgccgcccaccgccgacgagcgagcggcgctcctctacgacgttgccgaacaggtgagcgtcctcgagtcgactttcacgtggaacgaagtggatcgatccgcggccaaacgcgccactcacgcgctcgccgatctcgcgaagaatggtaaatcgatgcctccgatctcgccgtgtgtcgctgtgttcgtttggattgcggttgcggtgtgctgtttcttcttatgtgtttcctcgtgtcggttgcatgtccgtgtgtatgaatcaattcgtgcttgccggttgtgtttgcagaggaagtggtgaacgtgattgttgaaggaggcgcgattccggcgttggtgaagcatcttcaggcgccgcctctggttgaccgtgtcgagaagccattgccgttcgagcacgaggttgagaaggggagcgctttcgcactaggacttcttgccgtcaaggtgatttcatttccctctaactgttattttcgattctattccatacttaatcgtctatacatcgtaggtcttagcttgttttagtttggtacttcataatttggatagatgttccttcgtgttttgcgaatttggaagtatgagtgtgatttcggctgtagtttgattccaagttttgtaatgttcaattcgcttttgagtgttgattatttatttatgcattttaatctgtaatgctgtttcattattttttgtttaatggtgtgcgagtgatataatacttcaagtgtttgcacttttgaaagttttttggtttgtatttaactgacatttcaaagttcaacgcaatatttttttttttcatttatactcttatctatcgcttaatatttaatttgtttacatatatgcagttatagttatatagaaatgaaaataaatattttattcaagttaaataacattgcatttcttgggttatccagaaaaggtctaaaaaggaactaagggagtaatagtagagccagtgtcagacatcatgcctgatgctgtaatttgtaggttgggtttgctaaataagtactccctttaatcatgtttaaaggacttaaatataatcaaattccaatcatctcaattttatttaatgttattatttaaaaaatatccttatatttaaactggggcaccaatttccaataattatgactggtggtagtttgaaagatgtatttattttatgaaattaagaacgttaaatgaacttaactaagattcttaattagtgtttgagtctagcatagtactttctggtctttaattagcactatcacagaccaatgaaagtaattagttcagctaaattttttaaaacatgttaccagtgtaccttctaaaatgaaccttataatgaggattggatggagtgtttatttatttttgcaggatttattacgatgtgatacaatgggttgtttttgtgcatgacacatgactctgtctagaatcttaagaatcgtgatttgctgttcaatcacacctcagagccagcaaatcccgcagcactcttagtagttaatcacaaaatcggatgttgctgcccctccaagggtcatcttgttgcccttggcccccacactccaaacctacaacttcattgcttcagttcactgtcctgctctcatggctgtgcatctttttagtgggtcagagaagagagatggcccatttacagccctagttctaaatgacagtgtcctaggtttcctttttactttaagtaacttttgtttttatgttctagcacaagacaaactgtgtttggccttgggatgtcagttttaacattgttgtttgaactgttaattttttaattattggacctttattcatgtaagacttttttttttatctcttttagtcagcacttgtaaaaataaaattaaaaacgtaagtttagcactataataaagttgtatattttgattaaatttaaatagatatatttttcaaataagacatttcagaaactaaataaaaaagcttagttatcgatcatgaacttgtgcttttatgtcttttagcataaaaatatcatgttttattattgatcatgaatcttattattcacggtacaatttgattcgtgattcgaaaattagatgatcttattcacattttgtttctcgattcaactactatggagtccagaggtagtaccatttgatgtgtatcacgtggaattttggacgccataatcttcttgaattgaatggagttatttctgaatatacagtaatttgtgtgtgtgtctgttaaggtggagaacagaaatgttggtggtttatactatcatccactttcagttctgttctgtttcattttgcaagtactgtttcttcatggtatcccattctaaagatggggttcaattaaaacaaagagaatagaagaactgaggatgtgaggccaaagggtttagcattgatttaatataaccatactgttatttgtaataatgcttatggtttgtcctcgtgcatcaattccataatccatattaaattaagcacctgctggttggtaggaattatttatttataaaagattgagcttgtctgaatgcaatctggttctctcaaagcttgttgaattgccctttccatacactgctttgatggtagtcagcagtggtggaacttggctgaagattttgataggacaaaaattatagggtttatgtgcataagttagttagtgggggaagatgatgtgccaattcttgaaaactgtgggatctgctaattttatgatattacgtctgggctttggatactttagaagaagtattggatggaaacttgtttaaaaaatttaaatgatcaccaattgaatcaaattcaatatattggatgaagttagaagtaaggaagggatgttcttgagcattgtacttggtgcaaaaaccattagatttaatagaaagtcaattcgtggtgggttgaattcttgtgaaattcttcatcagagcaaatgtcccacatagattcacaaacaaataaattcgggaacgggagatggggggattgttccctttggtcctgatgaagatccacccttgaaagccagtctagcctactaggtccgtagtttttgtttgtaaccgtgggagtgtgtgagatactactgatttgatttctaaacggaaatttatgtatcctgtttgtcaattacaagattaatttagtgttggttgtcggatgtgaatatagaagcactgcccatctcctttttttgtaactatggtgaagcccaaataactaggactgatgactgtgtcatgtttgagtggagtttgaattgtgtgtgtgtgtgtgtatgacaatttcatataattggatgcaatttttagatttacttgtacttttctcgtctgacatatttcttttatctgttaaaaagaatattatttctaaactactattttatttgaaatgctttctacagccagaacatcaacagctcattgttgacagtggtgccttaatacatcttgttgatcttttaaagaggcacaaggacggcttaacgtcccgtgctattaatagtcttattcgtagggctgcggatgcaattactaatcttgctcatgaaaacagcagcattaaaacccgtgtcaggttttgccttcttctaaggttagcatatttaaaatttagtttggatttgttcttaatattattatcttgacttgatctgtaggatggaaggtggaattccaccacttgttcatttgcttgattttgctgatgcaaaggttcaaagagcagctgctggtgctctacgaactctggcttttaaaaatgatgaaaataaaaatcaggtaagttgttgctgaaagttgagctttggatattttacaaacaagtcacacaacatgatgattttccagattgttgaatgcaatgctcttccaactttgattttaatgctacgttctgaagacgctgctgttcattatgaagcggtgagggtaacgaaacctttaataataaatgcaagattttgcaataattttcagctctttgttcgcacatgtcttatgtggcacatgcctatgaaatggattgtatatcaggttggtgtgattggaaatctagtgcactcttcacctaatataaagaaagaagttcttctcgctggagctttacagccagttattggattactcaggtttatcctcaattctggaccctgataaactgcaatgccctttccctccctaccctgaacatgttttgtgattattatatgcctattttttttatggcaataacattctagcaaatgtgctcactgaaagatatcttccaattaacatatataatgttttactttatttaacagttcctgctgctctgaaagccagagagaagcagccttgttacttggacagtttgcagcaactgattcagactgcaaggtaagcgtaagcttcaggatgtaaaggacaaaagcaaaactttaattgggtggataactccagttttcaagtttaaattgtttaatattacacacaaacacatataaatagttcccttttatgcttgtatgcctgaatagtgaggagggggagataagaaccaattcataactgaactttagttgaagcaattgtctggtgacatccccatttccaatttgattgttttgtattatttatttcttgttaaataagattcaatgatagtagagtactgagcagtatagttgctactcttatgatgtatcatatatcatattctgttgaccttagtttttactgtttgtgctgcttgattttaggttcacattgtacagagaggtgctgtccaacctttgatagaaatgcttcagtcatctgatgtacaactcagggaaatgtccgctttcgctttgggaagattagcccaggttattacttttctttttttttcccctttataatttacttgcattagtttggaatataaagttgccattatatctttggaaataagttagttgtatctttctctgctggatagcatttggatctttaacacattcaatgcctttccatgttctcattagtcctcatatagttatgtgtggcttatctctgagaatggaaatcatcttagcgatatatcacacctttttatataaagctactatgcacctgtgtccatttataggttgaattggtggttctttcttttggctgaatataaatttatacgtttttgctgatttcaggacacacataaccaagctggtattgctcacaatggtggcttagtgccattactcaagcttcttgactcaaaaaatgggtctttgcaacataatgctgcttttgctctttatggccttgcagacaatgaggtatgatataactgaatttgattggactgaagattttctgtcttaattgcttaaaaagcttgttactttgagactttgagttaactaactattctctggttttgggttatttattttattttgtccaataggataatgtgtccgatttcattagggtaggtggagttcagaggctgcaagatggagaatttattgttcaagtaagctttctctttactacataccttgacttgcagtttccgcttttgccctttgatgcctttactaaaaaattcatcttggaccaatattgacatttacggaattgatttttgttgcaggcaactaaagattgtgttgccaagacgttgaaaagattagaggagaagattcagggccgtgtaagatgtcatattcatgatactttctgcttttggttattaatacttaatatctttaaaatgatgggagttctactgactactatattgattgtcagttttatagtattcaaatttgtaatgtgatgttttttcctttttataggtgctgaaccatctgttatatcttatgcgagtttcagaaaagggttgtcaaaggcgagttgctttggctcttgcgcatctttgttctgcagatgatcagagaaaagtttttattgatcactacggtatgtatcttagtaaaatatttttcatgggttttaggttcagttgggtttttgttttataaactcctttttattcttgttttgaagctgagcatctgtccatgcaggtcttgagttgcttatcgggcttcttggctcatctagctctaagcagcaacttgatggtgctgtggctttatgcaagttggccaataaagcatcaaccttgtctcctattgatgctcctcctctttctccaacgccacaggtaaatccagttgacttgacatcagttttcacaatttcactgcatagaatttaattataaaagaatgttttcataagttttatttttccttcaactttcatttaagggtagatgaaattgttacatccacagttttaggcttaaactttcttcataggtaagatctttataggcactcaagtaggtataagtgtaatttgcttatatgaatgtaacacgtgtttggaaatactttgttatttaaaatttctttaaaccctggtttcatatttagtagttagtagccaataacaatgactttttaacagatttatatgatattttaagatgactaatgacatgactatatataaatactgtggtacatttaatataacgagcatctaatgatctaacagccagcagtcatcttgatcaatgctttttgctgttttacatgcttgccatttgcataagaatcccgatgccaagttctctcttcagactgccttgtctaaataattctggaataagattttctaaaagctggtatgtttatgatcaaacactatttatcttgcaggtatatttaggagagcagtatgtaaacaatgctacattgtccgacgttacatttttggttgaaggtttgatgctttttgtccaccttgtttcatcattaaaattgtagcttgagaactaccttccctgaaatgtgttgtagcttcagttgacatgtgtagtagtaaacttggtgatctttgttcttcgttgcaggcaaacaattttatgcacatagaatttgtctacttgcatcttcagatgcatttcgtgcaatgtttgacggtggctacagggtgagtttattatatttagcttcacccatgaatcatctttatccttcaccctaccactaaagccactccaattaataaagatatcactagaagcaattcttgtaagtcctttacattgttacaaagtaagtgtgttggtcataaaaggaactcatttgttgactttcatgaggtatttatttttcacttatggttttactgttgatttgaacggtggatctaatattaagtaattaccaaaaattatgttttaatttgaagcattaagttatggttcatatctgtgaatcatgtattttattgcatgtcaggagaaggaggcaagggacatagagattccaaatattagatgggaggttttcgagttgatgatgaggtcactaaattctgctgtcttgcattttattaaagttggtctgtgaatgcttctaataatttctgggcatcttatatctcattgtttgtctgatctctattcagatttgtgtattgtggatcagttgatgtcacactggatattgctcaagatcttcttcgagcagccgatcaatatcttttggaaggacttaagaggctctgtgagtacacaattgcacaggtgatctaggaaaaccagtttttatttatgtatccatgtgctaaatattatacttgaaagtgggcttcctcattaccccatgtttttgtgacaggatatatcactagaaaatgtttcaagtatgtacgaactttcagaagccttcaatgcagtaccactgaggcatgcatgcatcctttttatcttggagcaatttgacaaattgagtgcgaggccagggtattgatccgatttcctcgtttccgtgtttacttcttgtgggcgttttattacctctatgatgtcttaattggtcatctggtttagtagtgttgtgcgtgctgtttcgagaagaatgttgttgacttaaaaggaaatttggatcttgaggcttgaaaatgtcactaatctattttttcatgaccatgttttgttttaattaaacagccatatccctcagtgcgtgaataatgtcactagtgaaaatagcaaatattcaaaaagcctattgtatccaaaaatcagtaaggaatagtcctttggaaacataaatattccatgcatactgtggtacaatgttgtggttgggggaggttccaataatatcttggatatgattatgtattccacattcctttcttatatgtgaagtaccattttcttcaaagattaagcagcaggtagaaggtttatttgtatggttgttttgtaccgtattcagatcagatacgagggatttgatatttttatacatggtcattttctgtttatacacagttgtgttctataagtagtttgaaataaactggataatcagcatcaaggcattttttgtgactgactgattcttcatcttatatttctgtttactctaattgtttgcaggcattctcttctgattcagcgtgtaataccagagatccgcaattactttgttaaagcacttacaaaggccaactcccataacaaccgactgtagtatgcacccattctatactcttgacctctaaccgattgtgttgtacagaatgtagtagatgttattccttttgttgtaccaggaaggggtctcctgtttgtgatatacaactcggctaaaagaaatacctaacgactgagtcgtgcttcttcttttctttttaaacgaggtgtaagccccttttggtctgtaacttcattatcatagatatagcaaatatgaccttcacgaacattttttttctctc

SEQ ID NO: 188 - protein, 704 aa, Phaseolus vulgaris
MENPNTVSRGLKRKPEGDLSQNQSDFKAQCLSSKFRKKILRQVSLLNSTTSDPLTLQKAIHNLSVLAEDEDLVDTVLDCGVVPALVRHFKLPDARNDDNSNIGKDSSDRVIDHEECEMAKGCALIIELLAVKQEYQDLIVGAGALPCLVESLKKHKICTISQPLINLLKRAADAITSLAHENSDIKTCVRREGGIPPLVELLEFGDIKVQRAAARTLRTLAFKNDGNKNQIVECDALPTLVLMLGSEDSKLHSEAIGVIGNLVHSSPNIKKDVLLAGALQPVICSLSSSSYCSESRREAALLLGQFATTDSDCKVHIAQRGAIPPLVDMLKSSDAELQEMSSFALGRLAQDSHNQAGIAQSGGIEPLLKLLDSKKTPVQQNVVFALYGLSDNEDNVVCIIKADGFQRLKAGNFKNQQTVECAMKTLKRLEEKTQGRVLKQLIRLMCYPEEVVQRRVAIALAYLCSPRDSKTIFIDNRGLNLLLDMLKSPNVRQMSDASAALHKLAAKAHSSVVSLFELPPPSPSPQVYLGEEYVNNPKLSDITFLVEGRTFYAHRDCLVSSDIFRAMFDGSYREREAKNVVIPNIKWDVFELMMRFIYTGTVDVSLDMAQDLLRAADQYLLDGLKRICEYAIIQEISVENVVILYKVAEDFNATSLRHACILFMLEKFDVLRSEPWYCSLVHHILPNICMFFSTLLVKSHPVDL

SEQ ID NO: 189 - protein, 707 aa, Phaseolus vulgaris
MDLHARPDHCLPERKGQKRKLEEDFEDDRQISAPPTGHARDALLSDVKEQVIVLDSTFSWKESDRAAAKRATHALADLAKNEEVVNVIVEGGAIPALVKHLKAPPLVGSDLLQRPMPFEHEVEKGSAFALGLLAVKPEHQQLIVDSGALKHLVDLLKRHENGLTSRAINSLIRRAADAITNLAHENSSIKTRVRIEGGIPPLVHLLEFADTKVQRAAAGALRTLAFKNDENKNQIVECNALPTLILMLRSEDAAIHYEAVGVIGNLVHSSPNIKKEVLLAGALQPVIGLLSSCCSESQREAALLLGQFAATDSDCKVHIVQRGAVRPLIEMLQSPDVQLKEMSAFALGRLAQDTHNQAGIAHNGGLIPLLKLLDSKNGSLQHNAAFALYGLADNEDNVADFIRVGGIQRLQDGEFIVQATKDCVAKTLKRLEEKIHGRVLNHLLYLMRVSEKAFQRRVALALAHLCSADDQRKIFIEHHGLELLMGLLGSYYNSKQQLDGAVALCKLANKGTTLSPVDAAPPSPTPQVYLGEQYVNNATLSDVTFLVEGKRFYAHRICLLASSDAFRAMFDGGYREKEARDIEIPNIRWEVFELMMRFIYTGSVEITLDIAQDLLRAADQYLLEGLKRLCEYTIAQDISLESVSSMYELSEAFNAISLRHTCILFILEHFDKLSGKPGHSHLIQRIIPEIQNYFGKALTKGISYNQP

SEQ ID NO: 190 - protein, 699 aa, Phaseolus vulgaris
MDSSARQSLKRKLAEEVKDSLCKRVPPTFTSIILKTLFLLNSFDHVLLNKLITILVKLCKTTKHEIHDDFIDILVNNGAVQALVRILHLPEKVVEDYSDRLIQARLLQLKKGCAFILGTLAKKSVYQQLIIDAGAFLYLLRLLKSHKTIPKSPSVPGFLRRVVDAISKLAYKNNKVKMLIRKEDGIAPLIELLEFKVKKVQVAVTNALGTLAFDNAHTVTKMVECNALPSLVLMLQSEDSVTQFTTVQLIKIMVDTSPHIGREVLKAGALTPVICLLSSSFSESQALAALLLGHFLGTDSDLKVHISQRGAIPPLVHMLQSQNTNLRKASAFVLVILAQDSHNQVSIAHSGGIEPMLNLFQSDNPTVQQYAARVLYSLADNEDIVANIIKVGGFEKLKDLHFTEEPISEFVAITLLRLERHMQGRTLKYLIHLMCSAEERVRNHVVIALAHLCSPPDHETVFIHNEGLELLLNILQSQCTIQKRKASMALSMLASRANFISSLIQTISPSPTSQMDLGEESINNPKLSDITFLVEGKIFYANKDRLVSSSVFQTMFEAEYFEKETKQAVIPNIKWDVFKLMMRFIYTGTVDVKLDDAKDLLRAADQYLLQDLKLICERVIAKSISPENVSLLLDLSEDFSANTLKNACILYMLEKFDRLHSKRWYYTMLHRIVPDIDTLFSTLLIMDQSNEDASVAYLY

SEQ ID NO: 191 - protein, 706 aa, Phaseolus vulgaris
MELQRRQDQSLSQRKGQKRKLDDEHHDEGQISAAPPTADERAALLYDVAEQVSVLESTFTWNEVDRSAAKRATHALADLAKNEEVVNVIVEGGAIPALVKHLQAPPLVDRVEKPLPFEHEVEKGSAFALGLLAVKPEHQQLIVDSGALIHLVDLLKRHKDGLTSRAINSLIRRAADAITNLAHENSSIKTRVRMEGGIPPLVHLLDFADAKVQRAAAGALRTLAFKNDENKNQIVECNALPTLILMLRSEDAAVHYEAVGVIGNLVHSSPNIKKEVLLAGALQPVIGLLSSCCSESQREAALLLGQFAATDSDCKVHIVQRGAVQPLIEMLQSSDVQLREMSAFALGRLAQDTHNQAGIAHNGGLVPLLKLLDSKNGSLQHNAAFALYGLADNEDNVSDFIRVGGVQRLQDGEFIVQATKDCVAKTLKRLEEKIQGRVLNHLLYLMRVSEKGCQRRVALALAHLCSADDQRKVFIDHYGLELLIGLLGSSSSKQQLDGAVALCKLANKASTLSPIDAPPLSPTPQVYLGEQYVNNATLSDVTFLVEGKQFYAHRICLLASSDAFRAMFDGGYREKEARDIEIPNIRWEVFELMMRFVYCGSVDVTLDIAQDLLRAADQYLLEGLKRLCEYTIAQDISLENVSSMYELSEAFNAVPLRHACILFILEQFDKLSARPGHSLLIQRVIPEIRNYFVKALTKANSHNNRL

SEQ ID NO: 192 - DNA, 9253 bp, Glycine max
  source 1..9253: mol_type = genomic DNA
ggttgcgttgcgtcgagggactcagcttcttcttcttcttcttcttcttcttcttcttcttcttcttcctcttctcgttcttctctcatccattccatggagcttcagaggcgtccagatcagtgcctcccggtgaggaaagggctgaagaggaagctagaggaggagttcgatgacgacccacagatctccgctcctcccaccggtgacgctcgcgacgccctcctctctgacgttaaggaacaggtttccctcctcgattccaatttctcctggaacgaacacgatcgtgccgccgccaagcgcgccacgcacgccctcgccgatctcgccaaaaacggtaataaatctattcctcctccgctgtttccctccgtccgttgctgcgcgcgcgtttcattcggtggttgtttttgtttgcagaggaagtcgtgaacgtgattgttgaaggaggcgccattccggcgttggttaagcatctccaagcgcctcctctggctgaaagcgaccgtttgccgaggccaatgccgttcgagcacgaggtcgagaaagggagtgctttcgcgcttggacttctcgctgtcaaggtaattttacttttctcctttcttccgactattagatagtagaaggaagctttgaagttaatgcctgatggtctaatattgtggtggtatgaaaatgctttgtgcagccagagcatcaacaactcattgttgacagtggtgccttaaaacatcttgttgatcttttgaagaggcataagaatggcttaacatctcgtgccattaatagtctcattcgtagggctgcagatgccatcactaatcttgctcatgagaacagcagcattaaaactcgtgtcaggtttgtttctttgattgaggactaccgtgctattgaaacttaatttggaatagttttgttctaatgattatctggagttaatgtgtaggaaggaaggcgggattccaccgcttgttcatttgcttgaatttgcggatacaaaggtgcaaagagcagctgctggtgcattgcgaacccttgcttttaaaaatgatgaaaataaaaatcaggttagtggtcttcagtgaaagttgggaatttaatttgacttccatatgatatgagtaagtcatatgacatcatcacttgtagattgttgaatgcaatgcccttccaactcttattctaatgcttcgctcagaagatgctgctattcattatgaagcggtattgttagtgcaaccttaattttaaatgttaaatttttcatgtgctgagtttggtctttacacttctcttactgggcacatgggatgaattttttgaattacaggttggtgtcattggaaatctggtccactcttcccctgatataaagaaagaagttcttcttgctggagccttgcaacctgttattggactacttaggtgtattttcacttcacattctggaaaactactctgctcctttcctttcctcccttctcccaagtctcaaccctaatctcaatttgtattgatataacccaaagttgccttttaatggcaataatcttcaataatatatatattgctgaaaatgatatctttctgttaacctattctaatgctgttttatgcaacagctcctgttgctctgaaagccagagggaagcagcattgttacttggacagtttgcagcaactgattcagactgcaaggtaagcatgaagtttagtgttctatctctgtacggaaaggtgagggagagaaaggtagcaaaggaaaaccctaaaacctcttactggatggtgtaaagtagtggaatgaacaataatacacaaggatttttagtttggattttggagcaataggacgatggtttctaactcatcaacgcttcatgtattatatctctgtttttaattcttaccttgttttgttttatttttgtaggttcacattgttcagagaggtgctgtccgacctctgatagagatgcttcagtcctctgatgttcagctaaaagaaatgtctgcctttgcattggggagattagcccaggttatttgttttcccttgtcttttccatgtcggagttcacatgtgtaagttgagaaggtttagtcatttttatattcatggaaatgatttaatgttatttcctctttatagttttcaatttgtaacatatatattctacacacttcgttctgtgttgagtattatatgtaatgtcttacctcggtacaaaagccatcttactaatttatattacagctttataaatgcaagtgttatgcactatttccatgtgtatgttgaatcattgcttcctgttaacaccacaaccttttccagctttcctttggcctgaaaatatttaattttaaatttcaggacacacataaccaagctggtattgtgcacaatggtggtttgatgccattactgaagcttcttgactccaaaaatggctctttgcaacataatgctgcatttgctctttatggccttgcagataatgaggtaaaacaaaccttgaattctaataaaagatcttgtcttgaccatggaaaaactcattacttcaagcccaagtcaattaactgttacatttttattttttcactgtcccataggataatgtgtccgattttattagggtaggtggaattcagagactgcaggatggagagtttattgttcaagtaagttagcctttttgttacctatgcagtatctctgttttcagggtttttttcattttccctttgttgcctatatgaatggggattcgatgcttcagataattgcataaaagttctctcttcttaagcacacactgatctatatggaattggtttccattgcaggcaactaaagattgtgttgcaaagacattgaaaagattagaagagaagattcatggccgagtaagcaccatgtcacattaacttgttacttgatgcattttactgaaattaacatggaaatgacaaggattctacttctgtatcaattataagttctactagaacaccaaccacctagccttatcccacaattttttagttctatatctcgttttaatttgtaacctattaattttcattttgtaggttctgaaccatttgttatatctcatgcgagtttcagaaaaggcttttcaaaggcgagttgctttaactcttgctcacctttgctctgcagatgatcaaagaaaaatatttattgattataacggtatgcatcttaatcaaatgtcctgattaagtttggtgtatgttgttttttgattttaaaatcctttttcttggtgatttattgttttttcttttctatttgaatctaagcatctgtccatgcaggtttggagttgcttatgggacttcttggctcttataaccccaagcaacaacttgatggagctgtggctttatgcaagttggccaataaagctatgactctgtctcctgtagatgccgcacccccatctccaacaccccaggtaggcttatatgaagcttggcttgtcctcattcttcatagcatctttgctaagagtttgattgtttttcccccaatatttttgtatgatcactatgcttgtatattgatgttttctaggttaagtttcttttccggtccttttcatgataatatgaaaatttgtttcctcttcctttttatattgataagatctctgtgtgcgcaccctcatgcttaatatggcaggtgtcaacagtgaggctgattattttttaaaatcctacctgatatgaccaaggaggcaggggcacctaccactctgccaaaaccttaagctgttagcttagatgcaacactttaagataaaacactctgcttagacactgtccttccctatttaagccattgggtcatcgggttgaaccaacccgcagagccaacatgtactatcatggccctttgggcatatagttttctcttagaggaggaggtttgtctttgaaccttgagataattggaaacatatcaaacccgaaatttgcatatgtatcagttctgataccaaatcatatgcctaagagtgcttcctactatgccaaaaacttaagctgttatcgtaacacgtgcatcagacatgggatcttccctatttaagccaccggacatgggtacactaggttgaaccagacccacaaacccaacatgcactatcacgatcctttgagcatatcagtgtatagcagtcaatgattaacaacactggctttcttttttctgatttgcatttttgtttgacatgtgatatctctttaaaattgatgattaatattgatttgaataatggggatggtgtctagttatgaatacatactctaattaattagcatctacacctgcagatccaataatctgtagttaacatggcctatgtcttcaaatattatttctgccacttgcatattcataagaagcctgatgcgctgctcactttctgtcttatctaaaattctaaatagttatggatccataagtaatttttgcaagttttaaaatctgtaatcctagacttttcttcttgcaggtgtatttgggagagcagtatgtaaacaatgctaccttgtctgacgttacatttttggttgaaggttgatgctttttcattcacattgttttgttaaaactgttgcttggaaaataatttacctaaaatgcagtgttgtagttttagttgacatttgtagataacctggtattttcatactttgctgcaggcaaacgattttatgctcacagaatctgcctgcttgcatcttcagatgcatttcgtgcaatgtttgatggtggttatagggtgagtatatattgatcttctctagtggtatcatatgtctcctctcacccaccttttcttgttattgttcattgactatcagtcgggaaaagaaaactgttattgactcccttgatttcatgagaaacatcatttatcttctattattttggttttattgtttgtctaccttggaaagcttttattggagacttggccgtaaaattgatgggtgaatttgaatatagctgttagatattgttgcatattagttatggtatcttgtgccttttgtcatgggcatattatatgatctacacaattatggtaattagttaattaggatatccgtaattaatctctcttttcttaaccatattatataataacactctccgctgtgtaactgacacacagattcacttatttctgttgttttcttttcctttcaacaataggaataaaaaaatttatttcatattttgcactataatatatttgatgtctgatatgcaagttatttattgtatgacaggagaaggaggcacgggacatagagattccaaacattagatgggaggtttttgagctgatgatgaggtcaaataaattctgcattcatgtgctttatgaaagttgtgctgtgaaagcttgtaataatttgtggacaacttaaatctttctccagatttatatacactggatcagtagatatcactcttgatattgcccaagatctcctccgagcagctgatcaatatcttttagaaggacttaaaagactatgcgagtacacaattgcacaggtcagctatgagaattttggtacccacacttgtcctcctgcactacaattagactggaaagtgaattcatgtgctctgatttgatgttttttgtcccaggatatatcactggagaatgtgtcaagtatgtatgaactttcagaggcctttaacgctatatcattgaggcacacatgcatcctttttatattggagcactatgataaattgggtggaaagccagggtatctatctgatccctcaatcctgtgtttgcttcttttgcggggatatatatatatatatatatatatatatatatatatatatatatatatattccttctttgcaatgcttaaaaggtgtctgaaataaataaacaatctaaatggaataaatatctgaatcatcttgtgtaagctggaggttttaggtcagttcagttgcacctacttttaatactaatttgtcttttattttacggcaaagcatatgtcaagctaaaaggcattcagatattgaaatttgaaagttttgggatctacttagtacttaaacaatgtcattattttacaggactaaatcaaaactatacggcctaccatatccagtaattaattagttcttcacttgattccatgaagctttcaattttagtgcaaagctgttacatttaatggctaaatggcaaccagaaagcatgttatcatgttattttattagtattcagatgagaaataattgactttttgtatatggttatcaaaatatggaaagctgtgtatttatttttctgtgatttgtgttcaatatattccctatcttttactttctttttctttttttataattttggctgcataataatttgtcatattcttagttttgtttgcttttgattaatatgatagacagggatcttaaactgttatatgatgaatgaattgaataattaagttgactggacaaataaataacaattatgatgaatgtatttttcattggttctatgtcttcctaatctttctaatttttgtgtgcaccaactactatttgcagacactctcaactgattcagcatataatacccgagatccagaattactttgttaaagccattacaaaggccaattccaatatccagccgtaatgtgctgttctactattgacatctaacccgttgcaatgtacataatgtggttgatgttctttttgttgaacctgcgaaggaagtctcctggatcaagtacagcatggcttaaaaaaaatatctaacatcacgtcatgtacgttcatttctgatgcagtgtaagtcccttctagctgtaacgtcattgtcttagatatagcaaatatgaccttcacgaacattgttttttactcgtgcaaatattgtgatggttgagactttctctttctcaagcatctaatgttgagtttatgagtagtataggttgcccaagcatctaatgtatatatgacaattagatagttgtcttcatattatataatgaaatcttaaagccttttcactggatgtatcagaatttctgttaggttttacacggacagatggaaggcctagtgataaaaaggctttgatggttatttttgaagacataaaaaagatcaagctgcttttttgttgggctatacttttatagaaaataattttctttaaaaatataaaaaagtaacgtattttattattcacatgtgagaaccatgattcttcgaaacattcgtataaataagttggaagttttaaattcaggaactctgtttgctttattttcatgaggcgtcaatgatccatagaataatttaatcctttttttttgttgggcaaaaggagcgacgaaaccaaagattaaaaacctctgaaaaagatacaccagaatgagccgtgttggttgctctctaagcacgtgagtgaactttatcaaggccctgaattccgtgagcttattgatctcctggactagattgtggcagggatgggtgatttcacaaccatccccgattaaggcaagcgcgattgtggaatcctctcttaattgctaatcccccaacccaaagagcttggcctacatcacttgattcaagtttaacataactgggcaagacttgaagtacagattgagtgagggtattcagatctaaatatatgcgcaaatctaaaaaaaaaatcagttccattagttcattcacgtagtattaagcgcaaatgattacttaggaggagaaatcagagtgaacaatgcatgcgcaaatcaaattgagatgtgatattatggataaaggatttcattaaacagagatcttggaacaagggaccggacacattattctaggaaatttatttaattaagaatgcccttgttataaggtgaaacgagcagatcctaattggtttcactggcgaagaaaattagcgacgattgttatcaatcttttggcttggtgagtttccatattaaacatgtgataaacatgatcctcttgttcctcttcaaagagttccacttggcctttccagccactctccttgacagccttatagtacaacagagttctgtccctgaagagtaggtgatccttaccggcaacagtaagaagcatcttagaacagccaagttgagccaagctgggtgccccaggagccaatggattgatcatggggttatctaagccaccaggtgcatcagggtacgcaaagttccaaatcaatgactgaggggtctcttcaaatcctataacagcttcagacccaattggctttgaaccccagaagtaagggtggttaagataagcaccgtaaacttttacaccgccgggcaaagcttcaaccccagcacgcatggccaggttatgaacaatattggcaccgctgctatcacccccgataaatattttgctgaaatcaccatgattgatgagccacgtgtcgctgttgctgttggtggcatgggaatgggatgcaacccatttgagagcagcccaagaatcattataagctgcagggagaaaatgctcaggagctttcctatgctctacggaaacaatgataacatttgcctgggaagctattaggttgcagtatttggtgtggtgcgctgcaaatgctgattcaaagcagaaggcaccgccatgggagtagaccaaaatggggattttttggttgggtggtggagttgttagttttggaaggaaaagtcttgcaaagaggaaagggttctttgagaagagaatgtctttggaagcgacacctgttgcagggtcctcaagtgagggaggagttcttgggatgtctatgggacgttcgatggagccatcattatagacatatatgtagggaggaatctgtgagactatgtgtttggtgttggtgttggtgttggtaccgctccaagccatttcaacaatgcaaacttgggtctgcagttttatgtttagacgatagtgtcccccccccccccccacacatatatatacaaaacgaaagaagagtgtgttaacttcaacttatttcctctttcatcttctttttactttatttttatttttctctttttttattatatctattattatttttattttttcaattcagtagcaaaaccttaaggattcataaataagaccaatgcagttcgcat

SEQ ID NO: 193 - DNA, 5529 bp, Glycine max
  source 1..5529: mol_type = genomic DNA
gaagctcacaagggccaattaatttattttgttttgatttcgttcccaaatcccatggaaaagcgttaccctgttgctagaagaagctcgaagcggaagctcgaagcagatctaaccgaagaccagacacataccaaggcgtcaaagatctctgcaaagattctcaaacaggtttctctcctcaactccgctgctattccgttcactgcgttggattgtgctaccgttaagagcgctgtccactccctctctgtactcgccgcaaatggtacttcacttttctttttcgtttctttaatttttgtgtttcgtgcttttattgaattttgcatttccgtttgattgacacctctcttttttttttctttagaggatcttgtggatactatactgaattgcggtgtcgtccctgctctggtgaggcatcttcggttgacagacaacatgcggaaatatgacggtcatgaggcagaaactgtgaaagattacagcgatggtgttacggaacatgatcagtttgatgtcgtcaaaagatgtgcggtcatccttgagcttcttgccattgaagtaaataagttttactttttcctttctctctaaatattttaattatatgaaattgtaactgtagtgttgattttagatttatccatcaaaaggtttcggttcaagctagatgaattatccattgatagatagttgtgcatgtgtgtaggtgtggaagcttacctccaagtcagaaaattctaaattacaaattttaaaccctaaatggatatcagtaaataataatttagaatgacttgtcaatcaatatcaatatttagttttcaattggcggttattggatatataagaggcaaatagattggaattgctcacttgtcgtgctcctgccccattgttttttattagtgcaaatcacctaaggtttctctgaattgtttattattcacctgctcaaagagcagctgccattacagtcttcacagacatgttgtaaagaatttgggtgtatggggttaattactcaatcatactacgtacaagtaataacaatattgaatctctatgtacattccatttgatcttctttagcagtatatccgtgacccttgtttccagaaaaatggctatgattttcttttctttaattcatttctctttttctttgtttcagattattttataaatcatgaagcatcttaattctgattttatttttgctatatctttatcgtgaaacagcaagagtatcagcagctcattgtagatgctggagccttaccctgtcttgttgattggttaaggatgcaaaagatcagtactacttctcaaccacttattgaccttctaaagagagtagctgatgcaataaccagcctaatccatgaaaataatggcattaaaaccctattcaggttttctctttttccataccttcaaaaatactgtattatttactcttatatacaagtggtatattcaggatggaaggcggtatagctcctcttgttgaattgcttgaattcaatgacataaaggtacagcgagcagctgcacgggccttgcgaactcttgcatttaaaaacgatggcaataaaaatcaggtagttgactttttgaagtaaattggtgtgatagatattgttggtatggttgtttacaagaataaaatattgcagattgttgaaagcaatgcattacccactcttgtactaatgcttcaatcagaggatcctaaaacacattatgaggcggtaatatgcttatatgactttacacagtccaatgcattttatagattgctgcttgcagagttctaagctactagcactagctgagttagcgctttttgtaggttggtgtgattggaaatctggtccactcttctccagatattaagaaagaagttcttctagcaggtgctttacaacctgtcatttctttacttaggtaatattatacttctatcttggtttttcctataagcaatccatagaagaatgatgtttattgaacattatagatgttttctgaaagtgagttactacttccatgttattattttgtaatttagtacttttccgttttccccctaagtttcaaaatttcaatgacagttcttgctgttcggagagccaaagagaagcagcccttttaattggtcagtttgccacaacagattcagattgcaaggtggatttagttttttgcaaacttgtaatatgatgaatctgtcagttatgaaatcctcttattgaattccatattttgtggttcatgtaggttcatatttgccaaagaggggctattccaccattagttgacatgcttaggtctccagatgctgagcttcaggaaatgtcagcttttgcacttgggaggttggcacaggtgattactctcaatatgttatgttctttttctattaattttaccatcatctttcatttttcattgttttgtattttatcatgctccttgattgatggtgattgtgtgtaaaactgcaagtctgtgatgtattgcttatcttgaatttctttaattttgggcttttagttttgatttttgataatttatgtgtagtgtaaactattcagttttcattataatatttaaaataacagttatctcactataacatttttagtattagctgctgcacaccaccgttttaaaattgataactattgatgtgttttaataatgtagcacacatagtcttaaagttacactaagtatttttggctgaatttggggttccctttcttaaacctaactcttaatgggtggattttcttaatttatatataaacgggcatcaaatggtgcaaaaaagtatgctcctttttctgtaattttatgtgttgttttttactcttaccattttcttgcataacctttttttgcacatataattctaatttcaggactcacataatcaagctggtattggtcaatgtggaggtatagagcctctgctcaaacttcttgactcaaagaaggtgccagtccaacaaaatgctatttttgctctctatagtctcgctgataatgaggtgaagttaatttccttgttctttacttggtcaaccattatgttgtccttagatatcattgatgtgcaatgataatatgatatgctgccactgatgtaacaactttgtatgataggacaatgttgctgccattattaaggctgatggttttcgaaaactgaaggctggaaatttcagaaatcaagtatgttcatttactcttcgaaataaaagcaatacacttgcattccttcttaatgataatttagttgttaatgttcacttacagaactcctttctctcaccaatttattaagtgggtttccttgtttgtgatcgtcttttaacttgcagcaaactgtagaatgtgtagcaaagaccttaaaaaaattagaggaaaagactcaagggcgagtgagttttcttgcaaattctatggggtgatttgttttagtcatagatgagaattataatctatttaaactatatttttttaatatatctttatgttattggatatgatttttatatctatacctctttggcaggtgttgaaacacctaatacatcttatgcgctttgcggaagctgttcaaagacgtgtagctattgctcttgcttatttatgttctcctcatgatcgtaaaactatattcattaacaataatggtaaataattaatctctacatttttgtaatttctcactcactgtacttcgaatgcattttcaatcaatatggtgctaaatattcaggattaaaattgctgctggatactcttaaatcttcaaacttaaagcagaaaagtgatgcttcagcggcgcttcataaattggctatcaaagccagttcttctttctctctttttgacattgcttctccatcaccaactctccaggtattttttgctctttatgtgtgggcttatcacattcgtttattttgttttttttcttatttattgaacaatttgtaccatgttatttaaattggaatagtagttattgtctttgaaattgaatttatggtattttactgtctatattttaagtgcatgaaaatgggaagctgagatttttttttcacattttttgttcacaatagtatttgttattggttgcatttgttgtagatgtactttggcgatgaatatgtaaacaatcctaaactttctgacgtcacatttctggttgaaggtggagtatctgctattaaaattttctgctgttattatttttcgttagttgtttgtaatgaaactgatttcgatatctgtactaatttatcgttttcctttcttcaggaagaagtttttatgctcatagagattgtttactttcttcagatatatttcgcgcaatgtttgatggcagttatagggtaagcatcaattgttttgtaattttgttttcaagtccttttttctttttattgtgacatggtctaccagtcaaaattcttcatcccttctttctcaacagttattctatgtataaaaggtcgtacattatctgtaactaccctcctttgttaatattagtcctatttcaatatccatataaatatcttgagattcatgatgcaggagagggaagccaaaagtatagtgattccaaatattaaatgggatgtctttgaattgatgatgaggtgcatcttctgctatccctttcttgtgttttttgtaatatcacaataagccttgtgtctgaattgatttttttgttggcattctagatatatatacactggaacagtagatgtcaatttggatattgctcaggacctgctcagagcagcagatcagtatcttctggatggccttaagcgtatctgtgaatatactatttctcaggtaggctcaattgtttttcacggtttttatttgttttgcttttgtaggaagtttttttttaatgactaaatttaatcacatggctcatctacttattcttataggaaatttctgaggaaaatgtttcactactgtacaagatgtcagaggatttcaatgctacttcattaaaacattcatgtatactgtttatgctggagaaatttgataaactgagatgtgaaccatggtatgttatattttttacaacctggagtacttccgtagtttactgcgtttatctggcgggttgcttgtgtactgggagcattcaattcatgaaatccaacctttcattcatcttcatcactataagttcatcttttcaacatgcaggtattgtcctctggttcgtcacattttaccagacatatgcatgttcttctcaactttacttgtcaaatctcatccaactgattcgtgagaatccctagattttagccatgacaggaagaaagttgaaaatgtacaaagctgtaaatgttagttagatatagaaatcactgatcattattttttagcatgtggtgggggaatagtcattgtttgagattgagtaatgataggcagatatatataaaatggccattt

SEQ ID NO: 194 - DNA, 9382 bp, Glycine max
  source 1..9382: mol_type = genomic DNA
gtagtagttcgcatttcccgcgaaattcctaaaacgccccttccaaatgtcacccattcaaatctccaattccacttcttaccaccctctctttctctctggccactgtctgttaacttgagcaatcactctgttccttcgcttctatcgttcatggagcttcagaggcgccaagatcagagcctctcccagcggaagggccagaagcggaagctcgacgaggagcagcaccacgaggaccgccagatctcgccggcccctcccaccgccgacgagcgcgccgccctcctctccgacgtcgccgaacaggtgagcatcctcgagtcgactttcacgtggaacgaagcggaccgatccgcggccaagcgcgccactcacgcgctcgccgatctcgcgaagaatggtaaaaaatcgatgcctcctccgatctcgccgcgtgtcgctgccttcgtttggattgcggtttcggtgtggtgttttcttcttctgagtttccgcgtgtatgttgcatgtgtgtgtttatgaagtggcggttgtgtttgcagaggatgtggtgaacttgattgttgaaggaggcgcgattccggctttggtgaagcatcttcaggcgccgcctctcagtgaccgtgtccagaatccgttgccgttcgagcacgaggttgagaaagggagcgctttcacactaggacttcttgccgtcaaggtaacttgatttttctctaactgttattattttttattttatatttaactgtttatagttatacttcgtaggtcgtagtcgtagcttgatttattttgaaactttataatttttttagatgttccttagtgctgtgcaagttctgaagtacaagtgagattatggttatagtttgaatccaagtatttgtactgtttcgttcgcttattcagggacggaggcagaaaattatacagttttttttttttttggggggggggggggggggaatcacgagaaagggttagaagaagttagaaaaacaattattttcaaatatagttccataaaaaaacatgtacatgaggaaattttttcattaaaagtaattaaggttcataacatttgttagcatcatttataaaaacttaaaagaaaaaaacaaatattaagtttttgcatgatataaacaatcattagattttaactgttaatgcaatcattaaaagataaaattcttgaaaaatacagaaataagaggtgagaaaaagttactgagagacgtgtataaaaacatttagataaaaaaaattattagtaggaataaaaaacagtatcaagagatttacatcattcacacatatggcttaaccaactgaattagattcccttggtacttagataaatttaatataactcttggttacaatctatttgattgaaatattgtaaaacaatattaatggtaattgttttattaaaaatagtattaattgggcattggattttcaccgaaggttgaaaaggttgtgatggaatttcaaaaaagttggcatcaacacgcagtaactaattgtgttcataagatgatggaatttactagtttattgtcattgttatcaattactaacttagttactaattttaaaaaaaaattcaggggggccaaggcccccccacctatacacatacctctgtccttgcgcttattgagtgttgattacttaattatgcatttaaaattgaatttttattccattttttttgttaaatggcacgagtgatttaataataataataaagggaggtttagtattcagcttgctatatactgtgttatgtgtattatatggaattttgggcatgataatcatcttgattgaatggagttttttctgagtcttcagtcatgtatgtatttcaagctgaagaatggaaatgttggtggtttgtaccatcatccagtttcagttctgttctgttctgtgctgtttcttcatgctagcccattccagagacggggttcaattaaaacaaagaggagagaagaaccaaggatgtgaggcaattagacaaatggttttaaaattgattgaaaatataacaatattgttattggaaataattcatatggtttgtcctcgtgaatcagttccataagccacattaaatcaagcatctgccagttgctaggaattataagagattattagtttgtctgaatggaatttgtttgagtcaaagctggatgaggcatctatcctttggtcttaatgaagatccaccattggaagcttgtcatctctattaggtccctaatttttgtttggaactgtggggagtgtgagatacaattgatttctgatttctgaacggcaatttatgtatcatgttgtgtcaattacaagacttagtcttggttgtgggctgtgaatagtagcattgcccatctcatttttaactgtggggagtcccaacatgtgcaatgactaggaccaatgaccgagccatgtttgactggagtttgtattgtgtgtgtgtgtgtgtgtatgacatgacatatagtttcatatgattgccatgtaacttttagatatagttatacttttcttcctttttttccctaaaatttctttctgtcaaagaaacataaaattgctaaactactattctattttaaatgctttctacagccagaacatcagcagttcattgttgacagtggtgccttaacacatcttgttgatcttttgaagaggcacaggaatggcttaacttctcgtgctattaatagtctcattcgtagggccgcagatgctattactaatcttgctcatgagaacagcagcattaaaacccgtgtcaggttttgcttcttcaagggataccatatgttaaaatttactttggattttgttcttaatattaactaaacttaatctgtaggatggagggtggaattccaccacttgttcatttgcttgattttgctgatgcaaaggtgcaacgagcagctgctggtgctctgcgaaccctggcttttaaaaatgatgaaaataaaaatcaggtaagtggtcattgctgaaagttggggtttgaatatgtttcaagtaagtcacacaacataatgattttccagattgttgaatgcaatgctcttccaactttgattctaatgctacgttctgaagatgctggtgttcattatgaagcggtatgggtaatgaaactttgattaaaaatgcaagatttttcaatagtattgagctctttctttccacatctattatatggcacgtacaatgaattggattttatatcaggtcggtgtgattggtaatttagtccactcttcccctaatataaagaaagaagttcttctcgctggagctttacaaccggttattggattacttaggtatattctcagttctggaccctgataaactgcaatgccccttccgtccccaccctgaatttgttttgctattataattataatatgcccatttttgtttctggcaataatatgctgagatatattccaagaaaggtatctttcaattaatgtattatgatgtttcatttaacagttcctgctgctctgaaagccagagagaagcagcattgttacttggacaatttgcagcaactgattcagactgcaaggtaagcataagcttcaggatggaaaggacaacaatagaactttaattgggagctattgtttaataacttcagttttcaagttcggtctgcttggttttatcatattttgtttttgatttgaactgaagggggaaagaaagagagtaggggtgatagggaagagacccttactccacttttatgcttgtttacccgtgaagtgaagaggggtagaaaggaaacaatccataaccgaactttcgttgggggcaattgtttaataacatctccatttccaagtttgattgttctatattttttatttcttgttaaataaagattccaatggttagagtactggaaaatatagttgctactcttgtgatgatgcatcatatattatattatgtgtcccttagtttttactgtttgttacacttggtctttttaggttcacattgtacagagaggtgctgtccaacctttgatagagatgcttcagtctcctgatgtacagctcagggaaatgtctgcttttgcattggggagattggcccaggtaattttttttccttgtttataattcacttgcattagttgggaatttaaagttgccattatatccttggaaataactttgtattttcttctctgtataatagtttttgggatctgtaacacattcaatgcatatccatctttgcattttcaggacccacataaccaggctggtattgcacacaatggtggcttagtgccgctgctcaagcttcttgactcaaaaaatggctctttgcaacataatgctgcttttgctctttatggccttgcagataatgaggtatgatataactcagaattcaaatgaaatgaagatctgtcttaattgcttaaaaatttgttacgttgagacttaattaactattctctgtttttgggccatttattttattttgacccttaggataatgcgtctgatttcataagggtaggtggagttcagagactgcaggatggagaatttattgttcaagtaagttttttctttaatacccactttagtttttatttcagggtttctgcttttacccttggatgcctaaatttaagaaaattaaaatacttaatgattgcatctgaacatttgtaatttaaagaactggaggaaaatagattcatctttgacctatattgacccttatggaattgctttttattgcaggcaactaaagattgtgttgccaaaacattgaaaagattagaggagaagattcatggccgtgtaagatgttatattcaaattacttctgcattttgttcttaataacatggaaaatgacgcgtgtgctactggctactctattttttttagtgtttaagtccgtgttcaaatttataatctgatatttttcttttctgtaggtgctgaaccatttgttatatctcatgcgagtttcagaaaagggttgtcaaagacgagttgctttggctcttgcacatctttgctcttcagatgatcagagaataatttttattgatcactatggtatggatcttcttgctgaaatgtttgtcatgggcttggttcatgttgttttgttttacaaactcctttttatgcttgttctattttgaagctgagcatttgtccatgcaggtcttgagttgcttattgggcttcttggctcatctagctctaagcagcaacttgatggtgctgtggctttatgcaagttggcggataaagcctcgaccttgtctcctgtggatgctgctcctccttctccaacaccacaggttataaatatatatatggtccatttaaataatgagcatctaatgatctaacaatcagcagtcattatgatttatgatcaatgcttgctgttttacatgcttgccacttgcataagaatcctgatgccgagctccctcttcactctgcctttgtcccttggctaaataatttccgaattaggattttctaaaagctggtatatttatgaccgtagactattcttcttgcaggtctatttaggagagcagtacgtaaacaatgctacgttgtctgacgttacatttttggttgaaggttgatgctttttgtccacattgtttcattcattaaactgttccttgaaaactaccttccctgaaatgtggtgttgtagcttcagttggcatgtgaagttaactgggtgatctttgttcttcattgcaggcaaacgattttatgctcatagaatttgtcttcttgcatcatcagatgcatttcgtgcaatgtttgatggtggttacagggtgagtttatattgagcttcaccaataaatcatctttctccttcctccccacctctaaagtccctccaatgaatacacaggccacaagaagcaatttttttaattccattacattattaggggaaaaaaaagtatgttggccataaaaagaactcctttattgactccacttgatttcatgaggtatattatttatcacctatgattttggctgttgatttgaatggtgaatttaaatattaagtacgtaactgttaaaacttgcattttaatttgaagcagaaagtgatagttaatatgagtggcgtaaaaatgtgttttattgcatggcaggagaaggaggcaagggacatagagattccaaatattagatgggaggtttttgagttgatgatgaggtcttgtaaattctgcagtcttgcattttgttaaagttgttctgtgaatgcttctaataatttctggacaacttatatcttgttgtttatttgatctttatccagatttgtatattgtggatcagttgatgtcactctggatattgctcaagatcttcttcgagcagccgatcaatatcttttggaaggacttaagagactctgtgagtacacaattgcacaggtgagctaggaaaattggttttatagatgtatatatggatgtatccctgtactaaatattagacttgaaagtgggctcctcattaccccaggttttttgtcacaggatatatcgctagagaatgtgtcaagtatgtatgaacttacagaagccttcaacgcaatatcattgaggcatgcatgcatcctttttatcttggagcaatttgataaattgagttcaaggccagggtattaatctgaatccctcagtactgtgtttaattcttgtgggtatttttttacctctacaatgtcttaatagcggattataatgaacttggtcatgggtttagcagtgcattgcatgttgtttggtgaagcatgttgttgacttaatttcttaaaataaatttggatcttgagactttttttttgctcagcaaaaataggtgatatattataaataagtaccagaggtactaaaatacataaaaggatgggtatacagcaggttcagagcgctatacaaggaatactaagaacctgattgaacccatagtaggaaataaaataccctgcatgagctattggaattactacatctgtcgtcactccctaattatagaaaaatgctttgagttgggaggaccagtgactaaagtgcactatgaaacccttctccattgccttaagccaagaccatagtaggaatagtgcatcgttcatcactttgcttccgttgaaggatttgttttcaaaaactaccccatttcgatgcttccaaatggtccatgttagcgctacccaccagcacttccatcttttagctttaattccagcaacacatccattatcatgttgcagaaagtggtgtttgggattttgtgggaatacacccaatgagttcacccatgccagagattcccaccatagaggtagggtttttttgcaatggaagaataaatgtgctgcatcctcctccgggctgttacatagtgggcaccgtgagtcatttatctccacctgtctgctcctcaggttggtcctagttggcaagcggtctctaatgagcctccatgtgaacactgctgctttaagtgggatcttgagcttccatagctccacaaaggtctgatcttcagcagcccccgttgagtagttcccactcgggtcagccttccatacccataagtctgctctgtgttgatgaactgttatttgtgctagctcctctaaaaattcagcagccataccaatttcgttttcaaaaagagacctcctccagctcaattcccattcccaccctgcatccttttgactccccacacagctgatgagttgatgtttctgattggagatctggtatagtctgggatattttaccattaatggtctgccatcacttgcccaagtatcctcccaaagtctgaatttatctccgcatcccaccttccattgtatctggttcttaattacatctgcgttctgctgttgattgatctgcataagatccttccactagagggagagatatctgctccttcttgcatcatcaagggatctccagccaccatacttggaagtgagtattctggtccacatgtccccctgtttctgaaacagttcccacctccactttcctagcaacgtcgtgttaaatacccgaagatcttttatgccaagaccacctctgtcttttgggagacacacggtttcccaattgacccaagcaatctttctgtgttccaagcctccaccccataggaatctacactgtatgttgatcagcttttcaacaactttgtccggtatctggctccttattcttccccactagaaagtggatcttgagacttgattaatgattactttcactagtgcaaataaaaaaaatatgcaacctattgtatccaaatatgaataaggactagtttttgggtatcataaatttatcatgcatgctgatttgtggtagatgaggttttctataggtgggcatttgctgtttattttcttttttgcgaagttgttatcttcttctgcttggttttgaaaaaaacgatgccgacctttggtttgaaataaactggaatagttcagttttaggaggtttcttaagtgcagtttctggaggttgccgtcatacttaaaatatggatatgatgatagaaattcacacttgtcaacgcatttttttgtgtctaattcttcaccttatatttttttcggcaccaattggttgcaggcactctcttctgattcagcgcataacaccagagatccgtaattacttcgttaaagctcttacaaaggccaactctcaaaacgaccgactctagtatgcacccattttattcttgacctctaaccgattgtgttgtacaaaatgtagatgttgttcctttttttgtaccaggtagcaatctcctgtatggtatacagtttggctaaaagaaatatctaacgccggagtcatgcttcttcttctttttaaatgaggtgtaagcccctttctgtctgtaacgtcattatcatagatatagcaaatatgaccttcacgaacattgtttttttctcatgcaatgtgactgctatatgatttaacagttcttctctcagatgcctacgttcagggaattaccattgttgactttatgattataggtgtaaatattgtttcccttatgtatatatgaacaaaaagttttctgcaaggaagttgtgccgctgggtttacttctgccagaccattaaatcctgtcttctgacatggaatgtgttgtaaactattgttgcaaatccttcattcaaatactcgaaggcatgctgctgacgtggcccaaaaatttaccattatgcatccagtcct

SEQ ID NO: 195 - DNA, 8378 bp, Glycine max
  source 1..8378: mol_type = genomic DNA
acctcatttctgaacagtttttggtttgggttgcgtggcgtcgcgttgcggcgagggactcaccttcttcttcttcttcctcttctcgttattctctcgtccattctatggagcttcagaggcgtccagatcagtgcctcccggagaggaaagggcagaagaggaagctcgaggaggaattcgatgacgacccacagatctcccctcctcccaccggcgacgctcgcgacgccctcctctccgacgttaaggaacaggtttccctcctcgattccactttctcctggaacgaacccgatcgtgccgccgccaagcgcgccacgcacgccctcgccgatctcgccaaaaacggtaataataaatctcttcccctcctcctctctttgctgtttccctccgtttcttcccgcgcgtttcattcgctgctcgtatttctttgcagaggaagtcgttaacgtgattgttgaaggaggcgccattccggcgttggttaagcatcttcaagtgcctcctctgcctctgcccgaaaccgaccgtgtgccaagaccaatgccgtttgagcacgaggtcgagaaagggagtgctttcgcgcttggacttctcgctgtcaaggtaatttcacttttcttctttctgctcactattagatactatatagttgaaggaagttttgaagataataatgcctgatggtctaattatgtggtatgaaaaaatgctttgtgcagccagagcatcaacaactcattgttgacagtggtgccttaaaacatcttgttgatcttttgaagaggcataagaatggcttaacatctcgtgccattaatagtctcattcgtagggctgcagatgccatcactaatcttgctcacgagaacagcagcattaagactcgtgtcaggtttgtttctttgaggactaccatgcaattgaaatttaatttggaatggttttgttctaatgattatctggagttaatgtgtaggaaggaaggcgggattccaccgcttgttcatttgcttgaatttgcggatacaaaggtgcaaagagcagctgctggtgcactgcgaacccttgcttttaaaaatgatgaaaataaaaatcaggttagtacttggtggtcttcagtgaaagttaggaatttaaattgacttccatatgatttgagtaagccgcatgacatcatgacttgtagattgttgaatgcaatgcccttccaactctgattctaatgctttgctcagaagatgctgctattcattatgaagcggtattgctagtgcaaccttaattatagatgctaaattttgcaagtgttgagtttggtctttacacttctcttactgggcacatgcaatgaattttttgaattacaggttggtgtcattggaaatctggtccactcttcccctgatataaagaaagaagttcttcttgctggagccttgcaacctgttattggactacttaggtatttttgcacttcacactctggaaaactactttgctcctttcctcccttctcccaagtctcaaccctatacttaatttgtattgatataacccaaaggtttttttccatggcaataatcttcaataatgtatattgctgaaaaggatatcattctgttaacctattctaatgctgttttatgcaacagctcctgttgctctgaaagccagagggaagcagcattgttacttggacagtttgcagcaactgattcagactgcaaggtaagcatgaagtttagtgttctaattctgtactgaaaggtgagggagaggaggttagaaaaggaaaaccccaacacctcttgtttttatgtttgtcgactgaacggtgtaaagtggtggaatgaacaatgatacacaagaaattttagtttggattttggagcaataggatgggtggttgttaactcatcaatgcttcatgtattatatctctttttaatttttaccttgttgtttgatttttgtaggttcacattgttcagagaggtgctgtccgacctctgatagagatgcttcagtcctctgatgttcagctaaaagaaatgtctgcctttgcattggggagattagcccaggttatttgttttcccttgtcttttccatgtcggagttcacctgtgtaagttgagaaggttaagtcatttttatattcatggaaatgatttaatgttcatttcctctttatagttttcaatttgtaacatatattctatgcacttccttatgtgttgaggtcttgaggattataattaatgtcttatctcagtacaaaagtcatcttactagtttcttgtagtacagctttataaatgtttataaatgcaagtgttatgcactatttccatgtgtatgttgaatcattgcttccagttaacaccataaccttttcctttggcctgaaaatatttaattttaaatttcaggacacacataaccaagctggtattgcacacaatggtggcttgatgccattactgaagcttcttgactccaaaaatggctctttgcaacataatgctgcatttgctctttatggccttgcagataatgaggtaaaataaactgtgaattttaattaaagatcttgtcttgatcatggaaaaactcatcacttctaaccaaagttaattaactgttccttttttatttttcactgtcccttaggataatgtgtccgattttattagggtaggtggaattcagagactgcaggatggagagtttattgttcaggtaagtttgcctgtttaatacctatgcagtatctctggtttggtttcagggtttctgcattttccctttgttgcctatatcaacggagattcaatacttcagataattgcatactagttctctcttaagcacacactgatctataaggaattgattatcattgcaggcaactaaagattgtgttgcaaagacattgaaaagattagaagagaagattcatggccgagtaagcaccatgtcacattaacttgttacttgatgcattttactgaaattaacatggaaatgacaaggatgctacttctgtatcaattataagttctactacaacaatcaccacctagccttatcccacaattttttatttctatatctcattctaatttgtcacctattaattttctttttgtaggtgctgaaccatttgttatatctcatgcgagtttcagaaaaggcttttcaaagacgagttgctttaactcttgctcacctttgttctgcagatgatcaaagaaaaatatttattgattataatggtatgtgtcttaatcaaatctcctgcttaagtttgatgtatgttgttttttgcttttaaaatcgtttttctaggtgatttattgctttttcttttctatttgaatctaagcatctgtccatgcaggtttggagttgcttatggggcttcttggctcttataaccccaagcaacagcttgatggagctgtggctttatgcaagttggccaataaagctatgactctgtctcctgtagatgccgcacccccatctccaacaccccaggtaggcttataaaaaacttggcttgtcctcattcttcatagcatcattgctaagagtttgattgtttttttcccaatattttcatatgatcagtatgtttgtatattgatgttttctaggttaattttcttttcatgtccttttcacaatgatatatgtaaaatttgtttcctctttttattttgtcatttttatatgatagcatctctgtgcacacatcctcatgcttaatatggctggtgttaactgtgaggctgattattttttaaaatcctatctgatatgaccaaggaggcaagggcacctatcattctgtcaaaagcttatgctgttagcttagacacaacactttaagataaaacactctgcttagacactgtccttccatatttaagccattgggcatgggtcactggattgaaccaacccgcagagccaacatgcactctcatgaccctttgaccatataattttctctctcttagaggaggtttgtttttgagccttgagataattggaaacatatcgaacctgaaattcaaatatgtatcagttcagatacccaatcatatgactaagagcgcttactagttactactatgccaaaagcttaagctgctatcatagggaaaacttttgacattaacacatgcatcagacatgggatcttccctatttaagccaccgggcatgggtacattaggttgaaccagatccacaaacccaacatgcactatcatgatcctttggccatatcactaccgacaagcttgttatttaaatttcttctcacctgtcatctgtgcccatatagttgacaagggtaacaacactgactttcttttttctgattcacatttttgtttgacatgtgatatctcttcaaaattgatgattaaaattgatttgaatattggggatggtgtctagttataaatatatactctaattaattagcatctacatctgcagatccaataatctgtagttaacatggcctgtgtcttcaaatattatttcttccacttgcatactcataagcttgatgcactgctcactttctgtgttgtctaaaattctaaatagttctggatccgtaaggtatttttgtaagttttaaaatctgtgatcctagacttttcttcttgcaggtctatttgggagagcagtatgtaaacaatgttaccttgtccgacgttacatttttggttgaaggttgatgctttttcattcatattgttttcttaaaactgttgcttggaaaataatttacccaaaatgcagtgttgtagctttagttgacatttgtagataatctgatattttcatactttgctgcaggcaaacgattttatgctcacagaatctgcctccttgcatcttcagatgcatttcgtgcaatgtttgatggtggttatagggtgagtatatattgatcttctctagtgggatcatgtttcctctcacccaccttttcctgttattattgttcattgactatcagttggaaaaagaaaactattattgactccttgatttcatgagaaacatcttttattatctactacctccgttcctatatataagaaacaaatgggaacatttttttgttcctaaatataagaaacatatggccacctttaaatgcattaattgctaatttccttctataccctgatttattgtaaagactactaatgagataagtcatacttattggtggaaaaagttatcccttaaaaatgagtagtgtcattaaatgctaccaccacttaaatcagttgattcaatgggtatttttggaataaaattcaaatttatgatattattaattaaagttaacaaaattaactacttttattggttttgatgaattgggtatttgtttcttatatataggaacaaaggtagtattattttggttttattgtttgtctaccttgtgaaagcttttactcgagatttcgacataaaattgactggggaattttgatatagcttcagatattgttacatactccctccggtcctttatataagaaacaaataactaatttgccaagaccaataaaaatatttaagttagttttaattaataatgtcatatattttgattttattctaaacataccatttaaattcattggttgaagcaatggttacatttaatgatactacacctcctccaataagtgtaacttgtatttttgatagaccaataaatgcgtcagaaatgagtggatgcctcattaatggattttcataaaatgaagtgtcaaaatgaaaactagcaattaatacatcttaaagtaggtctatgtttcttataattaggaattaggaccaaaaaaaaatacccttttgtttcttatttaaaggaccagaaggagcattagatatggtatccttttgtcatgggcttattctaggatctacagaattatggtaattaggatatctgtaattaatctctcatttcttaaccatattatataataacactctctgctgtgtagttgacacacagattcagttgtctgttgttttcttttcctttcaactgttggaatactaatttatgtttcataattcatattttgcacaataatatattttgtctgatgtgcaagtcatttattgtatgacaggagaaggaggcacgagacatagagattccaaacattagatgggaggtttttgagccgatgatgaggtcaaataaattctgcattcgtgtgctttatgaaagttgtgctgtgaaagcttgtaattatttgtgaacaacttaaatctttctccagatttatatacactggatcagttgatatcactcttgatattgcccaagatctcctccgagcagctgatcaatatcttttagaaggacttaagagactctgtgagtacacaattgcacaggtcagttatgagaatttttgtgcccacacttgtcctcctgtgcaatactattagactggaaagtagattcctctgatttgatgtttttggtcccaggatatatcactggagaatgtgtcaagtatgtatgaactttcagaggcctttaacgctatatcattgaggcacacatgcatcctttttatcttggagcactatgataaattgagtggaaagccagggtatctatctgaatccctcaatcccgtgtttgctttttctttgcaatacataaaagatgtctgaaagaaataaactcaatctaaatggaataaatatctaaatcatcttgtgtaagttggaggttttaggtcagttcagttgcacctacttttaatgccaatttgtctttattttacttgtagttttggcaaaagcatgtgacaacctaaatggaatattcagatattgaaagttttgggatctacttaaacaatgtcattcttttataggactaaatcaaaactatacggcctgccatatccagtaattatttagttcttcacttgattccatgaacctttcaattttagtgcaaagctgtttcatttaatagctaaatggcaaccagaaatttcatgttatttttattagtattcagatgagaaataatttttttatgtggttatcaaaatatggaaagctgtgtatgatttttctttgtgatttgtgttcaatatattccttatctcttatttctttcttatttattttggctgcatattatcatatttttaattttgtttgcttttgattaatatgatagacagggatcttaaactctttatacccttggtttgaaattttgaaatgaattgaataattaagttggacagtttaaataaatcccaaatatgatgaatgagtttctcgtaaacattacattggttctatgtcttcctaatctttctaaagttttgtttccaccaactactatttgcagacactctcatctgattcagcgtataatacccgagatccagaattactttgttaaagcccttacaaaggccaattccaacatcctgccgtaatgcgctgttatattattgacatctaaccagttgcgatgtacataatgtggttgatgttctttttgttgagcctgcgaagtaaatctcctggatcaagtacagcatggcttaaaaaatatatctaacatcaggtcatgtacgttcatttctgatgctgtgctagtcccgtctagctgtaacgtcattgtcttagatatagcaaaaatgaccttcacgaacattgtttttttctcctgcaatattgtgatggttctggcttgatagttctctttctcaattgatttggcattacaattgttgagtttatgagtagtataggtttcccaagcatctaatgtatatatgacaattagatagttgtttgtgattgctgatgaatgtattgtaaattaaatgcaaatgcatttaaagaattcgtcatttaagccatgctgaattcagttgctgcttataaaaattggctctttgtctatgcagtcaagcggcaacggaatcgaggtttcacgtacaagaattgctatgggtccctaccaacttttagaattcatggaaaaaattattttaccccagttcaaattcaccacatcctctcttcaatgtaatttttttagaatcatggttttatgtacaaaatctttgctggactagattgtggcagggatgagtgatttcacaaccatccctgattaagggaagcgcgattgtggaatcctctctaattgctaataattccccaaagctttgctgctaataattccccaaagctttgcctacgttcacttgattcaagtttaagcatagaaactatattaattaattcacggtactcgttgc

SEQ ID NO: 196 - DNA, 5904 bp, Glycine max
  source 1..5904: mol_type = genomic DNA
tctgattcctgatctcactcaaaccaagcctctcaaggactgattaatttattttgttttcgtttcaccgcgacgctccatggaaaaccctcactatgctgttagaaaaagcttgaagcgcaagctcgaagcagatttaatccacacttccaaacaacttcacccaaagatctctgcaaagattctccgacacgtctctctcctcaactccgctcacccatcctctgtctctgattgtactgccattaagagtgctattgatgccctatctctactcgctgaaaacggtactttttcatttgctaactgaaaatttctcttcaccctttggttgacatctcttcttgccttttgttagaggatcttgtggatactctactgaaatgcggtgtcgtccccgctctggtgaggcatcttcgattgacagacaacgcacggagagatgacggtgatgaggcagactctgtgaaagatgacagtgatggcgttaccaaacattttcagtttgaggtcatcaaaggatgcgcggtcatccttgagcttcttgccattgaagtaactaagttttgctatttcctttctctctaactattttaattatatgaaattgtaactatagtgttggctttagatttatcgatcaaaaggtttcagttcaagccagatgaattatccattgatagatagtcgtgcatgtgtgtaggtgtggaaacttacctgcaaattagataattctaaactacaatgttttagaccctaaatgaatattagtaaataataatttagaatgacttgtcaatcaagatcaacgtttagttttcaactggtggctattgaatatataaggggcgaaggaattggaattgctcatttgttgtgcttgtgccctattgttcttgacaagttcaaagcacccaaggttcctctgaattgtgtttattattcacctgctcaaggagcagctgccatcacagtctttaacagatgcatgttgtaaagaatgtggctgtatggggttaactgctcaatcatactacatacacataataacaatgttgaatttctatgtgcattccatttgatcttctttagcagtatatcagtgtggtccttgtttccaggaaaatgattatgttttttttatagttttaatgcatttctctttttctttgtttcagactattttataaatcatgaagcatcttaactctgattttatttttgctttatctttatcatgaaacagaaagagtatcagcaactcgttgtggatgctggagccttgccctgtcttgttgattggttaaggatgcaaaagatcagtactattgctcaaccacttattgaccttctaaagagagtagctgatgcaataaccagcctagcccatgaaaatactggcattaagaccctagtcaggtttttctcttttttccataccttaaaaaatatatattctacagctgtattctttactcttatatacaaatggtatattcaggatggaaggtggtatagctcctcttgttgaattgcttgaattcaatgacataaaggtacagagagcagctgcacgggccttgcgaactcttgcatttaacaatgatgctaataaaaatcaggtagttgactttttgcagtaaatcgttgtgatagattctgttgatatggttgtttacaagaataaaatattgcagattgttgaatgcaatgcgttacccactcttgtactaatgctccaatcagaggatcctaaagtacattatgaggcagtaagatgcttatatgactttacacaatccaatgtttttatagattgctgcttgcagagttctaaactacttgcactagctgaattagcactttttgtaggttggtgtgattggaaatctggtccactcttcgccaaatattaagaaagaagttcttctagctggtgctttacaacctgtcatttcttcacttaggtaacattatacttcggtcttggcttttcctgtaagcaatccatattattattttgtaatttagtacttttccccctaagtttcaaaatttcaatgacagttcctcctgtccggagagccaaagagaagcagctcttttaattggtcagtttgccacaacagattcagattgcaaggtgatttagttgtgtttcaaacttgtaatatgatcaatctgtcatatatgaaatcctcttattgaattctatattttgtggtttgtgtaggttcatattggccaaagaggggctattccaccattagttgatatgcttaagtctccagatgttgagcttcaggaaatgtcagcttttgcacttgggaggttggcacaggtgattagtctcaatgtgttatgttttttttctattaattgtaccatctttcattttttttatttcattattgtgatcttattgctcctagattgatggtgattgtgtgtgtaaaactgtggtgtattgtttatcatgaatctctttaattttgggtttctcgttttgatttttgattattcatgtgtagtataaattatttagtttccattataataatatttttaaaataacactcactataacatttttagagttatatgctacacaccactgttttaaaattgataatgtgtgtttataatgtagcacatgcaatcttatatggcattgcccacttaagaatttctttaaagttacactaagtatttttggctgaacttggggtttcctttcttaaacctaactcttaatgggtggattttcttaatttatatattaatggcatcaaatgatgcagaaaagctccttgtttctgtaattttatgtgttttttttttaactcttaccattttctagtataacctttttttgtgcacatataattcaaatgtcaggactcacataatcaagctggtattgctcaaagtggaggtatagagcctctgctcaaacttcttggctcaaagaaggttcctgtccaacaaaatgctgtttttgctctctatagtcttgttgataatgaggtgaagtttccttgatctttacttgggcaacattatgttgtccttttggaaatcattgatgtgcagtgataatgtgatatgcttccactgatgtaacaacttgtatgatagaacaatgttgcagacattattaagaaggatggttttcaaaaactgaaggctggaaatttcagaaatcaagtatgttcatttactctttgcattttacttaattgcattccttctcaatttttagttgttattaatgttcactaacagaactcctttctctcaccatttattaaatgggtttccttgtgattgtcgtttaactcgcagcaaactggagtgtgtgtaacaaagacattaaaaagattagaggaaaagactcaagggcgagtgagttttctcgcaaattctatgcgggtgatttagtttagtcatagatgagaattataatctatttaaactatttttaatatatttttacgttattagatatgatttttatatctattccactttggcaggtgttgaaacacctaatacatcttatacgcttggcggaagaagcagttcaaagacgtgtagctattgctcttgcttatttatgttctcctcatgatcgtaaaactatattcattgacaataatggtaaataattgatctctgcatgtttgtaatttctcacccagtgtacttcgaatgtattttcaaatttcaattaatgtggtgctaaatattcaggattaaaattgctgctggatattcttaaatcttcaaatgtaaagcagaagagtgatgcttcaatggcgcttcaccaattggctgccaaagccagttcttctttctctctttttgacatcgctcctccatcaccaactccccaggtatttttgctctttatgtgtgaggttaccacgttcgtttattttgatttttcccccttatttgttgaacaatgtgtactatgttatcataattgaattatttaaattggaatagtaattattgtcttagcaattgaatttctgatattttgctgtgtctatgttaaggggatgaaaataggaagctgagattatttttttcacaatttttgttcacggtatatttgttgattgcatttgctgtagatgtacttgggcgaggaatatgtaaacaatcctaaactttctgatgtcacattcctggttgaaggtgaagtatctgctgttaaaaattttggttagtttgtacacatactcattttgatatctgtactaatttactgtgttttcctttcttcaggtagaagtttctatgctcatagagattgtttagtttcttcggatatctttcgtgcaatgtttgatggcagttatagggtaagcattaattgttttgtaacttgttttcaagtcctcttttcttttatttattctgacatggtctaccaatcagaattcttaatcctttctttctcaacagtttattgtatcgaacacttaacaatcacttttcaattcaaatgggactaaaggatctctggaacttgagctgttaatcttaaatatccatattaatgtcttgaaattcatggtgcaggaaagggaagccaaaaatatagtgattccgaacattaaatgggatgtctttgaattgatgatgaggtgcatcttctgctatccctttctggtgtttttgcaatctcacaataagccttgtgtatgatttgattttctgttggcacttctagatttatatacactggaacagtagatgtcaatttggatattgctcaggacctgctcagagcagcagatcagtatcttctggacggccttaagcgtatatgcgaatatgctattgctcaggtagactcaattgtgtttcacggtttttatttgttctgcttttgtagaaagtttttttttaatggcttaatttaatcacatggctcatctacttattcttataggaaatttctgaggaaaatgtttcactactgtacaagatgtcagaggatttcaatgctacttcattaaaacattcatgtatactgtttatgctggagaaatttgataaactgagatctgaaccatggtatgcacattttttacaacctgaagagtactttcatagtttactgtttttctggtgggctgctggtgtactaagagcattcaattgatgaaatccaacctttcattcgtcactatatgttcttccatcttttcaacatgcaggtattgtcctctggttcgtcacattttaccagacatatgcatgttcttctcaactttacttgtcaagtctcatccagctgactcatgagaatccctagattttagccatgacaggaagaaagttgaaaatgtacaaagatgtaaatgtatgttagatatagaaatcgcagatcattattttttagcatgtagtgggtttctttgactaatgatattattcttgttcgattcgctgactttttcgttcagatcggcggtttcgtcaccaattttggcgatggcctccgatttacgattgtgggtgtggttctagtttggaggttgttgattttgttgttcttgtggttggggttggttgatttggtttttttgttgcatgggccatcgaaggggagggggagggaggagcggcgtgaggagagaaaaagagcttatctgagatgagaaagagacgtgggggtaagagaaagaaaaggaaacaggctgattcttttgcacatcctatcgttccacatcaccactattcaggcatcaatttcgaaggtttgctatataaaaattataacgattgttgttgtaaaattagaccaagtagttgtgtgtgtttatttttaatatttaaaaattataaaattggatatttgaaatccaataaatttacccattggtc

SEQ ID NO: 197 - DNA, 8707 bp, Glycine max
  source 1..8707: mol_type = genomic DNA
cgcatttttggcgaaattccgaaagcaccccttccagatgtcatccattcaaatctccaattccacttcttacccccctctttctcgtcactgtctgttaacttgagcaaacactctgttccttccttctctcgttcgttcatggaacttcagaggcgccaagatcagagcctctcccagcggaagggccagaaacggaagctcgacgaggagcagcaccacgaggaccgccagatcttgccggcgccgcccaccgccgacgagcgcgccgcactcctatccgacgtcgccgaacaggtgagcatcctcgagtcgactttcacgtggaacgaagcggacagatccgcggccaagcgcgccactcacgcgctcgccgatctcgcgaagaatggtaaatcgatgcctcctccgatatcgccgcgtgtcgctgcgttcgtttggattgcggtttcggtgtggtgttttcttcttctttgtttccgcgtgtcacttgcatgtgcgtgtcgtttatgaagtggtggttgtgtttgcagaggatgtggtgaacgtgattgttgaaggaggcgcgattccggcgttggtgaagcatcttcaagcgccgcctctcagtgaccttgtccagcatccgttgccgtttgagcacgaggttgagaaagggagcgctttcgcactaggacttcttgccgtcaaggtagcttgatttttctctaactgttattttggattttatttcatatttaactgtttataactcgtagcttgttttattttgaaactttatagttttgttagatgttccttagtgctctgcaagttctgaagtataagtgagattatggttatagtttgagtcttagtagttgtaaacttgtaatgttcagttcgcttattgagtgttgattacttatttatgcattttaaatttaaatttaattccatttttttttgttaaatggcgcgagtgatttagtaatagtaaagggaggtttcgaattcggctatgtggaattttcggcgtaatatcatcttgaagaatggaaatgctggtggttttatacaatcatccagtatcagcttctgttctgttttgcaagtactgtttctttgagctatcccattccaaagatggggttcaattaaaactaggggaggagaaaaaacgaaggatgtaaggcgaaaggttttagaattgattgaaaatatatattgttatttgtaataatacatatggtttgtcctcgtgcaccaattccataaaccatattaaatcaagcaccttttagttgctgaattatttatttacaagagtttattagttcgtatgaatgcaatttgtttgtctcaaaactggatgtggcatgtaatctctcttaagtttacccttttatgttgttctgatggtagtcggctgtggtggttgctaggaaacatttattgataagagttcgactgaatgcaatctgcttgtctcaaacctggatgaggcacgtagtctctcttaagtttaccctttttcttttgttttgacggtagccaggagtggtggaacttcactgaagaatttgagagggcaaaaaatatggggtctaggtggaaaaaatataatggggcaattcatgaaaaagatgacacttaccttatacaaaatttataagctgtgggatttgctaattttacaatattccttatatgattcaaatactttggatgttttagaaaaaagtttttgatgagaacttgtttaaaattttttaaatgatcacaaattgaatcaaatctcaatatatctgaagaagggtagaagtaatgaacgaaatgtccttaagcagtctacttggtgcaaaaagccatttggtttaacagatgaacaattgatggagggtgaattcttttgaattcttaattaaaacaaatggtcctcatagatttaaaaaataaataaatttggggtgggagtgggggttgggggtagggatgggaggagctgtcttttatggtcctaatgaagatccaccactggaagccagtctgcttattaggtccctaatttttgtttggaactgtggggagtgtgtgagatactattgattttgatttctaaatggcaatttatgtatcctgttgtgtcaattactagattaatttagtcttgtttgtgggatgtgaatagtagcattgctcatctcctttgtaaccatggggaatcccaacatgtgcaatgtttgtctagagtttgtacttttagattgccacataacttttagatttagttgtactcttcttccttttttttttcttaacaaatttctttttctgttaaaataacatataattgctaaactactattttattttaaatgctttctacagcctgaacatcagcagctgattgttgacagtagtgctttaactcatcttgttgatcttttgaagaggcacaggaatggcttaacttctcgtgctattaatagtctcattcgtagggcagcagatgctattactaatcttgctcatgagaacagcaacattaaaacccgtgtcaggttttgcttcttgaatgtatgccatgtatttaaatttagtttggattttgttctcaatattaactggacttgatctataggatggaaggtggaattccaccacttgctcatttgcttgattttgctgatgcaaaggtgcaaagagcagctgctggtgctctgcgaaccctggcttttaaaaatgatgaaaataaaaatcaggtaagtggtcattgctgaaagttggggtttgaatatgtttcaagtaagtcacacaacataatgattttccagatagtcgaatgcaatgctcttccaactttgattctaatgctacgttctgaagatgctgctgttcattatgaagcggtatgggtagtgaaactttagttaacaatgctagatttttcaataatattgagctctttctttccacatcttttatatggcacatgcaatgaattggattttatatcaggttggtgtgattggaaatttagtccactcttcacctaatataaagaaagaagttcttctcgctggagctttacaaccagttattggattacttaggtatattctcagttctagaccctgataaactgcaaggccccttccctccccaccctgaatttgttttgttattataattataatatgcccatttttggttctagcaataatattcaatcagatatattccgtggaaggtatctttcaaataatgtattataatgtttcatttaacagttcctgctgctctgaaagccagagagaagcagccttgttacttggacaatttgcagcaactgattcagactgcaaggtaatcataagcttcaggatggaaaggacaacaacaaaactttaattgggagctattgtttaataactccagttttcaagttcgaactgcttcattttattatattttgtttttgatttggactgaagggggaaagaaagataggaggggtgatagggaagagacccttactccacttttatgcttgtttacctgcataatgaagaggggtggaaaggaaacagtccatgactgagctttctttgggggcaattgtttcataaccatttccaagtttgattgttctgtattatttatttcttgttaagtcaagatttcgatggtcagagtactggaagtataattgctactcttgtgatgatgtatcatatattatattctgtgtcccttagtttttactttttgttactcttggtctttttaggttcacattgtacagagaggtgctgtccgacctttgatagagatgcttcagtctcctgatgtacaactcagggaaatgtctgcttttgcattgggaagattggcccaggtttctttctttttttttcatgtttataattcacttgcattcgttgggaatttaaagttgccattatatccttggaaataactttgtattttctctctctgtataatagtttttggatctgtaacacattcaatgcatttccatctttgcattttcaggacccacataaccaggctggtattgcacacaatggtggcttagtgccgttgctcaagcttcttgactcaaaaaatgggtctttgcaacataatgctgcttttgctctttatggccttgcagataatgaggtatgatataactgagaattcaaatgaaatgaagatattctgtcttaattgcttttaaaatttgttactttgagacttaattaactattctctgtttttgggctatttattttattttgtcccttaggataatgtgtccgatttcattagggtaggtggagttcaaagactgcaggatggagaatttattgttcaagtaagttttttctttaatagccactttagctttgatttcagggtttctgcttttacccttggatgcctatattaaagaaaattaaaatacttaatgattgcatctgaacatttgtaatttttaagaacaggaggaaaatagttcatctttgacctatattgatctttatggaattggtttttattgcaggcaactaaagattgtgtagccaaaacgttgaaaagattagaggagaagattcatggtcgtgtaagatgtcatattcatattactttctgcattttgttgtaaatatcatggaaaatgatgggtgttctactgggtaccctgttgtttttttagtttttggagttttgtgttcaaatttataatctgatatttttcttttctgtaggtgctgaaccatttgttatatctcatgcgagcttcagaaaagggctgtcaaagacaagttgctttggctcttgcacatctttgctcttcagatgatcagagaataatttttatcgatcactatggtatggatcttcttgctaaaatgtttgtcatgggttttgttcatgttttttttttgttttataaattcctttatgtgcttgttctattctgaagctgagcaattctccatgcaggtcttgagttgcttattgggcttcttggctcatctagctctaagcagcaacttgatggtgctgtagctttaagcaagttagccaataaagccttgaccttgtctcctgtggatgctgctcctccttctccaacaccacaggttataaataaatggtccatttaaataatgagcatctaatgatctaagaatcagcagtcattatgatttatgatcaatgcttgctgttttacattcttgccacttacaaaagaatcctgatgctgagctccctcttcactctgccttggctaaataattctcaaattaggattttctaaaagctgttatatttataactgcagactattcttcttgcaggtctatttaggagagcagtatgtaaacaatgctacattgtctgacgttacatttttggttgaaggttgatgccttttgtccacattgtttcattcgttaaactgttggttgaaaactaccttccctgaaatgtggcgttgtaacttaagttggcaggtgaagttaattgggtgatctttgttcttcattgcaggcaaacgattttatgctcatcgaatttgtcttcttgcatcatcagatgcatttcgtgcaatgtttgatggtggttacacggtgagtttatatttagcttcaccaatgaatcatctttctccttcctccccacccctaaagcccctccaatgaatacacatgccacaaaaagcaattttttttaattccattatataatagtgttttaccgtaatgttgtgtgtcaatgtagaccacacctcatgctatttataatatgaaaaaagatcagtattgattacaagatcaatcaattactgattaataagaaatagaatattctaataataaatacaatgtcaagaacaatatcaagacataatctcactctccttcaagttggagcatatatgtcatatgaaccaagcttgttacaaataggtaaacccaacataaacgaaaataaagatgattccaattgtgtggttgcgccaaaaaaccttggttgcagccaacgaaggcctctagtggcaatgggtattgttcacccgtgaataaagcacgctctgaggtggttccagtgtgactcttgtcggagatgcatcatgcattgtgtccgtgaacttctctcgtggaaaagggccctacgtggggttgatgtgacagtgtgttgaattggctgcaacgtgattggcgtggcattcttgaaaggtctctgatgcagactgataagagggtggcacattggttgccaaacaagcccaatagtgagggtgcacatatgtgtctgtgtgagggacattggtgaacgtcgttgcagaagcggattctgaaggagggtcaattgaggccatgaaacacatcgaaacagggccaaacaaagtgaaatagagtagatggaggaagaggaggatgacagcatggtcgccaaatgtccggcgagtttgtatgtgatgtcgccagctggaaaagagtggtggcacatatgtactgtatggcgcttagaagaaaggagaaagggccgtcaaaagaaggacaacgagcagaaaggtccactggggacagtaggtccttggtggagaatgactttcattattcctctatcaagaataatctggctctgataccatataacagtcttttactataatgttgtgtgtcaatgtagaccacacctcatgctatttataatatgaaaaaggaatcaatattgattacaagatcaatcaattactgattaataagagagggaatattccaataataaatacaatatcaaaaacaatatcaagacataatctcacacattacattattagaaaaaaaaaagtatgttggtcataaaaataactcctttattgactccacttggtttcatgaggtatattatttatcacctatgattttggctgttgatttgaatggtgaatttaaatatagtacataactatcaaaacttgtgttttaaattgaagcagaaagtgatagttaatgtcagtggcctaaaaatgtgttttattgcatggcaggagaaggaggcaagggacatagagattccaaatattagatgggaggtttttgagttgatgatgaggtctagtaaattctgcaatcatgtattttattatagttgttcagtgaatgcttctaataatttctggacaacttatatcttgtttatttgatctttatccagatttgtatattgtggatcagttgatgtcactctggatattgctctagatcttctccgagcagccaatcaatatcttttggaaggacttaagagactctgtgagtacacaattgcacaggtgagctaggaaaattggttttatatatgtatatatggatgtatccctgtactaaatattagacttgaaagtgggttcctcattaccccttgttttttgtcacaggatatatcgccagagaatgtgtcaagtatgtatgaactttcagaagccttcaatgcaatatcattgaggcatgcatgcatcctttttatcttggagcaatttgataaattgagttcaaggccagggtatttatctgaatccctcaatactgtgtttaattcttgtgggtgtttttttacctctacaatgtcttaatagccgagtataatgaacttggtcattgggtttagcagttcattgcatgttgtttggtgaagtatattgttgacttaatttcttaaaataaatttggatcttgagacttgattaatgattactttcactggtgtaagtaaaaaaaatatgcaacctattgtatccgaatatgaataaggacttagttttttgggtatcataaatttatcatgcatactgatttgtggtagacgaggttttctatagctgggcatttgctgtttattttcttttttgcaaagttgttatcttagttcttgcttttgacaaaaatgatgccatcctttggtttgaaataaactggatagttcagttttaggaggttgcttcagtgcagtttctggaggttgccatcttacttaaaatatggatatgatgatagaaattcacacttatctgtgcattgtttgtgtctaattcttcagcttatattttttgcaggcactctcttctgattcagcgcataataccagagatccgcaattactttgttaaagctcttacaaaggccaactctcatgacaaccaactgtagtatgcacccattttattcttgacctctaaccgattgtgttgtacagaatgtagtagatgttattccttttgttgtaccaggtagcagtctcctgtatggtatacagcttgggtaaaagaaatatctaacgccggagtcatgcttcttcttctttttaaatgaggtgtaagcccctttgtgtctgtaacgtcattatcatagatatagcaaatatgaccttcaggaacattgtttttttctcatgcaatgtgacggttatatgacttaacagttcttctctcagatagctacgttcagggaattaccattgttgactttatgattatatgtgtaaatattgtttcccgtgtatatatgaacaagaagttttctgcaaggaaattgtgccgctggggttacttctgccagaccattaaattctgtcacctgacatggaatgtgttgtaaattattgttgcaaatacttcattcaaatattcaaagtcgaaggcatg

SEQ ID NO: 198 - protein, 705 aa, Glycine max
MEKRYPVARRSSKRKLEADLTEDQTHTKASKISAKILKQVSLLNSAAIPFTALDCATVKSAVHSLSVLAANEDLVDTILNCGVVPALVRHLRLTDNMRKYDGHEAETVKDYSDGVTEHDQFDVVKRCAVILELLAIEQEYQQLIVDAGALPCLVDWLRMQKISTTSQPLIDLLKRVADAITSLIHENNGIKTLFRMEGGIAPLVELLEFNDIKVQRAAARALRTLAFKNDGNKNQIVESNALPTLVLMLQSEDPKTHYEAVGVIGNLVHSSPDIKKEVLLAGALQPVISLLSSCCSESQREAALLIGQFATTDSDCKVHICQRGAIPPLVDMLRSPDAELQEMSAFALGRLAQDSHNQAGIGQCGGIEPLLKLLDSKKVPVQQNAIFALYSLADNEDNVAAIIKADGFRKLKAGNFRNQQTVECVAKTLKKLEEKTQGRVLKHLIHLMRFAEAVQRRVAIALAYLCSPHDRKTIFINNNGLKLLLDTLKSSNLKQKSDASAALHKLAIKASSSFSLFDIASPSPTLQMYFGDEYVNNPKLSDVTFLVEGRSFYAHRDCLLSSDIFRAMFDGSYREREAKSIVIPNIKWDVFELMMRYIYTGTVDVNLDIAQDLLRAADQYLLDGLKRICEYTISQEISEENVSLLYKMSEDFNATSLKHSCILFMLEKFDKLRCEPWYCPLVRHILPDICMFFSTLLVKSHPTDS

SEQ ID NO: 199 - protein, 707 aa, Glycine max
MELQRRQDQSLSQRKGQKRKLDEEQHHEDRQISPAPPTADERAALLSDVAEQVSILESTFTWNEADRSAAKRATHALADLAKNEDVVNLIVEGGAIPALVKHLQAPPLSDRVQNPLPFEHEVEKGSAFTLGLLAVKPEHQQFIVDSGALTHLVDLLKRHRNGLTSRAINSLIRRAADAITNLAHENSSIKTRVRMEGGIPPLVHLLDFADAKVQRAAAGALRTLAFKNDENKNQIVECNALPTLILMLRSEDAGVHYEAVGVIGNLVHSSPNIKKEVLLAGALQPVIGLLSSCCSESQREAALLLGQFAATDSDCKVHIVQRGAVQPLIEMLQSPDVQLREMSAFALGRLAQDPHNQAGIAHNGGLVPLLKLLDSKNGSLQHNAAFALYGLADNEDNASDFIRVGGVQRLQDGEFIVQATKDCVAKTLKRLEEKIHGRVLNHLLYLMRVSEKGCQRRVALALAHLCSSDDQRIIFIDHYGLELLIGLLGSSSSKQQLDGAVALCKLADKASTLSPVDAAPPSPTPQVYLGEQYVNNATLSDVTFLVEGKRFYAHRICLLASSDAFRAMFDGGYREKEARDIEIPNIRWEVFELMMRFVYCGSVDVTLDIAQDLLRAADQYLLEGLKRLCEYTIAQDISLENVSSMYELTEAFNAISLRHACILFILEQFDKLSSRPGHSLLIQRITPEIRNYFVKALTKANSQNDRL

SEQ ID NO: 200 - protein, 708 aa, Glycine max
MELQRRPDQCLPERKGQKRKLEEEFDDDPQISPPPTGDARDALLSDVKEQVSLLDSTFSWNEPDRAAAKRATHALADLAKNEEVVNVIVEGGAIPALVKHLQVPPLPLPETDRVPRPMPFEHEVEKGSAFALGLLAVKPEHQQLIVDSGALKHLVDLLKRHKNGLTSRAINSLIRRAADAITNLAHENSSIKTRVRKEGGIPPLVHLLEFADTKVQRAAAGALRTLAFKNDENKNQIVECNALPTLILMLCSEDAAIHYEAVGVIGNLVHSSPDIKKEVLLAGALQPVIGLLSSCCSESQREAALLLGQFAATDSDCKVHIVQRGAVRPLIEMLQSSDVQLKEMSAFALGRLAQDTHNQAGIAHNGGLMPLLKLLDSKNGSLQHNAAFALYGLADNEDNVSDFIRVGGIQRLQDGEFIVQATKDCVAKTLKRLEEKIHGRVLNHLLYLMRVSEKAFQRRVALTLAHLCSADDQRKIFIDYNGLELLMGLLGSYNPKQQLDGAVALCKLANKAMTLSPVDAAPPSPTPQVYLGEQYVNNVTLSDVTFLVEGKRFYAHRICLLASSDAFRAMFDGGYREKEARDIEIPNIRWEVFEPMMRFIYTGSVDITLDIAQDLLRAADQYLLEGLKRLCEYTIAQDISLENVSSMYELSEAFNAISLRHTCILFILEHYDKLSGKPGHSHLIQRIIPEIQNYFVKALTKANSNILP

SEQ ID NO: 201 - protein, 704 aa, Glycine max
MENPHYAVRKSLKRKLEADLIHTSKQLHPKISAKILRHVSLLNSAHPSSVSDCTAIKSAIDALSLLAENEDLVDTLLKCGVVPALVRHLRLTDNARRDDGDEADSVKDDSDGVTKHFQFEVIKGCAVILELLAIEKEYQQLVVDAGALPCLVDWLRMQKISTIAQPLIDLLKRVADAITSLAHENTGIKTLVRMEGGIAPLVELLEFNDIKVQRAAARALRTLAFNNDANKNQIVECNALPTLVLMLQSEDPKVHYEAVGVIGNLVHSSPNIKKEVLLAGALQPVISSLSSSCPESQREAALLIGQFATTDSDCKVHIGQRGAIPPLVDMLKSPDVELQEMSAFALGRLAQDSHNQAGIAQSGGIEPLLKLLGSKKVPVQQNAVFALYSLVDNENNVADIIKKDGFQKLKAGNFRNQQTGVCVTKTLKRLEEKTQGRVLKHLIHLIRLAEEAVQRRVAIALAYLCSPHDRKTIFIDNNGLKLLLDILKSSNVKQKSDASMALHQLAAKASSSFSLFDIAPPSPTPQMYLGEEYVNNPKLSDVTFLVEGRSFYAHRDCLVSSDIFRAMFDGSYREREAKNIVIPNIKWDVFELMMRFIYTGTVDVNLDIAQDLLRAADQYLLDGLKRICEYAIAQEISEENVSLLYKMSEDFNATSLKHSCILFMLEKFDKLRSEPWYCPLVRHILPDICMFFSTLLVKSHPADS

SEQ ID NO: 202 - protein, 686 aa, Glycine max
MELQRRQDQSLSQRKGQKRKLDEEQHHEDRQILPAPPTADERAALLSDVAEQVSILESTFTWNEADRSAAKRATHALADLAKNEDVVNVIVEGGAIPALVKHLQAPPLSDLVQHPLPFEHEVEKGSAFALGLLAVKRHRNGLTSRAINSLIRRAADAITNLAHENSNIKTRVRMEGGIPPLAHLLDFADAKVQRAAAGALRTLAFKNDENKNQIVECNALPTLILMLRSEDAAVHYEAVGVIGNLVHSSPNIKKEVLLAGALQPVIGLLSSCCSESQREAALLLGQFAATDSDCKVHIVQRGAVRPLIEMLQSPDVQLREMSAFALGRLAQDPHNQAGIAHNGGLVPLLKLLDSKNGSLQHNAAFALYGLADNEDNVSDFIRVGGVQRLQDGEFIVQATKDCVAKTLKRLEEKIHGRVLNHLLYLMRASEKGCQRQVALALAHLCSSDDQRIIFIDHYGLELLIGLLGSSSSKQQLDGAVALSKLANKALTLSPVDAAPPSPTPQVYLGEQYVNNATLSDVTFLVEGKRFYAHRICLLASSDAFRAMFDGGYTEKEARDIEIPNIRWEVFELMMRFVYCGSVDVTLDIALDLLRAANQYLLEGLKRLCEYTIAQDISPENVSSMYELSEAFNAISLRHACILFILEQFDKLSSRPGHSLLIQRIIPEIRNYFVKALTKANSHDNQL

SEQ ID NO: 203 - DNA, 11478 bp, Pisum sativum
  source 1..11478: mol_type = genomic DNA
ggtttgtgtatttggggataggtgatcaattagaccaatgatattattacacgtggataaaagaagggttagagaaatgaatttaatcccaatttgttaattaataaataattcttatagtagtttaaaaaatctaaaaaaaaagggcagtattgacaaaccatacaattattttatgttggatagaatagtagaagtaaaactagaaggtaagtttttctctatttattactccaaatgagtttgatttaataaattttgatttgattaaaacaagttattattttccgtttacatgtaccttgcccgaaatacccctcccatctgtcatccattcaaatccgaatttccatttctcgccattttctatctattctctctctccccctctcctttctgttaaccagagcgccaacaacacactgtaaaaaactcgcctcttcttctcttgtccatggagtttcagcgacgccaaggtcactgcctctacgagaggaaggggcaaaaacggaagctagacgaagaatcgcaggacgaaccacagatctcggcggcgccgcctacctccgacgagcgtgcggcagttctaactgaagtggaaaaccaggtcaacatcctcgagtcgacattcacgtggaacgaatccgaccgagcagcggcaaagcgagctactcatgcgctcgctgatctcgcgaagaatggtaaatcgatgtctccgatctcgccacgtgttacttcgttcgcttgaattgatatggaagtgtggtgttattctctgttcctgtttatcgctcgcacgtgcatgtatgaatctattcgtggttgtgtttgcagaggaagtcgtgaatgttattgtggaaggaggtgctattccggctttggttaagcatcttcaggcgccgcctgtggaggattgcgataagaaggcgttgccgtttgagcacgaagttgagaaaggaagtgctttcgcgctaggacttcttgccgtcaaggtaatttgatttgtatgcaactgtttttttgttcttctttctgaaattccatatttaattgttttgaagcatatattgacaatttgtatgactaagggaaatgaatcagttgaagacttatttcatattgaatctacttattgagttgaatgataataatgctttttgtttcgataagtattagtattttggctaaagtatacaagtgaattgttaagccatttgtaggtgacatgttagaaatgagaaacttagaatagaacaggacaggagttggcataattagacggaggaaatatatcatattgattccatttctttttacgtgcatttaaagctatcaaatagcggcgccatggccgctgacatagctgttttttggctcgctacaatggtaaatatcggccgatattgcgggttttccccaccataatccactacaatggcgccttatagcggctggtatggcgggattttaactctcatggcgggattttaactcccatggcgggattttggctctccgccatggatcgccatccgccatcgacaacactgatttaaagattagagcacaaccagacacagttaaataaagttgtatgttttgatatgttaagagtttagctgagaagagcataacacactgttcctttctgttttattttcatatattaaacactataaactgtagtatacgtattatgtggaattttgagtgtgtcactgtcaattttaatctggttcttatttttatttttatttttaatacacaattacgtggaaatgttgatgttttatatcagcacccaatgtcagtactttttgtttaatttgttttgaccttaccgttgcttcgccccattccaaagacgagggatcgaaactggatgtacttgggtaaacataattttaaatgacaaggtagttttataaaatttattttggttataatatagtttgaagtaaaatgataaatatttggatttatttattacttctagtcaaactggtttagagggataatcattttttttcccgatagtaactattttaactaaactcacatcttttgtgaagtaaaatcaattttgttactactgtgtgaagccaaacacactaaatcacatagaagagccaaggaaaccaagcttatcaagatcgggaggggatgataagatcgtaaaacataagatcggaagatcctacccaattatttttgtaagatcgagaggggatagcaagatcgttaaacataagatcgtaaaaaaaatcgtaaaatattactacaataagtaatactctatatatttggagatttttacatgatgatttggtaggcaagtgtattcgtgggataatagcctccgacgaaccataattgttgcgcattggcatcttatcatcttctcggcttgtaatggtggtaagtgtagtcaagattgagtgctggatcgtaagatcgtaagatcttacttgccaaggatgcctaagagtgttacgattagagaaagatctttttcggtgccggtgtggtcaagatcgagatttttgaagcaagatcgtaaaaaaaaacgtgttgggcctttttttttgggcctaaattataattttcatgttttagttaatgtgtgtgtataaatatatatgaaattaccatttttccctttggtagaatttcgcatgccatgctaatgatccgagttttacgatctttcacaagccgtacgctcctacttaagatctcgtgcttgactacattgatggtggtggccaaaaatcggctgatcgtggccggaattggtcaagatcacactaaatcaatgtttttacgactttttttcaatgtttggctacaatgcacaattctactttcgtcaggggtgagtgagatcgcaaaattgtaaaattttaagatcgtgatcgagatcttggcaaccttgaaggaaacaaccatatccagtcataatttaggggcggaccgcaattaaggcggaaattccaacaataggtttaaaatagtagacaatagatcgggagaagggagctgtttccgttggtcctaacaaagaaccagcatttcgatttattctgggactctggtgagtgtgtctcttgctatgggttttggagttctaaacattcatttatgtatcctgtttcctttataaattcatgtgccgacactttccatgacgagtaccgtgtcacttttcaccagattttgcataatatatatgacatatatcatgtatatataactcttagccacacttttcttttggacaaatttatttatctctaaaagaaggtataattgctcaattactatcttatttgaaatgctttctacagccagaacatcagcagctaattgttgacagtggtgccttaacttaccttgttggtcttttgaagaggcataaccaaggcttaacttctcgtgccattaatagtctcattcgtagggctgcagatgctattactaatcttgcacatgagaatagcaacattaaaacctgtgtcaggtttgcttcttcattcactaccatatatgtagactcaatttggattttcttttatttcttagtattatatgtggactttatgtgtaggatggaaggtggaattccaccacttattcatttgctcgagtttgccgatacaaaggtgcaaagagctgctgctggtgctctgagaaccctagcttttaaaaatgatgaaaataagaatcaggtaggtggtggtcattttttgaaagttgagttttgaatatgatacaactagtaacacaacatcatgattgccagattgttgagtgcaatgctcttccgactctgattctaatgttgcgttctgaagatgctgctattcattatgaagcggtatgaataaggcaacttcaattataaattataggttttgcaataattatgagctgtatttctcatccaccacatgcaattaattggattgtattacaggttggtgtgattggaaatctagttcactcttctcctactataaagaaagaggttctttttgctggtgctctacaaccagttattggattacttaggtatattatcatctctggactctaattttgcaggtctctggactccaatatttttgtttcttgactataatttctacagtatatagttaaataggcatgtttcaattaatgtattcttataactttcaatagctcctgctgctctgaaagtcagagggaagcggcattgttacttggacaatttgcagcaactgattcagactgcaaggtaaatataaacttcacaactgaaaggatagtcaaaaacttagtttaaagtaatttttcaaaaactccaattcaaactttcaagtttagctctttttcctttattgtatattttatacttgtactaaaaggaaaatgagattattaagctgggaggaattcataattccatttttatgcttgttgcttgagtagttaagacttatgagagatagaaaagacataatcaactattgaacttctatatttggaataaaacgactaagttttagttgggggcaattgttcaacaactacaattccaagtttggttgtgttgtattatgtacatcttgttataataaagactccattggttgtagaatagtacctccatttttttggtcactttgccaatttcagacttaataaaaaatgtagttaattttgtatgggaaataaattacgatagatcttacaaaattattcttcattaatgatataagaaagaaaaattaaaagaattgaaaaaaagaggaagtaataaatagtaaatggtatgataggaacaaagacattaatgtttcattggtatcgtaaagtgacttataatttggtccaattatcttttgcaaagtgacaataaaaaatagggtagtaattgattacattggcgctagtgctactcctgtggctatgatgttgcaccatatattatatgttcttgctcacacttcttaccattcattccacttggtctgtttaggttcacattgtacagagaggtgctgtccgacctttgatagagatgctttcgtcttctgatgtacaactcagagaaatgtctgcctttgcactagggagattggcccaggttattttcttttcttcttttccttatttataattcaactgatttgccattagattcctggaaacatcttatttttttctttccttttgtaatagttttttgtatttgcaacacatcttatacatctccatcttcccgttaatcaatgtatctagtgggctcatagaacatactgttgaaatataatatattatttccttttcatattgttctaaatttatgtttattttattttccatctatctttcctgaaattatggaattgattgattgtttttctcctatataaggatcccctgtattcataacaatatatgacaatattattctctacaataactcatctcagtaatatattacaacattttatatacagtacaatgtttccatatataggccggttctttttaacatataaacattccttttggtatgattgggtttttcccctccaatttcaggacacacataaccaagctggtattgcacacagtggtggcttagtgccactgctcaagcttcttgactcaaaaaatgggtctttgcaacataatgctgcttttgctctttatggccttgcagagaatgaggtatgatataactgaaaattcaaataaagtggacatcttcagttttacaacatcaacaaccatgcctcgtttcactaggtgggactggctacatggatcaaaccataacattatatcacaatttgtgttaatacccaaaccattgacctcaatctttcttagatgttttgcccatagtttttcttggctttcatctatctctagcgattgagccattctccatcatatctacttccctatactaaatctgcaggactcctccacacatatttagaccacctaagtctatcttttctatgaataggtgctaccccaactccctgtctctaatgtaatcattcccaatccttttgtctagtattattatttccactcatccaacacaacattcgcatccttgatactttgagtttatttccatgttggcattttaccacccaacagtctgcgtcgcacatctgttttatcttttacatgagcagtatctcttcatcacatacagactcaaagacctccgtttcaaccaccccacttgaatgctatggtttacatatcctctaatttaaatagtggttatttcaaaaacataagcaattaattattctcttttttattttatttttccctacaggataatgtgtctgatttcattagggtaggtggagttcaaagactacaggaaggagagtttattgttcaagtgagttttctctttaatacctacttttagctttgattttctatccttggatttctgtataaaagggaattaccgaatggaggaaaatagattcttcctgggtgtatattgacctatatggatatgtctattgcaggcgactaaagattgtgtttccaagacattgaaaagattagaggagaagattcacggtcgtgtatggcgtcatatttctacattttgttgtaactagcatgggaaatgatgaacgtgcaactagtgtttcaattatcagttctatatgttcttgctttcaaatttgtaatccatcaattttcttcttataggtgctgagccatctattatatctcatgcgtgtttcagaaaggggttttcaaaggcgaattgctttagttcttgcgcatctttgttctgcagacgatcaaagaagaatttttattgaacaccatggtaaatgcatcttcacagcaaaatactttaacgggtttgatcattgttgtttcatgttgtataaactcctttttgttcttctatttcaaagttaagtgtctgtccatgtaggtcttgagttgcttattgggcttctttgctcatctagcaccaagcagcagcttgatggtgccgtggctttatgcaagttggccgataaagcatcaactctgtctcctgtagacgctcctcctccttctccaacaccacaggtaggcttaaatccatttggattttcctcaatcctcaaaatctctgtttaggcttactcccctgaagctcatatataagagaattaacaaaaaaaactcatatataagagaatttaaaaaaaaaagctcaccctttaagaaaagagattaattactatacactgtcagtgtaaaaagttttacaccgtcggttcatcaccatcacccgtttgtatttcaattaatctcttaagaaaaatgtctgaatgcattaaattcttgtgctgtttctaattttattcatatttttttgctttggaaatcgttacaaagataaaatgtaaaaaaaagtaggggtatatttggaatagtgacattgaatgtaataattatagatggcttttgcttatatttaagactattgaaatttttgttgttgtttatatttgaaaccggagggagtattaaaatacaaaggctttctttataatgtgaataggctttagccaaagttatcaatcccagatagcagaacgtaacaaagttatcaatcccaaatagcagaacgtaacggcaaccccaaaaatggaatagtgagatagcggataaaacacataacacaatatccataaaagaaaaaaaatagtagaaacagagtaagtaaaagtgaaagaggaagaagaggaataaacttattaaaatactattacttcgaaaaaaacactggataaatagtcaactgccatataaacatttatgcagtttattataataattaatagtatcaatcccagcctaggaaatctactacattaatatatacattaatgcactttattatcctaatgaataacaattaggattattctaaggataatactaacttgtgccctagaggtacatgttaagaaattcacaaataaaaaatttgttttgggaatagaaaatttgtattgaaaaaagtagttaaagaattaattacaagctttttataaaatcaaaaaacaattttcaaaaaaatatttctatgtttagttcttaacttgtgcccttagcattacccttatttattctaattagcaaatatcagttagaaatccggacactaaacctaatgacagaaatagcctaagtaaaagagcaagaagactttgaaaaaaaacagacagaggaagaaagaagaagaaaggaaagaagagaaaagaagtagaaaggaaagaagagaaaagaaagaagaaaggaaagaagaagagaagaaaacttgaaaaaatgtcaagcgaaagcgtgtgagaaaaagaccgattactctgttttgtgttctgtgttctgtgttcttttttattaagggtagatctgggttttcgctttcgaaactgatgaaatccgctcgggccaggaagcactccgctcccactatccgctaaacctcaaatagggtccgctatctcaaactaggatgagaaccgctcctccatagcggagggtcaccgctccgggacgctatcccgggatagcgcccgctatcgataactctggctttagcctttatgtattcaaaatagttagttttttcttttttctttttgatctctgacatgggaaaatgatgtatcctttttttatatcaatccttttttcactgatatgacctttcaacacacattcaagaagttaggagtgaggttttattttattttttattgcatacacaaatcctaccctttgtttaaaatactttggtatgtatgtttttcttatattgttcacatgccacgtatagtagtcagtgggtagtacaaggacttcttaatggacttacattatacatatgacattttcggactgctgtgttggcattttaaaagtatgtgaatacaagtgatggtgccttgttaataatatatggtccatttaaaatgagcatctgatggtttaataaccagaagtaaatatcaatctcttgctgttttccatgccttccacctgcataagaatctgggtgctgagctccctcttcattctatcttgtctatgtaattatggagtgaggtgttcctaaaggctggaatatttatgattatagactattcttcttgcaggtctacttaggagagaagtttgtaaacaatgctacactgtccgatgttacatttttggttgaaggtgatgatccctttcgttcacattgtttcactcttaaaactgttgcatggctaccttcttagatatggtttgtagcttcagttgtcatttacagttcatcgcgtaatctctgttcttttttacaggcaaacgattttatgctcatagaatttgtctacttgcatcttcagatgcatttcgtgcaatgtttgatggtggttatagggtgagtatgtacagagctcccacaccgaatcatatattcccttccctaaagaagctcccccaagaaataagataccacaagaagcaatttttcttttcttattacaaaaagtgtagtctaaatgaagaaagactgctttattgactttacttgttttattgagctacattatttcatccaatgttttttaattttttttattttcgtgctctttcaacctcttgataacttttactggaaacttagctgagttgaatggtgaatttgaattgaagtgtataaccatcaaaacttctattttttttcaaagcagaaaccgattgaaatgtctctgatgtacaaatgtattttattgcatttccatgacaggagaaggatgcaagagacatagagatcccaaatattagatgggaggtttttgagttgatgatgaggtccaataaattctgcagtcatgatttataaaattttaatgtgaaagcttctaataatttgtggatatgtctttaagtttatttgatctttgtccagatttatatatactggatcagttgatgtcactccagatattgctcaagaccttcttcgagcagctgatcaatatcttttagaaggactaaagagactctgtgagtatacaattgcacaggtgagttaggaaaattggttgtatggacaatatttactctatttctcctagaaataactctcgccagatgaatctttgtgtgtgcaacatgagtgcctcatgacctgatgttcttgttgcaggatatattactagagaatgtgtcgagtatgtatgaactttcagaagccttcaatgcaatatcattgaggcatgcatgcattctttttatcttgaagcactttgataagttgagcacaaggccagggtattgatctgattccctcaattctatgttggacatttatattgaactaactacttggtactagtacattgtttagtattgctccgtcttcatgtttgttgtagtttcggtgactatgttctttatctaaatggttgttgatatgtgaagtaccatgtactgaaatgttttttctagctttttttgagcaaggaggggcatattgtgacgtgggctcaatttatagctggcatcacttccttttcttttcttttcatctcggcttgttatgttatgctcttagttttgctttgctttgctttgcgttagacaaagttcattcggagggatactaaactgtattagccatagattttatggctgaagataccaacctgaggtttgaaataaactgaatagttcagtttcaccaggttgcttagtgcccaatttgtttagaatggtctcatgcttaaaattttatgatgattgaaattcacatttaccgtagcatcgtccctgtcttaattcttcggcttcttgattgtgtgttgcacaaattttctgcaggcactctcttctgattcagcaaacaattccagagatccgcaattactttgttaacgctcttacaaatgcgaactcccaaagacagtaatgtgcagacattctattcttgacctctaaccaattgtgatgtacagaatgtagatgttattgcttgagttgaaccaggaaaagggtctctcccttatggtatatatgttgattaaaagaaatatctttcttttttatccttttcattgatgcggtgtaaacccctttctctccctagcatatcatagatatagcaaatagccttcacgaacgttgttttttcttatgcaatactgtgagggttctatttctcatgtgatttgtacattcagggaattaggaatgttgtgtttatgatgataaatgtaaaatattgttatattgttccccaatgtatatatcacaattagatacaaaaaattaaactgctgggtaatttatgccagaccgttaaatcctttatctgacatggaactgttgtaagctattgtggcaaatactttatttaaatactcgtatggtccaaacttttatttc

SEQ ID NO: 204 - DNA, 8902 bp, Pisum sativum
  source 1..8902: mol_type = genomic DNA
agtaagttgactcatacgtagtgtaattagtaattatctttttgtaaattgaactgtttaccgcttcggaattcgaactaatgcggccgtttcacaagccgacacctttcttcatcttcggacaaaagaaacaaaaaaccgaaaaagaatacatgtgttattccacaagtgcccccaatctggaactccgtattcttcatctgttttcaaaatcccaaatccttttttttggatcactcttctctctctctcacctcattttccgttacactgtttctcccgtgtatctctaacttccacactcagagagagagagagagagggtgaggagagagagagagaaggagggaccttcttcttcttcttcttcttccttttgttggttgatggagcttcagaagcgtccagatcataacctaccggagaagaaaggccagaaaaggaaactggaggaggaatctcaacaggactcacagatctctcttcctcccaccggagacgcacgcgacgcacttatatccgacgtcaaccaacacgtttcaattctcctttctactttttcatggaacgattccgatagagcttctgctaagcgcgccactcacgccctcgccgatcttgccaaaaacggttttaaaattttcattgctcttgcttccttaaccgaatttccttgcatgccttgttttcggaatcaattcttctgttgttgcatctgcagaggaagttgtgaatgtgattgttgaaggaggcgccgttccggctttgattaagcatcttcaaccgcctcctttgcctgaacacggcgcgccgaagccgtttgagcatgaggtcgagaaagggagcgcattcgcacttggacttcttgcagtcaaggtaacttcacttcagcgtatttatgaattattgccgctgagaacttatttcggttttgaattctatattctgaactgtatgccttttgttagaactccatgatagttatttgtattctattagtatatcggtggaagaggtattttgctttatatttgcttacaagtgttgattatgttttcaaacttgaaatgttatttattcctctagtccagtgttatataatcagattatttaggttactgatatgaaggaaggattttagaatggtatagggaagtttacaagataaatatattgaattattccttagtccttacctaaactattttgtttgcaatgcattcattcttcagccagaacatcaacaactcattgttgacaacggtgctttgaagcatcttgttgatcttttgaagaggcataataatggcttaacatcacgtgccattaatagtctcattcggagggctgcagatgccatcactaaccttgctcatgagaacagcagtattaaaacccgtgttaggtttgcttcttcaaggactaccatacaaatgaaatttagtttgaaatgattatgtttataatgatctggagttaatgtgtaggacggaaggtgggattccaccattagttcatttgcttgaatttgcggatacaaaagtgcaaagagcagctgctggtgcattacggaccctcgcttttaaaaatgatgaaaataagaatcaggtaagtgacctttattgaaaaatggggatttagatgaattttaaaatgatatgagtgtatgagtaagttacataacatttgtcacaacttgtcagattgttgaatgcaattctcttccaactctgattctgatgcttcggtcagaagatgctgctattcattatgaagcggtattactagtgtagctttaattatagattcttaatttgcaatactgttgaaatttgggctttacacgcttctcttactgggcacatttgatgagttttgttttattgcaggttggtgtgatcggaaatctggtccactcctcccccaatataaagaaagaagttattcttgctggagccttacaacccgttattggattacttaggtatattctcaaattgaacccatgagaaatacaatgcatcctataggcctttacctaccttctgcaaccttaccctcaacttctattgatattatgacaagattattgttattataattttaatatcttcaaagctccctttttatggcaataatgttccaagaccaaaatatattagtgggaagcatatcttattaatctattctaatggtgttcgatgtaacagctcttgttgctctgaaagccagagggaagcagcgttgttacttggacagtttgcagccactgattcagactgtaaggtaaaaataaacttcagtcgaattccgtgttacttttttatggataagtatgtgttaattactgtttgatactgttaggatgtaaaatttaggacaattggagtagttaggagtttgttagtagatgtaagtaagttgatgattttgtttaagctttaacagccttgttattttggttattcttagaaagtctttaaatacccctcaattggtagatgggaaaaacaagttttggaatagctgatttttgggactggttattccagtatgagaggagagtgggaccggttattccagtactaaagtagagtgcttctctgtaaaccttttatattttcttgttcaatctctaagaaatacgaaatccttcattgatttgcaatttttaatcatttgaatatgttttcacaccattattctaggaatagccctcaattggtagaggggaaagacaagttttggaataactgatttttgggaccggttattccagtacgaaaggagagtgggactgtttatttcagtactaaaggagagtgctcctctgtatatccttttatattttctcattctatctctgaaaaataagaaatccttcattgattgatttgcaatctttaatcatttgaatatgttttcacaccattatcctaggaattctttcttgctctgttaactttatttttgtaggttcacattgtacagagaggtgctgttcgacctctgatagagatgcttcagtctcctgatgttcaactcagagaaatgtctgcttttgcattggggagattggcacaggtaatttgttttcctttgtcttttccatgttattgtacttgtgtgtgcaacttgagagggtaactttattatattcatggaaactattacctcttttttgttgttgtttttgaagcctaaacttttaagcattaaataaatggagcttagatttgagcatacaaactactgccttgtgaatattatgttgcaccttgttaaatttaggttttatgcactgtttccatttgtaagctgaattagagtcctcttaacaccatacccattttctctgggctgaatatattaaatttatatgtcaggacacacataaccaagctggtattgcacatactggtggcttagtgccattgctgaagcttcttgactcaaaaaatgggtctttgcagcataatgctgcttttgctctttatggccttgcagagaacgaggtaggataagctacaagaactctaataataaagactttctgtcataattgttcagagaagttattactaaaaacggaagttaatgctttttttttttactttgtgctgtaggataatgtgcccgactttattagggtaggcggaattaagaaactccaggatggagagttcattattcaagtaagttatttctttaatacctataggaattcaatgatactgttaactgcgtgcaaattttatctttatgaactggaaccattaggctttctgatgcacactgatcattatgaaaatgctattggtttctatgtaggcaactaaggattgtgtttctaagacattgaaaagactagaagagaagattcatggtcgtgtaagcccagtgtcacattggctttttactttactgagtttgctctttatactgtaattaatatggaaatgacaaggatgctattactgtttcagttagaagtttaataagttccacacaacaataaaccacgaagccctattattattttttttggtcaagtagtttagtggctggaatttcaccctttaaagatgaatagtgtcgtaggtttgaacctgcacccctgcacctgatgtccttgcacagctaccaactgagctggcttaacgggacatcacgaagccctattctatgagcaccaagtttcatattttgatcaaatttctaattattaattttttctttgtaggtgctgaaccatttattatatcttatacgggtttcagaaaaggcattccaaagacgagttgctttggctcttgcccatctttgttctgcagacgaccagagaaaaatatttattgaccacaacggtatgcatattctttgtcaacctttttgcattaatgttatttatcttacttcttgcctacataaataagtatgtttgtattgtatctaccgagatatgagcggtatttaattcaacaattaatataattctaagtgaaagatagtgagagttttgttcataaacgtaaatagtggtaaaagtagtgaaaataacaacgagataaaattgctgggattagatttcctcaaccactttctaatgcatcctaatggttagctacatacattcatgttaacattatcatcacaggttgctattcgaacaataataatttcttaataacaacgagaaatctatctgtcgtcttgtttaaatgccgattctttagatggttaactaagacaataacatcaacaactgaccatttgtaattattaaacttaaatccgtccctagagttttgattctatagatgtttatcattttaagagtattttccaataacaattcaaatcacaacatcatagtatgattgatccagtcataacaagcattaagaatgaagataaacattgtttaactgccgattctttagatggttaactgacaaaagaacttttaaaaatattttccaataacaattcaaatcacaacatcatagtatgattgagccagtcataacaagcattaagagcaaagataaacattgatattaatgagtttctagaatatatataacttgagatgaaaagagattcaaaagaatatgattgattatatctaatcccaacaaagagagaattagctatcatagacatgctggctttacacagttgagaagaaatgggatgaaaatgcttcaatggttgattcccctaactcctcatcttccttactcgaattcgtatggttctgtcttctctcagtgtgtatcttcaaatgacagtgttttgagatttcacttagtgaaattgtggtttgcttagcgagcctattcgtcctgaagtaatggctggccagctgtacaaaagtgcctttaaaccttaaatttgccaagtgaaatcgatgtccgcttagtgacatttgttctgctaaacttcacgaactctatagtttgtatttgctaagccactctactgctcgctcagcgaatcactacgccccgttttcttcaaattttggttccaatggtcttgattgcttttcctctttgagtgctaactctattttacctatcaacacaaaaatatgcaaatatcgccattcacatatctcaaaccctaattagtaaatatataccaaaattgggatttttcaaacagcttttgcactgagcctttaatgtttaaatttaaaccggaaagccttcattctcttatgtattactgaaataaggcaaaagcaatagaaacagcagtaaaatggaaacaaagccaagtaaaaatactgaatttaacaaaaataaactctaaatatagatataaactaggcttattaacaatgagattcatttggccaaaaataaattacaaactaggtaaatttgacacttaccaatactttgttgtgtattctattctgtatgaagccgcacatctgttcatgcaggactggagttgcttattgggcttcttggctcatcatgccctaagcagcaacttgatggtgccgtggctttatgcaagttggccaacaaagctatggctctgtctcctattgatgctgctcctccatccccaacacctcaggtaggcttattatatacagtttgcttcaccttcttgattcataatctcacacctaatagtttgatatttttctctcactataaccataatcataggatccaatgctttacctgtattcttgctcaaaattttatcactcttcaattttctaaatgatataggaatactttgtttcttctgcctttttggtcttagaaagtgttagttgcgcgagctcttcacttttttgaagttaattgaatatctagcagtgttgtcaaatagtggtcatggtagattgtggctgcggctattttgacaactaactaagatggctagtttgtgatgggtgttttatggcggattttggctttccaccatggtccaccatccacagtagttaaaactgatatctagatcgagaattcaaggcgtatagttatgaatacatgctatgtttaattaattggcggcttatgtctagctttgtcctttctccttattttccttcctgttttaaataattctggaaaaattgtttttcaatgttggaatcatcctagactatccttcttgcaggtctatttgggagagcagtatgtaaacaatgctaccttatcagatgttacatttttagttgaaggttgatactttctattcaaattggttcttcctggaaatgtttcttaagaaataacttacatgaaatgtcatgtcatagtttcaattgacatttgtagataaccaggtatacttaactgcaggtaaacggttttatgcccacagaatctgtttactcgcttcttcagacgcatttcgtgcaatgtttgatggtggttatagggtgggtatatctcctctctcccctcccccgacccttgttactattgattatctaccaaaaaagataactcctttactgatacctcttttcacaagaaacgtgtttatcacctactattttggtttaatgctttctctaccatgtgaaaactttagttggatatttttcatatttggcttttgtattgaatggtgaatttgaatatggcaataaaagtttatattgcaagtttaatttaaacatattccatgtccttgatgtacagttcatttactgtatgacaggagaaggatgcaagggacattgagataccaaatattagatgggaggtctttgagctgatgatgaggtctaatcatatgctttatgaaagttatgttgtaaaagcttttaaggcaacttaaatctcattgtttaatttttgttcagatttatatatactggatcagttgatctcactgttgaaattgctcaagatctcctccgagcagctgatcagtatcttttagaagggcttaagagactatgtgaatacacaattgcacaggttagctaagtgaattgggtttgttagtgcattgtttcctgaactaatattagaatagtaagtgaattcctcattaaatgtttttttgtctaatgatgtatcactacataataatataatagaaagtgcgtttctcattacttgagtttttattacaggatgtatcactggagagtgtgtcaaatatgtatgaactttcggaagccttcaatgctatatcattgagacacacatgcatcctttttatcttggagcacttcgataaattaagtgcaacaccagggtatctatcagatctcctcaatcgcacatttacttgctctttttcagaactctctttaccctgttgttgtctaaaaggaatttttataaactgatatataggcaacctaaatggattatatagctaggaatcctttttttgggggggaaacaatatatcttagaatcttggataagctatagttttagttttttttttattgtagtataggcaaacatgttgacctaaaaggaatccgtatattgaaaatttctggtacatactcggtaactaacaaggaataggtcttcataatcatgaattatttcaccttgagtaaaggtttcttagtgatatatggaatggggactagcaaatggttttctcaacatttgaagaaaagtaataaacttggttcttatcctcttctattcatcttgcttgcttttattttgaccaatatgattatagactgcagtcttatacatcactatagttagattgacggtagacaccaaccttcactttgaaataagatggataatcaagttttagttggtcagtttcatttttaaagaggagttttagttgatctgttaaagcagttgtttggagcatggttgcttccatatacttgaaatgataactgaagttcacattaatgttgcattagttcttaattatcttttaatttgtgcgctttttaaatatctaaattctgtttgcagacacactgatttgattcagcgtacaataccagagatccgcaattactttgttaaagctcttacaaaggggaactccaacatccaggcatagtatggttgacatctaacagattgcaatgtgtacataatatggtagatgttatcgattattatttaaagtgtgagggaggtctcctggattcagaactgcgtggttttgaagaaatgtctaacaccaggctgtgtctgttcttttttgatgctgtgtctctcccttctgtttgtaacaccgtggtcgttaatgtagtagcatacatgaccttcacgaacattgattttttccctcgtgcaatattgtgatggttatgaattgatagttctctatcccaatcgattatgcaatacagttgttgagtttatgattatgttaaagagtaatatatcagtcaaatacataattcttcagc

SEQ ID NO: 205 - DNA, 5447 bp, Pisum sativum
  source 1..5447: mol_type = genomic DNA
aaatattcagcgccaaacgttaccgctattccaattgcttcaattttattttttgcgccaaatggatgaaaatctttttgcctcaaaatctcgataagaggaagagtcttttcactttcaaaatcgaatttcaatctcttacgcatttcaaattgaacttcaacaccattttgattctcagaaaaaccataacctttaatctaatggaccgcaaggaaactttgaagaggaaattcgatttcaccgatgatgacgaatcaaccgatgaagttcttcacgaaaactctcgccgtctaactctcgccgacgatattactaaccgcatagatctgttaaactcggttttttcatcgtccgatccggatatcggttctgctcaaaatgctcttgtttttctttcggaatacgccaaagatggtatgtttgtttgcaatcccatttctttatcttgttttaaattttttgttattattattgatttttgaacgttttttctttgatttgttgtgatcaattttgctttagcagatgatatggtggattctatggtagtttgtggtgttgttcctgctctagtgaaggttttgcgtatggtgtctaatggaggtgatttcgatgctgatacttgcgatgttgaaaaagagtgtgtatacatcctcggtcttatcgctcccaaggtaatttcactgtactctgaaataattttgattatggtttacgatgtagaaatcaatttaaacaattttttttatttttagtttttaggtatgtctaagaatttgttacattatgaagtgtaataactcttgctatacttatgctgattttcatgttcaaatagccggagtatcaacaactcattgttgatgctggagccttgccttgtcttgtggaattgttgatgagacctaaagcccttggtgtttctcaatcacttttttctcttcttcttgggagagtagctgatgcaataaccaatcttgctcatgaaaatatcaatatcaagacccttgtcaggtttttttcatcttccaaattccaatactttaggatgttgtttaataatttggataccactgttgttctgtgatacactatttactgcaaaatgttgtctattagctgctatacatcatttaactatgaaacacagacacctcgaatgcgacccgacacttacatagagacaccattaataatttgaaaagatgaataaaataagtgtaattactagtgtttggtgcaagtgtttgatactaacacaaacatagtcatgcctttttctagaggtgtctgtgttacattgctatttaaaccccaatggtgggcctgttggcgggggtttgggtcttgagattgtagtcctcccaacgtcttgagtttgaatcttattaggtgctaacaatttttgtgttgggccaaattcatattgagttttgttttggatttaaatacattgtggaatgttagcaatctgttatctgcaattgacaacactgccttagttatattatagtccatgctctctaattgatgctatgttcaggttggaaggtggcattcctcctcttgttgatttgcttgagtccactgatacaaaggtacagagagctgctgcaggggccctgagaactcttgcatttcaaaatgctgagaataaagaccaggtagttaatttggcacaacaactttaatatggtggattctcttgttatagttgcttacaagagtcaaattgcagattgttgaatgtgatgcgttgcccactcttgtactaatgcttggatcagaggatcctgcaatgcattatgaggcagtaagagacaaatgatttcatatattcttttacattaaactctgcttcttacagttttctaagctacaagaacaagctgaatgaaattaattttgtaggttggtgtgattggaaatcttgtccactcttcaccagaaattaagagagaggttcttctagaaggggctttacaaccagttatttgcctactaaggtgacacatcttgtcttttattttctttaagctatccataggattaggagaatgtgatgtatttgtcaaacattgtagttgtctgtgctagtaagctattgcttccattttgacaaatctatgttttcattgatagttccccctgtttggagagccaaagagaagcagctcttttaattggtcaatttgccacaacggattcagattgcaaggttgattaagttgtgttttgcaaacttacaatgcaatagcccggtcacatgtaaaattctcttactgatccccatccttcgttcatgcagattcacattgcccaaagaggtgctataaaacctttaatcaaaatgctcaagtcttcagatttacaactcagggaaatgtcaacttttgcacttgggaggttggcacaggtgattatcactagcaactgatacttagcagtatgtgggaattgggttcctgagatcaactctaactgtttatataatccatgttaggactcacacaatcaagctggcattgcttacaacggaggtatagagcctctcctcaatcttcttgccacaaagaacccttctgtccaacacaatgcagcttttgctctctatgctcttgctgataatgaggtgaagttaatttccttgttctttactttgtcggcattgtacatggccctttattaatcattgatgcttgtggtgtgctgcctctgacataacagctttgtttgacaggacaatgttcctcttattattaaagcggatggtttacaaaaactgcaggatggacatttcagtgttcttgtacgttcatttactctttgccaatgataattttgtcctgtttatcaggatcaccattaaaatctcttactagtttattaaaaatttagttttgttatggtttttgtttgacttgcagcctactcaagagtgtgtagcaaaaatgttaaaaagattggaggagaagatgcaaggccgagtaagttttctcccaagttatcagttactatgaccaatgatttatttgtttagtcataagataatcacaatcaattcaaacattccttttactgttgtttacatcattgattttgattgttgtattaattactcttttgcaggtactgaagcaaatgttatatcttatgcgctctggggaaaaggttgttcaaaaacgtgtagctcttgctcttgcacatttatgttccgctgatgatcgtaaaactattttcattgacaataatggtaacaaactttaatatatacttttgtcccctttctctggcactacttagaaagtattttcaatcaatatgctgctaaatcttcaggattagaattgctgttggatctccttgaatctacaataaaaaagcagaagcgtgaagcctctgcagcgcttcacacaatggctaccaaaggaattggtgcctctattgttgatcttgcgcctacatcaccaacttcccaggtattttgcatttatgcttcattgggctcatcacgtttattttgttttttttccttctgcacttgctgaagcatatttctgtattatcacagttgcataattcaactgcagtttgaacttattgcctttgaaattgagttattttgttcatattctactgtgtatattatggtgatgatcctgagaatggaaaatgaaaattttgtttgtgttgtatgtaggtttacttgggtgagcaatatgtaaacaatccactactttctgatgtcacattcatagttgaaggtaaacaagctgttgctgatttttgttgttgttttctattaatttttcacatgtatgcatattgattatatgtactaatttactccattctcctttctccaggcaaactctttcatgctcatagagtctgtttagtttcatctgatatatttcgcataatgtttgatgggggttacagggtaagtattacctaatcatccaaattagtttcaagtcttcttttaattcattacctgtaagtagcaactattattcttttgcaaatattaattacctagctccacaagcattttgaaaattttgaaagccatataatcactttgcaattgaattaggattaatggatatgtggagttgaagtgtaaatatccttcataatgtcttacaatgtgcaatgcaggaaaaggaagccaaggatatagagattccaaatattaaatggaatgtctttgagttgatgatgaggtatgttggttcttccccttttcttatatattgatgtttttataatagactctgtttatgaactaattttctgttggaactctagatttatatacactggaacagtcgatgttgatttggatgttgccccggacctccttaaagctgcagatcaatatcttctcgatggtcttaagcgtatttgtgaatctgttatttctgaggtaggccaagaattgagtttcacagttgcttttatttcatttatttttgttgaatttttaatggtttattttaatattgttaaattattcttgcaggatatttctgtggaaaatgtttcactaatgtatatgatgtcagacacttataatgctacatcgttaaaatattcatgcatactatttatcttggagcaatttgataaattgagctccaaaccatggtatgtttacattctttacagcttgaaatgtagttttctttaagtacattgcattgatcatattttttgttctcaatcttaatatgcaggtattgtcactttatccgatgcattaagccggacattcggaacttcttctcgactttacttaccatgcctaaacatgctgactagtgcggatcctcagattttaatcttttcgtgaagaagtatgaaaatgtacaaagctgtggttaataatatatttgcatgccattctttcgtaacaaccttagagcatgtctgcttctgcagggttaacaaactcttcaaagtgtagcttctgtccaattgcacagaagcaccttgattttgtatttttcttaacacatttcatagtgaaagaatcatattttttatttagcaagataatttggccttattttaagctggtgaatactggttttggtctgaaattgttgatgttaaagtgcactttatttgcagcattttcattactttgacatttgtgttgcttttgggttccttatttatatcaagttgctactaggttacttgtatgttaagaaataagtttctacatttactggcatgaatcgagtgtagcaacttatggcaaattagttctattcaactttttataaagccaaaatggctaaataaaaccttagataaataaattatatgaatgtgttaattgaatttggacttaatttagagtctccttaaaaaagagtatagactgagtgatgaaaatggtttatatagttctcgttctatattttaaacgt

SEQ ID NO: 206 - protein, 704 aa, Pisum sativum
MEFQRRQGHCLYERKGQKRKLDEESQDEPQISAAPPTSDERAAVLTEVENQVNILESTFTWNESDRAAAKRATHALADLAKNEEVVNVIVEGGAIPALVKHLQAPPVEDCDKKALPFEHEVEKGSAFALGLLAVKPEHQQLIVDSGALTYLVGLLKRHNQGLTSRAINSLIRRAADAITNLAHENSNIKTCVRMEGGIPPLIHLLEFADTKVQRAAAGALRTLAFKNDENKNQIVECNALPTLILMLRSEDAAIHYEAVGVIGNLVHSSPTIKKEVLFAGALQPVIGLLSSCCSESQREAALLLGQFAATDSDCKVHIVQRGAVRPLIEMLSSSDVQLREMSAFALGRLAQDTHNQAGIAHSGGLVPLLKLLDSKNGSLQHNAAFALYGLAENEDNVSDFIRVGGVQRLQEGEFIVQATKDCVSKTLKRLEEKIHGRVLSHLLYLMRVSERGFQRRIALVLAHLCSADDQRRIFIEHHGLELLIGLLCSSSTKQQLDGAVALCKLADKASTLSPVDAPPPSPTPQVYLGEKFVNNATLSDVTFLVEGKRFYAHRICLLASSDAFRAMFDGGYREKDARDIEIPNIRWEVFELMMRFIYTGSVDVTPDIAQDLLRAADQYLLEGLKRLCEYTIAQDILLENVSSMYELSEAFNAISLRHACILFILKHFDKLSTRPGHSLLIQQTIPEIRNYFVNALTNANSQRQ

SEQ ID NO: 207 - protein, 703 aa, Pisum sativum
MELQKRPDHNLPEKKGQKRKLEEESQQDSQISLPPTGDARDALISDVNQHVSILLSTFSWNDSDRASAKRATHALADLAKNEEVVNVIVEGGAVPALIKHLQPPPLPEHGAPKPFEHEVEKGSAFALGLLAVKPEHQQLIVDNGALKHLVDLLKRHNNGLTSRAINSLIRRAADAITNLAHENSSIKTRVRTEGGIPPLVHLLEFADTKVQRAAAGALRTLAFKNDENKNQIVECNSLPTLILMLRSEDAAIHYEAVGVIGNLVHSSPNIKKEVILAGALQPVIGLLSSCCSESQREAALLLGQFAATDSDCKVHIVQRGAVRPLIEMLQSPDVQLREMSAFALGRLAQDTHNQAGIAHTGGLVPLLKLLDSKNGSLQHNAAFALYGLAENEDNVPDFIRVGGIKKLQDGEFIIQATKDCVSKTLKRLEEKIHGRVLNHLLYLIRVSEKAFQRRVALALAHLCSADDQRKIFIDHNGLELLIGLLGSSCPKQQLDGAVALCKLANKAMALSPIDAAPPSPTPQVYLGEQYVNNATLSDVTFLVEGKRFYAHRICLLASSDAFRAMFDGGYREKDARDIEIPNIRWEVFELMMRFIYTGSVDLTVEIAQDLLRAADQYLLEGLKRLCEYTIAQDVSLESVSNMYELSEAFNAISLRHTCILFILEHFDKLSATPGHTDLIQRTIPEIRNYFVKALTKGNSNIQA

SEQ ID NO: 208 - protein, 735 aa, Pisum sativum
MKIFLPQNLDKRKSLFTFKIEFQSLTHFKLNFNTILILRKTITFNLMDRKETLKRKFDFTDDDESTDEVLHENSRRLTLADDITNRIDLLNSVFSSSDPDIGSAQNALVFLSEYAKDDDMVDSMVVCGVVPALVKVLRMVSNGGDFDADTCDVEKECVYILGLIAPKPEYQQLIVDAGALPCLVELLMRPKALGVSQSLFSLLLGRVADAITNLAHENINIKTLVRLEGGIPPLVDLLESTDTKVQRAAAGALRTLAFQNAENKDQIVECDALPTLVLMLGSEDPAMHYEAVGVIGNLVHSSPEIKREVLLEGALQPVICLLSSPCLESQREAALLIGQFATTDSDCKIHIAQRGAIKPLIKMLKSSDLQLREMSTFALGRLAQDSHNQAGIAYNGGIEPLLNLLATKNPSVQHNAAFALYALADNEDNVPLIIKADGLQKLQDGHFSVLPTQECVAKMLKRLEEKMQGRVLKQMLYLMRSGEKVVQKRVALALAHLCSADDRKTIFIDNNGLELLLDLLESTIKKQKREASAALHTMATKGIGASIVDLAPTSPTSQVYLGEQYVNNPLLSDVTFIVEGKLFHAHRVCLVSSDIFRIMFDGGYREKEAKDIEIPNIKWNVFELMMRFIYTGTVDVDLDVAPDLLKAADQYLLDGLKRICESVISEDISVENVSLMYMMSDTYNATSLKYSCILFILEQFDKLSSKPWYCHFIRCIKPDIRNFFSTLLTMPKHAD

SEQ ID NO: 209 - DNA, 7770 bp, Eucalyptus grandis
  source 1..7770: mol_type = genomic DNA
agaattcctccctcatccatggactgcaaccgcagcgacgatctgcaggacatccaggagaagaagggccagaagaggaagctggaggacgaggcggccgccgccgacagcgagatctccgcctccgccggcggcggcggcggcggcggcgacggcggccggcagtcgctgctcagcgaggtggccgcgcaggtcaaggtcctcgagtccgccttctcctgggtcgagaccgatcgagccgccgccaagcgcgccacgcacgtcctcgccgagctcgccaaaaacggtgcggctcccgggggaagggtgggggggaggggggagaaaattgagattccgcgatctccgcttagtaacttgtccggagttgatttctcgctgctgattcgcgtgtttgtggttggatgcagaggagctggggagcctgcttgtcgaaggcggtgtggttccggccctggtgaagcatctgcgggcgccgccgtcggcggagggcgaccggggtgtgaggccgtacgagcatgaagtggagaagggatgcgcttttgcgctgggtcatctggctgttaaggcgagttgattgtgattctgattgctctaaaagcttggtgtattggctatatagctagcgattggtgttgtgaagttgattatctttgaagatatgatcgaagtcctgattatcctcattccagtatgcatatctacgaggcacactgtagtctggtcattgataggttagattgtgtggtttgaatgctcaagagtcgtttgttatggcgagtagaatgaccgcgaaggtatttggaggaggagcttgaagatatcttaggatgtaaattactttctggttgcgcaaaaaagagtgaaaaggaattgtcttgtttagctttctcagcaggctttgcatttacaccttaatttagtttccaccgtcatattgtgaggttatatgtagcttggtgtttaacgtattggctctacttgatttaatgaaatgcagattctgcttgagtgaaaagaaattgttacggttttattcattgaattgtctcgtttagctttctcagcaggctttgcatgtacacctcaatttagttttcactgttatatcgttaggttatataagtaggtcggtgttcaacatattgactctgcttgattgaatgaaatgcagagtctacttgagtgtgtcaatgctaaacttccatttgtgtcgtgtcacctcttttaatgtggtatcgtctgttgataaggggataactttgtttggatgagtcattgaagctcatcgtgttgaaagatgacgccttgagtattaattgtggcggattacatgtgctttacaaaagaaaacggaataggaaaaaatcagcagtgattgcagccttttgcacgcttgccagacattttggcatttgacatgctgatgagatatctaagctgatgtcattgagtgtcattgtgaattttagaagaatgttgtcaagccatcatactgtgggcttctgttatacttgtcattatctattgacggcacttttcaatattatctgttctactacttttttcttttaagcctaggtggtactggtactacagaaaattctaaccttttcccttgttatctcctcttggaacagcctgagcttcaacaacttatagtcgactgtggtgccttaccacatctaatagatctgctgaagaggcataaagatggttcaaccacacgagctgtcaacagtttaattaggagagcggccgatgctatcactaaccttgctcatgagaatagcagcatcaagattcgtgtcaggtgtgcttctgtaaataatagaatcaaatgatgccttagctccattttccttaatagtattgagattgatgtgcaggatggaaggtgggattcaaccgctagtagaattgctagattttatggataccaaagtgcaaagagctgctgctggagcattgcgtaccctggctttcaaaaacgatgaaaacaagaatcaggtgatgatttttcttaagaagatgttttcttgttttttatatcaagagtaggaattatgttaactcattgccttttcagattgtggagtgtaatgctcttccaacgctcattttgatgctccgttcagaggatgctgcaatacattatgaggctgtaaggccatggggatagtataattgatcagaatgaaagttgatgttttgtgtgattcctcaaattactttgttaattgcattctgtttgtggctttcaggtcggtgtcattggcaatctggtacactcatctccgaacataaaaaaagaagttctttctgccggggctttgcagcctgttattggattgctaaggtatgttgggaatctaggagttatgtggagcttgtgccgcttacagtctgcaaacggtctgatgatcttctttctctttcatgattgtttgtactgctcaagtttcaattgaacactttcttcttcaaacatgttgctttacagttcttgctgtcctgagagccaaagggaggcagctttgctcctagggcagtttgctgctgctgattcagactgtaaggtgaatgatggcagtttttttgtttgtatcctgttctgcaagatttgtataatttctgtctctctctctctcatgtgatttaaaattgatggaacaaagcaaccttaatctttgcttttttgggtcagtcaatgtccttaagtggttttagtttttttcctatccttctagtagataagtggtgcattcttgttgtcttctctgtcaagtgaggctggtcaacttctcaaccttacctctcgcctttttatcttggaaagtgtactgttgactttcttgacccattttctcatttccactgcaatggggatgcaaaaatgcaggttcacattgtccagaggggagctgttcgtcctttaatcgacatgcttcagtccgacgactttcagctgagggaaatgtcagcatttgcattagggagattggcccaggtctctctctctctctctctggtctctctctttctctggtctctctctctctctctctctctctctctctctccccacctttccctccccgcgcctacttgattaccaaaaagctggcttgatggatggttttcacagataggtagcttattcccgttttcccctaaaccttggcacttgtctatggtgtggcccttcagaaaggtccactgaaaataaacgacaaaagagcgtcttttgcttttctaaagatacggaaatcaagcacccactcaccaacactcaaacatagcttaataagtactctataggcatttattgaaattaacttatttaaaaagtttgcttcacacaatgaatttttgccagatgcaataatatggtgaaccatatgttcttttcggtacgtaatgtgtatttaatgaactattgtttccagtgaacttcagtttagaagtttagattggagacattctgaacatttctttttatcatttcaggacgctcacaatcaagctggtatagcttataatggtggcttgattccattgttgaagcttcttgattcaaaaaatgggtccttgcagcataatgctgcctttgcgctttatggacttgcagacaatgaggtaaaacctgtgaattttaatcaagccaaaatttaacaatgcttcccacccaaactccaaaatatggcaatgttgaagttttcttgatcactaggatgtcgttcaagctagttgtcgtaactgctatccatcttctctgtaggacaatgtctccgattttattagagtaggaggtgttcaaaagctgcaagacggagaatttattgtccaggtgggcaggagaagtgttaaatcacatagtatttagaattatatttcacgcaatgcataatatgagtgaagtggacatcatctttgcaggctacaaaagattgtgttgccaaaactttgaaaagattagaggagaagattcacggccgagtgagtatcttaattttgtagtctcatactttgaactgaactctgtattgttgtcaatgattttatgtctctttttgttgggtacataaatgaaaggacttctttcttttcctttcttgacctgttgggctttaatatgttggtttctttgtgcaggttttgaatcatttactatatttgatgcgcatagcagagaagactgttcaaagacgtgttgctttggctcttgctcatctctgttctccggatgaccagcaaacaatttttgttgataacaatggtgtgtgatgctctctctctctctctctctctctctctctctctctctcaatatttctatcattaagactgctttattctctttgtacttttaagctgtcagtgtctgattagtctgtattctctgaagggttggagctgcttgttggcctgcttatttgttcgagcgctaggcagcaacttgatggtgctgtggcattgttcaagttagctaacaaagcaatgtctctttctcctgttgatgcagctcctccctctccaacgccacaggtcactggccatctaatgggtgcttgattttcttttatcatttgaactgtcaattctggtcagatattgtggtccagaagaatataaggttatgcgtgtgcaaaagatctttgtcagcagtgttttttgattattagcttgccgatttctcataagttgccctttgtttcattacatggtccaggagaatttgcctgttctactggtttttctctttcaaagttttcaaatatatattatttgcccaggaaggagtctcttgtgcatatgagtattttagatctgttctgggaaataaaatttgatccattgttaaaagaactttcttattgcaggtttacctaggggaacagtatgtgaacaaccctacgctgtccgatgtaacatttctagttgaaggttcctgaaaattgtcgtgttctgtttcgttagtgactatctcatacatggatcattcatatacaagttatgatgaccgatttgaaagaatgcttgccttgtatatgttttgcaggaagacggttctatgcgcacagaatttgcttgcttgcttcttctgatgcatttcgtgcaatgtttgatggtggatatcgggtgagtgtcctttaattcttggtttcaggttttcgtttacattaccatatttgtgtcaacatgaaattggactctgctgagctttgtgatgttatgtttaaaagccgagtgcagcaccttatgctctgtgatctcttgattaggaagtgaaatctttgctctgacttggtttatgaaataaagtttgcgtgacatttattacaggagaaagatgctagggacatagaaattccaaatatcagatgggaggtttttgagttgatgatgaggttagttataacttttaagtctaaatccacataatatggtttgtgtgatattcttcaaatgactttcttcaatgacactacagatttatatacactggatcaattgatgttacgctggaaattgctcaagatctcctcagagcttctgatcagtatctcttggagggactcaagcgactttgtgaatattccattgcacaggttagctgatgaatgattgaatgagtttacctattgatgtttggtatataccttgacaatgagtgtaccttaattattgcaggatatttcgttggaaaatgtctccagcatgtatgaactttcagaagccttcaatgctatttccttgaggcactcatgcatcttgttcattctggagcattttgacaaattgagacctgggtaaacacttccagctaagctcctcttgtttggcaaaaatctgtttgaattctatttatcaatcccctcttctaagtatacttcactaatatatggaggaaatggtgggagttgtcattgggattatgtcaactctagaaatcttctcttccaagggcagtataaatttgtctttttgtgggtggaaagtggaggcaaagattggagattgatctcattctgccctgcttgttactagaatgacagtgagggacagattattacatcttgggaattatttccttcggcccataagttgcatgctcccctggttttgggagaatgtggaggaatttgattaaacaaccagttgtcttctgaaagttgaagtgcatctctatcattttctctcatggagaacaattttcatcccctccatttccttaatccaaatatctggaaataataaaattttcttgtctatgacttccatattcctgcctctcatttcccctctatatttttttgcccattcaagcaaaaggtaaacacacctagatttatatgaactttcagcctttttaataagtaataaaagccataaacattattcatcagacaaaaaaagtgatacttgtgacgtctttaagtcaatatcttcagttttggctccctttatttatctaggaaaaataccaaaaatgcacttcaccaaaattccttttttgtacttctgtttttgtaaatatcgctttactacctttagacaaaactcattcatggaaaagatcaaattgccccccttacagatccccaagcctccaaactctcccacagctctagcttatatcacccacaagccacaaacctcaggtcccctccaccatagaccatcgtccaccttccaccgtcaactcttccccactgccatcatcatcccttccccttgccaattgatctagatctggtagcaatgggtgcaagctcgaactttgagctccagcggccatgggccataagcccatagcttgaggcggtgagcttgagagatggagagaagggtgttgcgtgggtgaggggagggtgtaagtgtttttggaaagagaaatgacaaatgtagataggtgggcaatgacaacttctgtttaagtgaggatgcaaacgtgttttttaaaatataaagttatgcaagtggtaactaggtaataagcaaaatatttatcggtatttttcttaagctactggggcctctgttttgttttgttgaacttctcctgatctctttgtaactgttctgctctgaacttttgcaggaatttccctctcattcaccgtataataccagaaatccaacagtactttgtgaaagcacttactaagtctaaccagcgtagcaccttgaggccttaagaccctgtggtttcgctctccctactctaaccgattgttgtacaggaagtggtagatttatgagcagttggtagcaggtggatggctctgactgtttggtaattggaactcacattcttttccagacgcaagatgtggactccctgtaagtctccacccatttttgttgtaagatgtaactgggatggtgatcttcccattattgtcgaaatccaagcatgtagccatggattgtagcgtttcgagttagctttgccgacgtgcgttccatgaattgaaatgggatgtttcagtagacgtaagaaaaaaaggggaattggttggactctgttgactgtttcctcaaaaacgagtatgaagatgatgaatatcgtgtcatcttcagaggctcttgttgagggaacagatattggttccaatattcattgacatatttgcctgtggttcaatgtctcgggacttctggattgttgggcgtggttgtgaaagagtgtcattttctactgggaaacgctgtaattcatggaatgaaaggatggcttttgcttgtgtggcatgttcttcgacg

SEQ ID NO: 210 - protein, 712 aa, Eucalyptus grandis
MDCNRSDDLQDIQEKKGQKRKLEDEAAAADSEISASAGGGGGGGDGGRQSLLSEVAAQVKVLESAFSWVETDRAAAKRATHVLAELAKNEELGSLLVEGGVVPALVKHLRAPPSAEGDRGVRPYEHEVEKGCAFALGHLAVKPELQQLIVDCGALPHLIDLLKRHKDGSTTRAVNSLIRRAADAITNLAHENSSIKIRVRMEGGIQPLVELLDFMDTKVQRAAAGALRTLAFKNDENKNQIVECNALPTLILMLRSEDAAIHYEAVGVIGNLVHSSPNIKKEVLSAGALQPVIGLLSSCCPESQREAALLLGQFAAADSDCKVHIVQRGAVRPLIDMLQSDDFQLREMSAFALGRLAQDAHNQAGIAYNGGLIPLLKLLDSKNGSLQHNAAFALYGLADNEDNVSDFIRVGGVQKLQDGEFIVQATKDCVAKTLKRLEEKIHGRVLNHLLYLMRIAEKTVQRRVALALAHLCSPDDQQTIFVDNNGLELLVGLLICSSARQQLDGAVALFKLANKAMSLSPVDAAPPSPTPQVYLGEQYVNNPTLSDVTFLVEGRRFYAHRICLLASSDAFRAMFDGGYREKDARDIEIPNIRWEVFELMMRFIYTGSIDVTLEIAQDLLRASDQYLLEGLKRLCEYSIAQDISLENVSSMYELSEAFNAISLRHSCILFILEHFDKLRPGNFPLIHRIIPEIQQYFVKALTKSNQRSTLRP

SEQ ID NO: 211 - DNA, 4944 bp, Theobroma cacao
  source 1..4944: mol_type = genomic DNA
aaaacaaatcttcctccctatatttcactttcccaagattacactcttcgtttctctccattcttcctctggatttctccaaatggatcacctgaagaagccccaaacacgaagaagcttgaagcggaagttggagcaagatcttgaagaaggcaaagcagatcgctgcaaggtaccggtcgtcgaatctcgccttactcaccaagatctccttcacgaggttcgcctttacgtcggtcttctcaactccactctctccttttcaaaagccgatcgcgccgccgccaaacgcgccactcacttcctctccgaactcgccaagaacggtatgttttaattctccatttctgttgttttagtagcagttcgtttagaatgttacaaagatttcgttgtttatttcattatattttctttggcgattgcagaggatattgtgaatttgattgtggagtgcgacgcggtccctgcactggtaaagcatcttcaaacgccaccaccgttgagagaaggcgacgcgatgccattagagcatgaagtggagaaaggaagtgcatttgcgcttggactactcgccgtcaaggttgattttgaagacttttagttacttgatttcggttcaattacaatgttgttcttttccccacttacattggtagttactctgtttgctatttcatgttaagtagccagagcatcaacaactcatagttgacgctggggccctgccctatctcctgaatctgctaaaaaggcatagggatggttgtaattctcgagcagtcaatggagttataaggaaagctgctgatgctataacaaatcttgctcatgaaaatgccgacattaaaaccctcatcaggttcgcttgtttggatatctcttctcaattttcgtactattaatcatcacatattgaatggttctttttctatatgtttaggattgagggtggaatcccaccgcttgttgagttgcttgagcatcacgatgtaaaggtgcagagggcagctgctggggccttaaggaccctagcatttaagaatgatgagaataaaaatcaggtaaagttatcttttccaatatgtcgtattattttggtgctctattgtggatttgaatatattttgcaaatttgcagattgttgaatgcaatgctctacccaccctcatactaatgctgtgctctgaggatgtttccattcattatgaagcggttggttctcatctaagtgtttatatctgcaaacacatgttttggagctctattcctgttataaactcacataaaggatgttcaggttggcgtgattgggaaccttgtccactcctctccaggtataaagaaacaagttcttcttgctggagcactgcagcctgttattggattactaaggtaatcctgagttttacattgtgttttcttttttgcttaggagaatcgtgtcttttattagtctcatagtatttctagttttaatcatattgcaagtacacgctcattctaaaatgttactttgccaacagttctagctgtctggagagccaaagggaagcggctttactaataggtcaatttgctgctgctgattctgattgcaaggtcggttaagatcttggttctagtttgatacttgaattgtgctcataggtgaaggatatggattattatttgttgttgattgtctgttttaggtacattttaacacagggcttatgtgttttcttgctaaaagttaagaagatggagatcttgcaggtacatattgtccaaagaggagctattcctcctttaattgaaatgcttcagtcttcagatgtgcaactccaggaaatgtctgcatttgcacttggacgtttggcccaggtttgtatttctttgctgttattttgtattggtttgaacagtttatctagataagaactttaagcattatgtctgtcggtggacttaaattatcccatcagtaatttattatcttatgctatatgaatatatgatttaatttcttccccaaatgcttaataatagttatttgaagtatgcttaataataattattattttttcaggacacacacaatcaagctggaattgtgcaaaatggtggattagtgcccttgcttaggcttcttgattcaaaaaatggacctctgcaacataattctgcatttgctctatatggtcttgccgataatgaggtagccattggtctgttatgatatattgaacttgaactgcagtttttacttgcactgggagtctattgaagtttacatgtggtttattctgtaggataatgttgtagatcttatcaggactggaggtgctcagaaactccaggaaggggagtttattgtccaggtctgcttctttaatttcttgtgcttttgtatatgctgatgttcatggtcattgaattgtttcattccttttacatacccatagaatttatagttaggagaattataaatgtttctagcccatacattttttattatttgttttactcattaaggcactgtgtaatacttgcagccgactaaagattgtgtggcaaagacattgaagaggttggaggagaagattcacggacgagtgagtttatttattgctaactctcgaccttttcatagttgtgtgcttgcagtttgggtaggcctgttgtttgttaaaagttagaaagtggcatttatccaattgtgaaaacatttacaagtcatagtttgggagattaatgcatcattctcttgacaggtactgaatcacctattatacctgatgcgtttagcagacaaggctgttcaaagacgagttgctctggctcttgctcatctttgtgtccctgatgatcggcaatatatttttgttgacaataatggtaaaaaaaattttctgttcccattcttgtcaccactttctcttcttgcaaaatgattggctttagcagtttttctgtttttgaatttctaatatctaattgcttctctgaatgcacatcaatgttttccaggactggagctgttactgggccttcttgagtctacaagtttcaaacaacagcaagatggttcagcagccttgtataagttggccactaagggcaatccactctcatctgcagatgcagctccaccatcaccaactccacaggtaatttatgtctgctagctggtctattgtgagaacatttttacattcagttttgttttaaactcttctatgagcataggatgatatggatgcagattattggttgctttttcttgagagtggcatgaacaattcactagcaggataggattctttttgttattataaccacttttttgtagttaatttgtcatgatctgtatctctgttattattcatattcacctaaaatgtcctaaatttcaaattcttttgtctaattattattgtttataaggtcatggtttatatacgaggttggtaactaatttttttgccacctttttctttttaacattagatcctacatagcagtaattttttattactttaagcaatgtaatccttgggtggcattattttgcctaaaaactgattaaaatttgatgctctaggggtaattctttattagcttgggatatgaatggtgttaaaaatgtccttcctgatagattaagcgttcttctcttgtctttaattttttggaatgcaggtgtacttgggtgagcagtatgtaaataatcctacattatctgatattactttcttggttgaaggtacggacatttcttatgaaatgattttgctctttgcttgttattattcttaattcagtgtttaaatctttatatttcctcttttatgttaagttaaaaaattgttgcttaagttgtattcacctgcaatttgcatattcttctttcaggtaaacgattctatgctcacagaatttgtcttcttgcttcttcggatacattccgtgcaatgtttgatggtggttaccgggtgagttatacaattcaagtatattttttccatgatctgtttttaacttatgctactttgttgtcaccatccatagaaatagaaggcataacataactaacaagatggaaaaagaaatcataagtttgaggattacatcactagatagtacaataaataatttttaatattgtagatgtggagtaactcaaggtatagtattaagaacatgaaaattggcgttgcaggagagggatgccaaagatgtggagattccaaatatcagatggcatgtttttgagttgatgatgaggtagaattttgaattttcccttataagtataaaatgaattccttcaaacaacctgacttgtattgttctggtcttgtgcttctaggtatatatacacaggatcagtgaatgtggagattgatattgctcaagatcttcttagagctgctgatcagtatcttcttgatggccttaagcatctttgcgagtatgctatatcccaggtgtgttttagtgtgataattctagtacttggattataacagatacatgctgtttgttattctgatgactgaagagaaatggctttctattatccttcttaaggatatttctgtggagaacgttacgctgatgtatgaattagcagaggcctttaatgccatgacactgcgggaagcatgcatacttttcatattagagcaatttgaaagattgagtaccaagccgtggtatgttataccttcccttcccttttataataagaggacaaattgtgttttgttgtcgaaaaacttgtcaggctataagctgtttccactttcatggttcgaatcatgcaggtattctcgtttgattcaacgcatggttccagatatacggaattactttattaaagcacttgcgaagcctgttcaaattgacgcaacacaactataaatgattcggccttacttttggactaacattagagt

SEQ ID NO: 212 - DNA, 7446 bp, Theobroma cacao
  source 1..7446: mol_type = genomic DNA
gttccttcttgatggagcttcagaggagccaggaccagggcctcccagaacgaaaggggcaaaaacggaaactggaggaagaaaaccaagaggaccgcgaaacctctctccctaccggcgacgcccgccgtgctctcttggccgaagtcaccgctcaggttagcgtcctcgactccaccttctcttggcgcgaacctgatcgcgccgctgccaagcgagccactcacgtgctggccgagcttgcaaagaacggtaaatattcaaagtctccaatcccgatctcattcttttttacacttactgccattcaatttattgtgtttttactgtttttgaatttcaggtttaacggtaataataatatttttgtttttttgttttggcagaggaagtggtgaatgtgattgttgaaggtggtgcggttccggctctagttaagcatctgcaagcgcctccgtgtagtgacggcgaccgaagcccgaagcctttcgagcacgaggttgaaaaaggaagtgcttttgcgctgggacttctcgccgtaaaggtaattttactgaatttctagtttttttatagaaatttggttgttactatcgtgcttttattttatcgagtactatagttttgtttagtatctgttgtagtttaacttttgaattatttgttggaagttcacttgtttcgtgatatgcatgcattttttcttagttgaatcctttttagtagcattagtaaatatttgatgttttgtgcaaattttttctttattaaaagaatgttacacttacataagatgattatgcaatttcaattttaccatatatagaaaaagttgaactttgagaaagtttgaggagtgttaacctgttatataggctgtgattaaaagaaacagattctggtgcatagagatggtatcattagagcagaaaatgccatatagatttaggtggttaattttattgatcctgccactaaagcttggctatgtcttgagtctggtaattttctttggtttttcatggtttgtggtcgcactattactgtatgtaaaatgtttaataactgaatgtgctaaggtttattttggctttgctgggaacagccagaacatcagcaacttatagttgattctggggccttatcacatcttgtgaatttgttgaggcggcacaaggatggttctacttctcgtgctgtgattagtgtcattagaagagcggctgatgctatcaccaaccttgctcatgagaatagcagcattaaaacccgtgtcaggtgctaaaattgtgcagtttttcattcaagttagatttttagctctgtggctttttaatcactatcaggattaatttgacagaatggaaggtgggattccacctcttgttgagttgcttgattttactgatacaaaggtgcagagagcagctgctggggcattgcgaaccctagcattcaaaaatgatgaaaacaagaatcaggtaacagacttgcctttggaagttgattggataaaattgccttctgtgctagtcaatagagtgaatgctttgactttgcagattgttgaatgcaacgctcttccttctcttattctcatgctacgatcagaggatgctgctatacactatgaagcggtaggatgttattgcagcacaagttaattattttgccactgtccactaggtttaagttctttttattttttatgccagctgtagaatcaaactcttttgccctatggattgtaggttggtgtgattggcaatttggtgcattcatcaccgaacataaaaaaagaagttcttgctgctggggctttgcaacctgtcattggcttgcttacgtatgcttcaatttgttttgatatttcttttacttggtttagcagtgttcttaattgtgttacacttgggctgttattttgaactgcagtctgcagtctatccagagttctccacttttattaatttatttgtttcattggaaaacagctcctgctgctcagagagccaaagggaggcagctttattacttggacaatttgctgcaacggattccgattgcaaggtaattactttcttctctctttatagttcactaggcttaagagacttcttcctggctctatttgtctatttaggggacgcaggaagaaaaaacaatgattggctctgaaattattgtcctaatattttgaatgaattagctttttgtatcatttcctttgtccttgtaatggaataagaggagctctggtctctatgctttaccacttatcatttcactttatcttaattttcattgtttattgttttgacatatactgctgacatattgcaggttcatatcgtacaaaggggtgctgtcagaccgttgatcgatatgcttcactctccagatgtacagctgaaagagatgtcagcctttgctttggggaggttggcacaggttattatttttatttttcttagttgtacaatttcaagcttttgttaatgctgtgaacaatgcataatggcttgtcttcaagcttgtggatggttttacttttgctgagatatttatgacagaataatgagtttacttgtctttacattaaatttttgcatcattttgagtatcatttgaagttgaattatacttaatgaatttcagccagtttgtgaactaaattacacaaaacttgttccatcaatccgattgtttgttgttcacttggttttgcaattgttatatctcatgtgattaacgtggccttatattggaatctacccttctgtatcccttgttttccactcttttatgtttctcgtctctcaacttttcagcatgtctgttggcatatcaaattttctgcctgatgtcttaagagtctttgctccacagcactgaatggatacaagtttctctggagctcaatctttttgttttcgttacacattacaagggctttgctattcacattttcaacatgtgtagttataaaatctccagtaattgttgtcttatgttactgcgaaacttgaggctctcaactcatctctcaacattttggcatgtctgttggcatatcatattttctgcctgatattttaagagtctttgctccacagcattgaatggatacgagtttctcttgagctcaatctttttgtttctgttacacattgcaagggctttgctactcacattttcaacatgtgtagttataaaatctccagtgattgttttcttatgttgctgtgaaacttgatactgtcaactaagtttcctgtcttcatgtgctggaactagtagatagttctatgtcactgaaaggtaattctgatttcaggacacacacaaccaagctggtattgcacataatggtggtttggtgcctttgttgaaacttctagattcaaagaatggatctttgcaacacaatgctgcatttgctctttatggtcttgcagataatgaggtatggtagcatgtgatcattgtgaacctgggaaagtgcttgaatttattttttgttgtcctgtaacacggtgttaatatattcttctctccaataggataacgtatctgattttattatggtgggtggggtccaacggctgcaagatggagagtttattgttcaagtatgttaatcctttcagattttacctcttgctctccccttagttttgatgctactagtttctttattgcggcatgatatgcataagaacctcaaaagtttaccagctcttgttgtattttctccttaactgatttactattggtaatggtactttcaggcaacaaaagactgtgttgccaagacactgaaaagactggaggagaagattcatgggcgggtaagcattttcgttcttatttactaccctttactgttatacatttatttatcatattttgctgtttggactgcagaaagacctatctcttcagtgctctttaaggattaggtctcattaaatttgtgtataatttctgagattttggttttaattaccttttgtaggttttgaaccatttgctgtatctgatgcgtgtagctgagaagccagtccaacgacgagtggctttggctcttgctcatctttgttccccagaggatcagagaactatattcattgataacaatggtccatattcttcaccccttcttcagttatcccaaatatcagtcatattcttaattccatgcaatttaaattagggtattgcatgagtggagcacacatgtttggtctgctttgagaggctgattgtgctgtattttcttgcaggacttgagctgcttcttgggcttcttggttctacaagtcctaagcagcaacttgatggtgctgttgctctgtacaagttggccaacaaagctatgagtctttctcctatggatgcagctcccccttctccaacaccacaggtgagtttgtaacaggctggttagtctaattccatgcctttccagtgcctgaaatcctaaatttgaattgatgtatcatgtttgtgtattgttatatcatgttccatgattatggtaaggctagatttatgaccatgtttgatttcatatcaaaatgtaaagttgacagtggtatagaactaggctgactggatggctgttgcacccaaccaaatatttgagaatgatggagatttcacaaagtatctgtataggagaatacctcattgcagtcaatatgggaccttaatggaagatttcctatcatgaagttgtaggatcctttggttattttgctatttagtcagaggaatagaaatttgtgaaaaactgaagagctataaattcctatcttatggaacatgttcggattattatgtttgtggagcacactttggtaatgcgaagtgcaagtcaacgaacaacaaatataagatgtcaaaatcacatgccaactgtttggataccaaatataggaaagctaatgcatagttcacatgatttggccaacttttgggcgtatattaaaatacatatcttttcattcttttttgaattgtaattacattcatatccctcggtagtatatcttcttgaagtatgtgtttaatttgaagaccttgaaataggagctgatttggtaattaggacaaatttctaaaccaaaagaaagaaaaaagaaagtttgtcaaaataaaagcaagtacttttccagttttggacagattgatggaaagaacaaggaaattgcagaattgtcaactttctttcttctttctgttatgcttttccaaatgtattcaggaaccgaatgaaaaacctccaatctggattatgagaacttatttatagatatcattatttttgctccagagtctgatatatgtacggatgtgtgttcatataatcatttcaaattgcatgagtagattatagcattctcgtaactggttatgaggtatgagaatagtttatacttttgaaagttctattttaagtgcctcttataacatacaactttaatgcaggtctatttgggggagcagtatgtgaacaatgctacattatctgatgttacgttcctagttgaaggttgttatctgatctgattacttaaagctctaatacttgatatggagaaacatttggtgagggtcaaaatatagattttgttgtaattaagaccctgtcttgcttttcttctgcaggtagacggttctatgctcacagaatctgcctgcttgcttcttccgatgcatttcgtgctatgtttgatggtggttatcgggtgagttcacttttgcggcatgttaatgtctcagttggtcattcctcctcttcccaagagtggccaagaaatcccttcaccctgggtgttgggatgggagttattgttcaagtatcattctaacaacggggagagtctacattttatgctttgtcttccagctgatatgagatatgatcctttatttctgatggtcttggaaatgcactaaactcatctctttttgcaagcttaggcttttcacttgtaactgttagccttattttattctttttgaaagtagctactactcttattcttagttttgctttaatcttaaacctatagcagtccctacaggatggaaacaatgttttgtatctacatgatattcattcttaaagtcttcatggcatgtgctgcaggaaaaagatgcaagggatattgaaattccaaacattagatgggaggtttttgagttgatgatgaggtattacaaattctttgtcaatcccttccccacagtcccttccttttcgagcatcaataatttacttgatttcattcttgtacagatttatatacaccggatcagtagatgttacattggatattgctcaagatctgcttagagcagctgaccaatatcttttggagggacttaagcgactctgcgagtataccattgcacaggtaagccaaaagggttgtctggagatctttgaatccttttgctgctttaaaattgaaacttgacatctgatacttttttctgttttcattcaaggatatatcgctggaaaatgtttcaagcatgtatgaactctcagaagccttccatgctatatcattgaggcacacttgcattttgtttatcttggagaatttcgataaattgagcacaagacctgggtatgtacttgaatcaacttccacaactaggcttttctttaggaatttaacagtatgtcaaacatcacgtagtgttatttgtcgtatattccaatgccctttttgggtagttgtgtacctgcttgtctgcggtattttcatgatgtagcatgctttcatcttcctgcttgtctgcggcattttcatgatgtagcttgctttcgtcttcactaatattagttgcaggattaaaatttatctcaactgctgaaaagtttgtgcacatggtgtgtaactgcaggcacttgcatctaatccagcgcataattccggagatccgcaattactttgccaaagcacttacaaaacctaacccacataaccttcggctatagaaggctggtttttaactcctgatctctaactagatacgttgtacagaaagtagcagatcttctttgatgttgtggagccgatggaaggttctaattggttctttgtagcgtggttcataatcattactgatgccagagttaccgttgcttgtagaaaaagctataaggtttcttctttaattcattgtcttttggcctccacttttgatcttcgtggactgtgttggttattagatttaaatgtattccaactacttacaaagttggcattcattgaaaatgcttgtacttttttttttttttttttttctgttggcctaagaaaatgcttgttcaaatgagcagttacagtttcttggtgaacgcttgatttcctgtgtaaaagttgaagaatgcttgaaaagaccaatgaatctagtagtgcttcc

SEQ ID NO: 213 - protein, 705 aa, Theobroma cacao
MDHLKKPQTRRSLKRKLEQDLEEGKADRCKVPVVESRLTHQDLLHEVRLYVGLLNSTLSFSKADRAAAKRATHFLSELAKNEDIVNLIVECDAVPALVKHLQTPPPLREGDAMPLEHEVEKGSAFALGLLAVKPEHQQLIVDAGALPYLLNLLKRHRDGCNSRAVNGVIRKAADAITNLAHENADIKTLIRIEGGIPPLVELLEHHDVKVQRAAAGALRTLAFKNDENKNQIVECNALPTLILMLCSEDVSIHYEAVGVIGNLVHSSPGIKKQVLLAGALQPVIGLLSSSCLESQREAALLIGQFAAADSDCKVHIVQRGAIPPLIEMLQSSDVQLQEMSAFALGRLAQDTHNQAGIVQNGGLVPLLRLLDSKNGPLQHNSAFALYGLADNEDNVVDLIRTGGAQKLQEGEFIVQPTKDCVAKTLKRLEEKIHGRVLNHLLYLMRLADKAVQRRVALALAHLCVPDDRQYIFVDNNGLELLLGLLESTSFKQQQDGSAALYKLATKGNPLSSADAAPPSPTPQVYLGEQYVNNPTLSDITFLVEGKRFYAHRICLLASSDTFRAMFDGGYRERDAKDVEIPNIRWHVFELMMRYIYTGSVNVEIDIAQDLLRAADQYLLDGLKHLCEYAISQDISVENVTLMYELAEAFNAMTLREACILFILEQFERLSTKPWYSRLIQRMVPDIRNYFIKALAKPVQIDATQL

SEQ ID NO: 214 - protein, 704 aa, Theobroma cacao
MELQRSQDQGLPERKGQKRKLEEENQEDRETSLPTGDARRALLAEVTAQVSVLDSTFSWREPDRAAAKRATHVLAELAKNEEVVNVIVEGGAVPALVKHLQAPPCSDGDRSPKPFEHEVEKGSAFALGLLAVKPEHQQLIVDSGALSHLVNLLRRHKDGSTSRAVISVIRRAADAITNLAHENSSIKTRVRMEGGIPPLVELLDFTDTKVQRAAAGALRTLAFKNDENKNQIVECNALPSLILMLRSEDAAIHYEAVGVIGNLVHSSPNIKKEVLAAGALQPVIGLLTSCCSESQREAALLLGQFAATDSDCKVHIVQRGAVRPLIDMLHSPDVQLKEMSAFALGRLAQDTHNQAGIAHNGGLVPLLKLLDSKNGSLQHNAAFALYGLADNEDNVSDFIMVGGVQRLQDGEFIVQATKDCVAKTLKRLEEKIHGRVLNHLLYLMRVAEKPVQRRVALALAHLCSPEDQRTIFIDNNGLELLLGLLGSTSPKQQLDGAVALYKLANKAMSLSPMDAAPPSPTPQVYLGEQYVNNATLSDVTFLVEGRRFYAHRICLLASSDAFRAMFDGGYREKDARDIEIPNIRWEVFELMMRFIYTGSVDVTLDIAQDLLRAADQYLLEGLKRLCEYTIAQDISLENVSSMYELSEAFHAISLRHTCILFILENFDKLSTRPGHLHLIQRIIPEIRNYFAKALTKPNPHNLRL

SEQ ID NO: 215 - DNA, 6814 bp, Gossypium raimondii
  source 1..6814: mol_type = genomic DNA
cttccttttctttaagaagacaaaaccataacggaaagaaaaggaaaggaagaaaaaggaaaaagctccgccctttttttactaaatctccaaaatacccctgatccacactgtttcttttcaaatcactggtctcatttccgataataaaccttttcctctctttggttttccttcttgatggagcttcagaggtgcgaggaacagggcctgcaagaacgaaaggggcaaaaacggaaacttgaggaagaaattcaagaggatagagatgctactccgctacctaccggcgacgcccgccgtgctctcttggccgaagtcaccgctcaggttaaggtcctcgactccgccttctcctggcacgaatccgatcgcgccgctgccaagcgtgccactcacgtgctcgctgagctcgcaaagaacggtaaatatttttgaaatctccagcttccgatctcagtcttatttacacctttttttaattttgttctgtttttcactttttttttgaattttcgttattagacatgactagtaaaaatgtaggatattcggtactatccgatctttttttatttttggaaattcgggtaatggaataatttttttaattcgaatagaagatttacgttttagattccgatttataaaatatgaaaaaaaaaatatagttgcggagaagttcgagccttgtcaagtagtctttattactaaaagtttaagctagtaatccaatattagatattgtaatgataacatttacttaaaagttaaattatcaagcgtaatgaaacataataatgttttaatagatacttaatcggaaattatttttattaattatcttttagtatcttagaagtagactgttgttaattatgagtgaatttgaacttcaaatttctttattgtttgattttatcttttaactgctttctatattcaaacagataatgctatctaaatcggatctggatagtaatactaatattttctaacataatgggattcgcatacagatgctctaatagtaaacatccgaacagccgccatcccttttcaggatgattggtaataaatgttttcttcttttaatattctcttttgcagaggaagttgttaatgtgatcgttgaaggtggtgcgattccagctctagttaagcatctgcaagcacctttgtctgatgaaggtgacctaagcttgaagccttttgagcacgaggttgagaaaggaagtgctttcgctttgggacttcttgccgtaaaggtgattttattgaatatttatatttttacaaaagtagtcattatttatatagtttagtatttattgtagttaaagacttaaagttttgaattgtatattggaaattctcttctttcatggtatgcatgatttttttttttaatttcttgttagtagcattagtaaatatatgaagttttctgtaaaatgttattttggttaaaaagtatgttacataagctgattttttaatatcaattctacagtaggtattagaaattaaacttccagaaagtttgaggtgtgaaaagaaaatgattctggtgcatagagacggcatctgttcatgctatcattatgcagaaaatactatctagaattgttgattttatttctaagccaccaaagcttggttatgtatttagtcttgtaattttctttggttttacatgatttatgttatgctagtgatgcaaatgcaaataaatgtagcattcactattgttaatcactgaatctgctatttattacctttgctggtaacagccagaacatcagcaacttatagttgattctggggccttgtcgcatcttgtgaatttgttgaggcgacacaaggatagttctacttctcgtgctgtgatcagtgtcattagaagagcggctgatgctatcaccaaccttgctcatgagaatagcagcattaaaacccgtgtcaggtttgctaaaattgtgctgtttttatttcaagttatttgtttaactttatgtttattccaataactatcttgatttgtttgacagaatggaaggtggaattccacctcttgttgagttgcttgaatttactgacacaaaggtgcaaagagcagctgctggggcattacgaaccctggcattcaaaaatgatgaaaacaagaatcaggtaaccgacctgcctttggaagttgaatttgataaaattgccttcaatgtttagttaatggagtgaatactgtggctttgcagatcgttgaatgcaatgctcttcctactctcatctcgatgctgagatcagatgatgctgccatacactatgaagcggtagaattttattgaaacacaagatacttttgcaaattccactgggttttagtaatttttaccagctgtagcgttaaaaaaaatctcgtcaccttgtaggttggtgtgattggcaatctggtgcattcatcaccgaacataaaaaaggaagttctcgctgctggggctttgcaacctgtcattggtttgcttacgtatgttactatgcttcagttttttacttttcttttacttgtcatagcatgagtttttagttgttacttttgggctcttctcttgtgttgcagtttatcaaggttctcccttattaattaatttgttttgttgggaaacagctcctgctgctcagaaagccaaagggaggctgctttgctacttgggcaatttgccgcaactgattctgattgcaaggtgaagagtggattttcttttatactttactaggattaagatacttcttccttgttgactctgaaattactttccaaacatttgaaagaattttgcttttcatataatttcttctgtccttgtagtgattaagaggagactgatccctatgtttacttaatttcccttgaccattactttttcattgttgcttctttttggcatgtgctctggattgcaggttcatattgtacaaaggggtgctgtcagacccttgattgaaatgcttcactctcctgatatacagctgaaagagatgtcagcctttgctttggggaggttggcacaggttattattgttattttcttggctgtatcatttcaggtttttatcaatgctgtaaatgatgtgtattgggttttatcttcataccttgctgatctttgtcctttttcccgagctagtaatttgtttactccaaatatttacttttttttttttaaaagactgaagttaattttacttaaaggatttttccctgttttgaaaaaactagcttacacaaaattggttccatcaactggactgcttgttgtactcttgattttgcggttgttaaaagttgtgcgatgatcatggctttgcaggaaaatagcccatcatctcaatccttgttttccaccaaattaactatcctgcatctcaaacttttcaggatatgcatttgcatcttcccaaaaggcacaatgtgatttgttttctcaatggtttttcttgtttaggaggtttcttttacactcagtgaggccttttctagatgtgtaggtttaaaatttccaataattgttgtcctatgcttccaagaaacttagtactcaactaaagttcttgtttctataaactggaactagcagatagctcaatcactaaaaaacaatttttggtgtcaggacacgcacaatcaagctggtattgcacatatgggtggtttggtgcctttgttgaagcttctagattcaaagaatggatctttgcaacacaatgctgcatttgctctttatggtcttgcagataatgaggtatggtagcttgttatagttgtgacctgggaaatttgttcttctttttcttttttggagtaacactgttttattatatttttctttgccataggataatgtatccgactttattagggtgggtggtgtccaacggctgcaagatggagaatttattgttcaagtatgtcaaccctttcagatattgcctcatactctccccttagttttcatgctgctaattacttaattgctgcattatatccataagagctcaaaactttcccttcccattctgtgtttttattcgttttaactgattaaatatcggaaatggtaatttttaggcgacaaaagactgtgtagccaagacattgaaaagactagaggagaagattcatgggcgagtaagcattttcattcctttaacatcctttacccttatttatttagtatattttctgtttgggctgttgaatgaccaagctcttcgttgctcttttatgttttaggtctcattaaatgtgtatctttactctctgatattttggttttaataatcttttgtaggttttgaaccatttgctgtatctgatgcgtgtagccgagaagcctgtccaaagacgagtggcttttgctctagctcatctttgttctcctgatgatcagagaactatattcattgataataatggtcatatccttttacccttcttccgttatcccaaaatcattcattcatattgcattaatggagcacacatgttgtgtttttgttgcttcgggaggttgattatgctctattttcatgcaggacttgagttgcttcttgggcttcttggttctacgaaccctaaacagcaacttgatggtgctgtagctctgtacaagttggccaacaaagctatgacgctttctcctatggatgcagctcccccttctccaacaccacaggcaagtttgaaaaagttggttaatatagtcccatgcatttcgaagtgtactcaggaaccaaatgaaaaaccaataatcgtgattataagagttctttttacagattttttcgatgtttctttatgtaatcatttcaaactgcagaaatggaatgacaactttctgttaattggttcagatgtaggggaatactttatacatttggaagttatatattaagcttctgttataacatatgatttaatgcaggtctatttgggggagcaatacgtcaacaatgctacattatctgatgttactttcctagttgaaggttgtttaacaatccgcttgcttaaagctttgatacttgctatggagaaacattcgatgatagaagaaatacagcttttgttttaattaagattttttcctcttttcttctgcaggtagacggttctatgcgcacagaatctgccttcttgcttcttcagatgcatttcgtgctatgtttgatggtggttatcgggtgagttcccttctgtggtgttttaatgttccagttggttgtccttcctcttccagatcggtgcctagggtttctttcccccttggtgttcgggtgaaaattatgttcttattttgttctttgttaaaagtattagtactctagttctaagtttagctttgaacttaaaatgtagctggcttattttgcaggaaaaagatgcaagggatattgaaattccaaacattagatgggaggttttcgagttgatgatgcggtattacaaattcttcgatctggatatataaacactggatttacttcattttgtttattttgatcatcattttatgtagttgacttcgtttctttgtacagatttatatacactggatcagtagatgtttcattggatattgcacaagatctgcttggagctgctgatcaatatcttttggaagggcttaagcgactctgtgagtacaccattgcacaggtgagctaaaactaaggttgtctatatatagatatttcgaatccttttgctgctttgaaatcgggaattgatgtttgattacttctatgcttgggttgaaggatgtaacactggacaatgtttctagcatgtacgaactctccgaagcttttcatgctatatcattgaggcacacttgcattttgtttatcttggagcatttctctcaattgagcgacagacccgggtatgtatttctgccacatctctgcatttagcagtacaaagaacatcatacagtatttaactacttgttttagtcatccgtgtgcgtgataattccttgataaatgctttcagtcggtgtagtaccatcagttagaattttggaatgataaaagtgaatttgggctatttgaagtaggttcgaccgtcatgttggtatcgattttgtgtttttgcatattaaaatctatgaccggcggctgaaagttttcactcatgttaaatattatcgcaggcactcacatctgatccagcgtataattccagagatccgcaattactttgcgaaagcgcttacgaatcctaacccacataaccagcggccgtagaaggcaaccagtggctgtagaaggctggtttttaactcatctcatctctaacaagatacgttgatgtacagaaatgtagtagctgttgttgatgtggagccaattgaaggttctctaattcgtttctttgtagcacggttcgtaatcgtttccgatgcccgagttgtttcgtggtgtttgtagaaaacaaggtgtaagtttctcattttaattcattgtcttgtctgcatttagatgtttacacgaacaaaaacctgtatcacgatttgttagctattggactttgctttattaacttctgtgtatatccttacgtagaatctgatcggaactagggcatatattgtttcataaactaacaagatctgtagctttaaaggtttaaacacagtatctttgaggatcgctttcaaaagataggtgtaatgatatggtctacaaaagttagagccaaaggttatgttatatggtttacaaaagtatgattggatgcatatatgaatct

SEQ ID NO: 216 - DNA, 7036 bp, Gossypium raimondii
  source 1..7036: mol_type = genomic DNA
tttaaatcggccattaatctttcattttcattttagagaaaaaaagtaaaagaggaaaagaaaaagaaaagaaaagggaagaaaaagaatgaaaaagcttcccgttttactaaatatccaaaatacccctgatctagtctctctgtgtgtgtcaaatcacgcttctcatttccgataacaccttctctctctctctctttctctcgcaagtcccttctttaatccttcttgatggagcttcagcgttcggaggaccagggcctccctgaacggaaggggcaaaaacggaaactggaggaagaaattcaagaggaccgtgaaatctctctccctaccggcgacgcccgacgtgccctcttggccgaagttaccgctcaggttaccgtactcgaatccgccttcacttggcgcgaatctgatcgctctgctgccaagcgtgccactcacgtgctcgctgagctttccaagaacggtaaattttttaaatcttcaagttccgaattccgatctcgttcttttttatatctcttggctttttatttgggttggatttttactgtttttgaatttcaggattaacgctaatgatcttatttttgtgtttcttttgttttttttttgtcggcagaggaggttgttaatgtgatcgttgaaggtggtgctgttccggctctagtgaagcatctgcaagcgccgccatgcgaggacggcgaccgaagcccgaagcctttcgagcacgaggttgaaaaaggaagtgcttttgcattggggctgcttgccgtaaaggtgattttgctgaatgtttctcttttatatataaaaaatacttgttactattattttatatacttctgtttagtagttactgtaatttatgttttgaattgtttattggaagtttacttgtttcgagatatgcatttttttttttaaatttcctttcagtagcattagaaaatatctgaggttctttataaaatttattctctattgaaagtgtgttagatgatagcacaagttaaactttgagaaagtttgagttgggctaatatataggctgttataggaagggggccgggggggggggggaaagaatgatctgtcatataatggtttctattcatattatcactgagaagaaaattctacagagaattaggttgttggtttcattgctgaacaactaattcttgtctatgtatagagtccggtatatttcttggcttgcatgatttatgttcctgctattaatggtaatatgttcactctgtttgatcaatgaatctgctaagttgttcattgcctttattgataacagccagaacatcagcaacttatagttgattctggggctttgtcgcatcttgtgaacttgttgcggcgtcacaaggatagttctatttctcgtgctgtgatcagtgtcattagaagagcagctgatgctctcaccaaccttgctcatgagaatagcagcattaaaacgcgtgtcaggtttgctaaattgtgcagttttaactaagttatttttcgtaggtccttgtttgttctaataattatctttgattggtttcacagaatggaaggtgggattccacctcttgttgagttgcttgaatttactgatactaaggtgcaaagagcagctgctggcgcattacgaaccctagcattcaaaaatgatgaaaacaagaatcaggtaacagatctgcctttggaagttggattggataaaatcatcttcaatgctggttaatggagtgaatactatggttttgcagattgttgaatgcaatgctctacctactctcatcttaatgctaagatcagaggatgctgctatacactatgaagcggtaggattcttattgtttatgttacttggactaaggagagaggtggtggacatgggtatatgtccgtcactagtatgctaacttttttttcaaaatttccatgtatttggagattccttgaaggattttatcctcacacccatgtctgcatatgtgtcaaacataggtactttaagaaaattcaagagtaggagcaacatattttagcataagatgacctttaggaaaattctattgggtttggcatcattataccagctgttgcatcaaaaagtttctcaaatggcttgtaggttggtgtgattggcaatctggtgcattcatcgccaaacataaaaaaagaagttcttgctgcgggggctctgcaacctgtcattggtttgcttaagtatgtttaatttggtttcttctttctttcacttgttttcttttaacctggttatttgatactttggggctgctcttttgatctgcaatttatcctggtttctcattttttattaactaaccttttattggaaaacagctcctgctgctcggagagccaaagggaggcagctttattgcttggacaatttgctgcaactgattctgattgcaaggtgaagactgtactttctcttcatacttagctagtattaagatgcctcttcctggctctatttgtcagttaggggatgcatgatgaataaacgattattggctctggatttactgtcctaatatttgaatgaatttagctttatatgtgagtgcctctgtccttgtgatgattaggacaagcactggtctttgtgccgtacatataatttcattcccttcaccttaatttttcatcatttctccttttttgacctatgctgctttggattttgcaggttcatattgtacaaaggggtgctgtccgacccttgattgaaatgcttcactctcctgatgtacagctgaaagagatgtcgacctttgctttggggaggttggcacaggttattattgttattttctctgctgtaaaattccaagctattattagtgctgtaaaagatgcttaatggtttttgtctgctaatcttgttgatgctttctgagataataatgtgatttcttatctctactcaaaatatttgcattttaaataaaattagtttatgagttcctgccagtttctaacacaaaatttgttgtataatctgtaaatctaactgcttgttctcttggttttgcaattgttgtacatagtgtaattatcatggctttgtgggaatgtagccaatgtgcatcccttgttttccactcttttaagtatcctgcctctcacaagtttcagcatgcatgtttgcatataaattttttctgaatgatatcttaagaaaccttgctcctctgcattgcacataaggggctcattttatttgtgtttctctttggttttccttgtttgtgaggtttctgtttactgttgcttctgagaaactttgctaaatttcctttcttcataagctggaactagtagatatctctgtcgctaaaatatagttttgattgcaggatacacacaatcaagctggtattgcgcatagtggtggtttggtccctttgttgaagcttctagattcgaagaatggatctttgcaacacaatgctgcatttgctctttatggtcttgcagataatgaggtatggtagtgtgtgatagttatcaaccttaaaaaactgcttggacttaatttttggggttgtggtacactgtgttaattaatattcttctctcccataggataatgtatccgattttattagggtggggggtgtccaacggctgcaagatggagagtttattgttcaagtatgtcaatccttttagatgttaccttttgcgctcttagtttccatgctattagtttcttagttgctgctgcataatatccataagaaaacaaagcttttctaactctttgctgtgtttttatttttccttaaccgatttaatattattggtgatggtacttttcaggcaacaaaagactgtgtagccaagacattgaaaagactagaagagaagattcatgggcgagtaagcattttcgttgctttaactacccttttcctttatttatttggactaaagaaatgtctttcttttcaacgccctttctgttttaggccttgttaaatttgtgtttataaactcagattttggtttatcttttgtaggttttgaaccatttgctgtatctgatgcgcgtagcggagaagccagtccaaagacgagtggctttggctctagcttatctttgttcccctgatgaccagagaaccatattcattgataataatggtcatattcttttccctttcctcagttactcatattctttattatgtgcaattataagtagcatactccattaatggagcacaaatgttttgttgctctgagaggctgattttgctgtgttttcttgcaggacttgaactgcttcttgggcttcttggttctactagcactaagcagcaacttgatggtgctgtagctctgtacaagttgtccaacaaagctatgacgctttctcctatggatgcagctcccccttctccaacaccacaggttagtttgtaaagttatttagtctatgtcatgcatttccattgcctgaatttatgtcattcgaagaaaatggtgttttgtatggccatatcctgttccataattattgcaaggctagatctatgatggattggatttaatatcataacctaaggttcatgggtggcattggactaaccttatgaactttctatgtgggtgtggcatccttaccaaatatgacgatgatgaagtggttttttgtggtgcatcttattggattatgcgttttaatttgaagacctagagttacgaactgaaatggaaattaggagaacatggagtttaagagcttacctatagaaattcttattcttgccttttccaaatgcctttgtataagtgtttcaaattgtaagggtagatcaacaacattcttgtaattggtatgaggagaatagttcctacttatgaaagttctatgcaatttcgtgttataacatgcaattctcatgcaggtctatttgggggagcaatatgtgaacaacgctacattgtctgatgttaccttcctagttgaaggttatacgatcttgcttacctattgttctgatgcttgctacggggaaatagtcggtgacatgtcaaaaatggccatttgttgtaactaagataatttattttatcttgcaggtagacggttctatgctcacagaatctgtctgcttgcttcttcagatgcatttcgtgctatgtttgatggcggttaccgggtgagttccctttttcatccttttaatgttcaagttgtttgtttctcctcttctcaagagggttgaaggctaccttcatctgtggccttggggtgagaacttctattctagtacctttaacaactaggagactccatgtagtattgctttatcttgcagctgatattgagatacagtcctttatttctgatgattctgggtgtcctccaaaatcatcttttttttttttgaacttgggctttttcacttgtaattggtggccttctatttttcttttttaaaaaatatgagattgctcgtactcttattatcacattagctttaaacttttagcacttaattcaggacagaaattatgttgtcaagctacatgatgttcttttttaaattcctcgtgttgcaggaaaaagatgcaagggatattgaaattcctaacatcaaatgggaggtttttgagttgatgatgaggtaggacaattctttctttggtccagatgtatatacattggatttacatcgattttatttactcgattttattctttgtacagatttatatatactggatcagtagatgttactttggatattgcacaagatctgctcagagcagctgatcaatatcttttggagggacttaagcgactttgcgaatataccattgcacaggtgagctgaaaaggttgtgtttagatatttcaaatccttttttggcctttaaattgcgaattggaatctgattatttatgtttacattgaaggatatatcgcttgaaaatgtttcaagcatgtatgagctgtctgaagcttttcatgcaatatccttgaggcacacttgcattttatttatcttggagcattttgataaattgagtgcaagacccgggtatgtacttaaatcaacttgccatgtccctgcccttcattagtaattgaattgtatgtcaaaagatcatatagtattgagcattgcatgtttattgttttgtctactccttatttcgtcagttgttggaaatttcagaaggcccttgtttgtggctttttttttttgcttcatgaatatttgctgtagaagtaaaacgcttatgcaactgctgaaaatttcaatgcgtgctgaataaattgcaggcacttgcatctaatccagcgaacagttcccgagattcgcaattactttgctaaagcacttacaaaacctaacccacataaactgcggctatagaaggctgggtctttttaactcctgatctctagctaggtttgttgtacagaaagtagtcagatccgatctctttgatgttgtggagccgattgaaggttctaattggttatttgtagcgtggttcataatcatttgcatgtagagcaaatagcattagtttcttctttgattcatttttcttagatgtttggagaatatcatgtattgtgttggttgttactactttcggagtcggccctcattgaaaatgcttttgttaggtttgagcagttgctcgtttctttttatgccagaaattcgaatgcatgcatgattttaatgtgtaaaagctgagatctgagaatgattgaacaaggtttcgttgaatgaggcctaccaggcttgtgcaatgtcaatgtaaaccgtcttagactatgaaccaaaactcatacgtcacaaacagttcatggtagagttcggaaatcggaaacctgcattttaattgtggtgggtttcaaatttggatactcaatcctgtttttactgtgttaaagctttattgatactttttatatttattttattttgagattatattattaggtcaattataaatttg

SEQ ID NO: 217 - protein, 705 aa, Gossypium raimondii
MELQRCEEQGLQERKGQKRKLEEEIQEDRDATPLPTGDARRALLAEVTAQVKVLDSAFSWHESDRAAAKRATHVLAELAKNEEVVNVIVEGGAIPALVKHLQAPLSDEGDLSLKPFEHEVEKGSAFALGLLAVKPEHQQLIVDSGALSHLVNLLRRHKDSSTSRAVISVIRRAADAITNLAHENSSIKTRVRMEGGIPPLVELLEFTDTKVQRAAAGALRTLAFKNDENKNQIVECNALPTLISMLRSDDAAIHYEAVGVIGNLVHSSPNIKKEVLAAGALQPVIGLLTSCCSESQREAALLLGQFAATDSDCKVHIVQRGAVRPLIEMLHSPDIQLKEMSAFALGRLAQDTHNQAGIAHMGGLVPLLKLLDSKNGSLQHNAAFALYGLADNEDNVSDFIRVGGVQRLQDGEFIVQATKDCVAKTLKRLEEKIHGRVLNHLLYLMRVAEKPVQRRVAFALAHLCSPDDQRTIFIDNNGLELLLGLLGSTNPKQQLDGAVALYKLANKAMTLSPMDAAPPSPTPQVYLGEQYVNNATLSDVTFLVEGRRFYAHRICLLASSDAFRAMFDGGYREKDARDIEIPNIRWEVFELMMRFIYTGSVDVSLDIAQDLLGAADQYLLEGLKRLCEYTIAQDVTLDNVSSMYELSEAFHAISLRHTCILFILEHFSQLSDRPGHSHLIQRIIPEIRNYFAKALTNPNPHNQRP

SEQ ID NO: 218 - protein, 704 aa, Gossypium raimondii
MELQRSEDQGLPERKGQKRKLEEEIQEDREISLPTGDARRALLAEVTAQVTVLESAFTWRESDRSAAKRATHVLAELSKNEEVVNVIVEGGAVPALVKHLQAPPCEDGDRSPKPFEHEVEKGSAFALGLLAVKPEHQQLIVDSGALSHLVNLLRRHKDSSISRAVISVIRRAADALTNLAHENSSIKTRVRMEGGIPPLVELLEFTDTKVQRAAAGALRTLAFKNDENKNQIVECNALPTLILMLRSEDAAIHYEAVGVIGNLVHSSPNIKKEVLAAGALQPVIGLLNSCCSESQREAALLLGQFAATDSDCKVHIVQRGAVRPLIEMLHSPDVQLKEMSTFALGRLAQDTHNQAGIAHSGGLVPLLKLLDSKNGSLQHNAAFALYGLADNEDNVSDFIRVGGVQRLQDGEFIVQATKDCVAKTLKRLEEKIHGRVLNHLLYLMRVAEKPVQRRVALALAYLCSPDDQRTIFIDNNGLELLLGLLGSTSTKQQLDGAVALYKLSNKAMTLSPMDAAPPSPTPQVYLGEQYVNNATLSDVTFLVEGRRFYAHRICLLASSDAFRAMFDGGYREKDARDIEIPNIKWEVFELMMRFIYTGSVDVTLDIAQDLLRAADQYLLEGLKRLCEYTIAQDISLENVSSMYELSEAFHAISLRHTCILFILEHFDKLSARPGHLHLIQRTVPEIRNYFAKALTKPNPHKLRL

SEQ ID NO: 219 - protein, 697 aa, Gossypium raimondii
MELQRSEDQGLPERKGQKRKLEEEIQEDREISLPTGDARRALLAEVTAQVTVLESAFTWRESDRSAAKRATHVLAELSKNEEVVNVIVEGGAVPALVKHLQAPPCEDGDRSPKPFEHEVEKGSAFALGLLAVKPEHQQLIVDSGALSHLVNLLRRHKDSSISRAVISVIRRAADALTNLAHENSSIKTRVRMEGGIPPLVELLEFTDTKVQRAAAGALRTLAFKNDENKNQIVECNALPTLILMLRSEDAAIHYEAVGVIGNLVHSSPNIKKEVLAAGALQPVIGLLNSCCSESQREAALLLGQFAATDSDCKVHIVQRGAVRPLIEMLHSPDVQLKEMSTFALGRLAQDTHNQAGIAHSGGLVPLLKLLDSKNGSLQHNAAFALYGLADNEDNVSDFIRVGGVQRLQDGEFIVQATKDCVAKTLKRLEEKIHGRVLNHLLYLMRVAEKPVQRRVALALAYLCSPDDQRTIFIDNNGLELLLGLLGSTSTKQQLDGAVALYKLSNKAMTLSPMDAAPPSPTPQVYLGEQYVNNATLSDVTFLVEGRRFYAHRICLLASSDAFRAMFDGGYREKDARDIEIPNIKWEVFELMMRFIYTGSVDVTLDIAQDLLRAADQYLLEGLKRLCEYTIAQDISLENVSSMYELSEAFHAISLRHTCILFILEHFDKLSARPGFEQLLVSFYARNSNACMILMCKS

SEQ ID NO: 220 - protein, 687 aa, Gossypium raimondii
MELQRSEDQGLPERKGQKRKLEEEIQEDREISLPTGDARRALLAEVTAQVTVLESAFTWRESDRSAAKRATHVLAELSKNEEVVNVIVEGGAVPALVKHLQAPPCEDGDRSPKPFEHEVEKGSAFALGLLAVKPEHQQLIVDSGALSHLVNLLRRHKDSSISRAVISVIRRAADALTNLAHENSSIKTRVRMEGGIPPLVELLEFTDTKVQRAAAGALRTLAFKNDENKNQIVECNALPTLILMLRSEDAAIHYEAVGVIGNLVHSSPNIKKEVLAAGALQPVIGLLNSCCSESQREAALLLGQFAATDSDCKVHIVQRGAVRPLIEMLHSPDVQLKEMSTFALGRLAQDTHNQAGIAHSGGLVPLLKLLDSKNGSLQHNAAFALYGLADNEDNVSDFIRVGGVQRLQDGEFIVQATKDCVAKTLKRLEEKIHGRVLNHLLYLMRVAEKPVQRRVALALAYLCSPDDQRTIFIDNNGLELLLGLLGSTSTKQQLDGAVALYKLSNKAMTLSPMDAAPPSPTPQVYLGEQYVNNATLSDVTFLVEGRRFYAHRICLLASSDAFRAMFDGGYREKDARDIEIPNIKWEVFELMMRFIYTGSVDVTLDIAQDLLRAADQYLLEGLKRLCEYTIAQDISLENVSSMYELSEAFHAISLRHTCILFILEHFDKLSARPGYVLKSTCHVPALH

SEQ ID NO: 221 - DNA, 5622 bp, Lactuca sativa
  source 1..5622: mol_type = genomic DNA
ttgtataactttgtttctttctctacgaaaccgacacaaacatcccccatttcatataaaacactatccccaaattgcccctccctccactctctcgcctctcatcatcattcacttttttttttcctctcgctcgccctctctcatctctctctcatggagaaccagaaacgccatgaacaacctacaaactccgtgagaagaagcttgaagaggaagctggaggacgaattcatcgtggatcggaagatcacttcatctgatgacgcggctcaacaagatctagtatctgaagttcgcgctcaggtcgaaatcctcgactctactttttcatcgaacgaatcagatcgtgctctagtcaaacgttcgattcatatcctctccgagctcgcgaaaaacggtatgaatctacgcttaatttgtttttatgtttcaatttcacgtttctccgtacacatccccttttacgagtcacgctataacgtttcggtggtgttcaatttgtggtggtagttgtcgttgatttttgtttatgcggtggtgaaattgattattcttagcatctgcacatagctattgttttgttttcttaatcgcacctcgttgattttgtagttaccggtttaattcttcatttgcgcgagtagttgtggatgattatgttaatgcggccgatactttgcctgaattttttctatacgaattcggttctatgtgttgttggttagagttttgatgtgattaatatacatgactgcagaggatattgtgaatttgatcgtggaatccggggccgttccagcgcttgtacgccatcttcaagcgccacagtcaaaagaagtcgttgcaggaccaaggccatatgagcatgaggtggagaagggaagtgcttttaccctaggacttctggctataaaggtaattatcaagagaagctagattcttcatcattgttgcatgtcctatatcgttgtgtttggcactttggctggactagtggattattttcttcgaacttgtaacatggaatattgaagatgtgttcaatcatgcttagttctgtattctttttacttaagcattttcatgtggttttatttaaaatctacagtgtcacaagaaatgctactaaaacgttaagttgcgttttcacatgcatattttttatggaacacaatacagttggggcatgggacgaacttgcagatacagcatatcttttatttactatttagaagaaatagtatccaacatatatcagttaggcttgctattgagagaaaccaacactgaaagaagatattttaaacctcatgcttgtagtggaagattaaattgcttttcatgattgtttagttcccctcctgaagagcatcatgcactatgattccatgactcacccaatcacaattgattaaagtggttaggggccgccagttatttatttatttatttacttataattacagttgttttcttttatcaaattgtaatgatgtattggggtcatcctctaggctaccaggctgataaaacagcagatagtaaatcatttatctatataagtttcctttttgactagattttaggatgttttttttatgagcatttactccattgcatctttacctttttctatctaacttcaattcaaagcgatgatctacatcagcttccaagaactatatccgaagtttgattgattgtaatgattacacaatacacatggtcactaaagggatactacttttggtgatttctggtgttaacagccagagcatcaacaactcattgtcgatgctggagctctgccttatcttgttgctctccttaagcgacacagggatggccagaactctagagcagtcaatggtgttataaggagagcagcagatgcaatcacaaaccttgctcacgagaatagcagcatcaagacccgtgttaggtcagttcttttgttcccttttctgttacagttttgggtatttcagtttgtttgacatcacattcttaatttcttatgttcagggttgaaggtggaatccctcctcttgttgaattgcttgaattcattgatgcaaaggtgcagagagctgctgcaggagccctacgtaccttagctttcaaaaacgatgaaaacaaaactcaggttgaatgattgatataaaatgtgttttggtgattgtttggacaaagttttttaacattggaaccttgccatgtctgcagattgtggactgtaatgctttgcctactcttattctaatgctgcggtctgaagatgctgcaatacactatgaagcagttagttctagtttttaaattcactttttttctttttttcttttcagctcataagattgcttgtatctaggaatgatttttgaatggtatatctcaggttggtgtgatcgggaatcttgtccattcatcccccaacattaagaaggaagttcttcttgctggagcattacaacctgtaattgaattgctcaggtaacgtgatacatacctttaaagggttgcgttcaaaactgcaagttctgtctatgcctaaaactatcctgttggaacttattatgtcgcctacacataagatcagtcttcaaatattaaacaaaattggcttatttttgatagcaaagtaacaatttgttgaaaactacaacaattttaattcttgtattaattttacagttccagctgttcagagagtcaaagagaagctgccctattgcttggacagtttgctgctgccgatacagactgcaaggtttgaccgaaatgttgattcatttattatcatttatcacttaatttccatttctatattattattcatatgtcttgtctactgccaaccctaacaacacacgctcatgaatcttttcataggttcacatagtgcaaagaggcgctgttggtccactaatcgagatgctacagtcaccagatgctcaactacgtgaaatgtcggcttttgccctaggaaggttggcacaggtaaccgagttatagatatatatttatttattcacttaaattcacgaatctttattttattaaaatactatatcatagatttgtaagttctcactagcatctatgtatatgcacgggtttccatgcatgcaggtgtagtaattaaagctccaattttagtaatagcagtcataattacacacacgtgtgctactaaataagtgataactttgcatagtaaaaagatgtttattttagggtagtttatataattaatgattgtgatctacctatcatcaggatactcacaaccaagctgggattgcacatggtggtggtatacctccattgctgaaacttcttgattctagaaatggttctctgcaacacaatgctgcatttgccctctatggtcttgctgataatgaggtaataccatgttaaatcttattatcagaactactataatcccctgaagttaagattcctattctatgatctttgccttctattgaaataaatcccttttattttaggataatgttgctgatcttataagggttggtggggtacaaaagttgcaggatggtgaattcattgtccaagtaagtttgttatcttttgcagttccttagaatttttgtatcattttgcttggaataataaagactcatttgaatgacataatctggtttgacagcctactcgggattgtgtagcaaagacattgaaaaggctagaggagaagattcatggacgggtaattaattatcttaactacttgatccttttttgcaaaagatattaatttgtattattgtttttgtcctcaggtattgagccatttgttatacctgatgcggattgctgagagatctgttcagagacgagttgctttggctcttgctcacctttgttcgcctgacgaccagaaaacaatattcgttgatggcaatggtaaaattttaatcgccttttttaacacttgatatttatttagtgatgatttatattttacctttttctggatggataaatttcgtaggacttggcatacttttggagcttttggaatcaaccaatttgaagcatcaacgagatagttgtgtagccttgtgcaagttggctgaaaaagctagctcactttcccctgttgatgcgggaccaccatctccaatatctcaggtttttgttttttatttttgttctttttatttttttgaagttttgtatacattttaaactataatcgagggtgaaattttttcatactttgtgttgtaggtatatttgggtgagcagtatgtgaacagtcctacactctctgatgtaaccttcctaatcgaaggtggaaaaactatcttctacttttgtccaaaaaaaaagatttagttctattttagcatttcttgagcctgacaatttatatatgtataatatcttcaggcaaacgcttctacgctcacagaatttgtctccttgcttcttctgatgcattccgagcgatgtttgatggcggatacagagtgagtggcattaaatatctgttcgtttttgtcaacttttcgatccatttggttatatagtttttcaatgatgatttttatatccattttaggagaaagatgcgaaagacatcgaaattccaaatattagatgggatgtcttcgaattaatgatgaggttcatctatctataatctatatcttgcctttgatttcagttattgtacaggatttttcatatatattatattatgttacagatatatatacacggggtccgtagatgtcaatttggaaattgcacaggatcttcttcgagctgcagatcaatatcttcttgaggggctgaaacgtctttgtgagtacaccattgcacaggtgagtgacagctttgctctaaattcattaattattatatcagcagcatatgatgatgataataataatataaatataaatattattttatcaggatatactggtggacaatgtatcagttatgtacgacctatctgaggccttcaatgctgtgtcactaaggaatgcatgcattctatttgtgctcgagaatttcgacaagttaaatgctaagccagggtacaacatattaattaatttcaatttctttcgtgctctttttagattttggaaagtttgactgagttgactgaaatggtaaaaataaaatgaattaggtatgggggtttgatccagcgtataatgccagagatgcgtaattactttgtgaggacacttggaagacccgtggaagctgacatgcgacagtaggcgattgagtttcaaattttttgatcaattgatttttaaccaaacctagatgaaaaaaaaacaaggaagaagagaggatgtacagaaagttaagtggtttaggtttcatttgtcgaaaagaaaaaaaaaaggtggcgacttctgttttgagattggaactttgacaaccaacatggtggcagttgttttagtagatgggaaggaatgcttgcttgcttgttgtgccaaatgttgttgacatgcattgcatgtactgctctactactcttatcaactgttgcttatcttactatatataatatatacatattcttcttctcttctaatcatgaatttcatctcttgc

SEQ ID NO: 222 - DNA, 4659 bp, Lactuca sativa
  source 1..4659: mol_type = genomic DNA
cacatattcaagggcgggcgttgaatttctaattcatttattttaacctccgaaattgctttctcccatttcattttcacttttacacactcctcttgtaaaacgtaacttctctttccccaatttacccctacattcaatctctcatggcggaggatcggagacgccatgaacaacctactaactccggtagaaggagcctgaagaggaagctggaggacgaattaatcgtagatcataagttttcttctacagacgacgtttctcaacaagatctattatatggaattcgtgctcaggttgaagtactcgattctactttctcatcgagtgaagcagatcgtgccctagtcaaacgctcacttcacgccctctccgagttcgcaaagaacggtttggatttttcttattgagttttgtttttcaactttacgcagcgtaatttgatttgatttcgtttgcttataatttagtagttattgtgcaagatttagatttgtagttttgtgttaacgtgcggacgaatttttaatatctttcatttcacctactcttagttttcgttttttagattttatttatacttcgtgtgatatatatttacacatataggtatgtttatccgttcttatcgccttttaatatcgtgttgctcaacggaaatttctttttggcgactaggtagctgctgatgctttgtgttattactgcaaataaattgaatactttgccgacgagttcttaatatattcattacatgttctcttaaatttcgtttttagattttattcttacttcgtgtgatcactgatccttctatatttaattttgtgtttcttgattgttttgactttttgttgagtatctggctaatgatttgtgttagcaaagctgctaagttgaataattaatggcacccctgcttttatttattattcgctaagatttttcattttgttttcagaggatattgtgaacttgatcgtcgaatctggtgctgttccagccctagtacggcatcttcaagcgccacagtcaccagaagaggttgttactggcacaataccgtatgaacatgaggtggaaaaaggaagtgcttttactcttggacttcttgccattaaggtaggtactcatttgaattgcataaccttgtcaattaaaataaaggagaatccgaaagattatatttaataaaattactgttattaatggtgatagattgtttcctcttgaatctgttcacaaacaatttctgaacactttcaaaaaacctccactttgttttaacagcctgagcatcaacaacgcatagtggatgctggagccttacctcatctggttggtcttcttaagagacgcttggatggccaaagttctcgagcactgaatggtgccataaggaaagcagctgatgcaatcaccaaccttgctcatgaaaatagcagcatcaagacccttgttaggtctgtttccctccatctttttcagctgctattcatttattttagtacctttagttcatcacattttttcatgtttagggttgaaggcggcattcctccacttgttgaattgttagaatccagtgatgcaaaagtgcaaagagctgcagcgggggccttgcgtacactagctttcaaaaatgatgaaaacaaaaaccaggttgatgcttctataatttagtgaagcttcttttcgggatcaagaactaaattttttctaatatatccatgaaacatttgcagatagtggaatgtaatgctctgcccacccttgttctaatgcttcattcagaagatgctgctatacactacgaagcagttagtttctgtaccatttcttaaataccaattagtgtgcatacatccattgcattagatatttcagtatgtttttgactatctattgacttttgaatggtctcttaggttggtgtgattggcaaccttgtgcactcatccccaaatataaagaaggaagttctccttgctggagcattgcagcctgtaattgaattgcttaggtaccataatacccctctattgactaatgcaacctctgctcactttcttttggtcttgtttaattttatcttttgtcagcagttcaacttgttcagagagccaaagagaagctgcattactacttggacagtttgctgctgctgatacagactgcaaggtttctcaattttttatcatttatcaaatgatgctattgtgttgtaactgtatatctaacaataaaaaaaaatttgttttttatgcttaaatttggttatcaccataacccacataaccaaaaactttactttttcaggtacatatagttcaaagaggtgctgttggtccactaattgatatgttgcagtctccagaagctcaactgaaggaaatgtcagcttttgcacttgggaggttggcacaggtacatcatgaatttagttattttcttttatatttattgctataacatttatgataaaaaatcagttttttttttaaatgatgcttttattgtcatctatcaggacactcacaatcaagctggtattgcacatagtggtggcattgttccattattgaaacttttagattccagaaatggtactctgcaacacaatgctgcatttgctttgtatggacttgcagataatgaggtaaaaccttgaacattgtataaagttagaccaatataatatctgtagccaatagttacccttcaacttatggtaaaatcttttttgtaggataatgttgctgatctgataagagttggtggtgttcaaaagctgctggatggtgaatttgttgttcaagtaattactttacttatgaattatcatatcagtcatcaccaatgtctttccacaccctttaaaataataagcctgacttctgggacagattacttggttgaattcatgagtttatatttattgtgcagccaactcgggaatgtgtagcaaagacattgaagaggttggaggagaagattcatggaagggtaattattggtagataatatgtaggattcttaattgaaattttcaatcacacatgacatggtattactatttgttgtgtcaggtgttgagtcatttgctgtacctaatgcgtagttctgagaggaatgttcaaagacgagtcaccttggctcttgcacatctctgttcgcctgatgaccagaaatcaatatttgtggatagcattggtaaaaacagtctgttctttgttaaaatttgagtgacatattggtaattacacattttctttatatatatatttgatgacacctttcaggattggatatacttttggagcttttccaatcaagcaattcaaaacatcaagaagatagttgcgttgctttgcgaaagctggctgaaaaagctacttcacttaatcctgtggatgcagcaggaccatcatctccaatatctcaagttggctttccttttttttttctttttttcttagagataattacatttttggtccctgaagctttcaattttgatcattggttgtggttcttactgttgttgcattgcaggtatatttgggtgagcagtatgtgaacaaccctacactttctgatgtaaccttcctgattgaaggtacacatatgatatgatatgtttttaaaaaaagtaaaaattaagtaatggatgtggctgagaatgtttgtttggtatgatatcagggaaacggttttatgctcacagaatctgcctgcttgcttcttctgatgcgtttcgggcaatgtttgatggtggttacagggttagtctcaaactagaaacatgtagtatcatatatgtgtgtgtgtttatgaatgtggtttggttgcattgtaggagagagatgcaaaagatattgagataccaaatataagttgggagacatttgagaaaatgatgaggtacatttacagtggatcagtggaggtggatctgagaatagcccaggatctccttagagctgccgaccaatatcttctagatgggctcaagcgtctttgtgaatacaccattgcacaggtaaccttttcatatctgttatggaattggaactatccatcagttatggattttgttggctaacatgaacatcttgtttctgtatctgctgttaattaggatattacgcttgacaaagtcgcatatatgtatgacttatcagaggccttcaatgctgtctccttaaaggatgcttgtattctgtttattttggaacactttgacaaattaaattcaaagccatggtaagatataataaaccaatttaacatttttttttaatttataataatacttgcgatggttagttaaaaacttaaaatggaagtttcaatttcaggtatggtagtttgatgaagcggatgttgccagacatgtgtgattactttatgaagatacttggcaaaccactgaaatgaaatctgagagagatgatttagccatttaggtttgtttttttcaagggaaaatgtacagaaagtaatcagtttgtgttgttttttttcatgcatcacattcacagctgtagttcttcaacagaatgtgtatttccgaacatgattaatgcccttattgctaatttcctatacaagagtcgacaggggactaattactctgatggaacagtcttttga

SEQ ID NO: 223 - protein, 757 aa, Lactuca sativa
MYNFVSFSTKPTQTSPISYKTLSPNCPSLHSLASHHHSLFFFLSLALSHLSLMENQKRHEQPTNSVRRSLKRKLEDEFIVDRKITSSDDAAQQDLVSEVRAQVEILDSTFSSNESDRALVKRSIHILSELAKNEDIVNLIVESGAVPALVRHLQAPQSKEVVAGPRPYEHEVEKGSAFTLGLLAIKPEHQQLIVDAGALPYLVALLKRHRDGQNSRAVNGVIRRAADAITNLAHENSSIKTRVRVEGGIPPLVELLEFIDAKVQRAAAGALRTLAFKNDENKTQIVDCNALPTLILMLRSEDAAIHYEAVGVIGNLVHSSPNIKKEVLLAGALQPVIELLSSSCSESQREAALLLGQFAAADTDCKVHIVQRGAVGPLIEMLQSPDAQLREMSAFALGRLAQDTHNQAGIAHGGGIPPLLKLLDSRNGSLQHNAAFALYGLADNEDNVADLIRVGGVQKLQDGEFIVQPTRDCVAKTLKRLEEKIHGRVLSHLLYLMRIAERSVQRRVALALAHLCSPDDQKTIFVDGNGLGILLELLESTNLKHQRDSCVALCKLAEKASSLSPVDAGPPSPISQVYLGEQYVNSPTLSDVTFLIEGKRFYAHRICLLASSDAFRAMFDGGYREKDAKDIEIPNIRWDVFELMMRYIYTGSVDVNLEIAQDLLRAADQYLLEGLKRLCEYTIAQDILVDNVSVMYDLSEAFNAVSLRNACILFVLENFDKLNAKPGYGGLIQRIMPEMRNYFVRTLGRPVEADMRQ

SEQ ID NO: 224 - protein, 726 aa, Lactuca sativa
MAEDRRRHEQPTNSGRRSLKRKLEDELIVDHKFSSTDDVSQQDLLYGIRAQVEVLDSTFSSSEADRALVKRSLHALSEFAKNEDIVNLIVESGAVPALVRHLQAPQSPEEVVTGTIPYEHEVEKGSAFTLGLLAIKPEHQQRIVDAGALPHLVGLLKRRLDGQSSRALNGAIRKAADAITNLAHENSSIKTLVRVEGGIPPLVELLESSDAKVQRAAAGALRTLAFKNDENKNQIVECNALPTLVLMLHSEDAAIHYEAVGVIGNLVHSSPNIKKEVLLAGALQPVIELLSSTCSESQREAALLLGQFAAADTDCKVHIVQRGAVGPLIDMLQSPEAQLKEMSAFALGRLAQDTHNQAGIAHSGGIVPLLKLLDSRNGTLQHNAAFALYGLADNEDNVADLIRVGGVQKLLDGEFVVQPTRECVAKTLKRLEEKIHGRVLSHLLYLMRSSERNVQRRVTLALAHLCSPDDQKSIFVDSIGLDILLELFQSSNSKHQEDSCVALRKLAEKATSLNPVDAAGPSSPISQVYLGEQYVNNPTLSDVTFLIEGKRFYAHRICLLASSDAFRAMFDGGYRERDAKDIEIPNISWETFEKMMRYIYSGSVEVDLRIAQDLLRAADQYLLDGLKRLCEYTIAQDITLDKVAYMYDLSEAFNAVSLKDACILFILEHFDKLNSKPWYGSLMKRMLPDICSSSTECVFPNMINALIANFLYKSRQGTNYSDGTVF

SEQ ID NO: 225 - DNA, 6208 bp, Carica papaya
  source 1..6208: mol_type = genomic DNA
atggagcaagaagaacagcaacagcagaggcgcgaggatcagagcatcccggagaggaaagggcaaaagaggaaactggaagaaggaataaccgacggcgaggagcaggagatctccctttcctctgcagatgcgcgccacgcgctcctgcgagaggttagcgcccaggttactatccttgattctaccttctcctggaaggaagctgatcgcgccgccgcgaaacgtgccactcacgtcctcgccgagcttgccaaaaacggtaaacataaattttagagaaaacaaagatgggaacagaaaactcaaccgccggatctcgccacttcgtttctagtttagattgttttcttttattatgccatcacgtggtagtgttcctgggtgttctgtttggatttgaggattttgaggccacaaattgtcgtttgcagaggatgtagtgaacgtgattgttgaaggaggtgcggttccgggtctcgtgaagcatttgcaggcgccactgataagtgagggagaccatagctcgaagccgttcgagcacgaagtcgagaaagggagtgcttttgctctaggccttcttgcagttaaggttgcttgattatgttattattttttcacaaatatatcgcataatctttggatttcttttgttttggtcataatttttgcttagaacttccaaaaagctattctatagtatcggaattatttaatttgtgctaattggaatttggctttctttgtgcaccatgagtaaagtggataataaatagatgttcgcttggccatggaatggcgggttattccattttcttcttgttgctgtctttagtttgtctaacgcttttctgcagatctttaataattaaactgatttttgtgtgggaaaataaaaatgcaacattgagaatggcactttattgttcaaagcagcatattaatttatgtactgttttccagtccgaatggtaagttattcaattaagggctaaacctttagaaatggcttcctttttggttactgaatgcgtagacaggcattgctgtatatggaagaagcctggcaattcaactttcatgggttaacaaatgctcaaacttccattgaccttagtttttaagtcaaggatagtagtagtgtttattttcggaagctatagtgtggtattttcttagtttcggttatttggtgatcttagctttcaggatttagtgggttttcttgatcttttctggattttattgttagtcctgccatactagaaaatttttatggagcagaagcgttagaggttatagcttttggttagacatactttgtgtgatctctaaaccttttgcctttttgtggccttcaatggtaacagccagagcaccagcaactcatagttgacaacggggccttgtttcatcttgtgaatttgttgaagaggcacgaggatggttgtggttctcgtgctgtgaatagtgtcattagacgggctgctgatgctatcactaatcttgctcatgagaacagcagtatcaagacccgtgttaggtcagctgatttgtgttctttaatttcaaaattcacctctagaaccattcttttctcatggccatcacttctggataaacaggatggaaggtggcattccgcctctggttgagttgcttgaatttactgataccaaagtgcaacgagcagctgcgggggcacttcgcacgttggcattcaaaaatgatgaaaataagaatcaggtagttgatatatttgaactttgagtttaacaagattggcttgaagattaataattgatatggctgctatcatctcacagattgttgaatgcaatgctcttcctactctcattctaatgctaagatcagaagatgctgccatacactatgaagcggtaatagaatttttccacatgacttttatattagcccctataggaactcacacttatatggaatttcaaaatgtacttccttgctggatgtgttatcaaatgacctaccatgggttgcaggttggtgttataggaaatttggtacattcatctccaaacataaagaaagaagttcttgctgctggagctcttcaaccagtcattggactgcttaggtacattagatctgataatgtcatccttagtaatatttctctgcatggtcataggatactattctttttctgcatttattattttcttttacatgttacatggttctttttgtttactttcctattccaacgactcaaagtttatttatagcagttcctgctgttctgaaagccaaagagaggcagccttgttactaggacaatttgcagcaactgattcagattgcaaggtgcccttttctctattctatatctcctccttttccattgtcttatggagttgagacttgagagttaattcctccccaaaactttccttagtaccttggaatagggaagaattggattctgaacttaggataggctatctatcctgctagcactgataagacgagcattatcctcattggaccattttccttaatgccagccttcgtgcttctgagtttttttttcactctcctttcctcatattttttccattaaaaagtgggatgtttgcaggttcatattgtacagagaggtgcagttagacctttaattgagatgcttcagtcagctgatgttcagttgagggaaatgtctgcatttgcattggggaggttggcacaggttattatttttattttcttgtttatatctattattgaaattcaggaataaatatattaagatggctatctgtcctttatcttgagtagcatatttgggatttgataatcagatacttcaatattgctcagataagtttctgtttcaggacacacacaaccaagctggtatcgcacataatggtggtttagtgccactgctgaagcttcttgattcaaaaaatggatctttgcaacataatgctgcatttgctctttatggccttgcagataatgaggtgcaatatatatcttatgaatccttgtggactcgagctgaagtccttaaatttttgtttccaattttcatcaatctgtagttaatatagtgttctatccgtaggataatgtatccgattttattagggttggaggtgttcagaagctgcaggatggagagtttattgttcaggtattttattccctttgtttatttccaaacattagctgctattttataggtttatttcaatactcaatgttgctgatttcttacgatcacaattcagtgccactttcacatggctaagatattgagatgcttgtcaacttaatatacaccaagtagaactgtatagaatttgcatatatacaccaagtagaactgatagggaatatgcatatataattgcaggcaacaaaagattgtgttgcaaagacattgaaaagattggaggaaaatattcgtggacgggttagtattttctaatctcttattctgttctttttctcattttttgaaatgtggaagcatgtagtcaatgtaaactggtttggtctatgattccatgacacctatatttttaaccttggatattgtcttctcatgattttctgtgtagggtttaagtcatctcttatacctaatgcgtgtagcagaaaagtctgtccaaagacgagttgccttggctcttgctcatctttgttcaccagatgatcagagaactatctttatagataacaatggcatgtcacgttcttagtgaatctcccacggctatctcagaggctgttgtaattttcaattcgatcagggtttgggtgttgctaagttaagctgagatattcatgctagcttgaagatgctaatgatacaatagtttcatgcaggattggagttgcttcttgggcttcttggttctacgaatcctaagcagcaacttgatggtgctgtagctctatataggttagcaaacaaatcaatgactctttctcctgttgatgctgctcctccgtctcctacgccacaggttagctttctggacctcatagttccatgttatccacttttttatgttgtgaaaataagtgatttaattgttgagcatattctgaagctttccatgttggaacttggaagtatctacgtggttaaatgagcttaggtttttgtggttcattagcttttttagaaattctggaatttttaccctgggatgcaatctggcattgtcgaacaatgtcagcttttggcatgtatgttatcttagttcccttggaaaccagtgtcctttttttattggaatatccctcatgtcagcttttggcatgcatgttcttttagttcccctgtaaactggtggccttactttttattggaatatgcctcgagttcccatctgttttgttgaccctttttatacccagtgaattgtgggttggatgtacaaatacgagttttactagcgtagagagtgtttgaaagaaggaattggtactgaaggaagaactaattagtgtatatcaaaggcctttggccttaatccattttttggaaaggctcaggcttcgcttttgggaaaaaaaaaaaaaattgtgcatacactgaccagttgctcataccacttattttctgtatgcactctgcactagttagtaaataaactagtgtatgtttgtgggcaggcatattgtctctacggacctgcataatttcagaatatgagaataaattatacctgaacatttcttttgtgcatatttgatgcttattatcacataataagtgcactgcaggtctacttgggggagcaatatgtaaacaatgctacgttgtctgatgttacttttctagttgaaggtacacatttgaatctggtggttgtcatgatcagtttattatcatgaattgcattttaaaatagaagattgctcttttccattgtaggtagaaggttctatgctcacagaatctgtctccttgcatcttcagatgcatttcgtgcaatgtttgacggtggttacagggtgagcaattctttccaactctcaacttatcccttccagcagccctttcggctgctccacatccgtagtccttcgtgttgtaagccaaggcttgctgcatttgaacattctctgtttgcttatgagatgagatagtgttgtttctttaatagttcagggtttaccatttgaatttacttgttatcgggaattctctaagttcaaaagattttggctggtaatccaagtgttatatcagctcattactaaaaattaaaactggaatacatactgtagttgaaaatatcttcacatttaggatgttttgtatatgttacataatccttcgcttattctacaggagaaagatgcaagggatattgaaattccaaatattagatgggaagtttttgagttaatgatgaggtataatgattattgggcttctgttctcacaaatttctttttttccctaagcggtgatacttacagaagtaaatttcttgaacagatttatatacacagggtcagttgatgttacatcagacatttcacaagatctcctccgagctgctgatcagtatctattagagggacttaagcgactttgtgagtataccattgcacaggtgagcatctgtactggttggtttgcagtgttttgggtaatagcgcttttgaatctcaaagggagcatctcacggttttttttttttatatatttttttaatttttattttcattcccaggatatatcattggaaaatgtttcaagcatgtatgaactttcagaagccttccatgctatctcgttgaggcatgcatgcatcctgtttatcttggggcagttcgataaattgaatggtaggcctgggtaagcattctcactaacctgccatgttctggcaattctaagtaacattcccatgttttcagatgcattgatttttgctggactttaaacctgatgagagtggtctcttcatcgtgaatcttttggctgtagtgcagcaagctgtattcttgtagaatatattcatttttttctgcgtccatgtctgtctaaagtacttgttagaagttacttctgctgagattttcttctatgatgaacctttgcaggcactctcatctgatccagcgaattattccagagatccgcaattatttctcgaagacccttactaaacctaacctaaatagcttgcgcttgtag

SEQ ID NO: 226 - DNA, 5750 bp, Carica papaya
  source 1..5750: mol_type = genomic DNA
atggacgtctcgaggagaaagggcttgaagcgaaaactagagcaagatttccaggaggagaggcaaaattgcaagttggccctcatcgacccccaaccggagcacgatcgtcaaggtctgctcctcgagattcgctcccaggtggaaattctcgattatactttctcttctgaccaggatgatcgcgccgatgctaagcgcgctgctcatgctctctctgagctcgctaagaacggtacgccgctccttctttatgcggatcagggttgtaatacgtgcgcttactatgtccataagctgaacaacttctacttacgtgtttatacatatgcctgtcttgcaattctatttccaggagtaatcaaaatgattgtatttggccgtgtaggttttactgcctcgggttgatctagtactcatgtgaaatggtcactcgcggtgttcgcttgagttttagttgtcttattggtttttccattctccgcttttaatgaaccgcgtttgttcggtttagttttgtcgtagtttttcgatgaactcgttgcatatgatatgtgattccggttatttgagctgttttggggtctaggggtgttgattttggtcattttggcagaggacaacgctgacctggttgtcgactgtggagctgtgcctctgctagtgaggcatcttcaggcgccaccgccttcaaaagcagatgaaaatggacccaaacctctcgatcatgaggtggagaaagcatgtgcttttgcccttggatttctcgctgtaaaagtaattccaatgattcctcaccatttcaaaatttttccattaattctctttatgcttaatgccttttattttcttttattttaagctctcttcactctttgtctcttgttgtattatcaactgttaagtgtttgtgccaagtatataccctactaaaggattttatttatacgtccacttgttgttgcaactcctgcagaagatgtcaaccaacatcacttgctatcatattttcccttccattgcatccgaagccactagccttattgcctctatagctcgatataatttatgttcatattttgttgtagccggagcaccaacaacttatagttgatgctggagctctatcacaccttgtgaacttgttgaagagacacaagaattgtgataacccccgcactgtcagtggtgttattagaagagctgctgatgcaatcactaacctggctcatgagaatgctagaattaaaactcgtgtcaggtatacttgtttgtatgtttgctttctctcattgctgtcacatcctcatttgatatgatccagtttttatcctcagaaatgagggtggcattccacctcttgttgagctgctagagtttgctgatgtaaaagtgcagagggcagcagcaggggccctacggactcttgcctttaagaatgacgaaaacaaaattcaggtcaggtttctttccgctggtcatatcttttagtcacttgagcgttattgtttacatgatagaaaatttgcagatcattgaaagcagtgctctgcccacccttatactgatgcttcggtctgaggatcctcttatacattatgaagcggtgggctcttgtctaaacttttatgccttggtttgtgtccacttggagttttattgctttctttagctgacttccagaggattgtcagattggcgtgattgggaaccttgttcactcatccccaattataaagaaagaagttattcttgctggtgccttacaacctgttattggattactaaggtattgctggaatgcttgattttctatcaggtgtcactttttgcttagtgagattatagttttgatactctattgaaatttgcttccgtttctttctccaaactctattaatgtccttagtgccaaacagaaaaagaaagagcaacttgaagacataaaaagcaaagaatttagttgtttacatgctgaagcattaataactttggtgacagatcttcgtgttcagagacacaaagagaagcagcattgctagttggacaatttgctgctgctgattcggattgcaaggttgatatctctgttcaatgttggatttttagctatcagtactctgctgtattttatttgtttcttttatacgttataaaaagtgagactgctgcaggcgcacattgctcaaagaggagctatcccgccgttaattgagatgcttcagtcttcagatactcagctcaaagaaatgtcagcttttgcacttgggcgtttagctcaggtatttattttgtattactattattatctctatgtttataatggctctggaagacgctacctgcaatttatgagtgtaaaattttatttaaatgttcttggcaattagttatttggttttccaataaaacatatttaagacgtttaactaaattctttgatgattgggtggtaacttcaaatgtaggagactgttgcttgtctaattcgcaaacattagggtgtttatttagatagttatctgggaatcatagaaatcttaacatctgtttgctaatattgcttgatgccaggatgcacacaatcaagctggcattgctcagactggtggtataggtccgctgctcagccttcttgattcgagaaatagtactctgcaacataatgctgcatttgctctgtatggtatagcagataatgaggtaagtattgccggagcacttttttcatttgagtcatctaagagtgtagtgaagcttattttaagttttatgcaggataatgttgcagatcttatcaaacttggaggtgtccagaaacttctggatggagaattcattgttcaagtatgctttaactgctttctgtatttcatatatgggggtcttgacttttaccagcctttcatgctgttattctcctcacctatgcattaatgaattaataatttacgtccttgtttgcgttgggtttctatttggttcttatatttaaaatgtaatttcagccaactaaagattgtgtggcaaggactctgaagagattggaggataagattcacggacaagtaagttgatttatttttagttctttgcactttattctttcaaggtgcttattacacaagcagtggctcaccacagcacaaattctttttctgttttctcgataggtgttgaattatctcctgtatctgatgcgggttgcagataacactgttcaaaagcaggttgctttggctcttgctcatctttgtgcctcttctgatcgaaaaactgtttttattgataacaagggtaggaacgcatgagctgtcacttatccttcagtttctggaaaaacctttgctttattgttcatttggctctctattttcttacctgttcgcttttaatgcataccctgttcttttaggattggatttgctgctggagttcctccagtctgcaagcctgaagcagcagcaagatggttcagcagcattgtacaagttagctaccaagactatttcactgtcccccatggatgcagctcccctatcaccaaccccacaggtaccctttttaagcatctacatagttaaattttggagcatttatatttgttttagtttggggacccagctgaagtatatgatagcagggaacatggatatgctgatgcactgtatacttcagagagaggaaaggaagatttatctcactcattaatgtagatattacatcctttacctataactggtagtgaaagtactgtagcaaggagacttaagagttaacataggatgtgcgcgagtagagatagacacaaaaagacatgtagataaaagagtggttacatgtcctcatctatatgctccttcaagatgatgctcctgttggatttagcagtcttagaccctaaagcttgcagatgataatttggttgtgcctttataagaagttcagcaaattggtccttcctagaagcatgcttgacaaataattcagcagctgaacttccttaccaacgaagtgttaatcaagagcaaaatgcatcatctggctatgggaactgggtttgcatagaaattggcaatactaacattgttaaaataaacctcaagaggtagtagaggagccacttgagacccagctagtaataatagaatctaagataactaggcagtgagggatgtcacagtaggatgctttggcttagttgaagaaggggttatgttatgctgctccatgcggtatgctcaagagttttgaaatgtctgttgttgattatcaactatgacaacatcctgcttgggtcaacctttaattatacatgatttaagttgaattattatgtccagtttgccttcatacctgggactcggtttatatgatcacatgactttttcgcaggtttatttgggtgagcaatatgtaaacaatcctacgttgtctgatgtgacattccttattgaaggtatgatatggtttctctatgattttatacaaatgacaaatactttggtaaatgtgtatatatattgtttgttatcacactggtgcggagttttgaagcttattggaaaaatcattggttctcatggatctttttacataatcaggcaaaaggttctatgcccacagaatttgtctcctagcttcatcagatgcatttcgtgcaatgttcgatggtggatacagggtgagcattgcttcaatgagtttttgaatctttttcctatgagtttactcatttattacgttatatgaaattgtagacacttggcatagcataacttaaaatcattaaaaaaagtagcttaaagaagatttttcagtaagtaaaaagtgggtaacctttttaatgctaattgtttattacttacgtggagaaaacgaaaaattgaatatcaggagagggatgccaaagatgtagaaattccaaatattagatgggatgtctttgagctgatgatgaggttggtttcaaatcctcttcataatttcttgtcacacatgagcaattctgccataacatttcttaactttaacgggctttccgtacctctagattcatttacacaggatctgtagctgttaatgttgatattgctcaagatctcctgagagctgctgatcaatatctgttggagggccttaaacggctatgcgagagtgccatttcaaaggtatgcatcccggttggggttttttttaactaagggaggccaagaagtcagtgtcttttgttaaccttgatatctgctttttaaaataaatacttgatttgtctttttttttttaaaataaatttttctcaaggatatctcggttgaaaatgtatcactcatgtatgagttatcagaagcctataatgccgcgacattaagggaatcgtgcacactgtttgtcctggagcaattccaaaggttgtctcagaagccatggtatgttattcctgtgtatgataatcagatgtctctacagcatttaaaagttgaataccatcaaagacgaaccatattggctttttcctacttgcatttgctctacattccaaatcaatttaattctatcctgcttctactaattatggtgctcgtcagtccagttatgttgatataattacatgcatctgaaaggtcgggagtcaatttgtgatgactcgcaggttttctcgatttattcaacgtatcataccagagattcggaactacttaacaaatgcactcgatcggcctgtattacagaaccagactcagatgtaa

SEQ ID NO: 227 - protein, 715 aa, Carica papaya
MEQEEQQQQRREDQSIPERKGQKRKLEEGITDGEEQEISLSSADARHALLREVSAQVTILDSTFSWKEADRAAAKRATHVLAELAKNEDVVNVIVEGGAVPGLVKHLQAPLISEGDHSSKPFEHEVEKGSAFALGLLAVKPEHQQLIVDNGALFHLVNLLKRHEDGCGSRAVNSVIRRAADAITNLAHENSSIKTRVRMEGGIPPLVELLEFTDTKVQRAAAGALRTLAFKNDENKNQIVECNALPTLILMLRSEDAAIHYEAVGVIGNLVHSSPNIKKEVLAAGALQPVIGLLSSSCCSESQREAALLLGQFAATDSDCKVHIVQRGAVRPLIEMLQSADVQLREMSAFALGRLAQDTHNQAGIAHNGGLVPLLKLLDSKNGSLQHNAAFALYGLADNEDNVSDFIRVGGVQKLQDGEFIVQATKDCVAKTLKRLEENIRGRGLSHLLYLMRVAEKSVQRRVALALAHLCSPDDQRTIFIDNNGMSRLELLLGLLGSTNPKQQLDGAVALYRLANKSMTLSPVDAAPPSPTPQVYLGEQYVNNATLSDVTFLVEGRRFYAHRICLLASSDAFRAMFDGGYREKDARDIEIPNIRWEVFELMMRFIYTGSVDVTSDISQDLLRAADQYLLEGLKRLCEYTIAQDISLENVSSMYELSEAFHAISLRHACILFILGQFDKLNGRPGHSHLIQRIIPEIRNYFSKTLTKPNLNSLRL

SEQ ID NO: 228 - protein, 704 aa, Carica papaya
MDVSRRKGLKRKLEQDFQEERQNCKLALIDPQPEHDRQGLLLEIRSQVEILDYTFSSDQDDRADAKRAAHALSELAKNEDNADLVVDCGAVPLLVRHLQAPPPSKADENGPKPLDHEVEKACAFALGFLAVKPEHQQLIVDAGALSHLVNLLKRHKNCDNPRTVSGVIRRAADAITNLAHENARIKTRVRNEGGIPPLVELLEFADVKVQRAAAGALRTLAFKNDENKIQIIESSALPTLILMLRSEDPLIHYEAIGVIGNLVHSSPIIKKEVILAGALQPVIGLLRSSCSETQREAALLVGQFAAADSDCKAHIAQRGAIPPLIEMLQSSDTQLKEMSAFALGRLAQDAHNQAGIAQTGGIGPLLSLLDSRNSTLQHNAAFALYGIADNEDNVADLIKLGGVQKLLDGEFIVQPTKDCVARTLKRLEDKIHGQVLNYLLYLMRVADNTVQKQVALALAHLCASSDRKTVFIDNKGLDLLLEFLQSASLKQQQDGSAALYKLATKTISLSPMDAAPLSPTPQVYLGEQYVNNPTLSDVTFLIEGKRFYAHRICLLASSDAFRAMFDGGYRERDAKDVEIPNIRWDVFELMMRFIYTGSVAVNVDIAQDLLRAADQYLLEGLKRLCESAISKDISVENVSLMYELSEAYNAATLRESCTLFVLEQFQRLSQKPWFSRFIQRIIPEIRNYLTNALDRPVLQNQTQM

SEQ ID NO: 229 - DNA, 6205 bp, Ricinus communis
  source 1..6205: mol_type = genomic DNA
atggagccacagagaagccaaagtaaagatcaaggtcgtcctgaaaggaaaggccaaaagagaaagctggaggaagagatcgaagacgagcagcaagagatctctgcgtctgctacggcggcggctgcggcagcggttcctttcggggacgcacggcaagcgcttttatatgaggtagcttctcaggttaatatcctgaactctactttctcttggaacgaagccgatcgtgctgctgctaaacgcgccattcatgtcctcgctgagttcgctaaaaacggtagccttttgttttaatgtacttttatgaaatgaaatcaacatctcttactctctttgcttatgagtgctatcttgcatgttttatttataataaaaaacgagatatttttcttttgtatatagaggaattagtgaacgtaattgttgaaggaggtgcagttccggctcttgttaagcatcttcaagcgccaccatcatcatcgagcgaagttgatcgtagtacgaaaccatttgagcatgaggttgagaaaggaagtgccttcgcgcttggattacttgctgttaaggtcctttttgttagaactattttttttaataagtttccgtttcaatatttggcttttagataattgatgatctattatgggttgaagttaggtatattaatttgttcagggagtaaaagttctcatagaacttcaaatgttaggattagatatgttctttgaattattttccgtgtggaaagaaaatctgacttagtggaagatacagtttgcagttttggactatttgcttcatttcatgaaaattttagttgcagacgatatgcatttgtttcctgtttgtggcacttgtggcttttagctaatgatacatttatctacattgtgtaatataattcaatgattaaacatggcatgtaaaatttcttttgtatttgtacaatattttgatgagaaattctatgaacatagcccaattaataacctactttttatttattttccatgccattttcttacacaattgctgtcaacagccagagcatcagcagcttatagttgacataggggctttatcacatcttgtggaactgttgaaaaggcacaaggatggttctgtttctcgagcagtgaatagtgtaattagacgggcagctgatgctatcaccaatctagctcatgagaatagcagcattaagactcgtgttaggtttgctcattttagctgtaattttatttcattctgaatttaccgctacgtttttattctcattgctattggggatacagggtggaaggtgggattcctcctctggttgagttgcttgaatttgttgacacaaaggtgcaaagagcagctgctggggcactacgaaccctggcctttaagaatgatgagaataaaaaacaggtgacagacctttctctggaagttggactctatgaacttgctctttgatatgaataaatgatagagaatgtcttgcagattgttgaatgtaatgctcttcctaccctcattctaatgctacggtcagaggatgctgctatacactatgaagcagtaagatatttcagattgttttgtgttactagttctgaaatctgcattgctatgaattaattttacacttgatatttacttaagcatgaaatactttcttgtcgttctaggttggtgttattggaaatctggtccattcatccccaaacataaaaaaagaagtccttgctgctggagctctgcaacctgttattggcttacttaggtttgcttaagtcttgtattcatggcacttttaaatgtcttttcacttgctttcacttagcttctctttttgttttcttctgtgaagattttgttttgcaatttcttatttatttcttggaaacagctcctgctgctctgagagccaaagagaggctgctctgttacttggacagttcgctgctactgattctgattgcaaggtagacttggacttggattttttaacatttccttccctttcttgagttgagcaacttctgcacttctacatttaattgagagatggagagaagaaatcaaatatcgtcccctcttacttaggtctaagtttttgttccttgcactccctctagctgatgacaatgatctaaatttttgaacattgatggatttagcctcatttgcaaggcccttttgttctgctttaaaattgaaaaagtgatatgcttgtaggttcatattgtacaaaggggtgctgttcaacctttgatagagatgcttcagtctcctgatgtacaactgagagaaatgtctgcatttgcacttgggaggttggcacaggttattatttcttaaactctgttgcatggttgtattaaagtttaaagatcccaacaacattataaaatggctatttggtcttcacgctggtgaattttttatttatatactgttcttgtgaatgaatatataattgtcaccataaagataaatttttttatttctttttacattttgaaatactggaaacaagatatctaggaaaataaataatttattctattagaactgcaaagaatgtggaaaaatgtgtttccctatttagttactaaaaaatgtctaaagaaatttattggaggcctgttaattgcattagttcgttcctttgaataagtgactcgtttgcttacatttctggcagttttgatgtctgagcaaggctattatttgaatttcaacacaatttttttgcttccaggacttgcacaaccaagcgggtatagctcacaatggtggtttagtgccattgctgaagcttctggattcaaaaaatggatctcttcaacataatgcagcatttgctctatacggtcttgcagataatgaggtatgctgtaaattacaaggccttttgtactaaaggacccaaatttttatattttgaggatggcgattttaatcttctacaaccttattatgttcattggttttcctataggataatgtgtccgattttattagggtgggaggtgtacagaagttgcaggatggagaatttattgttcaagtatgttcataagtagcctactctatgatggtagcttgaatatcatgagttcgtgttggaattcaaagcactctttgctggacctatgatgattaatgtagactttataaacatacttgcaggcaacaaaggattgtgtagccaagactttaaaaagattagaggaaaagattcatggacgagtcagttcttcctcctgtggaaactgtaatggtgttatttgtttttcttccaatttagaatttcaacgtaatatttgaaatttataaatttctttgtaggtcttacatcatttactatatctgatgcgtgtaaccgagaaggctgtccagcgacgcgttgctttagctcttgcacatctctgttccccagatgatcagaggaccattttcattgataacaatggcatgttatgttcttcgtaatcttatcaattagaaaaattacattgagaaaaagaaattagtctggaatagtgttttttgactttagatgatcagtgttagtggagattgctgatggttttctaatgcaggattggagttacttcttggccttcttggctctacaagcccgaagcaacaattagatggagcagtggctctgtataagttggcaaataaagcagcgactctttctcctgttgatgcagctcctccttctccaacaccacaagtgagctttctgttgaaacctagccatttgattccattcactttcttatgatgtgaaacataaatttgagttgtaggtaactgtagttaacattgctaagatattcagtataaatggcctttggttactcacttgttatttgtataaatgggtgtcccttgaatttctttccactattactttttcatctctgtttctgatggttaaaaaaaagaaaaggaaacaattgggatttggcatgttacatatcattttgttttttcatttttattgtcacattatcactgtgtaaatatatcttactagaagctttattttagtgcactttagaatatttctcgtcgtcttgatcctcctcaagttgtgaggtctgtgcgcacaccaaatttttagaaaaagaacaagaaaaaacttctagctttaatatatttttctcccttttactaaatggtgagtaagatctggaaattgaatttctatgattaactagtctctcttcctgcaggtatatttgggagagcagtttgtaaacaatgctacattgtctgacgttacctttctagttgaaggtggatattaagttctggatatttacagcctgtcatacttgttagaattgtaatattttgcaattcttgctagttttcatctgagatttgttggcatgaagactcttatataatcacattgactgttgctgcaggtagacgtttctatgcccatagaatttgcttacttgcttcttcagatgcatttcgtgcaatgttcgatggaggttaccgggtgagtgagtatgcttgtcattcatggtctaattgccactatccggacactatttcttttttttttttttcttttgcaaagaggtatacagtctaaattctttgaatgaacttaaactattgatctatgttgctgttaatgacagatatactgttcagctatttagttgaaagccagagtcaatcttgtttattggattcatagttttaagaagtattagggaataacgacggttggaattcttttcatatttgtattttatttaatttttggcatgtgttacaggagaaggacgcaagggacattgaaattccaaatattagatgggaggtttttgagttaatgatgaggtttgataacttggaaaatcaatattatcctaaaaagtatttcccagatagattatttaatgagttatagtttctacagattcatatacactggatcagtagatgtatcattagatattgcccaagatctcctaagggctgcagatcagtatctcttggaggggcttaagcgactttgtgagtatactatagcacaggtgagctccgatggttggttacatgtgtgcatgtgatctgtgttttgctttttagttgacatcgaagttgaatatttgtttgctattctatttcattaaggatatatctttggagaatgttgcaagcatgtatgaactttctgaagctttccatgccatttcattgaggcacacatgcattttatttatcttggaacaattcgataaattgaacgctaagcccaggtacgtgcctgttctcttttattgttttggatttaagtaaatgtttttattgggattcacatggtaccttaacgatcctataatatgtacaaggaaaatgacaatttaatatctcgttccacatcttgattgttaaattgtttttccttttgcacaacagtacaatatattctctttgtggtatagaataagtaggaagatacatttctatgttctaggctctataattggaacttctcacgagtcatggaattttattgtgcatgctacaatttgcaggcactccaacttgattcagcgaattatacctgagattcggaattactttgccaaagcacttaccaaacctaacccacataactcgcggctgtagatggctggtatttgattcttgatgtctaactggaaaatgttgtacagaaagttgtagatcttcacattgttgtctagccatttgagcatcctaatggccgtaatcaccaatcacccctgatgcaagagtgttgtcacatttgcacgcattgtagcatcagttccattttcatggatattgatggagttatgtaaggtggtcatgtatcttgtatgcacccctttgatgagtctgcttgcatcgagtgtaagcaagatttcttctggaaataccaggaaaatttggggcagaagttcaggtctgtaatctaatctttgtctccaggactcggttgctaaaggtgtttgagcacgagaagcttttatgtaaagagactaggaaattaaaagaaaattgttacattttgaatttttttttcttttccaaattgtaatttagttgcagaggtttatatattgttttactggtgcgtgatcccacccaatctttgaacagaactgtgcaaggaactgaactttattcatgttctaatatt

SEQ ID NO: 230 - DNA, 5095 bp, Ricinus communis
  source 1..5095: mol_type = genomic DNA
atggatcaccaaacaatcaccgcaagaaagagcttgaagagaaagcttgagcaggacttccacgaagatagagatcacgatcgcaatcgcaagattcctgctattgaagccgacgatgatgacaccactcgcgaagatctcgcgcgagatattcaagcgcatgtggatgtccttaactccactttctcttctcttgaagcagatcgggctgctgctaaacgcgctgctaacttactctctcagttcgctaagaacggtaactttttttttcttttttatttaaatatatattttttatgtgattaaatttgtttgttaagtggattttattgaattctgattttatttgaatttaggatttaataggtttgattaactcgtgtatttttgcagaggaaattgtaaatttgattgtggactgtggtgctgtgcctgcgctggtgaagcatcttcgagcaccaacgccttctagaggtgaaagtggaccaaaacctaacgagcatgaggtcgagaaagggagtgcttttgcacttggacttcttgctgtcaaagtaatcaacggattttatttatcttcatatttgcatatttcttaggttattagcagcataataaactactacattgtgactctgatcagatggatccagtttccgctgttgctatattttatattgactcaatgtcgattttattttttattcattttatttttacttcttttgattatttttatttatcatttacatgtttgttgattaattgttgcaaaaggacaatgagaaacgtctatgatatggttaatactacttcatttgtgtttggaaactctagagacacaagaatttcaattcaattcaattcaattttatttggtcgattattgtgttttttgaaagcccatagttactattctctcaattaaatagaaagacacacaaggcattttgaaagaagtgaaactatgcttgagaaataacatatggtatactccaaacaaatcataaaagttgcctgtgattgttattggttccgtcattcaattggagtgacttaaggatgtccatagtgtatcttgatttcaatatctgttgtcaatctttttccctaatgattcatcttgatgcattcttaaatatagagtttgtatcttcaactttcagggttgagctatattgcaaacattggctttctgtgtgtaagctatgcatatgaaacttcttttttcctgtagttcttaattttgtaaattttctctatcacttgatgagtagcctgagcatcaacaactcatagtagacgccggggctctgccctatctggtggacctgttgaagagacataagagcagtggtaattctcgagcagtcaatggtgttactaggagagcagctgatgcaatcactaaccttgcccatgaaaataatggcatcaaaacacgtgtcaggtgtgcttgtttttatatttgttatgggttctaaagctagttaccattatatcccttctaacattttggactatacattcaggattgaaggtggcatcccacctcttgttgagctgcttgagtttgttgatgtgaaggtacagagagctgctgcaggggccttgaggactcttgcatttaaaaatgatgaaaacaaaaatcaggtaaatgaattttctcagtcactctttctgatttacttagtgggaaggggatactgtttttgggtgggcaatattgttgatatggaaaataaacttgcagattgtagaatgtaatgctctacccactctaatactgatgcttcaatcggaagatgctatgatacattatgaagcggttagttagctcgcaccttttatatattgcagtttctttcttttacattatgcttaacttggcattgaccgactttcaatgggttgccaggttggtgttattggaaatttggtccactcatctccaagcataaaacgagaagttcttcttgccggagctctacagcctgtgataggattgcttaggtaagaatgaaatttaaatgttttcccattgatgcttttgaagaatcatgtacttggtactaattgtacaactttgacagctcctgctgttcagaaagtcaaagggaagcagctctattattgggtcaatttgctgccgctgattcagattgcaaggtaggagaaatatcatctgtttgtgatgcttgaaaattgaaatttattttaacaatagggatataattttactggagcattgcttgcagactggcactcctcacacacatatatgagtgggaatacgtgcatttgaaatttattttagagtttaattgtaataatattgaggttaatgcaggtgcatatcgttcaaagaggagctgtccgacccttaattgacatgctcgaatcatcagatgcacaactcaaagaaatgtcgacctttgcacttgggaggttggcacaggttattatgtatatctttgacccattgcatggcatgtcttattacacacatgcatgaaactgttggatgacattatggttttgacatttatttcattttatttttaatatctgagtaagtaggaagcatgctatattagtgattctgctgtatgattcatacaattctaaggaatgattagtgtaaataattttataaaataattgttcatcaacatgttcaacaaatagtataagcatatgctactattgtatcaaagttataacctttaagtctaaatctttatcatctttagaagagagctctgcgccctttctcattatttggttctatattgagaccatgcatctctccctctttctctatttgtctctttcgctttcaatggtttgtagtatgctgtgaaagggttttctgctttacgtgcttgttagataccttttctaaatcattacttcttttcaattttaggagacacacaaccaagctggcattgttcataatggtgggatagggccactgcttaggcttcttgagtcaaagaacggatctttgcaacataatgctgcttttgcactctatggtcttgcagataatgaggtaggaattaatttcttctttgcctattttggtttatagtgcaataagttatttactcaggctgaaagttatttggattatttcgataggataatgttgcagagcttgtcaaggttggcggtgttcaaaaactccaagatggtgaattcatagttcaagtatgttttctgatgttttttatttgcaatggcttcttggtacttgagttgacttatgcgcttgttttatatttaatagagctggaaagttatagctgtcttcccttttctgattctgttcgtttgaatattactgtctagctcttattattctgattttgtgattatgcagccaacaaaggattgtgttgcaaaaacattgaaaaggctagaggagaagatccatggtcgagtaagttgtctaacaggatattttggtcattctttactttgattagatctttgattacttgatagacagttcaaggtttttctatttggactgagaatttgggcgcaatagttttctaaatccttttatgcctttcctttacaggtgttgaaccacctcttatatttgatgcgcgttgcagagagaactgttcagagacgaattgctttggctcttgctcatctttgtgctcctgatgatagaaaagctatttttattgataacaatggtagaatttctggtctgctaaatttttctacctttgtttctttatcagtcgcattcatatggactggaatggagtaattgattttataatatatgtatatnnnctgctcctctgtccccaaccccacaggtaagttattcatatgttatccttttgatgcatctgcaatttttccttaacaactctatgaatgttttgggggatatgacttttatacacgagtatgtgcttgaactgaggattttattttctaatcatatgtggttcactagtttatgtaattagttgttttttctttacataattgcttacagcgctttttttttttttttttttccaaaaggtgttgagacataattattatgattggttggtttggctgtcatcaatcaattcatctctagtgttttagccatttgttatcctctcatattggggtaaaaacagcagctgcaaaattcatttttgttcttattgtttttaccataggtatatttgggagagcaatttgtgaacaatcccacgttgtctgatgttaccttcttagttgaaggtaagataaatttgcatacaataacttgaacttccaaataccatactaatgtcaatattttccctttatagtcattactaagagcaatgattgtaattttgtttgaccaggtaaacggttctatgctcatagaatttgtttgcttgcttcttcggatgctttccgtgcaatgtttgatgggggttacaaggtgagaagttataacatcctaaaagcttgcttttatataatgaattttctatttattctttattgttgctcttgcaccaacttggccccctaacaaatgcatttacattagacagcatagggaaaagtagtcagaattactcagttgcagttgcgatcttactttttggtcaacagtaaactgtcaatttataaagaaatgtttgtttaattgatctgtacaatgtcttgcattctagttatatgtttgctttatgccaggtaaaaatgaaatttgcagttgctggtaaaatggcttattaatgtctgatttgttacttctgaaaattgcaggagagagatgctaaagatgtagagatcccaaacattagatgggatgtctttgagttgatgatgaggtgaggtgttgcctttgcttcttagttccagagcgaacttgccttctgctttctagtacctcactgatgtgtgttctgtttctaggtttatatatacagggtctgtggatgttgatattgagattgcacaagatctccttagagctgctgatcaatacctcttggaaggccttaagcgtctctgtgaatatactattgcccaggtcaggtcccgtgccttttcaatagctgctcttcaataa

SEQ ID NO: 231 - protein, 719 aa, Ricinus communis
MEPQRSQSKDQGRPERKGQKRKLEEEIEDEQQEISASATAAAAAAVPFGDARQALLYEVASQVNILNSTFSWNEADRAAAKRAIHVLAEFAKNEELVNVIVEGGAVPALVKHLQAPPSSSSEVDRSTKPFEHEVEKGSAFALGLLAVKPEHQQLIVDIGALSHLVELLKRHKDGSVSRAVNSVIRRAADAITNLAHENSSIKTRVRVEGGIPPLVELLEFVDTKVQRAAAGALRTLAFKNDENKKQIVECNALPTLILMLRSEDAAIHYEAVGVIGNLVHSSPNIKKEVLAAGALQPVIGLLSSCCSESQREAALLLGQFAATDSDCKVHIVQRGAVQPLIEMLQSPDVQLREMSAFALGRLAQDLHNQAGIAHNGGLVPLLKLLDSKNGSLQHNAAFALYGLADNEDNVSDFIRVGGVQKLQDGEFIVQATKDCVAKTLKRLEEKIHGRVLHHLLYLMRVTEKAVQRRVALALAHLCSPDDQRTIFIDNNGLELLLGLLGSTSPKQQLDGAVALYKLANKAATLSPVDAAPPSPTPQVYLGEQFVNNATLSDVTFLVEGRRFYAHRICLLASSDAFRAMFDGGYREKDARDIEIPNIRWEVFELMMRFIYTGSVDVSLDIAQDLLRAADQYLLEGLKRLCEYTIAQDISLENVASMYELSEAFHAISLRHTCILFILEQFDKLNAKPRHSNLIQRIIPEIRNYFAKALTKPNPHNSRL

SEQ ID NO: 232 - protein, 598 aa, Ricinus communis
MDHQTITARKSLKRKLEQDFHEDRDHDRNRKIPAIEADDDDTTREDLARDIQAHVDVLNSTFSSLEADRAAAKRAANLLSQFAKNEEIVNLIVDCGAVPALVKHLRAPTPSRGESGPKPNEHEVEKGSAFALGLLAVKPEHQQLIVDAGALPYLVDLLKRHKSSGNSRAVNGVTRRAADAITNLAHENNGIKTRVRIEGGIPPLVELLEFVDVKVQRAAAGALRTLAFKNDENKNQIVECNALPTLILMLQSEDAMIHYEAVGVIGNLVHSSPSIKREVLLAGALQPVIGLLSSCCSESQREAALLLGQFAAADSDCKVHIVQRGAVRPLIDMLESSDAQLKEMSTFALGRLAQETHNQAGIVHNGGIGPLLRLLESKNGSLQHNAAFALYGLADNEDNVAELVKVGGVQKLQDGEFIVQPTKDCVAKTLKRLEEKIHGRVLNHLLYLMRVAERTVQRRIALALAHLCAPDDRKAIFIDNNEQFVNNPTLSDVTFLVEGKRFYAHRICLLASSDAFRAMFDGGYKERDAKDVEIPNIRWDVFELMMRFIYTGSVDVDIEIAQDLLRAADQYLLEGLKRLCEYTIAQVRSRAFSIAALQ

SEQ ID NO: 233 - DNA, 7278 bp, Citrus clementina
  source 1..7278: mol_type = genomic DNA
tctgatcacactcctctcttcgcttcgccttctctctcagtgctttgtccctgatttgatggatccacagagacgccaagggccgagcgtccccgagaggaaggggcaaaagcggaaactagatgaagaaacagtgatcggagacgagcagcagcagatgcaacaacgagagatctcgtcttcttctgctggaacttcttcatccgatgcgcggcaagcgctattgagcgaggtcagtgctcaggttaacgtccttaacaccactttctcttggctcgaagccgatcgcgctgcggctaaacgcgccactcacgtcctcgccgagctcgccaagaacggtccgtaccttccaaaactgcctctcgatctcgagttatttacgcctctgtcactggttttttaatgcgaaggtctgtatttgtggttgcagaggaggttgtgaactggattgtcgaaggtggcgcggttcctgctcttgtgaagcatctacaggcgccgccgacgagtgaagctgaccggaatttgaagccttttgagcatgaagtcgagaaaggaagcgcttttgctcttggacttcttgctgtaaaggttgttttagcaattattctatttgcttagttaagcttggcttggagtctcattttattgatagtgattattttactcatgcatgttattattattttgaattgttctaattttactctttctggaaatagctataataataagctgctattggtttcattttagaataattagactaaatcccacagtatgcatgctatgatagttgttttgtcgcgattactataataattggtaaggctatatatttttggtgaaactaagaaatgtaaacaattcttggaaggcaagtgaagattagatgttaagcactacaaactattataatgtcgaaagtggtgtgctttatggttgtaagtttatgttaggattgaatggctgtattgaattattttactttagattttaaaggatttataatttaaagaatttacaatgttattgaatgggactaataaaagaaatttagaaacgccacctaaagaaatgaacaggatttcttttgagattcttatgacatgcttaatttttttttctctcccttttttttcaagaaattattttatccaagattcatcaccttgttcttgaaactatgtcctaaaaagattttttatcaatgttctagcattaagaagttgcttttgaaatttcaagggaaagtagaaaggtactattttgctggcatttatttttcttgattccaataagtcttagttgtatagcattgtcaattttattgttattgtttctgttgcatgactaataacaattcttgctatacttgcaaataaaatggcattgaagcatttaaaactgtaaaatagatattctattatgtatgagtactgaacctgtgaattttttatggattttgttggtaacagccagagcatcagcaactcatagttgataatggtgcattgtcacatcttgtgaatttgctgaagaggcacatggacagtaattgttcccgtgccgtgaatagtgttattagaagagcagctgatgctatcaccaaccttgctcacgagaacagcagcatcaaaacccgtgtcaggtctcatgatttttgtaactttttattttgagtcaggcgtttaccaattagtgccatgtttatctcattgttatcgtgttctggatatgcaggatggaaggtgggattccacctctggttgagttgcttgaatttactgacacaaaagtgcaaagagcagctgctggtgccctgcgaactttggcatttaaaaacgatgaaaataagaatcaggtaacaaacaatttgttggaagctgcatattgttaagctggcattggtatctacaaattatgaaattactatgtttttgcagattgttgaatgtaatgctcttcctaccctcattcttatgctacgatctgaagattctgctatacattatgaagcggtaggattttatcagagtgggttttctattagtttctgaaaattgtgcaagtgcaatattttatgcttttatttctctttggctatcaaatgaagttaattttcatgaattccaggttggagtaattgggaatctggtacattcatcccccaacataaagaaagaagttcttgctgctggggcattgcaacctgtcattggactacttaggtatgcataaattttgtttcttttacaacatttgtgatgttctgcctggtttaggtgttttggagaggttttcgcccttcttctgctattgctttagatattacggtttttaaccttagtagaacagcttagctctttttttctcaattcattgggtttgttaattggatgacagttcgtgctgctccgagagccagagggaggcagctttgttacttggacagtttgctgcaactgattcagattgcaaggtgggcacaacttgtcattgtctttatcttatttttccttgataaagtttattcttctcccaggttttctgcttggccgtgcaagatatgaggaatgaattgaaaatgaattttttaagtggaaatgtaaaataaattttgtttcctctgactatccttttagcagaagtattggtattggttcacttgttggtcatcatgtgcttttagccttctcatccttgtacaattttccatcagacttgtctctccttttatttattttaatatatatgcaggtacacattgtacagaggggtgctgtgcggccactaattgaaatgcttcaatcacctgatgtgcaactgagggaaatgtcagcctttgccttggggaggttggcacaggttatcacggtttcagtcttacctgctatccttatctttatcataattaatgaatgtcaactagaagttttggcttttgtgctttctgagatggtgctgctcttttgtagatagtgctatgatttgtatggtagattacatgtactttcattttcttgtaggaactagaaattaattcacagtttccctcaagcttttgtcaagttctattggtttttaatagtgcggttatgctatggtcatctttggtatccaaatacttcttcagaggtttttttctcttgcatatttgtttttgtactggtcatcnnnnnnnnnnnnnnnnnnnnnnnnnnnnnnnnnnnnnnnnnnnnnnnnnnnnnnnnnnnnnnnnnnnnnnnnnnnnnnnnnnnnnnnnnnnnnnnnnnnntttcccccccccccccccccccccccccaaaaaaaaaaaaaacaaaaaaaagtgcaagtaatattacatttttgtcagttttttgttctagtgccagaaaattaagttagcttgaaaatagaatttctttgcttaaatgtatttttccaatttaggacatgcacaaccaggctggtattgcacataatggtggtttagtgccattgctgaagcttcttgattcaaaaaatggttctctgcaacataatgcagcatttgctctatatggtctcgcagataatgaggtacattgtattcttttgaattcttatgaatattagaactgaaaaatttgagtttttatttcaagaagttattaacatactttgttggactcttctctcataggataatgtagctgattttattagggtaggaggtgtgcagaagcttcaggatggagaatttattgttcaggtatgctcaacaaattttcaaattagctgttatttctacaatttgtattaacttttatgactatatggttgcttaccattgttcatactcatgaatcggagactgagattcttgttagttcattttaaccttggacctacaatcaccagtatcgagaattgtacttgcaggcaacaaaagattgtgtggcaaagacattgaaaagattggaagagaagattcatggacgggtgagtattttgatccctatcttcgaagtattcagccgacatggactacttctaattttatgtttggatttttattctgtgatctcatgattttcttgatacaggttttgaaccatttgttatatctgatgcgtgtagcagagaagggtgtccaaagacgtgttgctttggctcttgctcatctgtgttcccctgacgatcagagaactatatttatcgatggtggtggtatgttgcattaccagatatactttttggtaattctgggttcatgttgccatgcatttgttctgatttagctggtgcaaagtcacggttgagatgttcatattggtgtgaatggtgctataactattcaatttcatgcaggattggagttacttcttgggcttctgggttcaacaaacccaaagcagcaacttgatggtgctgtggctttgttcaagttggcaaacaaagcaacaactctttcttctgttgatgcagctcccccatctccaacccctcaggtgaggtttaagaatggttttttacataccttgtcttatgatgaaaatgtaaaatagaagtgaagagttctctgatgtggggcaacttctatttgttatttattaggctttatgtatgttgaggaactcaaatcattcaagaaaagaaaacacaggaatcatttaaaagctttttacaatggcaactgagtcaaagctagtaatctcattatcttctatcaaacctattaaagaaataaccaaagctcaactggatacaaagaaaaattcttagaatgaaactgcgttagaaacaatcaaattagattatctttcaatgtttataattgctgagagtttggtgcctatgatgacagtcagtgcttggtgcaggtctatttaggagaccagtttgtaaacaatgctacgttgtcagacgttacctttctagttgaaggtttaaatttactttcttaataacatgagttcttgcttaattctgctgcatatgttggaatgacttgctaaatcatttttttccatagacgtttcgttagcacaagttctctttttgaattataaaattgcctcctttactgcaggaagacgtttctatgcccaccgaatttgtctacttgcatcttcagatgcattccgtgcaatgtttgatggtggttaccgggtgagtgtctatgtctactatcttggtccccaacccccactcttcaatcatcttatcttctgtatttgcgtgtgtagggtggggctgttgtactagagtttaaaaaaatttggctatgggagtgctgcactgtcaaaatctttgactttgtggctgaagtataacatttctttggattatacgaaatttaagctcaaacttatctgttttttttttaaaaaaataaaacattgattgcagattcattttctggttactcaaaagcataatcatctggtgctcttatctttcaatgcaaattgaagcactcgaaagcatagatgcttttaagatatgcattgaaagtatagctgcttttaagacatgcatattgtgactaacttacggtggattttattgtaggaaaaggatgctagggacattgaaattccaaacattagatgggaagtgtttgagttgatgatgaggtttgatgaattctgtgcctttaacttgagctctttataattgctttcccttgaacatctgggattactggtttattctgctgcagatttatctacactggatctgtagatgttacattggatattgcacaagatctccttagagcggctgatcagtatctcttggagggacttaagcgactctgtgaatataccattgcacaggtgagcttataaggcctttttttttaaaaaattttttttaatccctcaatgctgcttgtaaattgaaagtagttttctaatcaaatattctattttcgttgtaggatatatctttggaaaatgtttctagcatgtacgaactttcagaagcttttcatgctatatcattgaggcacacatgcatcttgtatatcatggagcactttgataaattgagtactaggcccgggtatgtgatcccactatcctgctatgttcctcatctttcttctttgactctgttaacttggaactttagtgatttggtaagttaagtagagttggaccaagtcctaaggtaggtgcccaattaaaatttatttgttatgccacagaaaattataatgagctggacggttttaagatagttattctcttcaatgcattgtgccatggcaattattttattttattattttgtcttatcgaggaaaaggggtttttgtagaatgctaagtatgttcactatttaatgaccaatctcttaggatcacttgtatgcttgacagtgattaccttttacaggtagaagatattgatgttgcattttgaggtctatatatgtggcctgtatgcataatctcagttgcttataattccttttactgatgtcacatagaagttagcaacataaaattaattgtcttaatccttcacatgggattttgtcttgttaaggtttttaagctctggggaaaagataagagaggaatagcttgaatcattgaaatgagcgatataaagcagcaaaatatatgattgccaaagtgaccatgtgctctttgcaaatcatatttgttaatggaaagtttgcttcagcatttaaagttgatattggttgtctctcctgccatcttcttttgtttttctttgttcaaattctgcaatagttattttcctgtagaaaacgggagtagatttttgtgtccacgtgaactttcctgctgctataaacatcttacaatcatttgctgaaaccatctgcttgttgaaaacttgcaggcattctaatctgatccagcgtatcattccagagatccacaattactttgcaaaagctctcaccaaacctaacccacataattcgcggctgtagatggccagtcattgattcttgatcgctaactagttatgatgtacagaaaatagtagatcttttcactgatatcaagtcaagtgaagctcctaattggttgattgtagtgtggctcataatcatttcctgatgccagagttatgttggttgtagactgtaagttgcttcttcaagttaattgttgtaggtactgcttgaaatataaccttcacaaaacattattgattttcatggattgtgatggttgtatgtctcgaaatgtattttatgactattcactgaaattgaattcgttgagatgtatcttttgcttgtgcaatagtaggcttctttgataactaa

SEQ ID NO: 234 - DNA, 5791 bp, Citrus clementina
  source 1..5791: mol_type = genomic DNA
cctagcatcgtctccatcatttacatccaattcttgatggatcgtcgggagcgccaaacctctccggctcgaagaagcttgaagcggaagcttgagcaagatttcgaagagaaacctgatcgcaaggtctcgatcgtcgaatccggcgccactcaacaagatctcgttcaagatatccgcgctcagattgatatactcaactccaaattctcttctgatgaaaccgatcgcgccgccgccaaaaccgcctctcacgctcttgttgaattcgccaaaaacggtactgttttcgacatttctatcctgattataaatatatatgtaactgcacaaatttgtgagggtgttgtttgtctttgtcgcacctggttctttcaagaaatggaatattgatggccaaatttaagcacttcgtctgaaatcacttcgcgttgattggctataataattatgtaaatttttcgtatttgtagtcattttttagtttattttcgttctggttctaacaaacaatgtgttggcgcagaggaaattgtgagtttaattgtggataatggagccgtgcctgcattggtggaacatctccagacgccaccacagttgacgaatgctcagatcccgtacgagcacgaagtggagaaagaatgtgcttttgcgcttggacttcttgctgtcaaagtaattgactaccttaactgaacgcatgaattgttacttcatagtatttgaaaaaaaggtgtcacggccaagtgacttatcttcatttttgtatctttgtagttttatttttgttagttgaacatttcttccaaagtagagtcatactattgtgctccggacattttgtttctcttttatgtgtctgcatcttggttgatgtttttagctgtttgtttaccttgtagtatttaccctgcttgttatgctttgttaaatagccagagcatcaacaaatcatagttgatactggagctttgccccatctcgtgagcttattaaagcagtataagaatggtggtaattctcgggcactcagtggtgttattaggagagcagctgatgcaatcaccaaccttgcacatgagaacgccaacatcaaaacccgtgtcaggtttacttgtttgcatattttgcttttcttatataaattattgtaccctctttctaatgtctctgtcgtacattcagggttgaagacggcatcccccctcttgttgaactactgaagtttgtagatgtgaaggtacaaagggcagctgctggtgccctgcggactcttgccttcaaaaatgatgaaaacaaaaaactggtacagttttcttgctaaattatacacttgaggttcttaagcaactttttcttcttatttttattgaaaataaataaattttgagttcgcagattgtggaatgcaatgctctacctacccttgttctaatgctgcgctcagaggatgctagtgtacacttcgaagctgtgggcactctttcaaattcataatatttgtagtttcaattcacaacttcatgatgctttgatcattgactgactaactgacttcacctgagattttcaggttggtgtgattgggaatctagttcactcttccccaagcataaagaaggaagttattcttgctggggctttgcaaccagtcattgggctgctcaggtaaatattgaattttgcaaagttcgcctttttctgagctgaattctaattactcttatggtgtcttatttacctgcctcaggctatatcataagatttgctttcaatttactctataaggttctttattattattaataaactaataattgaagaagctgatcaatttgcaacagttcctcctgttcagaaagcaaaagagaagcagctctgttacttggtcaatttgctgcggccgattcgaattccaaggtatactgaaataatttcctctttatgacttgactttttaatcttttatatcggcagtagtcaaggaaattaggtcataaatttatattaccagccccattttcagtgcaacaaaaatgagtttcatgcaggtgcacattgttcagagaggagctgtacggccattaattgaaatgcttcagtccccagattcacagcttaaggaaatgtctgcttttgcactagggagattggcacaggttattatttcctcaatcctgttgtgcctttttcaaagaagatactaatataaatggcattagaaggctgctatatttaattgttatcagctggacttgaatagtttgagctgttatactctactttcattttatgaggaaggttacttaatataaatgtaaactgaattctgttatgatggtattttagtaaacaattgtgtaaacattctaaggtgttttgcatggatgattattaggtttatgtagatatatctctgttatcatcttgttctattcttacagtaataagcatccactgattctgattcacggcaaatctttctatctgctttggtttttcctgaaagattttggtgcatcaaagtccttaattttgtgcataacaacttatgtggcaatcaatctttatgttatccatcctcattaaatttctctagtaactagtaacagaaaagttttgtttctatttgacaaatgtcttgttcaatatatttttatcctgaaaggtttgggtgctatgcagatgtgcgtgttttttccgagtatgctaaaactgtttaattgtaggacacacacaatcaagctggcattgctcaggatggtggtatattgcctttgctaaagcttcttgattctaaaaatggatctctgcaacataatgctgcatttgctttatatggccttgcagataatgaggtatggttaaggtcattcagtcattttattttgctgtaatctgtcatttgttatccatctaatttatgtatttgtacttacatcacaagttgtttccataggataatgttgcagatcttgtgagggttggaggtgttcagaagctccaggatggagaattcactgtgcaagtatgctcatgtttccattttactagaaactacattatagatacttccctttattgttccattcagagttttgttgctagctgttacaaaaattttcatgatacttgtagccaactaaagactgtgtagcaaggacattaaaaagactagaggagaaagttcacggacgagtgagttcgttcatctctactttttaggaaatctacttgatttgaattgtaaaatttagttttttcatggaagaaattgattgtataagcataagtttgtttgacctggtgtatcaattttgtcaatgttttgacaggtattgaatcatcttttgtatctgctgcgagttgccgacagggctgttaaaagacgagttactttggcccttgcccatctttgtgcccctgatgattgtaaaactatttttattgataacaatggtataaatacttgagctgagctacctactttgatcccagttgtctttgttgcatacgtttactccagcagttcaagtcaggttttctctggttcttggctccttcattgttcacttgtttttcctgcaggattggagttactgttggggctccttgagtctacatctgtaaagcagcgagaggaaagttcggtggccttgtataagttggctaccaaagctacttctctatctcctatggatgcagctcctccatcaccaacccaacaggtgtgttttctgaatttctgccagctttggggtataaattttctagtttcttaggtgaaatagaaaatgcgggctgaagatgtgcacttgatatgaatgtgcatttgctttctttgctgcgtcttatagttcaattcaagagagccaatgtaaattatttcctaggttatggagttttgaagagttggctattttgaccaccagctgatcttcaattacatgccttttttttggaaggggggggggggggggggggagttgatttgttaaaataacccttactctatccaccccgagcaattatcctataactactcttcttttgaccttttgcttgaaattcggaagattagcctgtaatttgagccatgacttttgtcttcctaaaacataaattaatgttgctcaataagcttccttctttttatgctcaatggtccaaagcactgattctagttctttatttcagactcaacattgtgttgacttcctcattcttgatatcagtttcatctgttcacattttgcattgtaacaatttcataattttgctgtaggtgtacttgggtgagcaatttgtaaacaatcctacgttgtccgatgtgacatttgttgttgaaggtatacatttgtttccactttgatttgaaattattgctccttttttgtgtttcttaatgacacgagcatactattctttcttaacgttgtcaggtaaacaattttatgctcacagaatttgtttgcttgcttcgtcggatgctttccgtgcaatgtttgatggcggttacaaggtgagcattgacttattttagagctatcttgtttcttgctaaatgcttaactaaaagaagatgaaataaaacagataaatctgcaaaataaaagactgagaatcatgtatgaggattcagtcatagtcagatttctttctgaacattctgcatctactgatctgtgcaatattttgcattctattggctgattgccatgtatcattatgaaatttggatttataacttattgaagctttataaaaatgcattgcaggagaaaaatgcaaaagatgtagagattccaaatatcagatggaatgtttttgagttgatgatgaggtctgagctttgcattctcccttaaaagatgaatgattaagcaaatatcccctgttgatattttattgtattttggatgtttgtagattcatatatacaggaaatgtcgatgtcagtgtagatattgctcaagatcttctgagggctgcagaccagtatcttttagaaggtcttaaacgactctgcgagtattccattgcacaggttggctaaatgttgagtttgatttgtgtttttaacagcattatagtattcttaatatttagtctaatgatttattttctctccttagattatttctgttgaaaacattatgctcatgtacgagttatcagaggcctacaatgctacgacattaaagcaatcatgcatactgtttatattggagaaatttgacaaaatgagaaacaaaccatggtatgctacctccttccaccttgattgtccatttttcaagctgctttgaacaattaatttcaatattcttggtgtataaatttctggccgttcttttaattagattttgggtttaaggagggaaatttatcttaactacctatgacaatcgtggtaataaatcatgctagaaaatttgctttcacattttttcaggactttgaatctttgtggtagtctgaaaaattgttatttctgcaatggctttgaagtgaaattattatctgaatcccatattcagtgggatttcctagaacatttgaatgatattaaacactgccaatgtctctagtctttcctgtgccattttagtttcgtgtagtcagtggtatatatgtttggaccctaactgaatttgagaaattctaattcaactatttgacaacacgcaggttctttcgtttgatccgttgtgtgttaccagagatacgaaattacttcacaaaagcattttcgaatcctgtcattgtgaattcaagccagttgtga

SEQ ID NO: 235 - protein, 717 aa, Citrus clementina
MDPQRRQGPSVPERKGQKRKLDEETVIGDEQQQMQQREISSSSAGTSSSDARQALLSEVSAQVNVLNTTFSWLEADRAAAKRATHVLAELAKNEEVVNWIVEGGAVPALVKHLQAPPTSEADRNLKPFEHEVEKGSAFALGLLAVKPEHQQLIVDNGALSHLVNLLKRHMDSNCSRAVNSVIRRAADAITNLAHENSSIKTRVRMEGGIPPLVELLEFTDTKVQRAAAGALRTLAFKNDENKNQIVECNALPTLILMLRSEDSAIHYEAVGVIGNLVHSSPNIKKEVLAAGALQPVIGLLSSCCSESQREAALLLGQFAATDSDCKVHIVQRGAVRPLIEMLQSPDVQLREMSAFALGRLAQDMHNQAGIAHNGGLVPLLKLLDSKNGSLQHNAAFALYGLADNEDNVADFIRVGGVQKLQDGEFIVQATKDCVAKTLKRLEEKIHGRVLNHLLYLMRVAEKGVQRRVALALAHLCSPDDQRTIFIDGGGLELLLGLLGSTNPKQQLDGAVALFKLANKATTLSSVDAAPPSPTPQVYLGDQFVNNATLSDVTFLVEGRRFYAHRICLLASSDAFRAMFDGGYREKDARDIEIPNIRWEVFELMMRFIYTGSVDVTLDIAQDLLRAADQYLLEGLKRLCEYTIAQDISLENVSSMYELSEAFHAISLRHTCILYIMEHFDKLSTRPGHSNLIQRIIPEIHNYFAKALTKPNPHNSRL

SEQ ID NO: 236 - protein, 704 aa, Citrus clementina
MDRRERQTSPARRSLKRKLEQDFEEKPDRKVSIVESGATQQDLVQDIRAQIDILNSKFSSDETDRAAAKTASHALVEFAKNEEIVSLIVDNGAVPALVEHLQTPPQLTNAQIPYEHEVEKECAFALGLLAVKPEHQQIIVDTGALPHLVSLLKQYKNGGNSRALSGVIRRAADAITNLAHENANIKTRVRVEDGIPPLVELLKFVDVKVQRAAAGALRTLAFKNDENKKLIVECNALPTLVLMLRSEDASVHFEAVGVIGNLVHSSPSIKKEVILAGALQPVIGLLSSSCSESKREAALLLGQFAAADSNSKVHIVQRGAVRPLIEMLQSPDSQLKEMSAFALGRLAQDTHNQAGIAQDGGILPLLKLLDSKNGSLQHNAAFALYGLADNEDNVADLVRVGGVQKLQDGEFTVQPTKDCVARTLKRLEEKVHGRVLNHLLYLLRVADRAVKRRVTLALAHLCAPDDCKTIFIDNNGLELLLGLLESTSVKQREESSVALYKLATKATSLSPMDAAPPSPTQQVYLGEQFVNNPTLSDVTFVVEGKQFYAHRICLLASSDAFRAMFDGGYKEKNAKDVEIPNIRWNVFELMMRFIYTGNVDVSVDIAQDLLRAADQYLLEGLKRLCEYSIAQIISVENIMLMYELSEAYNATTLKQSCILFILEKFDKMRNKPWFFRLIRCVLPEIRNYFTKAFSNPVIVNSSQL

SEQ ID NO: 237 - DNA, 5922 bp, Citrus sinensis
  source 1..5922: mol_type = genomic DNA
atggatcgtcgggagcgccaaacctctccggctcgaagaagcttgaagcggaagcttgagcaagatttcgaagagaaacctgatcgcaaggtctcgatcgtcgaatccggcgccactcaacaagatctcgttcaagatatccgcgctcagattgatatactcaactccaaattctcttctgatgaaaccgatcgcgccgccgccaaaaccgcctctcacgctcttgttgaattcgccaaaaacggtactgttttcgacatttctatcctgattataaatatatatgtaactgcacaaatttgtgagggtgttgtttgtctttgtcgcacctggttctttcaagaaatggaatattgatggccaaatttaagcacttcgtctgaaatcacttcgcgttgattggctataataattatgtaaatttttcgtatttgtagtcattttttagtttattttcgttctggttctaacaaacaatgtgttggcgcagaggaaattgtgagtttaattgtggataatggagccgtgcctgcattggtggaacatctccagacgccaccacagttgacgaatgctcagatcccgtacgagcacgaagtggagaaagaatgtgcttttgcgcttggacttcttgctgtcaaagtaattgactaccttaactgaacgcatgaattgttacttcatagtatttgaaaaaaaggtgtcacggccaagtgacttatcttcatttttgtatctttgtagttttatttttgttagttgaacatttcttccaaagtagagtcatactattgtgctccggacattttgtttctcttttatgtgtctgcatcttggttgatgtttttagctgtttgtttaccttgtagtatttaccctgcttgttatgctttgttaaatagccagagcatcaacaaatcatagttgatactggagctttgccccatctcgtgagcttattaaagcagtataagaatggtggtaattctcgggcactcagtggtgttattaggagagcagctgatgcaatcaccaaccttgcacatgagaacgccaacatcaaaacccgtgtcaggtttacttgtttgcatattttgcttttcttatataaattattgtaccctctttctaatgtctctgtcgtacattcagggttgaagacggcatcccccctcttgttgaactactgaagtttgtagatgtgaaggtacaaagggcagctgctggtgccctgcggactcttgccttcaaaaatgatgaaaacaaaaaactggtacagttttcttgctaaattatacacttgaggttcttaagcaactttttcttcttatttttattgaaaataaataaattttgagttcgcagattgtggaatgcaatgctctacctacccttgttctaatgctgcgctcagaggatgctagtgtacacttcgaagctgtgggcactctttcaaattcataatatttgtagtttcaattcacaacttcatgatgctttgatcattgactgactaactgacttcacctgagattttcaggttggtgtgattgggaatctagttcactcttccccaagcataaagaaggaagttattcttgctggggctttgcaaccagtcattgggctgctcaggtaaatattgaattttgcaaagttcgcctttttctgagctgaattctaattactcttatggtgtcttatttacctgcctcaggctatatcataagatttgctttcaatttactctataaggttctttattattattaataaactaataattgaagaagctgatcaatttgcaacagttcctcctgttcagaaagcaaaagagaagcagctctgttacttggtcaatttgctgcggccgattcgaattccaaggtatactgaaataatttcctctttatgacttgactttttaatcttttatattggcagtagtcaaggaaattaggtcataaatttatattaccagccccattttcagtgcaacaaaaatgagtttcatgcaggtgcacattgttcagagaggagctgtacggccattaattgaaatgcttcagtccccagattcacagcttaaggaaatgtctgcttttgcactagggagattggcacaggttattatttcctcaatcctgttgtgcctttttcaaagaagatactaatataaatggcattagaaggctgctatatttaattgttatcagctggacttgaatagtttgagctgttatactctactttcattttatgaggaaggttacttaatataaatgtaaactgaattctgttatgatggtattttagtaaacaattgtgtaaacattctaaggtgttttgcatggatgattattaggtttatgtagatatatctctgttatcatcttgttctattcttacagtaataagcatccactgattctgattcacggcaaatctttctatctgctttggtttttcctgaaagattttggtgcatcaaagtccttaattttgtgcataacaacttatgtggcaatcaatctttatgttatccatcctcattaaatttctctagtaactagtaacagaaaagttttgtttctatttgacaaatgtcttgttcaatatatttttatcctgaaaggtttgggtgctatgcagatgtgcgtgttttttccgagtatgctaaaactgtttaattgtaggacacacacaatcaagctggcattgctcaggatggtggtatattgcctttgctaaagcttcttgattctaaaaatggatctctgcaacataatgctgcatttgctttatatggccttgcagataatgaggtatggttaaggtcattcagtcattttattttgctgtaatctgtcatttgttatccatctaatttatgtatttgtacttacatcacaagttgtttccataggataatgttgcagatcttgtgagggttggaggtgttcagaagctccaggatggagaattcactgtgcaagtatgctcatgtttccattttactagaaactacattatagatacttccctttattgttccattcagagttttgttgctagctgttacaaaaattttcatgatacttgtagccaactaaagactgtgtagcaaggacattaaaaagactagaggagaaagttcacggacgagtgagttcgttcatctctactttttaggaaatctacttgatttgaattgtaaaatttagttttttcatggaagaaattgattgtataagcataagtttgtttgacctggtgtatcaattttgtcaatgttttgacaggtattgaatcatcttttgtatctgctgcgagttgccgacagggctgttaaaagacgagttactttggcccttgcccatctttgtgcccctgatgattgtaaaactatttttattgataacaatggtataaatacttgagctgagctacctactttgatcccagttgtctttgttgcatacgtttactccagcagttcaagtcaggttttctctggttcttggctccttcattgttcacttgtttttcctgcaggattggagttactgttggggctccttgagtctacatctgtaaagcagcgagaggaaagttcggtggccttgtataagttggctaccaaagctacttctctatctcctatggatgcagctcctccatcaccaacccaacaggtgtgttttctgaatttctgccagctttggggtataaattttctagtttcttaggtgaaatagaaaatgcgggctgaagatgtgcacttgatatgaatgtgcatttgctttctttgctgcgtcttatagttcaattcaagagagccaatgtaaattatttcctaggttatggagttttgaagagttggctattttgaccaccagctgatcttcaattacatgccttttttttggaagggggggggggggtgggggagttgatttgttaaaataacccttactctatccaccccgagcaattatcctataactactcttcttttgaccttttgcttgaaattcggaagattagcctgtaatttgagccatgacttttgtcttcctaaaacataaattaatgttgctcaataagcttccttctttttatgctcaatggtccaaagcactgattctagttctttatttcagactcaacattgtgttgacttcctcattcttgatatcagtttcatctgttcacattttgcattgtaacaatttcataattttgctgtaggtgtacttgggtgagcaatttgtaaacaatcctacgttgtccgatgtgacatttgttgttgaaggtatacatttgtttccactttgatttgaaattattgctccttttttgtgtttcttaatgacacgagcatactattctttcttaacgttgtcaggtaaacaattttatgctcacagaatttgtttgcttgcttcgtcggatgctttccgtgcaatgtttgatggcggttacaaggtgagcattgacttattttagagctatcttgtttcttgctaaatgcttaactaaaagaagatgaaataaaacagataaatctgcaaaataaaagactgagaatcatgtatgaggattcagtcatagtcagatttctttctgaacattctgcatctactgatctgtgcaatattttgcattctattggctgattgccatgtatcattatgaaatttggatttataacttattgaagctttataaaaatgcattgcaggagaaaaatgcaaaagatgtagagattccaaatatcagatggaatgtttttgagttgatgatgaggtctgagctttgcattctcccttaaaagatgaatgattaagcaaatatcccctgttgatattttatagtattttggatgtttgtagattcatatatacaggaaatgtcgatgtcagtgtagatattgctcaagatcttctgagggctgcagaccagtatcttttagaaggtcttaaacgactctgcgagtattccattgcacaggttggctaaatgttgagtttgatttgtgtttttaacagcattatagtattcttaatatttagtctaatgatttattttctctccttagattatttctgttgaaaacattatgctcatgtacgagttatcagaggcctacaatgctacgacattaaagcaatcatgcatactgtttatattggagaaatttgacaaaatgagaaacaaaccatggtatgctacctccttccaccttgattgtccatttttcaagctgctttgaacaattaatttcaatattcttggtgtataaatttctggccgttcttttaattagattttgggtttaaggagggaaatttatcttaactacctatgacaatcgtggtaataaatcatgctagaaaatttgctttcacattttttcaggactttgaatctttgtggtagtctgaaaaattgttatttctgcaatggctttgaagtgaaattattatctgaatcccatattcagtgggatttcctagaacatttgaatgatattaaacactgccaatgtctctagtctttcctgtgccattttagtttcgtgtagtcagtggtatatatgtttggaccctaactgaatttgagaaattctaattcaactatttgacaacacgcaggttctttcgtttgatccgttgtgtgttaccagagatacgaaattacttcacaaaagcattttcgaatcctgtcattgtgaattcaagccagttgtgaatgtaaatgatttagctttaattttgatattgaaacagaatagtagatgaagaccaagaatgtaaatagagcttgggttattgttgttgagctagtggaggaaattttgctgattcctcgtgttaggtgtaagaagacttggcgacttctcagataatgtaaatccca

SEQ ID NO: 238 - DNA, 7445 bp, Citrus sinensis
  source 1..7445: mol_type = genomic DNA
cttcgccttctctctcagtgctttgtccctgatttgatggatccacagagacgccaagggccgagcgtccccgagaggaaggggcaaaagcggaaactagatgaagaaacagtgatcggagacgagcagcagcagatgcaacaacgagagatctcgtcttcttctgctggaacttcttcatccgatgcgcggcaagcgctattgagcgaggtcagtgctcaggttaacgtccttaacaccactttctcttggctcgaagccgatcgcgctgcggctaaacgcgccactcacgtcctcgccgagctcgccaagaacggtccgtaccttccaaaactgcctctcgatctcgagttatttacgcctctgtcactggttttttaatgcgaaggtctgtatttgtggttgcagaggaggttgtgaactggattgtcgaaggtggcgcggttcctgctcttgtgaagcatctacaggcgccgccgacgagtgaagctgaccggaatttgaagccttttgagcatgaagtcgagaaaggaagcgcttttgctcttggacttcttgctgtaaaggttgttttagcaattattctatttgcttagttaagcttggcttggagtctcattttattgatagtgattattttactcatgcatgttattattattttgaattgttctaattttactctttctggaaatagctataataataagctgctattggtttcattttagaataattagactaaatcccacagtatgcatgctatgatagttgttttgtcgcgattactataataattggtaaggctatatatttttggtgaaactaagaaatgtaaacaattcttggaaggcaagtgaagattagatgttaagcactacaaactattataatgtcgaaagtggtgtgctttatggttgtaagtttatgttaggattgaatggctgtattgaattattttactttagattttaaaggatttataatttaaagaatttacaatgttattgaatgggactaataaaagaaatttagaaacgccacctaaagaaatgaacaggatttcttttgagattcttatgacatgcttaatttttttttctctcccttttttttcaagaaattattttatccaagattcatcaccttgttcttgaaactatgtcctaaatagattttttatcaatgttctagcattaagaagttgtttttgaaatttcaagggaaagtagaaaggtactattttgctggcatttatttttcttgattccaataagtcttagttgtatagcattgtcaattttattgttattgtttctgttgcatgactaataacaattcttgctatacttgcaaataaaatggcattgaagcatttaaaactgtaaaatagatattctattatgtatgagtactgaacctgtgaattttttatggattttgttggtaacagccagagcatcagcaactcatagttgataatggtgcattgtcacatcttgtgaatttgctgaagaggcacatggacagtaattgttcccgtgccgtgaatagtgttattagaagagcagctgatgctatcaccaaccttgctcacgagaacagcagcatcaaaacccgtgtcaggtctcatgatttttgtaactttttattttgagtcaggcatttaccaattagtgccatgtttatctcattgttatcctgttctggatatgcaggatggaaggtgggattccacctctggttgagttgcttgaatttactgacacaaaagtgcaaagagcagctgctggtgccctgcgaactttggcatttaaaaacgatgaaaataagaatcaggtaacaaacaatttgttggaagctgcatattgttaagctggcattggtatctacaaattatgaaattactatgtttttgcagattgttgaatgtaatgctcttcctaccctcattcttatgctacgatctgaagattctgctatacattatgaagcggtaggattttatcagagtgggttttctattagtttctgaaaattgtgcaagtgcaatattttatgcttttatttctctttggctatcaaatgaagttaattttcatgaattccaggttggagtaattgggaatctggtacattcatcccccaacataaagaaagaagttcttgctgctggggcattgcaacctgtcattggactacttaggtatgcataaattttgtttcttttacaacatttgtgatgttctgcctggtttaggtgttttggagaggttttcgcccttcttctgctattgctttagatattacggtttttaaccttagtagaacagcttagctctttttttctcaattcattgggtttgttaattggatgacagttcgtgctgctccgagagccagagggaggcagctttgttacttggacagtttgctgcaactgattcagattgcaaggtgggcacaacttgtcattgtctttatcttatttttccttgataaagtttattcttctcccaggttttctgcttggccgtgcaagatatgaggaatgaattgaaaatgaattttttaagtggaaatgtaaaataaattttgtttcctctgactatccttttagtagaagtattggtgttggttcacttgttgtcatcatgtgcttttagccttctcatccttgtacaattttccatcagacttgtctctccttttatttattttaatatatatgcaggtacacattgtacagaggggtgctgtgcggccactaattgaaatgcttcaatcacctgatgtgcaactgagggaaatgtcagcctttgccttggggaggttggcacaggttatcacggtttcagtcttacctgctatccttatctttatcataattaatgaatgtcaactagaagttttggcttttgtgctttctgagatggtgctgctcttttgtagatagtgctatgatttgtatggtagattacatgtactttcattttcttgtaggaactagaaattaattcacagtttccctcaagcttttgtcaagttctattggtttttaatagtgcggttatgctatggtcatctttggtatccaaatacttcttcagaggtttttttctcttgcatatttgtttttgtactggtcatctttttatgctcaatatttatgcgtgcatgtttgtaaatgtttatgccatggtgctggttgtcaaactcttccccaccccccccccaaaaaaaaaaaacaaaanaaagaagnanaatatactattntttnntttgttttntntgcncaataaattagtntntaanaanattatttnttntatatntttcttactagtagatnnnnnnnnnnnnnnnnnnnnnnnnnnnnnnnnnnnnnnnnnnnnnnnnnnnnnnnnnnnnnnnnnnnnnnnnnnnnnnnnnnnnnnnnnnnnnnnnnnnnnnnnnnnnnnnnnnnnnnnnnnnnnnnnnnnnnnnnnnggttgtcaaatttttccccaccaccccccccccccccccaaaaaaaaagtgcaaataatattacatttttgtcagttttttgttctagtgccagaaaattaagttagcttgaaaatagaatttctttgcttaaatgtatttttccaatttaggacatgcacaaccaggctggtattgcacataatggtggtttagtgccattgctgaagcttcttgattcaaaaaatggttctctgcaacataatgcagcatttgctctatatggtctcgcagataatgaggtacattgtattcttttgaattcttatgaatattagaactgaaaaatttgagtttttatttcaagaagttattaacatactttgttggactcttctctcataggataatgtagctgattttattagggtaggaggtgtgcagaagcttcaggatggagaatttattgttcaggtatgctcaacaatttttcaaattagctgttatttctacaatttgtattaacttttatgactatatggttgcttaccattgttcatactcatgaatcggagactgagattcttgttagttcattttaaccttggacctacaatcaccagtatagagaattgtacttgcaggcaacaaaagattgtgtggcaaagacattgaaaagattggaagagaagattcatggacgggtgagtattttgatccctatcttcgaagtattcagccgacatggactacttctaattttatgtttggatttttattctgtgatctcatgattttcttgatacaggttttgaaccatttgttatatctgatgcgtgtagcagagaagggtgtccaaagacgtgttgctttggctcttgctcatctgtgttcccctgacgatcagagaactatatttatcgatggtggtggtatgttgcattaccagatatactttttggtaattctaggttcatgttgccatgcatttgttctgatttagctggtgcaaagtcacggttgagatgttcatattggtgtgaatggtgctataactattcaatttcatgcaggattggagttacttcttgggcttctgggttcaacaaacccaaagcagcaacttgatggtgctgtggctttgttcaagttggcaaacaaagcaacaactctttcttctgttgatgcagctcccccatctccaacccctcaggtgaggtttaagaatggttttttacataccttgtcttatgatgaaaatgtaaaatagaagtgaagagttctctgatgtggggcaacttctatttgttatttattaggctttatgtatgttgaggaactcaaatgattcaagaaaagaaaacacaggaatcatttaaaagctttttacaatggcaactgagtcaaagctagtaatctcattatcttctatcaaacctattaaagaaataaccaaagctcaactggatacaaagaaaaattcttagaatgaaactgcgttagaaacaatcaaattagattatctttcaatgtttataattgctgagagtttggtgcctatgatgacagtcagtgcttggtgcaggtctatttaggggaccagtttgtaaacaatgctacgttgtcagacgttacctttctagttgaaggtttaaatttactttcttaataacatgagttcttgcttaattctgctgcatatgttggaatgacttcctaaatcatttttttccatagacgtttcgttagcacaagttctctttttgaattataaaattgcctcctttactgcaggaagacgtttctatgcccaccgaatttgtctacttgcatcttcagatgcattccgtgcaatgtttgatggtggttaccgggtgagtgtctatgtctactatcttggtccccaacccccactcttcaatcatcttatcttctgtatttgcgtgtgtagggtggggctgttgtactagagtttaaaaaaatttggctatgggagtgctgcactgtcaaaatctttgactttgtggctgaagtataacatttctttggattatacgaaatttaagctcaaacttatctgtttttttttaaaaaaataaaacattgattgcagattcattttctggttactcaaaagcataatcatctggtgctcttatctttcaatgcaaattgaagcactcgaaagcatagatgcttttaagatatgcattgaaagtatagctgcttttaagacatgcatattgtgactaacttacggtggattttattgtaggaaaaggatgctagggacattgaaattccaaacattagatgggaagtgtttgagttgatgatgaggtttgatgaattctgtgcctttaacttgagctctttataattgctttcccttgaacatctgggattactggtttattctgctgcagatttatctacactggatctgttgatgttacattggatattgcacaagatctccttagagcggctgatcagtatctcttggagggacttaagcgactctgtgaatataccattgcacaggtgagcttataaggccttttttttttataaatttttaatccctcaatgctgcttgtaaattgaaagtagttttctaatcaaatattctgttttcgttgtaggatatatctttggaaaatgtttctagcatgtacgaactttcagaagcttttcatgctatatcattgaggcacacatgcatcttgtatatcatggagcactttgataaattgagtactaggcccgggtatgtgatcccactatcctgctatgttcctcatctttcttctttgactctgttaacttggaactttagtgatttggtaagttaagtagagttggaccaagtcctaaggtaggtgcccaattaaaatttatttgttatgccacagaaaattataatgagctggacggttttaagatagttattctcttcaatgcattgtgccatggcaattattttattttattattttgtcttaccgaggaaaaggggtttttgtagaatgctaagtatgttcactatttaatgaccaatctcttaggatcacttgtatgcttgacagtgattaccttttacaggtagaagatattgatgttgcattttgaggtctatatatgtggcctgtatgcataatctcagttgcttataattccttttactgatgtcacatagaagtatagcaacataaaattaattgtcttaatccttcacatgggattttgtcttgttaaggtttttaagctctggggaaatgataagagaggaatagcttgaatcattgaaatgagcgatataaagcagcaaaatatatgattgccaaagtgaccatgtgctctttgcaaatcatatttgttaatggaaagtttgcttcagcatttaaagttgatattggttgtctctcctgccatcttcttttgtttttctttgttcaaattctgcaatagttattttcctgtagaaaacgggagtagatttttgtgtccacgtgaactttcctgctgctataaacatcttacaatcatttgctgaaaccatctgcttgttgaaaacttgcaggcattctaatctgatccagcgtatcattccagagatccacaattactttgcaaaagctctcaccaaacctaacccacataattcgcggctgtagatggccagtcattgattcttgatcgctaactagttatgatgtacagaaaatagtagatcttttcactgatatcaagtcaagtgaagctcctaattggttgattgtagtgtggctcataatcatttccggatgccagagttatgttggttgtagactgtaagttgcttcttcaagttaattgttgtaggtactgcttgaaatataaccttcacaaaacattattgattttcatggattgtgatggttgtatgtctcgaaatgtattttatgactattcactgaaattgaattcgttgagat

SEQ ID NO: 239 - protein, 704 aa, Citrus sinensis; identical to SEQ ID NO: 236

SEQ ID NO: 240 - protein, 717 aa, Citrus sinensis; identical to SEQ ID NO: 235

SEQ ID NO: 241 - protein, 720 aa, Citrus sinensis
MDPQRRQGPSVPERKGQKRKLDEETVIGDEQQQMQQREISSSSAGTSSSDARQALLSEVSAQVNVLNTTFSWLEADRAAAKRATHVLAELAKNEEVVNWIVEGGAVPALVKHLQAPPTSEADRNLKPFEHEVEKGSAFALGLLAVKPEHQQLIVDNGALSHLVNLLKRHMDSNCSRAVNSVIRRAADAITNLAHENSSIKTRVRMEGGIPPLVELLEFTDTKVQRAAAGALRTLAFKNDENKNQIVECNALPTLILMLRSEDSAIHYEAVGVIGNLVHSSPNIKKEVLAAGALQPVIGLLSSCCSESQREAALLLGQFAATDSDCKVHIVQRGAVRPLIEMLQSPDVQLREMSAFALGRLAQVITDMHNQAGIAHNGGLVPLLKLLDSKNGSLQHNAAFALYGLADNEDNVADFIRVGGVQKLQDGEFIVQATKDCVAKTLKRLEEKIHGRVLNHLLYLMRVAEKGVQRRVALALAHLCSPDDQRTIFIDGGGLELLLGLLGSTNPKQQLDGAVALFKLANKATTLSSVDAAPPSPTPQVYLGDQFVNNATLSDVTFLVEGRRFYAHRICLLASSDAFRAMFDGGYREKDARDIEIPNIRWEVFELMMRFIYTGSVDVTLDIAQDLLRAADQYLLEGLKRLCEYTIAQDISLENVSSMYELSEAFHAISLRHTCILYIMEHFDKLSTRPGHSNLIQRIIPEIHNYFAKALTKPNPHNSRL

SEQ ID NO: 242 - protein, 712 aa, Citrus sinensis
MDPQRRQGPSVPERKGQKRKLDEETVIGDEQQQMQQREISSSSAGTSSSDARQALLSEVSAQVNVLNTTFSWLEADRAAAKRATHVLAELAKNEEVVNWIVEGGAVPALVKHLQAPPTSEADRNLKPFEHEVEKGSAFALGLLAVKPEHQQLIVDNGALSHLVNLLKRHMDSNCSRAVNSVIRRAADAITNLAHENSSIKTRVRMEGGIPPLVELLEFTDTKVQRAAAGALRTLAFKNDENKNQIVECNALPTLILMLRSEDSAIHYEAVGVIGNLVHSSPNIKKEVLAAGALQPVIGLLSSCCSESQREAALLLGQFAATDSDCKVHIVQRGAVRPLIEMLQSPDVQLREMSAFALGRLAQAGIAHNGGLVPLLKLLDSKNGSLQHNAAFALYGLADNEDNVADFIRVGGVQKLQDGEFIVQATKDCVAKTLKRLEEKIHGRVLNHLLYLMRVAEKGVQRRVALALAHLCSPDDQRTIFIDGGGLELLLGLLGSTNPKQQLDGAVALFKLANKATTLSSVDAAPPSPTPQVYLGDQFVNNATLSDVTFLVEGRRFYAHRICLLASSDAFRAMFDGGYREKDARDIEIPNIRWEVFELMMRFIYTGSVDVTLDIAQDLLRAADQYLLEGLKRLCEYTIAQDISLENVSSMYELSEAFHAISLRHTCILYIMEHFDKLSTRPGHSNLIQRIIPEIHNYFAKALTKPNPHNSRL

SEQ ID NO: 243 - protein, 715 aa, Citrus sinensis
MDPQRRQGPSVPERKGQKRKLDEETVIGDEQQQMQQREISSSSAGTSSSDARQALLSEVSAQVNVLNTTFSWLEADRAAAKRATHVLAELAKNEEVVNWIVEGGAVPALVKHLQAPPTSEADRNLKPFEHEVEKGSAFALGLLAVKPEHQQLIVDNGALSHLVNLLKRHMDSNCSRAVNSVIRRAADAITNLAHENSSIKTRVRMEGGIPPLVELLEFTDTKVQRAAAGALRTLAFKNDENKNQIVECNALPTLILMLRSEDSAIHYEAVGVIGNLVHSSPNIKKEVLAAGALQPVIGLLSSCCSESQREAALLLGQFAATDSDCKVHIVQRGAVRPLIEMLQSPDVQLREMSAFALGRLAQVITAGIAHNGGLVPLLKLLDSKNGSLQHNAAFALYGLADNEDNVADFIRVGGVQKLQDGEFIVQATKDCVAKTLKRLEEKIHGRVLNHLLYLMRVAEKGVQRRVALALAHLCSPDDQRTIFIDGGGLELLLGLLGSTNPKQQLDGAVALFKLANKATTLSSVDAAPPSPTPQVYLGDQFVNNATLSDVTFLVEGRRFYAHRICLLASSDAFRAMFDGGYREKDARDIEIPNIRWEVFELMMRFIYTGSVDVTLDIAQDLLRAADQYLLEGLKRLCEYTIAQDISLENVSSMYELSEAFHAISLRHTCILYIMEHFDKLSTRPGHSNLIQRIIPEIHNYFAKALTKPNPHNSRL

SEQ ID NO: 244 - DNA, 18405 bp, Miscanthus sinensis
  source 1..18405: mol_type = genomic DNA
tcatttctacatttctgtcgaacaggtccctaccgcgccggaatcgcactgcttgtgccttttcctcctccacaatccgtcacgccctgcgcgccgccgtcgacctatcgaatggaggcggagcagcaaaagcagcagccccagcgcccgcgccgcaaggggcagaagcggaagttggaggacgaggcatccgccgccgccgccgccaccgcgtcctcgctcggcagcgcgggcgccgacgatgacaacgaggaggaggacggctcggcgggcacccccgagatctgctgccgccactcccacgcagcgcttgcccgcgaggtccgcgcgcaggttgatgtcctcgtccgctgcgcctcttcgtggcgccacgccgaccgcgccgccgccaagcgcgccacccacgtcctcgctgagctcgccaaaaacggtaacctcccttcgccaaacctcactccggccgcgccgatccgtgcacccgcatccttaccgagtggatctggtggttgtcaattgagcagaggaggttgtcaacgtgattgtagagggcggcgccgtggcggccttggtgtgccacctagaagagcctgctgtggcggcgccaacgcaggaggaacaacaactgcggccgtttgagcatgaggttgagaagggcgctgccttcgctctgggcctcctagctgtaaaggttccttcattaattccctaattgagttgtagatgcacttttggtaccaatgcaattacttgtattatcgacgaatttatgttctaaatagggctgtgaattttcaagtttcctgtggcataggattacaaactttaagaacttaaactatcccatgtatatatatactgtaattctgaaggcccaaacctcatcctcatatatctgtatttcttgtaaaaaactgtaagatcccatgccttttaatagttagaaaaacctaggaacttccaagtgctatatacttggtgtctttctagtcattctcaccctttagaaaaacttaggaacctaatatatcataatcgctctagttctgtagggatcttttaatatttgtgttttgagcaattgatgctttactcttatgtacttttcatcaagttattattgctatggtcaatttaatcatttattctgtgttcactgtaacagcctgaacatcaacaacttatagttgatgctggtgcactacctcctctagtgaaactcttgaaaaggcagaaaaatactacaaattcgagggtggttaatagcgttatcaagagagcagctgatgcaattacaaatcttgcacatgagaatagcaacatcaaaactagcgtcaggttttgttttatgcctctttgatcatttgataacgttttccttgagaagttttcacttgctgagggttttgttttactgcagaatggaaggtggaatcccaccacttgttaaattgctagaatcgcaggatcttaaggtgcagagggcagctgcaggtgccttgcggactttagcctttaaaaatgatgaaaataaaactcaggtgagatatcaaaatcaatgaaggctataattatgttagattttgacatctgaacttgcatatgccttttacacatattcacgacatggtaaattcctgtaatgcagattgttcaatgcaatgctttgccaactttgatcttaatgctgcgatctgaagatgctgcaattcactatgaagcagtaaggccttatgctattctccagttttgattatgaggcactgaatattctgatgtcaactccacttctctaagagcactttctcacactgttgagatgtatcgtttgattgattatgagcaagttaatgttgttacagataaatgatcatatcatttgaaattgtgccattctacaattttgcacaatccttaatcagcatttatcattgcaaggccttgtgaaatatacaattttaatgctccatcttgaaacttaatgctggatcataacactgtatatttagcgttaaatctcatgctagaccatgtttcatcctcgattacatggacaattttgaattttgaatgtatttccaaagttgaaaatgagcctaccccaacttgcttgggactgaaaggctatgttgttgttgttgttgtatttccaaagttgaaaatagaaacttaattttgttggctgttagcagttaccttacagatattatgttgtcctacaacacatttatatcataggctttgcataatttattcaatatttcctgccatgtaagatgcagtttgattaatattttctgatcccattgatgaaattatattaatctggattcatgattaccctgaagttgtgcactgatattgatctattgcatataaccaaccttagtgaaaccactagcagtgcgtttggcaactattgggaaggggcatgggaattggtggtgggagttgtagcgaattacgagaatttgatttttaggtccaatcacttgtttggttcattgagggaaataagacacggaaagagtgtgtgcgtgtgtgtgtgtgtgtgtttctgtgagaaagggaagtgattggtaggagttagccctgtaaactcactttcccgtcccactaaacaaacaaaagatttctaaactcttaccccccaaactcccattcccttttaccaattacccccaaccaaacgtgccatagaggttattgaattgactaaggtaaatatcttgaacgcactttctgttttctttttgtcaactggcgatagaccttaatggctgtattaagctagttcgggcgatctttgaggctgaaattgaagatttgaaaacttagcaatacacccaaataagtttgagggccagtggtgcagccgtgcagttaagcctgtatcatggtgcatgtacatggatgcttgaagaattaaatgtttatttgaatgcataaatgtgcggcaagtactgagacaacactagaggctgaggctatttactacttggttcctgaaatatttcaaaaagtaatctgcacctgctacttgtaacaggtttgctaagtaaacttgattgtagaagcttatgcaaaacaaataaattgcatgaaattggtccgacgctctgagttacctccttatattgacttgctgttctatgctcttttatccgttgaataaacttctacatggtgcaaggttacctttctgtactaacatccttatcaatccaacatgtttgctgataaactttcatagaatatcagcacaatcttggatctaatctattcacgatttctttaattttattgcaatgcactctaaccatttttctcgactgacatgttaggttggtgtcattggaaatttggttcattcatcaccaaacatcaagaaggaggttcttaatgcaggggcactgcaacctgtgattggattattaaggtatggtcatcatagggaagtgcagctttatgaggtgcataaagaactttataattgtatatatttgttaggttctgctccaatactgctagcatagttgtgcattatcactagcaaatacgtctgtgcgttgcaacgggaaaaagagtttttgtataaaaggggagaaaagagtaaggtccttagcagaaatgcccgcgcgttgctatggaaaatactaatcctttacatgagaaagggggaccaaaatagatgtatacctccaaagtagaatagttattgcaaaggtactccttccattccaaaggaatggatgtcgacatgcagtgcaacatggtgttctaagaagtaagaactcaagctggtatgggcccaacctagtgttctaaggactaaaacattaagttttctgggattatttttgaatcctaaaacatcacgtgttctgaaacggagggagtaagatggaaaaaagataaataaatttctcaaaaagttggtctgcttcaaggacatcaggtgagatcagagttaaattctcatccatgattgatgattccttctggctccgtagctgtgggtaagtttttagtgcaagttgagtgaatgtcttggtaacaatcaacactgccgagtttctctacatgtgaatgtacagaatacagtctgatattggtaaggagctagctccttcgattttcatctgttagtagagacatcaagagtttccatgcacctacgctggacctacttctaaaatctaggaaacatgccccttctaaaatataggatatatggatcatctaggatacatggccctccctttttaaaatatagaacatatggaccattggccgctcttttttctctgaagctaaaaactgttcagttagtgtgggttagatggacttccttgtacattagttagtcgttatgttatgtggggccgacaattccaagccactccagggctcaagatgctgccaggagcgcagcaatagaggtgcatgcagctgtgatcaatagcaattagggcctgtttggttcccattgactaaaatttagctactaaaactagtgactaaactttagtcacccctgtttggttctagtgactaaaagtgactaaaggctattgaaacagttcaacaaaggccaaactacccctaatgaatgcatgcccaaatcagggtgggggaccagcaataatgaggggcagcccttgtccactaggcactttagcccacttttagctactcttgggtgactaatgtgactaaactactttagtccctttttagtcaatttgtttggcagtttagtagctaaagtgactaaagtttagtagctaaactttagtagggggtaaccaaacaggcccttagtagatgattggggattagtagttattgctgcagcaatagaggcgcatgcagctgccagaagcacagcagtaagagcatgcggctgtaatcaatgagaattagtagtatggttgagatattagagttaatggtggggagagaaacgaggagctagaggctgggcgcctagaggctgggcagctctatttatacccctgtaatcagcttatgatgaatcaagcaatgaacaacaaacaatccagttaccccaaatattctagtctccctccacgccgactttgcctggccttcctcttggcaatggttatcctccctatccccgatatgaactaaggttcataccatgttaaactgttgcatgcccaaacaaccagaagagagttccatattgtttctcaggcatgggagttgcttgtgggttgattcaactcaattagcattgatatgatgtctggttgattgagcaacacacatttattgaggccaataaacacacatttattgaggccaatgttcaataattgaataagatgtgaatctgaagaaacacagatagaaaaggagaagaattgcagacctcgccatcaggttccgtgggagtgggttagcagctcggttgtgctgcccacgactagatctcaacaccactcgttgatcgcggaggaagccaaacctctaaaagccatggactccatgacccatgggcctccaccacgacgtgccggatgcctggatccggtatcccaggttggagggggaggatggagcttccaatactgcgctgtcgcaaggaaggcgaggggcatgctaagaagctctacgcttggccgtggagccggtgccgtcttctcacaggtgttctccagatctccacccatggggcagtcatgcttcatgtccgtcgtgtgggccaacggccgtgtcgaaggcggtgtagcatgcaggcaggcggaggtgtgagccaagggcggggtcttggacagttggacaaaagtcagggtgcagcattggacgagacgggggaacatacgttcacgcggagggaccgctggtgaggcgatgaatgtatgaatgggcttggctgacggacaaaatcccgaggagataaacttttgctctttaatactcccactgtccaaaaagaatgtaattctctgttccctaggagtcaaacaatgtaaagtttgaccaaatctatactaaaaaaatactaacatttatgatacaaaatatgtatcgttagattaactataaaatatatttttatagtaaacctaaatggaaacataaatgttgatacattttctttaaacttagttaaacttaagaaagtttgatctgtttcaaatctataatatacattctttttgggacggaaggagtattaggtatagatatatactgcatgctctgttgagcatgccttacaaatgttctattagagcatctccaacagattacttatcctgcatcccctaaaagtctatataggtgatctattatgtattattagtagtttagctctttcttctcctctcccaacagattaccaatacttttaaagtggataggggagagggagtggatagggattttaagtagttacttaaaacttcaatcccttatattgcatatttttagtatcagggatgagataagtaatctgttggagatgctctaattttgaggacaccagtgtacatgaagctttaatgattaagccaaccaaaacaatgctaattattatgttcgagtgtaggctaggccattcctagtcctcctattcagatccttgtcatttttatattatttctagagaaacacttgaccatggctttgtcttaaagagggggagtattgaacaccggttgtccaaaaactcgctgaaaccggttcagtgaggtatctacatttggcgagggactggaattttgggtgggcggccttcttgttgggaaactgtaccagccaagctactggctcctttctcatcttgtattctagaataccatcttattcaaatgagaaggttctttgtattcaagttttaaagggtgttctacgatttgctctacactggcaactcacctcaggaatatctgcttgatgtatgaaacattgctttctttatttttttcagctcatgttgtacagaaagccaaagagaggctgctttgttgctagggcaatttgcttcggccgactcggattgcaaggtgcttaacaaatatggaatacttattgtttacaagtcatcagtaaattttgcaaatccactggtaggttagtcaaaactaaagagagaatcgcaccactaatccgtgaatttgcatggttgtctctcgcacacccctcaatttgtaacttacattgtgagcccttctaactttggacccattgtggcatcggcccaaattaccgttggctacttagtttaattgatggtgctgatgtggcaacaaacatgggctattatactggattgtttattttcttttatcgtcgcttccttcccttttcttttccattgatcaatacatcactgacatggatatgtagatgatgccatcaaattgactaattatttgaccagtcaacaaaatattttgttttcgtatgtgtcattatttatggtgtactcaactggtagccgtgtcttcttgtgaacaggcccttattgcagttaggcattatttatgaatgtgactttcaataccatgtatatttggctaatattagactatcaatccccttctttttcaagaagtatttattttgtattattgttccataatttgatggaatttagccacccatgttatttatttgtgatccatgttatttatttgtgattggaatgtatattgcacatgtcttatggttataggccaaaacctgtgtcaacatgccatggagagcaggtcccatgtttaatgctcatgtcaacacaatttgttatgttaaggtgatttgggccaatgttgcaaacagacctgaagtttaggggggctagcaaagtaatttgcatgttgagggaagttggtgagagtgagacaacaacacaactttaagggctagggtgcaattctctctttttcagaagtactggtgatttacatatgtaacatttatgtgcactgtatgttgggatagaagtgaaataagtagtaaaccccatttctggccatgcacatcaggtgcgacagattctcattgctgggaccgtctggcgccttttgacatgctgctggccagtccatgcatgacctcacttattctccttgttgctcttttctaactatgcctctgcatctcttattcttggtctgatctgggtgccacacaatcacgaatccagattggtgtgccatatggcagcctctgctactgccctatccggtgctggcacacttatcttccttatctagtccatcctcacaaggagtcatggacatgttctgcaaatatggtgggctcatgtttccagtgtctgcacgtgccaagtccccagctctgcccttacctgcattgcgtcttcatcactgtgcttggcaacaacacaccctgtgttctatgctcaagctgaacctagctcggctaccacgcatttcaattgctccaccactcctggcttacaccacaccctaagccctcccctaccaataaatcattggatataaaatttaagtttttgtagaagttagtttctttgttgcagaggtaggttttactttatttttttagatgtttccttgggagatgggagagaggacagccattgggaccacttgtcgtctgttctttgagtggagagatgcagaaggtagaaaaagaatgaactcaacaattgaatataatgttcagtataaggaaatctagaatgataaatcttattatctaaggaatgacacaaaagcaaagagatataagatgttttcttcagttaattcgtttctgaacttgatagattaatatatatgtttgtttacaggtccatattgtgcaaaggggtgcagtccgtccactaattgaaatgctacagtcagttgatgtccaactccgggagatgtctgcttttgcacttggcaggcttgcccaggtttactttttatttttaatatagcatattttttaatgtttataaggtactttactgttttcttgctctcttacaaaatccacacaatgtatgactttatcaaaattagttcccttgctcctctgttgatgggaactatatgtggggactggggatgcaaagatcataatatgtttagggcaaaaccatattgagtttgctggcaccacataccttccttatccagttcatcctagacatggacagattttccaaatatgcgggcttcatgttactggtgtctgcatgtgccaagtcccttgctctgcccttatctgcattgcatcttcaccactgtgattatcaacaacacacccagggtgctgctgtattcgaggtacctctggtaccacacacattccaattgctccgccaagtaattgaagttatgcagctattctccatatgttggttcaagagcccatatgttggttgcacagaattatgtcttttgtttttgagttaaatgcaccagaggtccattaacttgtgttggggtttgtccatcaactctaaaagttgattttcgaatccataaacttttaaagtggttcaccacaggtccatatcccttcgtttggcccttagattctacttccgtgtccacaaacttttaaagtggttcaccacaggttcatacccccccttcgtttggcccttagatctgatgtggtatgcagccagcatggcatgaaatttgctgagcccatgcttatcctccacctgtgctggtctcctttccgctccctcaagcctggcatctgtgcctttgttctatctctgctccagtgctcgccaccaccattaccggtcaccgagctcccactaccgtgcctggcatctgtgcctctgctgtatctctgctccagtgcttgtcaccaccattaccggtcaccgagttcctgctacggccgctgttccttgccttgtgcttcagctctgtcctagaaatgagctctactgagtccatctctgcctcctctaccctttgcgctcgttgaacgcacagacaccgtgtcggagctcctagcccaccgtactgcagctgtcctgccatggtctgctcacttgcgctaccattcttgtcggtataggacatcaccgcttcaatgagtgtgcggttgagtccgctgtggtcccatcgtcctagtgcgcacgcatttagggcaagtctatgccggacccaccatctaccttctacctgccgtcgaccgctggattggcacgcccgtggccgacctgctactggcctccatcggacaaattaaaaccaccctcgggtgcgctggtagctcgtggtcccatccattgccgccgccgagtgctcccttggccgaatcggcccctccacgccatacttgtgcctatgttgatttggggaagaaagaagaggaaggagatgattcatgggacacatgtgccgtcgtgtctctgccatgcgcccctgtggccctatgtcgcgtcaccgggccttcgtcgcgtgccaccgccctctatgctcgtgccgcttaccggcacttgcgctcactgctgcacactgccgctcagggaatagagcaaggagaagggagggaggaggggctaattgcaaatttcatgccatgctggctgctgactccacatgccacatcagatctatgggccaaacgaaggggtatggacctacgatgaaccacttataaagtttatggacccagaaatcaacttttagagttgatggcctaacagaaacccccgcataagttaatggagtgcatctaactctgttttttttgtaagggaattatgtcttttggtttttgctccaccatatgctctgaccactaaccattcatatcttagcaaaacttttgaacatttgtaattcctaggttacgccatcctggcttgatccctagcttagttatcctagcccaatgatgggtgcttggagcattccctgtgactttggccctagctaatcgtcaattaggtgctaggagctggtctgctgtctgactatcactttgtcagtggtacattctagcagagcgataatatttctgacaattgcaaccaaccaaacttcgtagcatatattttccttgtgagattgtttggctagttttatacagagtgcaacgtggagtgaaccagttaaaaagttgacccagatcctcacttgagagattatggacccagttgagtatctgggaaaagtttaactatctaacgcattttcgataatgtaaggggaaatccccattcatcttttcctttcacttatgggttagtggggttgtttcttttgcttagttgcaactcgtaatctaatctaaagagtcttttatcaggacacacataaccaagcaggtattgcatataacggtggcttggtgcctttgttaaaacttcttgactcaaaaaatggatctctgcaacataatgctgcatttgccctttatggggttgcagataatgaggtaatttacgatctttttttttttcacaaggtttgccatctctctcaaatatcccttttccactattggttaataattccacactccatgttcctttctaatgggattaactcattttttataaaatgtttatcttatatttcttatcttcattatttctgaagcaaatcactgttctttcttataggactatgtatctgacttcattaaagtaggaggtgctcaaaagttgcaagatggagaatttattgtccaggtacattggccttcattgtatattggtcactttgttgtgaatgcttgttattaagctattcttaatttcaggcaacaaaggactgtgtggcaaaaacattgaagaggttagaggagaagataaatggacgagtaagttctgcttgcaaggtttctgtatttcattgtttgcgatgtgcttgactatagtatttatgaagtttgttcccatgtgatggtttacaggtgttgaaacacttgctttatttgatgcgagtaggagagaaatctgtgcaaaggcgtgttgctctggctcttgcacacctttgtgcccctgaagatcaaagaacaatttttattgataataatggtaaacaattttgcaaccactgaaaaattgtaccttttcatttccattctactgtatggtgttcttcatgaatttaaattatgggtcatccaggtctcgacttgcttcttgatcttctgatttccatgagctcaaaacatcaacaagatggctcagcagcattatacaaattggccaacaaagctgcagcactttctcccatggatgctgcccctccatccccaacacctcaggtatgcaaaagaattattaaatttaaatttactttgtattacgcaggtctggtgcagtggtgaaagctgtctcattgagtcaccatgtcgtgggttcgaagcagcctctccgcagatttgcgggaggaaggcttgcctcggtttttcccttacccagaccccactcatgtgggagcctctgacactgggtctgcccttacgtatgctgtttgagttgcagtgactttatgagctgactgtggtatggttaaaaatagtatcacaatggcatgatcttcagtgtgctaggatgcacatgaatttattttgattcatcattgtggaatggtgctttggttcaacaaggtatataagggcccaaacgagtcttgtagtccaacctgttgtgaatgatagtgtgtacaacctgctggaggaaaataaatgttcctctggcatgccatgaaaggtaaatgttggactgctgatcagcttgcaaaacatggtctgtctcatccggataaatgcctactctgtgatcaagaggaggaaacagtccagcacatccttacaacctgtgtctttgcaagacagttttggcataggttcattcttcattgcacttaacttgcagcagcttttgcctagcattactaaacatagtttcactacttggtggcggagagctagcaaaagagttagcaaagatcaaagaaaaggggttaacaccctcatcatcttgggtccctggatgccctggaagcagaggaatgcgtgtgtttgagggagactctccagtgtccctactacacctagaaacctgaagttagaagctcatctctggacgcttgctggggcttccaagctacaggtcttgggctaagtcagttagaaatctaggctagcttagttttctttgttgtaaccccccttaccttggtcctagtaagaggggtgcttgtatgtaccatttcttttccctataatacaaagatacgcagctctcctgcatgttcgataaaaaaatatcatgtcaatatttttatagtgcttggcattgtcttaaaaattgtggtcagaatttagctatcattggcatttttaacaagatttccaaacactgcctgtattttgctatcctaaataaagtcattgtgacattgtgggatttttccatccaattgttccggtaatggctgaggcactggcaattgttacaacaacaacaacaacatagcctttcagtcctaagcaagttggggtaggctagagttgaaacccaccaagagcctcaagtcacggttcaggcacttcaatagctgctttccaagtactcttattcaaacatagatatctaggtatatctcaagctttcaaatatctttttattgcctccccctatgtcaatttcggtcttcctctacctctcctcatattattagcttggcttaagactccacaatgcactggtgcctctggaggcctcctttggatatggccaaaccacctcaaccgatgttggacaagcttttcttcaattggtgctacctctaggcgatcacgtatatcatcgttccgaacttggtccattcttgtgcgaccgcaaatctatcgcaacatacgcatttctgcaacactcaactgttgaacatgtcgaatctttgtaggccaacattctgctccatacaacatagccggtctaatcgtcgttttatagaacttgcattttagcttttgtggtatcttgtcacagagaatgccagaagcttgtcgccacttgatccaccctactgtgattctatggctaatgtccgcatcaatatctccatccctctgtagcatcgatcctagataccgaaaggtatccttcttaggcactacttgaccttccaaactcacatctccctcctcctatacaactccgacaaagtcgcatctcatgtattcggttttagttctgctcaatctaaaacctttagactcaagggtctgctgccataactctaatttcctatttactcccgcctggctttcgtccactaacactacatcatcaacgaacaacatacaccaagggatatccccttgtatgttcctggtaacctcatccattaccaaggcaaagagatacgggcttaaggctgacctttgatgaagtccaattttaatcgggaagtaatctatgttaccatcgtttgttcaaacactagtcacaacattgttgtacatgtccttgatgagggtcacgtattttgatgggactttatgtttgtccaaagaccaacacataacatttcttggtatcttgtcataagtcttctcaagtcaatgaaaaccaagtgggggtccttcttctgttctttaaaccgctccataacctgtcttattaagaaaattgcttctgtggttgaccttccgggcatgaaaccaacttggtttgttgatatctgcgtcgttcctcgtaggtgctgctcgatgaccctctcccataacttcgtagtgtggcttatcaacttaattccttgataattagtacaactttggatatctctcttgttcttgtagattggtaccaatatgcttcttctccacttctcaggcatcttgttcgatcgaaagatattggtgaacatcttggttagccatactataactatatccccgagacatctccacaccttgattgggataccatcagggcccatcgctttgccccctttcatctttttcaagacttctttgtcctccgattcttgaatcctccgcacaaagcgtctattagtgtcatcaaatgagtcgtccagctgaatggtggtgttctcgttctcaccattgaacaatttattaaaatactcttgccatctatgtctgatctcatcctccttcaccaagagctgctccctctcatcctttatgcacttgacttggttgaagtctcttgtcttcctatcgcgagccctagccatcctataaatgtccttctctcattcctttgtactcaaacgtcagtagaggtcctcataggcccgcccctttgcctcactcatcgcttgttttgcagtcttctttgccaccttgtacttctttatgttgtttgcacacctgtcatgataaaagcgcttataacactcctttttttccttaatagccttttgcacatcttcattccactaccaagtatctttcgagtcgcatccgctctctttggtcactccaagcacctccgaagcaaccttccgaacgcatgtagccatcttctcccacatgctgtttgcattgccttcatcattccaagggccctcttcaatgaccttttccttaaagacctttgatgcctcaccttctaattttcaccacttcgttctagcaaccctagcttgtttgttcccacgagcttgcatcagaaagcggaagtcagccaccaccagcttgtgttgagcgaccacacattctccaggtttacagtccatgcatgttcgtttatccctccttgtaaggacaaagtcgatttggctagagtactggccgctactaaaggtcactaaatggaactgtctcttacggaagaaagtgttagctatcatcagatcaaaagctatggcgaagtctaagacttcctctccctcctggttcctactaccatatccgaaacccccatgaaccacctcgaaacctgcacttgatgtacctacatggccattaacatcacctcctataaagagcttctcgctactagggacagctctaaccaagcgatctaagtcgtcccagaaaagccgcttagctctctcatcatggcctacttggggcatacgcactaattacgtttaagaccatatcactaatgacaagtttaactaagatgatcctatccccttgccttctcacctccaccacaccatccttgaggcttttatcaatcaaaactcatactccatttttatttgaagttgtccctgtgtactagagcttgaagccggtattgtccacctccttcgccttctgccccttctatttagtctcttggacgcataagatatttacacgtctcctaaccgatgtgtccactaactctcttaacttacctgtaagggaccctacattccagctacttaaacagatcttagttggctcgactagcttccttacccttcgcacccgctgaggtaggtgtgaagacccttgctcattttgcaccacacccggacgccgatgtggcgcgccactaagaatgcgacgacccgatccttgctcacttgacaccgtgtttagatcgcgacacggcgcgtcacgggggtgacgacccggcccttgctcatttaacaccatacccgggttccgacatagcgcgtcgctaagagggttacgccccaacaggattcttttgggtttcatctccattaaagtggctaagtttttacattggctcgccgcgcctaaaccctactcctttaccagggcttgtgacctgctatgctgtgacaccaaaggcactggcaattgttactgaatttatatttcattgcaggtttatcttggtgagcaatacgtgaatagttcaacactttcagacgttactttcttggtagaaggttggtactatttcatgacagtgatttcatcagtaggtactttaaataattcttttctatcgtgtcccagataatcttaatcccttcttctacaggaaagcgcttttatgcacacagaattgctttgcttgcttgttcagatgcatttcgtgcaatgtttgatggcgggtacagggtgagttttgacttgccacaacataatgtgcttttgctggttttagtctgttgatctctttccatagttgatatattgttgctgtatatagtatgttagttttgaacaaaccttgaatctcatgtttaatttaaaggtcattttcttaaccaggaaaaggatgcaagagacattgaaattccaaatatcagatgggaggtctttgaactcatgatgaggttagtaagtcattgacccccccttctcatttggccacagttctcattctgttgatgaatctgcaactatttttcctcttttcttttttatgccactgtatgctggattaaagtctgaaaccctctttggttttgcagatttatctatacagggtcagtgcaggttaccagtgaaattgcacaggatcttcttagagctgctgatcagtatctcttagaaggcctcaaacgcctatgtgaatatactattgcgaaggtgattagaaaagctactctctattccttgtttaaactgcatattagatattaatttgaatgccattatttgccttgtaggatgtgaatctagataacgtatctgacatgtatgacttgtccgaagcctttcacgccgtgtcactgagacatacatgcatcttgtacgttctggaacattttaacaagatctgcaccagagctgggtaccttctcttgctaataacctttgatctgagaccagtacgatttcaagtaactcaaatattaacacgcaatcttggcatgcagttctccacagctgatccagcgtgtcattccagagctccgcaatttcctaaccaaggcactgagttcatcaagaagtccaagtccaagctgacaggaactcacagacttgatttgagtcccaattcattgacaccgacgccgtcatctgaccaaagttgctggagatcctgaacagtaacgtttctggcgctgagcgttcgatggtatctattgtgggtacatggtggccgggtccttcaaattaacatcagcaatgtaacaaacttttctaagatttagtagaggatatgggtaaagagaacctgtgtcttagtcatgcatcggccagcttacactgggatagggctgtagttggatggtcctaattcgtcggtctcagctttgtttctgagtttagtgtttgtttccagttcacagttcagtgtatgcccgcatttgtttaaagtatgaagcttgagcaagttagaaattatcccccgtagtgataaagttgtccgttaatctcctagtgtggaaccaccgattggatttaccgagacaacaatgtaacatcatagatgcaattagatgcatgatatttgctgataaggtttgctcaaagtctgaggcagagccactgatcatcgctggttaatcc

SEQ ID NO: 245 - DNA, 35397 bp, Miscanthus sinensis
  source 1..35397: mol_type = genomic DNA
cctaccgcgccggaatcgcactgcttgtgccttttcctccacaatccgtcacgctctgcgcgccgccgtcgacctatcgaatggaggcggagcagcaaaagcagcagccccagcgcccgcgcccgcgcccgcgccgcaaggggcagaagcggaagttggaggacgaggcatccgccgccgccgccgccgccgccgcggcctcgctcggcagcgcgggcgccgacgatgacaacgaggaggaggacggctcggcgggcacccccgagatctgctgccgccactcccacgcagcgcttgcccgcgaggtccgcgcgcaggttgatgtcctcgtccgctgcgcctcttcgtggcgccacgcggaccgcgccgccgccaagcgcgccacccacgtcctcgctgagctcgccaaaaacggtaacctcccttcgccaaacctcactccggccgcaccgatccgtgcacccgcatccttaccgagtggatctggtggttgtcaattgagcagaggaggttgtcaacgtgattgtagagggcggcgccgtggcggccttggtgtgccacctagaagagcctgctgtggcggcgctaacgcaggaggaacaacaactgcgtccgtttgagcatgaggttgagaagggcgctgccttcgctctgggcctcctagctgtgaaggttccttcattaattccctaattgagttgtagatgcacttttggtaccaatgcaattacttgtattatcgacaaatttatgttctaaatagggctgtgaattttcaagtttcctgtggcataggattacaaagtttaagaacttcaactatcccatgtttatatatactgtaattctgaacgcccaaacctcatcctcatatatctgtatttcttgtaaaaaactgtaagatcccatgccttttaatagttagaaaaacctaggaacttccaagtgctatatacttggtgtctttctagtcagtctcttgtaccctttagaaaaacttaggaacctaagatatcctaatcgctctagttctgtagggaccttttaatagttgtgttttgagcaattgatgctttactcttatgtacttttcatcaagttactattgctatggtcaatttaatcatttattctgtgttcactgtaacagcctgaacatcaacaacttatagttgatgctggtgcactacctcctctagtgaaactcttgaaaaggcagaaaaatactacaaattcgagggtggttaatagtgttatcaagagagcagctgatgcaattacaaatcttgcacatgagaatagcaacatcaaaactagcgtcaggttttgttttatgccttttgatcatttgataacgttttccttgagaagttttcacttgctgaggattttgttttactgcagaatggaaggtggagtcccaccacttgttgaattgctagaatcgcaggatcttaaggtgcagagggcagctgcaggtgccttgcggactttagcctttaaaaatgatgaaaataaaactcaggtgagatatcaaaatcaatgaaggctataattatgttagattttgacatctgaacttgcatatgccttttacacatattcacgacatggtaaattcctgtaatgcagattgttcaatgcaatgctttgccaactttgatcttaatgctgcgatctgaagatgctgcaattcactatgaagcagtaaggccttgtgctattctccagttttgattacgaggcactgaatactctgatgtgaactccacttctctaagagcactttctcacactgttgagatgtatcgtttgattgattatgagcaggttaatgttgttacaaataaatgatcatatcatttgaaattgtgccattctacaattttgcacaatccttaatcagcatttatcattgcaaggccttgtgaaatataaaattttaatgctccatcttgaaacttaatgctggatcataacactgtatatttagttgggaaatttcatggtagactatgtttcatcctctattacatggacaattttgaatgtatttccaaagttgaatagaaacttaattttggctattagcagttaccttacagatattatgttgtcctacaacacatttatatcataggctttgcataatttattcaatatttcctgccatgtaagatgcagtttgattaatattttctgatcccattgatgaaattatattaatttggattcatgattaccctgaagttgtgcactgatattgatctattgcatatagccaaccttagtgaaaccactagcagtgcgtttggcaactattgggaaatggcatgagaattggtggtgggagttgtagcgaattatgagaatttgatttttaggtccaatcgcttgtttggttcattgagggaaataagacacggaaagagggtgtgtggttttttttttctgtgagaaagggaagtgattggtaggagttggccctttaaactcactttcccgtcccaccaaacaaacaaaagatttctaaactcttaccccccaaactcccattcccttgtaccaattacccccaaccaaacgtgccgtagaggttattgaattggctaaggtaaatatcttgaacgcactctctctctctctctctctctctctctctcttgtcaactggctatagaccttaatggctgtattaagctagttcaggcgatctttgaggctgaaattgaagatttgaaaacttagcaatacacccaaataagtttgagggccagtggtgcagccgtgcaggttaagcctgtatcatggtgcatgtacatggatgcttgaagaattaaatgtttatttgaatgcataaatgtgcggcaagcaatgtttttaaggcggtaaggcgaggcgtggcgagtgactaccgccttacgcttaggcgactgaggcgtgaggcaaggcgacgccttacggatttaaaaaaaacataaaacaacagcttagagtagtagatgatgaagaaaaaagaaaaggaaaaaagaaaaagagaggaggaggagtaagaagtgggctggcccagcccaccaggcggcccatgtgcccctccccctcctggcgtggcttatcccaatgggaatcccctccagcgctgctcctcgttctccaccactcgtccgcctctgctcgtctctccgccgctccacttccctctgcggctctgcttccgtccgtggctcctcccctctctccggatgcgctgctctgctcccctccctcgctgctccccttccagatctacagtcgccgccatccccttccagatcgagcagccgatggcgagaaggtggaatcgagcaggcgacggcgaggagacggcgcaattgagcggaatcgacgaggagacggcggatagagaggacccgcatcagaatcgatgaggagacggcggaatcgagggggcatcagcatgtgcataaggcgacaaggtgccgccttacccctaaggcgagcttggatgcctaatcgcgctctctctttcctttttttcgcgcctattctcctgcgttttcccactgtccagagcagaggcttcctcgtatggcgcccgccatgcgcgatttggcgcgatttggacgccaaagcgacgttttttggacgcctcggctgtaaggcggacgccacacgaatctaaggcgagtcgtctgctaaggcgtcgtgcgtgcagcgccttggcgcttaagcgacgccttaaaaacactggcggcaagtactgagacaacactagaggctgaggctatttactacttggttcctgaaatatttcaaaaagtaatctgcacctgctacttgtaacatgtttgctaagtaaacttgattgtagaagcttatgcaaaacaaataaattgcatgaaactggtctgaggctctgagttacctccttatattgacttgctgttctatgctcttttatccgttgaataaacttctacatggtgcaaagttacctttctgtactaacttctttatcaatccaacatgtttgctgataaactttcatagaatatcagcacaatcttggatctaatgtattcatgatttctttaattttattgcaatgaaccatttttctcgattgacatgttaggttggtgtcattggaaatttggttcattcatcaccaaacatcaagaaggaggttcttaatgcaggggcactgcaacctgtgattcgattattaaggtatggtcatcatagggaagtgcagctttattaggtgcataaagaactttataattgtatatatttgttaggttctccaatactgctagcatagttgtgcatgtttttttttaattattatcactagcaaatatgcccgtgcgttgcaacgggaaaaagtttttgtataaaagaggagaaaagagtaaggtccttagcagaaatgcccacgcgttgctatggaaaattctaatcctttatgtgagaaagggggaccaaaatagatgatctccatgtagaataattactgcaaaggtactccttccattccaaaggaatggacatgcaggctgcaacatgatgttctaagaactcaaactggtatgggcccaacctataacattaagtttttctgggattatttttgaatcctaaaacatcacatgttctgaaacggagggagtaagatggaaaaaaggtaaataaatttctcaaaaagttggtctgcttcaaggacatcagatgagatcagagttaaattctcatccatgattgatgattccttctggctccatagctgtgggtaagtttttagtgcaagttgagtgaatggcttggtaacaatcaacactgccgagtttctctacatgtgcatatagagaataccgtctgatattgataaggagctagctccttcgattttcatctgttagccattctaatggagatgaaacccgaaagaaaaccgttggggcgtaaccctcttagcgacgcgtcatatcggaacccgggtatggtgttaaatgagcaagggccgggtcgtcacccccgtgacgcgccgtgtcacgatctgggcacggtgtcaagtgagcaaggattgggtcgtcgcatccttagtggcgcgctacatcggcgcccggatgtagtgaaaaatgagcaagggtcttcacatctgagtcgacgggtgcgaagggtaaggaagctagtcgaaccaactaggatccgtttaggtagttggaatgtaggatcgcttacaggtaagttaagagaattagttgataccgcgactaggaggcgtgtaaatctattatgcgttcaagagactaaatggaagggtcagaaggcgaaggaggtggacaatacaggtttcaacctttggtacacagggatagtcgcgaatagaaatggaggagttttcattgataagagcctcaagaatagtgtggtgggagtgagaaggcaaggagataggattatcttagtcaagcttgtcattggtgatatggtcttgaacgtaattagtacgtataccctccaagtaggcctcgacgagagtgctaagagaattctaggaagacttagatgacctgattagagctgtacctagtagtgagaagctttttataggaggagatnnnnnnnnnnnnnnnnnnnnnnnnnnnnnnnnnnnnnnnnnnnnnnnnnnnnnnnnnnnnnnnnnnnnnnnnnnnnnnnnnnnnnnnnnnnnnnnnnnnnnnnnnnnnnnnnnnnnnnnnnnnnnnnnnnnnnnnnnnnnnnnnnnnnnnnnnnnnnnnnnnnnnnnnnnnnnnnnnnnnnnnnnnnnnnnnnnnnnnnnnnnnnnnnnnnnnnnnnnnnnnnnnnnnnnnnnnnnnnnnnnnnnnnnnnnnnnnnnnnnnnnnnnnnnnnnnnnnnnnnnnnnnnnnnnnnnnnnnnnnnnnnnnnnnnnnnnnnnnnnnnnnnnnnnnnnnnnnnnnnnnnnnnnnnnnnnnnnnnnnnnnnnnnnnnnnnnnnnnnnnnnnnnnnnnnnnnnnnnnnnnnnnnnnnnnnnnnnnnnnnnnnnnnnnnnnnnnnnnnnnnnnnnnnnnnnnnnnnnnnnnnnnnnnnnnnnnnnnnnnnnnnnnnnnnnnnnnnnnnnnnnnnnnnnnnnnnnnnnnnnnnnnnnnnnnnnnnnnnnnnnnnnnnnnnnnnnnnnnnnnnnnnnnnnnnnnnnnnnnnnnnnnnnnnnnnnnnnnnnnnnnnnnnnnnnnnnnnnnnnnnnnnnnnnnnnnnnnnnnnnnnnnnnnnnnnnnnnnnnnnnnnnnnnnnnnnnnnnnnnnnnnnnnnnnnnnnnnnnnnnnnnnnnnnnnnnnnnnnnnnnnnnnnnnnnnnnnnnnnnnnnnnnnnnnnnnnnnnnnnnnnnnnnnnnnnnnnnnnnnnnnnnnnnnnnnnnnnnnnnnnnnnnnnnnnnnnnnnnnnnnnnnnnnnnnnnnnnnnnnnnnnnnnnnnnnnnnnnnnnnnnnnnnnnnnnnnnnnnnnnnnnnnnnnnnnnnnnnnnnnnnnnnnnnnnnnnnnnnnnnnnnnnnnnnnnnnnnnnnnnnnnnnnnnnnnnnnnnnnnnnnnnnnnnnnnnnnnnnnnnnnnnnnnnnnnnnnnnnnnnnnnnnnnnnnnnnnnnnnnnnnnnnnnnnnnnnnnnnnnnnnnnnnnnnnnnnnnnnnnnnnnnnnnnnnnnnnnnnnnnnnnnnnnnnnnnnnnnnnnnnnnnnnnnnnnnnnnnnnnnnnnnnnnnnnnnnnnnnnnnnnnnnnnnnnnnnnnnnnnnnnnnnnnnnnnnnnnnnnnnnnnnnnnnnnnnnnnnnnnnnnnnnnnnnnnnnnnnnnnnnnnnnnnnnnnnnnnnnnnnnnnnnnnnnnnnnnnnnnnnnnnnnnnnnnnnnnnnnnnnnnnnnnnnnnnnnnnnnnnnnnnnnnnnnnnnnnnnnnnnnnnnnnnnnnnnnnnnnnnnnnnnnnnnnnnnnnnnnnnnnnnnnnnnnnnnnnnnnnnnnnnnnnnnnnnnnnnnnnnnnnnnnnnnnnnnnnnnnnnnnnnnnnnnnnnnnnnnnnnnnnnnnnnnnnnnnnnnnnnnnnnnnnnnnnnnnnnnnnnnnnnnnnnnnnnnnnnnnnnnnnnnnnnnnnnnnnnnnnnnnnnnnnnnnnnnnnnnnnnnnnnnnnnnnnnnnnnnnnnnnnnnnnnnnnnnnnnnnnnnnnnnnnnnnnnnnnnnnnnnnnnnnnnnnnnnnnnnnnnnnnnnnnnnnnnnnnnnnnnnnnnnnnnnnnnnnnnnnnnnnnnnnnnnnnnnnnnnnnnnnnnnnnnnnnnnnnnnnnnnnnnnnnnnnnnnnnnnnnnnnnnnnnnnnnnnnnnnnnnnnnnnnnnnnnnnnnnnnnnnnnnnnnnnnnnnnnnnnnnnnnnnnnnnnnnnnnnnnnnnnnnnnnnnnnnnnnnnnnnnnnnnnnnnnnnnnnnnnnnnnnnnnnnnnnnnnnnnnnnnnnnnnnnnnnnnnnnnnnnnnnnnnnnnnnnnnnnnnnnnnnnnnnnnnnnnnnnnnnnnnnnnnnnnnnnnnnnnnnnnnnnnnnnnnnnnnnnnnnnnnnnnnnnnnnnnnnnnnnnnnnnnnnnnnnnnnnnnnnnnnnnnnnnnnnnnnnnnnnnnnnnnnnnnnnnnnnnnnnnnnnnnnnnnnnnnnnnnnnnnnnnnnnnnnnnnnnnnnnnnnnnnnnnnnnnnnnnnnnnnnnnnnnnnnnnnnnnnnnnnnnnnnnnnnnnnnnnnnnnnnnnnnnnnnnnnnnnnnnnnnnnnnnnnnnnnnnnnnnnnnnnnnnnnnnnnnnnnnnnnnnnnnnnnnnnnnnnnnnnnnnnnnnnnnnnnnnnnnnnnnnnnnnnnnnnnnnnnnnnnnnnnnnnnnnnnnnnnnnnnnnnnnnnnnnnnnnnnnnnnnnnnnnnnnnnnnnnnnnnnnnnnnnnnnnnnnnnnnnnnnnnnnnnnnnnnnnnnnnnnnnnnnnnnnnnnnnnnnnnnnnnnnnnnnnnnnnnnnnnnnnnnnnnnnnnnnnnnnnnnnnnnnnnnnnnnnnnnnnnnnnnnnnnnnnnnnnnnnnnnnnnnnnnnnnnnnnnnnnnnnnnnnnnnnnnnnnnnnnnnnnnnnnnnnnnnnnnnnnnnnnnnnnnnnnnnnnnnnnnnnnnnnnnnnnnnnnnnnnnnnnnnnnnnnnnnnnnnnnnnnnnnnnnnnnnnnnnnnnnnnnnnnnnnnnnnnnnnnnnnnnnnnnnnnnnnnnnnnnnnnnnnnnnnnnnnnnnnnnnnnnnnnnnnnnnnnnnnnnnnnnnnnnnnnnnnnnnnnnnnnnnnnnnnnnnnnnnnnnnnnnnnnnnnnnnnnnnnnnnnnnnnnnnnnnnnnnnnnnnnnnnnnnnnnnnnnnnnnnnnnnnnnnnnngggtttcaactctagcctatcccaacttgtttgggacttaaagactttgttgttgttgttgttgttatagagccatcaagaatttccatgcacctacgctggacctacttctaaaatctaggaaacatgccccttctaaaatataggatatatgtatcatctaggatacatggccctttttaaaatataggacatatggaccattggccactctttttttctctgaagctaaaaactgttcagttagtgtgggttagattgacttccttgtacattaggtagtcgttaaactgttgcctacccaaacaaccagaagagagttccatattgtttcttgggcatgggagttgcttgtgggttgattcaactcaattagcatcgatatggtggctagttgattgagcaacatgttaggtttcacgcaccaaccaagtgaacccaaaagcttaagcgattgggaaaaggtgggcaatccactaatacttcacagcactcccactcacgtgcagccagaacaaggcgcaaacgtggaaataaaggagggagcggaggacttaaaagatgcctctacgaggactcgaactcgagacctctggctttgataccatgttagtttcatgcaccaaccaagtgaacccaaaagcttaagcgattgggaagaggtgggcaatccactaatacttcacaacacaacacacatatttattgatgccaataaacacacatttattgaggccaatgttcaataattgaataagatgtgaatctgaagaaacacagatagaaaaggagaagaattgcagaccttgccatcaggttccgtgggagtgggttagcagctcggccgtgctgcccacgactagactccaccactcgttgatcgcggaggaagtcaaacctctaaaagccatggactccatggcccatgggcctgcaccacgacacgccgaatgcctggatctggtatcccaggttggagggggaggacggaacttccaatactgcgctgtcacaaggaaggcgaggggcatgctaagaagctctacacttgaccacggagccggtgccgtcttctcacaggtgttctccagatctcccacggggcagtcatgcttcatgaccgtcgtggggccaatggccgtgtcgaaggaggtgtagcaggcaggcaggcggaggtgtgagccaagggcggggtcttgaacagttggacgaaagtcagggtgcatcattggacgagacgagggaacatacgttcatgcggagggaccgctagtggggcgatgaatgtatgaatgggcttggctgatggacaaaatcctgaggagagaaacttttgctctttaatactcccactgtccaaaaagaatgtaattctctcttccctaggagtcaaacaatataaagtttgaccaaatctatactaaaaaaatactaacatttatgatacaaaatatgtatcgttagattaactataaaatatatttttatagtaaacccaaatggaaacataaataggacgcacccagtgcagagagcatgtgaccagcacagtcccacaaagaccagcccacacatgagacttatcccatcattctccccctaagtcttgtgcgtcgnnnnnnnnnnnnnnnnnnnnnnnnnnnnnnnnnnnnnnnnnnnnnnnnnnnnnnnnnnnnnnnnnnnnnnnnnnnnnnnnnnnnnnnnnnnnnnnnnnnnnnnnnnnnnnnnnnnnnnnnnnnnnnnnnnnnnnnnnnnnnnnnnnnnnnnnnnnnnnnnnnnnnnnnnnnnnnnnnnnnnnnnnnnnnnnnnnnnnnnnnnnnnnnnnnnnnnnnnnnnnnnnnnnnnnnnnnnnnnnnnnnnnnnnnnnnnnnnnnnnnnnnnnnnnnnnnnnnnnnnnnnnnnnnnnnnnnnnnnnnnnnnnnnnnnnnnnnnnnnnnnnnnnnnnnnnnnnnnnnnnnnnnnnnnnnnnnnnnnnnnnnnnnnnnnnnnnnnnnnnnnnnnnnnnnnnnnnnnnnnnnnnnnnnnnnnnnnnnnnnnnnnnnnnnnnnnnnnnnnnnnnnnnnnnnnnnnnnnnnnnnnnnnnnnnnnnnnnnnnnnnnnnnnnnnnnnnnnnnnnnnnnnnnnnnnnnnnnnnnnnnnnnnnnnnnnnnnnnnnnnnnnnnnnnnnnnnnnnnnnnnnnnnnnnnnnnnnnnnnnnnnnnnnnnnnnnnnnnnnnnnnnnnnnnnnnnnnnnnnnnnnnnnnnnnnnnnnnnnnnnnnnnnnnnnnnnnnnnnnnnnnnnnnnnnnnnnnnnnnnnnnnnnnnnnnnnnnnnnnnnnnnnnnnnnnnnnnnnnnnnnnnnnnnnnnnnnnnnnnnnnnnnnnnnnnnnnnnnnnnnnnnnnnnnnnnnnnnnnnnnnnnnnnnnnnnnnnnnnnnnnnnnnnnnnnnnnnnnnnnnnnnnnnnnnnnnnnnnnnnnnnnnnnnnnnnnnnnnnnnnnnnnnnnnnnnnnnnnnnnnnnnnnnnnnnnnnnnnnnnnnnnnnnnnnnnnnnnnnnnnnnnnnnnnnnnnnnnnnnnnnnnnnnnnnnnnnnnnnnnnnnnnnnnnnnnnnnnnnnnnnnnnnnnnnnnnnnnnnnnacttgattgttggaatgacaccacttgtagataccacttgtaactcataccacttgtatcttgtataaggcttcttaagatacaatacataggatctttgatcttgataccaatttgtgtgacacctctccctatgggatagcatgggtcatccattcgatacacttgagctcttgtaggtgaaggatgtattcttcatttgatgatcacttaaagttgaggatcacttgtggaaccatcatcttgcatgattgatgccatgtgtagatatgatatcacttgaaagaatcttctactatggaaccacttgttggatttatcaataaaaaccatttcttgaacatttgctatcttcatgagtaccacttataggatgtcacttgtgagttgatctagacatcatttgtaggttcttgatgaaatgcttgagtctagataccacttgaaataaaatgaactagatatccatttgcattgttgtcttgtgcttgtactcttatcactatcatcaacttctatggttaacttgatctaaattgacttgcctaagcttccaagtccggtttgaaccaatgactagcttcttcacacctcttgcaagggttatcttgccaatgttgtacttgtcacttgttggcaatccaaattaaatcaagtacttgggtttacttagctcatgaacaaattcatatactaaccactagatcaattaatcattcatgcaatagtggtaggctatgaatgtaaacatttcatttgttatgcatgatcctatgaagtatgtactatatgcactaaccgcatactagtaagggatgaaatgatcatgcacattacaatgatacctttgctatgttggagtagaggatagtcacatagattccaattcattactccaatagcaatgtgaggtccaattataagcttggtgaagaccaatagacaccattttaaattctactcttcacccatatgaaatgaataccacttatgatcaagtgcactttcttgttgtggttgacttgcttcatctttgatcaatgcttgcatgagagcatcaatttgagaatattacttgaaatatcatgactagctctcttttggnnnnnnnnnnnnnnnnnnnnnnnnnnnnnnnnnnnnnnnnnnnnnnnnnnnnnnnnnnnnnnnnnnnnnnnnnnnnnnnnnnnnnnnnnnnnnnnnnnnnnnnnnnnnnnnnnnnnnnnnnnnnnnnnnnnnnnnnnnnnnnnnnnnnnnnnnnnnnnnnnnnnnnnnnnnnnnnnnnnnnnnnnnnnnnnnnnnnnnnnnnnnnnnnnnnnnnnnnnnnnnnnnnnnnnnnnnnnnnnnnnnnnnnnnnnnnnnnnnnnnnnnnnnnnnnnnnnnnnnnnnnnnnnnnnnnnnnnnnnnnnnnnnnnnnnnnnnnnnnnnnnnnnnnnnnnnnnnnnnnnnnnnnnnnnnnnnnnnnnnnnnnnnnnnnnnnnnnnnnnnnnnnnnnnnnnnnnnnnnnnnnnnnnnnnnnnnnnnnnnnnnnnnnnnnnnnnnnnnnnnnnnnnnnnnnnnnnnnnnnnnnnnnnnnnnnnnnnnnnnnnnnnnnnnnnnnnnnnnnnnnnnnnnnnnnnnnnnnnnnnnnnnnnnnnnnnnnnnnnnnnnnnnnnnnnnnnnnnnnnnnnnnnnnnnnnnnnnnnnnnnnnnnnnnnnnnnnnnnnnnnnnnnnnnnnnnnnnnnnnnnnnnnnnnnnnnnnnnnnnnnnnnnnnnnnnnnnnnnnnnnnnnnnnnnnnnnnnnnnnnnnnnnnnnnnnnnnnnnnnnnnnnnnnnnnnnnnnnnnnnnnnnnnnnnnnnnnnnnnnnnnnnnnnnnnnnnnnnnnnnnnnnnnnnnnnnnnnnnnnnnnnnnnnnnnnnnnnnnnnnnnnnnnnnnnnnnnnnnnnnnnnnnnnnnnnnnnnnnnnnnnnnnnnnnnnnnnnnnnnnnnnnnnnnnnnnnnnnnnnnnnnnnnnnnnnnnnnnnnnnnnnnnnnnnnnnnnnnnnnnnnnnnnnnnnnnnnnnnnnnnnnnnnnnnnnnnnnnnnnnnnnnnnnnnnnnnnnnnnnnnnnnnnnnnnnnnnnnnnnaacatcttcatcaatatccccgtctctctgtagcattgatcctaaatattgaaagatatccttcctagacactacttccttccaaactaatatcttcctcctcccgagtagcagtgccgaagtcacatctcatatactcagttttagttctattgagtctaaaaactttggactccaaagtctcccgccataactccagtttctgattcactcctgtccaactttcatcaactagcactacatcgtctgtgaaaagcatacaccaagggatgtctccttgtatgtcccttgtgacctcattcatcactaaggcaaatagataagggctcaaagctgacccttgatgtagtcctatcctaatcggaaagtcatccatgtctccatcacttgttcgaacactagtcacaacattgttgtacatgtccttaatgagcccgacgtacttcgttgggactttatgtttgtccaaagcccaccacataacattccttggtattttgtcataagccttcaccaagtcaaaaaaaaaacatgtgtaggtccttcttcttctccctataccgctccataacttgtcttattaagaaaattgcttccatggttgacctaccgggcatgaaaccaaattggttcatagagacccgcgttattgctctcaagcgatgctcgataactctctcccatagcttcatagtatggctcatcaacttaattccccggtaattagtacaactttgaatatcccctttattcttgtagatcggtaccaatatacttctccacttgtcaggcatcttgttcgatcgaaaaatatggttgaacagcttggttagcatactatagctatgtccccgaggcatctccacacctcgattggaataccatcccgtcccatcgccttacctcctttcatccttttcaacgcctctctgacctcagattcttggattctccccacaaagcgcctattggtgtcatcaaaagagttatccaactaaaaggttgtacccgtattctcaccattgaacaatttgtcaaaatactcttgccatcgatgtcggatctcatcctnnnnnnnnnnnnnnnnnnnnnnnnnnnnnnnnnnnnnnnnnnnnnnnnnnnnnnnnnnnnnnnnnnnnnnnnnnnnnnnnnnnnnnnnnnnnnnnnnnnnnnnnnnnnnnnnnnnnnnnnnnnnnnnnnnnnnnnnnnnnnnnnnnnnnnnnnnnnnnnnnnnnnnnnnnnnnnnnnnnnnnnnnnnnnnnnnnnnnnnnnnnnnnnnnnnnnnnnnnnnnnnnnnnnnnnnnnnnnnnnnnnnnnnnnnnnnnnnnnnnnnnnnnnnnnnnnnnnnnnnnnnnnnnnnnnnnnnnnnnnnnnnnnnnnnnnnnnnnnnnnnnnnnnnnnnnnnnnnnnnnnnnnnnnnnnnnnnnnnnnnnnnnnnnnnnnnnnnnnnnnnnnnnnnnnnnnnnnnnnnnnnnnnnnnnnnnnnnnnnnnnnnnnnnnnnnnnnnnnnnnnnnnnnnnnnnnnnnnnnnnnnnnnnnnnnnnnnnnnnnnnnnnnnnnnnnnnnnnnnnnnnnnnnnnnnnnnnnnnnnnnnnnnnnnnnnnnnnnnnnnnnnnnnnnnnnnnnnnnnnnnnnnnnnnnnnnnnnnnnnnnnnnnnnnnnnnnnnnnnnnnnnnnnnnnnnnnnnnnnnnnnnnnnnnnnnnnnnnnnnnnnnnnnnnnnnnnnnnnnnnnnnnnnnnnnnnnnnnnnnnnnnnnnnnnnnnnnnnnnnnnnnnnnnnnnnnnnnnnnnnnnnnnnnnnnnnnnnnnnnnnnnnnnnnnnnnnnnnnnnnnnnnnnnnnnnnnnnnnnnnnnnnnnnnnnnnnnnnnnnnnnnnnnnnnnnnnnnnnnnnnnnnnnnnnnnnnnnnnnnnnnnnnnnnnnnnnnnnnnnnnnnnnnnnnnnnnnnnnnnnnnnnnnnnnnnnnnnnnnnnnnnnnnnnnnnnnnnnnnnnnnnnnnnnnnnnnnnnnnnnnnnnnnnnnnnnnnnnnnnnnnnnnnnnnnnnnnnnnnnnnnnnnnnnnnnnnnnnnnncgccgcacgcgctgcatccgccgccgtcgctgcttccgcctccgctctggctgctgccagctccacgctgccagcctcgacgcccttgccgctgccgcagcggtctctgccgccgctcgctcacgttcctctgccgtggcaagttcggcctcctgccgacgccgcatgctcgaggcgaccgagcgctgagattgccctgcggacatgacgcgctaccggggggctgctgcgtggggagagggctgcttcagatgagctgctgctcgtctgcgcagagggagaggagtgagcaggagcggccggagctgctgctgctcctagctggggctgttgtgcggctgggaaaggagatgagcaagagatgctcaggctacaggatagtacggctctaataccagttgttagtcgctgaattcttactcttggtagtagtagaattcttactctcatcgagagaggatgacactaggagttggggcaattttctagtttatttccaaatgccatgccaacctgaagggttgggggtacatatttataggttgctagtcagccaagcatatgccaagatgctagtctaagatgtcgtcctagatgctaagatgctgtcctcgaagatgttgtcctctagtctaagatgctgtcctctaagatgctgtcctctagtctaagatgctattctaaaaacagaccatgcagccacaaggaccatatgaccagcacagccccacaaagaccagcccacacatgagacgtatcccatcaagccttaccctcgcctgtgcaatacgaggagaccgcgactcgaacccgggaccttcctgtcacaggcggtaagactctaccgcttgcaccaggcccgcccttgaaatggaaacataaatgttgatactattttctttaaatttagttaaacttaagaaagtttgacttgtttcaaatctagaatatacattcttttttggacggatggagtattaggtatagatatatactgcatgctctgttgagcttgagcatgccttacaaatgttctattagagcatctccaacagattacttatcctgcatcccctaaaagtctatataagtgatctattatgtattattagtagtgtagctcatctcctctcccaacatattaccagtacttttaaagttgataggggagagggagtggatagggattttaagtagctacttaaaacttttaggtattggagataggttgagtaatctgttggagcaaccacaatcccttgaattgcatatttttagtatcagggatgagataagtaatctgttggagatgctctaattttgaggacaccagtgtgcatgaagctttaatgattaagccaaccaaaacaatgctaattattatattcgagcataggctaggccattcctagtcctattcagttccttgtcatttttatattattctagagaaacactcgaccatggtatcccaatcgaggtgtggagatgccttggggacatagctatagtatggctaatcaagctgtttaaccatatttttcgattgaacaagatgcctgacgagtggagaaaaagtatattggtaccgatctacaagaataaaggggatattcaaagttgtactaattatcggggaattaagttgacgagccatactatgaagctatgggagagatttatcgagcatcgcttgagagcaataacgtgggtctctatgaaccaatttggtttcatgcccggaaggtcaaccatggaagttattttcttaataagataagttatggagcggtatagggagaagaagaaggacctacgcatggtttttattgacttggagaaggcttatgataaaataccaaggaatgttatgtggtgggctttggacaaacataaagtccaaacaaagtatgtcgggctcattaaggacatgtacaacaatgttgtgactagtgttcgaacaagtgatggagacacggatgacttcccgattaggatagggctacatcaagggccaagttgagtccttatctgtttgccttagtgatggatgaggtcacgagggacatacaagggggcatcccttggtgtatgcttttcgcggacgatgtagtgctagttgatgaaagtcggacaggagtgaattagaaactggagttatggcgggagactttggagtccaaaggttttagactcagtagaattaaaactgagtatatgagatgtgacttcggcactactactcgggaggaggaagatattagtttggaaggtcaagtagtgcctaggaaggatacctttcgatatttaggatcaatgctacagagagacggggatattgatgaagatgttagccatagaatcaaagcagggtggatgaagtggcgccaagcatctggtgtcctatgtgacaaaagggtaccacagaagctaaaaggtaagttttataggacggcgattagacctgttatgttgtatggtgcagaatgttggcctacgaaaagacgacatgttcaacagataagtatcgcggaaatgcgtatgttgcgttggatttgcggtcatataagaagggatcaagttcggaacgatgatatacgtgatagattaggggtagcaccaattgaagaaaagcttgtccaataccggttgagatggtttggacatgtccaacggagacctccggaggcaccggtgcgtagtggaatcctaagccaggatagtaacgtgaagagagacagaggaaggccgaagttgacttaggtagatgcaataaaaggagacttgaaaggatggaatatacccaaagacttagccttagataggagtgcttggaaaataactattcacgtgcctctgctgggtttcaactctagcctaccctaacttatttgggacttaaagactttgttgttgttgttgttgtaaacactcgaccatggctttgtcttaaggaggagtattgaaccccggttgtccaaaaaactcgctgaaactggttcagtgaggtatccacatttggtgagggactggaattttgggtgggtggccttcttgttgggaaactgtaccaaccaagctactggctcctttctcatcttgtattctagaataccatcttattcaaatgagaaggttatttgtcattgttatttaagttttaaagggtgctctatgatttgctctacaccggcaactcacctcaagaatatctgcttgatgtatgaaacattgctttctttattttttttcagctcatgttgtacagaaagccaaagagaggctgctttgttgctagggcaatttgcttcggcagactcggattgcaaggtgcttaataaatatggaatacttattgtttacaagtcttcagtaaattttgcaaatccactggtaggttagtcaaaactaaagagagaatcgcaccactaatccctgaatttgcatggttgtctctcgcacacccctcaatttgtaacttacattgtgaacccttctaacattggacccattgtggcatcggcccaaattaccgttagctacctagtttaattgatggtgccgatgtggcatcaaacatgggctattatactggactgtttattttcttttatcgtcgccaccttcccttttcttttccattgatcaatacatcactgacatggatatgtagatgatgccatcaaattgactaattatttgaccagtgaacaaaatattttgttttcgtacatgtcattatttatggcgtactcaactggtagccgtgtcttcttgtgaacaggccttattgcagataggcattatttatgaatgtgactttcaataccatgtatatttggctaatattagactatcaatccccttctttttcaagaagtatttattttgtattattgttccataatttgatggaatttaaccacccatgttatttatttgtgattggaatgtatattgcacatgtcttaaggttataggccaaaacctgtgtcagcatgccatggagagcaggtcccatgtttaatgctcatgtcaacacaatttgttatgttaaggtgatttgggccaatgttgcaaacagacctgaagtttaggggggctagcaaagtaatttgcaagttgagggaagttggtgagagtgagacaacaacacaactttaagggctagtggtgcaattctctctttttcagaagtactggtgatttacatatgtaacatttaatttatgtgcactgtatgttgggatagaagtgaaataagtagtaaaccccatttctggccaagcacatcaggtgtgacagattgttgttgctgggaccgtctggcgccttttgacgtgatgccagggcaccatcaatggaggctaacactcttagtggttctagtacaaataaagtgatccacatagactagggaatgttgggactactattcacacaatgcaaactatcactacttgtggtttacaaagaaactttttcctttcatcatgcctcgcctttatttcctctccctcttcttttttagcatggaccaccttctctctccccaagcatatgtagcttctgcaagccactatgacaagtgtagagcacctactttttttatccgatcctacatggcctctggggctaccagtaaaaaagcagcgttggggaaggcctaggcctacatgctgctggccagtccatgcatgacctcacttattctccttgttgctcttttctaactatgtctctgcatctcttattcttggtctgatctgggtgccacacaatcacgaatccagattggtgtgccatatggcagcctctgcaactgccctatccggtgctggcacacttatcttccttatctagtcccagctcatgtttccggtgtctgcacgtgccaagtcccagctctgcccttacctgcattgcgtcttcatcactgtgcttggcaacaacacaccctgggttctatgctcaagctgaacctagctcggctaccacacgcatttcaattgctccaccactcctggcttacaccacaccctaagccctcccctaccaataaatcattgataagatttaagttttttttagaagttagtttatttgttgcagaggtagcctaccccaacttgcttgggactgaaaggctatgttgttgttgttgttgtttccttgggagatgggagagaggacaaccatggggaccacttgttgtctgttctttgagtggagagatgcagaaggtagaaaaagaatgaactcaacaattgaatataatgttcagtataaggaaatctagaatgataaatctcattatctaaggaatgacacaaaagcaaagagatataagatgttttctccagttaattcgtttctgaacttgatagattaatatatatgtttgtttacaggtccatattgtgcaaaggggtgcagtccgtccactaattgaaatgctacagtcagctgatgtccaactccgggagatgtctgcttttgcacttggcaggcttgcccaggtttaatttttatttttaatatagcgtattttttaatgtttatgaggtactttactgttttctactctagagaatcagtggaggcagtgaaataaaaacaccacagattttttcttgctcttttacaaaatccacacaatgtataactttatcaaattagttcccttgcttctctgttgatgggaactatatgtggggactggggatgcaaagatcataataaatatgtttagggcaaaaccatagtgagtttgctggcaccacataccttccttatccagcccatcctagacatggacagattttccaaatatgcgggcttcatgttactggtgtctgcatgtgccaagtcccttgctctgcccttatctgcattgcatcttcaccactgtgattgtcaacaacacacccagggtgctgctgtattcgaggtacctctggtaccacacacattccaattgctccgccaagtaattgaagttacgcagcttgtcgggtatcgatattaggaatacccaaaccaaggaagttagcgcccacgttgactttcccggatggatcaagacatattaaaaggcctcgcccgaccccaaggccgcgggctccgtctcgcccgacctcaaggccgcgggctctcgcccgatccctaggacatgggttctgtctcgcccaaggccgcgggctctccgtctcgcccgaccccgaggccgcgggctccgtcttgcctgaccttgagctcgcgggctccgtctcgcccgaccccttgggtgcaggctccgtctcgcccaaggccacgggctccgtctcgcccgatcccaaggacgcgggttctgtctcgcccaaggccgcgggctccgtctcgcccgatctcgaggccgcgggctccgtctcgctcaaagccacgagcttcgtctcgcccgaccccttgggtgcgggctccatctcgcccgaggccgcgggctccgtctcgcccgaccccttgggtgcgggctccgtctcgcccgaccctaaggacgcggtttccgtctcatccgacggggacccatacggccgccaaccattccaggtccaagcgtatggccctaagtcaaaactctgacaccagggaagagactggcacgcctcgatgtaacccgtggcaatgaagggccatacctgaggattcgcatcaagaacagtgtcgggcgtgccggtggtgttctgcctaaccctcgtacggacgctgacagacgcgtcagttcaccacgacgtccgccatgaccggcagattacgcctgcgcatggcgccagtaacgaacagggccgcgacgtggagccgtccctgttgacatctacaggatcggcgggacccgcatgaaggagaagaaggacacggcgaccctggaagccttcttctctctctcgttcttctcattttcctctgctgtaaccctcgctttcccttcgtctataaaagggaaagcagggtgcccataccaggggatccggacagagaataaaaaacacaagagcacgacatgagcacacggctgagcggcaatcgagctcttagcacccgttcactccttccaccagagacttgggatcctttccctctctcgcctgtttgtaacctctaccacaaaccaagtgccggtaacacgagcaacagcgaactggacgttgggacgtttcgcccgaaccagtataaatccttgtgtcttctgagcacaccatccgagccagacacgtaaatacaaatttactcgtcggtggtccgaaaacaccgacacaactattctccatatgttggttcaatagcccatatgttggttgcacagaattctgtcttttgtttttgagttaaatgcaccggaggtctattaacttatgttggggtttgtccatcaactctaaaagttgattttcgaatccataaacttttaaaggggtttgtccatcaactctaaaagtcatgccggcggccagccacccgacggggaggggagcggacggctggagcagtaccggtggggacgggaagccgccggcgggagctcgagcagcaaaccggcggggatgagcgcgaccggcgggaggcggcagggcacgaccggcggtgaggggcgcgaccggcggagagaagttgcgggtgcgacggcgtctttccctcttatactctgccgcccgattccatctgcgcgcgctcctcactttcttttcccatgcccgcgcgtgggcctgatgccagcttcacgcgcgcgcttccgcggcggcaaaattttcgcgcgcctcgctcgcgccgttcgcccaggtgccgccttacgaagcctaggcgctgcgcccgccttggagtccgcctacccccataggctaggcgagacccatcgcccagcgattaggcgcgcctaggcggggatgaggcgtcgcctttttgaactttggggtggatcaagtggcgacaagcttctggcattctctgtgacaagagggtatcacaaaagctaaaaggcaagttctatagaacgacgattagaccggctatgttgtatggagcagaatgttggcctataaagattcgacatgttcaacaactgagtgttgcagaaatgcgtatgttgcgatggatttgcggtcacacaagaatggaccgagttcggaacaatgatatacgtgatcgcctagaggtagcaccaattgaagaaaagcttgtccaatattggttgaggtggtttggctatgtccaaaggagacctccagaggcaccagtgcattgtggagtcctaagccaagctaataatacgaggagaggtagaggaagaccgaaattgacatggggggaggcaataaaaagatatttgaaaacttggaatatacctagagatctatgtttgacaagcagctattgaagtgcctaaaccgtgacttgaggctcttggtgggtttcaaatctagcctaccccaacttgcttgggactgaaaggttatgttgttgttgttgttgctgcatatcatataatgcaaggggaaatccccattcatcttttccttttacttatgggttagtgggattgtttctttttctttctttctttctttcttttttgcttagttgcaactcgtaatctaatctaaagagtcttttatcaggacacacataaccaagcaggtattgcatataatggtggcttggtgcctttgttaaaacttcttgactcaaaaaatggatctctgcaacataatgctgcatttgccctttatggagttgcagataatgaggtaatttacgatctattttttttcacaaggtttgccatatctctcaaatatcccttttccactattggttaataattccacactccatgttcctttgtaatgggattaactcattttttataaaatgtttatcttatatttcttatcctcgttgtttctgaagtaaatcactgttctttcttataggactatgtatctgacttcattaaagtaggaggtgtccaaaagttgcaagatggagaatttattgtccaggtacattggccttcattgtatattggtcactttgttgtgaatgtttttttattaagctattcttaatttcaggcaacaaaggactgtgtggcaaaaacattgaagaggttagaggagaagataaatggacgagtaagttctgcttgcaaggtttctgcatttcgttgtttgcgatgtgcttgactatagtatttatgaagcttgttcccatgtgatggtttacaggtgttgaaacacttgctttatttgatgcgagtaggagagaaatctgtgcaaaggcgtgttggtctggctcttgcacacctttgtgcccctgaagatcaaagaacaatttttattgatagtaatggtaaacaattttgcaaccactgaaaaattgtaccttttcatttccattctactgtggtgttcttcatgaatttaaattctgggtcatccaggtcttgacttgcttcttgatcttctgatttccatgagctcaaaacatcaacaagatggctcagcagcattatacaaattggccaacaaagctgcagcactttctcccatggatgctgcccctccatccccaacacctcaggtatgcaaaagaattattaaatttaagtttactttgtattacgtatgctgtttgagttgcagtgactttatgatatggctagatgattgggtttattaaatctggggctgcctaaatctggctagacttagaacaatggcaaggttgtgatcctgatcgccctccctaggaggctctgatcataataactcacttcttgcttattcctcttcgcttagccggcccttagttatagcacctaatggccggctgtcaactaacagagtcaataaccaaacgcatgcagatcctaaacccaaacgcatgcagatctatcgtttagccaaagtcccctaaacagataactatggctgtttttagccactaacagttcctgacaccttcgtcttcttcttgctgtattgcttcccaatgaaagtgtccacaacacttctaccttcctttcggaactggggctgagcaatactgaaggtgatgaagcacacttgagcagtcagctgctggaataagacaatcatggcaacgacggaagatgaggtctgaaattgcgccactggagtcaattcagccagtgggggtgttggtgctggtgtcattggtggtgccatggtggtcgcaggggaaggagatgccactgccgtcaggatgtgttcgacaaaggctgccaatactgatggggcaggcatgtccacagctgacgaacatggcggcaatgtcggatacggtggcacatttggcagctgcaagaacggcgctgatgccatgggtgtcaccacaattgacggagttgctgttggcaaggctgttgatgtagaagacagtggtggtgtggtgcccaagactgaggagaacacacgctctggtggagcggacaacgaggccagagagtttgctattccgccaaccctgtccgacggcttcagtcctggcggtgcggatagcatcactactgatggcgttgcaagggctccaagtagggttggaaaattctatatatggtggggtgggcttgtagatgatgcgcttagcttagtcactactgatagcatcactactgatggcgttgcaagggctccaagtagatgatgcatcactacccatcgttttcttcgtgcaaattgttagtagcttctttggaaaaatcagtccacttcgtttttggatttagatggaacaatcgtgcggttgtatacggaactgaatacgatacgcttattcagtcaagcgcacgaccgcaacttttcgggtgtacaagtcgtccagtagcggcccacgtttgactaggcgggagctgcaatgcctgaagcgcagacactgaccccgaccggcatttgtttttttgatgctatacgacatcgtattcatgaccggagtgtacaacatcgtattttcgaccggaggctccaagtgttgcaggccttgccgatgaagtggccagggccaagcaggacgctcgcattggtggagtggacatcaacgctggacatgcaatcgcctggtgcttctccttcaccatggctggcgcaaatgtgaccggaggagtaatcacaggtggggatggcgctgatggtggaagcagtggcgacattgtctggcgacagccatcggtggaagctgtggggaagttgtcggtgtagccgcaattgttggtggaggtgaagctgttggtgttggctgtagaatagaacagagagatagggaaacaccacacacccccatggggggggtgaccttcatatatatatatagccaatatggcagggtgtacatgcgtgtacatgctttacatagcaggtgctaatcacactgattgtgtggttgcctattatatacttgcctaatatacacttgcctaatatatctatcagcctcccgcagtcgaagcgtcaagattccggatgcagagactggaccgaaaatcgtcaaacagctgaaccggcaaaccctttgtcatgatgtcagcgaactgaaaccgtgacggcacatggagaactcgaaccttgccgagagccaccttctcacggacgaagtggatgtcaatctcgatgtgcttggtacggcggtggtggaccgggttggctgtcatgtagacagcgctgacgttgtcacagtagacaactgtggcgaccttcaagggaacatgaagttcctgaaggagttggcgaagccaacagcactctgcaaccacgtgagcaacaacccagtactcagcctccgcactggaccgggacaccgtggtctaccgtttggacgaccaggacaccagactgtcgccgaggaagacgcagaagcctgatgtagagcggcgggagtctgggcaccctgcccagtcagcatcggagtatgcaatcagcttgtcgataggcccagtgctgatgtggaggccagccgacagggtgcccttcacataccgaaggatgcgcttgatcagcgcgaggtgagcttcgcgcgggtcatgcatgaagaggcacacttgctgtacagcataggccaggtcggggcgagtgagcgtcaggtactggagagaaccggcgagactccggtacgcagcgggatcagcgacaggggcgcccgccgaggcagagagcttggcacgagagtcaacaggtgtcgacgtcgagtgacactcggtcatgcccgccttctgaagaaggtccacggcgtactgccgctggctgaggaaaaggccgtcggaggagcgagtgacggatatacccaggaagtgatgtagttcctctaggtccgtcatggcgaactcagggtgaaggcggtcgatgatgcgtcgaagcagagcggccgaggaagccgtgaggacgatgtcgtcgacgtacagcagcaagtaggcggaggagccgccctcggtgtagatgaagagggaggcgtcggtggtagaggcgacgaagccgagctgtcggagaaacgtggcgaagcgttggtgccacgcccgaggggcctgcttgaggccgtagagggagcgctggaggaggcagacggcgtcgggttgtgccgggtcgacgaagccggggggctgctgacaatagagcgtctcatgcaggtggccatgaagaaaggcattcttcacgtccagctgatggataggccactggnnnnnnnnnnnnnnnnnnnnnnnnnnnnnnnnnnnnnnnnnnnnnnnnnnnnnnnnnnnnnnnnnnnnnnnnnnnnnnnnnnnnnnnnnnnnnnnnnnnnnnnnnnnnnnnnnnnnnnnnnnnnnnnnnnnnnnnnnnnnnnnnnnnnnnnnnnnnnnnnnnnnnnnnnnnnnnnnnnnnnnnnnnnnnnnnnnnnnnnnnnnnnnnnnnnnnnnnnnnnnnnnnnnnnnnnnnnnnnnnnnnnnnnnnnnnnnnnnnnnnnnnnnnnnnnnnnnnnnnnnnnnnnnnnnnnnnnnnnnnnnnnnnnnnnnnnnnnnnnnnnnnnnnnnnnnnnnnnnnnnnnnnnnnnnnnnnnnnnnnnnnnnnnnnnnnnnnnnnnnnnnnnnnnnnnnnnnnnnnnnnnnnnnnnnnnnnnnnnnnnnnnnnnnnnnnnnnnnnnnnnnnnnnnnnnnnnnnnnnnnnnnnnnnnnnnnnnnnnnnnnnnnnnnnnnnnnnnnnnnnnnnnnnnnnnnnnnnnnnnnnnnnnnnnnnnnnnnnnnnnnnnnnnnnnnnnnnnnnnnnnnnnnnnnnnnnnnnnnnnnnnnnnnnnnnnnnnnnnnnnnnnnnnnnnnnnnnnnnnnnnnnnnnnnnnnnnnnnnnnnnnnnnnnnnnnnnnnnnnnnnnnnnnnnnnnnnnnnnnnnnnnnnnnnnnnnnnnnnnnnnnnnnnnnnnnnnnnnnnnnnnnnnnnnnnnnnnnnnnnnnnnnnnnnnnnnnnnnnnnnnnnnnnnnnnnnnnnnnnnnnnnnnnnnnnnnnnnnnnnnnnnnnnnnnnnnnnnnnnnnnnnnnnnnnnnnnnnnnnnnnnnnnnnnnnnnnnnnnnnnnnnnnnnnnnnnnnnnnnnnnnnnnnnnnnnnnnnnnnnnnnnnnnnnnnnnnnnnnnnnnnnnnnnnnnnnnnnnnnnnnnnnnnnnnnnnnnnnnnnnnnnnnnnnnnnnnnnnnnnnnnnnnnnnnnnnnnnnnnnnnnnnnnnnnnnnnnnnnnnnnnnnnnnnnnnnnnnnnnnnnnnnnnnnnnnnnnnnnnnnnnnnnnnnnnnnnnnnnnnnnnnnnnnnnnnnnnnnnnnnnnnnnnnnnnnnnnnnnnnnnnnnnnnnnnnnnnnnnnnnnnnnnnnnnnnnnnnnnnnnnnnnnnnnnnnnnnnnnnnnnnnnnnnnnnnnnnnnnnnnnnnnnnnnnnnnnnnnnnnnnnnnnnnnnnnnnnnnnnnnnnnnnnnnnnnnnnnnnnnnnnnnnnnnnnnnnnnnnnnnnnnnnnnnnnnnnnnnnnnnnnnnnnnnnnnnnnnnnnnnnnnnnnnnnnnnnnnnnnnnnnnnnnnnnnnnnnnnnnnnnnnnnnnnnnnnnnnnnnnnnnnnnnnnnnnnnnnnnnnnnnnnnnnnnnnnnnnnnnnnnnnnnnnnnnnnnnnnnnnnnnnnnnnnnnnnnnnnnnnnnnnnnnnnnnnnnnnnnnnnnnnnnnnnnnnnnnnnnnnnnnnnnnnnnnnnnnnnnnnnnnnnnnnnnnnnnnnnnnnnnnnnnnnnnnnnnnnnnnnnnnnnnnnnnnnnnnnnnnnnnnnnnnnnnnnnnnnnnnnnnnnnnnnnnnnnnnnnnnnnnnnnnnnnnnnnnnnnnnnnnnnnnnnnnnnnnnnnnnnnnnnnnnnnnnnnnnnnnnnnnnnnnnnnnnnnnnnnnnnnnnnnnnnnnnnnnnnnnnnnnnnnnnnnnnnnnnnnnnnnnnnnnnnnnnnnnnnnnnnnnnnnnnnnnnnnnnnnnnnnnnnnnnnnnnnnnnnnnnnnnnnnnnnnnnnnnnnnnnnnnnnnnnnnnnnnnnnnnnnnnnnnnnnnnnnnnnnnnnnnnnnnnnnnnnnnnnnnnnnnnnnnnnnnnnnnnnnnnnnnnnnnnnnnnnnnnnnnnnnnnnnnnnnnnnnnnnnnnnnnnnnnnnnnnnnnnnnnnnnnnnnnnnnnnnnnnnnnnnnnnnnnnnnnnnnnnnnnnnnnnnnnnnnnnnnnnnnnnnnnnnnnnnnnnnnnnnnnnnnnnnnnnnnnnnnnnnnnnnnnnnnnnnnnnnnnnnnnnnnnnnnnnnnnnnnnnnnnnnnnnnnnnnnnnnnnnnnnnnnnnnnnnnnnnnnnnnnnnnnnnnnnnnnnnnnnnnnnnnnnnnnnnnnnnnnnnnnnnnnnnnnnnnnnnnnnnnnnnnnnnnnnnnnnnnnnnnnnnnnnnnnnnnnnnnnnnnnnnnnnnnnnnnnnnnnnnnnnnnnnnnnnnnnnnnnnnnnnnnnnnnnnnnnnnnnnnnnnnnnnnnnnnnnnnnnnnnnnnnnnnnnnnnnnnnnnnnnnnnnnnnnnnnnnnnnnnnnnnnnnnnnnnnnnnnnnnnnnnnnnnnnnnnnnnnnnnnnnnnnnnnnnnnnnnnnnnnnnnnnnnnnnnnnnnnnnnnnnnnnnnnnnnnnnnnnnnnnnnnnnnnnnnnnnnnnnnnnnnnnnnnnnnnnnnnnnnnnnnnnnnnnnnnnnnnnnnnnnnnnnnnnnnnnnnnnnnnnnnnnnnnnnnnnnnnnnnnnnnnnnnnnnnnnnnnnnnnnnnnnnnnnnnnnnnnnnnnnnnnnnnnnnnnnnnnnnnnnnnnnnnnnnnnnnnnnnnnnnnnnnnnnnnnnnnnnnnnnnnnnnnnnnnnnnnnnnnnnnnnnnnnnnnnnnnnnnnnnnnnnnnnnnnnnnnnnnnnnnnnnnnnnnnnnnnnnnnnnnnnnnnnnnnnnnnnnnnnnnnnnnnnnnnnnnnnnnnnnnnnnnnnnnnnnnnnnnnnnnnnnnnnnnnnnnnnnnnnnnnnnnnnnnnnnnnnnnnnnnnnnnnnnnnnnnnnnnnnnnnnnnnnnnnnnnnnnnnnnnnnnnnnnnnnnnnnnnnnnnnnnnnnnnnnnnnnnnnnnnnnnnnnnnnnnnnnnnnnnnnnnnnnnnnnnnnnnnnnnnnnnnnnnnnnnnnnnnnnnnnnnnnnnnnnnnnnnnnnnnnnnnnnnnnnnnnnnnnnnnnnnnnnnnnnnnnnnnnnnnnnnnnnnnnnnnnnnnnnnnnnnnnnnnnnnnnnnnnnnnnnnnnnnnnnnnnnnnnnnnnnnnnnnnnnnnnnnnnnnnnnnnnnnnnnnnnnnnnnnnnnnnnnnnnnnnnnnnnnnnnnnnnnnnnnnnnnnnnnnnnnnnnnnnnnnnnnnnnnnnnnnnnnnnnnnnnnnnnnnnnnnnnnnnnnnncctgctttagggagtgaaaaccctcaagcaggaagacggcccggggtgcgcggttggagcggaatagggcttcgatttccacccacagctcgcgggcggtctggttctcgtcggtgatggccagatcaagaaccgagtcgtcgacggtgttcaggatccaaccgcggacagtgcactcggcaattggccacgatggatcatcagcagggggagcagcagactcgctgatgtgtgggaggagactgaatttcccacacagagccttgaagaaggaagcccacttggtgaagttgggattcttcatctccagagtcaccgggatgtgagtcttcacgttgacggcggtgtaggggtggacgagcacagcctgcggtgccgcggcagcggagccgtcggcggtgacagacatgtcgaccaggtggtgtggcgcaccgacgggagaagggtggacggcggcgtcggagttcagccgccggggaaaggtggagaggagcggaagcagaaggccgggatctgattgatcacgcggtctgtgataccatgtagaatagaacagagagatagggaaacaccacacacccccatggggggggggggggtgaccttcatatatatatatatagccaatatggcagggtgtacatgcgtgtacatgctttacatagcaggtgctaatcacactgattgtgtggttgcctattatatacttgcctaatatacacttgcctaatatatctatcattggcgatgctgccggcggggaagatgtgatggctgctggtatagcagattgggtcgtcgctggtggggaagaaggcggtgatgccgttgtgcccagggacagggacgactggattggagctggtgacgagtcccgagccttcatccgatcgctaagttggaggaccgtctcatagatccgatccatccctgcagagatgcgatcatacctcgcagagatgccctcagcggtggtgaggaggtcgcccatggctaggaattgtggacgagcagatgtgatctgatggtgggactgggtgggaatgtgcggcggcggtacagtaccacggggtttatggtgacggaagcagatgtggtcgcaagatcaaaggctctgaataccaagatgatatggctagatgattgggtttattaaaaatggctagacttagaacaatggcaaggttgtgagcctgatcgccctcccttggaggctttgatcataataactcacttcttgcttattcctcttcgcttagccggcccttagttatagcacctaatggccggctgtcaactaacagtcaataaccaaacacatgcagatcctaaacccaaacgcatgcagatctataggttagccaaagtcccctaaacagataactatggctatttttagccacttacagttgctggcctggtgcaagcggtagagtcttaccgcctgtgaccggaaggtcccgggttcgagtcgcggtctcctcgcattgcacagacgagggtaaggcttgccactgacacccttccccagaccccgcacagagcgggagctctctgcactgggtacgcccttttttttttttttttacagttgctgacaccttcgtcttcttgctgtattgcttcccaatgaaagtgtccacaacactttatgagctgactgtggtatggttaaaaatagtatcacaatggcatgatcttcagtgtgctaggatgcacatgaatttattttgattaatcattgtggaatggcgctttggttcaacaaggtatataagggcccaattgagtctcttgtagtccaacctgttgtgaatgatagtgtgtacaacctgctggaggaaaataaatgttcctctggcatgccatgaaaggtaaatgttggactgctgatcagcttgcaaaacatggtctgtctcatccggataaatgcctactgtgtgatcaagaggaggaaacagtccagcacatccttacaacctgtgtctttgcaagacagttttggcataggttgttcattcttcattgcacttaacttgcagcagctggtgcctagcattactaaacatagtttcactacttggtggcggagagctagcaaaagagttagcaaagatcaaagaaaaggggttaacaccctcatcatcttgggtccctggatgccccggaagcagaggaacgcgtgtgtgtttgtgggaaactctccagtgtccctactacacctagaaacccgaagttagaagctcatctctggacgcttgctggagcttccaagctacagggtcttgggctaagtcggttagaaatctaggctagcttagttttctttgttgtaaccccccttaccttggtcctattaagaggggtgcttgtatggaccatttcttttccctataatacaaagatatgcagctctcctgcatgttcgataaaaagaatatcatgtcgatatttttatactgcttggcattgtgttaaaaattgtggtcagaatttagctatcattagcatttttaacaagatttccaaacactgcctgtattttgctatcctaaataaagtcattgtgacattgtgggattttttccatccaattgttctggtaatggctgaggcactggcaattgttactgactttatatttcattgcaggtttatcttggtgagcaatacgtgaatagttcaacactttcagacgttactttcttggtagaaggttggtactatttcatgaccgtgatttcatcagtaggtactttaaataattcttttctatcgtctcccagataatcttaatccttcttctacaggaaagcgcttttatgcacacagaattgctttgcttgcttgttcagatgcatttcgtgcaatgtttgatggcgggtacagggtgagttttgacttgccacaacataatgtgcttttgctggttttagtctgttgatccctttccgtagttgatatattgctgctgtatatagtatgttagttttgaacaaaccttgaatctcatgtctaattcaaaggacattttcttaaccaggaaaaggatgcaagagacattgaaattccaaatatcagatgggaggtctttgaactcatgatgaggttagtaagtcattgacctcccttctcgtttggccacagttctctttctgttgatgaatctgtaactatttttcctcttttcttttttatgccactgtatgctggattaaagtctgaaaccctctttggttttgcagatttatctatacagggtcaatgcaggttaccagtgaaattgcacaggatcttcttagagctgctgatcagtatctcttagaaggcctcaaacgcctatgtgaatatactattgcgaaggtgactagaaaaactactctctattccttgtttaaaccgcaaatttgatatcaatttgaatgccattatttgccttgtaggatgtgaatctagataacgtatctgacatgtatgacttgtccgatgcctttcatgccgtgtcactaagacatacatgcatcttgtacattctggaacattttaacaagatctgcaccagagctgggtaccttctcatgttaataacctttgatctgagaccaatacgatttcaagtaactcaaatattaacacgcaatcttggcatgcagttctccacagctgatccagcgtgtcattccagagctccgcaatttcctaaccaaggcactgagttcatcaagaagtccaagttcaagcgacaggaactcagacttgatttgagtcccaattcattgacaccgacgccttcatctgaccaaagttgctggagatcctgtacagtaaagtttctggagctgagcgttcgatggtatctattgtgggtacatggtggccaggtccttgaaaattaacatcagcaatgtaacaaacttttctaaaatttagtagaggatatgaccaaagtcatgcatcgactagcttacactgggataggctgtagttggatggtcctggccgtaattcgtcggtctcagctttgtttctgagtttagtgtttgtttccagttcacagttcagtgtatgcccgcatctgtttaaagtatgaagcttgaggaagttagaaattagcccctgtagtgataaagctgtccgttaatctcctagtgtggaaccaccgattggatataccgagataactatgtaacatcatactccctccctcctaaataagggaaaataattatcgttttcgcttctcg

SEQ ID NO: 246 - protein, 732 aa, Miscanthus sinensis
MEAEQQKQQPQRPRRKGQKRKLEDEASAAAAATASSLGSAGADDDNEEEDGSAGTPEICCRHSHAALAREVRAQVDVLVRCASSWRHADRAAAKRATHVLAELAKNEEVVNVIVEGGAVAALVCHLEEPAVAAPTQEEQQLRPFEHEVEKGAAFALGLLAVKPEHQQLIVDAGALPPLVKLLKRQKNTTNSRVVNSVIKRAADAITNLAHENSNIKTSVRMEGGIPPLVKLLESQDLKVQRAAAGALRTLAFKNDENKTQIVQCNALPTLILMLRSEDAAIHYEAVGVIGNLVHSSPNIKKEVLNAGALQPVIGLLSSCCTESQREAALLLGQFASADSDCKVHIVQRGAVRPLIEMLQSVDVQLREMSAFALGRLAQDTHNQAGIAYNGGLVPLLKLLDSKNGSLQHNAAFALYGVADNEDYVSDFIKVGGAQKLQDGEFIVQATKDCVAKTLKRLEEKINGRVLKHLLYLMRVGEKSVQRRVALALAHLCAPEDQRTIFIDNNGLDLLLDLLISMSSKHQQDGSAALYKLANKAAALSPMDAAPPSPTPQVYLGEQYVNSSTLSDVTFLVEGKRFYAHRIALLACSDAFRAMFDGGYREKDARDIEIPNIRWEVFELMMRFIYTGSVQVTSEIAQDLLRAADQYLLEGLKRLCEYTIAKDVNLDNVSDMYDLSEAFHAVSLRHTCILYVLEHFNKICTRAGSPQLIQRVIPELRNFLTKALSSSRSPSPS

SEQ ID NO: 247 - protein, 717 aa, Miscanthus sinensis
MEAEQQKQQPQRPRRKGQKRKLEDEASAAAAATASSLGSAGADDDNEEEDGSAGTPEICCRHSHAALAREVRAQVDVLVRCASSWRHADRAAAKRATHVLAELAKNEEVVNVIVEGGAVAALVCHLEEPAVAAPTQEEQQLRPFEHEPEHQQLIVDAGALPPLVKLLKRQKNTTNSRVVNSVIKRAADAITNLAHENSNIKTSVRMEGGIPPLVKLLESQDLKVQRAAAGALRTLAFKNDENKTQIVQCNALPTLILMLRSEDAAIHYEAVGVIGNLVHSSPNIKKEVLNAGALQPVIGLLSSCCTESQREAALLLGQFASADSDCKVHIVQRGAVRPLIEMLQSVDVQLREMSAFALGRLAQDTHNQAGIAYNGGLVPLLKLLDSKNGSLQHNAAFALYGVADNEDYVSDFIKVGGAQKLQDGEFIVQATKDCVAKTLKRLEEKINGRVLKHLLYLMRVGEKSVQRRVALALAHLCAPEDQRTIFIDNNGLDLLLDLLISMSSKHQQDGSAALYKLANKAAALSPMDAAPPSPTPQVYLGEQYVNSSTLSDVTFLVEGKRFYAHRIALLACSDAFRAMFDGGYREKDARDIEIPNIRWEVFELMMRFIYTGSVQVTSEIAQDLLRAADQYLLEGLKRLCEYTIAKDVNLDNVSDMYDLSEAFHAVSLRHTCILYVLEHFNKICTRAGSPQLIQRVIPELRNFLTKALSSSRSPSPS

SEQ ID NO: 248 - protein, 744 aa, Miscanthus sinensis
MEAEQQKQQPQRPRPRPRRKGQKRKLEDEASAAAAAAAAASLGSAGADDDNEEEDGSAGTPEICCRHSHAALAREVRAQVDVLVRCASSWRHADRAAAKRATHVLAELAKNEEVVNVIVEGGAVAALVCHLEEPAVAALTQEEQQLRPFEHEVEKGAAFALGLLAVKPEHQQLIVDAGALPPLVKLLKRQKNTTNSRVVNSVIKRAADAITNLAHENSNIKTSVRMEGGVPPLVELLESQDLKVQRAAAGALRTLAFKNDENKTQIVQCNALPTLILMLRSEDAAIHYEAVGVIGNLVHSSPNIKKEVLNAGALQPVIRLLSSCCTESQREAALLLGQFASADSDCKVHIVQRGAVRPLIEMLQSADVQLREMSAFALGRLAQDTHNQAGIAYNGGLVPLLKLLDSKNGSLQHNAAFALYGVADNEDYVSDFIKVGGVQKLQDGEFIVQATKDCVAKTLKRLEEKINGRVLKHLLYLMRVGEKSVQRRVGLALAHLCAPEDQRTIFIDSNGLDLLLDLLISMSSKHQQDGSAALYKLANKAAALSPMDAAPPSPTPQVYLGEQYVNSSTLSDVTFLVEGKRFYAHRIALLACSDAFRAMFDGGYREKDARDIEIPNIRWEVFELMMRFIYTGSMQVTSEIAQDLLRAADQYLLEGLKRLCEYTIAKDVNLDNVSDMYDLSDAFHAVSLRHTCILYILEHFNKICTRAGSPQLIQRVIPELRNFLTKALSSSRSPSSSDRNSDLI

SEQ ID NO: 249 - DNA, 10860 bp, Beta vulgaris
  source 1..10860: mol_type = genomic DNA
ataaacccacgaaacttttgacaacaacaacaagaaaaaaaaaagttaaaaaaattacaaaaattccttccactctcactcacacttttttcccgaaactacccttttctccgtctatccagatttcctctctcctcccgctgcagctgcttaccccgtccgccatggatctcggcgagcgaagatcaggtggtaccgctcgaagaagcttgaagcgcaagctagaagaagacttccatggaaatcacaagatcaagctcgatcttcctcaaaatcggcatcatcaccataatcatcaagatctgttatcggagatcaattcctatgttcaaattctctttcgttgtttctcttggtgcgattctgatcgcatcgattccaaacgtgcctctcatttcctctccgaactcgccaaaaacggttcgctcttgttttttcagcttttgtgtttttcttgattgattggatataggttttcttttgtgattttgatatttttttcgttgtttcagaggaaatggtgaatttgattgttgaatgtggagcagtaccagctttggtgatgcaacttcagtcaccgccatcggaggatggcggcgtttcgaaacctcttgagcatgaagttgagaaaggaagtgcatttgcgcttggacttcttgctgttaaggtgactaatatatttaatttcgttatataagctcatttcttgcaatttttttatgtagagaaatcacagtttatggcaattaagagtgtgatcacagcctgtttggataattggctgttatctttttcaagataagctgatttagtataaatgaataccttgtttagaaatgttcagccggtgacatgtccatttcttttggtttagagattaatttctttgagtggtctttcatgtcgtggtgattgctcactgtatgtctattctatgtctgactacaacttctaagctaattttaatcttggtcttattgcgcgtttagtaggcattactaaatgatcgtattggtattgaaattatgaagtttataatttggaaggaaaatccccaacttgttacaatggtaacggaattccatctccaaatatgtgattttcttcagatatatcattctcactcagaccacatgtttatgtgataatggatcgtaacgaattataagaagaatagagctgtttcagtatgaagtaacatttccatgagtctttacttacacactaacactaacattgcattactattacaaccaattatgattgcttaccaaatgggctgcaaaagtatttatgtctacaagtgtagccaacaatcctgagctgttatgcatactttatcagctaatttgtcgggagttgggtttatgtgcttgtacagttaatatactggtactttgaataaaaagaatacatttttggaattttatttggtgatttattacttattttgatctttcttaccttgacagccagagcatcagcagcttatagttgatgctggtgctttgcctcatcttgtggctcttttgaaaaggcatagaagtggagatatatctcgatcagtccatggtgttgtaagaagagcagccgatgcaattactaaccttgctcatgaaaatagtagcataaaatctcttgtcaggtctgtagtattatgcatgtctccagcaattataccgttgattaaagagacatatttggtctctattgacattttaaaatctacacagggttgaaggtggcatcccaccacttgttgaacttctagaatctacagatgttaaagtccagagagcagcagcaggtgcactaagaactcttgctttcaaaaatgatgagaacaaaaatcaggttcatatgcttactttgcttcatgtagaacttttttctgaaagggcatgtgatatctgaacttgttttgttcctgtattttgcctctgcagatagtggaatgcaatgccctgcctaccctaatcttaatgcttcgttctgaggatccagctattcactatgaagcagtcagtgtttttactgctcactggaatacgttgcaaaactatatggctgatgctattattaattgctatcagttgttcatttgggtgatgtgtcaatctttgcaggttggtgtgattggaaatttggtccactcatctcctaacattaagaaagaagttctcctagctggtgctgtgcaacctgttattgggctgcttaggtgtgttgatgcatttctttgtccataattccctatagtcttcctaaacatatttttagttgcttaattttgtctacttgctattgctgcagctcctgctgctctgagagccaaagggaagcagctttactccttggacagtttgcgtctgctgattcagatagcaaggtttgttggcaactctaattgcaaatggagtggttaccttaggcagatttaaagtagtgtgattgcttcttattcctgcatttcagaagaatatacatggtgcctttaataatgatttacatgcaggtacacattgtccagagaggtgctgtcccacctttgatagagatgcttcagttgccagatgcacagcttagagaaatgtcagcttttgctcttggaaggttggctcaggtgtgcttcttgtttccttcattccttgtatttgaacactggttctctgtgtattactagaattctttaccagtggtgttcctgtatgtttttttttttttcaatatttgctagttctatgagtatcacatcattattgtgttggtctaaagtttaggcgttcatattgtggacttgaaccttttccttgttttttttttttgaaggattcacataatcaagctggtatcgtccaatgtggtggtatcacaccattgttaacacttcttgaatcaaagaatggtcctctacagcataatgctgcatttgcgttatatggccttgcagacaatgaggtagagtaggaaaatgctagaagattgcctgctttgcaggcttgtactgtttcgatacttttttttcttaaccaacttagctcatcaggtgtctgtgataggataatgttgcagatcttattaaaattggtggtgtcgaaaaactccaagaaggggatttcatagttcaggtatgatctcataatacttgtacttgaatgaattgggtcctttggttctgggttgctgtctcggttttttctttgtgtttctcattgtttaattattaatgtgactttgaagatggttttagagttgcatctatatgccatggtgtatggcctgaaaagtatttggagaaaaagctatgtattgtccgaagtaacatacttaaaagtactacttgtaatgatatttaataagctctcttttaaaaatactctacattaataaagtagctctaaagacatcgataacattatgaagctaacaaagtaacaacattatacaaatatttagatttccaacgacaaaccaattgattatgttattcttggacttataaaaatctgacaaactgttgggttcaataaccataatagaggtagaagaaccaattagttcagcattggatgtacaggatgaagtttcgaagggaacaccttgtcatgccaaatttttaatatcaatttttttcatataatctgttataggtagtcaagcactttggcgtaagcataagttatttttatagttaaagtgctttttgagggtttagaaaatttgatcataaccctccttatttctacggctagatgtattttgtaaactaataaggtaacatattattttacctatatataagcctatagatgaaagatgaatcggaggtgcaactttacatgtgatggattaggttataggtttgcaggtcttgatcgccttttaccatctcttcctctgccttcattgtgagattcgagatcaatgcacataacttgaatgtcttctattgcaagaactcacttgccatgttctttccctactgcagtaacagatacatcatgcagtttatgctctgctgaatcagagttgtagaaacagcagcactagtggaatcattcttttgttgggtcatcatatctatatgctttgtattcaagctcttaagcctttttggacttacttttcaagttttttagaagcttctatcatctgaattcttattcctctagctagtaacagtattttgatgcttgagcttatggaatgatacttctacctcgcaagagagtgtctcaagattaaagtctcaagatatacacaaattgcaagtagtgtttctttggtcagcaaaccgaactattagcacaaagcttaatgtcgttaatcacaaactcagacatttcctgcgtacagccccatagctttgcttatagtaggagtaggtctaagttattgaggaaacaaatgctaacaactacttagtaggattctgagaagcaaattagaaattgatttatacttccctgagaccagcttactaacaaaagtaaactaaaagagtgaaggaaactcttttgttaggcaccaaggatatgcacggccaccctttataaagttggatttgggaaaaaattaagaaacactctacttgctgcccaaataactaagctcaaattttattgcagtccaagtaaagcccaaaagtaacttggaaaaaattgctcctaaaaaactaataaaattagacattttttgctaaggtcaaatagaccaaattagaatcttaataagtcaaaggaaccttatctaacattttttacaaacacatagttgacaaatcattaaggaaccttatctaacatctaaatcattaaggaactctttatatgtgtaattcctcccaatcatgctaaggtcaaatagaccaaattagagggcaagctgtccaaaacacccctatataagattcatcaggtagctaattctagtttatggaatataaatcatgaaatcaaatatcatgtgttacatactagataaggaattaacttatactccatagctaaattacgacataataataataatgatgatgaactctgttggtcttgaacatctgtttggaaccgctctttcatttctcgatttacatcacttttatgctggtttatgcgcaatctgtagaagtgaatattgtttcagagttcacacatatatttacattaatttgtgcaggtttttttattttctaattgatttttgtatacttagcttacttgtagtacatttggttgtcttttctgcagccaactaaggattgtgtggggaaaacgctgaagaggttggaggaaaagatccaaggacgagtaagatctcagcatgttattcagtaacctgatttaactatctacagcagtgcagttctttttttggttttgttctagtctaacggtgtttcttgtaaatctgttcacaggtactaaaccatctgctatatctattgcgggttgctgataaagttgttcaaagacgaattgctttagctcttgctcatctttgttcacctgagcatcagaggaggatcttcattgacaataatggtaaatatttcgtaagatcatacccaggatttgatattgcttcttatcaggtctttgttacatctcgattggggcacctagtatttgattgcttatctattacactggtacagacttttttccccatagaaaataatttttcaatattttggctactttttctttaggtttggagctgctcttggagcttctcgaatcttcttgtattaagcaacagcaagatggttctatggctttgtacaagatggctagcaaaacaacattactttcaccagctgatgcagctcccccgtcaccgactccacaggtgtgtgccattgggcttatttgctacgggtggagttaaagtgctgtatctccactggaactctgcttctttctactgtaccatctctacgatatgtatacagttctttctgtgatggatcaattgctctatgaaattattctttctttcagtgttaaggatgcctagtaattagaattctttcatttgtttggcaggtttatttgggcgagcaatatgtaaataattcgacgttgtcggatgttaccttccttgtagaaggtaaaatgtctgtaacctatatgtagacctggcaaaatagtcggtcagatggattttgggccgttaattatgggtttgggtgatttttgggccgggttatattgggtattgagttgacaacccttgactatgatttagaatgtttactttgggttgaaccaatgtgtcaagttgtttacgttatttcagtttttggcagaagttatattgtccatttattctatgtattttttcaaaataaatatatacgagtactctactaatgcataaatgatatgaacaactaaaataagttttcataacaatatagttcatgaataccaaaatattcaaattgtcaaactgtgggttaatgatggcaacaaagtaaaatctagcctagtccatttaaacttattaatcaatgaggaaatttaaatgcatgatggcgtgccactaactatgatttattgaaattgggggaaaggtaggggcactaaggaagaataaatatgcatgaatgatttattggtaagttttatttgggaatttttcaataagttttggtcatgggtcaaatcgtattggcctattgggttgtatttggcgtgctcatggttagtattgagttgacaacccttgactatgatttagaatgtttactttgggttgaaccaatgtgtcaagttgtttacgttatttcagtttttggcagaagttatattgtccatttattctatgtattttttcaaaataaatatatacgagtactctactaatgcataaatgatatgaacaactaaaataagttttcataacaatatagttcatgaataccaaaatattcaaattgtcaaactgtgggttaatgatggcaacaaagtaaaatctagcctagtccatttaaacttattaatcaatgaggaaatttagcatgatggcgtgccactaactatgatttattgaaattgggggaaaggtaggggcactaaggaagaataaatacgcatgaatgatttattggtaagttttatttgggaatttttcaataagttttggtcatgggtcaaatcgtattggcctattgggttgtatttggcgtgctcatggttagttttttgggtctgattattttcggatttcaatgtcatgagtttgtgttgaatcccagttttctcgagttggattttgagtgaggtcaatttttgtcaggtctacctagatgcttttgttccagataatctctttagatgtttacttatagtatctacacctctggttgctttcaggtaggagattttatgctcaccgcatatgtctacttgcatcttctgatgcatttcgtgcaatgtttgatggtggatatagggtaagtgcaccatagtttaaacaatcttttactagttatatggttgtaattggaattcaggttaaaagtatgtattatgaccattactgcagtttacttgttatttatcaactgatttattttaatatcaaattcacacttactgtatgtaatatcctgtttttttccatgtctctgattgcaggagaaggatgctaaagatattgagattccaaatattagatggaatgtctttgagttgatgatgaggtggatctttttctcttcaattgttcttggaatttgaaactttgcctgagggcggttgataaatctagtgtcgtggttttgcagatatatatatacaggctctgtgaatgtcaatttggatattgcacaggacttgcttagagctgctgaccaatatcttttagacggccttaaacggctttgtgagtatgccattgcccaggtaacaaccatgttatcttcttatgttggatatctagatttaagcaacatccatgttcttcgatttttttttaaaactttcactctttcaggatatctctgtggagaacgtcatgctcatgtatgacttgtcagaggcatacaatgccacatctttaaggcattcttgcatcttgtatatcttggagcagtttgatggattaagttccaagccctggtaagattttgctaacacatcagaaaatgtagctcattttctccactctgctgccttgagctaagagctctgtgaacttataatattgtagaacttattactgcagagtctattatacaactttttcactgttgaagtctattatacaactttttcaccgttaaaagaactccctatattgctgcaaacatattgcaacatgatcacaatgtcaatcttacttacaaggttaacatgataacatcactgatataaagtgtttgcaggctccataaatgtttgcttctgtgttagcgttgcatcttgtcttattaaattttttgaatttggcaatgttttgttcaccacatggcaaatacctcttcaattgaatgtctatatatgcataatttttagtatggaaaaatgaattggtcttgagaggaaagtgaatggtcaatgcctttatgtaaagtaattatggccaatgcctagtacagagtgtgagtgctgctgactcatttcgtgatatgagttagtacattatgtaacctcacacttctatttatgtgcttgtttctttatgctctaatctgtgtgcttgttcatatcacaggtatcctcgcctaattcaacgtattgtacctgagattcgtgcgttttttgaaagagtacttaccaaacctagttttgttgaattgactcaggcatagaggatccaaacacttctctcaaatctcaatcattgactaaccatttaggaaatccttacaatcacatgtcgttttagtgtcataccattttttgagcttgaagtgtagtatttagattccattgagtgtcttggtccttatagtgtgtaatgcgatggtcaaaatgtcatattgtagttgtttaccgtattagccttagccctctttttcgtgttctttttcatgttttgtttaatataagtgatgtaaatcttcgtcaatacttccgcacatcttgggctattgtgatggactgacatattcatgtaagatctttattgtgtatattgtttgacaagttcgaattcgaagcgggtaaaagttttgtcacattaaacaccaaacttgacgcacgaatatatatacttcctccgttccaaattagatgttacattttctattttaagaagtttcaaattagatgttacactttcattttgggtaataatttctctttatctctctcctatcacatgggacctttttgttttctttctctctctcctctccaaaaattgtctaggagttcgtaatttcaaaagtgtaacatttaaaaagtaacggaggaaatcgttccaatcatgggtgttctatcattctcaatcccaatttttgattatttttcagtggtcccagctttggtgtatgttttataaaaatggtctcaattgattgataacctatttaataagttgatttttttaatcggttttcattcttcctccttttctctctcctctctcctctctcctctctagtctctcccctgtcacccctttacctccccttgccaccattcttctcccctaagcccctcccctgccactctcctcctcttcctagccaccccgtcctccttgccctccactaccaaaaattcacatcatgttatggattaagtacattgtgattcctttgcttgaaaaatataataagaaatctttatgtgctcactgcctcacacaaaaaaacatttgataacttgaatgattttatttgaaaaatacaacaaacatcaagatagtagatcaaaacacaaacatggtagaagttaaacatgtttgaatcaagctagtagatcaaaatcagcatttactatatgttattcaaaaggttcaataatgtgtgtatattggattttttgaggcaattgtagatccttggtggaaattctaattggtcaataaaaatatatttcaatgcaatttttttttttttttgtttttccttagtttagccaatttcttgtgaaggtaaaaagggataaagaatctttgtgttgattgtcctctaaatgtaagttttcttcttctgcatgtagaaaaggaataaataaatcaattaaatttcgggaggcttcataaagtgcttctttcggagttaaactgccatttgtccatatttcgagaaaaaagtatctcttgtttttcattctcatttccataagaatgaataatatgattcacgtttcgaacaggcatgaataaacatctataggataacttccgtcttgaaagttatttggtgcttttatatgatatctgcgatttctctcaaattgtaatccaatacacaaatcaattggtttcgtcaagctatttgtcaactatttcaacataaggtggtaagatgatatcttgagtagttacacacctggggcccctaacgtaaatagccgcctcacaagttccatatagattacttctcaatactatttctttcaaattcattaaaatttcgtgtactgattcttgaatacctaatatggtcgagtattcgtgtggtattttctcagattttgcacgtgtgttgaatcaagaactgatagtaaatgcctttattatgggcgctttattctctctccacttatgaaaggtcaaggtgatacaataggcattgcgatgcgaagagcgttgcttggagaaatagaaggagcatgtatcacacgtgcaaaatctgagaaaataccacacgaatactcgatcatattaggtattcaagaa

SEQ ID NO: 250 - DNA, 21486 bp, Beta vulgaris
  source 1..21486: mol_type = genomic DNA
cttcttccggagtaaattccatttgcaaaattgagcgcacgttatactacttgaaccggagaagaccgtaaaccggtctatcaacattgaaccggctacttgactcaaacgactggtaaagtgcaaaaatataaataaaaaatgtgagatcagtataattccaaaattaccccttgcttacccatctatttctggaatccaaaacagttcaatctctctcttcgtcctttgtggctgcaatggggtccaaggagtggcaaggcaaggaaaattcgagcgacaggaaagggcaaaagaggaaattagagcaacaatctgaggagagagaatccgccattgttaccggcgaagctcttcaacgagaggtaactactcaggttgatattctcaaggcgaattactcgtggactgaagccgatagagccgccgctaaacgagccactcatcttctggctgaactcgctaaaaatggtacaaattttgatccctaatttgaagtttctgcttaattaattagggatttcaattggtgtgattgattagagatgtttgttgaattgtttttttttttttttttgatagaggaagtagtgagtgtaattgtagaaggtggcgcggtgccgatgttagtgaagcatctttcagcaccaccgtcgatggtggaagatgatggtgtgaagccttatgagcatgaggttgaaaaagctagtgcttttgcacttggccttcttgctgtcaaggtcagtcaagatattttagtgaatgtttattgcaaaatgccgaactgaagcgttatcgaatgtttttttattttattttattttttttaaaattaggtaataggtagcgaattttgttatgatgttttggtagatggccaagagtaatgtggaatgtacctcacgtatgtttaagtttgggtaatggaaaggacaggaaacatcattttagtaccaagtgaatttctttgtttaaacagttagacaatgcgaatttgttagctggaaatgttggttaaactctgcagagatgtttgcaggaggaagaatatatatacagttgcataattagcttatcacttgttggaggtggttattttctgttttcatatgtcgtactattgtttagtgtactttgttcaacttgcatttccactaaaaagttcatgtaggagtttggacaatattggcaacattgatgaagtatcagtttaagattaagctgttggtgatacaaattgtgttgtgcagttggtgatacaaattgtgttctgcagttggcgataaaaattgtgttttgcagtattgcttctaactgatgattaaaatttcatgaaaattttctgctttggttttgtgggtgcttgattcaataagatgctacatccttagcatctcttcctctggcatgtttagctaggatgaaggattttccatcgtgtgacttataacggcaccttatacctcatattcttagatttgctgtacattttattcttcttttttttctggttggttggtaattccttttctgtttatgttttcggagcgccgcttatgtttatcacactttcgttttccctgtgcagccagagcatcaacaactcattgttgatgctggggccttgccccttcttgtagatcttttgaagaggcacacaagtggcttgaattcacgggctgttaatggtgtcattcgtagagctgctgatgccatcactaaccttgcacatgaaaatagcagcattaaaacccgtgtgaggttcgtttagttgtgctgtaactgaactgaaaatgtcatttgttttatttgtctgactgtcgttcctggactctgaatccaggacggaaggtggtattccacctcttgttgaactacttggatttaatgatgcaaaggtacagagggcagttgctggggcactgcggactctagcttttaaaaatgatgaaaataagaagcaggtgatggatctttctgaagccagtttgtggatgctatccttaacaattcaataagtttttctgagttttcttttctaacaaattcaagtttatgacgacgcagattgttgaatgtaatgcccttcctgctcttattctgatgcttaaatctgaagatgctgctatacattatgaagcggtatatttacctttacatcttaatccagtggttttcagtgtggcgggatgtggtttaccatatttcctacatttctactgacatagatgaggttttgtgtatgtttgggactttgcgtgtcatgctaacttgctgtctactttataaattttcaggttggtgtgcttggaaatttggtacattcgtcgcccaatattaaaaaagatgtcctgcttgcgggtgctttacaacctgttattgggttactcaggtaatcgcacacaacagtcttccatttgcatgctgtagttaattctgtacgttaggttttttttattatatattttatttcttcatctctataagtatggtgttttgatgtgaattatttggatgagtttgggttgcaaaattaggtaaaacccttaaagtagtgtatggaacaaatcgtttaaagtgattttaggatggttaaatacttaaatgtcactcactgatctgcttctcaaataactaagcaaaaacctaacccacaaattcattcaatcatgtccaccttgaagatggcgtatgagacttgattttataacaaagcaaggctagttccctttttgacttgaagtaggaacctaaagacataccgatcagactatgaatagaactatagaagtgtgggtttaccatgcaaggcttgtgatctagatgtcaagtaggatagaacaatctaagtccaagtttacattaccccaaataaactaattcaagtaaacacccccattacctatgcaaaggcccataaacactaaataaactaaaacccatatgtaaaactcctgctctagggagaatgataagggagaatggtaagactctgtacctaacgtttcttgcttttacacatgcaatttataaaaatttgttttattaatccaatcatttatgcagtttttagaaatctattttactaatccaaaaaggtaaaataaaaaccgggaattatattatttgattagctttgaacaatatatcgaacctaccgtgaaacttgattagactagtccatatcaggaatggataattagttgcagtgttctcttggtaccctgtaaatgtgacttatgtgttcagcgtcttgagcaaactttgatgattgattcctatctcttcattgctctttcttctcttaggggtgtgtcctcttcacctgtacttatctagaactaaacttgtttttactttatgggactggatcatttcaccttatcggacttgattaaacctgaaacttattgatttaaggtgaagaaaacacaccctaaatccttgagtaatttgtatgttcagcaaggaaggcttttactgctgtttgaataaattaatcaactgctgttggatggaagtgttaatagtactatacattttcttcttcatataattttaaccagtgtttcattgttgtgaatgtcacaaattccatttcagattgagtggccaaagttatcttttgaaattcccctgtcaagtatctgccgatatagatgtattatttaattcatttttttcccccctgaatcctgcttatgctgggttcatattaaacagttcatgctgctctgagagccagagggaggcagctttactacttggacagtttgcagcaactgattcagattgcaaggtttgtcacataatttttcctaattttttaaatctatagtttaggatattccaaggcatgtcatatctacttcacattcttgttgatagacagatttttcttttctcctttttttatgtatttatgaaagttaccacaaatttgatgcttttatattattagtttgtatttttattgttaagaatatctgttcttttacttttgaattgagggtacagcagaatttttttgttgatgacttaagacagttcattagaacaaagaacgataatgcttgaatcactgaaggtgttgcttaggaaacatcatagtgaaatggaatgattttttggctattcacacttaggtgtcctgacattctgataataaacttatctagttcaggtatgctgatgcttaagattcagtgacactctaatctttggtgcctatagatataccatcattgttaccttgattaatatgttagatttctcaaaaatcaagtctctctccgtttaagtttaagggctccttggccgaagataattacaacacattaagaggatctatataattttttagagtacttctgtgcactgcctcaatgcttgcaattgtgatgctgggacttgtcactataccttgctatacctatgttgacatgggatggtctaggtgtagacattgcgtatctattaaatcctagatgatgaaaatagacttgggcctctctgcagttgctggttgttcgacacgatttttagcagggcgaggatatgccagtggaatccccctccccgctcctcgattagtcttctttccacttcttctgagttctgctttcccattcactttctcctcttttgagatttcttctttaactggaacagagagctgatgttgggacttcagacttgcaggccttttgtcttattcttttatttgcttctgtcagtaacccggttgactggtaaaattaaaatgtacaacctaggtacctttcttttgcaagaaagaaaggccaggcaactgttaacttttctctgtttttttatttttttggctttgtaaaaagtaatcctttgattcgagtcagacttatcctcattttttcccttaaaaaatactctctccattcttaaataagtgaaacacttctctccaaaataagtgaaacacttctctcctttatgtgagaactttttaagagaagtgtttcacttatttcaaaatggaggaagtatatattctagctttttattgtaaataagaaatttcttttacaatatttttttttgtaattaacttctaaactactactcgactattgaataactatccctcagaaaaataaatagtagtactcgccaagacgccaactgatccttttgttcagaaagcagtaacctataatattgatgtcttcaattttgggggatgcaaataatgtttattctcaatactaaaagagtactatttgaagtaattgtggtattgtgaattgtttgtgtcctgagtccatatccaaaatgcggatgcttgttaaatgtgtcccagtatcttcaaatttatattttcccaagccaaagctttcgatccatagttccataccagatatcgaaacttccagatacaactgtccaagtccaagcatcatagtgccatatttactcacatttttggccaaaattgaagtgtcccagtgtccctaatctttttgaagtgtcaagtgtcaactgacatggatactcgagttaaaatgaagagtctgagcatgatagggagcttgtgtggtgttacagctcaggttggttgagtttaggattgctttttttttttttttttgaagcaagcattgatagtttttttttttttttgaagcaagcattgatagttttttttttttttttttttgaagcaagcattgatattttttttttttttgtaagcaagcattgatagtgtttttttttagcaagtgctttttttgaagcaagcattgatagtgtggtgctttattacaggttggttgagttcaggagtatgtggtatgggtgggacgaatgggggagttttgggaatactcgctattgtgtgctggagggcacttctggagttagatgctaggatgtaaaccttttcaccttctcttactttttcctttttgtgagtggggttggagggtggatgaggcatgtaatttacattcttccattatgttatgtaaggaaatttgaacatgtcgtcctgctaactgctgttacatgacgctgtatccaaattcacgttcttcttgcggcgactccccgtgttgaatcgttgtcattgtgttacatgcattccgtgtcagtattggcaaaaaagaaagggaaaagatacattgccatagtaaaagaacatgcacacgctgaggaagggagaagaatgcgacagggctttcaaattgggtgatatataggagttgtatctattgacattaataataggacgagtcattcatgttttaagtaattatccattcactaactatgtaactctcatatgataggtttgctcatataatgttacaagaatacttctgaatctagaaaatgcaaatttgagtttaaaaattcatcaatatgaagtttcttcaagatattcatgccgcggttcattcaatcgttcattacaagccgcttgtgagacattgcgaccaccactaatgaccacatatgaccgcatacccgattgtttttccttgggatgaggagtctttggggtttaactattttgaaacattttttctattttgttctctacttctctcgcgggaaatcagtagtttaggttcttgtgctgcagcggatcctcattgatcttttcttgatttaattgtgcttgggtatttattgatgttcctgagttatttgtcttatcttatttatctatttatttatatgttaagccgtcctatatagttagtatcgggatagatgttgttctgttggcttgttgattctccttaggaatcgcaacctttatgcattgccttctgtcactggtaatcttacttttgagacacttcctttgatgttttctaggttcacattgttcagagaggcgctgttccacctttgattgaaatgctccaatcacctgatttacagctgagggaaatgtccgcctttgctctcgggaggctagcacaggtcatcacctataacttcgctccacctctttgattgatagttacatggggcatatatatcagttaaaaggcgttcatgcttatgagttagaattgaaaattttctgctacagtcttatgattacgtctagtattggcagaaatgatttatagatggttggacaaattgtaggaattgggagtggttgttagtcaagcgaatttcattattggaatacttaggacaagaatggatactttaatagacaaacaatatgtgttatgagggggaatgggggtgggggcggttgccgggaattggtgtagagcagtatgagggttttactcaaataccggatttctcgagaccctctagttaaacatgtgtgctgaatcattattgtacataatggggttaaagatctatgaaacatatagctagtacgctggattgagcttgttggatggttcttagctatgttacatggactcaagtaaatatgttggacacacattcatgtcctaagtgtccatacccatttaattagtttgacccaaaatgaagtgtcgtagtggtcatacccatgtcggagtgttgaggatctgataggtgaaatgcaaagtccaaagcaccaatgattcctaatatttgatatattcttatgaggcagatggagcatggaaatgcagctcaatggtaccaagcatattcaatttttttttatctacaccttggccacaacaattggccatatcaaccaagccctcttgtgctcttatatgtcacattattataacataagttgttccttggctatatgaatgtgaatatcaactctttctttttcaattaggacaaattattctaaattcttgattactatgagttcccgaggcatttagctttgtggaagaggaaattcttttagccgcgtatgacccgaactcaggcattgtcttctcctcatgatttttctgatcgagggatttttggacctaatgatggtacctgttctttggtggtggttattctctttcatatatgttaatacttcctccattttttttagatgttacacatttgaaaatttgggttccctaggcaaaaattgaagaagtgattaggagagaataagggtaggggattaagcatgtggggaccattgtacatggggtttaagggaagggaggagagagaaaagaggaccctaacttggttccccaccaccaccccagcatcccagcgaacttctaccaccaccccaccacccacccgaaattcgaaccacccacccgaaagtcccacacagccacccaaaaccccacccacccacccgaaaatcccaccagccacccaaaaccccaccccaccccacccgtcgaaatccccacccacccaccagaaaaccccacccagccaccgaaaagcccaccccacccgccaaaatccctacccacccacccgaaaaccccaccccaccgccgaaatccccacccaccccaaaaccccaaccacgcatcgaaaacccaccccagcctcgcgaaaccccacctctaccgccgaaaactccaccccagcctcgaaaaccccacctctaccgccaaaaatggaggacatgtggttttgcgcaaagaaaattgcgtggttttcggtgggtgggggtggtggggaaggttttcgtgggtgggggtcgggttttcgggttggtggggtggggttttgggaggctggatgggattttcgggtgggtaggtggggatttcgggtgggtggtgggagttcgctgggcttctgtggtggtgggtaaggaggctgcgagatgggggaagggatggggcagccgaggtggtgggggaggggtggtggaagagaagggaggaggtttaattaatttagattagtatataataaggttaaattaagttagtttaattttgattgacccttataagtaagggtaagtgagtaattttacagcataaaactttccaatttaagaaataaaaaaaagtgtaacatctattttgaaacatgcaatttaaggaaagtgtaacatctaagaaaaacggaggaagtaataaaatttagtgtcttaggtgggcaggaggatcttgggtgcgaaaaacatatggaagagcacgacaatggagtttaatttttaatgccttttctttccatttacatgtatgtaattagtttgtttgaatcctttgagatgtcaccatatcaaaggctaattagccatatctcatagctcctgttatataaagccatgcactgctttgtgggaaatttaaaagacattgggtaaatatatcttactcagtttatagccttgtgttcaatccgtatcactcttaaatcttaatcatcttgcgtgctatattgtatcctgccgaatgccaatagaagcttcctcttaggtattacaacataccaatgtcaaccacagcatgtacactattatcacgatgtaaagttcctaaaactcaatgggagttgcaaaagtaagttaacttgaaagtcattttagataaaattcaatgattctcaactttgacaattctggactctttcatataattttcaagattttctcagtgatctcatgtacgttagggatttgggttacctcaaggagtcatcttgtaatgattcaactttcaaccattcactagaccacccttttaaaataatttgcttacatattactactttattaatgatgtgttgatgcttgttaaagtattgtggaagctccaatattttactgttaattatacatcttaccctattattagtccctcaaccttgatatggcagaatgctatgaatcgatttagggggtaagggtattttggagagtctctttattagttagctcggggaataagctaggtagctgtgctaaggaaattactctatatatagggatgattaaagagtgaagattatgttgaaaattgttgaaaatattggtgagctttcaacaattcaattagaagagaatcaagcctcttgaaagcttgaatatcatttattttttctgtaattttcagtttatcaagcaaatactcatcttctttaatttctgcctttaatggtgtccaagctatgttactttatagcaaatggtatcacagcagaacgattctgggagattagagtgctgatattcgaattaaaaaaaaaatatgcaatggagttcggcggaaaaaactgcaggcgaaacaaatgcaaatgtgaatcaatgaggagttcgcctacatcacacgcaagagaaatcgaggatttttagatgtcgaagaagagcggaggatccagagagagcttccacttccaaagtttaacggaaggaatttttgaagggtggattctggaattgcaggacaacttccattttttccagttagatgagtcggcgaagttaaaggcttccatcataactcttgatgaagacgtgcagcggtggtttgaatgggaacaccagtgactaccattcaatgagtggagagaactgaaggcactggtctggcgatattttggtttgccatcggtgctttcatggcaatcagatctagagaaaggaaaggtggtggtgaaaacgaatgttgttcaaccaaccacctttagcttcctagtattcaggagacgaggaaattggctgccttagtacggtggaatcttttcctgaaccgaaggaaaagaagctgttaatcgttagtgttagccaagggtttgaaatagtcaagggcttaaacagtggtcctgctgcttatttaggaggcttgactgctccggtagatggagaaattaatggaaaacaattgttgagcaactttcaaaccagaccagtgagtaggaaagaggtggtgaaaacttccacctatgactttccacagccacggaaaaagaaattgaagcagaagaagagcctaagaaaaatggattggggaaggtgctttaggtagtggtcaaggttgtcacgccggtggtagatggtagatttcgtagtggaataagtggagttactagtaggcgaaaaggaggaagagaaacgaaggaagaagtgcaggttgtgagtctggtggtggtccaggtttctctggtggtgatggcgattatggtggttacatgagaggagctgaagctgctgatgtagggtggctagttagaggagatcttttgggaaggttcagatctcttttccggcgaagattttgaaggtgaagaagagcagcgcttacgttgggtcttgttgcagaactcttcagaagatgagcataagaggagcatggttggcttgaagaagaagccaattagggaacagactagtaacggcttttttgtaaaattgctaaaaacaagtgacagcgtagcaaaaaggcacaccctactttaatgaatgatacaaggcctgaaattggaccctttcatatcaaacccatttattgttcgatttcggatgactggttttcgaatgggctcactaattctaaacccacttccctaccaccaatgctgaaacccctttttttccattccagcccactacagagaacagaggaagggcttatatctattttcactaaatcccagcccaaccactcctcccatttttaatttcccatttttcaccccttgagcccaaactgccaccaaactaccaacctacttttgagatccttacatctagaactaaactcacttctccagctcatgtttctacactcaaaccagcaaacccaactttccctcaccaaattaaaatttccgtttctatcttttccgcccagctcaaccataagatactaactcttccatgacaacttccatttaccggcaacattcaacaaagaggagctagaacttctaacgcaacagtcttctgatacttttgcacatagcattgccccacgttgccaaggccgataatcgagtgcggactactacccacctcgaggacaaggtggaagtttcagggtccggcgatgctatgaatcgttttagtgggtaagggtattttagagtctttattagttagcttggggaataagctaggtagttgtgctaaggaaattactctatatatagggatgattagagagaagattatgttgaaaattgttgagaatattggtgagcttttaagagttcaattgggagagaaccaagcctctcgaaagcttgaatatcatttacttttctgtaattttctttttatcaagcaaatactaatcttcttccttaatttctgtcattaatggtgtccaagctatgttaattcatagcacggaagccaatgtattgaattgatgtgtttgtatatggaggatgtagtagtgcaagttttgacatcatttactaggtttaatatattgtttaatcatggaactgtttctagtatatttctttgatttttatttacaaagtatgtgatgttttaataagcaagacaccgaggagagtgtcggtcataaaaaaaaaggactatggttataaacctcatgcttaaagctatcattaaacaatttatctacaaaatcagaaaaacctcaagctagcatctatttggcagaactgttctattgagaaagcttgattgcaatttttccgctctgcagccgtatatgatttcttttgtcatgattttgctgtttttttgtgccactttttcgggccatctgatgaaagatatatgggttctgtttaggagtcacataatcaagctggaatttctcatagtggtggcttggtgccattgttaaagcttcttgatgcaaaaaacggttctcttcaacataatgctgcttttgctctgtatggtcttgcagataatgaggtatcttcaatatgaatttgagatgctcagagttgcattaattgggattttgttaatttctgcatctttactttcttttgcttaatacagaatggtaatgtcatgcttttattacttacttaaataccaggataatgttgctgatttcatcaaagtgggtggtcttcagaagttgcaggaaggagagtttattgttcaggtttgtttcccgttttggtatatagaactgcttactgttctattctctttgcaatttggtatgagttactatgattgagacaaggacttgaggatttggccaattggctattttttcttgtgggagtcatcacgtattccagttcattattgaatatattgatcttctatccaatgatttatgccaaatatttgctttcaggcaacaaaagattgtgtagccaagacactcaaacgattggaggagaaaatacatggtcgagttagtattatggagatcttttgatttcatatgcctttaatcaaacaatcattataaaccactgatatccagcttttatcgttttatgaaggtcttgacctacttgatgtacctcatgcgtgtgggagaaaaagctgttcaaagacaagttgctttggctcttgctcatctgtgttctccagatgaccagagatcgattttcattgataacaatggcatgtcttatatctatggctttatggtctttgtattatttctattgcgttgatatttattttttgacattgttgacatcatggtctaattgttttggctaggattggaattacttcttgggcttctcaagtccactagtgctaagcaacaacatgatggtgctgtgggcctctgtaagttggctagcaaagctatgactctttcccctatcgatgcagctcctccttctcccatatcacaggtaagctttgtctgatttgatgctccatgtaccttgctgattgaatattgtacagccgacagcagcactttgctttgcttatataattgttttaagctttattagtaaactgctgttcaagggcagcaccccaagatcttactgttggtgctgcttgtggatgttaggtggagacagtctaattttaaaggactgttctagacttgtactcagggaaaaaaaacgcgttcgcggtcgcgggaacggcttgtactgggaaatagaacgtttcgcggccgacacggcgtgatttttttttttttaaattcacattaatatattctaaccttatttgcatttttttttgtttatgaagcattattacaacataatatactcaaatctaatagaatatcatgtttcctcaactatataactaaatcataaaaaaaatttggccaatgtttgaaaagaacggatgtaacggggataaaagcgttctaacgcggcgagttcgcgttacggaatggacaatgcggggagaagtatgtgaatttaattatggcgtcccgtaacgagatttcgcggaacggcaaatccaaaatccgttacagaacgaccgttctgtaacggaatgggagagttttaattccctgcttgtacttagttgatctgatcaaagaaagttcagtaacatgtctcaggaccgcggcaatgggaactggacttctgttttccatttgaatcaagagatttttgaagataactagataagacagaagtattggtttctctgcacagtactcctgtcatgtcctgatttacttctttttgctttgtactaactccgttttcctaagttctactcacttttattttacacggtcgccaatgcactcctttgacgattaatgtctttcatgacattgttaaaaattatgaaaaattgatattatatacacatcgagacgaactttgaaaatcctacatgataatatttttcatataaataaataaaaaaagatggtcaaagttttgtaagtttgaccacttgaaaagtaaataggtagaacgtaggaaatagagggagtataaaattgtgaattgacttcaattttgtgattaagttacccttacttaagtgaactttttccttagtgtgaatctatattctcaaaagctactcatttaattattttccatctaacaagctagattaataagcatgtattttcctgttgtcaacatccttaatatagaacacttcttatatgagaacgtgagaacggtggaatagtattacactttagtaaaagtataatcctttattaagataatacatggtattttcttgaaaatgtaatcctgaggaagattggccccgcaagggaaaatatgattccattttagccaaaatggattacttgttggctaaaaaggattactacttagtgttctcactttctcattaagtagtgttcttaccaaatcccaaccctatatatattgatcatccgtataagggctatatttatacgcaaatatgtatgcgagtatgtacatccattatcctgtgcactatttaaagagttgcacgtttagctgaaaatagctcacacaaccccgtactttctctacaggcgcagacacacgctaagatttatgtataaatgtatatatgtatatatgtacatgtaattctgtttggcccattttgtaatgatatattggtggactagaagcaacgtctttgatatggtaggtggtagtttttaggaaggcttcgggtagaataaatgttaatgactttgtgttctattactatatgaagttcgtcttgcaagtttattactttgcggtttgggaatctcatcaatattatttaatctttgcaggtttacttaggcgaacagtatgtgaatagtccgacgctctccgatgttacctttctagttcaaggttccacatgtgtcaccaatcattgcttgttttgatacttctattatttgcttgtgctgaactaccaagctgattatctgagcatattgctcaagttctaaaaatcatgcgacttccgttttgaattgtgtgcttatgcctcacatttcaggcaaacggttcttcgctcatcgaatctgccttcttgcatcatctgatgctttccgcgcaatgtttgatggtggttatcgggtgagtttttcttgtctaattatatgagttagacctgaggtcttccatcttctattatttattatctttgggtaacataagattaaggtttccgcctctatattgttatgaagagctggaaatatgctcaagggaaataatgtacatttatttttcaattttattattaggaaacccttgaaatgtgctgtgagcagtacatggcaggttgccttaccatatatgttattaagatatgtacgacgttgggagagggatgggggaaagggcaacattgatagaaaagggtgaattgctggcatcaaggtcactgaaactttatggcatagggatcaatttgctatgaaatgacatgcatcatacaccatttgatgttctcgcaaggaactttagcttctatgtagtccttatgatcatcaataaatatggaaaaactattcattgagcttcaagctttggatttatgactgacgtttcttttttgtacggtctactatgctctctttttactgtttggaacttttgctcataagatttttgctgatatcttgatgatacaggaaaaggatgccagagatattgaaattcctaacatcaaatgggatatttttgaattaatgatgaggttattttaatatgtacttttgtggcatttcttaagatgatatgtgaataagaaatagaattgacgtggctgtctttgtcactctgttgcagatttatatatactggatcagtagacataaaaccagatattgcacaagatctcctcagggctgcagatcagtatcttttagaggggctaaaacgcctatgcgagtataccatagcccaggtgagctgaactaagaactgctcatttcttgggtatatctgtttctgttgaatggaggatggcatatatttatgttttggtttcctgatatatgaaggatgtatccctggaaaatgtgtcaagcatgtatgagctttctgaggcattccatgctgtttcattgaggcaggcttgcatacttttcatcttggagcagtatgataaattgactgctaggcccgggtatgcagtttctccaatctctttttggtagtcttatcagttttccttctattctgtgagcagactatggaaactacagtattaatgcagctgaaaaaaattggtgaagttattaggtttttatgttctgcaatatctgcctgttgcactaagtattggtaaatggtcattgtcaaattaatcttgttcctactgtacatacatgttgatacttgcaagacactgcctgttatatttttttgttttgttttttcgttttgaattagcatttatgatacttttcttggttagttactactctttctttgactctgtcccataataaagttccccttttttttttataatatttaaagtccaattgtaaagttcctgccagtcactcacacacaagcaagaataatgatagagaagatagcagtgttgtgatagacgcaatcaacgaaacaaataacaagtgaacaatcaacacaagaattaacgtggttcaccaacaatgtgttagctgcgtcgagaggcagagagaaacaattttattaggtttaggagagagtacaaattacaaaatgatgccggaataacatataccggaaagttcgggggcgtcaatcctagcgccagattaataattcaaggcataattcaaagtagcctggagctttcaagaggctcaatgtctcccaatacaaactacaacagatcaagcaatatcctgccttctttcgattcacccttcccctttatgtacaaaatatctctctctagccaaatattccctttttctaaccaaacttctgattacatgtacatgagccactacctgaccccagcaagaccataacttattgctttccccttggctgatttaccccttactagccttgtgtttctggtgacccgccctttttcttgcgacgagtataagtcagcatatgtggagggttgtgattcattacacaaagctcataatttttaccgttaattatcaccaatatataagaagtaatatagttatgtggggtattgttagatttgtctcaatatggacattcatatcatctactttttatatattttattggtgtgtaattaaagttgttcctgggtggaaatgcatggaactcgccgataagaatccttcgcctgtagccaagataatctgcaatgcagtaaacgtgaactgcccgcaggttgattgttaggaaacccctcgaatgcataaattagagatttaaatgggatgagatgtagagaaagattctagtgagagaaatataagaatagaacaaaaagtactaaatgtcggagtgtccctttaccaagtatgcccctggtattttgaagttgatggttccattagatgactccatgtgtatgttacagatgcaaggcatctcttgccagctattaaggcttttcatgtttcaccggcaaggttatgaggattgttgaccgcccaactacattttgttccagtatcgatatctgtgattgttttcttcctggctatatttctagctgtgttgaattattcttatcgtgtacagaagttttaaaagtcaaagaagtgtctcagagactctgcgtaagcaaatgagaactttaaatggaacagagggagtacctttttaaatcaaaatattagcctaagtggatatttgattgatcgtcattttgtcaatcacggatgaaattgaaatgtttgatgctctcattaggcaacttggaatttaaacaattgagggtcaaacattttagcttgaggagtgttacaataatattgtcataaaaggttgactgtccctgaggtattaacttgcaataagtgatatttgaaagaacttgcaataagtgatatttgaaagatagctgctaactcttgccaaagaaaaagaatgtagttggcaattatccgagcagaaaataatttttttgaagtttcttacctttgtttgcagaagtgaagctaggatttttcgattaagggaccaatacttacataaaagtatatagaaccagagagggtttacatcatcgagctcccattattcatattttttttttgaaaaattaagtgtttttttatcatcatttaaccagccaattccccaacataagaaaattatagttattatatgtgcagtataatgagtacttgatccatgtgagaatggctcgtttcctacaagtcctagttcttttaggactcctttacttcgtctcctagttctgttgggattttaggaaggctatgtaaattaggtttttttttatagttaaattagaagtctcgtgcatgtaagtctttactattctacttagaataggtttttcttactttaagcaccttgggagtctaattacactaagagaataaagcataataggcgtgtgactagtattgcttgccccccaaggtaaatttaaggtgtgttctcttcacctcaaaaagtaattttcaggtccaataagttcagatgaggtttaatcaagtttgattaggtgtaatacaatactaaaaaataagtttcaataagggtaaatcaggtttaataagttcataagttcaggttatttcaggtaaagagaactcacccttagttagagcagatacaagtttgttatttcatgttatctttgtaattagtttcctaagtctagcctaattagttttgtatgcctacataaggccacgattctcattaataatataggttgatctgagttaaagaaattgcctttgttaagtgtgtgaattgtaaatttcaactgcataacacttcactttcatgctctcttgaagcttagacttacaagaaaccctcttaaaccgcgatttgagagatatattttattaagatgcaaaagaattgatatgtggaaaggtactttcaacaatcattgattatatattcatataactacaattgagtaaaaagaaattaagaacatacaacagcaactgacctttttgatgtgtttcggtgtataatgggaagtgctcccagaatgaagtaatttcattgctgaagaaaattgaaaactaggggaagaaagaaaaaaagaaaaacaaaggctgaaggcaatgaaaaaggcaaatgatgaggaaaccagttgttcaatgaaccaatcaaactctgacctttgcttgcaatagaccaaaaggcacgatcgtaattgacaccaaaaccaagtaaacctttcatgtttatttagtaaacaatcaattatgtgaactttcatgttcattcagtgaacaagcaattatgtattactattatccagctttatgacagaatgggcttcaaagctgggctatgggggctaggcatccccagccccctcatggtgccaaccctgtttgtccgattggaggagtttctgattctttactatcctaccaaaatatcaaatcagttagttttataaggcaatacaaatgcacttttttccaaaggagatttagtttgaataatagatctacttttgtttctctggcaaatgttactgtaaggggtttgttgttatgcaagtcttcaattctaatggagctaccatatgcttgtggtctcttctgctatttaacattttcttgtggcttatataggtgtaatagtgcttgtatgaaaaataaaaaatacatgaaatgaactttagttagattttatctgctcctgaccttttccactgtggaactgtgcaggcattcatctcttttgcagcatatattgccagaaattagaaattactttctcaggttacttaccaagcctaatgctctaaattagcgacttaagctgccaattttatctcgtttctagaaatggtatggttgaagctttaagtcaccgacaagcctggctttcatctctccattacgtgatctcaagttgtctcttacggcttgcatatctaactttcaccaatatctgtcatttggctgcttgatgactctaagccacctttaattccaatctttaacgttttgttctcatgagagcaatactggtggtttttatagcaagtcctgtgcgaatttctaacaaagcactgaaatactagactgacaacttctggaagcagttatgagttgtgcatcaatcacatgtgaagtctgatctggtatgcgagtagcagttttaggtagtatttcgggttcttgcagctgcattaggctcatacctatctcactgttaaagcatatatatatgtgaccttcatagcctaaggtcatttttcacggttgagtttggaatgtgtacgaggtcaaatggcacaaattataggatgctaaatggctaggtgttgtgtttgcttcacagagaagctggaagagttgtaccatgcaaagaatagtatatcgcttttgtctctattttctgttaccttacgctactactaactctgcaaaagtgtaattatgttgtcacgactttacaagcaggtgatatgaggtgtatttgtgtaatcagtaatcaatatattgacagtttcaactaatgacattgtcgtggtcctaaatgttttccccatatgtttttctagaagtt

SEQ ID NO: 251 - protein, 744 aa, Beta vulgaris
MDLGERRSGGTARRSLKRKLEEDFHGNHKIKLDLPQNRHHHHNHQDLLSEINSYVQILFRCFSWCDSDRIDSKRASHFLSELAKNEEMVNLIVECGAVPALVMQLQSPPSEDGGVSKPLEHEVEKGSAFALGLLAVKPEHQQLIVDAGALPHLVALLKRHRSGDISRSVHGVVRRAADAITNLAHENSSIKSLVRVEGGIPPLVELLESTDVKVQRAAAGALRTLAFKNDENKNQIVECNALPTLILMLRSEDPAIHYEAVSVFTAHWNTLQNYMADAIINCYQLFIWVMCQSLQVGVIGNLVHSSPNIKKEVLLAGAVQPVIGLLSSCCSESQREAALLLGQFASADSDSKVHIVQRGAVPPLIEMLQLPDAQLREMSAFALGRLAQDSHNQAGIVQCGGITPLLTLLESKNGPLQHNAAFALYGLADNEDNVADLIKIGGVEKLQEGDFIVQPTKDCVGKTLKRLEEKIQGRVLNHLLYLLRVADKVVQRRIALALAHLCSPEHQRRIFIDNNGLELLLELLESSCIKQQQDGSMALYKMASKTTLLSPADAAPPSPTPQVYLGEQYVNNSTLSDVTFLVEGRRFYAHRICLLASSDAFRAMFDGGYREKDAKDIEIPNIRWNVFELMMRYIYTGSVNVNLDIAQDLLRAADQYLLDGLKRLCEYAIAQDISVENVMLMYDLSEAYNATSLRHSCILYILEQFDGLSSKPWYPRLIQRIVPEIRAFFERVLTKPSFVELTQA

SEQ ID NO: 252 - protein, 714 aa, Beta vulgaris
MGSKEWQGKENSSDRKGQKRKLEQQSEERESAIVTGEALQREVTTQVDILKANYSWTEADRAAAKRATHLLAELAKNEEVVSVIVEGGAVPMLVKHLSAPPSMVEDDGVKPYEHEVEKASAFALGLLAVKPEHQQLIVDAGALPLLVDLLKRHTSGLNSRAVNGVIRRAADAITNLAHENSSIKTRVRTEGGIPPLVELLGFNDAKVQRAVAGALRTLAFKNDENKKQIVECNALPALILMLKSEDAAIHYEAVGVLGNLVHSSPNIKKDVLLAGALQPVIGLLSSCCSESQREAALLLGQFAATDSDCKVHIVQRGAVPPLIEMLQSPDLQLREMSAFALGRLAQESHNQAGISHSGGLVPLLKLLDAKNGSLQHNAAFALYGLADNEDNVADFIKVGGLQKLQEGEFIVQATKDCVAKTLKRLEEKIHGRVLTYLMYLMRVGEKAVQRQVALALAHLCSPDDQRSIFIDNNGMSYIYGFMVFVLFLLRLELLLGLLKSTSAKQQHDGAVGLCKLASKAMTLSPIDAAPPSPISQVYLGEQYVNSPTLSDVTFLVQGKRFFAHRICLLASSDAFRAMFDGGYREKDARDIEIPNIKWDIFELMMRFIYTGSVDIKPDIAQDLLRAADQYLLEGLKRLCEYTIAQDVSLENVSSMYELSEAFHAVSLRQACILFILEQYDKLTARPGHSSLLQHILPEIRNYFLRLLTKPNALN

SEQ ID NO: 253 - DNA, 3862 bp, Brassica napus
  source 1..3862: mol_type = genomic DNA
atgaaaatctccaaatcgctcaaactccaccgctccaatccaccgtcgaatctcctcctcgtccgtcgtccgtcatcgatctcaaaccttccacctatggagaacaatcttaagcgccagcgaacaacacgcgtcgccggaagaagctccaagcgcggccgggagacgtacgcggtttcgataatcactcagatcaccgagatcgaggaagaagaaacagatctcgtcgtcgcgatcagccgccacgtggatgttcttaactccagcttctcagatgcgggagatgtcaaaggagctgctgctgctctctcctccctcgctaaaactggtaccgtaactgtttgaatcgatgcagatctgtgattctacttagcgattgatttgttctagctcagattaggcgagatctagattgtttttttgattcgtaactgtttgtattagacgaaaacgtggagatgatggtggagaacggagcgattcccgctttggttagaaacttggaatcgccatggtctttagcaatcagcgggaacgttgccaagtcttgtgatcataagctggagaaagattgtgctgtttcacttggactcattgctgctaatcaggtaacacttgtgaatatcatttactgcttcttgcactgatgttttttactaacgttagctttatctgttaaatagcctgcttaccagcagctaattgtagatgctggggttatagctccgactgtgaagttgttgaagagaagaggggtttgtattgggtgcatggaagctaatgctgttcttaggagagcagctgatatcatcactaatattgctcatgataatccaaggattaaaactaatataaggtacggtttagtgtttgatgatccttatgctttttttggtcttggctataagttgttttcacttgacagggttgaaggtggtattccaccgcttgttgagcttttggattttccggatgttaaagtacagagggctgctgcaggtgccttgcgtacagtttcttttagaaatgatgagaacaagaaccaagtatgttttgcttttgatgatgctttgtttgagcttatgagaggcatgtttcttacataaaaaaacatttgtgtagattgtggagttgaacgctttgcccacgcttgtattgatgcttcagtcagaagatccttctgtgcatggcgaatcggttggttcttttatcttgctttggatttttggaattggtttgctatgtttagttccttctaatatactattgaaatatcagattggggcaattggaaatcttgtccactcatctcctgacatcaagaaagatgttatccgcgctggtgccttgcaaccagtaatcggtctacttaggtatgcttattttctttattctgtttttctacttctgctgaaaatagatgtttactcttgatgttgtgaaacatcttttgtaactgtttctgcttgctatgatatctgctacagctcaccttgcttggagacacagagagaagcagcattgttaattggtcaatttgctgcgcctgattcagactgcaaggtataagtttgtctctttcttgacattgttgtgctctaatctgaatatatgctcactcaaactcttttgttttgacgatatcaaaaggatggattcagagtaaagaaaacgtactaaaacataaatggcaatatgattatgcaggtgcacattgcccagagaggtgccattacaccattaattaagatgcttgagtcatcagatgagcaggtcacggaaatggcagcgtttgctcttggtcgtttggcccaggtagttatgtttttgaataagcatgtgaatctttttgacgctttgtgtcataagaacaatggttgtaatttgtttgcttagagcataacttaattcgcatatatcaatgctttgaatgtcgcaggacacacacaatcaggctgggattgggcaaagaggaggcattatttcactattaaatcttcttgatgtgaaaactggatctgtgcaacacaacgctgcctttgctttgtatggccttgcagataatgaggtaaactaatctcataatgaatcgttttcaatacatctacactttttgctaactataaataacaatggttaattaatttttcgtaaacaggaaaatgtagcagatttcataaagactggaggtattcaaaagcttcaagacgacaacttcaccgttcaagtatgcatttcgctgcttatgtttgcaaaaacaatattataggctttccaaattctaaattgcaagtcttctctttgcagccgactagggactgtgttgtgaggacattgaagaggctagagaacaagattcatggacctgtgagtacctatctgttagaccgtctggttcttataagtatggccttggttctagagtcccttaatgtcatactcttctttcaggtactaaaccaactattatatctaatgaaaaccactgagaagaatatacaaatgcgaattgctttggctcttgcacatctttgtgaccctaaagatggaaaattaattttcatcgataacagtggtaatattctcatctcaaaattcatcagtttttcttttcttgtcgatttttttctgttcctgatcaatcgactattatttatgctatgttatacaggaatggagtttttgttggagcctctatacatctcaagcatgaaacagcagaagtatagcgcaagagctttattcgaattagctacaaaagctacatcctttgcaccagaggactcagctccttcctcacccacacagcgggtaagaaattttcattacttctttcaattataaaaatataatttctgatttgaggtcttgacttgttattggctgtaatactgaaggcgtttttgggtgaggaattcgtgaacaaccctactttgtccgatgtcacattcctgatcgatggtaaaacatttaatcccttctatgtttatgttaaatctacctgtgatcacactttttactgagtgtttgcatggcatatattaggtaaacaattctttgctcacaagatttgcttggtagcttcctctgatatatttcgtgcaatgtttgatggcctttacaaggtaaccttcttaataaattattgtgctacccatttcatgatacaaagtatcaatcaactaacttgagaattggttttaggaacgcaacgcccaaaatgtggagatcccaaatataagctgggaagtgtttgagcttatgatgaggtaaagttctataaaatcaaacattttgaatacttaccattataataagctaagaatctaaagcataaaatgcaatggtgcagattcatatacacaggaaaaatcaacatcacaaaatacttggctcaagatctgcttgtagcagctgatcagtatcttctcgaaggtctcaagcggctttgtgagtacacaatcgcgcaggtaaatacacaaaaccaacttcttattcttctccttgtcagagtggcttgtctatgtgtataactaaatggactcctctaatgttggtgcaggacatttgtgtggaaaacataccgttcatgtacgacttagcagatacattcaatgcgtcagccttaagacgagcatgcactctcttcgttcttgagcattacactaagctcagctctgaactgtggtatgcaaaaaatcattacatcatttatacaatgaaataacttttcttttacttaatcaggttttatgttcttattttcttacgcaggtttcccatgttcataaagaaaataataccagaaatccggagctacatcactgatattctcagacggccagtccaagctagcagctag

SEQ ID NO: 254 - protein, 706 aa, Glycine max
MELQRRPDQCLPVRKGLKRKLEEEFDDDPQISAPPTGDARDALLSDVKEQVSLLDSNFSWNEHDRAAAKRATHALADLAKNEEVVNVIVEGGAIPALVKHLQAPPLAESDRLPRPMPFEHEVEKGSAFALGLLAVKPEHQQLIVDSGALKHLVDLLKRHKNGLTSRAINSLIRRAADAITNLAHENSSIKTRVRKEGGIPPLVHLLEFADTKVQRAAAGALRTLAFKNDENKNQIVECNALPTLILMLRSEDAAIHYEAVGVIGNLVHSSPDIKKEVLLAGALQPVIGLLSSCCSESQREAALLLGQFAATDSDCKVHIVQRGAVRPLIEMLQSSDVQLKEMSAFALGRLAQDTHNQAGIVHNGGLMPLLKLLDSKNGSLQHNAAFALYGLADNEDNVSDFIRVGGIQRLQDGEFIVQATKDCVAKTLKRLEEKIHGRVLNHLLYLMRVSEKAFQRRVALTLAHLCSADDQRKIFIDYNGLELLMGLLGSYNPKQQLDGAVALCKLANKAMTLSPVDAAPPSPTPQVYLGEQYVNNATLSDVTFLVEGKRFYAHRICLLASSDAFRAMFDGGYREKEARDIEIPNIRWEVFELMMRFIYTGSVDITLDIAQDLLRAADQYLLEGLKRLCEYTIAQDISLENVSSMYELSEAFNAISLRHTCILFILEHYDKLGGKPGHSQLIQHIIPEIQNYFVKAITKANSNIQP

SEQ ID NO: 255 - DNA, 72 bp, synthetic construct
  source 1..72: mol_type = other DNA
atatatggtctctggcgacctggggggatcagccggaagttttagagctagaaatagcaagttaaaataagg

SEQ ID NO: 256 - DNA, 52 bp, synthetic construct
  source 1..52: mol_type = other DNA
ttattggtctctaaactccgcttctcggataggttatgcttcttggtgccgc

SEQ ID NO: 257 - DNA, 20 bp, synthetic construct
  source 1..20: mol_type = other DNA
ggcccagagccacaagataa

SEQ ID NO: 258 - DNA, 20 bp, synthetic construct
  source 1..20: mol_type = other DNA
gcttgtggaccgaaacgaag

SEQ ID NO: 259 - DNA, 20 bp, synthetic construct
  source 1..20: mol_type = other DNA
catcctcgtcactcgctaac

SEQ ID NO: 260 - DNA, 25 bp, synthetic construct
  source 1..25: mol_type = other DNA
acatgaacgcgtactctttattatc

SEQ ID NO: 261 - DNA, 20 bp, synthetic construct
  source 1..20: mol_type = other DNA
cgagatggcgaaggttgacg

SEQ ID NO: 262 - DNA, 20 bp, synthetic construct
  source 1..20: mol_type = other DNA
aatgtccgctgcttcctcag

SEQ ID NO: 263 - protein, 125 aa, unidentified
  VARIANT 3: note = X is E or D
  VARIANT 4: note = X is K or R
  VARIANT 6: note = X is K or Q
  VARIANT 15: note = X is I, S, M, L or V
  VARIANT 16: note = X is T, S, or deleted
  VARIANT 17: note = X is N or deleted
  VARIANT 18: note = X is L, I, A or deleted
  VARIANT 19: note = X is N, Y or T
  VARIANT 21: note = X is K, R or S
  VARIANT 23: note = X is P, G, S, T or deleted
  VARIANT 24: note = X is T or deleted
  VARIANT 25: note = X is T or deleted
  VARIANT 26: note = X is A, S, G, P, L or D
  VARIANT 28: note = X is D or E
  VARIANT 29: note = X is S, M or T
  VARIANT 37: note = X is E or D
  VARIANT 38: note = X is T, P, A or S
  VARIANT 39: note = X is A or T
  VARIANT 40: note = X is N, S, C or T
  VARIANT 43: note = X is K or R
  VARIANT 47: note = X is I, V or A
  VARIANT 50: note = X is K or R
  VARIANT 56: note = X is V or I
  VARIANT 67: note = X is V, I or L
  VARIANT 68: note = X is Q or L
  VARIANT 75: note = X is R or K
  VARIANT 78: note = X is D, N or G
  VARIANT 82: note = X is E or G
  VARIANT 86: note = X is E, D or A
  VARIANT 88: note = X is S or A
  VARIANT 89: note = X is R, H or Q
  VARIANT 90: note = X is V or C
  VARIANT 93: note = X is L or H
  VARIANT 96: note = X is L, K, V or I
  VARIANT 99: note = X is L, A or T
  VARIANT 100: note = X is Q, D or E
  VARIANT 103: note = X is S, K or R
  VARIANT 106: note = X is T, A, S, V or T
  VARIANT 107: note = X is E, D or N
  VARIANT 108: note = X is I, A or V
  VARIANT 110: note = X is R or K
  VARIANT 111: note = X is E or Q
  VARIANT 113: note = X is T, S, A or L
  VARIANT 116: note = X is K, H or Q
  VARIANT 117: note = X is E, D, N or S
  VARIANT 119: note = X is V, L or I
  VARIANT 120: note = X is D, N, T, S
  VARIANT 121: note = X is M or V
  VARIANT 123: note = X is M or V
  VARIANT 124: note = X is N, S or D
  VARIANT 125: note = X is M or V
LSXXRXALFEPLEPXXXXXGXRXXXXAXXLLPPPDFXXXXYPXGWLXGKXRKLVNXDVVESMRRIAXXEMNRKDXEIXGLNXQLEXDXXXLEXLQXQLXXERXKRXXXEXXNXMLXXQXXMLXXM